European Patent Application EP 4 141 103 A1 - sequence listing, part 3

SEQ ID NO: 10 - DNA, 294049 bp, Chitinophaga pinensis
  source 1..294049: mol_type = genomic DNA
acttctggaatcatggctgggccggggtgctcaggggggccggggtggtattctttgctttcattggttttgatgcggtatctactgctgcacaggaaaccaagaatcctaaaaagaatatgccgatcggtattcttgtatcgctggctgtttgtaccttattatatatcctgttttcttttgtgctcacaggtattgcaccgttcaccgacttcctgaaagcaggtggtgaagcttctgtagcttatgcgattgatacttatatgcctggttattcctggttgtcgactttcatcaccgtggccatcctggcgggattttcctccgttatcctggtgatgttactgggtcagacaagggtattttactctatgagtaacgatggactggtaccggccgtatttgcgaaactgcatccaaaataccgtacaccttaccgctcacagtggatgttctttgtttttgtatccctgtttgctgcgttcattccggacaatgtggtgggtgatatgaccagtatcggtaccctgtttgcctttgtgctggtgtgtattggtattattgtaatgcgcaaaaccaacccggaactgccacgcgcctttaaaacgccgtgggtgccatttgttcccttgctgggagcggctttctgtcttactatgatcatcagcctgggtattgaaaactgggcgcgtttatttgtgtggctggctattggctttgtggtttacttcggctatagtgtaaaacacagtaaggcccgtaaaatgctggaatagtttacggagattaacatttccggatatcatacgaagcggagaacagaacaaaggggattacccttgttttgttctccgctttagttaaaatcaggggaatccgctattctggtacctgaaaatccttatttttgcgttctgtttttaaaagtcataataaatatataccactccaatgggaagaatatttgaagtaagaaaatcgaccatgtttgcccgctgggataagatggcgaaagcattttcaagaataggtaaggaaatagccatcgccgtgaaggcctctggtcctgatccggataataaccccgcacttcgtcgctgtattctcaatgcgaagagtgttaacatgcctaaagaccgtgtagacgcagctatcaagcgtgctatgggtaaagacaaaaccgattatgaggaagtggtgtatgaaggctatgctccccatggcgtggcagtgatgattgataccgctactgataatactacccgtaccgtggccaacctgcgtatgcactttaccaaaggtggcggcagcttaggcaacagcggctctgttggatttttatttaaccgcgtaggcgaattcaaaataaagaatgccggccaggacctggaagaactggaactggaactgattgattttggtttggaagaagtgggagaagatagtgagggcaacatcattatccgtgctgcattcaccgagtttggcaacatggccaaagcgctggaagaaaaaggactggaagtgatcagctccgagctgaaacgtattccgactactaccgtggagctgaatgacgagcaggcaaaagaagtgctggaactggtagaccgtttggagcaggatgaagatgtgcagcaggttttccacaatctgaaataggatattaatacatataaaaaaggaaacgtccgccattacggtggacgttttccattggatacggttaactttccagaaccaaaaaacagctaaactttagcgatggtgtgtgtgcgccccaggtcatcagcgatgaacatgagtcccttgccgtggtaggtttcgagttttacggcagggtcctgcgcaatgtgtttacgaagacgggtcagataaacgtccatcacacgtgaagcgaagaagtcttcctgtccccagataacagacaggatatcatctttcttcagttttttgttagaattttcgcacagaaagcgaagcaactccgcttcttttggggccatacgaacatgggagtcggcatctttatgccggatatgatattgtgaataatcgaagatcaggttactgatagtatataccacgcggcgctcacttttcagcaggcggctgcgtttcaggtatacttccacgcgacagatcatttcctgcatattgaagggcttggtgatatagtcatccgcgcctgcttcaaatccctgcagcctgtcctgttccatataacgggatgaagtaaaaatgatgggaatgttttcatccattgaccggatatctcctgcaagggcgaaaccatcttttttaggcatcaccacatccagtatgcacaggtcaaacacatgtttctggaatttttcccaaccttcctggccgttttcacagaagtttacgttgtaaccggcgcgttccaggtgtctttttaccactttggcaaaaaatacatcgtcctctaccaaaagaatgcttgattgcatgtaacgttggttttaagcgaataaatagattttagttgtatgcgtaccttttaaataagtgtagcaggtacctttatccaaaaataaataacataatcataaccctggccatccatcccattcacttctgaaggcatcattcatttcaaccattcagttacgcggtataccccaaagcctattattttctgtttgcatgctacttactaataacctgtttattcgcttaacgggtaatcctaattgataatatttttaggatttccttcgaggaaggcttttacgttttccaccgatgtatacatgagtcgtttccgggccgcctgggtagcccaggcaatatgtggtgtaataatggtattaggcgcagtgatcagtggattccccgcaggcggcggctctgcagataatacatccagcgcggcaccggcaataattcctttctccagggcatccgccagatcggcttcacagatcaacgggccacgactggtatttacgaggaaggcgttctttttcatggtacgcagcagggcggcatttacaaactctttattggcagcattcagcgggcaatgcaacgagataatatccgcctcccggaagcaggtagcctggtccacaaaagtaacaccgggcatcccgtcccggtcaggatgtttatggtgggcaatcaccttcatcccaaatgccaacgcaatacgggccaccgcctgccctatctgcccgagacctactatgcccaacgtattgcccgccagctccgtgagcggcgttttccagtaactgaaatcgatgctgctgctccactcccctgcccgcacacttacagcatgcaaaccggtatgatgacataattcaaggatcagtgcaaaagtcagctgcgcaacagatgccgtgctgtaggcaggtacattcgttaccgggatatgccggcttcttgctgcatgcgtatccactatgttgaatcccgtagccgtcacgcctatatattccaggtgttccagctgccggatggtttccccgcttacaatagccttattggttaatatgatatgtgcatcctttgatctggcagccacttcatgttcgggtgtacggtcatacaatgtaacgttgcccaatgcctgtaacccgctccagtcgaggtcgccggggtttaacgtatgcccgtcgagtactacgatgtttttcatggtcttcgttttgccgacaagatacatcatacatgaaataatcattaactcacctgtaaacactttatacattcaaaatatccctgacctttgctgcgccataataagccaatactgctaagcctgcaaactgcttaatgtaagaagccaccatatcagcagattgatgctgttatagtggcttcgccaattaaaggaaaagccggctcctgttaaggcaaccggcttttgtatgattttgaaatgcaactattcctgcatcatctccataattacttttactacatcttctgtattgggcttggagaaataatccccgtcggagccatacgccgggcgatgggcttgcgcactcatggtgcgtggcgatacatccagccagcggtagccgccttgtttttcaattacctgctggaacatgtaagcagttccgccaccgggtacgtcttcatctataaagaggatgcggttggttttctgcaatgattccacaatactgtgatggatgtcgaaaggcagtaaagtctgcacatcgatcagctcacaggagatgcctgtttccgccagcgtcaccattgcttcttccacgatacgcgtcatagaaccatacgtaacaatcgttacgtctgttccttcatgcagtatttccgggatgcccaggggtacggtatacgtttccaggttggccggtaatttttctttcagacggtagccgtttaaagattctatcaccagggccggttcgttggcctgtaacagtgtgttatacatgcctgctgcctgtaccatattacgtggtacgcatacgtgcatgccgcgcagggaattgatgatcatgcccattggagatccgctgtgccagatgccttccaggcgatggccgcgggtacgtactatcagcgggcaatgcataattcctttggtgcggtattgcagggaggccacatcatcgctgagtggctgcaggccgtagaggagatagtcgaggtactggatttcagcaatggggcgcaggccgcgcaatgccagtcctattccctgccccatgatagtcaactcccggataccggtatcggctatacgtactttaccatgtttctgctgtaatccggcaaagccctggtttacgtcgccaatctttcctacatcttccccgaaagcaaatacgcggtcgttgttggtaaacagctgatcaaaatatttattcagtatttcgtacccgtttacggtgatgctgtctgcttcgtatgcggccggaactaccggtacattcagggcagagtttacgccggtggcgtgaagcagtgtattgtacacttctttttcgccggccaggtaggtatcataatattgctgcaatgcctgtacggcggcatctgatttcaggtgccggtgtttcaggagaatcatggcgctggccttcagaatatcgcggcggagcggctcgcggttattctgcaggtcgcggatgaaggtgtttatcatgtttgcatcggcgcctgcaatagcagctaccggtgcggccagtgcggtaaacgactgtacctgttccttgatcggtgatatatatttttcccaggcagctttccgggcgtgctgtgcttttacttttgcttctgcttcaacggcgcgcagggtttcttcctcgcacaaagcattttcaatgatccaggaacgcatttttacgttacagtcgaactcccgttcccaggaaagacgttccttgcttttataccgttcgtgcgaaccactggtagagtggccctgtggttgggtgatttcttccacatgaaacagtgcagggatgtgtgtttcgcggatcttgcggatagccgcttcgaacacttcacacatgccggcataatcccagccttttacattatatatgtcaaagccattggattcttccgttttgcggaagccttccagtgcggcgctgatagaccctttggtagtctgatatttacggggtacggaaataccatagccatcgtcccatacaaatacggccagtggcacctgtaaaacaccggcggcattcatggtttcccagaaatgaccttccgacgtagaggcgtcaccgatagtagcgaaacagatttcgttaccgttgttggaaagatttttatattgacgcaaggcttccacctcacgaaacattttagaggcataggcaaggcccagtgcgcggggcatttgcccggcggtaggcgccatgtcggcagcagagtttttcatctgcgtcagattgagccagttgccatcctgatcaagattaggagtggcataatgggagttcatctgcctgccgcctgaaaaaggatcattttccaggtcgggatctgcatataactgcgaaaagaattgttcgggagtggcgataccagtggcaaatgcaacagtttggtcgcggtaataaccggaacggaagtcccctggctgaaagtattttgacattgctatctgcgccacttcttttccatctccaaaaatgccaaactttgccttgcctgtaagcacttccttacgggccagcagactaacttccctgctttcgcaggccaacctgtaatcattaagcacttccttgcggaactcttcgaatgataaccggctttctaaattcatagctagttcgttattttctatcatgcctcatggttaaagtacaaaagtaaggttaattatacagttgaaaaatgctgtgaatctttcatttaaaataatctgattttttttaataagattttaataaattgtaaggtttataatgctttttggctgtaaatttgttctaaccaagaaagatatcaatattttttaaccggtcgctttaaaaccatcatatgaaaatgaaaaaatttatcttatccctgtttgcgagcatgctgctgactacagcgctgtgggcccagaccgctccagcacagaatccggcagatacaaaagtaaaatttgccaaagaaactgttgattttggtaaaactgaattaaacaagccagttactgttgatttcgaattcactaacatttccaaagaaccggtgttgattgaagctgcccgcgctagctgcggctgtactacgcctaagtggacgcaggagcctattttacctggtaaaaagggtaaagtaaccgcgagctacagtgcaaacggtttaggtcagcagaataaaaccatctgggtaaagttcagaggcgtggatcaggacaaggaactgcacttaacaggtacagttggttccaacaacaagtaactccacactttaaaacatactaagaccttacagcacatgctgtaaggtttttttgttgcccatcgtatcccctatctttgcaatgcaaaagtcaaaacaattttatgcctaccattagccagagaggtgagcaaatgccatcttctcccattagaaagcttgtaccattcgccgaagcagccaagaaaaaaggggtgaaagtataccacctgaacatcgggcaaccagacatcgaaacaccaaaacccgtactggatgcggttcgccattcagaattcaagatcctggaatacagccacagcgcaggtttcgaaagttaccgccgtaagctggtcacttattacgaccggtttaacattgctgtgaaccacaaccagatcattgttaccaccggcggttcagaggcgatcatatttgccttcatggcctgcctggatccgggagatgaagtaattgttccggaacctttttacgctaactacaacggttttgccgtagaagcggaaataaagatcaaaaccataacggccagcatcgaaaccggctttgctttgccggcaatggccgattttgaaaaggcgattactccgcgcaccaaagctatcatgatctgtaatcccaataaccccaccggttatctttacagcagggaagagatggaggtgttgaaacagctttgcctgaaatacaacctgttcctcttctctgatgaggcttaccgggagttttgttatacaggagcgcatttttccgctatgaacctggaaggcatggaaaataatgtgatcctgctggatactatttctaaaagatacagtgcctgcggaggccgtatcggtgcttttgtaaccaggaatcaacctgtgctggacgctgtaatgaagtttgcccaggcccgcctgagccctcctacctttgcacaaatcgctggtgaagccgctgtggatctgcctgctgattattttgacggtatcaaagcggaatatttaagccgccgggatatcctggtaaggatgctgaatgagatcccgggcgtattttgtccgaatccgggtggcgccttctatgcaatggccaggctgcccattgatgattcagataaattctgccaatggatcctggaatccttctcttacgagggccaaacggttatgatgtcacccgcaaccggcttttatgcgacccctgggttaggaaaaaatgaagtgcggctggcttatgtattaaatacaacagacattagtcatgcaatggtctgcctggaaaaggcattggaggtatatcccgggaaaattgccaaataatttttatgtcaaaaccaggtataaaatccgacatgagagccgttaaatacattacaataaattctatatatgtatttttaaagaaaaaagcaattatttaacactcaacgcttggaattttgatattttgtttcgtatatttgatgtagaaataacaacaacgacaaaatttatttaattataaaaatatttacagatacgatggactgcaaaatctaaacttgtttaagaaaaatttaacctgcattatttcttataacgtttatttggtccgacctttgaattattaaaacaagaagatttatcagtcttctgtaaaactcaaagattaactaaaacgttttagcaaaatatcgtatttttgtatcagtttttcataacgtggaatttataaaggcaaacggctctgatcacagagccgtatttttttgtcctaaccttaccttttcccaccactgacggcggaatccaacagaacaaacaaaatattctgaaaatattccccctcctgtttaccttttttcgataatattgttatgtaataaaacgggcggagctaccggcgctttcagcaatggtaatatccgtttgttttcataacgtggaattttaaaatgcaacggtcccgattcctcgggaccgtcttcatttccaggcagcatggctgccgtatataattcctttagttatgccttattcgctttaatcatctcaaagaaatcatcaaacaggtaacggctatcaaacggaccaggagtggattccgggtgatactgcacgctgaatgcaggtttatttttgatacggatgccttctacggagtgatcattgaggtttacatgggtaacttccacattttcactggccgctactgctttcgcgtctactgcaaagccatggttctgggtagtgatttcgcacaaaccagttttcaggttctttaccgggtggtttaaaccgcggtgaccatggtgcatcttgtaagttgggatatcattagcgagcgccagcaactggtgcccgaggcagataccaaacataggtctttctgcagccaggatctttttcaccgtatctactgcgtaagtcagcggagccggatcaccgggaccattggaaataaagtaggcatgcggtttaaattcctcgcaaacctcaaaagtagtgtcggttgggaatacctgcaggtaagcgcctttatcagacaggcatttcagcatatttcttttcacgccgttgtcgagcactgcaatacggatctccgcagccgggtcgcctacatagtaagcttccggagtggtcacttctttgcagagggccaggccttccattgaaggcacctttgccagttcaactttcagttgatccaggtccaggatagcagaagagataatgcagttcatagcacctttgctgcggatgtgggaaaccagcgcgcgggtatctacgtcataaatggctaccaggttattatcggtcaggaacgtatccagtgacccatcggccattttcctggaatagttgtacgcaatattttttgcgatcaaaccattgatcttcacactgctgctctctacgtcgtcctttttggtgccgtagttcccgatgtagcagttgttcattataagtacctgtcctttataagaagggtccgtaaacacttcctggtaacccgtcataccggtattgaaagctaattcaccggcggctgtgccaattttcccaaaagcttttccctgaaaaaccgtaccgtcttctaacagcagtatggcaggttggatggttcttgtctgaggcatttctggtatctgtcttgttttatattttaaaaaaaaccttcaagggtacaaaaattgccctgaaggttcggataaaaaaccgtgcaaaggtatgaaatgcaacagttaaatacagattttttttaccagaaagaaaagatgttacttaatttttacagatttaagcacgcgctgtgccacctggcggccaatagggtcatcgtcgcggtaattaatctggatttgccagcggttgcttcctttgatcattaccaggttacaaaatgccaggcggatgccgcctttatacagataattcccttcttccagcaccccctgcattccggaaatgagtacgggtattgatttacagtcgatatccgtagcggtttccttcagttgcatgctgttatgggaggcggccacagcatcttccaggctgttagctacgctgctgatataactgaacatatttaccgcgatgcggatacctcccccatcttcattagtataggttttcgcgtattcaatcactttagcttcttccccttccagcggctggtcgtgtacccataattttaccggagtactgatttccagtgcctgacggcctatggtagcagtgtgccaggtgctgtacaaactggccagtggtaccttgggatacagaagggtaaacacggctcttttaccgaacagcgtgccggtaatagctaccagcaggaaaacgagtgaaaaaaagatgactattttccttttactggcggattgcagctggtttttaatccaatatagcgggccggtcgtttttttctctctcagtgagatgcctactgcctgggtatattccgggaatgtggccattggatgaagctttcgccattcggcgaagctttgtggcagcttttttccgcacgcatcgcaaaaagtaaggtattcagatttgagtgggttgggatgaccacaactatcacaatgcaggtatttcatagggatactcattaaaactgctgtaatattacgaaatatatgcatttattagcgcataaaaaaggacaaagcctggctttgtcctttttcgtatcgtttgatataagattactcagcagatttttcttctgttgcagtatcagcagctttagtttcagttgcttcttctgctttcttcttagcaccaccggcacgacgggttttcttagcagcagctttttcttctgatttaccgtagatttcgttgaagtctaccagttcaatcagcgcaacttctgcgttatcgcccacacgtttacccagtttaatgatacgggtgtaaccaccaggacgggtagctattttctcactgatcgtgctgaacagttccttgatagcttctttatcctgcaggtagctgaacacaattctacggttgtgggtagaatcggttttgcctcttgtcagcagcggctcaacatacacgcggagggctttcgcctttgccagtgtagtggtgatacgtttgtggctgatcagttcgcaagccagattggacatcagggctttacggtgggaagcagttctgcttaatttgtttaatttaactccgtgacgcatgacattatttgttttaacccttacaccgtgtcaggaattgcaaggtacttgttaattataaagtagttaagccaaagctattgcggatgcaacggctttggcttaacagataaatactattcttcttcgagtttcagtttagacagatccataccgaagtgcagacctctttcgcccaatacctgttcaatttcgctgagtgatttctggccgaagtttctgaacttcatcagttcttcctgttcgtattgtaccagttcgctgagggaattgattttagctgctttcagacagttgaatgcacgtacgctcagatcgagatcttcgagtggtgttttcagtatcttacgcagttgcagtgtttgttcgtccaccacatcttctttttcagtgtctttggtatcaaagctgatgttttcatcagtgatgatcatcaggtgctgaatgaggatacgggaagcttgtttcactgcttcttccgggtggatagtaccgtcggtgatcacctccataacgagcttctcatagtcagttttctgctccacacgggtattttctatgctgtactttacgtttttgataggcgtaaagatagagtcgatcgcgatgtagccgaatactgcatccttgggtttattttcctcagccggaacataaccacggcctttaccgatagtcagttcgatatccagcttggcagaaggatccagggtgcagattaacagctccggattcatgatctggaaagcactggtggctttttcaatcatatcagcgcggaactctgttttacccttaatggacagtgtgatcttttcgttcgttacatcactctctgaaatcctcttgaaacgaacctgtttcaggttcaggatgatttcagtaacgtcttcagtaacacctttcagtgtagcgaactcgtgatcggctccttcaattttaatacccacaatggcatagccctccaaagaagacaacagtacgcgacgtaacgcattaccgacagtcacagcataacctggttctaatggacggaattcgaattgagcttcaaagtcggtagacttctgcaatacgatcttatcaggtttctggaaatttaaaattgccattgatatgatagatttatttgttaaatatgaggttagtccgtgacctttggccacggactaattatttattacttagagtacaattctacgatcagttgttccttgatattttcaggaacgctctctctctcaggataagcaatgaatacacctttcatttctttctcgttccaatccagccagctgaacttaggattttttccacggataacgctggtcagtgcagaattgtttgcagttttgtttttcaggctgataacgtctcctggtttcagttggaaagaaggagtgttaacaacgataccgttaacagtaacgtgcttgtgagaaaccagctgacgggcagcaggacgtgaaggagcgataccaagacggaaaacggtgttatccagacgggcttcgagcagtttgatcaatacttcaccggcaacaccttttctgcgggtagcttcatcaaacaggttacggaactgacgttccagcaaaccgtaagtgtatttagctttttgtttctctctcagctggagtgcgtattcgcctaattgtttgcgtttacggttagcaccatgctgacccggagggttactgttcttacttaaatacttgccattaccgagaatgggctcaccaaaaattctggaaattttggttttgggacctgtgtaccttgccatgttttaaatatactttagattttttagttaatgatgcatgctcttcaaaaaatctgaaaacctgatcatgcatccatttatttaataatattacaacgtccagataccaaacttctaatgaaatctggtatctggatgctgtaaatatatattactatactcttctcttcttaggagggcggcaaccgttgtgtggtaaaggcgtaacgtctttaatcatgttcacttcgataccggagttagcgatagcgcggatagcactttcacgaccagctccagggccttttacaaatacatctgctcttttcagacctgagtccattgcaactttagcagcatcctgtgcagccagctgagcagcatacggagtgttcttcttagaacctctgaagcccattttaccagcagaagaccaggatataacctgaccatgcttgttggtgatgctcacgatgatgttgttaaagctagcagagatatgaacatctccgtagttatctacctttactactctctttttattagcagcagtttttgtattatttgcttttgccataatgatttaaattccaaatatgaaattccgcatcccaaattacacgactcacggtcattgaaacccctcagattcggatttgggatttcaacctgggattttatttattatttcttagttgcttttttcttaccagccactgtcttacgtttacctttacgggtacggctgttggtacgtgtgcgctgacctcttaccggtaagcctttcctgtgacgcaaaccgcggtaacaagcgatatccagcagacgcttgatattcatttgcacttcggaacgcagctgaccttctaccttaaactcaccgttgataatgttacggatggcagcttgatcatcatcattccaatcacgcacttttttgtttacatcaatttccgccttgttcaggatatattgggcggtagaacggcctataccaaagatataggtgaggccaatttctcctcttttatttttaggaagatctataccggctatacgtgccatatttctattttagattttatgattctgattaaaaaatcaaattccgttaggggaaccgattaaccctggcgttgtttaaaacgaggattctttttgttgatcaccaacaaaacaccttttctacgaactattttacaatccgcacttctttttttgattgcagctcttaccttcatgattaatactttataaaaggttatgatatttgttaaattattattccaatcccctctacgctgttcccacttatttgtatctgaaaattatacggcctcttgacaaatcgtatgggctcatctccacgccaaccttatctcctggcagaatgcggatgtagtgcattctcatttttccagaaatggtggccaggatctcatgcccgttttccaattttacacggaacatagcgttcgacaaggcttctaatataattccatcctgtttaatgagtgcctgttttgccataaaaatttttaggactgcaaagatagcatttatcttttgaaatagaaaaatttcccctgattattattaatattgccagtttttttaccaaaacctgtcctttttaccctcaaaacccctgctatattagataaatccaaaatcctatactagtaatttgaatttaattcggggttgtttttctcttctttttctatatccacataggtagataacacatccgccttcccttttccaacagccaccgtatgttcaaagtgaacagacgggcttccgtcgcgggtagctactgtccagccgtcttccaggtactccacgtctttcgagcggagattgatcataggctcgatggctatcaccagtccttccttcatcaccggaccactacctcttttaccatagttaggcacctgagggtcctcatgcaggttccggccgaggccatgccctaccagttcccttactacgccgtaaccgcgctctttttcggtatattcctgtattgcataagagatatcacctatcctgttgccaacaatcgctttttcgatgcctttgtacagggaagctttggtggcagtcatcaggcggagtacgttttcgggtacattaccaatggcaaaggtgtaggcgctgtcggaatggtatccgttcatgtaaacccctacatccacggtgaggatatcaccgtctttcagcacatatttatttggaataccgtgtactacttcttcatttactgaaatgcagcaggcattcgggaaacctttgtaatttttgaaggaaggtgttccaccattttcaacgataaacttatcagcaacagcatccacgtccagtgtagtcatccccggtttcagggtcctggctacttctgccagggctgcactgagaatcagggcacttttacgtatcaactctatttcttccttcgtcttatagtgaatcataacatccttgtttctgtcgctgttagtgatcagcatcagctttctgcgtatgcttttaactgaagctaaggactaactgttctttattcaaaaataatatagccaccaaagcgggaaagcttctgtggctattttattgttcttgtaacacttttgtgttcaattacttatgcgttagccggggcagttctgcctttgatacggccggtgctcatcagtccatcgtaatggcgcatcaggagctggctttcaatttgttgcagtgtatccaggataactcccaccatgatcagcagggatgtacctccgaagaaagtagcaaagttgctgttcactttaaaggcggcagccaggccgggcatgatacccactattgccaggaaaaatgcgccgggcaaagtgatacggtccattactgcaccaatataatcagcggttgctttacctggtttgatacccgggatgaatccgttattacgtttcatttcatccgccatttgggttggattgaaaatgagcgcagtatagaagtaggtgaatacaataacgagcaccgcgtaaatgaggttgtaccagccgttcgtgtgatcactgaagatgcggataaagccggacgcactttctgaggaagtggcaaagcctatggcagttgcagggatgaacatgatcgcctgggcgaagatgataggcattacaccggcagcattcactttcaggggaatgaactggcgtacaccaccatattgtttgttacctacgatacgtttagcgtaattcaccggtattttcctggtaccctgaacgagcaggatgaggcccacggtgattaagataaagatggcaatttcaatgaggaacaggatcggtccacccgcttcacctgcaactttactggaaaattctgcgactaaagcctgtggcaaacgggcaaggatacccatcataatgatgatggaggtaccgttaccaattcctttgtctgtgatcttttcaccgagccacattacaaacagggtacctgcagtaagtaaaacggtagtagagagccagaagaaaaaggtgccatattcggcaataatagcgccacctgactgattacgcagataagcaacgtaagcactcgcctggaaacctgttacgataactgtgaggtaacgggtgaactggttaatttttttgcggccgctttcaccttctttctgcattttctggaattgcggaacagctatagttaataactggatggcaatggacgcagagatgtagggcataatacccaatgcaaatatggaggcccttgaaaacgatccgccggcaaacatgttaaccaaacccaggataccctgattagaatttttctcaaagtcggtgagcgcatttgcatcaatgccgggcaaagcgatataggatcctacgcggtagatgaggaccaggagcagggtggtcaggatgcggttacgcaaatcctcaatactccagatattcttaatcgtttcgataaatttcttcacaggaagataaaggtttaatagcgctattaaatatgaaaagacgcactactccgtaggcgtctcctcagtcgtaaagtcttataccagttctactgatccacctgctgtttcgatggcctgtttagctttttcgctgatagcgttaactttaacagtcacctttgttttgagttcgccggtagcgagaatcttaactttagctgttctgttaatcagaccgttcatgaacaaggtttccagattaaactcctggaggccatatttctcaactaattgatccagctgacccaggttgaagattttgtattcttcacggttattatttttgaaaccgcgttttggcatacggcgttggattggcatctggccaccttcgaagcctcttttgctcgcgtaaccagcacgttgctggatacctttgttaccttttgtagaggtaccacctttaccggaagcctcaccacgtccaagacgtttttctttatgtacagcgccttgtgcaggctgtaatgaatgcagattcataattaattgtttttacttgcgcggaaattaaccgctcgcttttattctaaaataaaaatggtaaagtcacaaatgtaaaggtaagattatcaacagacaatcccacagcagtgttacttaattaagcgttaactgtttctaccgttacaaggtgattaactttacggaccatacccaggatctgaggagttgcttctacttcaacagtagcgtgcattttagtcaggcccagtgccttcaaggtcagtttctgcctttccggacggtctataccacttttcacttgagtgatcttaatctttgccataaacccctatccgctaaaagcggagtaatttaattgttaatgaattattttcaaaattttccggaggtacccagcttttcagcgggtataaatcaaccgttgaaaactttcttcagggaaacgcctcttgttttggcgatgctgattggttcgcgtaacatacctaaagctttgaaggtagcttttaccacgttgtgtggattagcagaacccagagatttagccagtacgtcggttacaccaacgctttccagtactgcacgcatggaacctcctgcgatcacaccggtaccgtgagcggctggtttgatcaacactttggcggcgccttctttagcaaactgatcgtgaggaatggtaccgtgcataacaggaaccttgatcaggttcttcttagcatcgtctatacctttggtgatagcctgctgtacttctttggctttaccaagaccgtgaccaacaacaccgttttcgttacctacaactaccagtgcggagaaactgaatgtacgaccgcctttagtggttttagtaacacggttgatcgccactactttttctttcagctccagatcaccagcctttactttattgaatgaattctttgccattttattttataagaattacttgttcagaattataagattcggacttcgtgattaaaactgaagaccgccttctcttgctccgtcagctacgcttttcacgcggccatgatataaataaccacttctgtcgaaaacgcaggtggtgagacccagtgccagtgctttagcagccagcgctttacctaccagtacagatttttcgcttttattacctgcctgtgctttgatatccttatcacgggaagaagcggaagccagggtagtgccattggtatcgtcgatcaactgcacatagatatcgctgttgctgcgaaatacagataatcttggttgctgtgcagtaccggaaattttcttacggatgcggtagcggattttctgtctcctgttaacttttgtgctcattttgagttttattttattaccccgatgctgccggggtatctgttaaaatcagctaaccagctatagtagctgattagccaattaaatattttacttaccggctgatttaccagctttcttacgtaccacttcatcgctgtagcgaacacctttacctttgtatggttctggtttacgcagaccgcggatcttagcggctacctgacccagcaattggttatcgataccttccagcatgatcttagggttctgacctttttcagtcagggtagctaccttcagttctttcggaatttcgaaaacgatattgtgagagtaacctaaagcgagatccagtaactgaccgttgtttgctgctttataaccaacacccaccagttccagttgttttttgaatccttcagtaacaccctgaaccatgttagccagtaaagcgcggtataaaccgtggagtgctttatgacggatctgttcagttgggcggattactgttaaaacgccgtccttcacctcaatcttcatttccctgtcgatgttctttttcagttcacctttagggccttttacggttacttcattggaaggggaaacagtaactgtaactccgctagccaatttgataggacttttacctatacgagacataactttaatttaaagttgtttgatattgatgtaccggttatccgtgttcagcgccgtatagagagcttaattgtcagataacttaagtgaatgactggttgggtaacaaccagtcattcaatatattaatagatgaagcaaactacttcgccacctacattttgagcttttgcttccttatcggtcattacacctttggaagtagagataatcgctacgcctaaaccgttcttcacgcgcttaaactcttctggtttagcgtactgacgcagacctgggcggctgatgcgttgtaattccttgatagcgggttctttagagatcggatcgtacttcaaagcgattttgattacgccttgtttagtatcttcttcaaatttgtacttcaggatataacctttgtcgtacagaatttctgtaatgcgttttttcagcttggaagccggaatttccacaatcctgtgggtggccatttgcgcgttccggatacgtgtcaggaagtctgctattggatcagtaaccattgttgtaatagtttgataaatgtttacaatgcgatatccaatcgtaataagatgggaatcaaataactttttcgggatttacacctccggtaggccggaagataaacaccttgaattaccagctggcttttctaacgccagggattttacctgcgagagccaggtcacggaacatgttcctgcagaggccgaagtgacgcatgtatcctttaggacgaccggtcagctggcatctgttgtgcagacgaacaggggaagcattttttggaagttgatccagtgcagcgtagtcaccggcagctttcagggcagcgcgtttttctgcgaacttagctaccatagcttctcttttcctttgtctggcttttacggattcttttgccataattatattatcgtttcgatttactgattatcttttttcatacccttgaacggcatacccatttccttcaggagctcgtaagcttcttcgttggtgtttgcagtggtaacgaaggtgatatccataccggacattttcgttactttatcgatatcgatttcagggaagatgatttgttcggtgatacccatagtgtagttaccacgaccgtcaaaagctttttcgttcacacctttgaagtcacgtacacgtgggagggatacagcgatcaaacgatccaggaagtcgtacatattagtgctgcgtaaagttacacgtgcaccgataggcatgttctttctgagtttgaagttggagatatcctttttagacatggtagcgatagctttctgaccagcgatgcgggtcatttcgtctactgcgatgtctaccagtttcttatcacctactgcaccattgataccctggttcaggcaaatttttaccaggcgaggaacctgcataacacttttgtagttgaatttcttcatcagtgcagatttaacttcctcgtggtatttagtctgcagtctcggagtatattttgtgtttgacattatttaatttcctcccctgattttttagcgatacgaattaatttaccgttttctctctgcctgttaaccctggtaggtttaccagttttagcatcccacagcattacattagagatggcgataggagcttcctgcttaacaataccacctttggtattctgggcagttggcttcgtgtgcttggtaataatgttaacgccttctacaagaatgcgggctttctcaggattcacttccagcactttacgcgctttggttctatccttgtcatcaccggcaattaccgcaaccaggtcgcctttcttaatgttaaatttaggcttaaatctagttttcattactttgatttatttataaacgccaagcgaaacaatagtttcgcttgattaatgttttttctcgttttgcaaacgggctgcaaagataagaaatattttcggatttcgggattttggctttttttgataaaaatcataaaaattccaaaatccctgtaccgctatatctttataatacctcaggagcgagggagataattttcatataacccttgtctctcagctcacgtgcaaccggaccgaaaatacgggtaccgcgaggttcgtctgagttattgagcagtacaaccgcgttatcatcgaaacggatataagaaccatctttacgacgtaatttgttcttagttcttacgattacagctttggtcaccatacctttcttcacaccgccacctggcattgcgtccttaacggttactacaattttatcgcctacgccagcgtagtcctgaccggagttacctaatacgcggatgcacaatacttctttggcaccgctgttatcagctacactcagtcttgattcttgttgtatcatcgaaatgagatttgatattgtttagtcagcggctggcaccggggttgccggcagcagcttgaaacaaataaataattattttactttagcgattacttctaccagtctccagcatttgttcttgctcagagggcgtgtttccgcgattttcacggtatcgccgatgctgcactcgtttttatcgtcgtgcgccatgaacttggtagtttttttcacgaatttaccatagatcgggtgctttaccttacgctccaccttaacggtaatggttttatccattttgttgctggcaaccacaccaatcctggtttttcttaattttctttcggtcgtcattgttgaaagtatttaaccctccgtgaggaggtcataaattgtattatactaatgctatgtcagcagtcccggtatcaccgggactgaagaatcagaagcccagttgtcttttacgcagttcggtattcatccgagcgatatcgcgtcttacggcgcggatgctcattggattttcgattggcgtaattgcgtgaccaaaggtcatttttttcaagcggagttcttctgcagagattttctctttcagatcttgttcgctcaggcctttcagttccagcttttcttttgccattgtattgagtttgattcggttagctgccggggcagtgttaccggatttttagttattgtgtacctgtaattaagctacgaagtcgcggctggttacaaattttactttaatgggcagtttctgtgctgcgagttccattgcttcttttgctacctgtaaggaaacgccatcagcttcaaataaaattctacctggctttacaactgctgcccaatggtcaggagcacctttacctttacccatcctcacttccaaaggcttagcagtgataggtttgtcagggaatatgcggatccatacgttaccttcacgtttcatgtgccttgtcagcgcaacacgtgcagcttcgatctgcctgtcggtgatccacttaggttctaatgctttaagaccgaaagtaccaaaggagagggtagcgcctcttttagcgttccctttgatgcggcctttgtgcatcttcctgtgtttcgttctttttggctgtaacatcgtctatgttgttaatgttaatagtaattgttaatgtctgcttaaccgccagatactatctgcggccaccgccacggtgttctccaccgcctcttctttcgccaccaccgcggttatctctgcgttcaccgtgatgttctcttctttcgccgccatgaccagtaccacggttatcaccttctttaccggttaaaacgttcgggttcagatcgcgtttacccagtacttcacctttacagatccatactttgataccgattttaccataaacggttaaagcgaacagggaagcgtaatcgatgtccatacggaatgtatgtaaaggcacgcgaccttgtttcatttcttcggagcgggcaatttcagcaccacctaaacggccgctgattttaaccttgataccttcagcacccattctcagagcggtagcaatcgccattttgatagcacgtttgtagttaatacggctttcaatctgttttgcgattgtttcagcaacgatgttagcatccatttcgggacgacggatctccaggatgttgatctgtacatcttctttgcctgtcagcttcttcagctcttccttgatgcgatcaacttcgttaccgcctttaccaatgatgataccaggcttagaagtatgaacagtgatgattaacttacctaaagttctttcgatcacaactcttgagatgccacctttgttgatacgggcattcagataagttctgatcttgttatcttcgatcagtttaacagcaaagtcttttttgctgccataccaattagagtcccatcctctgatgatacctaacctgttaccaataggatttgttttctgacccatgttctggttatttgtctattagtttaatagttttgtttctattttgtttccggtttgcactgaattactgtgctttaccgtccactacgatcgtcacgtggttacttctcttgcggatacggtaaccccttccctgtggagccgggcgcattcttttcagggtgcggccgccatcaacaaaaacggtttttacgatcaggttagcatcttctacccttgcaccttcgttcttcactttccagttggcgatagcggatatcagcaacttctctaaaggtacgcttgggtgtttcggatggaatttcaaaatattcaaagccttttccacatccagaccacggattaagtccgcgagcaaacgcattttgcggggagatgtaggattattattcagcttagctactgcttccattgttattaatttcttttattatttaatgtctgacgtctggtgtttgatgttccggtttgaaacgaatacttcaaacctcaaacctcagactataatttacattttcttgtttacgtgtcctctgaagttacgtgtaggtgcaaattcgcccagtttatgaccaaccataaattccgttacataaacaggaataaatttgttgccattatgaacagcgaaagtgtgaccaacgaaatcaggagtgatagtagaacgacggctccaggtcttgataacagaacgcttggtaccggtattcatcttttcaacttttgtttctaatttcaggtctacgtaaggacctttttttatggaacgagccatgtcttactgatttatgatttttcaaacccgggatccggtattgctaccggagccctgattcagaaatactataattttttaccgttttttctgctaatgatcagcttatcagaactcttatgcggttttctggttttcagacctttcgcatatttaccagttcttgatcttggatggcctccggaagatttaccttcaccaccacccattgggtgatccacagggttcatagccacaccacggttgcgggggcggatacctctccaacggttagcacctgctttaccgatggattgcagtgcgtggtcggagttagaaacagtacctacggtagctttacaagtatttaatactttgcggagctcgccggaaggcattttcagtacggcatatttttcttccttgttggacagctgtgcgtaagcgccggcgcttcttgcgattgcaccacctttaccaggctgcagctcgatgttgtgcacaacagtacccagtggcatattcttcagtggtaaagcgttacctacttcaggagctacatcggagccgcttataacggtaccaccaacctgtaagccctgtggagcaatgatataacgtttttcaccgtcagcatagtttaccagtgcgatgaatgcgctacggttaggatcatattcgatcgttttaactgtagcaggtacattctctttatcacgtttgaaatcaattacacggtattgtttcttgtgaccaccacctatgtagcgcatggacattcttccttgcgcatttctaccgccggtccttttgatgggctccagcaggcttttctcaggggtatccgatgtcagctcagcgtaagcgttgcctattttccagcgggtaccggccgtcattggtttgaacttcttcagtgccattacttcctaaaaagttaaatgttgttattaaatataaatagtgatctgtatatacatccacatcccggctgttcaggccggaacggcactacatgttagcatacagatctatagtttcaccacttgcaacggtaatgatcgcctttttgtaagacggttttttacctgcgatgaaaccggctttagtaaagcggaattttgctttacctggcattacagcagtatttacttctgctacggttacgccgtaaaattcttctactgcttttttgatctccagtttgttggcttttttgtcaacaatgaagtagtagcggttgaatttttcggttgctttgttaaccttttcggataccaccggtttgattaaaacgtcagaaagtttcatcttctttatagcattaagctgttggcgttagccgcaagctgttatttaattggttttgacatcctatgcttccgcttctgcaggctcttcagtgaagatctttgcagcgctttctgtgaacacgatataattgctgttcatgatgtcgtaagtgtttacgtcgctcagtacagtaccgtctacagtaggaatgtttcttaaagacaggtaaacattgtcattgtattcaggcgtgatgaacatagtctttctgccttcaacattgatgttcagattcttcaggaagccaacgaattgtttggtttttggtgtttcgagctgcagatcttcaacaatgatgatgctgttttctttagcttttactgacagggcggagatctttgcgagatctttcacttttctgttcagtttgaaaccccaaccgtgcggttttggtccgaagatggtaccaccacctttatacaatgggttacggatgttacctttacgggcgccaccggtacctttctgtttgtgcagtttgcgggaagcaccttgtacttcagctctggtttttaccttgtgggtaccctgacgctgagcagccaggtattgtttaacagccaggtagattacgtggttgttaggctcaacaccaaagatctcctcaggaagatcaatagtccttccggttttcttaccttctatatttaaaatatcgatttgcatgttacttctggattaaaacgattgaaccaatgtggccgggaacggaaccacttaccaggatataattcttttcagggaatattttcacgatcttcagacctttcactttcactctttcgttacctgtctggccggccatacgcatacccttgaaaacgcgggaaggataagaggatccaccaacagaaccaggagccctgcttctatcgtgctgaccgtgggtagcttcacccacaccactgaatccgtggcgttttacaacaccctggaaacctttacctttggaagtgcctacaacgtcaattgtttcaccttctgcgaagatttcgcaggtgatagattcaccgagggctttctgtacatccgggttgcggagttcttttacaaaacgtttgggagaggtgcttgctttcgcgaagtgactgctttctgctttagtggtgtgtttttctttcttctcaccgaaagaaacctgaattgcattgtaaccatctgactccagggtttttacctgagttacaacgttgggacccgcttcgataatggtaacagcagtttgcttaccattagactcgaagatactggtcataccaatctttttgccaataatacctttcattttttatatgattttacccagcgcctgggggatttcgtgctatccccaggatgggcggtttaaatacatttattgggcggccgcccagaaggcgcgacctatgtttgcttgttaaaattgctatcctgctggtaatcaacatgataaccataaatcaataaaaggccggcctttcgcccgccttgctgttgtcctatgctttaatttcaacttccactccggaaggcagatcgagcttgctcagcgcgtctacagttctggaagaagacgtgtaaatatccagtaaacgtttgtgtgtacacagttggaactgctcgcgcgctttcttatttacgtgcggagaacgtaatactgtaaatattttcttctcggtaggtaaaggaattggacctgttaccacggcacccgtgttacgcacggttttaacgatcttctcagcagacttgtctaccaggttatgatcgtaggacttcagcttgattcttattctctgagacatatgcaatgaacttcttcttgttttttcccaatacaatttgggagggcaaaggtaacccgttttttctatttggcaaataaatctcaggaaaaaataaaagaaaccgggcaaggggctggctccggcggcgaaagaggtgcggtaaaattgctgttaccggggatgacggcttcagaaaccattcattgtgtgtatgttaagccttaaggtaacttcacatgccccgttttgacaaatataggaaaacatatttcaaaaccaaaaaaaggagaatttctttacaatttttttcccgggagatggaaaacggaacggatacctctcaacagtatccgggaacggggagccggggagcgtaaagcgatatcaggattatttctttccttgtatagccctgtcaggacgggatagtgcatggggagtgcatgcttagtgcattaagagtgcatcaggagtgcatgaggagtgcatcaggagtccatgctaacagtattcatactgcatacatagtccagggtatacgcaggtttgaggcatgggagaaatatcagtaaggtaaccgctgccctggaaggtaacttccccggtgtaaggatcaaaaataccagcagcgcggctgacaggttccataaatccttacttcaggaggaagcggagccatccctgtcagatggcaataacccaaaagagaaagggctgttcccgcttacctggaacaaccctttctgaataattgaaatggtttgatgacttgttggtcaatcgacccaacaatgattagagtggtaaaccacctaataatgacttaactaatcctaagattaatgccagcagttgattcagtaaatccatggaaaaaggtttttataagatactgcctactctattacctggttttcggcgatgcccagttgttattcagttaacatgtctaaattaaaagctctcattcaatatccggccgttcattttattcattccaatccaatcgcaattatttgttcatttagccaccatagccatgttacgcggatactgccaacaaaaaaaagaggctgttctggtattgaacagcctccggatgatgttgtaagggaaatagtatcatttaagtacggaaaaatcccttaccgaaaggagtccttattacaggccacccagcagagatttcagcagggcaaccagcgttgccagcagttgattcagtaaagccataagatagtttttactacgggtgacacctactctctttatttggttttcggcaatcccatgtacacttcttgttttagtgcctgtcgaaattaacggctattcacagaattccgctcgttcattttgttcagttcggcatcctgatattatactgttcaataggctgccatggctcatttacattaaaagaaaaagccccggcaaaacataccggggctttttgttcagaagttgttaaatcagcttcctgtctgaagcgcgattcgtgattcaccggtaataagcattgtatttacattacggaaccatatgcaggtactttcatatgttacaacctcggccggggttagtgctaactaacaatacaggttaaatgccgccaagcgcagacaccagcagcgccagcaatcctgtcagaaatgtgtttaaagcatcaaggatcataaggtgttgttttcatttgtgcctactcttacttgtgattttcggcaatttccattaattaatatccttgtgtaacaaggtgtaaaatttacagtgcgccagcaacggttgccaggaacttcagcactgccaggagaatagagtttaccatatccggagttttatggatgtaatgcttactctgttccgggttttcagcttcccccttgtctgcgtcttcacagacaactactaaaataaatggttccggcttaaaagccttcgttcagttaattcattcctgcttctgctgttcattttattcagcgcccttaaaagacaggactccttataacagcagcggcggcaataatcattgccgccgctgctgttgaattgtattatatactaaattattttcctgtttcttccctgtaaatctgtttcgcctttgctgaaggcagatagatctggaaacctacacccagattcagtctgtttgaagtagtagagctgccaaaacctactgtgagatcgtatttcagcaatccttccaaaccaatattaggggtaataaaataggaaatgccagggcctacacctatattaagaccgttagttgaagccccgttagcaacattggtacctgcaaaaccaacgtttccttccacgaagaaacgggtacgtttggagaattccagtttccttacatttttatcctccacaaaataacgggcaagtgcacctacgccgtagtttgtattggtacccgggttgtcagttgtcaaaccaaagtttacgtagcctcccaatgcaagaccatccctgataaaccaggccgcttttggtgtgagatccatactaaactgggtgctttctttctggaaatttaaacccaggttacccaaggtaccacctaccataatatttcctttctgaatctgggcgttagcagcagaaccaaacaatacagccgcaagtgcaagggttaagagacgaattcttttcatagtctgatttttagttttaacaatttacatgttgaatgaataagaaattagcacgcaaacgctttccgtttgcaactaaagctgctgatcagccgtaaaaaaataaaggcaggggataatggggagtaatcttacctcgtcaaacaaacatcatcacagttaacaatacgtattgtatcacaaaactactgaaaatgagtctaatatgtgcgcatctttcaaaaaaaatctaaaaaaacaccttatcagatcccttcagatattatacttattcgattcattattactataacatccagaacttaaatgttgttgtataaaaacctgaatcaatagaaaagaaaagggagatcatccagccgtagtcagtcaggacatgcctttcagcagatcggcgtgtgtgcagaaagttccgttttgttgcaggaaatcaaggaataaatccatcttttgctgcattcttttcccggatacacgcctgatataaccaggtaattcatacgcattgatgtcgctcaactcccagggatggaagtaaaaagaaaggtaggagtccttcttcaaaattcttttactgaaatgccgggttacccacaggggcatattttttacgctcagccagaacaggggatacctgagaaaaggagatacggaagatggaatgatccaggtatcctggtctttgaacacggttctcggcagatgccggttattgtatcttccgggaagccaggtggggtttaccgaggcatcatacaggtagccggcggctttcagcgcctgcatatttactttacggaggcgcggcatgcgaaacccctgtaccggctgactgctgatttcctgcagagccaggcgggaactttccaggtccgcttctgtaaaagagctatggtaataggcatgagaggctatttcatgctttactgccatttgcctgatcagttcaggataatgttgtgcccaataagcggtaacgaaaaacgtagcgcgtacattgtatttgtcaaataaagccagtgtggcctgcaacccgctcctggaaacttccagtttctcctggagggttacctgctggccgaattcttcggggatatcaaattcctccacgtccacactgatcagtatcctgtttctttgttccataaaaatttaagcagccgatgagccgaaaacaatcctgcaataattcatcatttctttcattaaaagtttcaccctgaaagatgaaaactggatgcctggccggcaagatactgcgactgcgccaattttgagatgggaacgtttgcctgcgtggtataaaaattcgctgtcgtacagaaagccattgatgcgggtggagagcaggatattctttccataggcattaaagccctttaaaccggcctgtgcgtcttctactttgaggtccagcactacccggttcaacaggcggctgatgcgggtaattatacggcgtttgcggggtaactcacggaggtaggcttctcccctttccccggctaccacatccaggccctgcattagacgatcgtaggcttcttttaccgccgatacgccaaaggggaaatcgaggtccgtatacacctggaaagtgtgttgtgagcgcttcacgccttccctcacagcgtatcctttaccgcggttacgggaatagctgacgataatgatgtccgggatagctgcctccagccagctgatatgctgccgggtaaagttttttacagagccgtcgttcaccaggatgagctgaacgggtgcggttcccatcagggttgttatttcgtggtaatgcctgataagtgattccacccaggggcccgacgggttccagcagggcagaatcaagtccagaccgggagttaacgtaaccatttctcccgaggtatgtaccacagttgtaggaggtgcttgtaataactctaatgacataattcaaaggctatcagtaaataataccggttgagatggtttatatgctatacctatgacgtcgaaagagaaacctccccctatcaccggggtttaaataataaaaaaggtcctgtaaaacaggaccctggcagttagcaaaaagtaaattgcagttgtaggttatcgttattgtaaaatatcgaatattcttgtcatggcaatagcatgttcatgtcagttagtgctgtaaaagcagaaaggttgttccgctttggcagaacaacctttccggtataaaagaaactatgattaagcgtttactttgcctttcactttagctaccacttcttccgctacgttattcggagcaggagcatagtgggagaattccatgatagagcttgcgcggccggaagacagggaacgcagctgagttacgtaaccgaacatttcgctcagtggcactttagctttgattacctgaacaccatttttggagtccataccttccagcatgccacgacgacggttcaggtcacctgtaacatcacccatgtattgatccggggtaagtacttctactttcatgattggctccagcaatactggtttagctttgcgggcagcttcacggaaagcggatttagcgcacaattcaaatgacatcgcatcagaatccacctggtggtaagatccgtcgaacagacgaactctgaggttcaccagcgggaagttagcgagtacaccctggttgagggattgttcgaaacctttctgaactgcagggatgaattctttagggatggaaccaccaaagatatcattgatgaactggaaggatttaccttcgttttctttcagccattctgcgtctgcaggtccgatttcgatctggatatccgcgaacttaccacgaccaccggtttgtttcttgaatacctcgcggtgttcaactttggtagtcagtgcttctttgtaagcaacttgcggcgcaccctggttaacttctaccttgaattcgcgacgcatacggtcaacgatgatttcgaggtgaagctcacccataccagagaggatagtctgaccggtttcttcgtcagttttagctctcagggtaggatcttcttctaccagtttggagatagccagacccattttatcaacgtctgcctgagttttaggctcgatagcgatgtggataaccggttcagggaaagtcattgattccaggataatcggtgatttttcatcacacagggtatcaccggttttgatatctttaaaaccaacagcagcaccgatatcaccagcttcgatgaaatcgatcgggttctgcttgttagcgtgcatctgcatgatacggctgatacgttcatttttgccggtacgggtattgagtacataagaacccgcatccaggtgaccggaataaacccggaagaacgccagacgacctacgaaaggatcggttgcgattttgaaagccagtgcagacagcggagctttagcatctggtttacgttcaacttcttcaccggtgtcagggttggtacctttaaccgcttcaacgtccattggagaaggcaggtaacggcaaaccgcatccagcattttctgaacgcctttgtttttgaaagaggaaccgcacatcatcgggatgatagcgatatcgatagtagccttacggatagcttcgtggatttcgtcttcagaaattgaattcggatcttcgaagaatttctccatcagtttgtcatcgtattcagcaactgcttccacgagtttagctctccattcttctgcttcagctaccatgtcttccggaataggaatttcctggtaagtagcacctttaccttcttcgtcccagataatacctttcatggtaatcagatctaccacacctttgaagctgtcttcagctccgattggtaatgttaaaggtaccgggttagcgcccagcatttctttaacctgtttaaccacgttcaggaagtctgcaccggaacggtccattttattaacgaaaccgatacgtggtacacggtagcggttagcctggcgccaaacggtttcagactgaggttcaacaccggatacagcgcagaacaatgccaccagaccatccagtacacggagggaacgttctacctctacggtaaagtccacgtgacccggggtatcgatgatattgaatttatattgtttggtatcaggtaaggctttaccttgtaaggttggaaaattccagaaacaagtggttgccgcagatgtgatggtaatacctctctcctgctcctgtgccatccagtccattgtagcagcaccctcgtgcacttctccaattttgtgggatttacctgtataatacaggatacgttctgtggtagtggttttacccgcatcgatgtgcgccgcaataccaaagttcctttgaaattttaagtctgccataatattaaagtgactaaataatgcaatttggggggcaaaggtaacttatttttgacaataaataaaatgaccttcttttccaaattgttatttctttttaacaagcgcgggcgttattcacattaaatttaataacgataaatagttccccgaaaaccagtttttagatggtagcgaccacttgtatatgaaattcaaccaaacattaaattagcattttccgggtgccataattctgtcatattcgtagtaagttataaaaaggatatacccactgaagaagaatgctagtgaaatagtccaaaagtagaactgaaatcgatttccctaaaaatgaaaaacaacatgaaataaaagttactcaacgcgcttgtataacaggctgataccttatttactattgtaccccttcctgtcccggcgctgtagcggttcccgaacacttatttacttataaccatacataatatgagaacaattgtactcagatgcactccagcactgttgctgctgatgtgtgcctgtatttcgtcctccgcccaggtagcgcttaaacgacaggtagttgccgtcacaggtggttccgccgtgatccagaacatccagttccagtataccgtaggagagcccattattttacctgttacagatggcagggtgttactcacccagggattccagcaacccgaagatttttcaaagccgacacccggcgtaaacccggtaaagagctacctactgttccccaatcctgctattaccaataccagaattgtatttgacctgctgtcgaaagtcagtgtaacgatcgaactgattaaccccgccggtcaggtgatacatcaccaattcctggaaatgggtccgggtaaaagcacggtggtattgcctgtgaaccattttgccgcaggtatttacaccgtgatgctgaacgtaagcgggaatgtattcttcgagaaactcattgtgcaataacactacacaatcaccctttaacagatgacaccatgaaatacggttatacaattgtacttcttgcaggtatactgacaaccagtatgcggctgtcggcacaaaaagcaacccaaaagcctccgaatatcggcgccagcttcctgctggtaaaccccgacgccaggagcagcggcaccggggatgcagctatcggcttatcgcccgacgccaactccctgttttcaaacgctgcaaaaatagtgtttgcgggcgactggggcgtgagcgccaactactccccctggatgtgggaactgaataataataagtcaaatatggcttatgtatccggctataaaacatggaacggatcggaaggagtaggactttccatgaagtacttcaactatggctccgttacattccgggatgataacggcacggtactccaggactataatcctaaagaatttgcgatagatggcgcctatgccaggaagctgggaaaccatacatcgctggcactcagcatccggtacgttcgcagccagctgggacaaggttcctacaataatattcagcagaaacccgcatcagcagtggccggcgacatcgcctattattaccagaacagtgtggataaactggatttcggtaaccgctactgctttggcgtaagtattaccaacatcggaacaaagctgcaatactcagacgataacaaccggaaaagttttctgccgatgaacctccgtatcggtggcggctatacgtttgtgcatacccacgaacatgaatttaccctttcggtagacatcaacaagctactggtacctaccccaccgctgtatgccctcgattccaacggaatggaaaccagccagatcctgaaaggaaaagatcctgaccggggcatagtagacgctatgttctcttccttcggcgatgcccccggcggcttccatgaagaattaagggaattcaccattggctccggtattgaatatgcttacagacaggcattttttgtacgtgctgggtatttttatgaacatcctaataaaggctaccggcagcatttttctgcggggctgggcgtacgcgtatcaaaccttgcgctggatatcgcctatcagcttcctaccggagaaagcctgattcagaaaaggaccctgaagttctcgctggtttataacattggcggaacgcgggatgaagccattcaacaaccgtaattcatctactaaaatatccaacatgaaaagcgaatttataacacccaataatatgaaatcactgatcatacttgcatttcttttgtttgccggattcatgcccggtgtttttgcacaggaatctgtaaaaccagataacaccggcggtagtaccggaagagtaaaggacatgcttttccctacttttcagaaagatcttgctgacctgaaccagcggtcagctatacctcctgctgaccgtgccgttgtgtctaaagacagcaaatcgcgtcttttcaccaaataccaggcgccacgcagcaatgctgctccacaactgcgagcagctaaaagcaggccgcttccttctgacagtgcagcaactgcaaaaccggatacccaggctcctaaaattgttcctacacctaaccaggatggcggatcatcacccaaaaagaattaagcgcatcgtaaactatcacaaaaatgattattatgaaaaagatatgttacctgacctttctcctgttgacggtatcatttcatattgtatgggctcaaagcggattaaccggaaccaactaccaggcggtagcccgcaatacaaatgggacagtactcagcaaccaatccttaacggtgcgtttttctattttgggaggttccgcagcaggacctgtacaataccaggaaacacatagtactaccaccaataccctgggattattcactttacagattggtaaaggaactcccttaacaggcacgtacagcggtgttccctgggcgaatgccaatcaatttttaaaagtagaagtatctataaacggcggcaacttcagtgaattgggtacttcccagttaatgagcgtaccgtatgcgttatttgcagccaatggtactcctggtccggccggggcaacaggaccagccggccctaaaggcgatcctggtgtagcgggtcctgtagggccgataggaccagttggtcccgtgggacctgccggcgctaagggagatcccggtgtagcgggtccggtgggcccaataggaccagccggtgctaccggaccacagggcgccaaaggtgatccgggtgtggccggaccagctggaccgattggacctatcggacctgctggcgccgtcggaccgcagggggcgaaaggtgatccgggtgtagccggtccggttggaccgattggacccgccggtgctaccggaccgcaaggtgatcccggcgtagctggtccgcaaggcattcagggcgtacccggcgcccctggaccagttggcccgatgggtcctgcaggtcctgtggggccaatcggtccggccggtgatattaacggcgtagccgcgggtggtgatctttcaggtacctatcccaatccacttatcgggaatggaaaggtgacgctggcgaagattgccccgggtgtgatcccaaccaccctgcctcccaacggtcctgccggcggagatctttccggtacttatcccaatccggttgtaaatgccttacaaggtaaaccagtgagtaacgtagcccccgcagcaggacaaatcctcaagtttgatggtgcccaatggttagcaggcgcgcctccgggaggtggtctcacactgccatttgtagctacagaaaacaatgcggccacgcttttcagtattacaaatgatggcgacggcacttccctggaaggggttaacaataccgcgaccagcagcattgcagctgtgagaggcattgtttcctctgcttcccccggcggattttccagcgcggtaagaggtatcaataacggcaccggtggtttgggtataggtgtatggggctcccaggctggttcaggctggggcgtgtatggtgtaacgccgaacgggctcggtgtatatggcaatagcagcgccggtggtaccggcctctatggaaacagtaatactggtaccggcttaacagctaccagtaacaacggtatagccgccagtattgccatcttcaataatgccaataacaataatgctttaaatgccagcagccttggaaatggtactgtggtgaatgtaacttccagcggtagtggggcaggcgtacgtagcagtaccggcgccggttttgccattcatggtattaccagtgcgcaaacctcagctggtgttataggcgataacaacggagccggagaggccgtagttggaaggaccaccagtgacattgcgggggccgtagttggacggaacgacggtggtggatatggtgtacgcggttttatttcgaccaacacttcaggcacagcaataggcgtattaggccaggtaggtttaaacaacagtaccggaagagccggacgttttgagaatttcaatgccaccaatactaccggaaatgtgttggaagtagcgaccaatggtaacggtaatatcccggataacacacagggtaatgcttcttccttcctggtagacaataccaatagtgtgggcgccgcagtaaggggcgaggtaaaaactatttttggcaacttcggagcggctgctttgtttggtgtttcttccggtactggtggatttgcggggttgttccatgcttccaatgctgcaggaaacggtgctgcactggtagctataacggatggaaatggtaatgccattaccgccaatgcgagcaaaaatggcaatggggtagaaaccaatatagacggcggcggaaatgccttgtatgcctgggtacccacctttgccactggcagggcaggcagatttaatatctttaatgaatccaataccagcgatgcagttaccgttacaacggtaggtaacggcattgccggcaacttcaaggtagacaaagtaacgggcacatctccggcagtaaaaggagaagtaaactcccagttttccaattttggtacggcaggtattttcggattatcgtctggtaccggtggttttggggggctgttttatgcatcaaacccttcaggaaatgcgccggctattgtggcgcttaccgaaggcagtggtaatggcattaccgctaatgccggcaaaaatggtaatggtgtagaaggaagctctgatggcaccggaaacggcgtttatggatgggtccctaactttggtaccggccgtggcgcacgctttgccaactttaatgccgctaactccagggaagtggtattaatcagtaatgccggtaccggtaccggtttgttgatcaaccataccggtccttccggcaatttagctgtttttcagagtgccagtgcaaatgtggcccgtatcaataaggccggacgaggtttcttcaatggtggtacacaagccagtggagcggatgtggcggaatcatttgccgtatcaggcgaacgcaatacttatgaagccggggatgtactggtgatttccactcataccgaccggatggtggaaaagtcatccgaaccttattctaccctggtagccggagtatttgccactaagccgggtttgttattaaccgaaaaggatattgacgccaatttagatggtgaagtacctatgggtgtgataggtgtaataccaaccaaggtttgcaatgagaatggcgctattcgccgtggcgatctgctggttacttccagcagggctggttatgcgatgaaggcggatattgataaagtaaagccaggtcaggtacttggcaaagcgctgcaggaatttagcggtgcagaaggcaagatcaatgtgctggtgagtgtaaaataagtgattccgaaatagcgaaaggcgggcatctgcggatgcccgcctttttgtttgtggccttcgccacttaaattgtctttcgcggattttgtcttggctcaggattacgctgattatactgattagctggatttttactttttggattttctttggattaagggagatggaagcggaggttatctttcctttatcaacacaaaaaggcaaacagctccaaaaggaactgtttgccaaatatattgagttgcctgtgagggctataactagattctgaagtgagagaaagctttgttcgcttctgccatacggtgagtatcttctttcttcttgaacgctgcgccttcacctttgcttgctgctacgatttcattcgcgagcttgtcagccatgcttttaccgtttctttcgccggcgaagcgtactagccatttgatgctcagggatatctttctgtcaggacgaacttccgcaggaatctggaaggtagcaccaccgatacggcggcttctaacttctacacccggagtaacgttggccaatgcttttctccaaacctcgtaaccgttttcaccggtcatcgtgcttaccttatccacagcatcgtagaaaattttataggcaatgctcttttttccttgttccattacgttattaacaaagcgggttaccagcttgtcattgaaccgaggatccggagccagaggcaatttctttgcagcttgctttctcatttattgaaaattacgactatttataattattattttttagccttttcctttttagtaccatatttggaacggctctgctttctgtctttcacacctgcagtatccagggaaccgcgaacaatgtggtaacgaacacctggtaaatcttttacccttccaccacggatcagtacgatggagtgctcctgcaagttgtgaccttcaccagggatataggcaatcacctcaactttgttggttaaacgcactttcgctactttacgcagagcggagttcggtttcttaggcgtggtagtgtatacacgagtacaaacgccacgacgctgagggcagctatctaatgccctggacttagacttagcccggataatttctcttccttttcttactaattgttgtatagtaggcattctttacctagtttttttatgtcggtttacaatgacatccaaattccccacatagggattttgggacggcaaaggtaaaactatatgtgtgaataacaaaattgtttcgaaaatatttttgccggaatgatctcccgggtaaacagggaaaggtcttattattttggtagcagctcaggattaccaaaaaccggattgcaaaggtatgatatccgttagaaactaccataaaaaaatagggcctttttatcggccctattcttatctctataataatatataaaacgcttatttcttgtctattatgtaattccaatgccggatatcggtggtgcggccggtgcggatatcatcgagccgctggattacttccgcccctacttcatatttggtagtatccagtttgatcttcgtatccaggtaatcaagctgttctacataagccacgctggaggcggtgcctgtaccaaatacttcgcggagggtaccattattataggcagttaccacctcatcgatagaaattggcctttcttcaattttaagtcccatatctgccagcacgtccattacactggcgcgggtaacgccttccaggatggtgccctgggtaagatcgggcgtgatggcggtattgccgataatcgcaaaaacgttcatggtaccgcattcctgcaggtatttatgttcgtagccatccacccagaggatttggtcgtagccctgtttccttgcctgcatggtggggtacatggtaccaccataattgccggcagctttggcgtaaccaacgccgccggggaaggcgcgtacatatttatcctgcaccagtaatttgatgggcttattgaaataaggaccggaaggtgagttgatgatggcaaacttataggtatcagacgggcggacgccgataaattcatctgccgcaatcataaagggacgcaggtagagggaacagccttcaccggtgggtacccagttgcggtccaggtctatcagtaaatccaatccgcctacaaacaaccactcgggtacctggggcatgcccattctttctgcagaggtattaaaacgtttatagttatcatatggcctgaagatcatgggatgaccttcgggatctttataagctttgatgccttcaaaaatggcctgcccataatgccaggcagcattggaaggacttacagacaggttctggaagggcagtatctccgcatttttccattctttaccatcaaaatcggccaccagcatatggtcggcgtacattttaccaaatgccaggttgttgaaatcaacctcactgagcctgctgtgcgtagttttggtgactttaatcttctgaagtgcctcttccttaactgttgatttatctaccatcatggttaatcaattttatctcaatatttttacattttaatcgctgtgccaccggagccctggtggaaccggcagtgcaaataaactgatttttccccagagggggttttcatattaaactaaacgataataaacatgtcgcttgagcaaaccgaacttgacccgtactttctggctaaaatctttacccagccaatcattcccgggaaaagcatgccggctgaggccgtagaaaaagtgacgcccaaagtcaaatatttaggagaaaatcaaaaaaacattgcgctcttcatacaaaacgaaaacgaagcgtatttaaacgaagaattattcaacctccttactaatatattaaatgcctgtaaactggggatgcaggatgtatcactgattaacgtaatccactacccttccctcacatttcccgactggcaggcggcagtgaagatagaacggagcgttgtatttgggattgcaccggaacaacttgggttaaatgatataccaccatatcagctggtaactgtaaacggtaccaccttgttgttttccgatgaactatccttgataggcagcgataaagtactgaaggccaggctatgggccgggttaaaacaattattaggcatttaaacttcttttccaatcatatgaaattgatattcgccaccaataacccaaacaaagtaaaagagttccggtcgttactgggaaaccagtttgagatcgttaccctgctggaagccggtattgatatagacattccggagccacatgatacgcttgaagccaatgccaccgaaaagtcggccaccattcaccgcatgaccggggaaaactgtttcgctgaagacaccggcctggaaatagcggcgctcaacggtgcgccgggcgttttatctgcccgctacgccggggaacagaaagaggccgccgacaacatcgctaaagtattacgggaactggaaggccaaagcgaccgcagtgcgcagttccgcaccgttatttccctgatactggatggtaaggaacaccagtttgagggagtgagtaaaggtcatatcaccaccactgtaaaaggggaaaagggatttggctatgatccgatctttgttccggaaggtgaaacacgcgcctttgcagaaatggatctcacggaaaagaacaaatacagccaccgggcacgggcctttgagaaatttgtggccttcctgaaacaaacagcaaacgtttagcatctccctaaaaaataaatatggcaagagtcaaaatagatttacctgcaacattcccgttcagcgtacaaattcccgtaaggatacgggatattaactatggcaaccacgtaggcaatgacgccatcctgtctattattcatgaagccaggatacagttcctcaacagcctcggctataaagaactggatcatgaggccggcgatggttttattatggcagatgtagccattgcatacaaaggcgaaggattttacggagatatatttgacatcgccattgcggcgggtgaatttagtgccctgggctttgaattgttttatcgcatcaccactaaccgtaacggacaaacgattaccattgcagaagctaaaaccggtatgatatgctttgattacaaagcacataaagtagcaaaactgccagccgatatgaaggcacgactggaaacaggaaaataaaaacaacagactatggatgaagcaaccacctccactgcagtggagcaggcgattatagcacgccgcacggtgaaacccaccagcatgaacggccggaagattgcagatgaaacggtacaacagctgttgcagctggcagattgggctcccacacacggatatacagaaccctggtactttgtggtatacagcggcgataaggtacagcagttttgtgcagatcatgcggatatgtacaaacagtttaccccggctgataaatatattccaggtaactacgacaaactgaaaacacagggcaacctggcatcgcatgtactggcgatttgcatgaaacgcgggaacaatccgaagatcccggcgctggaagaaattgccgcggtatcctgcgcagtggaaaatatctggctgggcgctactgccctgggtattgctgcctactggggttccggcgggatgacctaccaccctgccatgcaggaatattttggtttgggagaagaagacctggtactgggcttcttttatatgggctacacagatgagcctgtgcaaccgggaagaagagtgaaaccttttaatgagaagttcaaatggatgtaattttataggaagatggggacctgttgatccccatcttcctataaattatttcaacagatacccgttaacttcggctgcaaagctgctgatctgcgtagctacccaatgttcatctttatgtaattcttctgccataatccgggctacggcaggggctatacgcagcgcttcctttgcatcgaggaacaacaaacgcgtgcggcgggccagaaaatcttcaatattgcgggccatttcctctctcacagcccataccacctgcgctttaatgatatgatattccccgctcagcacctcctgcagatccggctgacgcgcgaccatctggtgcaggtgcaatacatcactgccatagaaataccagggatcttcccagttcaccttatcagtagcgccatgtattttcaggtgatgggtaacggaggatgtttccttccacttcagcaccacttccagcttatgtatgacgtcttccgccatcctgcggtaagtagtccatttaccaccgattattgtaataagatttgacgcagacacgattattttatggctgcgggagatttcctttgttttatgtccctctgctttggcggcggcaagcgggcgaagaccggcccacacgctgcggacatccgagcgttgcggcgcctttgacaaatactgaccggctgtgcggagtatgaaagcaatttcctcctccagtgcgcggggttcaaggctgatatgattcaccggggtatcggtagtacccatcactactttattgtgccagggcacaataaacagtacccttccatcgctggtagacgggatcatcagggcgttatgcccgggtagaaatacgctgtcgagtaccaggtgtactccctgacttgccgcaatagattttggcgcagccgggttatccatttccagtacatcatctgcaaacacaccggtagcattgatgactgcgcgggtgttaagatatatttcctctcccccgcccagggtatcctttaccgttagtccgctgattttcccaaagccgtcttttcgcaaaccggtaacacgcatatagttcagcaccgtaccgccattatctgaaatggactgcaccaggttaatggccaggcgtgaatcatcaaactgtccgtcgtgatacaacacgccaccagcaagccggtcctgcttcagggtagacaaccgctccagggtagccgatctcgaaatatgtacggacttccccaaactgagccggcctgccaaccaatcgtacattttgaggccaacagtatatttcaggttctcccagaaattaaaagtaggaataacgaaagccaggttacgtaccaggtgtggagcattggcagccagcaatccacgttccacactggcttcccttaccagcgacacattgccctgtgcgagataacgtacgcctccgtgtaccagcttcgtgcttttactggaagtggattttgcgaaatccacctgttccagcagcaaggttctgtaaccccgtgttaccgcttccagggcggcgccaagaccagtagcccctcccccgatcacgatgatatcccagggttcgagatcctttcttaatgaggtaacaagcatttctctgttcataagctagttttcattggtctgccaatcctatacaaaatactgaggaatcggataccggacaaataaagcagccgattccagaaaacttaacggccgggagagttaaaagttttaaattcaggaacatttaggcattaaaaatgttcctcctagagatcattcaattttacagcttcatatgtttaccaggattcacctcaattacagatatttttttcagctgctgatactgctggtagtgatggccgggagctacaacgccgatgcacaaagccgtaagcgtaagcccaaaaccgataccattcacctggtagctgttgacagtgctaccatcagcaagaatatccaggcgttatcgaaagataccaaccgggtaagaaagtcggacacgtctgtatccatcctgatcaaccgcattgagagttacactttgacgctgaacgaccttatgagttccctccgccgtgggtttgacacttcacggatcactgccggcctgccgctcacagatacttccctcgcgctgatcaggtacaatattgccagtttgggccgcacacccaatatcaacgacatatataccaacaaagtaatgctggagcaggtgcaacgaaagctcacatcgtggcagggcgcccttttttcctattacgagaaactgaaaaacattaacgacaccatccgtcttatccggggagataccgccatgcggaatatcccttctgaagatgagctgtatggtttttacctgggccaggtgaccaacctcgtgcttaaattccgttccgtagacagcgcgaataaggccagtcttattaagatagggctgctgcaaaaccaggtggcgaaccggtatattgaagcctccaatctttacgaggacatggactaccggttgcaacaatacgcctccaacatgtttgtacgggattaccgctacctgtggaagccgcaccgcgacagtattaacccgcttgaatttttcccggtactgaaaaactctttgcataaaagcacgaaagtgctcgacatctttttttctatccaatggcctatattctttgtgtggttactattggccatattattttcctggtgggtacacaacaatattaaacgcatccggcacaatcatcctgaacaggaaggggaaaccattctccaacacgcgcgatacctgtaccgcaacccggtggcctgtacggtggtactgattgccactttatcctccgtactttctgtacgttatcccattctttttacggaaatcacctggggtttaaatgtgatagcgctgacctttatctttcgcacacatcttcctaaaaccttattcaaaagctggttattactggccggcctgctgtttatttacagtctgaataacctgctgatagaggtcacctataccgaacaatggggattattgataggcgccattctttcgctactgctgggcaaccggctgctgaaagaatcgtcgcttaccacttttgcacaaccgaaatttacccggccggtactgatattatttatgatgatcagcgccttttccctgatcatggtaatttttgcgcgggtaggcactgccaaaatcatgggatctaccgctgttgtgagcacagtaatggcgcttagtttatttacgctggtaaaaatactgatggaagccgtttatctccaggtagaggccaataaagattccagcaccttcatttcttttatggactaccaggaagtacagaaaaaactgaggacattcctcacgatcctgggctttgtaggctggctggtaattttatcgcgcagtgtttatttatacgatattatttacgaggttattaccgatatcctctcctccaaacataagctcggcaattcggattttactttcagcagcgtcatcatttttatcctggtaatatgggtggctactgtggcttcgcagctgattgcatatatgtttggtaacaccggtcaaagcgccaatcccaataagaaaacaaaattcggttccgcgctgttgctactccgcctggcagtgcttgccggcggcgtgttgctggcatttgctgcctccggtattcccatggataagatcactattgtaataggcgccctgggcgttggtatcggttttggtttgcagaacatcgtgaacaacctggtatccggtattatcctcgcctttgaaaagcccatagaagttggtgatgtgatagaactgggaccccgttccggcgttgtaaaagaaataggcatccgctccagcaagatcaatgccttcgacggttcagaagtaattgttcccaacggcgacctcatatcccaacaactgatcaactggacccggagcaaccggaataaacgcataacaattgcgctgggcgttggctatggaagtaatattgaccaggtgaccgctattatcaactccgcctttaccgatcgtaaagatgtgcttactgctcccgctccttttatacagctgaccgacttcggagataacgcggtgaatttcaaggtctacttctgggtaggcgaccttgataatgcaggcaggcttcaaaatgaggtgatgtcgtttatttacaccgcccttaatcaggccggtattgaaatcccttatccacagcgggatttgcatatccggtcggtggatgagtcgttgttgaaaaaatgggataagcctgctccgggcgatcccctttaaaaaaagttctaaaaaaacgttggattcattttgaattttcatttttaagccgttatctttgcactcccgttttggagcagcaggcgctactgatagtagttatagcgatccggatggagaataaggcgaggtagctcaggtggttagagcgttggattcataacccaaaggtctcgggttcaactcccgatctcgctacagataacgagccgtaaattcttgataaaagagtttgcggcttttttgtttggagaagtggtcgattgattggccacactatcattcaaacaaaacatccatcttcaagctgttctgcacgagtgaattcgaataattatttttattcaatccaaaagttgttatcatagttagaaaaatagctttgcgtgtttttgtctcctctttaaaaatgccaatcttatttctcaactcttctgcatattttttgtcgattgtaaaattattaatagagaatttcatttcgcaaatattgatcacctgatcacgcctgtcaatcaccaggtcaatttgcgcacctgtatctgtactggtacttatccatgatgacgttgttgtttgcacaccgctgatacctagtgccttttttatttctttagtatgagcaaggcatacctgctcataagcatagccgctccaggaacgctgctccggactatccagcccattaatccaactattttcacccaatatactagcctttcttataaactttaaatagaacagtgagtaaaaatcagttaactgataaagactatttctttccttttttccgtatgagatatatttgcgaataaaatcactttcctccaattcttttaaaattctggtgacgcccccgcccgcggagagcttagcccctttgattaactccccgcgagttagcccttttgcttttttactcaacgtttcgataaccgcaatgtgtttttctgcattatcgaatagggattggtagagattatcaaattcggaacgaagcatttcatccttctcaaaacataacctattaatattctgggcggcactttgcgctacatctacctgttccaggtaaaaggggattccccccatgaccatgtacaattgtataatctgatacctgtcaaatatagctttcttatattttaagaagtcttcacactctttcaatgtaaaggactctaatctaatccgatgagtcacccgattatgcaaaccacctttgttattaatgagtttgttgatcatccatcccgctgccgaaccacaaacgattaataccacatcatttctcgcacttgcccaggaattccaaaaatgttccagtgcaagtacaaaatcagattgtgcggtatcaagccagggaagttcatccaggaaaataactttctttttccgcttactggattccagcaaaatagagagctgttggaatgcattgaaccaatcggcaggaggttttctttcatttgctgacgaatcatatctcgtcattgcaacatgaaaattggctaattgctgtgacaagttaacattagacatacctgtcagataaaaatcaaatttattatcgaaagcctgcctgattaaaaaagtcttcccaacccttcttctcccatacactgcaacaaaagaggaagatttgctatcttttatttgattgaacaaatcaagttcttttttacggccaataagcttatccatgtcattaaatttggccttaagtacacaaaaataaatagttaaggtcaaattgacgaacctaggagcagccaaattgcatgacaataaaataaaatattaattgacattcaattcattatctcctgtatttcagttaataatgaaatccgtagttccaacccatctcattcccctacgaattttaaaaggctatcgggcagattgggggtgtggcaactgtggttaccttgcccatgaagatgaatcctttgaaagaacatattcaacttgtaacaccaaaactgaatccagattagaagatgatgaaaaaatttactggtggtgttcccgtgaggtaccattaacttcggagaaatgatgtaaatgttcttttaacaggttagatattctgcccgttcgggctacgaggtctttcgtcagttggtcgtgtgcataaaatatttcgcttaatgtttcatccaacgcttttcctgacaatggtatcaacggggctgaacatgaaacacaggcaaaaaaaagctgcctgcaagagtaatggaacccttactaaaaaagaggctgtcagtctaagactgcctcttctacttacatctgattaatttcagctagtgacattgaaattatcatcgtacgccacaactccctctgatatcccccctggaaataactgtacctggaaatactcagtaggagcatatgtccattcaccaaaaattaatatattggaacatgaaaaaaatcatcctgatttcttttttactgatagcggcgatagcactgaacgcacagcaactgacctacaaaaaccccctggctgttgatttgggcgatccttatgtattacatgtcgagggcgacaaatactatatgtatgggaccggtggcgccaggaacggcttcgccgcctattcttccaccgatctggttaattggaaaaacgagggccaggtgtattttcacgataacaaaaatggctggagcgatccaaaagccgcctgggagggcgcttattgggcgccggaagtatatgctataaatgggaaatactacatgttttatagtgcccaatggaaagacaatccaacgaaggaactcgaaaactttcgcattggcgttgccgtggcagataaaccaaccgggccatttatcgatgtaaacaacaaacctgtttttgaccctggctatcctgtcatcgatgcaaatgtgctattcgatccaagtggaaaagtatatctctattattcccgttgttgctacaaacatccggtacagagtgaaatagctgcctgggcaaaaaataaaggctggttcaatgagatcgaagaaagctgggtatatggtgtagaattaaaaccagatttcagtggcgttatcggtgaaccggtgctgctattgcgcccaccggtgagcatgaaagataaacaagccgaatgggaaagccgctcggttacatccaaagaagtgaatcgccgctggacagaaggttcctccatcttcaaaaaaggaaatacctactacatgatgtattcggcgaattacttcggcggcaaaaattatgcggtgggttatgctacttctaaaagtcctttagggccttttaaaaaggctgctaacaacccggtgctgcaaaagaacgttgagcaaggcggtgtggtaacagggactggccacaatagcatcacgtattcaccggatggtaaagaaatgttttgtgtataccatggccgtacattggaaacgggtgataagcgtgtcgtttttatcgaccggatgaatatattgcctggtggaaaattggtggtgcagggcccaacaacagcaccgcagccatttcccggtggagccaagtagcattgatcttcagtaaatttttttagttgtaacaaaaacaacttgttcactaagtcgcctaaaatatagcgttatggatcatcttaagagagtctttttactggcaggcataggaatgtttttcagcattcacgggttttgccagcaactagccgatgccagctggctactgggaaaatgggaacaaaaaacgaataaagggactatttatgaaacctggaaaatcagtagtgattccagctacgcagggaaaagctacctgttgaaagaaaaagataccgttgttttagagactgttagcctgctggaaaaagatggcgctttgctttatatcccaacggtgaccaatcagaataataatatgccggtatcttttaaagtaacattttcttcagataataaattaatttttgagaatccggcgcatgatttcccgcagaaaataacctatacacttatttcatccgattccctgatagctgaaatatcgggggtaatgaataataaacaacagttccggcagtttccaatgagaagagtacaataacccttaccggtaagtcgcccatcccagccctaaaaatcccttatgcttttcaatatgaaaagtatctccttcttcaaactgcgcgtatgctgattccgatatatttttagcctgaaaaggaccatttaccttctgcattaaaaaataatactgacgtttagcgaatggcgtttcttttttagccaatatcatatattccgcatccccaaatttcatccttttatattgctgaccgccacgatattgaccataggttttctggtttacttctacccattgggcagggttagaaatactgtctacatgaatgagatcaaaataatattgatccgatcctgcatccccatgatcatatggaacgcttgcataatacttgtttgccaaaaaatatttctccaccgcaggattagacgaatcaaacgcataatttaacgtgagaaggaaagtcagtatgtaagaaagtaatccaccccaaaaaattcctttactcattacgggaacaggttcccggccaaataaaaaacaataaatgatggcgggcagaaaaaggctgacggaaagcgataaaaattctgactgatatacggataaaacatgaaacagtataaagccatacagacacggcgtgatcaggtcgagcagtaaattatatatattatccggcctgggtttaatgaaatagaaaagcagatgccttgcaactgaaataaggaataaaattataaggagatatctgaacctgaatgacaggggatcagtgtatagcaaattaatacccaatgcgagtctcaccatcgcaagaaatataccgccaattgaagccgctccggttggattaacaaacgctttattttttccgttactcatgtataatactataatggattccctttcgtaatacaatttaccatttttgtgcagcatttggttacaaagaaagaggagcatgttaaccataccggttacatacaaaaaagtatataaaaagagtcgcttccggaaaggatatagatttgccggataaaaaataacggcttttatgaacaagctacaaactaaaaaagagtggataacaactcccatactcccctgttcttccattgaggaaaccctggcattctgggaggtacttggataccgtaccacttataaactgacgcgcccttaccagtatgggatcagtgagcgcggtggatatgaattacattttgcccgtgttaaagatatgaatactgcttacagtggttgcctggtaacggttgccgatgcaagggcagtgtacctggagtttaccggaaaactgaaagcatcgcttggaaaggtgcctcataccggcattcccagaatttcgagaatgaaaccagatgccacacgctttacgttaacagatgtttccggcaactccatcatctttgttagttttggggagaaggatgaagaagtgtggcagcgtgcagacaacaaaaaccaaagcatgctgcaaaaatctattgccgttgccgccaggttccgggactacaaaaatgatgatgtggcggctgcgaaaacattggatgtcgcattagcccggcacgggaatgaatcaaatactgatatcgcggaggcattgatacttcgcattgaactggccggagcgctgaatgagcccgagcgtgcagcagcgtgcagattacagctggaactgatatcgctttcaaaagaagagctgaatgttttgaagttaaaacattcagtagcggtgtagtgtcatttcttccatttttgcgcaatctgcatggcggtatcaatcatataaggttcccagtgctcaatttgccaggcggtatgtgcaagcgaagaacccttgagcgatcgaatagcctcttcgcaggaggtggctgattccagtatatcagaaagttccagctgctgatggtgtaaaacttcatcttccacaacctcagctgttactatggggaatgatggtaaaaaagactggtaagatgatataccgggcatgcttttcttttttacaatattttccatctttccaaaatcattgtaaaaagtagttctgctttccgcggtggtaagggcatttccaagttgttccagcacaacatatttaagatgggggcaacgcgctatcgtgttttccagtaaatgaaatacttctgccggaacggcatcatcatgtgtatccctcctgattctcttcaccgggctattgggagcgtcctcccagctaccgccggaaatatgtatctcccttactttatctaacgggtagcgggtaataatttcttcgaacggaatattaaaattgtggatctggcaatagaggttgtgcagatcgaggatgataaaaccatttacaggttccaggagttgttccaaaaaggcgccgtgacgttttacctcgtcgagcgaataggaaaaggccaggttctccagtcctaccgggcattcacatgcttcgtagatccgcttcagtctgtctctcccaatgtcgagtgtggatttcgtatagggaatattcagcggagcgccgtgatgaaagtctttccccgtcatgaagccaaaatgttccgttacatgatcaaaccggaattcttccctgacccttttcaattgtttcagccaatcggcttgctcctggcgccactttcctgaaaaaagggaaaagaatacgccatgaccaatcagtcgttgttcatcgctgtaggctgtcagcagttcaaggaaccaggatgggatctcctgcactttaaacaatgcgtcaaacgaccattcaatggcttgcagtcttgatgcttccattagcggaagacatgctgccagtatgtcggcgtccaggttgcaggcggctgctgatagaatttccggcaccttttggaattaaatgtgaatgataaacgatgggctcaacccattccgcaggcagggcaaccattttcatatggctttttcacttcttccttcttttcctttggtttaactgatttatccttgttacaggaactggttgtttgaacggtgataccaatcaggatggcgccgagtaatgattttggcagtttcatttgatattatttaagggatgaaatgctacaatatgcttgtcaaaacaagattacctgttaaacgaaggcgaatatgaaaaagttacaggaaaacagatccttaacattggggagccgctgtaattatcatgagcctgaaggaagatgacaactgcaggagaggccactactcctgcagttgttgcttaaaacttaatggtgaggttagccgttacgcgtgttgggttttgtgctgccagccggttcgaccagtacttttcattggtaatgttatccacttttaccccgatgcggtaaacgggtttgtcgtagaacagggagccatccagcacggtgtaggaaggtatggtaaaggcgaaggtgttggtgttggtttgaaacgactggctgccatagttgccgccgaaagcaaagcccagtcctttggctgtgccacgcaccaggcggtagctcacccacaggttggctgtggtggctggtccggctgaagacggccgcagtccctggaatttagcatccgccttatccattttactttcgttataggcatagcctgcaatgatatttaatcccggaacggggttagcaattacttcggcttcaaagcctttgctgagctgggttccatcctggagagaaaatccgctgtgagcgggatcatcatatacggaattggtaaccgaaatatcgtagtagctaagcgtagcatttaatttctcattaaaaagatctgctttaataccaccctctatctggttggcctgttgcggtttaaacgtgttgccgctgtaatcagtacccgactgattctggaatccgttcatatagttggcaaacacggaaacccggtctttaatgacctggtatacgacgccgaatttaggtgataaagctgtttgggtataatttcctgttgtaagatccttactgggataataagcaccgagattgtggtagttatccagcctcaggcttgccatcaccaacagctgctccgtgatattgataacgtctgagaaataggcgctgtaagtgttttcgcggttactgtcgaacgccaggaactttaattttgcgaacaatggtgttacattatccttattgaaattatagtaggcatcaccgggagttctgtaattgatggccggcatattcacgatggtatcattccgcgaggcgcgcaggctataaaaatccacccccaccaccaaccggttacgcattttaccgatatggaaatcgccgataaagttttgctggatatctgtaccgtagtatggataggtttgcgaggtaactgcctgccgcagggtgctatcgcttaagatgttcagttgggtagtgaatccgtcggagctggagcgggtgcgggaaaatacggtttgcgacgtccagcttccggacagtttatatttgatctggccaaaaacgtttaactgctggctgttatagctcatggtattgttggcataggagagtttatagggcatgcccagttccgctacgctatgcgcctttccttttgtgtaaggactcaccctcatgggagaagtagctttgtaaccgctcatttccacgtccagcaaaatggtgagccggtcgtttactttataggaaaagctgggcgcgagcaaatagtttttgctgaagccggcatcctggaagctacgttcgctatggatggcgccattgaagcggaacagcgctgttttttcctcatttacgggagtgttgatatccagtgtgaggcggttcaggtcccagctgccaccggagtaagccacttctcctttgaagctgtcgaacggctttttggtaacccggttaaacagcccaccaaaagaagaaagggtgctgccaaataatgtggcggaggggcctttgatcacttctatgcgttccaggttagcgggatctacattggtatacacaaaactgcctacgccgttgcgtaccaggttggcggtggtgaagcctcttgatgtagcggagcttcttccctggttgtaaacaatgggaatgcccgcccccggaatatttttgaaggcgctattataatctgttaccagttgttctttcatcagctcttttcctactacgctgtatacctgtgggttttcgagattttttagcggcagtttggatacatcttcgctttcctttttggcaaagcggtttcccccggtggccaccaccacttcttcgaggttttgggaagatgtttttagttctatttgcagcagtacgcttttgccgtttactacagcaaccgttcttctgatggtttcaaatcccaccatagatacctccagctcgtagttgccatccggaatatttttaaagaggaattcgccgctctggttggtgatcattccttttgaaatgcctttcaggataacggttacgttggttgccgggtgaccgtctgatgtggtgataacgccctgaatggtattgttggctccttcgtccggcacgccagcatatatcaaggtaaatgggagtagaaaaagtgctagaaacaggtatgcccttgtcatgttggtcttatcgtttaccatgcaaaggtgcattgagaaaagaccaaattatctactgtatcgggaaaacgatttacgcaatcgggaaataattatttatgcacagcggcaaccggttgactggcggggtgcgtcaacgcaaaatacgccaccagcaaggttagccacgcttatcattcttcaaaagccttagatccctggcggacccaaaaggtccaccaggatgaccatataaagcaaatccctgccactacccattgaagggcggtgggcaacaagcgtcaaattgtttaaagtaaggtttcccggattacaggtgggcaggtgtaaaataaccgcgtaaaatctttacagcagtaccaatctggtttttcaccgtttgaatgctggtgttcatctcttccgctatttctttatggcttttctgatcgtagtgtcttaaacggaaagccgtagaggatttaggcggtacttttttcttcagtgcgatattcacctggcagtaaatttcttcgctttccaacggatcgtttggtacaaaagcttcatccggaataacacaggaaaatttcctttcccgcgtaattttgttaagacagcggttccgtatgctcgcatacagataacttttcataatacaggaactgtcccggttctggtaattagcatcaatcttcaggaacaatttcttctgccagaagtccagaaaaaattcctggagaacatcttttgctttttcttcgtcctttagcatatctatagccagcagtagcaggatgcggctatattttttgtacacacttgtaaatgcttcggtactaccatctttaagcagttccagcaggacggcatcttggttgttatgttgcattctcatttcctttttgagagactggtttaggaaaaatatttcgacttttattgacaatacaggtgttagaaaatcaagctttctaatggtttactacggtggttaaaagtggtttattttgcattccgtttttctaaatctggaataaaagtaacgttataaaacatcccgactggttaatccattgttaagcacgaatgttttagaagtggtaagattcaatgccatggctgcttggcaaggaaaaattaacattaattaaaaatacaatgtaatttccgtgggtgaggcctgagggagggcttaacgggcgtagcaatagcacccggaaggacggattaaccggcccggaaagaagaagagaaataagagaggaattatacggataacttcagaaaatcaccgtctatgatcaggagtttaacaccagttgttgaaactgaacggtgactactcagatcatctgtcaccacataactcatgccttcagataattcaaagttttcaccactctgcaactcgcttacaaaagcaccttgcaggcaatgtacaatatgcccttttctgcaccaatgatcagccagataaccgggagaatactccaccatccttatccggagcccggggaactgcaatgtttgccaccacgcggtaccgttttctcctgggtggactgttttcggaattaatgaccaatcgatagcttgaaagggaatattgctgctcatggtaaaataacttaacgtacacggatatacgcttccaggatttcctggttaacgttgaggctatcaatcttttctataccacgctgaatcagcgtatcatgctgtaggctaagtgtgaaagtgaaatgcatgtcttcccaggcgcggtagctgcaatactgcaagtgctcctcgtatttgtcgcccgttaactcataagtgcctgcaccggaatcgaaaacagcagtgctgctgtcgcttcctttcgaaacatcatgcttgaaaaacgcaaaatgactgccattaaacattttgatcatctcctgaccttttacgggatacgtatcagtggtatctccgttcttgatcatcttactgtatgctaatttccacgtacctattaaagataacgctgtagcagcttccggcgcctttgcttccccgcaggaaacaatggtccatccaataataccaataatggcgggtaatcgcaggttcataacgttcagatgtttgagtgaaaagttaataaaaagatgttgattttaaaatatatggtaaaataaaaagggaacaacatagtgatatgctgttccctttctttcataaatctgttacatcaccggattacctgcaactggtcactccctgcgggcttatgcagtaacaggttatatatcttatacttattgtcggtaatgccagccagggccgattctcccctcagttcatcatccgtgcggatcaatcccactaccctgccgtcgccaaaaaagcgcagttcataatgctccaatggcagcatctccaggtgataagccttgatctggtcaaaccggttccaggtttctgctgcatcagcaggcttgttctgaaaataagcctgttctgtttccagttcccggttgtagatcagctccgccacggcattcatgttaccatctgccatcagtttgcggtactggttgtaaaaggccagcacttcttttgtgagctgcgttttatcttctttccgcagatcctggctctggctccatcccttcagctggtaaggggtagaagcctcaaaggtgcctttaaattcgaggtagggtacattatccagttttatctccggcattttataataaaagagttgtttgtattctttaggcttttctttttcttcatcgccatacagcacctttacctccaggccgcagttctttgccagtaaaaacggttccattttatcatcgtcatctacttttgggaataccctgatagtaatggtttgcttaccgcttttcaggatattgggagatattggccatacagcaccgccctggttcccgccgccaaagtccgaataggcgggcatatcgttaaccagtatttcataggtacaattgtagctgttaaaatccaggataaaacgcggattatagtcgtatttttttaccagtttataactgttcagatatttttcctttatgccctgattcatgctttctttttttgcatttgttccctgcccgcagctatgcaggccgatcagtaaaattaatgagatgatgattgctggtttactcatccgtccgattctttttttgttaagtatatttttttcaaagagatctttttctcatcgataccgatttcaaaagacgctttgggattggcttctaccagtttattgtactcggccggtttctccggggcgcctttcttcttctttacctcttttgttttttcccctacgttcacctttgcctccacatacccttcaatttttatgccttcaaaaatcaaatcaaatcctacaaataatcccgcgtcatcagaaccaatcctggcctgcaatcccaggccggaacttccttccagtcctattcccagcgccactactacttttaccttgaatgcggtggccgttttactcagatacagtttacattccagcttcactgacactgctgcccctccctttatcaggtcttctttcttttctgatgcaccggctgtccgggtgaatacattccctcccaccgtgttatgtttaaaggtggcttccaggtctattttaccggagagggttacactgatatccactttactgtcgtcgtctgcacatatgtacagcaacgcgtctacggcctttaagatggcataggcaatggggtgccggcggcaaagcagttccaggaaatcccacttcaggtcgatccctaccaacggtttggcatccagctttaccagcacggttttgcccgcgccccacaacttgctgtcgcctttttgtggcggcatggtttcgtagtaccacgaagcggccagccccagctttggaaactgcagctcataatcaaatggcttgcgctgcatccgctgaataagcccctggatatttttatcggggttccctttgtttttattgataaactcgtcggggtctttcccgtcgtcaccggaagtatccgctttattggtatggttgccatgaataatattcctgaactcctttaccaggttccatccggccttcagcacattgtaatatttggcgatcatatcctcaataggatccacgctctcggtatcattattccattccaccttgatggagaaatcaaattctttcagcagctccaccagctctgcaaacttgcctttcgatttcaccggggttggcgccgcctttttatcttttggcagtgcaaacatttcacccaattcagtacctaactcttcattgtggcggtccagcgtaggtgtgggcttgctccagcggcctttcgcagcctccccgatcttttccacgccttccagccggttcatggtaaaccgctgcaaggcattctttattcctttaccattatttgcttccgcgaatttggttttcagcgcatcaaaatcggctttgtccatgttaaacgccagggctgctgtccactttatatcgggatacaccgcaaagtcgataacatgtttccagcgacaggtttgtatagttaccgggaaatggtcggcttgtgccgcaggaatccacaaatagcccaggatccgctcaaaaagcacatgattgttttcatcaaagaaattatacttgtactgcgcatcaaattccagttcttcatccgatacctttatcacaccggaaaaagaagcgttggtatctcttttaaacttatagttattggcctttatttcaaatttcccctttgcggcactctctttttctttctcccgtttcacaccggccttcacgtcttctttcttatatcctttggcgccaaagctgctcaggtctattacatggtccttatgcttcggtgacgctgtacattcatcttcatgcgtcaccaggctttgcacgctgagcttgatggttttcttcgcggtatcacttcctgccacgatgttataggtaagattttccgggggctgaaagtccagtacgttttcatcaaagatggtttgtgtgccgtctttgtcttccacggtgatcatgccatacttacaaggctggaacttgcgcgtattggtaggaatatctcctgccagcaccggcttattaccgccatacatcaggggagattcttttactttgggatcttcctttacattaaggaagcacttcgacaatgttttagagagcttgccatcgcgtgtttttacgatgggatatatttccagtacttcgcctgcaccgggcttccagaggtcatcgaggaaaacgtctaccactattttttgcacaaagttctggtaggtgatggagccggtggccaccttcatatctttccccgacttatcttttattacaaaatcacttgtctgcagcgtctccccacggctggtttcatccgacagcatgggcattatttttacctgccgggtgaaatatttgatggcatcatcgggtgtttctttccccggctccttctgtgcttctcctgcaacccgctcccagggtggcagatcatcatccgctgtagcagtatcattgtccatcagaaaaatccgtagttcctgcccgtacaaggcgcgggtataaatatgcagctgtacactttccctgaatttcttagtaccagcggtgataattttaccgtcattattgggtgtaaactcccgccactcggccgacataatcgccggctttccgcgcgcagcaataaagtagccatgtgccgctgaattggtaggttcatgcccgtcgaggaaaggctccagccaaccaagtccgccaccttccactatcttcgggaaattgggatgcaccaccggcccgttcagtgcttcgttcacatccgttttcttaaatgtaagtgtgcgcaacatcgaccagatccagcggtaaggggttttatcaccttccggcattttcatgggaacgctgatcttggcaggcaccggcagtttttccaccatcgtggtaatgcgtttcatttctgcccgcactgttccggcctcgtttaatacggcggtggaagtttttacatctaccgatcctttcgctgccgggatggtgactaccagctttttattatcagacatggcaactatttttaaaacggttgtccctgtggaaaccggatcagaaataaatcttcttctactttctgtacatccatcatgggattcaggtgtgtttgtacttccttgtcagctttctccgcatccttttttgtcatatcggctgtttgcccgtgaaaggtgatagcgatacaatcttttccaccggtggcgcaggtcgccttactatcttccagcaaaatataagcatctcccggtaataccactttatcataaaaaccgctccaggccgtaactgacggcgtacagggagtattattctttttactgcaactaccaaaggtattggcttcaaaaggctgaccaatatctttggtattccccaacggtttctctgcaccgtctttgtcgttgatataatgcacctgctgactcttcactttcaatttatccggggcggtaccaaactggcacttacaaacggcgccctggcaaaccagatgtttttcgctcatatctttttaattttccctgcggttgaaaaagaaggaaaaaaggcttttcttcttcccggacaactccttctccggcaacagcactgacattgccggagcctgcgttttatccttttcccgcaaatgatagatcgtaaatgttacttttttatcctggtcaggtgtgtgctgcaaactgcattctcctgtgatggcattgatcgaataatcggtctggtataatttataagtgatatccacctgcccttttgcaggtgtgtgaataccatgtaactgccgggacaagggaatttctttttccgcggaaatgtcttccgcactacgcgggtcactgcaactacctttctgctgaagcaccaaactaccgctggcggtattgtgctgtatgggttgctgtgtaacgttatacagcacgggcgcagtataaggcattaccggcaatgctgcagtgagctggcgtttcatgatatcgctgccgggctgatacaggtcggcaaaataaagggccataaaccaatcgcgacacagcgactggtaaatatgtggttcgctgcttactgccaggtccatatatgctattatttcgtctgtaatatcgccggtataatactgttgaatgtccggtttggcggcagcccaggcagcagcaatctgtaactggttggcgatgccggtaaattgcccggcttcgttcacctttatctgcaatggatacaatactttcccacattgctctgcaagcttatcaatcattttttccggcgcctggtcattcatgtacacctgtcctttattgatttcaaacaggaacatattaccgggtaatcttttggagcagctcaccgttatctcataactgatcgcctgttccctgccggccgattgaataatataggttacgccgtaagttctgctgagatgtaccgggttaaaccggaaagaacgattactcataggtatgctacttttttttattcccttcagtaatcagttgcgatacctctttttttacgcttcccacgtaatgcctgatagctgccggaatgcggctggtgtcggcatctatctggtacgacatagggggccttttatctttaaacccaacttccactatgaccaccggctgctctccgcaatacaggcaaccccagctatgggtagtagtaccggcggttaacaacagcgatgggatggaatccagtacaaaacggcttcgttgccattggccggaggataaagtttgcacggacgaatctatttttacgccagtggtatccagccagtatcgctccagtacttcaggcgtaacgcgatacttcacccggatgccggtggagaaaacaccaaagtgaacccaggccactgcaccggttccgggttttgtttgtgccggtagtatatccattaccgttagcatcaataaaagcgtaatcaaactcccgcgcatactagtaatttaaaattaaactccggtcctgtctcatgatatcccactggaacttaaaaaaggaccgcatattatctttggcattgtgtggattcagattaccgtttgtttgccaggtataatccatgatgttgtcggtatggccctggtaaaaagtgtagggtggcggctttagtcccgccataggctggccggcgctgaacgtatgctgcaggcccagcgaatgccccgcttcatgcaacagggtacgccgttgattgagccctttcaggaatacaacgaaggcatttccccaaacaaattcctttataacgtctccgtcggcggcagcagcgatgccgttaaaatcggcgggtaaatccgtgaggaatatataggtgcgtttgttggcatcggcgttaatgcggccgccattgggtttgtgctgcccgtatttttcatacagcttcatcacttcctccaggaactgttgctcattgaaggctgctgctccgccaagaacattgttccaatagctggtaacgtcatggtcggttaaagggagtacgccggtttcaaaaatggtgtcggttttaatttcggcgcggatgagcgcctggttatatgaacctcttttaaactggtattctatgtcctttaccatttgctgatcaatagcaggaagactgtttgcctgtgtgcctaccttcaccagtatcagctccattttgggaatgacgtgattattatacaccatcagcttgcccacttcttccttcttattgcccagttttgcaaacacttttatttcttcatgctgttgcagcggagcattggcatttactacattcacggcgcctttcaacgtatagtacttaacttttacgccgcctggccggaagcgcgtttgctggccgcttcccattaatgcagcgatatttactttctgcggggttattttcaggttaggattttttgattcgaagataatctcggtaccatcgctgactacttcctctatctcttccagttcaaggtccagccgggcgccatctttattcatggaagaaccgtatttaaactgttgtgaagtagtataaggaaaaagtgacaaccaggcggggtaatagtcaacgccgtatggcttcaccgggttctttacacctttcaggtattcgctttttgcggcggctacgtcgctaaccagtggcactgtgctgttacacggctggttattattatcgcgttcaatgtaaataaggggatagatatattcgtcccggagccagtcgaacccatattcccctttgtaacccgccggccgcctgaagtgtaccaggaactttttcagttccttctcttttgctggcggcgccttatacttgtcataaataattttctctgtgctgcgcagttttacctggctggcggcattcaagctgatatcgccattggtggcataggtagttgacagctcggagctttcaacaatcgtttttgctactgagatcatatttcccatctgtacctggttgtggggttaaaacattttcgccttgtcgccgcttttgttcacgatctgcttggcgctgtgcatttcaatattttctttggtactgttcatactcactttctcggcggtcttctcaatatttttagcagtgcgctggagtgtatcatccgccacctctttgatattggcagcaagcaggctaaagtccttcaccgcagtttgcgacaggtttttaccggcgcttacctgtatattttcttttgccgtaaagctgatatttttagcattgatggtgatgttttccatcgcggcgatgttaatactttgggcactggtatccattgtaacgatgttaccggatttatcggtgatggtgatgctttctgccccatcggtatcatccaggcggatgatatgcccgctgcgggttttaatgaccttcaggttattttgcgcgtcaccgaagcccgttttcgcgtttccattatacacggtgccaagtacgactggcacttcaggattacctccttcaaaatctacccatacttcctccccgttttcaggtataaaatagaaccctttctcagtacctccatgcggggataccaatcgtagccagggcgtagttccttgttgctgccattgaaattttacccgtacacggcccagtcctttggggtcattattatcggtcaccacagcgctttgcgcttcacataccggcgtgcggtacaggtctacctccggcatggctgctgcggcgggtatggcttcaaaggtatttttatataatccgttttctgtgcagtagtgcgcgagttgagttactacaaactcgccatggtgctcattggaaagtaccgattcattaacggtaatgatatccccgatgcgtaatgcactttgctggctggtgcctttcaggacggccatttgcgaaagccttcctttcttttgtacctgcgtatatttatccagttgcgattttgcagcggtaccaaacgattggttcagtttatactgcgacgtttttttatacagccgttcacttacttctttcaggtggctcgtatatacgtcggtgttacctgcgggcaccgacagggtatcgttgcttaccgcctggttttgccggtaatcatagccatagaagcggctattgttggacttcacggtaagatcgaggttaaacccgatcaggtctacctggtgtgtaagcgttgtcttctgcggacggtaatttccaaacaccaccttctctccatcataaaaaaaccattccccgaaacgggcggcgagcctgtctataaactcgtaggtggtttctttatattgtacaatatatttcagggcatcggtatgcgccggatctaccgcgggcgatttggcgtaaggcccgcatcccttcagggcttcattcacaatagccgacaatgttttctgctcataacaggcaatatgttcatcatcttccagcaggatagttacactatgtcctttgatcacgcaaaatccgtgcgtaccatcggtttcctttcccatgctgataccactcacaataccattaaaatttaaaggcttgtatacggcatttgattcaacaggttttacagagatagaaatttcttttcccaggaactccttaccggcattaaacaatccttttccgagtttggtaagccagtcgtacccgatcatgatctcaaagctatgatggccgcggatagtctgatgcaaggcaagggaatgaaaagaagtaaactgatgatcaccaatagtgaatgaggtgtgcgtatacaatgacatttcgcagcttttacggttttaaatatggttatacctttttatcaccatagaaatgatatcgggtaactacttcaaaaaattggaattaatatctgctgttgccattaacgggttaaaacacgcaacaggagattgacatggttacagtcagcaactaatatacaacaagtgtcacaatttcaatcatacgcgaacaaaaaaataacgctggcgatgcgataaaataaaagagctctgccgttaaataataagcaggacacctaatgtttataatcaaatgttcaacagtgatgaaagattaacttatctagcatgccaacactcaccaaacgccagtactgttattgaaagcagctttcaggatacagccggtaatttatcatgtaaagtttatgaaataacgattaatttaacccctgcttctccgtacggaggaaattgcattttatacaacttaaaacggaaataatgaatctgaaaggatggatgcttgcctggatagccattacaggaagcatagcagcagcggcacaggaatatacattgcgttcgcccgacggcaaaataaatatacgtataaccgtaagggatagtatacagtattccttatcctacaatggccaggtattgttgcagccggccactatcggcgtggctacctctgttagccctgatggtaactggaaagttgccggcactaaaacgtcgtcggtaacacaaacgcttcgcccggtagtaaagcagaaaagtaccttcattgaagatcactacgatcagttgcagctcaattttaaaaaccgcacctccctgcaatggcgcgcctacaataatggtattgcatggcgatggctcattaataacaaaggcgcctggcaggtggtaaacgagcaggccggcttcgccctccaggcgaaagacagcgcctggtacccggttgaaagcgggttcttctcccataacgaacgcctctataaaaaactgaccatagatagtatccgcggcccgaaaagcctggccagcctgcctgcactgttcagcgtaaacggcgccaaattactgatcaccgaaaccggtctccttaatcacgcaggaatgtggcttcagggaaatggcagcaacacactggaggccgtatttccccactacccgataaagaaaaaagtaacctccgaccgtgatgaagaagtggaaaccagggaaaactttattgccaaaaaagaaggcgcttcccaattgccctggcgcattgtgatgatagcaccggaagataaagacctgctggtaaatgaacttccttatcaattggcggaaccagctaccggcgactacagctgggtgaagcccggcaaggccatctgggactggtggaacgataataatatttaccaggtggatttccgggcgggtgtcaacaccgacacttacaaatattacatcgactttgccgctaaatacaaactggaatatgtagtactggacgaaggctggagcgatacccgcaacctgctgaaaacagtacccgacataaatatggaagaattatcgcgctacgcggcttccaaaaatgtaggcatcatcctgtggacgacgtggctggcactggatcagcagctggacgccgcaatggaacgctttgccaaatggaatatcaaagggattaaggtcgacttcatgcagcgcgatgaccagccaatggtgaacttttatgaaagggtggccaaagccgctgctgcacataaaatgctggtagacttccacggcgcgcataaacccgcggggctccaacgtacataccccaacgtaatttcctttgaaggcgtgtatggactggagcaaagcaaaggcgatcaaagcaaatccattgcaccggatcataacgttacctttccctttatccgtatggcagcaggaccggcggactatacacccggcgctatgctgaatgcacaaaaaagagactgggcaccacattacagcaatccaatgagcatcggtacccgttgccatcaactggcaatgtacgtggtatatgaaagcccgctgcaaatgctggcagataatcccacgcactattacaaagaaccggagtgtatgcagttcctcgaggcggttcccagcgtatgggataccaccattgccctgcaggccagcgttggcaactatatccttaccgcgcgcaaggccgctaacggcgattggtatgtaggcggtatgacaaacttcacaccacgcaccttaacactggattgttctttcctgccggaaggtacctatatcatgcatgtctggaaagatggtatcaacgccgacaggaacgcacaggattataaaatggaacagataacggtagataaaaactcgaaagtaccggtagtaatgaacgttggcggcgggtgggccgcaaggatcgtgaagcaacaataaaataacattgccggtaaaccatttatattcactttgcaatgatgaaccgtactttatttttagctgtcctgggtagtctgtttaccagtagcgcaatcgcacaacaaccgatagatgtacaggcacatcgcgggggaatggccctgatgccggagaataccattcccgctatgatcaacgccgtaaaattaggcgccagaacactggaactcgactgcatcattacagcagatcaacaggtagtcgtatcgcacgatgcgtatatgtcggcagaatttatgcgtaagcctgatggctcggatatctccaaagccgaagaaaaaagcctcgcgttgtataaaatgtcttacgacagcatccggaaatatgacgccggtacaaaaccacatccccgctttccgcaacaggaaaaaatgatggttcaccggccactgctaacagacctgatagatagtgtggaaacgtatgtaaaaacacatcacctcaaaccagtgttttacaacatggaaaccaaaagcgctcccgatggcgatggcatctataatcccggaccagcggaatttgtagcccgcgtaatggaagtcatcaacaggaaaaaaattacggaccgcgttattatccagtcgttcgacatccgcacactccaggaattgcataaaacccatcccggtcagaaaaccgctttgctgataggtaacaaagacagcttcagcgacaaccttgagaagctgggattcacgcccaccatctatagcccgaactacctgttggtaacgccgaccctggtaaaagaagcacacgataaaaaagtggcggtgattccctggaccgtagatgacgaaagcgaattaaaaaaactcatctcctggggagtagatggcattatttccaatgcacctgataaactcataaaactggtgggcagctaccagaagtaatacttactttaaaataaagcgcgggccgacaaatgatgtcggcccgctctttactttttattcttatctatgcattttctttaaactgttccagcacctgcccgatctgcttcaggtacttcccataactttgtttgatccatatttccgttaaggcggtaatcagtaacaccagcaaaacaaaagctgcagctaaacccagcgcaattccccggtgatcagcagcctttgccagcaagctggtcatctcgctgcttttatgactcaccatgtacataacgccaatgatcagcgcaaaaggaagcagtgtataggtgtaagctttatacatttcaatattcagcctggcctcgtaatacaaagcatatagattgtcttttgagctgagggtatttgtaccaagactcttataaaaagtattgaacttataataatattgaacagagatggcgatcaccaccaggtacaccgcataaaaaggcaccaccatcacgggatcgagtggaaaaattttaggtgtaaacgctatcagtaccaggctgaaaagctgtacaaaaaattccatttgcatcgctttacgcagtttttccaccggcagttgtaaagtttttaactggtctacactggaaggaaccactacattgccgctttcattatcgttgttccatgcagattttatatcatcaaaattcataaccttgttttttaatcagttcttttaatttgtcttttgccctgctgagcttaattctggcatttccttcggagatacccaggttttcaccgatctctttgtgggaataattttccaggtgaagaaaaaccaatgccttttccaatctttccagtttctgtaccgccctgtaaaagtgtgccagttgcagttcttttgtagctgttacattttcttccatggccatgtgttccggcatggtgtctgtaacagccatttttcttttttcttttttgaagaataccagtgcggtattcagcgcaaccctgtacatccaggtggagaagcggctttggtgctgaaaggagtcgtaagatttccatagctggtagataatttcctgtgtcagatcctgctgatcatcttcagcatccatatacatcctggaaatcttatgaataattcctttgtgggcttcaaccagttcaagaaattctttttccttgtttttcaatcggtgatagctttagttcaaaataggtgtaaccgtatatcctttctctcttaataatttaatcaatccgatagggcctgcaagatgggcgccgcccactgcaaagaaagtgctttcctgctgcatcattccgggcattttatcaacccagtttttgttccgcacttccagcatccagtgaatggtattttcatccatctggtccggagtagtcatcaggttgtacatattactcagctcttctgctttataggctgccaccagtttgttcatgtttatactgctgctgtcgaaagcctttacctgttcaacaatttgtttatcggtataagatttcagcaggtatcccacctgttcttctaatccttccaggtaaccgacatgcttcttatctgcctgcattgtttgtataaaagtagtttcataagattttaattcctggcagggaaatgatttcatggccagcagggagatagtagcgaccagctgatagttttcaaatggcgccaaaggcacgccacatttacttttcaggatagaatccacgtcgtggtagtcggcaggagataattttttactcaacggcacatcagacgccatggctttagccataatggtgttaatattggggtcgaggatattggcttcaatgaccagttgcgccgacttacttaatgcctgtttggttttttctgttactttaaaatcattttcacaaatcatgtggatggtgccatacaaataagagggcttcgataatccgttaccgctgacttcccacaataatgatttgtcctggctggttggctgctgtgcaaccgctttacctgcaaataagcctgtgattaccaatgtagctgctgcgatattcctgaagatatttttcatatgcttttgattttcttttcagaattagtaggcgatggaatcacttcgttacagattatttcaactttttttcaaaaaattcctaaaccagccaccagtaagagaaaggtctgctttgcagcagaccttttcctgtaaaagaggtatccttatttatcagcgggcaattcggccctgcgggtaacgatgtggttcaggttatgatggatcattttctccagcaggtcgtagcctgcattaggccgggagtgcgcatattccctttccagtttggtgatgggggccagccagtataagttcaccttatcgccatatacctccggcagcccgatggcggggccattatataaggcggaggataccactacgctctcgaaaggcgcaggtagttcctcagagctcaccgtatggccttctcccagccaggtaacctgtttccagggcctgtcggccatatcagacatcaggccggccatcgccatgatctctttatccgtaaaatctttgctgctcactgccatcgccagttccatccggcgaaacccgggtgcccggtcgctgtacaggagttctacccatggcatcgggcggatactaatccccagggtgagcaggtataccacctcatctttctcaaatttacccaatgccatcgggggccattgtccgccgtcgatggcgtagtacttctggatgggaccaaactcggcttcataggctttcagatactggtcctgcaaaatgctccatgcctggctggtttcgccttcccagtctttccagaaggcaatggcctggtctacgcgctcgtacatggcgttggcgccccgtttgcccagtggcatcagccggtcgttttcgccggcgccggtacaatcagcagcataggctaccgcgtgttcgtcattatacaaactccagcccggtatcacacccagtatttcattatcatataataccgctgctccatctccctcttccgtccatacaattgttatacgctctttttccagcggttcacggccttcggggtggttgcagtaggctgcttccaacataggcgccatgccttctttcatggctgcaacgtctttcgatgcgggcgccggctgcaggttacgtaaccagcatggtcgcggcgaatactttgtggtcaacaattccgatggatacaggtaaaaataagccactctgtcgtcctgctccactacggcatataaagttcccctgttattaggctggtctatcaacattaccggctcagacataattattcttttaagatcgaaaaataacacaatcccggcaatactataattcctgcctcaattgctgtattttgtcaggtatacaattaattttttatgaaaagatattccaccctgttaatggcactcatgatgttttgttcagctacactcactgccaaagaacgacaattttatcagatcaaaatctaccacctgaaaacaaaagcgcaggaaacactggtagataattacctggaaaaagcatttctcccggcattacaccatgcaggcatcaaacaggccggcgtgtttaaaccggttactgccgatacggccgaaatccggatctatgtattgatcccattccagtcgctcgaacagttcaccaacctggataaaaccctgcaggccgacaagtccttccaggctaacgggaaagactatacggatgcagcctggaacaacgttccttttaccaggatagaatccatcctgttacaggcgtttcccgggatgcccgtactggaggctccctcattgaaagctcccaaaagtgagcgggtatacgaactacgcagttatgaaagcccttccgagaaataccacgtcaataaagtaaagatgttcaataccggcgacgaaatcggcattttcaaaaacctcaactttaatgcggtgttttatgccactgtcatttccggttcacgcatgcccaacctgatgtacatgaccactttcaacaataaggaagaccgcgatgaacactggaaggcatttagtgcagatccgaaatggaaagccctgtcggcgctggaagaatacagtcacaatgtatctaaatcagatatcctgttcctgagaccaacagactattcagacctgtaataccatggagtggcaggcatgcacctgccactccatttatcatactgccaccgtagccctcactgttccctattaccgccatggctttgtttccaggccggtaaatgctgacccacatttgtcgtaaaagtataaataatatttctacagacaacacctccccgcgcaggcgcttacctgccccgcccacagattaaaaatgtgcgccgataattaaacaaaaaggcttaatttaactgctattacacccaccggcgggagtgaaaatgagccaccacacatttttgctcccggtcaatgacaccacaattatttaaaattcaaaaactgatccccacatggctgatgaaactcaacagaaagttcagaccgcactaggcgacgtcgccgcaagacagcttgccattgccacccgtacggtcccgcaaatgtctaccattaccccccgctggctcacgcgattaatgagctggatcccggtagaatcgggcgtgtacaggcttaacaaagtaaaagatgaaagcaatgtaaccgtggattgttccggaagggatgaacgcgaactgccgcaaacctttgtggattacattgataacccacgtgagtacaatctcagtgcagtaaatacggtgctggatgtacatacccgcgtgtcggacctctacagcaaaccttacaaccagatcagcgaacagttgcggctgatcatcgaaaccattaaggaaaggcaggaaagcgaactgattaacaacaaggaatatggtttgctgaacagcgtaatagcctcgcagcgtattaaaacacgcaccggcgcgcctactccggacgacctggatgaacttatcaccaaagtatggaaggagcccggtttctttttactgcatccgctcaccattgccgcctttggccgggaatgcaccagacggggtgtgcctcctcccaccgtttcccttttcggctctcaatttattacctggcgcggcattccgctgataccatccgataaagtgcccatcgaaaacggtaaatccaagatcattcttttacgcaccggcgaaagcaggcagggagtagttggcttgtaccagcctaacttaccgggagaacagtcgcccgggttatctgtgcgcttcatgggcattaaccatcaggccattgcttcctatctcgtatccctttactgttcactggcagtattggtagacgatgccattgctgtattggatgatgtagaaataggcaagtaccatgaatacaaataatttccaacccgatggattaccggatattgccgcattggaaaaactggccaaccagttgttttcctccctgcaatccggtaatgatgcgccctccgcaggctacgcatctgctgcccccatccaggacccgttactgcaacagggaagcgtaacggatgttacgcaggcgcccaccagtttaccggatcctcacttttccggtaacggcggcattcctgcttctgtggcaggcagcggtatttcaccggctgcgctcacgcatccaacaacggcgtatgatccttcttttgaacaggaactgcaacgggcactgaaaagtataccgtcatccacctatacatcgcagctgccttccgcaggcacctcctactatttcttaccggaaaaagcagcaggtatcaccggcgctacccagcctccgttggatatcaaccgggtgagggcggacttccccatattgcaggaacaggtgaacggccgccggctgatatggctggataatgccgctactacgcagaagccgcggagtgtcattgaacggatcagctatttttatgaacatgaaaattcaaatattcaccgcgccgctcatgaactggcagcacgcgccacagatgcttatgaaggcgcccgcgaaaaggtaagggcttttctgaatgctgcctccgtgaatgaaatcgtatttgttcgcggcgccacggaagccattaacctcgtcgccaaaagctggggcgaacaattcctgcaggcaggcgatgaaattattctgagccacctggagcatcatgctaacattgtaccgtggcaacaactggctgccaaaaaaggattgctgataaaagtaattcctgtggatgacgacgggcagatcatactttctgaataccagaaactgcttggcgctaaaacaaagctggtgtcttttacacaggtgtccaatgcactcggtaccgttacaccggcccaacaaatagtggaactcgcccaccaggcaggcgctaaagtactggtagatggcgcccaggcggtatcgcatatgcgcgctgatgtacagcggcttaattgcgactggtacgtattttccgggcacaaagtttttggccccaccggcatcggcgtattgtacggcaaagaggcattgctgaatgaaacacaaccctggcagggtggcggtaatatgatcaaagatgtaacctttgaacacacccaataccacgccgcccccgggcgctttgaagccggtaccggtaacatagccgacgccgtaggactaggcgctgccattgattacgtaaatcatataggcattgatgttatataccagtatgaacattacttgctcgtatatgccacacagttattgaaagacatacctggtttgcgcctgataggcaccgctcccgataaaacaagcgtgttgtcttttgtgtttaaagatttcacaactgaacaggtgggtgcggcgctcaaccaggaaggaattgcagtaagatccggccaccattgcgcacagcccatccttcgcaggtttggcgtggaaagcaccgtgaggccatcactggcattctacaacagttgtgcggatattgatacgctcgtaaatactttattaagattacgaagaagcaggatataattttttttagaaagaagagatggctggcagtttattcatatcaaactattagtcatctcttcgatcaaaaatatttttcatctcacagaaaataaaaaagaagcgcaagaccaattccatcaaacgcgctacggcactacattataccggatctgtttttccacgcaaaaacctcattgccctggaacatgcggctgtgctcataaaaaacaacatttaaattttgtggtttaaattatttacctacatttgcactccacaatgcgaggtagagcagaggtagctcgtcgggctcataacccgaaggtcagtggttcgaatccgctcctcgctacaaaaagtaaaagtcctgtactgaaagtgcaggactttttttataccgcaacagatcgaaaataaatagtattattacaacaggccatcaatacctgaaagcagtttttgttagccatcaacccaatccctaaacaaattttattactcaatgaaacaaaaaccatcaatggcatttattgccgcctcctgggtagcggtatttgcaggtatcctgggctttatcatcggcctgtggaatgcatccactatgcaactgaatgaaaaaggatattacttcaccgttttaatgtacggcctgttcgcagcggtatctgtccagaagtgcgtgcgcgacaggattgaaggtgttcccgtaaccgacatttattatggtctcagctgggtgtccatgttgcttaccatcctgttgcttactatcggattatggaatgccacccttgcaccaagcgaaaaaggattttacgcatttgcatttttgctgagcgttttcggcgctatcacggtacagaaaaatacccgcgatagccaggccgcgaaagcaggcaacagtcccgtttccggcgatatctaatactttcttttacagggaggccggttagtctccctgttactccccccctctttttccggaatctataaatacttttcctgaatcgtcttccacagcaattgctgcggcggtacatttacattgtcacctgtggacatgtgcttaaacaggatatcaaatattatatctatcctccaatcccttataatacatctcctgaagtgattaacagtattcctgctaatcacttttttttgcgccatattataatatatttgttgatagttaacctttttatccatatgggaaacaaaacctatactgctactattgtatgtattgcagcaatggtggttatttttattacagtgcgaactgtgcgtaaaagcagccagccggaatatttgtcaaatgacaaagccggagcagctgccgctgttgcgctggatgaagcgacagtacaggccgcagtggcggtagacagcgttacctatgaaatgaagaccgctgcagaatttccgctcagcgtttcccagctccgtgatgctactgcctatctgttgcatgaacagctgcaactggacagccatgtggtgaaaaaaaagcaaacttttgatctcgcactgatgtggcattcatatgtacaaccgctgtattatgaaggagaatcggaagatccgtataacacaaccgcctatacgaaaaatcacgggttagagcccgctatccggcaacttgcctggactggccgcgatgaggcccggctgcgtgcatccttcgccagttataaaaacctgttatacgaaatgctgccgtataatacttaccaacgttccccggcacgttattatgtggaaaaattattactcacttatagcgcactccaggcaaatgaaaacgtaacggcacagctggaaaaactctatattaagatggccatcagtactgatcatggcccctcagaaaatttcattggagaggtaagacaggtgttaagtagcatgattcgcgtagatccttcactgaataacaacgacctggatgcacaccggatgaccgtttggctggtttctttctgggcccgacgctataacgaaggtaatcagcaggccgtttatgaaatcctgaaagaaatcagcgatatgtacagccggtgattgatccggtatatcccttcgtttgacccggatctcaaaaaaaaatgttaaaaatgatttcatttaatacaaataaatattacttttattccgggcaagagaaaaagtgctgcgttatttgacttgttatttaataaaagattcacatggatcttttttttggaacctattgctaaatcgattttttaacggagactatgataggcgtcgggaaatctatgcattacacaccgcgtatgaacgaaaaaaatatagtaattaaaatatattccaggtaaaaaagctaactgaacttgttattcttattgtttgctaaatcgatatactactgactaaacagtactgtaaggatcgtacattttgcttatgcgaatataatgggaaccattgcatgcctgaccggaaaccaggcagcatcttcattcaggagatatttttcactatttaaatgataaaaccagtatctgaaaaattttaaaaatcagcctgtaggcttattgctaaatcgtttttcctaataagcaacccggcttttctttattaaccaacttcaattaacgtatatgcacaaacgatccacgttttgggcacggacctgctttgccagtatggtactgatgctcttctcgctgtttgccttttcacaaggcaaaaccgtatccggaaaagtaacggatgccaatgacaacaccgcaattcccggtgtatctgttcagataaaaggaaccagcagcggaaccatcaccaaacccgatggtacctttaccctgcaggcgccggaaaatgccgtgctgatatttacttttgttggttacctcccccaggaagtaccggcatcagctaacgccatgaatgtaaaactggcagcttccgtaaagtcgctgcaagacgtagtggtagtgggttacggtacccaaaaaagaaatgaagtaaccacttcagtagctactgtaaaggcggaaaacttcaaccagggcggctcccgctctccaatggatctgatccagggtaaagtagccggcttatccgttaccaggacccaggggaataaccccaacagcggcgcttctatacagatcaggggtatcagctccatatccggtgatatgaagccgctgatcgttgtggatggtattcccggaggcaacctcgacctgctgcaacaggatgatatcgctactttcgacgttttgaaagacggttccgcagctgctatttatggtacccgcggtaacaacggggtaatcctcatcactactaaaaaaggtaaagcaggtgatccgcagtatacttactctacctacctgcaacgcgaagctgtggccaaaagacccagcatactcagcgcagcagaatatgtaaaagtggccggcgccaccaacgaccagggcgccgatgtggatatgtatgatctcctgctcgacaaaaacaatcttagtcattaccacaacttcgcagcctccggtggtactgcaaacagcaactaccgcgcatccctttattacaacgatgccaatggtattgccctcgaaaacggccgtaaacaatacggcggaagggtgaatgtaaaccagaccggcttacagggcatgctcaccatgcagttcaacctggcaggcaatttcagtaaagccaacttaaacggtggaaacagcggtgacggtgataacaaagccggcaacccaggcgccgattttgagcaggcagtacaacggaatcctactgcgccgatttttggacctgatggtaaatatgttgaaacaaacggtttcaataactacaatccactggcccgcttacagcaggaattatacgaaagggatcagaaaacctattcaggagatgcacgtataacgctggagcctattcaggatttgaaattttctgccttcggcgctattgtccgtgatgagtatactgaccgccagtataaaatgaaggcttcccgctcttccatccaggacttccagggtggcggttatgcgtataaagccaattccgccgctatggataaaacttttgaagctacggtagactatacaaagacaatcaattcagaccatacattcaatgtgctcggcggctacagctatcagtacagcaccctggaaaagtatgccatggataacaacggcttcctcaccgatgcgtttgaagactggaacatctctgcaggtaacgccttaaatgatccaaaactgccacgccctacacagagcagcaacaaggtagacaataccctcattgcattcttcggcaggataaactataactacaaacagaaatacatgttgcaggctatcctgcgccatgaaggttcttcccgcttcggtgccaactacaaatggggtaacttccctgcagtatccgccggatgggtgatttcaaaagaagccttcatgcaggacctcactgttatcaaccacctgaaactgcgcgccggctatggtgttaccggtaaccagggtattcctaactaccaatccctgatcacattgggaacagggggcgcttacctccagtatggtaaatggatccagacttatggccccaataaaaatccaaacccggacctgagatgggaaaagaagaaagagttcaacgtgggtcttgatttctccctgctgaaaaacagaatcggcggttccgttgatgtatacagccgtagaacagaagacctgttattcaactacacggcacagctgccctccaatatcctggataatatcttcaccaacgtaggggagatctccaacaacggggtggaagtagtgatcaatgcggtaccggtaagaagcaaagatttttcctggaacagtgatctcgccttcaactcccagcggaataaaatggtgtcattctccaaccagatttataaagccactgaacagttttatggagatctcccatctccgggtaatcttggccaggccatccgcgtagtagaaggcggtccgctcggcactttctatggctaccgctacgcaggtcttactgacgacggcaaatggcagttctataaaaaagatggcagcaaagccactacttctgaaatcaatccggacgataaaacagtgatcggaaatggtattcccaagtacatggcttcctggaacaatactttccgttacaagaactttgacctgagtatcctcttccgcggcaaattcggtttcgatatcctgaacctgcaggatatgtacttcggtaataaaaaatggaaaccgaataacatgttatcatctgctatcggtaaaaatgataagctgaatgacgatccacagttctctgattactacctggaaaaaggcgatttcgtgaaactggataacatcaccctcggttataatttcaaactgaaaaccaaatatatccgcaacctgcgcgtgtatgcgagcggccgtaatatcgctaccatcaccaaatacagcggtcttgatcccgaactgcaggatactgcgctggattccggtatagatggaagaggattttatccacgcacccgctcctacactatcggattgaaccttggattttaaaagcagcaaaattgtaacgtatgaaaaaaaataaagcatatatcagcgcagccttgctggccctcggattgagcgcctgtaccaagctcgatgaaaaaccatacagcgaaattatttcagataatttttatcataataaagaagaagtactgtctgccgtactgcgtccgtttacgcatgccggcgcatgggccgctcctaccggtcaaaccggctactggcgcctgcaggagctttccgccgatcagctggcatggccgcagaaaggcaaacacggttatgatggcggcaactggatccgcctgcataaccatacctggattgccaatgaagacaatgcctggaacccgtggagactgatgtactggggaatggggttctgtaacaatacactggtagatctggcggctatggacttcactaaaattggtatgaccaatgaagacaaagcctcctttattgcagaaacaaaagtggtgcgcgcctggcattacctgaaactgatggacctctatggtaacattcccatcgtaacagaagtaggtacaccggcatctccggctaccaaaacccgcaaagaagtatttgagttcgttgaaaaagaactgaaagaaaatgtggaactgctgaaaccattatccgcagacatggtaggccgcgccaccaaagcgggcggctatgcgatgctggtagagctctatctcaacgcacaggaatggacaggcaccccacgctgggacgactgtgttaactattgcaataagatcattgcaggcgacggcggctccctcagcggcgctgtacccgcactggaaccggatattttccgcgcttttgccaacaacaacaatacctccccggaagacctattccagctcgcctatgacctgagagccggtaactcccgcttcggatggcaaggtgatttttggcactaccgtcaacgccaggtctacaacgccgacgtagatggaaacaatagtatcgttgtagttcctactgcttatgatgcgtataaagacaatgacctccgcaagcaaaagtggatgctgatcggaccacagaaaaaagatccggcactacgcaccagcgttgcagacagtttggtactcggcacagaggaatacaatggaaaaccgcttgtatttgtgaaagaaatccgcagaaacacagaaggagaaagcggcgccggtggcatgacgcagggtgaagagaacagcggcgcacgtttcgcaaaatatgttcccggcacacaaaacgatcctaactactggggcaacgactttgtattataccgtttgacagaaatttatttcaacaaggcggaagcactgatgagaaaaaataacggcatcgcaacacaggatgcagtagatcttatcaacacctgtaaaaagcgtgctttcaaagcggaagactgggcagcagaggcttatacccctactacgctcaccatgaatgaactgcttgctgaaagaggccgtgagttcatctttgaaggtaaacgccgttcggatctgatccgctttggcaaatttaccaccgccacctggtgggatcatcagccatctgctgataagtacaagttgttcccgattcctttcaaacaaacaagtattaatcctaacctggttcaaaaccctggttactgataaactggttgggtaaagtagtaaacgactttaacctggatgcggaaaacccaaaacggccgtctcttaattgagatggccgttttcaatttagtatcgtgatggtcaataggctagcagttcgctgatagcagctgctacttttgcaggcgtgggcaacatggctgcttccaggccggtgttaagcggcactgccggcaaatccagcgcccccaccgtaaatacaggagcatcgaggaaccggaagcatgtttgctgaatgcgtcctgccaatgcctgtgcaaaagaattattgagttgttcttctgtaaggatcaggcatttcccatgttgcttcaccatgtcaaataccagttcttcatccaatgggaaaagggtgcgcaggtccactatggttacctggccaggataggccttggcagcagctttggcccagtaaacgcccattccgtaagtaattatgcaaagcgcattgccctgagcagtatcttttggatgtgcgcgttgtattatatttcccttccctaacggcagcaggtaatcagctgcaggttctatggtcatggcatcgagtgtaccgggtactttgctccagtacagtcctttatgctccagcatcactaccgggttgggatccaggaatgcagctttcatcagtcctttcatatcggcagcattggagggatacaccactttgattcccttaacgcttaacagtgtggattccacactgccggaatgataaggaccgccaccgccataggcgcccaccggaacgcggataagggtttgtacgggaaatttaccattgctcaggtaacacgactttgatatttctgtaaccagttgattgaatccagggtagatataatcggcaaactgtacttccacaatgggttttacgcctacggcagatagacctgcagtagcgccaataatgtacgcttcctgtatcgcggtgttatatacgcggtgtggtccgaatttttcgcccagggtggccgcttcgcggaacacgcctcccaaccttacgcctacatcctgcccaaataaaatagcttccggatactgctgcataatctcttccacagcgtgaagggctgcatctaccattactactttggtcttaccggctggtgtgcgggtaccactttcagctgttaccgcagcaggcgcaaatacgtgctcctgcaccgtttccggcaatggttccggggcatgtacagccttgtcaaatgctgcctcaatatcggccgcggcagtctgctcaattttgtccagctcctccggagtaatgccgtgtttcaacagcagcgctctcattttaggaaccggatcattggctgcatgcttttccaggtcttccgcggagcggtaccattcttttcgcacgccggaagtatgatgtcccagcaggggtacatttgcctgtaccagtataggccgtcgttcttgtcttacataactgatagcggtttccatcgcagcatagctggcggtgaagtcgctgccgtctacccgcatgcgttccaggcctttaaacccggcagcatattcatatgcatccattgttcttacttctgccgccgtggcggagataccccaatcgttgtcctgtaccaggtaaattaccggcagctgtttcagaacggcaaattgcagggcttcgctcacctctccttccgttacgctgccatctccgagtgaacagatcactaccggcaattccccatccggccctgttttcagcaggggagaatgtatttgttccaggtattgcagtccctgcgccatgccggtggtggggatcacctgcataccggtggcgctgctctggtggggtatctgcggtttatcggccgctctgttgttagggtgactgtaataagatcttccggcggaaaaagggtcttctcctttcgccagcaattggagcattagttcataaggggtaaaaccgatggcgagcaacatgctctcatcccggtaataggggcttacaaagtcccacggccgcaattgcagtccggtggctatttgtatggcttcatgtccgcgggaagtagaatgcacatatttgcagatttgccggtttgcctcataaatggcggccatactgccggcttcacacatcaatcgccaggctgttaataactccgcccgttcgccggcgttactacccctgttggaggccggcgtttttaaagttgaaacgcttgtgttatctttaaacacagtaagactgttttggtgatgatggtaatttaaaaacaatagttgccatagcaacagttgctaatgcaaattaattaatatgcctgatactttcgtcagtaatccctctttttttaagttggatgctacgctcaaaaaattgcgcaactattggcaaaaaacgtttgatgcccaacagaaggacattacagtggatcagtggttgctgattgagaacctgtataaacacaaaaaaactacccataacgagctggcccgtaatacctcaaaggatattaccaccatttcccgcatcattgagctgctggtaaaaaaagggctggtaaaaagggaggccgatgtgtacgatcgccggaaggtatatttacagctcaccccggacggagtggaaaaatataaagatgtaaagtcgctggtatacgatatgcgtaaaattggctggaaaacgctgacagaaacggattatgccgagttaacccggatcctggacacgatttatgcaaatattccgtagcgtaggttgtctttctcaggattacgctgattttactgattagctggatttttacttttggattttttttgatttttagatttaataataattatgggagataagagcgaatatatccgcttctatctcccataatcctttataaaatccaaaagtaaaaatccagctaatcagcaaaatcagcgtaatcctgagaaagacaacctacgctatctaacagagaattccagcaggctgtcgttttcaataaatgcctcgaagtcgtctccgatttccgttggtcctacgccggcgggggtgcctgtaaaaatgaggtcgcctatgttcagggtaaagaagcgggaaatataggctaccaggaaatcgaaggagaacaaaagatcctgtgtattaccggattgcgccaatgccttgtttttatacaggcagaaattgatatcttttttatccatttccggggtaatagggatgaaattacccaccactgcggaattatcgaaagctttggctatttcccagggtaatcctttcgctttttgcttatcctgcaaatcccgggcggtaaaatcgatacctacggagatatgatcgtagtacttatctgcaaatttttcctggatatgtttaccgtttttactcaccctgagtaccagttcgcattcgtagtgcaggttggtagtaaattccgggtaatagaacgggtgcccgttttgcagcaacgcattctttggtttcataaataacaccggttctgtgggcacttcattcttcaactccctggcatggtcggcataattcctgcctacgcaaataattttcataatgcgtttgttttaaagtataaaaaaagcagataggaaccagatgaacaaatttatttcacagacgggaaggtcagtttattactgtcgttcatagtacgggcaatgccgatactggcaaaactttcaatgatatccgaacatttccatattttctcttctacaatccgttcttctgtatttttccatttactgagtacaaattccacctggcggcccttgggataattattacctaccccgaaacgcaggcggggatactggttggtacccagggattcctggatacttttcaggccgttatgcccggcatcactgccgccggggcgtaagcggagcacatccagcggaagggccaggtcgtcgaggatcacaagcaggttttccacgggtatcttttccttgtccagccagtatttgatagccttaccgctcaggttcatgtaagtggtgggcttaataacaataaacgttttccctttccatttacattccgccacatcagcgagccggtcgttccggaaggaggctttatgcctggcaacaaaatcatctaccacatcaaaacctatattatgacgggtatgccggtattcctcgccgatattgcctaatcctgctattaagtatttcatacgggtcgttttcgtacctggagatttccaaaattaaaaagcccctctaaaagtagagaggctttttggaaaaatatatctaaaagattatttctttttagcatctttttcagcagttgcttcttcctgacgcagctgacgggtcattaccacagaagcgattggaatacgcggagagttggtgatttcaacaccttcaattttcacgtcttctacacggatgttcgcgttcagttccaggttatcgatgttaacttcgatattttcaaccaggtgcttaggtaaagcttttactttcagcgctttcagtttgctaaccagtttaccgccggctttaacacctgcagaagaaccaaccagtttaattggaatggtaacagcaacctgtttgtcttctaccagttccatgaaatcgatgtgagcaagtgcatcagtaactacatcaaactgcatatctttcaatacgcatctgtaagttttagcacccagtttaatttctgcaatctggaaagctgcagtgtaaaccagtgttttgaatgctttggcaggagctgaaaaattaacagtttctgcacccccgtaaataacgcaaggcacttgttcctcagaacggatctggcgggtggcttttttgccgaattcgctcctgagttgtccttcgatggttattgtgttcattgtttagacaatttatattgattattaaaatactatgttatcaatctccccggcggtgactgtgaataaacaggctggtgattgatttgttttcgtgcatgttacggatggctaccgcaaaaagctctgcaacagatatcaccttgatcttggaaccggctccctgtggtttgataggaatggtatcacataccactatctcctgcagtactgatttttcgatattttcgtacgcatttccgctgaaaacgggatgggtacaaaaagcacgtacactccgggcgcctttttccattaacaggttggcggcttttgaaagtgtgcctgcagtatcgcagatatcatcaatgagcacaatgtccctgtttgtcacatctcctatcactaccattgatgctatttcattggctcgtttacgatgtttgtcgcaaataaccatttcagcattaaagtaagacgctacttcacgtaccctattggtacttcctacgtcaggggacgcaaaggtaagattttccagctttaaattctctatataaggaataaaaatagctgaactatcaagatgatctaccgggatatcaaagaacccctggatctgaggtgcatgcaagtccatggttatcaccctgttagcccctgcagaagtaagcagattggccaccagtttagagccgatagccacgcggggcttatcttttctgtcctggcgggcgtatccgaaataaggaattactgcggtgatatagccggcggaagcccgcttggcagcatcaatcatcaacagcagctccagcaggttgtctgaaggcgcactggttccctgaatcaggaaaacatagtcaccccggatactttccaggaaaacaggctggatttccccatcgctgaatttctgaatctttactttgccaagaccgccattaagacccttgccatatttcttggcaattttctcggccaaggccggattactgttgcctgtgaaaatttttactgaaggttgcatactagatactagtggaaaagaggttgcaaaactaggattttttgggagtacccgcctgattttttttgaaatacaaattatatagctgttaaaaaccagctataattatcacattatcataacgttttaagagataataggtcccgaaaaattcctataacgatcggtaccgaatataacgattttataacgatccactggtaaaaggaaaagaaaaatgtggttggaagaacaggtgtgtcatgataggttcgtatatttggataaatggaataagtcatgtttgttgatgttaacccggctccccacctggctattcataaatggccggataatgaaaagccaagagaaaaactgatcaatataggccccactgcgctaagcgatgcagagttactggcaatcctgttgcatacagggcataaaagcaaatccgcccttgagctggcaaaggaaatcctccgcctggccaataacaacctctccgaactgggaaaaataaacgtaaaaaagctgcaaaaaatccggggagtgggttatgccaaggctgttaccatactggccgctatggagctggcccgcaggcggcaagccggcaccatccataaaaaaacagtgatcaacaacggatcggatgcagccatgtttttcaagcccatgcttgcagaccagccctatgaaaccttccatgtcctgttcctcagccacgccaacaaagtgcttcattaccgccacctcagtaccggcggcatcaccagcactgtcgtggatccccgcattattttccgggaagcactggatacaggcgccaccaagttattactctgccataaccatccttccggcagcctccgccccagccaggccgatctccggattaccagccgcataaaagatatgggaatgctcttcgatatccaggtaatggatcatatcattgtatccgaaaccgggtattacagcctcgcggaagaagggatgatataaatcccgaaatgtgttttactttcgcacatatttattcattttccatatgctcaaaataggactcttcggcgtaggacatttaggtaagatacacctctctcaactggccactatgaaagacgtagaagtggtaggcttctatgatcccaacaatgcaaatgcagccagcatctccgagcaatataatattcagcggtatacaaccgcggaagaactgatacagtcggtagacgccattgatattgtggcgccaaccaccctgcacttcaaattatgcgaactggccatccgcaacggcaaacacatattcgtggaaaaacccatgaccaacaccatggacgaagccaaaacactggttaaactggtggaagaagcgaatataaaattccaggtaggccacgtggaaagattcaatcccgcttatctcgcactccggggatatgatctcaaacccatgttcattgaagtacaccgcctcgcagaattcaatccccgcggtacagacgtaagcgttatcctcgacctgatgatccacgacatcgacatcgtgctgagcatcgtgaaatctaccgtgagccgcatctccgccagcggagttgctgttatgagcgacaccccggatatcgccaacgtacgcatcgaattccataatggctgcgtagccaatctcacttccagccgtatctccctgaaaaagatgcgcaaaatgcgcctcttccagaaagatgcttacatcggcatcgatttcctcgataaaaaaacagagatcatcaaactcaaaacaccggaagacgaaggcttgtttaccctggatattgaaaccaacagcggcagaaaaacaatcgccatcgataacccggaaataaaacaatccaatgccatccgtatggaactggaaatgttccgcgacagcatcctgcaaaataaaccggttgccgtaaatgcgatcgacggcctgcaggcaatggatgtagcccaccagatcctcgcaaaaataaataaaggcctgtctgaaacggcctccgctaaatagttatgctggtaacccggcgcaggtaattatgccggcagtgatacacttaccaatcgccgggttactgcattcgtcgtttttgtcaatactgcaaaagcagcaggctttaccggcaggtaacgttatctcctataacaggcactttagctgcgctctttcagcaacacttctgcaatagcaagatcaagcggtttcgtaattttaatattggactcttctcccggcagcagatgcacaggataccccagccgttccactacggtggcttcatccgtaaacaacggatcatagggcagttcaaaggcaggcaggatcaactccgaaagaaatgtttgcggcgtctggataatcctgaaacggtcgcggtccacagcagcattgctgccgcctgatatctcccggatactgtctttcatatcaatcaccgggatagcgctaccatggataagtgcggcttcataacaggcacggatcaacgtagtagataccagcgggcgcaccccatcgtgtacaaataccaccgacgggtgttttacctgctgcaatccattctgtacagaatgaaagcgggtatttcctccttttataatggtgatgtccggcagtttatcaaaagcctgcaggatgtggttggcgaaagtaaaatgagcttcaggaagcaccagcacaatttccatatccggaaaggcggccgaaaaagcggcaatagtgtggtacaatacaggtttaccggacagttccaggaactgtttgggaacagcgctctgcatccgggtaccggacccgccggcaactatgatagccacttttttatattccataaaaaaagatcggggattttctcatccagttggctgaataagaaaatccccgaaaagtgctttgtaattaaacgatcagcatggcatcgccatagctgaagaaacggtatttctctttaatcgcctgctggtaagcctccatgaccaggtcatatcctgcaaaagcgcaggtcatgatgagcaggctggttttaggcaggtggaagttcgttaccaatgaatttggaatagcaaaatcatatggcggatgaatgaacgtattcgtccatccttctgctgctttcagatggttttgcgcagttacggaagattctacggcacgcacagaggtagtaccaatagcgcagatcttgcggttttcttctttcgctttgtttaccactttcactgcgtgttcttcaatatgaaaatactccgcatccattttgtgtttgctcaggtcttccacttcaatagggcggaaagtacccaaacccgtgtgcagcgttacttctgcaaacttaacacctttaatttccaaacgtttgatcaactcacggctgaagtgcaaacctgcagtaggtgcagctacagcgccttcgtacttggcatacacggtctgataacgctctttatcttcgtcttccggtttgcgtttgatatacttaggcaatggcgtttctcccagctgatcaagcacctgtttgaactcttcatcattaccttcgaataaaaaacggatggtacggcctcttgaagtagtgttatcaattacctctgctaccaacgtctcgtcgtcgccaaaatacaacttgttgcctacgcggattttacgtgccgggtcaacaattacatcccacaggcggttttgcttgttcagctcacgcagcaggaatacctcaatttttgctcctgttttttctttacggccatataaccttgccggaaatacctttgtattgttcacaatcattacatccttgtcgttgaaataaccgaggatgtccttgaatactttgtgctcaattttgccggtattacgatgtaccaccattaaacgtgattcatctcttgtcttggtagggtgctgggcgatcagatttaaaggaagatcgaatttgaactgtgatagtttcatattacggtatgaataaattttagaggtgcaaagttatcaattattatctacatcatcaaaaaatgatgtataacgtataataaccagataattatatattatattcctttaggaatggctgctatcagttgttgcgtatacgggttttccggatggttatacaccctgtcggctgcgccctgttctacaatctttcctttctgcatcaccatcatccggtcgctgataaaccttaccacggaaagatcgtgtgaaataaaaatacacgtaaagcccagctcttcccgtaaacggatcagcaggttcagcacctgcgcctgcacacttacatccagcgcagctaccgattcatcacagatgataaaagagggctccaccgccagggcacgcgctatcacaatccgttgccgttgaccgccggaaaattcatgcggataacggttaaaatgttccggcagcagattcaccttctccagtaattcctgcacttttgcttgctgctgccgctccgtaccatacaaaccatgcactttcattggctccaggatagcggccccaatggttttccggggattcaacgatgcatatgggtcctggaaaatcagttgcatatccttccgcagcgcacgcatcccggtggccgacaaacttcgtatatcctgtcctttataaataatacttccggcggttggtgctgcaagtcttagcagcgaccggcccaaagtggttttaccacaaccagactcgcctaccagcccaagcgtttcaccggtgattacccggaaactcacatcgtctacggctttggcccattgcagtactttacccgtgatacttcttttcacgggaaaccacgttttcagctgatgcacctccagcagaggtggcgcggctgccagctgttgctcccgctgccgcagcgctgcgtcggggattaccagcgactgcatcacatcccggatggcgcctgctttttcgtgtatctgtccccgtgagtccgtctccataaaatcccggatcacgggcaatctcaccaaacgtttatccagcgggggccggcaagccagcagtccctttgtatacgggtgttgcggatgcaggaacacctctttcacagttccttcttccacaatattccctttatacatcaccactaccctttccgctatttcagctaccacgcctaaatcatgggtaataaaaataacgctcatctccatctgctgttgcagttcccggagtagttccagtatagctttttgcacggtaacatccaacgctgtagtgggctcatcggcgatgagcaggcggggatggcaggagatggccatcgcgatcataacccgttgtttttgtccgccggaaatttcatggggataacggtccatgatcgctgcaggatcagggagttttaccttttggaagagggcgatcacttcctcgcgggcggccttgcggcttatgccggtatgcaaccggatagcttccgccacctgctctccgcaggtatgcagcggattcagcgccgtcatgggttcctgaaaaatcatggcaatttcgttgccgcggtagctacgcatggtagcatcgggcaactgcagcaggtttactgctgtttcatccgcagcctggtaaaggatctttccaccggagatggtaccaggcatatcaatgagtcgcatgagcgaaagggcagtaacggattttccggaaccggattctcctactacgcctacaatttcaccctttcctatggaaagggaaatctgattaacagctgttgttgttgtttgtccggacctgaatgttacctccaggtcctgtatctctacccgcgtggaaagcatacccggaagatacaacaattctaaaaacgcaggtgcttcacggtctggtgactttcaatcagcttctgtaaggagtcgatgcctactttaagatggcgttccacaaatttagtggtcacctttttgtcgctttcttccgtttttacgccttccggcaccatcggctgatcagataccagcaataaagcaccggtagggatcttgttaaagaaaccaacagaaaagatggtggctgtttccatatccactgccattgctcttatcttttccaggtattgtttaaatgcggcatcatgctcccatacacgcctgttggtggtatagcaggtgcctgtccagtaatcgtaaccggaatcacggatcgtggtggaaatggctttttgcaaagcaaatgcaggcagtgcgggtacttccggggggaaataatcgttgctggtaccttccccgcggatagcggcgataggcagtatcaggtctccgatgttattcttcttttttaatccgccgcattttccgaggaataatactgctttcggggagatggcagataacaggtccattacggtagcagcacccggacttcccataccaaagttgataatggtaatatcacctgccgtagcgcattgcataggccggccaacgccaacgatttccacgttgttccattcggcaaacattgttacgtaattactgaagttggtgaggaggatgtgggagccaaattgatccagtttctcacccgtgtagcggggcagccagttagctacaatttcgtcttttgtcttcatagctttttgacaagcaaatataaggttttgttcgctaacctcaatattatcctaatgtaactatcttcgcaacggtattaaatcagttatatcttgatcgcgatcagcttccctccacccgatttcaaaattatgaaagaaggcagcaaagaactcatctttgaccgcttccgtaaaaaatatgtggtactcacaccggaagagtgggtacggcaaaatttcctgaactacctggtgaaagtgctgaattacccggcatccctgataggtattgaaaaggaaatttttctgggagagatgaagaagcgattcgacatcgtgatctacaaccgtgcaacacaaccctggatgctggtggaatgcaaagaaatgaatgtaccgctcaccgagcacaccatgcagcaggtgatccgctataacatggtaattcccgccacctacctggtgatcaccaacggcctgaacaccttctgcggcaattacgtggcggccgaaaataaatggcggttcctgcgcgagttgccggggtttgcttagcgcgccttcggcgcgggaaattgtcttggagcaggattacgctgattatactgattagcttgattttgattttgtttgattttataaaggattaagggagatagaagcggatattttcgcttttatctcccttaactattataattaatcaaaaaaaaatccaaaaaatccaaatcaagctaatcagtataatcagcgtaatcctgctccaagacaatttcccgcgccgaaggcgcgctacgcgcatcaagggaaaatgcccagttgctcgtaagccgcacctactttgttaatggctactacgtaagcggctgtacgcatatcatggatctgcgggtttgccatcattacgtcgcgtacttcgtggagtgcagcgtgcatggtttcttccaggccggaatataccaggtctacttcatccgcaccatgggcaatgaattttctttctttatcagaaacagttttgccggtcagctcttcgatggtttgcaggatatgaatgttcatattttcatcgaagcgtttgcccaaacggccgtaacgcacgtggctgaggtttttcagccattcgaaataagaaacggttacaccgccggcgttcaggaacatatccggcaccacgatcacgcctttcttattcaggatttcatccgcttccggtgttaaaggaccattggcagcttcaccgatgatctttgctttaacgttgggagcattgtgtttatcaattacattttccagggcagcaggaatcaggatttcacaatccagttccaggccatctgtatttttattgaggttggtagcaccggcgaagtttacgatagaaccggtggcttttttgtgcatcagtacttcatcaggattcataccctgttcgttatagatggcgccatcccactcgatcaggcagattactttggcgcctgcttcatggaagtatttagcagcgtggtaacccacgttacccattccctgtacaatcactctttttccttcgatgccggtagtaagaccaaggcggtccatgtcttccttgatgttacacagttcgcgtaaaccgtagaacacacctaaaccggttgcttctgtacgaccgcgcacaccgccctgtgatacaggtttaccggtaacgcaaccgtagccgtcaatttctcccgggcgcaggctcatgtaagtatccaggatccagctcatttctctttcaccggtaccgtaatcaggagcaggaacatctgtacctggtccgataaagtttttctttaccagttccgcagtataacgacgggtaatcgcttccagctgaaagggcgtatagttgcgggggttgattttcaaaccacctttggcaccaccaaacggcacgttcacaatggcgcatttgtaggtcatcagggatgccagggccattacttcgtcctggtttacttcatcgctgaagcggataccacctttgcagggaagtttatgatgtgaatgttgtacgcggtaagcttcaatcacctgtacagaatcgcctattctcaccgggaatttaatctggtaaacggcgttgcaggccttgatctgctccaggatacctttgtcccatttagtgaatgcagctgctttgtcgaagcttttctccacactctggaagaagctataatgctgatcttgcgacataaattattgttttggtataacgattagattttaaattttcgggttactgatttttatctttttcttccagcttaccgatctttctgtccagattgataagaaataacacaattcccaggaagatgatcactaaaacaccgacaatgacataaattttatcgttgctgcggaagaattcgttgaccgctcctttctctgtattctgctgttgtgcatttgccagtaccgaaatgaatagcaaggccagggtcaggcaaaatgaaaacgctctattgatcatttaaaaatatttttaagctgtaatttcctgtaacgtactaccagtgtgaatatccacacactcagcagggtccagccaataaaggcgggatacaacaccagtttcatggagccatcggtatcttttgacgcaaagcctggtgtggtagcgcttcccggatgcagggagtccaccatgcggggaataatataggttaagggtatcagcaatgcaaacgcaaaaatgttgaaaactgcggatatccgtgcccgtttgtcgagatcgtgtatgctcatgcgcagcaccaggtaagccatatagataagaatggcgatggcggtgcacatctgtttgggatcgtctgtaagcgtgccgccccaggtataggtagcccagagcgtacctgttgcgaagcccaatacgccgaagaaggtacccactcctgcagcgctggaggcaatcacatctttctttaaatcgtatttcgacagataaagcagcgagttgataatagatatggtgtacatggtatacatacatatccacatcggtacgtgaaagaacaatccgcgggatgattgtccgttggttcctattataggtattttaacagtgaacccggcgataattacatataaaagaagcagtatcgctaatgctttccaccaatgtctggccattttttaatagctatattcgggggcaaacctacacgttttaaacctaatcacaaagattttcggggattttaagtttatccaacggcagtaattccccgttaaatatcctttacagaagtgagctttttgtttgatatttctaatatcagtctttccacaaaaatgggaaaaggatcattgtcagggcaataaccagtatatccattcccccgagcaacaggaacattttaggcagttccggctgatatacggttacaaaggcagataaagagatgttggccagcagcatcaacaccggcataatcagggggaaacccatcacggccatcagtgcggcattgtgattggcctgggcggcaatagccgccagcatagtaaatagcagggagatactggtaccgcccaggagcaccatccccacaaaataaacggggttgataatgggattgcccaggaaagcaatgctgcaaaccaaagcaataatgctcatgagggtcattaatatcacattgtagatcagcttggccgcaataaaacagcgcggattcaccagggaatagaaatacaggagccgtcccctgctttcctgcataaaacttttagcgacggcatttactgccacaaacagctgtatcacccagaaaagggcattccatactttgtcgtccggtcgtcccatcatcaggttgatgacaaaaacagtagacacaatatagagcagtaccccataaaaagcatactgctggcgtaattccagcgtaagatcctttttcacaagggtaagtgtctgatgtatgggattgctttttttcatgatcaggcgcaaagatagttattcacaattagctttcagccgttacccatttttaagtatatttagcccctcattaaaaaatgacatccccatagcaaaggggccttgttaaaagcaaactgctgatgaagaaaattctggttgccaatcggggagagattgcattacgcattatgcgttctgcacatgaaatgggtataaaaacagtggcggtatattccgaagcggatcgatccatgccctttgtacaatatgcagatgaagccgtttgcattggtcccgcaccttccaatcaatcttacctgctgggcgaaaaaataattgccgtggctaaagaaaaaggagcggatggcattcacccgggatatggttttttaagtgaaaatgcccgttttgcacagcaggtaacggatgccggtattactttcattggtccgtctgccgcttccattgaggtaatgggcagtaagctggctgccaaacaggcggcgcagaaattcggcgtccccatggttccgggcacagaaacgcctttacgcagtgtggaagaggccagggaagtggtaaagaaaacaggctttcctatcctgatcaaagcttccgccggtggtggtggtaaaggaatgagggtggttaatgccccggaagaactggatgagcagatcaggatggctaaaagcgaagccctcagcgcctttggtgacgacgccgtatttatagaaaagtatgtgggttcgccacggcatatagaaatacaggtattgggcgaccgccacggtaactgtgtatatttatttgaaagggagtgttctattcaaagacgccaccagaagctgattgaagaggcgccgtcgtcctgcctcacaccggccatccgcgccgctatgggccagtgtgccgtagatgtggccaaagcctgcaactattatggcgccggcaccgtggaattcctggtagatgaccagttgaacttctacttcctggaaatgaatacccgcctgcaggtggagcatccggttacggaactgatcaccggtctcgacctcgtaaaagaacagattaaggtggcccggggagaaaaattatctttcacccaggaaagcctgaaaataaacggccatgccattgaactgcgtatctgcgctgaagatccgggcaataactttctgccggacaccggtaagctggaaacctatatccgtccgcagggttatggcgtgcgggtagatgacggatatgaacaaggcatggatattcccatttactacgatccgatgattgccaagctcatcgcctggggcagcaaccgggaagaagcccggcttcgcctgatccgcgccattgaagaataccaggtaaaagggatcaaaaccaccctgcctttcggtaaatgggcactgcagcagcccgccttcattgaaggagattttgacaccaactttatcaataaatattttacgccacagtcgctgcttacagacgaagcagacctcaataaactggcggcaatcctggctgcatacgtatggcagcaaaacaatataaatttacaggaagcggctatcagcaatcatccacgtgaatcggcctggaaaaaaaggaatatgttaagataagccaaaacagttgttaactttcgttaaagtgtttcctgaaaacccgaaaacgcataactttgcgccaattttaattatgttacgtaacgtcatcttacagatccttcagttcttttaccaggcacttccaaaggtggttccctggcaaaccttccgctacttagcatgtggcgggggcaatacggtattggatatatgcctgtattatgtgtgttataattttatactgcaccagcaaatggtgcacctggggccggttagcatgagcgcgcatatcgccgccctctttatgtcaatggcggttacctttcctaccggtttcctgctcagcaaatatgtagtgttctctgaatccaatttacgcggacgcgtacaattgctccgttacttcatgctggtaggcatctgtattgtactgaactatttattaatgaagatatttgtggaccacctgcacttgtatgccaccgtaggtaagatctgtaccactgtgctggtagtaactttcagctatctgacccagaagaaatttacctttaaagtgaaacaacaggcataaagtaaaaaggaaggtcgctgaccttcctttttactttatcatacattttcgtaatagcaatgcctgcatctcggttcatacagatccttctctcccagcaacaatgtttcttttgatgccgatttacggtaagagtaattggcaatatgaccgcacttcacacagatggcgtgcaacttagtaatataatctgcttttgccagcaggaagggcatctgaccaaatggcttgcctgtgaaatccatatccagcccggcaacgattacacgcaccccacgaagcgccagctgatcacatacattgggtaactcatcatcaaagaactgcgcttcatcaatacctaccacatctacttcctgggccagcaacaggatttgctgggaattttctattggtgtggaaataattttattgtcgtcatgcgacgtaaggcttctttcatcaaaccgggtgtctatggcaggcccgaatatttctacctttaaattggcgatacgtacccgtttgagccggcggatcagttcttcggttttccccgaaaacatagagccgcaaattacctcgatccagcccctccgccctcctgcaagagaaggttcaataaacatattatactaatttgattattaattaattaaaatattctaattttatgaaaataaaataattctatcactaacccgttaacaattaaggcatggaaaaaattaatgcattaattgaaaaactacaggaattaaaaaattccggggctgagctttctgcaatttcgtactacgcgcaattgctccaggcagaggtgttgcatgcgcgtaacaagctgcatcagcaacaggtgcaatctacacaaggaaatatcgcggtgatcatgcctgcgcaacaaccgataacggtaccggcgccggcagcaactgcgccgcaaactacaacattaccttcaaataaaccggcggaagcgccaattgccaccgctgagcctgaagatatcaatacccgcgcagccaggctaaatgatacgcctacccgtaatacggtaatacttactgaagatattaatggccgcgcctccaggacagaagaaccttcagccaccaaacctgtggaaatgcctaaagccacgccgatggaaacgccgatagcggctgtgcctccggcggccgacctggtaccacccaaaccggaaccggttgtcactgcccaacccattcccacgctggcaattaatcaatctcctgttgaaaaaacaaaacccgcgcaggctgctaccctgttcgacgatatacaacctgtaaaaaacacgccgccggtggccaccaacggcgaactccgaaaagatctcaacgaacttgccggcagcaacggtacttcactaaacgaccgtttgcggcaacaacaggtagaagtagcgcagaaacttggtgagatgcctattaatgacctgcggcaggccattggtatcaatgaaaaataccagttcattcaggagctgttccggggcgaccgtgacctgtacgaacgttctattaaaaccatcaatgaatgtagtaatctccaggaagcggattactggatccagcgtgaaataaaaattatacagggatgggaagacgaccatcacctggtgcagcacttctattcgttgctcaaaaagcgtttctcctgaatataatctaacaccttttgggtagctccggtattggcggctacataatttccagcgatggcggctacttcagcataggctaccttgtctgccaggagcatctccatacaggtgtggaggtttctgtaattatgcactaccaatgcgccacccgcggccaccagctccactgcttcgaagtatttcccgaattccggtcctatgatcaccggcttgctgtaaacggccggctccagtatattatgtatgccgtccttgccaaagccccctcctacataagtgatagcagcataacgatagagcgtagtgagcatgccgatattatctatgatcaatacatccccctgcctgttatttccttgctttagttcagagaagcgctgcgcatccggaaacaaagccagtatcgactggatatggtgatcatcaatttcatggggtgcaaggaccagctttacgtctgtttcttccttttctttccaccagtcgcccaggattttttcatcggatggccaggtactaccggctacgactaatcgcttttcgccggcaaaaacggaaatttcaggcaattcccggtattcattgagcagggcggccacccggtcgaaccgtgtgtccccgctgatgctgctattttgcaaccctattccgcgaagtaattgaagtgatgcctcattctgtacaaaaatatgcgtcaggtggcgcaggagcccccggaacatgttgccatatcccttaaaaaatacctgatcgggccggaaaatgccagataccagcagggtcgggatattcctttgatggagggtagtcaggtaatgataccagaattcgtattttatgaagatagccagggcgggctgaacaatatctataaaatcccgggcgttgctgcgggtatccaggggcaggtaataaacatggtccgcgcctttatagtctttccggacctcataccccgaaggcgaaaaaaatgttaacaaaatttcatatgagggccaggcagcgcggattgcctccagcaccggccgtccctgctcaaattcccccagggaggcggcatggatccatactaccggacgggagccgattccgtccttccgcatacgcgattgccagttctgccggccttccagccagcgccgggctttggttttgcctgccaatgcggccaggtgaactcccgctttatacaattgaagccctgcattataaattcctgttgctatcattcgcctgcgtacttttacttaattttcagctgaatgcaaagataatccccagccaatcccaaaatttgtaaatttgcacactttaaacaaaataaaaatatacgatcatatggttcctattcagatggtagacttgaaacgccagtatacgaagattaaatcacaggtagatgcagccatcggcgaagtgctggatagttccgcttttattaatggtggcgcggttcagaagtttagcactgaattgcagtcatacctggacgtaaagcatgtgattccctgtgcaaatggtacagacgcgcttcaaattgccatgatggcgctcggactggaaccaggcgatgaggtaataactccctcattcacctttatagccaccgcggaggtaatcgccctgttacaactgaaacccgtttttgtggatgtagatcctcaaacctactgcgtggatgtagctgccatagaaaaagcaattacccccagaaccaaagccatcgtgccggtacatttatacggtcatgtaacggatatggaaccgttgatggcgctggcggcaaaacataaactgtacgtgattgaagataatgcccaggctattggcgccgattatacttttagcgacggcacaaagaaaaaagccggtgctattggtcatattggctgcacttctttcttcccttcaaaaaatctgggttgttatggagatggtggcgccatttttacaaatgatgatgaactggcggcgaagattcgcatggttgccaatcatggccaatctgcccgctattatcatgatgtcgtaggctgcaactcccgtctcgattctgtacaggcagccgtattgcgtattaaactgccattactggatcaatatattactgcacgccgtaaggtggcagacgcatatgatgctgcatttgcagatatgccacaaataacaacaccttatcgcgctccgtacagctaccatgtatttcatcagtatacactgcagttaaatggcgctgacagaaatgagctgcagaaatacctggcagaaaaagaggtacctgcaatgatatattatcctgttcctgcccaccgccagaaaatgttcgagcattttggtggcgcggcctttgatcttcccgtaaccgatagtctcaccacaaaggtgatttccttgccaatacacactgaaatggatcccgatcaattggagcacattatccaatccgttaaatcatttttaaaataatcaccccgcatgaaaattacagtagtaggaactggttatgtaggtcttgtaaccgggacttgttttgccgaaacaggaaatgatgtcacttgtgtagacattgatgccaacaaagtaaaaaagctttcgtcaggtcaaattactatttatgaacctggcctggaaaaattatttgagcgcaacctcaaagaggaacgtttgttctttaccactagtttggaagagggcattaaagatgctgaagtaattttccttgcattgcctacccctccgggagcagacggagctgcagatctttcctttgtgctgaatgtagcagagcacctgggtaaaatcatgactgactacaaagttatcgtagacaaaagcaccgtacctgtgggtaccgcagaaaaagtaatcgctgccatcgcgaaaaattgtaaaaccccatttgatgtagtttccaacccggaatttttacgtgagggggtggcagtagacgacttcatgaaaccagacagggtggtgattggcactatgtctgaaagggcacgcaaagtaatgggagaattgtatgctccttttgtgagacaaggaaatcctattcttttcatggatgaaaaatcggcagaactcaccaagtatgctgccaattccttcctggccacaaagatttccttcatgaatgaaattgcggtattatgtgaaagactcggcgctgatgtagatatggtgcgcaagggtattggtagtgatgaccgtattggtaaacgcttccttttcccgggtatcggatacggcggcagctgtttccccaaggatgtacaggcattggtaaagtcatcacaggatgcacagtacgaatttaagatactgaatgccgtaatggatgtaaatgaaaatcagaagctgtttcttcttccgaaaataaaaagtttctttaaaaacgatctgaagggcaagcattttgcgctctggggacttgccttcaaaccaaatacagatgacatcagggaagcaccggcattgtacattattgaagcattgctggcagaaggcgccactgtaagtgtttttgatccggaagctatggcaaatgtaaaacaggtagtgggagataaaatcatctacgccgaacatcaatacacttgcctggaaaacgcagatgcgctgattattgctacagaatggagtgtattcaggactcctgacttccataaaatttcggccagtcttaaaaatcaggctatttttgacggcagaaatcttttcgaagtctcccgcatgaaagaactcggttaccattacgaaagtgtaggacgtataccagcaacattgtaattacttataacaacaacatggaaaagaaaaaaatacttattgccggtgcagctggatttcttggctcccacctttgtgatcgttttataaaagagggttttcatgtaattggcatggacaacctccttaccggcaatatcaaaaatatagaacatctttttccgttaccggaatttgaatactatcaccacgatgttaccaagtttgtgcatgttccgggaaaactggattatatactgaactttgcttccccggccagccccattgattacctcaagatgcctatccagacgctgaaagtaggatcattgggaacgcataacctgctgggactggcaaaggaaaaaaaagcacgtatcctcgtagcttccacttctgaagtatatggtgatccaaacgtacatccgcaaccggaagaatactggggtaatgtaaatcccgtaggtcccaggggagtatatgatgaagccaaaagattcctggagtctattaccatggcttatcataatttccacggtgtagacacccgtatcatccgtatcttcaacacttacggtccgcgtatgcgactcaatgacggccgtgcactgcccgcattcatgagccaggcgctgaatggtcaggatctcaccgtatttggcgacggcagccagacccgttccttttgttatgtagatgacctcgtggaaggtatctatcgtttattattaagcgactaccacctgcctgttaacatcggcaatccacaggaaatcacattgaaccagtttgctgaagagatcattgcattaacaggttcaaaacaaaagattgtttaccatccgttaccaaaagacgatccgaaacaacgtcagcccgatattaccaaagcacgtacactgttaggttgggaaccaaaagtaggcagacaggaaggattaaggatcacatatgaatattttaaagaagccttattaaaataaacttttctccggaatgaagcgaaaactattaattaccggtggtgcgggattcatcggttcacatgtggtaaggctatttgtcaataaatatcccgactaccagatcgtaaatcttgatgctcttacctacgccggtaatctggaaaacctgacagatgtaaaagataaaccgaattacatttttgagaaaggtgatatcacggaagaatcttttgttgatgaccttttcaccaggtatcagttcgatggtgtgatccacctggctgcggaaagccatgtagaccgctccattatggacccgctggcgtttatcaaaacaaatgttttaggtactgcagtattgctgaacaatgcacggaaacactggaaagataacatgaacgggaaacttttctatcatgtatccacggacgaagtgtatggatcactgggagaggaaggtttttttcttgaaactaccgcctacgatccgcgttctccttactccgcttcaaaagcaagttcggatcattttgtaatggcctattatcatacttatcacttacctgctgttatatccaattgttccaataactacggttctcatcatttccctgaaaagctgataccgctggctattcacaatatcaaaaacaataagccggtacccgtttacggaaaaggggaaaatatacgcgactggttatacgtaaatgaccatgcccgcgcaattgacactattttccatcatgggaaagtgggagaaacctataatgtaggcggattcaacgaatggaaaaatattgacctgattcaattattgtgtaaaatcatggataagaagctggggcggccggaaggcgcctctgcgcagctgattacttttgtaaaggacagggccgggcatgatctccgctatgctattgacgctaccaagctcaataaagaactgggctgggaaccctctctccaatttgaagaaggcctggaaaagacggtcgactggtacctggagaatgaaacctggctcaacaatgttaccagcggaaactaccagcaatattataacgaacaatatcaaaaaagatagctgccggcggttggcttttataagctaaccgctcacagcttttagttattacacatgccttttcaacaaaccggaatacctgacctgttaatttacgagccaaaagtttttggcgatcaccgtggttactttttcgaaagctataacgccaacaccttcagtgcagaaggtattgagtataaattcgtacaggacaaccaggcacgttccacctatggtgtgctccgtggactgcactaccagttggagccttatgcacaaacaaaactggtaagggtactggaaggaagcatcatagatgcggtggtagacatccgcaaaggctcccccacttacggcaaatcttttgcaattgagttaagcgccagcaataaactgcaactactggtgcctaaaggatttgcgcatggttacgcagtgatcagtgaaacggcagaagtaatgtataaatgcgataacttctaccataaaggcagtgaaggcggcatcatctacaatgaccccgccctgggcatcgactggggtatcaacctgaatgacgcggtagtttcagacaaagacctgatcctgcccacgcttgcagatattcaacataattttatttttaacagctgatcatttgccatgaagaatattcttgttaccggcggaaacggacaactaggacaagccctgcaaaaagtagcaggcgattatccgcaattcaacctgttatataccgactaccaggaccttgatatcacggacgcggatgccctggccgcttattttgctgcccaacagatcgatgcctgtattaactgcgctgcctatacagcagtagataaagctgaagaagatgaagacaaggcattcctcctgaatttccaggcggtactgagcctggcggaaatatgcgcccaatataatgcccagctgctgcatatctccacggattatgtattcagcggaaaacagaatctaccttacacagaaagcgacgatactgatcctgaaagcatttacggcgcctctaaagtgcgcggggaagcggcggctgccggttataatcccgacaccattatactccgtacttcctggctctactccgaattcgcagttaacttcgttaaaagaatgaaacaactgatgcaggaaaaacaggaactgaatgttgtttttgatcaaaccggcacccctacttacgcaggcgacctggctaaagcaatcctggacatcttacagtataaatcagccaatccggatgcagccatcggcggcgtatatcattacagcaacgaaggcgtaaccagttggttcgattttgcagtaaccattaaagaaatgacgaacgctacaaccgccatatacccggttacttccgacaagtataaaacggccgctaaacgcccggcctacagcgtattaaacaaggaaaaaattaaaagcacttttgggattactattccttattggagagatagtttggcccaatgcctgaaaaatatataaccagcgcggaggttgtctttctcaggattacactgattatgttgattacgctgattttatttttttggattttaaaatgattggggagatatatgacggggattgcttgaggattgactcggggatacttcattgatacccaacagatacttagcatatgcttaatacatgcagataacccggaagtgacgtggaggtgacgtggacttgatgccaggaccttttaccacagggctttatagaggaaaagatacaggacgtttatgcgagcgctaccatataaatgaaacggcgttcttacatactggtgaaaatgggtgagcagtatttaagacaggaattagcatctgaccggtgtattaatcttcaaaaatccctccaaaatcacaaaaagctaatcagtaaaatcagcgtaatcctgagaaagacaaccttcgcgttaaagcatttttatttcttcagcgccgtgatcatagttcctcccatgtccttcccatccttactggaagaagttttcaccggtccgaagtcaggggcaaaccattcgatagcactgaatttcatcggaattccctgccccatcattttcatctggaaattaatatcataagctattttgaaacaatcccagctgcctgccggtgtagttactttttcttttcccaatactttccggttgctgattacataactgatccccatttccatgcctttcacattaccgttcatttcaaaggtgccacccggtaagtcttgtccggcgtgcattccggatggataatccagaaaagaagcattggttttgccttccatcttcatgtctttcatctgcggcattacaggaacgctcatcttcatatcaatggctaccccgtttccgctgcatttaaaatgcccggtaccggaagttacctccttattacttttgtcataaaaggtattggtaaaatcagacaccgttccagtctcatctttgtgcacgttcgtgattttgtaaatagttttgccactggccacgcctttcgcatccaggatggtcatctcaatttccgcattgttgagcaggtaatagtatcctttgcaatcctgcgacagtgccggtaccgtaaatatcagcgccaataaaagaaagagtgcttttttcataatattttatttgggggtaagaaatctcagaccgcggcaggtgcaaacagcaggtcttctttataaatttacaccgatatttgttataccagcccggaatccttaaaatgggcgaatcctgcgaattttatgtaggtttgcaaaaattgttattaaaatcatgaatctgatagaagagctgcgctggcggggtatgctacaggatatgatgcctggcacggaagagcaactgaataaagaaatgaccactgcttatattggttttgatcctacagcagagtcgttacacatcggcagcctggtacccatcctgttactggtgcatctgcaaaaggcaggacataagcccctggcgctggtgggcggcgctaccggaatggtaggcgacccctcctttaaagcggaagaacggaaaatgctggacctggataccctgcagaaaaatgtagccggtatcaaagcccagctggaacgcttcctcgacttcaatgctgccaaacccaatgcggctgaaatggtgaataacttcgactggttccaacatatttcctttctcgattttattcgcgataccggcaagcacatcaccgttaactatatgatggccaaagattccgttaagaaaagaatcgaaggcgacaacgggatgtcattcactgaatttacctatcagctgatacagggttacgatttctatcatttgtatactgccaaaaactgcaaattgcagatgggtggctcagatcagtggggtaatattgttaccggtacagaattgatccgccgtaaggcacggggggaagcttttgcatttacctgtcccctgatcaaaaaagcagatggtaccaaattcggtaaaacagaacaaggcaccgtatggcttgatcctaaacgtacttctccctactccttctaccagttctggctcagaacaaccgatgtggatgcagaaagttatatcaaaatattcaccttcctggaacaaccggaagtggacgctttgatagaagaacacagaaaagatccgggacagcggttgttacagaaacgtcttgctaaagaagtaaccgtatttattcacggggaagaaaactataatttcgcggtagaagcggcgtctatcctgtataataaaaacactgccgaattactggtgtccctttctgaatccgatctgatagaagtgatggatggtgttccgcaatacgaagtaccaagagccgacctggaagccggtaaggatattgtaagcctgcttgctgaaacaggcattttccccagcaaaagcgaagcccgtaaaacagtacagggcgggggcgtaagtgtaaataaaataaaagtacccggcattgatatgattgtaaatacatcttcattgctgagagataaatatattttattgcagaaaggcaaaagctatttcctggtaaaggcggtgtaattctccggttatacctggtaagaaatatttaaaaagaagagggaagaaaaagcaattgtccgctttctcttccctcttcttctttcaaaaaaccatctgctactatttcaacccatacttcttttcatatttctcatacaactgcttctgtttattatccaggtttatttcccttccctggataaatgcccgcgttatcacgctcgacttcatatccaggatatcgccggtacttatggcaatatttgcatccttgccggtttccagtgagccggtagttttgtcgatccccaggattttagcggcattgagcgtaatcgccgacagggcctcttcttttgttaaaccataggtgctggcggtacctgcttcaaaacccaggttacgctgctgccagaagccttcgttgctcaggcaaaacagtacgccggctttctgcagttgtgcagcggttttgtaaggctgatccacatcgtcgtcctgcatcaccggcaaagcatgcggctgtgccagtactaccgggatattattttgtttcaggatgtctgcaatgagccaggaatcagccccgccaacaatcaccacatcgagctggaactctttggcaaagtcgatcgctaccagcatttcctttaccaggtcgcagtggataaacagtttctgctcccggttaaacagcttgcgcatcgactcaaacttcagattggtagcggtgtgtttgccttccttctgataagcctttgcctcgcggaaaaatgttcttaccgtttctatttgttccagggctgctttcagccggtcgttgggaacagccccacggcctccgcccagcggcgccagcggtggcataaaaaagtgcagggcattatccgttttgtaagcggcatcttcccagttccaggcatccagctgtactacagaagaaacaccgctgacaatacctccttccggtgttacctgagccagcaggatgccattggaacgcagggtgttgattactttggaatcggcattatacgcaatgatggagcgtacggaggggtttatttctcctacttcacgcacatcgatggtagcccgcacgctttcaaattccaccagccccaggttggattcgggcgcaataataccagggtatacatgctgtcctttcatatccagaaccatagcatcgctgctggcagcggggatattactacctactgcggtaatttttccatggctgaatgcaatggtgccattttcaatcacctgcccgttgcctacgtgaatagtggcattggtaaggtatacaggcttgttttgcgggcctgccggagatatcgtttcctgtgcccggacagtatacattcccagggtaaggcttaataaaattaattgtcttttcatcgcttgtagcatttagcggtgcttaaaaatttctaacagatcaataaccaatagcttgctgatgtccgccctgcaaatcttcgcagtggtagatttcctccggcgtcagcgaagctttacgggtaggcgtaccttttttcttttctgccagcaataactgggtaagccggttacgctccgttgcaatgcgcttacgcagctgcagatcgttgtcgcggtcaaattccacgataccatccacgatggtcttttcggctttggcataaatgcttagcggattatcgctccacaataccacatcggcatctttacccactttgatgctgcccatgtggttgtctacatgcagcagtttagcggggttgatagtcaccagcttaatggcttcttcttccgtcataccaccgtatttgatgctcttggcggcttcctggttcaggcggcgcgccatttccgcatcatcggagttaatagcggtaagcactccggcgccctgcatgatggcagcgttgtaaggaatggcgtcctgtacttccattttataagcccaccaatcggcgaaagtgcctgcgcctgcgccatgtgctttcattttatcggctactttatatccttccaggatatgtgtgaacgtattcactttgaagtgaaaactatctgctacgtgcatcagcatattgatttcgctctgcacataggagtgacaggtaataaaacgcttctgatgcaatatttccacaagggcgtccagttccaggtcgcggcgcttgccggcgccttgtttttcatagtcgagcgcacgggtaaatgcatctgtataaatttgctctacgcccattcttgtttgcgggaaacgtacggtattacggtcgccccagttggattgcttcacgttctctcccaatgcaaatttgatgaaaggatcccagttggtcactttcagtgcttctgcattttgcccccaacggagtttaatcagctgcgactgcccgccgatggcgttggcactgccatgcaataaatgagaagcggttacgccgccgctcagctgacggtagatattcacatcatcggggttgagtacatctgcaatccttacttcagaagtaactgactgcgacgattcgttcactcccttactgatggcaatatgcgagtgttcgtcgatgatgccggcactcaggtgtttgccggtaccatcaattacgcgggcattgccggcagccaggtttttacccacctgtgcaattttgccgttgcggattaaaacatctgtattttccagtttcccttctttttcgctggtccacacagtagcatttttgataagcaggtcctgctgcgatggtaacttctcccagccatatccattcaacggataatacagtggcccaatggccaaaggtgtttctttctttacggaatctgctttttccggggcggcctttacaaatacagcattccattttacaagatttccgctggtatcggcgccggtgccgttccagctgttatcgccgatgataccgctaagacgtacattgcttttactgttctttgccagtgtcagcgacagggataccagtttgccgtttacatcgatacggccgggaagggtatctttctgcaacacagacagtaacggtgcaacagcggtacctcttacttccacggagtagctgccgccggggataagatttacggtatagatgccgcgtatatcattccagccgtcggccttgatggtataacggttaccttgtacccagttctggtacaggatggttttttcgttgaaaacgggaccggaggtaatgaggaaattggccagtttacctggttccaggctgcccactttatcataagcctttataagtgtggccggggttttggtcagggcttccagggctttctgttcgctgaggccatagctgatggctttccgcacgttggccagaaattgctttacatctttcaggtcggcagcagttagacagaagggaatatttgctttctcaaaagcagcaggctccgtaggcgccatttcccagtgtttcatttcggccagtgatacatagcgtgcatctgcgggatcctccatatcgatggcgcccgggaagttcagcggcaatgcgaacgtggctttggtggcggccatttcactgatacgctggtattcattgccaccggctttaataatatactgtaccccgaactcgtctcctatcttatctgcgcggagcgcatcccatttatcggtcacttcaaacagctgaggcagctgctgactggcattccaggcttccaggctgagattgactccttccctggcgggctgggatttataccactgggcatccaggaacgtttgtcgcaggagggcgatgcaacccatgagggagttaggataattttgcgtagaggtgcctttatcaaaagaataggccgcagcggctttctcccggataatgactttgttttcttttgcggtggccagggttaccaatgcggcggtaccacgggcgatgccatcgggctgttgggtaagcacggcgccaaatccggcttcccgcaggggcgttgccttttcatcatctgcagaaaaaagatccacggcatttacttcgcttctgatggcctggttccagccataggcccctttggtgttagacaggaactgaggaggtgcattccatgcggaaccgccccgtttaggctccgacaaaccataattgctgaagatatccacaaaggaaggatagatatatttccctttacaatccacgatcactgcatctttggggatggcagccgatacgccggcagacactattttcccgtcgcggatcaccagtgtggcattgttcagggtggtttgcgggtcttttacaatggtggtatgtgtaaaagcaaagcacccttcgcggggatcggcgatcccgttgaccggataggtttcctgtgcgctgactgcctggccggttgccagcagggccagtaacagcagtttaccgcggtgccgcttcatagcataggtaatacaccgcaacagcagggctgtcccgggtttctcaaaagctcttttcatgtaaattttttattttttcggttcagattcagttgatccgctaaatgtaataaatcattaaggcgggactaaataaaacggcatattttttatgagtggtaagtggattttggattcacatgaaaaagggataatttgaaaagggtttaccgcttaagtttgtttaaattcgtataatacttgctgactatgaagtttatttctgtttatacatggatgttgctcaccgttttttttgcagcaactacctttactaccagtgcccaggtaaaagatagtgccaatgcaaaaggccgctggacagcggaaggaagagccgataaaatcacggacaaaatctcccataaagtaaatctgaacaaagaccaggaaaaaaagatcctggtaatcaatcaggatattgtgcgccggatggatgcagtgaaaaacaatccttccctctccaaaaaggagcgcatgacacagtttaaagccctggatacggagcgcagccagcgtttcaaaaccgtatttacgcccgcgcagtataaaaagtggaatgattgggaaatgactaaaaaagaacacctggaacaaaaaatggaaaaaaagcggcaaaagaaggaagctaaagactccacccaaccgcaataaatttcttaacttgaaagatattggcagtgagtagtctcactgctttttttatgccgcgaaaacatgaacaacactactgccgatataaaagatattttcctgcagggcgttgcggcagtgcatccgcagcagctgatcaggaaaaatgtgcaggtaatacctgccacccgtgttattaatatttcgggagatagctacgtcctcccggagcatgcggctgtttggatactgggggcaggcaaagctgccgccgcgatggcacaggagctggaaaacatactcgctgcgcatttcccggtaaagggaatggtggttacaaaatacgggcatgcgttaccattacagcaggtggagcttatggaggccggtcacccggtgcccgatgaacagagtgtagccgcttccgttaaactgctggatatggctgccaaggtgcagccgcaggacctggttatctttttactttcaggcggcgcctccgcattgctggcagatgtgccggcaggcagcagtttacctgaagtacaacaattgtttgaaacattgctgaaaagcggcgccgacatccgcgaaatgaacaccgtaagaaaacatctttccggtatcaaaggcggtcagctggcaaaaagcatatatccggctacgttatgcacccttgttctcagcgatgtggtaggcgatgacctcagcgtgatagggtcagggcctacagtggccgacccgtctacctttgcggataccatgaatgtactccgcaaatatcatctcccggaaaaaatatccgcgttcctccttcaacatattgaagacggcctcgctggcaggatacgtgaaacacccaagccaggcgatccatccctgctgcatacacacaactatctcaccggtaccaaccgtgtggcattggaagcggcggctgcaaaggcccggcagctgggttatcacccggtattgttatctgatactataacgggagaagtgcacgctgtagctgccagcctggtacaaacggcgctacagtacaacggtcctttgccggcctgtttgctggcaggcggggaaactaccgtcgaggtaactgggaacggccttggtggcaggaatcagcaactggcgctggcagcaggcattgcccttgccggttatccatcgcttactttcctgagcggcggcaccgatggcagtgatggtcctactaatgctgcaggagctatcgtagatgcatcaacgataaaaaatgcagtaaaaatgcagctcgatccaaatagttttttacaacagaacgacgcgtggcacttcttctcaaaagcaggcgggttaatgattacaggccctacccaaacaaatgtgatggatctcatgatcatcctgatcgccgcagacggccctaaaatttgaaatcaaagtttgtatatgtgtggatagattatatttttggggtttggaactagaaattctggatttactaaacgtatttgcattatgctgagaatggaacagacatggcggtggtacggacccaatgatccggttagcttgtctgatattaaacaggcaggagctaccggaattgtaaccgcattgcaccatgtgcctaatggagtggtatggacgaaggaggagatacaaaagcggaaagccatcatagaagcagcagggcttacctggtctgttgtggagagcgtgccggtacatgaagatatcaaaacgcaaagcggccgttttaaggattatatccacaactaccagcaaagcttgcggaacctggcagcatgcggtatacgtactgttacgtacaacttcatgccggtactcgactggacccgcaccgatctggcgtataccgtagaagatggttccaaagcgctgcgctttgaaaaagcggcgttcatggcattcgacctgttcatgttgcaaagaccagatgcagagaaagattacagcgaggaagaaatagcccgtgcaaaggagcatttcgacagcatgactgcggccgacaaagagctgctgcaaaaaaatattattgccggattacccggatctgaagaaagctttacgctgcaacagttccaggccgcattggataaatataaaggcattgatgccacccagctgaaactgcacctgttttatttccttcagcaaatagcgcctgttgcagaagaagccggtattaaactggctatccacccggatgatcctccgttcccgattttgggactgccgcgggtggtaagcaccgaacaggatgcccgcgaactgctcattgcggcgccatatgcctccaatggactgtgcttttgcaccggctcctatggcgtaagggccgacaacgatcttcccggcatgatagaacgcctgggcgatcatatccacttcatccacctgcgcagcacacaacgggatgcattgggcaacttccacgaagccaaccacctggaaggcgacgtagacatgtttgccgtagtaaagaacatcctgctcaccatgaaacgccgcaatgtttccattcctatgcgcccggatcatggccaccagatgctggatgacctgcacaagaaaacaaatccgggatacagcgctatcggccgtttacgcggactggcagaactgcgtggactggaaatgggtatcgccggggctttaggctctgattgactgacgtctaccagcatcaggtctgcacaaagagtaaaggtggggataagcaataccatcgtcggactgagatgctacaccagggcagaaagcgtatttgaacatataccgtaatggctgattacgtgtacaaataacactactctgaaaatatattaaagacccgccttaccggtgggtcttactttttttagcaccggctaagcacaaattttaaaagcagcgcgcaaaaaatcactgcttttttgtagcattgcatcaggacaagattttatcaactgtacacttttaccaaacctacaatatgatgagcgcaactatagatgcgagatatgaggcatgcctggccaaaagacctgacagcctcgcccgcctgatcaatttgttcaaaaaagatatagacctgcgtattacacaaaaactactggagcgcggatacaagaattttaaactgggcgatatggtactcctggtacacatcgatgcgcagggcaccattaacaacgacctggccaggaaagcgcgcatcagtaaacaagccatgagcaaagtggtaaagaacctggaagcagataactacatcggtacccgcaaacacgataccgacaaccgcgccagcattattttcctgacagagaaaggaaaagagtttatgattaacgcctacgaagcggtagatgaagtacaggacctgtatgctggtattataggcgaagaagcttttacacagctgaaaacgatccttaaacaattaacagcgggcttaaacctgagctgaccattctttatttcaacgttatgtaataccggttggcactgtctttcaccaaaggtacctttaacatcttttgcagtaattccagtgtttcttctgcagatttattttcaaagtcaacagtcaggctgcgtttattcacgcctgctgcggatggtggcacccgtatatcaaggtggaagtagctgttcaccgcatcaatgatttcttccaggggaatattccggaacttcaggcggcctgttttccaggcgagcaacgactggcttttgactgttttgaactgcagcggctggtgctgttcccgctttgcctgcatatttgcggtgaggtatactttgttgccctgatcctgcaccagggttacctttccctttatcaccagtactttgaagaggttattggttttatgcactgcaaatacggccttcagcgtatacagatcagtgtgctcatccagctgcatccgggtgcgggttggcaatgccacatcaaaccaggcatcgccggcaagcatatgtaattccggcgttacatcaagctctttagcatagctgaacgacgcgccgttgccggcaatcacggtacagcccggggcaagcaataggctatcggtatggccggtattgttaacgtaccccaattgcttagccggagctggccagcaatagtaaacaatcaccgctgtgacgagcagcatcaccgcagcagccaccagccatttacggttaaaggcgcgtaccggggagcgtttggataaagcgggtgaagatgacggaaccgcgctttccacatcatggggaacaggtatcccctctgcaagccaggcggttaagcggctttccacgtaagcagcctgctcaggtccctcgcggcataaaccggccacatgttcctgtaaaaacggatcctgtggagcatgtatatatcttgatatcagatcatcgatatcctgttccggttgatacatagtgattggaatacacgtggctatagctggtatgtttggcaagatacttaacttccctgcaagttccatcgcgcaggcattacatttgtacagacagaataaataattaggtcacttccgcaaggtttaatatttttagcacagaggaaccggcaaaaacgatatgtatgtcacctgaacaattaataaataacgaccaggaatatattgagggattgcttcaccatacaccagcagtaattgaaaatatttatcagcgctttgcttccaaagaaaagcggttcatcctgcaaaagagcggtcacgtaaaagatgcggcgcatatttttgaagaggccctgatggacatttattacttcgcccgccgtcacccgctgaaagtctccgactttgagccctttctgcaactgctgtgcaagcgtatctgggaacaggaactggaaagaagaggacaacggattcccggcctggaagcagaggagctctctaccatgagcagagacgatatccaggatgtggaagatgtgctgaaagaaggagaaaaaagaagactcgcctatcactattacctcgccctctcggacgactgcaaagaattactccgctggtcactcacagatggctgcctccaggaagatattgccgcagaaaccaacatccctattagtgaactgcctggcagacgagccgattgtttccgcagcctgttcagggatatcgacataaaactaaaagccaacagcctttcagaaaaagacctgctggaaacagaccgtttcctcagcgggcaaatgagtgaggcagagcgcaaagctttctccgaacgacttcaaaccgaccccctgcttacacaacaggtaaaacgctttgatgctgtccggcaactgctgggccagaaaatctgtaacgacgccaaccgggatgagttgcaacatttgctgtttacccaccgcaacgcctggtacacgctgaaagacagttcgcccatacccatccgcaattatgtaatccttactgcattgatagcagcaggactggctatcctgctgtatgtaagcccctggagaaaaaatatctaccggcaattcgcttccactgaaatgcagattccggatatcgacagcctgcggcttccggaagaagcgatcgaacagttcaatcgcggccatttcaacgaagctgtattgctattgaataaagcactggcagccaacccgggcaacctatacgcccgctattaccgcggcgtagccctgatcgaccaaaaccagatggaaagcgcacgacaggacctcactactgtttttaacaacagcagcgaactccggtacgaagcagccttttatatggcgttgagctacctgcgggaaggacgtaagcagcaatgcctcgaatggttattaaaaatcccatccggcgcgccgaattacctcaaagtgcagaaactgatagaagaattaaaataattaactcaggtattgtcccttactgtagtggataatattttctacttctcccttaattaactcataaacaggcgccttacctgttttgatctgtaccagttgttgtaataccaggaaatagatctctccgcggttacagccatcaatctgggcttttaaaatgtcatgttttacctcttcacaaccggtggcatccagtttctggtaaataacatacaagtcatccatccaactcatttctctaaagtttaaacatagtgtatagtctcctaaagttaaggatttatattaagaaaataaaacatctgaatcttaaataattgtaaattctaaagcgctcataaccagatcagaggattcctcacgggaaggtttctaagcacttcttcctcctccggatcctggttaagcgacagccatagccggtagtattccggccgctgaaaagcagccgcaccgaaaatgaggaagggctgcgccaccggccagctgttccagtacatcacatcatgtgcataaggccagctgtttttattatttacatatggataaaggaaagcgattcctctctccatatttttactactgtcggctgtaaagcgccacagatcattatccggcgtactcagcaactggcagatggtgctcatggcatccaggttaaacagcgagtagccgtaaggtttagtacgtttcaattccagtggaaaactgccgtcagcagccatctggtgaggcagcaataccgttttataacgattgctgcaaaattccaacagctctttatcatccacaaaacgcgcaaaagcggccacctgcatcacccagcacgtgccgtgattattggcagcattcatttcatccttcccaaaaggatgtgtggtcagccattgcaggtattcactgaaccagcttttaaacgctgtaagatccgccggcggaatggcgccggctttctccataacacttaaagcctgcaccacttccatcaaatggatcgtatcaataatgccgatacccctgccggttacctttcctttgatggcctgcgcatacagcagcgaaggattcatccgggtagccgctgtttcaaaccaggccttcgcatgcagcaatgcctgctgtagataagtgttgtctttggtggcaatatatcctgccgccagtgcgcccatcacccggctgaaacggatcatggccagccggtgcgctacaaaattttcagggttggtttggccatcccgctggatataagctccgtttggatttgccggatcgggccaccagtaatccccttctgaataaaagtcatgtatgcctccggcgctgcggtcgcaacggaaggcggtaatcgtttgtggtggctgctgcatggcccatgcggcccgtttgatcaccgccacccgtgtatctttaagcagctgctgctgatagggtgattgcgcctgcattatgcaggaaatactgatgaataaagctgccaggaacgtacgcatggaattatttttttggtgttaatagtaatacccggccgtcatgtcctgccagctccatcacaaaagaaccggtgtgtaaacctaaaccagcgcctgtccagtaatctgatatttggtatggctgatcaagtttcaccgttattttttttgaagatgactgccagttgagcaaaatcacctgtttgcctgccgcggtagtaacccttcctatttcaaaatcagtgccttcaaaagctgctgcctttgcggtgggaggcaatgccttcttcaaaacgttgagccgttcccgtgatatcttcgttaagtcatcgccacttagtaacataccaccggtagcgtacagcaaagctgcatggaaattaaattcgttgtcaggcatgttgccggtgagtaccaggcaatcaggatcgttccaccataaacggccattttgccaggcacggtaaaggttttcacgaccggaacgctcaaataccggccaggtacgtttaatatccattgagctgcggctgccatgcaccaatcctaatgatggccacagcggatgattacagccaagtataaaagcatccctgctgcctttgagaatggcttccatgccacgccggtatgcttctacccttgtagctttagcatcataaaatttgccgccatgaatagcgccccagaaattagcatccagtttaaaataagtaacgccccagtcgttgcgcatggtccggaatagttgctccaggtgttgctgcaccgcagggtttgtgccatccagcacaaaccagggcttcatccgccagcccccaaatgtaaccaggtcgctgcgcaaaggtgcaccagacgcgtctttcaccagccagtccttatgatttttataaatagtggagttgctgtcgcaaataaacggcgctacccaaatagccggctcaaagcctttttcccggatggctttcagcacctgttgcacattaccgccaaaagaattacccgactccagccagtcgcccatatgcggctgataaccgtcgtctacctgtatatattttagcgccggaatgttactttttatgtaatcaaggttatcgtaaatattctgtgcggttaccttcggaccgaaacaataccaggagcaccacccggttggtggctgcttaaactcaagccgtggatgatgctcctggatcctgccggcgaaacggtccagcaaagcgttgccatccttacccgtgatcaccattaattcctccagcttaaaatcagctccgggagcaagttccaggttctccaggtcggttactgttttgatggtatccgcagaaatataaaatttgcccacaaaacgcctgctggaagtatatcccaataatatctgttcctcatttgcagggtacaaacgcagcaggttgtatactgccaggtaaccctccggttgcggaattttataatgcccggcatccgtataattccctaatgtttcaggatgagcaagcgtaccggctgtttgcgtcagcatctggaaaccctccgcataaaagggcgtggtgggcaacaatatcttacctgtcgcaccggtaatcacttccttcaatcgcaccgcggtactaccggtgttgactatacgtatttcacagtgatcatttttccagttgcggactactttaatataatccggcgctatactgccattggcagcatacactacagctgcactgcctttcagcgcctgtacaaatgctgcgggggttcctgccatggcggtgagggcacaccacagtaaaccggcagttaaaagccaactattttttttcatcgtggatattattttggtggcatcgtgagttcaaatagtttcatcaattcttttcccgttatcccgtttgccttaattgttatgtcatattcgcctgccggcagataaatatctttcagtgactttacggttgttttaaccggttgcacagtttcctttataacatgatcgcctatacgcagtatgaaactgccaccggcatctgcaccatacttaatactaagcctgtacgctgcatcgtgtacggtacgcaccttccagctgatgtactgcgcagtgtctttccagttatgtacgtcataattattcttctttccgtcgctgtactgccagccgttgccatgcagggtggcatcaaacgccctgagtacattcgtaatgttataagtatccaatactcttacgctatctgttttaagctggtctgtttcaagtacaataacgctgttaatgctatcgggcgcgtgtgcaggcaatgcaatcagccaatctttggactgctgccgctttaacggcagcggctttttacttttgtcgcccagcaggtacgccttgcggatattgctttccagtccgcctacatataaggtagattgccaattaaaaacgtgcaggtataatttgttgtccttccgcgtgctttcaccccagggctgcaccgttagtggacttgcagtagtgccgtaaatgctttcgccgtattgttgcatccacgctccaatggtatgcagtattaccgtatcacgcgggtcaatgctgccgttgccttccgggccgatgttcatgagcaggttgccgcctttgccggccgctttggccagcagccggataaaaaagcccggcggcttatgactgctgtcgtacttcgaatatccgtacgactcgttggtggtgggaatggcttcccaatcgccggttaccgggtaaaactccgcgggccggtcggccgtgttcacgtaatcgccgaaagaaacgccgggagcgcgtgccagcctgccattcactactaccttattatctgccgcccggatcgcctgcagtatacggatgttttcactgagcggtagcttatgcggcgtatcaaaccaaagaatatccggatgatatcttttcaacaactctaatatttgcgggattgctttttcattcacatacctcaccgccttaggcagtaattccggatgtgcattataccaggtgacgccaccatacaggttcttatctcccccgggatttttataatcccagtcgttacccggtgcatcgggatgctcccagtcgaacgcatgggagtaataaaagccgaaccggataccatatttcttacaggcgaccgacaatgccgccaaaggatcctgctgaatgtgatagttgccgatagcagtgggatacatggccacgccatcatgatgcttggcggtgatgaccaggtatttcatgcccgccgctttaatcatacgtacccaggcgtcggcatcaaaatttcccgggttaaatgattgaatgagcttatccgcatattccttccggctgatcttctccttccgcatcaggtgctcggcgtagccctccaccttctttccattccattcgccgccggcggtagaataaacgccccagtggataaagcatccgaatttagcatcccgccaccaggcaatgcgggcattgtggtttttcatggatgctttccaccagccattcagcgcgccgttgactgctatgctgtcgcgcgctgcggcctgctggctcaggatgccatcatcatcgcctttcacctgcgcaacagttactgctgttataacgctaaaggctatacttaatatgcacctgcgatagttcataagatatcataaattttaccaggtgcagttgaaaaatcatactcaaaaactttttccaactgcaacactggtaatttcgttgcgtcttttacaatagtgttcccccggatctgcaactggtagaatggatttatgttgttaccaaccgccacctttaccggttgtccgttcactttaacggcaacgcgcgtacgaatacggcagttaccacccaatgctgaacggataacggcatgcgtgagctgcccatttttccattccatatctacttcaaaaccacctcttgcttttaatcctttcacactgccggaaggccacgcatcgggcaatgcggggagcaggtacagtgcgccatcatgactttgcagcagcatttccgtaatcccggaagttaccccgaaattgccgtcgatctgaaacggaggatgcgcatcaaacaggttgggataagacccgccgctgttgtcggctacgctcactgtttgaccgcccgccagaaataactgcttattcaacatggtatacgcgtgattgccatcttccaggcgtgcccaccagtttatcttccatgatttagaccagccggttccgccatccccccgcagcagcaaactgcgtgtagccgccgccgatagtacggtatcccttcggggcgaaatgaaattgcccgggaataagccatacaggtgggatacgtggcggtgagcatcttttggatcgtcccagtctttgtaccactcctgcaattgtccatactgaccggtatggaaaggatacatttccttcatggtttgtttgatacgggctaccagggctgcatcctgttgcaacactactgctgcccggatcgtattattaaacaggtcgtgaataatggaaagatccatggtggtagcaatgctcacagaaccttcccgcttgccgtttaccataaagttattctccggcgtggtagaagggcttgtgatccattgtccctctttatttttcaccagccagtcgagcataaataatgcagcgcctttcagatcgggatatacctgttgcagcattttcttatcgccggtaaactggtagtgttcccacaggtggcggctcagccaggctccgcccattggccatattgcccatttggggttaccgctgggatcggaaaaatcaataccaccggccggattggtcataccccatatatccgagttatgatgcgccgtccatccttttgcaccataatttatggcggcggttacacgcccgtgttgcgccagctgaccaataaattcaaataaaggcgcaccgcaatccgataagttggcggtttcggacggccagtaattcatttccgtattaatattgatagtatagttggagccccagggcggttgcatttccttattccacagtccctgcagattcatagccggaccgcctttacgggatccggatatcatcaggtagcggccgtattgatacagcagcgtagttaattgcggatcgcggttgccaccggcgagcgtatatactttcagcctttcatctgttggcagcaatgcggaagtgtcgcttccgaggttgagcgatacccggctgaacaacgacgtatagtcgtttatgtgaccagtcagtaattgcagataattgcctgttttttgtagaggcgccacagctgccgcatgcggatctttcccgttgggtaatccatctttaaaactagtgccaacagataccaggagtactgcttccgttgcgccggaaatgtgtatgccggcagtatctgtatttacgtgtcctccgtttacgcgcgcatcaagatgtacttcataattgattcctttattgccataaacaatctgttttggctcataagcccttgccgccacatattcggggcatctgcccttcatgaccaggtaatgcgggttaaccacgctgttcgtatgcggcatcgggttggcaaaacgggtgctgaagctaagctgcccggctttactggccgtatagcgtattaccagcaattgcttcggataactgcaaaacacttccctcgtatagtcgacgccgttagctgtataactaacgcgtgctaccccgttgttcaggttcagttcacgtttatattgtatggcctcctgtggtatatcgttgtttataaaaagacttcccagtgtgagatagcgggcgctgtaggtacccatcatcttgcgggccacctgatctgcttccatatatttttcttctgccagcagctggcggatgacgggcagcagttctttggcggccgggttattgccatcacgtggaacgccggaccagagataaccttcattgagttgcagttcttcctgctgtacgccgccaaagatcatggcacccatgcggccgtttcctacagggagtgcctctacccattgtttggccggttgccggtaccagagttttaacagggaatctgccggtgttgcggcgccggtgtttccggccaataacatcagcgaagctgctaacagatactttatcatcaatatattatttttcaagttgagtcatgctgtttccattcccttgcttacggctgccactaccttaccatcgttcataccagcctggacctccatagtaattctgatccggctatgatggcaaggcaggtggccattcctctgattaacatttgcttttaattttttttggcgaatctgttttaaggaaatgtttgctgcaggctttctttttttagaaaggggaatgtatatcagttacctgacattcgttctttcatcatggaattaatctctttcagcaaacgtttgcaaaacatccttagttgaccttaaccggtgttttcactacttctacgggtattttaaaaactatgctttgctaatataatccgaaactatgcaatcggttgcaaataaatgtatgcaattttacccatttcaggtatctttttaaggcagcgtaaaaaagagggaataaccggttatgagatgaggagaccgtggaaggttcctgtcttgcaaacgcaaaaaaagaaaattatacaataaatgttttgttcgatcgtctggtaataaagtgaggatgttgttatgaaaaaaggaaaacaatccatcattgcatcataccggctggaagagcttctggttgttccggggttgatgatagatgttcatcataaacaggccgtggaaccggcccaccaccccaatgctgatttaacggcggcccaccggcacgagttttacacattggtgataacaggcaggcagcgaagccggcacatggtagatttcaggctgatagacatgccaccggagagcatgtttttattaacaccgtggcaggtgcacctgtcgatggatggagaacaggtgcaggatgtgtacctgatctccttcacgcgtgattttttacctgttggctttgctgctttgcctttatgtgtggagcatccggtaacacccgacaacgctgcttaccaggaaatatggcatttgtgtacacagatgctgcgggaattcaatacgcgtaaggcgctgcaggagcaggtgttgcaacattacctagcagtattgctgacgcagtttatgcggtatcttccggaaaacacccaaagctctcctttacaatcaacattattaaaccgttaccgggaactgatggagcaacacctgctgagctggaacagcgccggggaatacgcgcgggcgctgtatgttaccacagatcatttaaacgaggtagtaaaacaggaaacagggcaaacggcttccgcgttgctggctgccagacgtatactggaagccaagcggatgttgctgcattccacgcatggcatcaaggaaatagcctggtacctgcaattcaatgaggtcacttatttcaaccgttttttcaaacagcataccggtcaaacgccggtggccttccggatctcaagccgggaaaagtataactataacccggaatagtataataacagagaagtgtgggtccggtagttttgctgaaacaatttttgagttatgaaaccactagtaatttttacgaacgacactaagcatctgaaaataaagagtaacccttaaagaggcactgcagccgttctccgccaggctctggtaatatcagcccctttattctgcaacttacccgccgcaagccggtgcgttttaatcatcaaacacatttaataaatgccttcaattaaagaaagggcgaccagtttactgatgtcgcgcatagggaaaactgcgcacgtaataagcgtagcacgtataggaaattttttattagagatagatttgcaactgtcgcaggccctgccagaacgcagcacccagcatctcaaatgtgaggtggctccatatgcgtatcgcgattacactgttgcatgctgggacactgctgcacaaaccgccacccttatagtggattgcggacatgagggagccggcagctcctgggcgctggaactgcaacctggtgatgaagtaaattatgccgggcccggtggtggtcagcatcagccctccggcatgcaacacctggtgtgcataggtgacgccagcgccgcagggcactttcattctttatacctgcgtaaaaccaaccaacaacaatttcattgcttcctgcaattggaagatccgcttacccggcagatattacaaatgccggtacagccgctttccaataacggtcattatttcaccgatttacatgaatggttataccattatgatttcccggtggcaaatacaacttattatgtggcaggtaatcaacaggtggtgatacaggtacgcaaattattacgtcagcaaggcaaacaggtaaaggcacagggtttctggggctaaacgctatggcatcagaccaggtgttctttcattgcctttacaatagcgttggagcgggattttacatcgagcttgcgataaatattcatgatatgggaacggaccgttcccacactgatatggcacccttctgctatctgcttataggtgtcgccatttaccaggcaacgtaaaatctccttctcccgcggcgataatccgtaggggtcctgataaacctgtttctccttgcggaaaaaggccagtactttgttaaccgccactaagttcgactgcaaagccgtctcatatatctgagaaataaactctgtcagggagaccgggggtacatgatcgattttaaacgcttcagttgctgccggcacctgtattaatccctgttccgtttcgttcagggtaagcaatagcacatttatatcagggtaagctgcttttactatgctggcggcttctattgcggtcaatccgggtatctctatatccataaaaaccaggttgcagatatcttttgctaattgttgtaacgtttccgatgattcgctgtacaatcctgaaacctctaaaacacgcgttcctcccaggttagcagaattaataggccgcacttttttcataatattccttttgggttatgtatattcatatgaaatattccattaataactgcaggttttccggaagctggtatggttgataaattataaatggaaagaatcacacggttcccatacccgtcgcaaatttgaaacaattacatgcagtagtcaatcggatacatatatggtttttcaataaatattaatatacaattcattttatattagcaataaaatgaaaatataacgtggtatctgacagtttattaaaggattaacctggatacaattacttactaatcaactacttaaaagtcaggacttctatcatttaaaacaaattatactttggtatatatattatggttgtacttttcctgcgggtctccgctcagttcccttagccccggtaaggtcgtcgccaagcgtcgaccggtacttttctgctatcgcctgcagggatttcaccacctccggaaactgctgttgcacatccaatgtttcacccgggtcacaccgcatgtcatacaatgccatagggacgtctacttccggctgcgcaccgggaaaaccatcatatcccggcaggtttaatttatacgttctgcttctatgcgggagcatcagtttccacggccctttcctgatggcctccaaactattcacctggtaatatacggccagctcatcccgcgggtttgcttccggctcattaaataataatgacttcatatccactccgtcaattttccggactggcaatgcagccccgcataaattggccactgtaggaagcagatcaatggtagcagccattttgttgcaaacagtaccggcaggaatcttccccggccagcgcatgatacacggtaccctcgtgccaccttcccaggaagtacctttaccttcgcgcaggccaccggtatttccggcatggttaccataagataaccagggaccattatcgctggtaaaaatcaccagggtgttatcagacaaaccattctcctccaacgtttttaatacctggccaacagaccaatctatttctgctatcacatctccaaaaagcccatccttactttttcctttatacttctctgacaccgcaataggcacatgtggcatactgtgcgccaggtaaagaaaaaatggttgctgccggttattctttataaaacggcaggccctttctgtataaagcgtagtgagttgcgactgatcttccagtgttttaatatatctgagtggcttattaccttctatcagcggcagtggcggatactttctccgcggatgcgtagaggtatcggaataaggctttccatcataatgtaccggccacatatcattggaataaggcagtccgaggtactcatcaaaaccatgctgtaaaggcaaccatggttccctgcttcccaggtgccacttacctaccatcccggtgcggtaaccccgtgcttttaaaacagatgcaatggtttgttcggcggtgtccagcgcaataggcgatgccggcgacaaagcgccattaatgcctaccctgttaggataacagccggtcagcaatcctgccctcgatgcagaacaaactgcctgcgctgcataaaaataagtgaaacgcatgccctgagcggccatacggttgatattgggagtgtgccagggagtaccggcaaaacattcaaggtcaccataacccatgtcatccatgaagatgatcacaatattcggcttttttgccaccggcggcagttccctaaagctgaatgatacagccgccaatatgaatgtgctcaggcaaaaaaaagctcttttcatccgggacgtttaacaataaataatggtgagtataaaaatatacatcttccgcggatttcctagaaaaatttgtcttagcgagttttgtcttgagcgctgattacgctgattataatgatttaggggattgacctttgggattttattatgattaggggagatagaagcgattgatcttttggatttttataagattagagaatatataagcgatttgttatcataagatgtattaaagattaagggagatataagcgaatagatccgcctatatctcccttaatcataacaaaaataacaataaaaatctcaaaagatcaatcgcttctatctcccctaatcataataaaatcccaaaggtcaatcccctaaatcattataatcagcgtaatcagcgctcaagacaaaactcgctcattgcaaaatcagttctatcaccgggatctccacgtcaggtttgcgcaccggtagttccagggcaaggtcgcctttgtcggtgccacgcattttcacttcggagccatcgtttagtagctgcgcgtattttactttgcctttcatgcccggcagttcgaaacgctgtaatgggtagtcgagcaaatgcacatacaaacgtttggtggttggattgtaagtcagcaaactgttatcagggcgcttgaactccgctggtgcttcggtgcagccgtaaatggaacggccattcacctgcatccactcacccattcctttcagcctgtcctgtgcgcgggcatcaaaagtaccgcgggaggtaggtcctacgtttagcaacaggttaccgcccttactcaccgattcaatcagcaacaccagtaactgcttgttatctttccaggaagtttcatcacggtaatatccccacgaaccggaaaaagtctggcaagtttcccaatgaatgcgcttgccattacgggtaggccattcggatactttgtattgctccggtgtggcaaaatcgccgccgtcttcatattctccaaggtccaggcggtcgttgatgataatgcctggttgcagcttgcggatcattttaataagatccagcgaattccagtcgttatgatcttttccatgttcacccggaaaagaaaagtcggtccagaggatgtcaattttaccgtagttggtcataagttcctttacctggttcttcaggtaagtacggtatttttccatatcgcggcccttattcagctgctcataatccttcggatcggaaggacgctgcgggtgcacacggtcgatggtataatccggatgatgccagtcgatcagcgaataataaaaccctacttttaatccttctgcccggaaagcgtctacccattccttgatcagatcccttttagctgccgtgttaggcgctttgtaatcggtgtatttagaatcaaataaacagaagccttcatggtgcttggtggtgatcactgcatacttcatacctgccgctttcgcctgccgcgcccattcgcgtggattgtagaggtccgggttatagaggtcgaaatatttctggtaggcactgtcggtaatatgctcgttactttttacccattcgtgccgggaaggcatggaatacagtccccagtgaataaacatgccgaagcggtcgttcacccaccaggccagccgttgttctttctgtgcatctgtttcgttgaatattttcttttcctgtgcgttaactgccgacaggaataccaggaaagtgagaatacaaagtgatagtttcttcataactaataaattatacattcggtttgatacaaggttactcggctaccagccaggtgtagccatttgcggggatggttactttcacatgagcgcggtaactacggtcaagggtatacgtttttagcggtccttctttttcccggatacgcacgctttgtttgagcccgctgtaatacagcggcagcgccacttcacgggtaatggcctgttgtgttggattgtacagcatcgccagggccttttgcggcaattgggcgcttatatgcataatcccgtcccagtcgcggccatcagccctgcgcaggtgaatgatatccgtattgagaatgtcgcggtactttttataccagttgaccatgttctttaccactgctttggtgctatcggtgtcgtataaacgcggaccacggtagcaggcctgtactccggcgccgtaatactgtgccatcagctggtcgtaggcgtccaggtgatctttcagcggttcaagggtagcagctgcaccgccgccctggtattcgctgagcggtacaaagccccagctcatagaaggggttttctcccaggtgccatcaaaaatattctgcctgttcaggatcagttgttctgcgcgtggcagggaaaaatttacttcgcggtagcccaatgctattttgttggtaccatccaggaagtaccaatcgggggcatttacatacacccctttttcgttgagccagtgataaagccctttctgtaactgcatttgcttccactgggaatcttccagcccggtgtggccgggatgcgttgtggaggcgcaaacatctccggggtaaggaccatcattttcaaaaatatcgaagccggtagcgctgataaaacttttaatcttctgcagataactcagaccccatttgctgcccatacagggagcattcccaaaaaatgcaccgcctgttttaccggttgccgggttaatcacatcatcttcctcactgatacgcctgctcgaaaacagggagtaaccgcccagcagcacctttttactatgtgcataatccgccagcgctttgaatttagcgatgttggcagcgcctgtatcttccatattcaaaccactgccaaagctgaggatcacgccttcatagccggttgcggcgcattggtcaatgatcgcttttactttcacggggtcggtacttaccaggtgcatgaaaataggattttcggtggtccacggtgcgatggtgcggtaaaatcttctcttagccaatccatttctttcgcggtcgtatccgtcaaacaacagttcgtaggtacggatcgattcaaaatgttcaccggcggctaaggtgatgcctaccggcacacttgggtatacttccagtacgcagggcgtttgcaggtcgtagtttacctgggaagtgtaggtgctgtcggctttccagtgggtggtctgatcgctgagatttgccttcatggcattattgaaagcgtaattactttcgatataaattccgtgcggtacctgcattttattcacgctgcctactaccgcagattcctcttccggcgttgccagtatttcattcactacctgttgcagctttatgggttgtccgctcttgttggttatttccagccatttcgagaggagcgggatcccgtcaaaaatatcgtagtgcactttaacgctgatgcctttcagttcaggcgcctgcgcctcatacgagaaggtaagctctttgccggagggctgctttggattgctgcaccagccttttgcctgccattttaaatagggagagatggcggttacctggtggccactgtaaataaaatctgttgacccggctttcaggttatccagccacgcaggaagcagatatgcctgttgcttttggccccgggcgccgccaatcatatagtcgtgcccgttaatagtaagcctggcttcgggcttaatggcacgcagcagctgttcaccgctgaccaggttacggtaatcggtgcagattacgttaggggctatacgaaaactccggctcagcaaaccattgctgagtgtaatttccttttccttttccgttaccgtggcgatatacgactggtggctgatgagccagtcgggcgcaggggctttcacctgtgcgatcgctataccggaataaagactggtaaccagtccaaacaggaggtgtgttcttttcatgttcttgttctctgataaattattatttcactggctgcaggatcactttccgcaaccagcataattcatttttatttccggaaaccggtttcactgtcaggttttgtttgcccgccttatcaatatgtataatgccaactgcgtgttgaataaagttcatgggtttgtggctgtcgtagctgccggttaccagtgtgaggaagggcagttgttgcccgccaagggttaccagtccctgctgcgaggcgcttcccggttcgcaggcgtaatccagtataattttatagtcgcctgcgtcctgtacttccagtggaaatacaatcgcgtcatcgggagttaccataccggtgatacagttatcatgtttccagtcgccgaagtaatgggaatacgtaaagagtttgcttttggcagcgccgttgaaaacggcccatacagcgggtatttccgcctgcgcatattcgctgctcacggtttgtgtgcgcagctgtgataaatctgtttgctgcccggtatacaccacttcaatcacggtacttcgggtatccggcaatgttaccggcagctggataacggtttcttccggcagctgtttccacgcaagctggtctttagtacccaggatttttaccgatttaatttttgctgtgagtccgggtacccgtaactgcctgttggctggcatttgccagatatgcaggaataactttcctggtttactggtggttacgccccagggctgtgccgggatcagtccccagatggtgccataaatgctttctccataggtttgcagccatttaccggtggctttcaggtatgctatggaataggcaggccattggccattgccgtcgggaccaacattcagcatcaggtttcctcctttggaggctacattgcccaggagccggatgatttccgttggtgatttaaagttcaggtcgtgccggatatagccccaggagtcgttgtgggtataaatagattcccaggcgcccgggatgggaaccgggggtacttcagaatcgccaaaatcgcggtagtcgccaagatcatgtcctacgcggctgctgaacaggcagcctggctgcaatagccggagactgtcgatcatctgtttggtttgtgctgcggttaagccgccgggcatatcaaaccaaacgaggccaagcggaccgtagttggttaacagttccttcagctgcgggattgatttggtgtggtagtattgctggtaatctttctctttatttttaaaatcccagttatttccgccgccgttaggttcgtgccagtcgaggaactgggagtaataaaatccgaagtgtatgccttttgtgcggcaggcgtcggagagcgccttcatcggatcttttttatagggagaagcgtcaacgatatcaaagtcagttactttggaatcgtacatgctgaagccttcgtggtgtttggcggtgatcaccatatacttaatccccgactgcctggctgtttctgcccattcttctgcgttaaacccggtggggttgaatgtttgtgctactttggcatattcagcagccggggcttttgcgcggttcatgatccattcgccgctgccgtagtagctgctgtcgttccagcggccaccgagtttagaataaagtccccagtgaatgaacagcccgaacttagcttcgctgaaccatttcagcccgggatggagcttattggctacggcatctttgttccacatatccggcatgtcctgggcattcccttttagcgaagtgagcaggcacaggaatagtaataacgttggaatccggtggaacatatagctaagtttagtagtacaatccgtaaaaaatatacatatcctgcggtatatgcaaatgcgtggaaaatggtatcagggaaagggaaaatgctacaatcagcggagggaggcgggcgcttcgcgtcattaaccaacggttaacgattattccggatagtaatatctaatttcgggttcgacaagttacaatccactaagcaaattggtaactttccaaattcagcaatcatcttatttagcttaatagcaggctataaatgtgttatcagcatctgacgcaatgccgcaggtgccatgtgaatgttttttttaaacccttgctgtggtcatcagcaagggtttcttttttgccctttctccccgttatttcaattcttgtttaggtttaattaacgctctgcacacccagtccggctaatattgttttatcgttatgttcagtctgataactgaaatgcatacaactaacaaatatctcagcagtacctgttggccttttcaggccgacggggattttcctgtgttaaacaatcacccaccggtctgacgatcaatgggtttttgatttaatcatcatctagctacagcgcctctgcggtttccactgcggaggcttttttgatcttgaaaatgaatatttattcgcttatctttgtaatgtgaaactgaaagatgataaaaaagtagcccagatttttcaatcggccctcaagctggtggccaaaaagggattatccggcattaccatgggcgacatctccagggaggccggcattgccaccggcaccctgtatgtttacttcaaagggaaagatgaactgatcaacgccttatttgctgcctgccgggaaaactcggtacaggtatcttttaaaggctataacccgcagctccccttcaaaccagggttcaaaaatatatggttgaatatcctgcgctataagctgcagcactttgaagaagtgattttcatggagcaatgctatcactccccttttattactgccggtacgcgagaaaaagcgcaacagctgtcggcccccttctacgcattgatggaaagaggccagaaagaacaacttatcaagcaaacagatattggacttttgctcacctttatgatgggcgctatgaatgaactggtaaaacaaacgcattacagcagcattacccttaacagaagccggatcaacagtacgttcgacctatgttgggatgccctgaaagcataatgataaatgaataaatattcacaaattaatccacctgcatatgtcagacatcatgatcgcagtagacctgagcagcttttcagaaagcctgatcaggaccggccttgaactggccgataaaatgaatgcttccgttaccctcttttccgtggtagaaataggcattggcatcggcctgccggaaggcggccccgtgtttaccgacgatattccggcccgtatccgtgaagtggaggaaagactggaggcttacaaacagctttacccggataagcagaacatcagcattgtagtaggtaccggcaaccctaaaaatgaaaccctggtacaggcacatgacagcaatgccactatgctggtggtaggcactcatggccggaccggcctggatcatatgctgctgggcagcaatgcggaatatataatccgccattcccgcattcccgtactggtagttccctataacctggaggaacactaaaacaacactcaacaattcatacaaccgcaactcccggcaaaacagccgggagttgctttatatcctgcaacaaccccaacacctggcagattaaaatagccttaaactccccgtagcctaaaagattcgtttaaaagttggtatacctttgtggtcattgcgaacaacagacctaacgaaacccacgaacctttgaaaaagaaattttttactgcagcgtttttacgtaagctccacctcaaagagctactggccgtgttattcatattactggctatttatttcttccggtcacagcgtcatgaattatactccctgatccctgctattgaaaaggcccagagaggttgggtggtgctgggagtagtagtaactatcgcctatattttattacaggcaggcatgtatgtattcagtttccgagcggtaggcgccaaactggatgcaggccggagtaccgaattattcctgaagcgcaatcttctatccgtatttctcccggcaggcggtatcagctcactggcctatctgccacagagcttacgccgcaccggcttgcataagcaacaaatccaccaggcctccggcatctatggatttgtaggcatcctgtctgttttcctggtgggtattccggttgttgcttatgcgatgtttcatgccgccaccatgaaagatgctttgtggggactcatcgccatttgtgcgctgctgctcggcgtagtatggctggtacgttccatgcaattgaaaggcaaagcctaccagtggctggtgaaatattttccgggagcagcccggcaggcagatgaaatatttacctttcaattgtcggtaccctctttcatgaatacggtactcgcctcggcgctgatagaaatagcgggcatagggcatctttacctgagcatgctggcagtgggtgttaccccgtcgctggaagcggcctgcgtaggctatattgtagccactattttcctaattatttccccttttctccgcggattgggcgccatcgaactatcgctggcttatatcctcagcaattatggattcagtacactggaggcactggaaatcactttattattccggctgtttgagttctggctgccgttggttgcgggcatgatcgcctttgccctgaaaggcagggaattggtattacggctactcccacctatcctgatcttcctgttgggtatggtgaacatcttttcggtgcttactcctcccctggctaaccgtattcatttgctgcgggcttatattcccggaacgtctattcacgctactaacttactggtggtgttcctgggcctggtgttgctggtaacggccacctttttgttccggggtctgcgcagcgcgtggattgtggcgctggcagtttccctgttgtcggtatttggtcatatcggaaaggcgctggattatgaagaagcttcactggcgctggttactagtgtgatattacttatcacttcgcggcaataccgggtaaaaagtaatccccagctggtaaatatcggcgtggtaacggcattggctacactgtttgtcgtcctcatttttggtaccgttggtttttattttttagatgtaagacatttcgggatcgatttcacctggcagcaatctatccgccatgctttccattgttttatgttgctggaagatgacggactgcaacccgttacccggttcgggaaagaatttatgtcggcgatccgtgtattaggcgtaagtgcatgggccttcctgttttatacgattatacggccttacctgcatgttacccagcaaacgaataccagcctggagaaagcacggttttacctgagccagtacggcgactccccgatggattatttcaaaataggccaggacaaactgttgtttatgtctgagcaatatgaaggctttatcgcttaccggatagcgggcagctttgctattgtactggaagaaccggtgtgcagcgaagataataagctgctggttttggaagaatttgaacaacaatgccgtaagatgggcctccggcctgctttctaccgggtggatgaagatagtacctactatttcagtcatcttaaaaagaaaaaaatgctgataggccaggaagcgattatggatatcagggacttcacgctgagcggcaaagacaaaaaatcactgcgtaacggtttgaacagcctcgccaataaaggttatgtaactaccttccatgccgcgcctcaaacgactgctatgctgcaggatttaaaagcggtgagcgatgaatggcttcaccagtatgaagtaaaggaactcactttttcgcagggcttatttgatgaagacgtgatccgtaaccaggatatcattaccgtaaccgatgcagaagggaaagtagcggcgttcctcaatattattcctgactatgcccccggggaatgcacttatgacctgatccgcaaacgtgccgacgcgccgggcggagtgatggatgcgctgatcattgcgttgatccaggatgcgcagcaaaaagagttgcactacctgaacctgggaatggtaccgatgtccggcattatccaaccggaaaatactgcggaaaaaatggtgaagtatgcatacgagaagctgcggtttttccgtcactaccaggggttgcgtgagtttaaagaaaaatatgccaccgaatggactaacaaatacctggtatatggacatgatttcgatttgatacaattaccttctgccctcagtaaagtaatgcagccctgaggccggcgaacaatagcggaacggattttgttttacaggaggcgttaatctggtatatgagtaagttattccatgcagccatgctgctcagcttttgtctatttttcacaacgtttccgtcaaacgcacaaagcgggattaataacctgccggtggttattaaagcgcctcccgcaggcaatactgcaccattgattgtgtatataaccggtgacggtggcatgaagaaattttccgcaaatgtaattgaatcatttcatcagcagaactacccggtagtagcattgaatgcattaaaatatttctggagtaaaaaatcgccacagcaggcggcaaaggatatagcatcattgattacgtattatcagtcgcagtggggcgggaaccacggggtagtgctggtcggatattcgctgggggcagatgtactgccgttcatttacaccggtttaccaccggaagtggcggcacaagtaaagcacctggtatttttgtcgccatctctttataccgatctcgaagtgcatctttctgatatgctgggtagatccggcaataagggaatgagtgttcccggggagatcaacaaaattaccaacaaacctttgctattggtatttggtgcagaggaaaaagacttcaacctgtcagccctgaatgtccggtatgaaaaaatgatcctgcccggcgggcatgcttatgatgaagatgcgggcggcgtggcgggtaagatactggcggcgctgcatacaggcgctactccataggcagctggtatcttttagccagttcctttcttacttcttttgtcagggtaatcctggcgtccccaatcattacatgatcgtctgccagtgctgtgatatggcggaatcctatcacgaaccagtgatgcacccgcataaaagcatttgccggcagctgtgaaatgatccagtcgagtttttcggtggtcaccattttctgatcgcggagatgaagcatgatatgatcatccattacttctacatattgcagatcatcataaaatactttctcaaaactgtgctgtgttttcagcgtgaaataatccgctgaatatttggtggggctggtaattgcgtccatttctatggtcttataaattttagagaacacattatttaacgtttcggcagtaaagggcagttgcaggagtgctgccgggaggaaatcgaatcctccgggtggcgtatcgttatacgtcatcattaaaacgggcaatatgcctgttatggtcattggaagggaaagcggatcatcatattctcctgctatcagtacatgaatggtttgtgtttccagccaaaaacgtgcttccgccatcgtttggcttctgcaaaccaggtaaacatagggaatagcagacaaataattctccagctcttcaaatccctccgggttattacccaaaataatacagtttagtaccatagagctgatttgttcaaatatgggtacgtaaatttactccagtcagttgccacggaaagagaggatttaagtagggcaggtgactgaacagaaacccgcgtataatctaaaatctaatctaaaccgcgttatgaaaaaaactattcttcacagtaaattcttattaaaaagctgacaataatttcagtcgtaaaattgaagctattccgggtagcaatagttaatcgaatgttaaggattttggaaaaagaaggtggacagatcaagctactgtccagaaagacaatactttccctgtccaccagttaaggaagattacataaaagatcctggaacagctgccttacagctgtgcaacagatctaaggccctgaaagggcagcgcgggcgcagggagagctaacagggaggccggttaactggtcagtgcgcggaccatgttcaccaaataaggaagcataaaagaaacatcgtactcacggcgatcaggttttttgagaacctgacgttgaagccgcctttttctgagtagaagtaactttctttgtaccggtcgtactcaatgggagcacctaactccttcatcattttgaggaattcatagagtgttctttcggaaatacgaagccgcttggctaactgagcgggcttaccggtccctttgatcctaatgaggtaatcaatggtctgtagtctgtcaaaataacgctttggcatgtggcatagaggggtcttaacggttatttactgaatatacgatttgtgtctttattaaaccagcattatcatatatatatttaaacgtaaatattaacaatctggtttaaatgggttttcgaaattttagctgcggaacaatggcgctgatgcggataagctgcgtacttttactaaacgttgctaccttggttttattggctattaccctgaaaaaaactcactgcaataatgcttcatagataatgttggtaagcgctgtaccgcggtctactgcgggatccggaggctttatagcatatacttttccattctttccaacaatgataaacgaaggatatttactgatgttgtattgcgtaagtacgtcgcggtgctgttcatccagctgccatatccatcccggcaaaccccttacagcattgccatcgcagcagatgttcacaaacgtaacgctatcatcaaagcaattttttatttctgtaagtgcaggcagcagcggatctttcccactgtagaaatgcagcagtactacctttccgctgaattgcctcaggctcaccaggtttccctgcgcatcgggaaaactgaataccggcgctgtcacacctctgctgatacccttcctcgaacgaccgtaaagctttgcgatggcctgcttacatgcttcatcctgcaccagctccaggtaatcacgcacacaccattcctgttcttccggcgaattgccggcagcaaaacccaacatcagcgaatgcgccagcaacctgtcgcgtaaccggccactgtaatgcgttttaagccattcatagatcgccctgttattacattcataacgatgctgaataaaataatctgcttccgctttttgcaacagataattcaaataacgtatagacgtcaccgttgtatctgaaagaatgatctccggtaatgcaggcaatatattatccttataaaaaagcacttgtctttcttccagcgtactatccggcgctacggccactttccatacagtactcaccagccccgcggcggcttccgctaatacatgcgatcttaccagcgcccacgtggcagtatttatgctgtcgcggtaaaccgccagtaccttgtctgccgcctgcaaccgctgccgccacgccgctgccagccggaacgcatcaggcaatacaggaagctgcacggcagactgctcccgcttagcagtataaacagccctgttcaacactgcaccgctgccgccaaaccggatgctgtcgtcctgcatcaccatctgcaggctatccccgccgcggatcatcccataaaaattatatccactacccgcatctgcataaaaaaatattacccttcctgccggaacggatatacggaaataaaaagaatcagattttagcaaagtatcctgcgtaactgccggggaaattcccggatcataccagtaagataacgacaccttttgcacaggatggtccactaccctgcccgtaatcaccgcggcggattgttgtgctgcagctgttcctgccagcatcaaaaaaatacagctgatacgcagcagctgcatcatcataggaggacggttcataattagattttaaatggtgaaaatccccgtagtaaaaactacagggagataatattcacaacgatagtaaatgaaaactttatatatatcttaacgggcatacccgttctattacgccgaacttgtggtgcaatgataacgggtataaaacggtaaagtgttaatcgaatcttaactgttaatacgaaaacggatttttagagattaaaccaatacaccagcttcagcaccaaagcacggtttctcacataaaatggctccgggagataattgtcggtatacactataaaaagatcggatgcaggccggtagcgccattggaagcgggtattcaggttcatattcttctgctggccattgtattgcataaacccggtaaagaaaagggtgtttgtcattgtaacatccaaccgcgggcctaccagccagaaagaattattgccccagggctttggcaggttgatattgttatagttagcgcttaatgcaatgctcacatacggctggaagcgatatcccagttccgtattggtcattaaccggctgccatctgcataataacctccatagcgggccgataacgaataggtaaacaaactctgtggctttgacacgtaatcagcgcccacagtgttccagttatgctgactcccgttcaccaggctatctttaccggtattggtagggtcaaaaggctgcagcagtttgatataagtgttggacgcccagatattgagcgtgtttcgcttccggaacacaatgccatagtttagcatggtttcgttatcagtacggcgcatatgcgcttcgtcaaaaaaccaggtactggttacctgcggcccatgactcaacaccgcacccgataagggaaagaacaggcgggtaacctgcggcgccacttttatatatccctggcggggcacatatcccacctccgcattgtaattacgtcccacatactcatgctgccacccaatgttccattgcttgctggtatactgcagattagcggcatgcgccacatcatgaccggttttattgggggtatacgacttcagcaacatggccttgcccgtccagaaattgttggaggaagccaggttatactccagccccatgttccggttataccggttgtaaattggcttatccgttactttagccggatcatagtttaccgactccttattgataaaaataaaacccaggttggagcgggaaaacacccggcgctgtaaagccgccaccgtaaagttttgggccggcaacccggtttcctcctgcttcccggtttgcatattcattacccctaagcgccagtctttattcagtttaccactcagcctggcgccaaaacggattggcacgccaccaagaccaatacgcctcgagaaaaaaggacggatcgtggaatacccgaaatttgaaaactggtctccgttttcgagaaagaactgccgcttctccgggtaaaacaattcaaaacgatccaggttggtcacctgtttatccacatctacctgcgagaaatccgggttcactgtgaggtcgaggttcagcgaggaagtaaccgctactttggcatctaaacctgcatcccgccggtatttggtgggagtagccttatcataatcctttaacatgcctcccagcaggtaaggaatcagcgacacatttgcgcccgcagcaggtggagcagcatcccataccaggttgcctgtatacgccagcgaggcagtgggaaactgccgtggcaccggcgcccatgccgatttctctgttgttttcagatcgttcctactgaagttaataccccaccgggtaattccttttttataccggatggttttaaacggtatcgcagcttcaaaaacccatttatccgggtagttctttactaccgatgtccacttattatcccagctcaggtccacctttccgccatcatacatcaaaccgtcccattgcgcaccggctgcattggcgccgaatgaaaagccgttggtctgatcatcaaacgggtccatgaataaaaggaagttatcattcttcagaaaagcaaaatcgcgtctcaatgattccaccatataaggcccgtcgcctgtcgtgtagttttctactatgaggtaaaggttcttgtcgtcgtaggtcatccgcacatctgtacgcaaccgggctgcactggtatccattggcagcaccatgtgaaaaccggtggcaatatccgcctccagccacgctgcttcatctgctacaccatctatcttaacaggcgacaccgctttgcggatctgcaattgataagcatcatttttcttttgtgcaaacacagcgcatccaacaatacaacagctaataataagtggaattatgcgaaacatcaggttgatatgggtttaacgaacaaaatacaaaaattgcaaaaggagaagcaagaaaatggatgaagggtaaatgcagcggatttaacttgtcctgccgttatcttttttgaaagatgatttccggataataacccgtaaataaaaacggtaagcaacaggaagatcccgttgctcaccgtctttctttcttccggaaaattataatttattattcttcatctgcgtatcggctaccggcacttttacggtagtagtcctgctgctgcggcctttagggctgaataccttcagcttcaccgttttaccgcctgcagctaccggggtagtatacaccgggctcttcaacgtaggctcgtcgccgttagtagtataccggatcactaaacccggcatctggatgtttgcactcagcacgccattttctactttcgcgcccgcggttgggatgcgccagttgaaacccccttcataataatccaggcgcggcatttcacgcttacccattacattgctgaatacactccatgcctgtgcatacaatgcatcggctttagcggaatccttttcggtagcccactccggatcctgcgcccacgcacgttctgcaagcccaagtagttttggcaacatcatatattccatacggtcagagctggttaccgtttcactccacagcaatccctggatacctgggatattggaagcaccaaaacctgttaaccggtccttacctacaaacaactccggtgtaaccgggttgcccctgccatctacttttgagttcttgtagtagtcgaacggaataaaataaaacggcttatccacgtctacaaatccaccccagtaaaatccgggttcatcaaaagatttcatgtaagccatatcaaaataaaaattgcttacaccagacaggatgactttatacccggcatttgccaggcggtaggataaatcttcctgtccgccgccgatcacgttgttccatacattcagctggaaatgatcgtttacaaaatcggggttaggaatgctctgtgattcgccaccgaccgttgttttacgcatcccggcttcttcccatcctgctacagataatccacgggccttcagcagctcattcaccttgcggtagtaataataccagagatcatttacatctttcagtgatttatcctgctgcatcaacgcgatacaggcaggcgatttttcaaatacgccgcctggcacttcatcgccgcccatatgcactgattccagcggagcgccggcttctttatacatcgactggatttcttccaccactttatcgaggaagtggtaagtagaaggcagcgctacgttcatcacgttgtcgttccaatactgaacagagtggtattcagatttatcctgcaaatcggtcagcaggtattcattggcttcctggtcgcgaccagccgctttcaggcggtagtagcgggattccatggctttcaccgcagcgcgggcatggccggggctttctatttcaggtaaaacgcgtatatgccttgccgttgcatagcggaggatttctataaaatcgttgcgtgagaaataaccactacctgcagtgttggtggtatcgggaccggagccataagacggcggcagcatatttttccagtcgctgctatggccgcgcttagcgcctacggaagtaagttccggcagggaagggatttccaggcgccagccttcatcatcgctgaaatgaaagtgcaacacgtttaatttatacagcgccatcaggtcgatgatgcgtagcatatcgcgcttgttatgaaagttacgggccacatctatcatgaaagcgcggtaaccaaagcgtggctcatctgtaacctccacacccggtatggtaatggctttctgattgccggcaaacgccgttggcggaaccagtgtttttaaagattggatagcatagaaggcgcctgcttcagtgccggcagtaatggtaattccttccggcgccactttcaaacggtaaccttccggagcggtgatagcagcgtcataaaccaggctgataactgccgttcctttttttcgtttacccagcaacgttagcaactctgcatccagcattgccgcgctggcagacaactgcggatcggcttttacttccgggaatgcatccagcaccaggcctttaccggtggcagtgtaagacttcggcgtcgggaacaccagcggcagctgtgatacgggaatatcctttactgcagcattctgtttaaatatatccgttggcgttactactgcagttttatcaccgggataacgcatcaattgctttgcggtagtagaagggcggatactataatccttgattgagaagcctttttccggctgttcgtcccataccaggtacaacccggtgggcgcatccgtaaaattcacggcccaggcatcgccggtaatagcgagtttcagggagtcgccgggagcgataccggtaaaaccatccgccggtgtaaaccggtacaggtcaccgttaatatgctccactttcacatgccccggtaattccccgggagcaaccatcctgataaaattgaaatacaactgccatcctttggcaggaaacggcttaacggccgtattcacaaaggtgaaggccgactggaaattatcgcggccctggtaatggttttctaccacttcccagctggttttcagccgggcagcatcatagggggtggcttgttgcgcccggacagccgctacagtactaaataagaacaggaaagttgctaccaacttaccaggatgaatgtatcttttcatttggtggattgattgaagattggcttattttgaaagataataaataaatttaaaaactgcgcggattttagcgaaggttgtctttctcaggattacgctgattacattgatttttgggattttgttttttttgattttgtttttgattttgtttttgattttaaaagatttgggaagacagcagcggatattttgtttttgtcgttccttaccttttttaaaaaatataagaaaattaaatcctaaaacgtatatctccgctgccgtctcccaaaatcctttataaaatcaaaaaaacaaaatccccaaaatcaatgtaatcagcgtaatcctgagaaagacaaccttcgcgaagatttaacaaatttatctgctatacgttaagtagatttataagaacaatagcgaaggaagtattcggcaatctcctgtggttaggagcatcaaaaaatcaaaaattacagtctatggtcaaagcatttattggattttcaggtgttagtttaggtgttatcgttgttttgggtttatttttcccgtgggttttctggttactggtgctggtattgcccattattgtgatgggtgtccttgacttgttgcaaaccaaacacgccatcatccgcaattacccggtagtggggcggatgcgttactggatggaggcattacggccaaaaatttaccagtattttgtggaaagcgatattgatggcagcccgattaaccgggtagaccgctctactatttaccagcgcgccaagcgggaactggactcccagccatttggtacccagtttaatgtatacgcggaaggatatgaatggatggcccattctattcagccgcaaaattttgatcacctggagaaggacccgcgtgtaatctttggcgggaaagactgtaaacagccttattccggcagcatcctcaacgtaagcgccatgagctatggatcgctcagtaacaacgctgtacaggctttaaatggcggcgccaaaatagggaacttcgcgcataacaccggcgaaggaggtatcagtgaagcacatctcaaacaaggtggcgatatcatatggcaaataggtaccggctatttcggttgccgcgacgatgacggcaatttctccgatagtttgtttgcagaaaaaagtgcgctgtcacaagtcaaaatgatagaactgaaaatttcgcagggcgccaaaccgggccatggtggcatattaccggctgctaaaaacacgcccgaaattgcagccatccgtcacgtgaaaccacataccaccgtattttctcccccttaccataaagcatttaacagtccgcgcgaaatgatgctgtttatccagcgcctgcgtgatctcagcaagggtaaaccggttggattcaaactgtgcatcggccagcaacgggaattctacgccatctgcaaggccatgatagaaaccgatatctatcccgatttcattactgtagatggtggtgaaggcggtacaggtgccgcgccaccggaattttccaactcggtgggcatgccgctgatggatggactttcctttgtacacgatacccttaccggattcaatatccgtcatcatatgaaaatcattgcctccggcaaaatactcaccggctatcacatgctgcgggccatggccctgggcgccgatacctgcaacagtgcccgtgccatgatgatggcgcttggatgtattcaggcgttggtatgcaacaccaataaatgccctaccggcgtggctacacaggacaaatggttatctgccggcctggtggtagacgacaagaaacaccgcgtagccaactatcaccgcgataccattgaaagcgccatagaactcgctggggcagccggtttaaaagatccgcatcatattaccaggcggcatattttccgccgggtatttatgaaccaggtaaaaacttttgaagacatatacccaagtgcagctccgggtacattgttaaacggactaatgcccgaacatctgaaaaaagaaatggaaaccgtgggaattgatacgtggatatagtataaaaagattccggcttttattccctgtggaataaaagccggaatctttttatctctcaaaatatttttaaaaatataatccccaacatcatcataatcctgagccagacaaaatccgcggctggtaaagcgcgagggcgttttccctgcatattttggcggcaatatctgccgggaaattctggaggatcagttgcagatcggaggcggcaaatggccgtggcgcccgtgtagaaggcaaatcggtgccgaataataaagcactggcattaatagctgtaatctggcgcatggcggttaacacatcaaaatcacaacgactgaaacccgttgcttttaccctcgctcctttttctaccaatggcaataaatatttgaacccggcttttgataaccccaggtgatcaataaccacggcaggcagtttatgcaacgtagtggataatccgggcagttgccgggaatccacatacagctccacatgccatttcacgagttcatacacacgtaacgccagccgttcgaggtgtttcacactctcggaaccgccgcgctgcacattaaatcttacggcgcgtacacctgcttcatgcagggctataatttcttcgtcgctggtaccggcaggtatctgcgttacgcctacataaccggggcccagctgcttcaatgcttccagcaggtatccctgatcaaatccctggaaagagccggacaccactgcgccgccgcctacgttcagcgacgctacctgttgctggtagtcggctactgaaaattccgacggcaaaaagccttcgtttggctgcaaagggaaccggtgatcaatgatatgcaggtgtgcgtcgaatatgggcttatcaaacataatctcatcgttgttacaatacacaagctacagaaaatagctgaaagcagaaagcagaaggcccggagggatctcttaatccgcccgggcctttaccgcaattgctttatgttttgttaaatttccattgcgccggcagcggcttcgtccacaaaccaatgcagctcgccttcttccggcctgatgagctgggaaggatatttctccgcatcgaaagtgccttcaatcacacttttcagcgtaatggctttattggcgccagtggtgagaaacaatacacaggcagccttattcaccaccggtgcagttaaggtaatgcggtacatgtcctgtgcttccaggaaaaatgattttacccaggctttcttttcgtgcacaatgggtaatccggggaacaacgacagcgtgtgtccatcatctcccatgcccagcagcaccaggtcgaacgtggtatcatcttttccgaaatacgatttcaggatcttttcatattcggcagccgattcttccgggccgatatcggtacgcattacatggatattatcggggtttacacttactttatccagtaatgattcaaatgccatgcgggcattattgcgttcatcttcaaaaggcacatctctttcatctccccagaaaaaatgtattttctcccagggtattaccatgttgtaaggagcttttgccagcaggctgtatagctgctttggcgtattaccaccggacagtacaaatgtaaaccgttcctgtgtttgcaatacttccagtatgtagttgctgatccatgcagctacattttcactcagctgggcaggatcttttgcgatatgtagttccataagacaaaaaagttacggaccattttcacaaatggtccgtagttattatttagtaggtaaattaatccaggtatgaccgtcgcgggcaacgagtgcatctgcatcgtcggggccccatgaatcgggtgcatagttcgggaagtcctgcggcgtgcggttttcccatgtttccaggatgggcatgatcactttccaggcagcatctacctggtcgccgcgcatgaacagggtagcatctccttccattacatccagcagcagcgtttcatatgcttccggtgcatgctcgccattggcagcatcatagttaaaggtcatgtctaccgggtccagcgtcatggtttgaccgggacgttttgcctggaagcggatccgtatatccatttccggttgaatgctgatggtgagcctgttagggcgccatgtttgcgcagcttctatcgggaaggaataagggggtgcttccttaaaggtgatgataatattggtagctttctggtggagatatttacccgtccgcacatagatcggaacgccctgccagcgccagttgtcgatataaaatttaacggccgcataagtatcaatattggatttgggatccacacctttttcctcgcggtagccggctactttgttgcctttcatccagccggcagaatactgtccgcgtacggcatgttcatgcactttacccggtgtgatacggcggatcgcgttaagtacatccactttcttgtttcgcacttcattggcatcaaaagataccggcgcttccatggccaggatacacatgatctgcaggatatggttctgcaccatatcgcgcaatgcgcctgccctttcgtagtaaccgccacgaccttccagtcccacgctttcagcagcagtgatctggatattgtcgatgtaattgcggttccacaccggttcaaacaatgcgtttgcgaagcggaaagccaggatattctgaatggtttctttaccgagatagtgatcgatacgatagatctgctcttctgtaaatttctttgccagcagttcattcagttcatgcgcgctttgcaggtcatgcccgaatggtttttctactacaatgcgggtacagtgtttatcggagcaaagattcagctcacccaaacgggtggctatgttcggcaccagctgtggcgctacggccaggtaaaagataacggtaggatgtacgctccactcttcttccttctgcgttacaaaatcggtgatcttgctgtaagatgcaggatcttctgcatccatctgcaggtaagtaacatgattactgaaatctttccagtgaccattctgctcgcccttccgacgggaaaacttactgatcccttccagcaggtgtttgttatagtcttcgttgctgtatgggctgcggcctaagcctgcaatggcaaattgctcaggcatccactcatctaaaaagagattatataacgcaggcgttagtttccggtagtttaaatcgccactgcctccgaatatgaacaggatggatgcaggcgggcgtttatggatctgcatatgtttaattaaagatgaacattttttagtgttgctgccactctgtgtggaaagtacctggcatatcaatacgctggtaggtgtgcgcgccgaaatagtcgcgctgcgcctgaatcaggttggtagccatacggccggtacggaacgcatcgaaataagacaaagcagacatgaatccgcccacaggaatacctgcggaggcggcctgcgcaattacgctgcgggtgttgctttctaccgattgtacgagataagctacgccttcatccagcaggatgttggccaggtcagcatttttctggtaagcttgtgtaaatatttccagcagggaagaacggatgatacaaccacctctccatactttcaccacttccggtaacgggatctccattttcagatcaccggaggcttctctcagcatagccaatccctgtgcatagctcaggatggtggcaaagtagagggcatcgtgtacctgtttgatccacatttcagcgtcggcatgaatggtattttcaggtgctttatagatcgcttcagcttccaggcgctgctctttgtaaccggaaagggtacgcatcgccacggcggtatcaataaccggaacggctaccggcaattccattgcatcctgtgaagtccatttaccggttcccttggagccagccttatcggagatcacgtctaccaggcgtttgtcagatttatcgtcgttctgcaggaagatatccgcggtaatttctaccaggaatgattgtaaagcgccctggttccagcttttgaatacttcgtgcaattgatcattgttgaggccagcgcccttttgcaacagggtatagctttcactgatcagttgcatgatggcatattcaataccattgtgtaccattttcacataatggccggcgccttctttacccaggtaagccacacaaggcgtcccttttactttggcggaaatcgcctccagcatgggttgtacctttgcataggcgtcgaggtcgccaccgggcataatgcttggaccactacgcgcgccctgctcaccaccggaaacgccgatacccataaaatggatacccttttcgcggagttgtttcacacggcgtaaagtgtccgtatagtgggagttgccaccatctattactacgtcgccctgctccagcagcggcaacagggatgctatcacgtcatctaccggctgaccggcgggtaccaacatcattaatttgcggggacgttccagcaactgtaccatagtggccagctctgcaacacctttaacggtagtaccgggggtagcggctgcttccagtgcgctgttcttggcagcgtctttatcaaagccgataacggaaaagccatgatctgccatgttgagtaacaggtttctacccattacgccgagaccgatcattccaaagtcatataagctgtttgccatatatagagaagttacttaaggaggtgtaaaagtagggaagaattacgaaatacaaattacgaattacggagttatatggagacagccgctgatgttgttcaccgccactatttccacataactccgtagccggatgatgaataatttttatgctgagtttctgccagcattgataataccaaaagagcaacgcatgatgagcttttcgtaggtttccctgccatgtccgttgtcgggatgtgcgtccagctcccggatgcgcgtaagcgcatattgctgggtagtaagcaaaggcaacacaatccgttcgcgcatctggatagacagcaaatcgatcgggctgccggccatcagttcggattcattagtgagcagcagcaggtatttcttcgtcagctcaaattcattatagatcatctgccatacttcaccgtattgcggatgcttggccaggtaagcggtgagcgggaaataactcttcttcatcgccattacacagttatcgagcagggtcctgaaaaacagggagtgtacatataatgcctggacctcttcccatttaccttgcttttccagctgttccagcgcactgcccacgccgtaatagccgggcacattctgtttcagctggctccaggcacctacataaggcactgctctcaggtcattaagattgagtttggcagaagcattacgtttgctgggacggctgccgatattcgcctctgcatagtaacgcagcgggctggcatgatcgagataagccaggaaatgaggatgtgtttttaatgtattgtaagatttatatccttcgtccgccagtagctgcagcaaatcttcttctgatttactcagcgttacttcccgggaagaaaatagttcattgctgatgccggcgtgtatcagctgttccatattgaactgtgctgcatccacggtgccgaaattggagctgatggtttgcccctgaatggtttgctgtatttctttattggcaatgttcctgcccattgaagcatagaactggtgcgtttttccaccgccacgggccggaggacctcccctgccgtcaaagaacaccacgttgataccgtattctttggagatagtagtgagttcttctttggctttatagatgctccagttggccatgagatagccaccatctttggtgccatccgagaagccgagcataatcgtttgtttgcattggcgacgacgcagatgctcgcggtagtcggcgttttcatacagctctttcatcacctgtcctgcatggcgcaggtcatcgatggtttcaaacagcggcacaatatctaccgtcatctcttcttttttccagccgctcagcaggaacagcccgtatacttccattacgttgagtacactggtactgtgactgataatataacggttgcagccttcttctccattggcagcctgtatttccttaatggcggcaatggtttcaagcgtatcctggtgcaggggattttccagcgctttaggatctgcggcttcttttatattcagtaacaggttgatcttttctttatctcccagggaagtataattatccggcagcgcggttgttctggcagctatggcttccagtacggcttcatgaatggagctgtcctggcggatatccagggaagcaaagaacaacccgaatatttccactttgctgatcaggttatctacaagatgtacaaacagcccgttcagatcagcgataatggtatttcgtatatccgacaacgtgtccagtatttcctggcggctaatatccgctttatgcccgggaataaagaggttgcgggataattttgattccagggcggctactacattttccacgcctttaaaggtaaggcggcggcgcaggttgcgtacttcccggaagtaacatttcatgatagacgcgcgcagggcggcggctacttccacggtggtaggcgctttcacaaacgggttcccgtcacgatcgccaccgggccagaagcccatgcggatcacggagttatcgctgctgatggcgcccgggaactgcgcccggatagacgacaggatgcggccggccgactggtaaaatatattttccaggaaccacaccaggctgatggcttcatcatacggggtgggtttttcttttttgaagaacggtgtttttcccagctgttgcaggtacatatttacctggctggtattttcgtcgatgagggctttcgacaggtcgttgataatacccagcacctcgctgggataaaattgtgtcggatgcgccgtcagcaccaatctcaccgaaaaatccttcagtttatccctgagtttatcctgggcttgttcctggatcacttccgactgcagatggcgcagggtgccggcgccctggaggtcacggatattccggaacgcagcatcttccagtgcgtcaaacagtactacctgtctttcagcgtattgcacgaagcgaaacagcaggtccgttcgctgtttttcttccgtataagtggtatactgggaaaaaaaggagtccattatttcctcggggctgttacctttggcgtatccttcttcacaatgaagcaggaacagggacaggaagatacctgtcttttccacccggtggaaaggcaaagaggtgaagaggctattatacagctgaaacttggtcccaacgaggtttttgaactgttgcagcgaattatttaccggcgcttccatactaattatccgtttatagtgctaaagaagaagactaagcggctgttaaattaataattattatgttaatttcttagatttttgatttttgtttgatataaagtgataatgtttgaatattatctaataagaagcgagaggattaaaaggcaatcccggccgctatatgcgggccgggactggtatcaggaatcagaatgcgcaggttaaatggatgtaagccggataaacaggaattgtaagaattaaagagataataatataggaagtcacgccgtcaaacgatgacagcactttccgggttattaataaagtgtttattgaaaaaaatgaggaaaggtgaaactagttgccgcttaaccggaagctgaccgggaggttaaaatataccgccacatactgaccattctgtttgccgggtttccacttgggcattttactgatcacacggaccgcttcttcttccaggcctccgcctttcgctgcgcctactgttttcacctgtgaaatagtgccgtcgcggtttaccacgaactggataaatacggtgccttgtatttcattctcctgggcaatgtgcggataccggatattgttacccaggtatttcgctaatgcagcttcaccgccgggaaattcaggcatgatttccacgaatgcaactggaacatctggattggctgccggaggagcctttactacaccggaaccgccgttgccacttgcacccaggtcaatgtccattcctccttctactccttctgaagtagtaaatcctactacctgcttgtttacatcagcatttctcggaggcatttcatccggcggaacatctgtgttaacaatcatcggtgtagttaccctgatagaagcagccaatggcggcggtgcggaggttaccgggggtggaggaatggtaaccgggggttccggtggcatttccaatgcctgtaattcaatttttttctctgccaatacaggccggtgtacattttctgcggccatcagcgtgttgttcaacacgtagccgccgatcattaccagcataatagaagcggtgcccattactgcgttgcgaacacgcctgtcgtaacgactgcgtaattcataggccccataatctttgttccttccatagaagagaatgtcgaggaaatcattccccgggattttagctgagtccatggtaaatatgtttctaattagatgttgcagtaaaatattttccataaggtttttgaaaatatattttcagggagatgggtaacggggcggggtatatataatagcgtaagatacaggtagtattaaaaatagaagtcccgacacgtgtcgggacttgctggcactggggaccttacctgaaaacaagtggttccttcattttaattaggctttccgaaaaaagtataggcttatacgttatcacgtattttgcccggctgcttccggataatatctttataacagttggtttggaagcagtcctaaatgatccgataatgcttcagtccctggggcagttgccgacaaaacccaccagtattgtttgagacaacgccccttttgaactgaagttgatcgtttaatttcaatggatagtaacccaattctattccgttaccaatacactattaaaatcgtgtatccgtatacgttatattatcttatacagctgttattgccgggctgccgggtaacggcatcaggactgaacagttgatgtttgttttcatgttaaataaaatgagaaagactggtttaagatttcagttgataaatgccaggaggatgcggggaggtacgttgctgataaatttaccaccaataaatttgcagcccacctttcccgcaagcctgaccaggcattctatttacagcttacagaacgcaagattttctttcaacagcggctgcaataacagcctgctatttgaatgtaacggggacaggtgatatttaccacggtattttgcgtgtggtaacgcattccactagttagcgtgtgccttttcatagtgtatttttatttacacattttcaataaatgatggcagcaacaccttgctggtggtcaaaggatgccggaagcgtttgcctgatacttccctgtggtggtagattttattagtctactgatttggtagacaaatatacatcgagttttattaattccaaataattgcacaattttttttgtgattttttgttcgtggctggagaagcaggccatatccaagtgcgacaaaagcgtatttttgcggcatgaaagagcatgtgaaaaacatattactcattatagcaggtgccttcatctttgcagcaggcattaactacctggccattcccaacaaattatctgagggaggcgtcatcggtattaccattgtaacttactactattggggatggtcgccgggcattaccaacttcatcatcaatgccatcctgattgtaaccggttaccggctcctggataaaaggagcatggtatataccatacttggcatcctgttttgctcgttgttcctgtatctcacggaaaacaaactcgccccggttaccaccaatcctttgctggcggctatcttcgcagggttgctggtaggtataggcatcgggctggtattcctttccggcggcaccaccggcggatcagctattgtagcccggttatttaataagtatttcggctggacactgggtaacgccatgctcatttttgacatcgtggtgatcatggcttcttcctttattataggcatagaaaaaaccatgtacacttttattgccgtatacattggcgccagaacagtagattatatcgtggacggccttaacaccaaacgcgccatcaccattatctccggacgcaccgaagctattgcggctaagatcaccggcgaaatgaaacgcggcgccactgtgctgcacggccatggcgcctataccggcgcccccaaagaagtgttgtatgtagtgatcggcaaacaggagctgatgcgccttaaatcactggtgcacgaaaccgacccggaggcctttgtggtgatacacgaagtacatgaagtactggggagagggttttcaaaatagcatagctgccggctgcctgtatcgggaagccggcaaccaccattacttaccggttagcccacggatcactttcacttcttcttcgctgtaaggcgtgccatccggccggaaaatatcatgaaaccaggtaggcggctcgccaccatccggcataggcgtactccaggcatatttggtattggttttacccgctaccagtccccagttaatggcgccgatattttcttttttcagcaacggcataatattatcaaaacggctgctgcgcgtacgggccatatattcggtacaaataagcggccttcccaggcggcgcagggtatcaatatcccgctgatgctcttccggcggagaatagttgtggtaggtaattacatcggaatgcgtttcctggaagttggaaaggtccttcagcttccaatcccatatccctgcggacaaaggctgcgaaggatttacttccctgccccaggcaaatactttttccagcaggggcaaactcctgttgccatgaccggagttaccgggttcattatacaggtcccataacaggatacgcttatcatcagagaaggaggtcaggatatctttcacatatctctccaatgtatccaccagctcaggacgttgatgaatggctaatcccgggtcctgtacccagccggaattatggatgcccggccttggcgcccgctgcggccccgcctggtaggtactgtcccagcaatcgtcgaagaatacaaacaaagtagagatatgatgcctgtctgcaatatcgaggtaggtattgatcctttgcttaaaccctgcggagtcaaccacccagggcacatgatgcaggtacacccgcatggtgttcatgcctatcccttccgcataacccagttcccggttaatggtggcagtatcaaaagtggcggcctgccacatttccagctggttgatagccgtactgggaatgaaatcgcttcccctgatccagtctttacctgcataccaggtattggccctttcctttgaccacaaacctttttcgggctgcttacagctcatctgaacaagcacggccacacacaacgcaataaatctgtaattcataacgtaacttttttagtggagtcaccaaaatagtgattatacgtgtctcacgttagccgatatgtctcaatttgttttcccggaacgaattcatatttggattttgaaaattagatgtatatattgtaggcagctcaacgctttttctatccttaccatcttatcaaccaatacaattaaagggaaatgacacaaagctctcaacgctttttaccgctggacgtattccgcgggctgaccgtttgtttcatgatcatagtgaacacaggcggcactggtgggacctactggccacttgaccatgctgcctggcatggctggacacccaccgatatggtatttccttcttttctttttgctgtgggcaatgccatgagcttcagcatgaagaaatatgttcaactgggaaattcagcggtgctgggaaaaattttcaaacgcaccctgatcattttcctcctcgggtacctgatgtactggttcccgtttgtagaccatactgataacggacttcaattcaaaccatttagtcatacccgcatactgggcgtgctgcaacgtatcgccttgtgctactgtattgcctccctcctgatccactactgctctaaaaaagtggtatgggctgtgagtgccatattcctcctgggatactgggccgttatgtggtacttcggtactcccggcgaacagtacagcatgggtggcaatgccggcatcctgctcgataaacttattttaggagataaccacatgtatcatggcgaaggcattgcctttgatccggaaggcatcctcagcaccattccggctgtagtaaacgtggtggcaggttattacaccggcctgtttgtacagcaacagggcagaacaaaacccggcctgctccgcatggtgggcgccggcgtattattcctgctgctggcatatgcctggaacacggtattccctatcaataaaaaattgtggaccagctcctatgtattactcaccatcggaatcgacctgttgctgttatcactcctcatttttgtgatagatatcctcggcttcactaaaggcgccggcttctttaccgtgttcggtaaaaacccgttattcctctacctgctgtcggaagtaatggccatcctgttctatttctttatggtcaatggcgtgtcgctctataaatggatcaacgacaccatcttccagccattgtcgccgggcaaattcggatcgctgctgttttcactggcattcatgctcacctgctggctggtaggatttattctcgacaaaaagaagatctacgtccgcgtataaccatattatcttactgaattataaaagcaaagggaaggtcgcatggccttcccttcgcttttatacgcgtcagacattttcgctaaattgtacataaaattatcacggatggatctctcactcaaaggaagaacagcgctggtgtgcggtagctcacagggaataggactggccaccgcaaaggaactggctttattaggcgctacgtgtattttattggccaggaatgaagacaggttgaaaacggtactgccaacactgagtacctccggcgggcaacaacatagttatgccatcgccgatttttcagatgtggcacaggtaacggcagcagcagaaaaagttgctgcacgtggtccggtgcatatactgattaacaacaccggcggtccggcgggtggtcccattttagaagccaatgcggccgcttttaccgcagccttttcacaacacctgctgtgcaaccaggcgttggcgcaaatatttgtgcctggcatgatcagcgcgggtttcggccggatcatcaatatcatttccacttctgtaaaaacacctataaaaaatttaggcgtatccaatactacccgctgggcagtggcggcgtggtcaaaaacccttgctacagaactggcgccgcatggcattacggtgaacaatgtattacccggctccacttccaccgcgcggctggaaggactgtttaagagcagcgctgctgcccgcaatgtatctccggaagtaatagaagcagaatggctgaaagaaatccccatgcagcgctttggagaagcccatgaaatagccgcgctggcagcattcctggcatcgcctgcggcggcctacattacgggtaccagtactgctgtagacggaggcaaaacacccgtgatgtaactcaacaaggaataaaattaacgatcttcaccaggcggccatcttcaaaatataactgcacactgctttcgctgtctttgctgtaggaatcgcgcaggatgatcatatctcttttaccttcgttttccgcctgcaatactgcattgggatacaactgttttacttcttcccaggtagtattgcgggtaagtgtaattttaccggaagtaagtgagttactatctgtaaaaacaaattcttcacaggccagtgaatctttacagtgttcaaaagtagatccatctttatagaaaaaatcaaaatcctccgcaaactgcgacccgcagatatcttccccatttgcagagatgatgctgtcggccgcacctatggctgcttccaggcgctgcctgctggtaaataacggtactttgttattgatgagcgctttggcaaagaggaaaacctctatctgttcccaggcaatgttccgccggatttcctgcagggagtcttcctcttccgtaagcggccggatgttttccgaaggcgccgctacggcaatgttatccgtttcttctgttttgtgctgctgacaggctgttaacgacagcaataggacgatactgaacacgcgctttctttcttcgttcagccgataccgtatattccgcatgatcccgataaatttaaactggttactttgaaacacataattaaaataatttatattaagaaccaagttatttttatgcaatcgtttgcaataatgataaatgcgggctatattgtacatacaatttccacatatgaaaaagcaaacccttgtcttactcctgggcataaccctcccgttagccgcgctgtcgcaggacaattccaccgacgcagcagtggtgaaaaaagtagccgactatgctgtggcacacgctgccttccagtttaaagatgataacaaccaaacctggaacaccagcaaggaaataccagccggcacaacagccaggatatccgaccacctgagcgaatggcattatccaaacggcgtattgaatatcgctatgacggatctcggcaattacctgaaagacgaaaaatatactgccttcgcgcagcggcatgtagcttttgcattcgacaactacgcctattttgaagcgctcagcaaaaaaggtgtgaagtacaaaagttttccattcaaccagctaatcaacacccgcgtgttggatgactgcggcgccatgggggccagcctgttagacgtctaccaaaaagtaaaaagaagcgattacaggacctatatcgataaagcagccaaccatatcagcaaggtacaggaacgactggcagacggcacgttatgccggccaacgccttataagtggacgctctggggagatgatctgtacatgagcgttccctttctcgcacgtatgggtaagctcaccggcaacaacgcttattttgatgatgccgtagcccaggtaaaacatttttcgcattacctctgggatgaacggaatgaattgtatgtgcactattattacgaagatctgaaaagacagggcgtagctcactggggccgcgccaatggctggatcatgctggcaaaagtacagctgctgaacgacctgcccgccaatcaccccggcaggaatgaagtaattgcagatgttacccgtcaaatcctgggcgttgcaaaataccagtcggccagcggcctgtttcaccaggtactggaccgtaccgattcctacacggaaacttcctgtaccgcgatgtttgtatattccattgcgcgcggtgtaaatgaaggctggctcgataaacgctatatctccatagcggaaaggggttgggaaggactggtaaaggagaaaattcaggaagatggacaactgaaagatgtgtgcatcggcacaaacacttcggcggacctgtctttttactataaccgtcctacagaactgaacgattttcacgggatcggaccggtgatagaagcgggtattgaaatcatgcgctatcgcgcgaataataaaaaataaaaaggacggatttgcagtaagtcgttacctgcaaatccgtcttctttttcattttttttagtacatatcaaaccaaaccttcgtcgtcagcagatctgcaccctggcgggcaacagctgctttgtagttggcgccgttcagcgcctgctcacttgaaggatacgttaaacgcagcggcattttgccctgcagtgcgccggtataagcgggcttcaactgtggataatccaatctcctccattctgcaaaggcctccaggccttcactgaataaggccagccacttctgctctcctattgatttcttaaaattattggcgtcgtacgctacggccggttgtgcgaggtaagcatctacctgggcgccggtaataccgtattgtttgaaggatgcgcggatagcctgtgcatacaaatcggccgcgttgccgctgatcaggttacgctgcgcggcttccgccaggataaacaattgctctgcatacgtaaatacaaaggcgggcgcctgggtagcagtaaaagctgcaccaacatcagaggttctactgaaacccaggcgtgaggccgagtcagcagacaatccattggtaacgccgatatatgcattggtatcagctggcagtgctgcgtatatgcttaaccgtgggtcgttcagcgctttcagtttatcgaccactgttttactgatgcggtaatcgtttctcgtttccctgtttttaccaaccgggttctggttgggagaagtaaggtaattcagtttcacttcacggtcgccggcagtgaggaaaaagttgccttctgccgccagttccgcgaacaccgctttagcggcagcaggatcacgatcggccaggcgtaaggcaatgcgcgaacgcagcccgttagcgaattttttccagctattcatattcccggccagtaaagagtcgccgaggataggattgtctgacggggaaatagtgttcgccgcatttttcagttcagccaggagtcccctgtataccacccgctgactgtcgtacaccggtgttaggtacttatcgatattgcctgcttgtgtgtaaggaatatccccgtacagatccgtcaacacctggaaaatccaggaacgcatgataatgcctacggccttataattaggattgtgcaacgtgtcgcccaactctgccagcttggtaaaatcagcgattccctgtgcgtaaaaattgttccacaccgtttggatattagtagatgcggggatataacgatccgggtcggggtactggatcttagcccagtactggatgtacagcagggatgtttccatggtggcatcactgccccagtaggtatccacgttggatttaatgccgttgctcagcaggtagtccggctgtacaacggtaggttcattcggatttatgttggtgcgctccaggtctttctggcaaccagccagccatgcagcagcgaatattaagcaaaaaggtatcaacaactttttcataatcaatcaatcattaaaatgaaacattcaggttaaagccaaagctgcgggtagtgggtatctgcagcgtttccagtccctgcccgttaccggtattaaaggccgtttcggggtctatgttcggtgtattcttgtgcaggtacccgagattccgtcctaccagcgccacattcaccgcctgtagtccccatttcttcaccagggaaaccggtaaagtatatcctacttttatttcacgcagtttaacaaaggacgcgtcatatacagcgctttcattcaggttgctactgtatacggccttgtaatagttttgtgccggcaggatagcggtattcttcttaccgtctgctgtgtagccgtcgaagattatcccgtcgtgtttcacggtaaagccgccaggtgcggtggcgttatgatccggcagctgaacatttttggagccatcattatagtaaggcaacccgccatgttcctggtcgcgacctggcatggttgccgccagcacaccggtactcataccggtggcattggtacctgaccagatagatccgccttgtttggtgtctaccaggaagctcaggttaaaccctttgaaggagaaattattattgatgctacctgtccactttggtgtgtagtaacctaatatttttttactcggatctacagccggggtgccatctgcattaaccaggatcctgttctcgctgtcccttttataggcagtgccataaagagcgccatagcgctggcctttgctggcaagtacctggatattaccggagctgccgagtacatagttggtgagatatccatctgcatccagttctattactttactcacgttacgggcataattgatgttcgcatcccagcggaagccggagcgtgtagtgatgggcgttagtcccagcatcacttccacaccatggttactgagttcgcctgtattaagcagtttcttcagatagccggtagttgaactcacatccgccagcaggatctggttacggctgtgggagctgtagtacgtaacatccagccgtacgcggttgtcgataaacccggcttctacccctacttctgttgaagtggtgatttccggtttcaggtctttattcaggtacttatccgacacagtgagtaacggcagtgagccaaacggctggttgaatggataggtattgatttcctggtaaggatcggtgtcctttcctacctgtgcccatccgccgcgtagcttcagcagggagagtacctcgccctggatatgcagcgcttcagacagcaccaggctggcatttacagaaggataaaaataagagttgctgcctcttgggagggtggatgaccagtcgttacgcgcggttaaattcacgaacgcataattgcggtaacctacctgcgctgctgcgaatccgctgtacactttctgcctgttgagcaagctggtagagatgagcggatcgcgggagttgttgagtgtgtatacatctttcacagccaggcgtggcgcctgctggtagttttgttccagctgattagagcggaggttggcgccggccagcacatctatatcaaaatcgctgtttagttttttcttggcgtttaatgtaaactcgccattggtttcgctaactgcgtaggcatcttctgtataagaaccgaatggcgtaccattggtgtagtaagctattttatatttgcgtctgtcctggtagtagtcggtaccaatgcggaagctggcggtgagccaatcctggatctggtacgacagccgggcgttaccgaggaagcggttgcgcagcatgcctacggtattctcgttctggatccagtagggattgctatagtaactgtggttccagttgtaatcggtaccatctgcatttttgtagttcttcagtttgctcacatctacctgacggccaaaccagatgaactggagggtaacgctgttaccgcgccggccatctacaccgggaagattatcagcagcgctgcgcacataattggcgtaggtactgagagtgagttttggtgtaatacggaacgtattactggcggtgaaagtattgcgggtaataccggtgtttggtaaaataccaccttgcttggtgttgttataagagaaacggtaatccagtttttcgttggtgccgcctacagataaaccgttattcagtgtatagccggtaacatagaaatcttttacgttatcaggatgtggtacaaacggtactgcttcgccattggagaagaactgcgggataaggcgtccgtccattttcgggccccagctttcatccacgccatcgttgataccgccgcctttaccgtctttataggagaattgtccgccggtaccttgtccgtaggagttctgaaagtcgggcaggatgaggagtttttcaaaggtggcgccggaatttacggtcacgcccatgcctcctttggtatcttttcctgtttttgttttgatgacgattacgccgctggaagcgcgcgatccgtacaatgccgccgcattggggcctttcagaacgctgatggaggcaatgtcatcagggttgatatccgaaatggcattggcaaaatcgcggcctgtgccaataccgagctggctgttgtctaccggcacgccatccagtacaaacagtggctggttataacctgcaatggaggtttcgccacggatcacgatgcgggaagagccgaggttaccctggctgttggtcacctgtacgcctgctatctttccggacaatgcgtttaccaggttggtttcctttgcttcagaaatgtcttttgattttaattcctgcacagcgtagccgagtgatttcttttcgcgggaaatgcccagggcggtcactactacttcttccagtttcctgttactgttttccagggagatgttgatcactttattgtttccaacaacggcaaacgttgtttcaaagcctagtgaggaaaattgcagcgtatcattcacctgcgcactgatcgaatactttccgtccggatcggtttgtgtaccgcgaccggttcccttcacctgaacaattgcgccgggtatgttctgtgcatccgaacgggatgtgactaccccgtttaccctgatttcctgggcaatgctctgctgcagccacagtaaaccgggcagcaggcataacagcctttttacgtaattcatgctttgtacttgatttataagttgactcagatctttgcggatatggttacaccgttcagattttggcatttattttttggtgtataatcagttggtgatatcgggggcaaaagtaaggcacaattactaatctacaaaatttatagactatatgggctgtgaaaatagcgggaggatgctgctaaatatttagcagggaagggctgttgggcgggcattgtgcgtatgggatagcggtaaccgcggggtgattccggtcagagagtttatcactgaaatgagcaggtaacggatacatggagatgaccccgttgttacttcacggatgcttcagccatgcctgaaatatgcgtatgctatggactatctatacacttcccatgcactcctcatgcactattaatgcactccccatgcactcccaatacactatctcttcctgaggccggtttataacacaggtgagatagtcctggttttggcttacaccagttttgggtaatcctgcatttggtttacaggtaaccggcttcgcaggaatttaccgggaaggcatttcccggtaaattcttttgaaaatgtcatttacttcgccccgagcagctttttgagctcagacttacagtcttcaatattctgccagatcatcctgtcgtcgcaaatggtgcctttatatttgatggtcacctttgttttgcgcagtactacctggtaatattccggggcgtcgggagaattttcccaggtgaccctgccgctttcttcgataccaccggcaagtttatcttctatgatgtcgtttacttttttgtgcatattatctgcaaaatcgtagctgacatctgttttcaccaggcaggaagaatcttttgcgggatggtctgtttgtgcggtggcctgttcacggggccagcatagcaatgcgaggctggctgctgccagcagtaacgggaatttaaaagaacgtttcataacaagaaagattagtataacatggagattaggtataataacaagtccgggaaaatgggtctcttgattgctgattttggtttatatctctttttaactcattattaaaatatgatatttatcccactccacaaaataatctttgcagaaacataggggtaaaagtaacgttgggtgtctttctaacagatcactggtattgctgctgcagattgaacattatcttcctgccggcgtcattgagacccgggaggctgtcttccggtataaagtggcgtttaaaggccatgatggcggcggtggagtctttcacatcgtacccgatgatgcggagcgagagcaacgggtcaaatgtttgaggcacgatggtattgctggtgtctttataccagaggccaaagcctttatcggccagttgatgccagggaaaccaggcgctggggtctacttttctgcccggagcgatatcgccatggccgatgaagttggcggcggggatattgtagcggtgctgaagggtgtccagtaatactaacaggctgcggatctgggcggaatcgaagggttccttgccgttgttgtccagctctataccgatggaagaagaattgatatccgtgaggttgccccatttggcgactcctccgtgccaggcgcggagataatcgttcagcatatgatggatggctccgttacggcatatcacataatgggcgcttacctgggttctttgcagggtaaacgtttgcagtgtttgtccacatgaattctgagcggtatgatgtatgataacaagactgggtttcctcatattgaagttcaccgtgcctacccaggagggggcttctgcgccgccggcgccattcagcgctcccggctgttcacgcaacaccttcgcgtaggatttagcttcctgccggtaaaccttattggtggcggcatatgggttacgggcgcaataagaaaggccgccaattgctgccagcaggcagccgtatctcgcaaatcgggctatggtcttcatctggaactgttaaagtttagacaacactacctgataaagatactaaatgaaccaatgcatcgttttttttacggatactatgaaaagtgttctttaaggtatacatttacattttcaataatacttttcgaagtatcaaaaacctgtgccacattgtctgctattgcctactacttactgttaccactgatctacgcgttatcgctactgccgtttcgtgtgctttacctggtttctgacgcagtatatgtgttgttatattacgtgatgggctaccgtaaaaaggtggttcttcagaatttgcggaattcttttccagaaaagagtgacgcagagatccaacgtatatgcaaagatttctatcattacctctgtgatcttttcctggaaacgtttaaaacgcttaccatcagcaaaacagcgatggtgaaacactgcagctttacaccggctacagtggagctttttaaccagctcgaagcagagaaaaaaagtgcggtacttgtaatggggcacaaaggaaactgggaatgggcaggaaatacgtttagcatactgtgccgccagcagctttatgttatctatcacccactggccaacaaacattttaacggtctcatgtaccgcatgcgtacccgctttggcaccaagctgattgccatgcaggataccttccgcgacatggtgcaaaaccgtggagaagtaaatgccactgcttttattgctgaccaggccccacagccgaaaacagcgcaatggctcaacttccttcaccaggatacgcctgttttcaagggcactgaaaaaatagcacagaaaatgaattacccggtagtgtatgtaaccgtgcaacgcgaaaagagaggctactacaccgtgtcggctgaattactgaccgccacgccggctgaagaaaaagacggcgccattacctccgcacatacccgtaaattggaggaggacattgtttcccagccagcaacgtggctatggtcgcacaaaaggtggaaacacaaacgccctgccgttatttaatcattttacaaacaacaacttaagatagatcatcctacgacaattatgctggaagggaaacaactgatactggctaccaagccatatgcgcgcgaagagagagccaaaagctggctctatacaatatcaacattactactgttgatgctggccttaacaggcaccctggtattgcctaacctggtacttaaaataatggccagtattctttccggattactgatcgtaaggatgtttgttatttatcatgatcatcagcatcatgctattctgcataaatcctggttagcggaagcaatcatggttactttcggggtgtatgtgctggcgccttccagtatctggaagcgttcgcacgattaccaccataaacataattcgaagttgttcagcgccagtattggctcctaccctattattacccgtaagaaatttgaatccatcacaccggcagaaagaagaacttacctgttcagccgccacccggtaacaattgcagccggttacctctcgatgtttatgatcggcatgtgtgtgcagtcttttttaagcagtccgcgtaaacacctggattctttactggcgctgatcatccatatcggtggcagcgcggcggtgatttacttcctgggctggcaaagctggttgttgtttatcctcattccgtttaccattgcatgcggactgggcgcctatcttttttatgcgcagcataattttccgggcgttacgtttaatgtaaacaaggaatggtgttatgataaggccgcattactgtcttccagctatatggtgatgaatcccgtaatgaaatggtttaccggcaatattggctatcatcatattcatcacctgaatgcacgtattcccttttaccgtttaccggaagtaatgcaaaagatccctgccatgcagtctgttaaaaccaccagcctgggcttccgggatgtgtgcgcctgtttccggctgaaggtatgggatcctgaacaaaaccggatgatcagcctgcgcgaagtacgtagcatcaggagggccctgctgaggagggagcgcgatcctgcagtagttgccggataattttcttcctggcatccagcatctgcgcgctgagttcttttgctttttgcagcaccggcaatcccgcggtatgtggcgatcctgccctgaatggcggcgcgggattatattccagttgcagctgtataattttagccacttcatctccggctataagtgctgtcagcaccaatccgaaatcgatgcctgcggttacgcctccgccggtaatgcggctccggtctctcactactctttcttctaccgtttccacaccgaacatccgtaacaattccagcgaacgccagtgagtagtagccttgaatccatcgagcaatcctgctgcggccagcaccaatgcacctgtacaaacagatgtgatatactttgcctttaccgcctgatcctgcagaaacttcagcactacggcgttggtaagtaacgcattgattcctctcccaccgggaacaaaaatgatatccagttgcggacaatccgccagcgctacctgtggctgcagcaacaggccaccttctgcctggataataccagtggtttccccgataacgatcacttcaaaacagggcgccttcacaaatacatcgtaaggtcctgtaaaatcgaggacggttaactcaggaaacaataacattcctactttcagtttttgcataacagcggctttagatggggtacaatataatgtaagcagcatgaaggcagggagcagcgcaaattgctaccggtgctgatcatacgtgtttatggttactgcctgttgcagtttttttatttcatccggcaacagtgcggcggatttcacagcgcgcagtgcatcttccagttgtgcggtggtgcgtatgcctaccacagcgctggaaaccgccggctgctgcaatacaaactgcagcgccgtttgcgcggcatcccgggaagccgtgctgaacgcttttaccgcagcggcggcagcgctcacttcttccgcagtatagttgaggtaaggcgccgcgggtttatttaccagcaggccttttgccacacttccccttgccagtacaccgatgttgttttccagcaataaagggaacgctgtttcttccggacgccggtccagcaggctgtattgcatcattacacttaccatacccgaccgctgtacatactcgcggatcacattgggacggatggaagagatgccataataccttattttcccttgttgttgcagggtttcaaaggcctcaattgtttcctcaattggatcgtcaatagtgcctccgtgcagctgatacaggtcgatataatctgttttcagccgttgtaaacttgcttctacagccgccatgatgtatgctttgcggggattccagtcccatccgctgccatcttctttccactggttccctactttggtggcgatgattacagatgatcttctgtcctgcagtgctttgcctatggtgatttcattttgcccgtgttcatagaggtcggcggtatcaaagaaattgattccctggtcgcaggcgtgatgaagaaggcttgcgttagcggcatcatcatttccgagcgacatgcagccgaatccgatttcactgacggcgaggtctgattttccgaggaggtgatattgcatgcgtttccgggtttacgatgttttcaacaagcgctttctgtgaaagtgcaggtaacgaagttatcaccaaaactttcatttttcacataaatccggtttaaaatagtgggctgttttgataaacagccccgatatcaatttacgtccacctcaaaaatgagctatgttgcagtaagcgcggcactgccgctgcgttaccatgtgttggtcaggagatggggccgcctggaaaaacagcccctgttttttagtatgtccgatccattgttgaatgaatttcgtcaggatgatccggaggaagaaatcaggaccatctggaaagatggtcccttcctttcccaaatcaaattgaacctatgaaaaagcgttgtatcaggaagactgttgccagcctggttttcaaagatggggaccgcctggaaaaacagtcccccggttttccgaatcaatcgcagcataaatgatctcgttttctacactgatcggtttaacgtatggctttatatttaaacaatatgcagggtatgcgccttcatattggtgattccggtaatggggaccgtttagaaaaacggtccagggcataaagcttccatcgtgtatgttgcactccaataatcttttcatataaaatttttatgggattgaaaaacaggggactacctgaataagtggccccgtttaacatgcgtcgcaaagacttcaactaaatgttcatctcaatgttaaaaaaaccggactgcctggaaaaacggtccgttcttgtatgtactatcaccccatgtgaataggatttgattggttaactgtagccgggaacaaacaatgaatacctttagctgcaagtgtacatgctgctcccctaacaaccatccggtaaaaccaggtctgaccagttaccgcatatcaatgccggtaatacatcaccattttcctatgcctgatcttcctttatcctgatcaggacctggcgtaccgaaagcaacagctgttccgctaattcaacacaaaaaaaaataactgatagtggtaatgtccaagaaatgtgcatgtttgaaaatgccggttgaacaaaaaagattgcatgtgggttaattttcgttttcaataaataaatacaaggaatagccagctatttggcgctgctaataatggttgaataacctttgtattgtaaccgggttaactgtgacaacaaggttatataaatgctccagacaaactaaaaaaacagattttcggtaattcttttcagcgatatgttcatcgtgataatgcaaaggtagggagttaccgttcccggagaacatgttttgcagccattattacaatgaacaatcctgaataaaataaaaaaatgctgaataaaatgaataccggagatcaaaaaatttgttgtataaatatcatattctgatggtcagaattaacaaatcaaccgtatattcattgctataatttcatatgtaccttaacgttagttattctatcccatgcaacaagaaattacaggcgctttttacggtatcgctatcggcgatgcattgggcgtaccggtagaattcaaaacgcgtagttatctctcagaaaatcccatcaccaccctcacgggatatggatgctggaatcagcctcccggtaccttttcagatgattcctccctcactttctgcacagcggaaagcctgataaccggttacaaccttcaaaacatggcgcagtcgtttgtgcgctggtcatcggaaggttactggggcgcgcataacgaggtatttgatattggtcatactacccgccgggcgctgctgagggtaagtaccggcacgtcgcccctggtaagcggtggatttgaggaatttgaaaacggcaacggatctttaatgcgcatgatgccgcttgccctgttcctcaccaacgaaaatgatatccatacgcgttaccaggttatccgggaagtgtctggcatcacgcaccagcatttccgctcggtactgggctgttttatctacgtggaatttctccgggcgctgctttccctgaaagacctccgggaggcctatttgcagatgcagcggggtgtaaacgcctacctgggcacccagccttttaacccggcggaaataaagcgctatgagcgtgtattacagcaaaatatagctgctatccctgaacaacagatccttagctccgggtatgtaatacataccctggaaagtgccctctggtgcctgctcactacgcaggattaccaaagctgcgtgctcactgctgtaaacctgggaggagatacggataccaccggcgcagtggccggtgcggcggcgggcctccactacgggtttgaccagctgcctgcccagtggatcaaccaggtggtaaaatcagcggagataggaaatctcgccaaacgctttatggcggccattaatactactagcacccagtaaacagccgcatttcagcaaaccggccgcatttttgcattatatggtattgcagttaaacttcaagccccctttaccgtctaataaatgacagcgaaagagaactgaagagacgattaccaaatgttaaaaaaatgaaaaacagactttatatactgtttgtgctggttggcctgttgggcacatttacagtaagcaacgcctatgcgcaacgtgttagctcaggtcagggcggtggccgcggtggaggtcatcatggcggtggcggaggattccggtcaggcggtagcggcagggtatacgcgtccccccgcatgtattctccacgggtagtggccccggtaaacagaggctattatcacggttatcgtggtccggtttaccgcggacgcgtatattacggacgtccctggtacagaccttactacaacccgttcttcccgccattgggattatatgtttcctcattgcctttcggttacttctccctgggcgcctcctttggtccaatgtactattacggaggaacctattaccagtcgaccggcgataccaaaggctataaagtagtggaagctcccgtcggcgcagcagtaccggacctgccggaaggcgcagaagaaatacaggtagacggaaatacctattacgaactgaatggtacctattaccaggagtccatgacggataacggcagacgttatgtagtagttggcaaaaatggtaaaataggcaataaaacagtgaccattaatgatgaccagggaaataacaatcccgataacggcgcaggcaacagtggtacagatatggtttcacagctgccggataacagccgctccgtgaacatcaatggtcagcagtattacttatcaccagacggcatgtattaccagtctgttctgaacagcgataattctatcgcaggatataaggtggttggtaaaatgaatgccgataattaaaacaacatagttattcagtttaacaggagagccggttttacaccggctctttttttattccgggagaaaggatttaccagctgctgcttgctccgccaccgcccgaagacccgcccccccagctggaagaagaggacgacgacgaagagcttccggaagaagaagatgatgatgatttggatatctttggaataacaaactggtagtcatgtgcataagcacaaaatgcacaggcatattccttgatgccccacccttcggaggaagtggtggcgcgctttttcgtcaccgttttcttacacttataggttttatgtttgcaagatgggcaatctgccagcgcggagcgcatattcgtgtaattcagtactgtttgggtattgcaggtatcgcagcgccatacgtcatagtcaaccgaatccagttcttcctccaccacctgccccttttccaggtaggtgttatcatctgcttcatccagtttatgcatcgcatgtgtgcattgcgggcaatcatacacgtcgttccgcagatgattgagccggttcttcagccacatcatatacagccataaatagggcagcgggaacacgtaaccggcaatccgcagatccctcctcaatacctccagccgcagccatttcaggtggcggtcatcatttctcagcatcactgcagaacggagcatgatcagcaacaccgctgcatgcataaacaccagccacaccaggtagtagaccaggaatactttcagaaagcctacatctgtgtgccgctttgtagcgatataaaaaatggtatagaaagcgatagcgtgaataatgatcaggccaatccagcgtggacgcaggaattcattgggaacagccgttatagccaatggttctgcatccggatcatcttcgcgccgctttacctttttcccgaagaaaacatgcatcattgccgccgaggcgaataaccagaagataatggcagtaaacgagaaatcgccggtatagtcattggaagcggaattggtagcctgatctgtactggcaaatgattggggagctacgtctattacgtcaccatctgtcgccggcacggtggccggcatggtggcctcatctccggcaataactatggtatcggcagccatcagggaggaatcagcccggggcagatccggcagcatattgtatgcatagttgccgttatcaaacagggaggccactgacttaataccgtccgtaaaggctgcatcatagttgtgctctttgatgcgcgggatcatatattcctgctggatacgaaaacagataatatccggcatatctgcctcaagaccataccccgtttcaaattcaagtttacgggcatcttccaccatcaggatcagcagcccgttatttttttccttatctcctattttccagtaattaaacagcttatgggcaaagtcgcgcgtttcattgtcgccgatactgtgcagtattaccactgccacctgcgccttaccggcgttatccagggctgataacttttcattcagttcattcacggcagctgctgaaatcagctggtcgggattacttacataccccccgccggattttttgggatccggcacatcttccacgctgaacttttgttttttgctttgattacacgaaggcaggaaaccaatcagcaatgccagcaacaagcatctcaataaaaacggttgatacttcatcagaatattttctgtgccgaagatatgtttatttaattttttctttcaacagaagaaagtattttaactgccgatgaagcccgtaataaccacctggataataatattatgctttgccgcgacccgcagttttgcacaggccaaaactgccgataccaccacgaaaccaccggtgcaactgaaaacagtgaatattgtccggtataatttttttaaagattctgccgccttccgggaagaatacagcaaagagatgaccttccgccggcctaaatggttcgaagtttacaagatcaccgccgtagatatcaacaaactataccgggttacccaatttaagaagaataaaaagaagatcgccttcaaacatatgttgctggataaagaacaggagatgtacgtaaacagtgtatacaccccctccatggtgaataaagtgacccggctcgatggcgacagtctccagctttttatgcggtactaccgccctgactattcatttattaaaaacgcttccgactacgacatctatgcagatataaaaaagcactacggggcatttattaaaacccgcgacagtataccatctccaccataaaacacgccgcaccggcatttctttggcgtcccctgcctctaaaaatactatatttcagtatccatacgttttactaattcccgctattattgcggtaatggtaactgctgtggcaaagattacataaattagtgatctcaaaccagttaacgttgttagttttaaagattctcaatacagctcacatgaaaaggcttttcatattggttgcccttctcgtgccggtggtactcaccgcgcaaacgaaactcagtcaaaatatcgtagacgatttctccgcccgggtggccgctcactaccagctgccgcatgattccatcaccgggtacatcgcagaacagctcacccgcagcggtaatgccggactggatatcgactctactgtttttgacctgaaaaaagacccggtagctttcgatgccgcgctgaaatacctttaccagtacagcgactgtaaccggcaacggtttattaccaacctgcgcagtatgggacttcaaaccaacagcgtattccccattgccacctacaccgccaacaaatataagggcgaagtgaaagcgctcatggaagataaaacggatttcctggccacctatacaggcccggtaaccggtaaaaagccacctgctaccattgcggaagtagcagcagccaaccaggcagcagccaccgccccggccagcaccagcagcggcaatgaaagcaccgccaccacggcaactggtaatgcggaagctaccacctctgcaccggcagcggatacacgtaactgggaagtacgccccctgttccaggtacgcaccccggaacaactggtggaaatgtacggcgtcaataacgttacccagcatgatgccatcaacctctccggcgaaaaagaaggcgaggcttacctgatctatcctgataccgacaatgaactggaagtacagtttgacggcgaaaatggcaacatccttaccttttcgcactacccctccaaatggaaatcgccttatggcatcaaagccggcgacccactggataaactcatcaaggtaaatggccgcccctttaagctgaacgcatttgaatggaccaacggcggaatggtatccagctggaacggcggcgccctggaaggcaaaagcgtgatcgttatactgaaagccaataacaccggcgatcccaagcaatacgaccaggtcaccggcgacaaaatactccgctccgatatgcctgcactgaaaaaactggacgtggttattgaatcggtggcattcaaagccgcgaattaagcggatgttgtctttctcaggattacgctgattttactgattagtttgatttttactttttgattttataaaagattttaaaagattttgggagatatcagcgatatacccgctgatatctcccaaaatcttttaaaatcttttataaaatcaaaaaaagtaaatcagtaaaatcagcgtaatcctgagaaagacaacatccgctcttgcacttttcatttgtgctcattatcttgtttgtatgaaaaagtttttattatccggcggcctcctctttctggcgcttaccggtatttctattcacatgagcggacaagcaaagaagtatccatcgctgaaccacatggcgttgtacgtagtagatctgaaaataagcacggaattttaccgggatattattgggctggaaccaatggaagagccctttaaagatggaagacacagctggttcaaagtgggtgagaacagccatgtacacgttatttccggcgcagccaaagccactgcgcacgacaaaaacacgcacctttgcttcagcgtgcctgatatgcaggctttcgtggaagtattgaaaaagcaccagattccttttgaagactggccaggcaaagccggtgctatcaacaaaagagtggatggcgtacagcagatctacctccgtgacccggatggctactggctggagatcaatgacgataaatactgatcatacgcggattttgtctttctcaggattacgctgattatactgattaatttgatttttacttttggattttttctgatttaataattaagggagataagagcgaatatatccgcttctatctcccttaatcctttataaaatccaaaagtaaaaatcaaattaatcagtataatcagcgtaatcctgagaaagacaaaatccgcgttatttcaattctttctccagcgcagcagctttcgccgcagcagaggcatcggccggaattttctttaaccaggtcaatgcctcctttttatgctgcgcctgtgcgtgatacagggcaatataaaacacagcatcatatttaaatactgattccccttcgtatactttcaccaggtctttcatacctgtttgcaccgcacccgtttggataaggactattccccggtaataaagggcggtttgactgctactgtctgttttgagatagctctccagtaaagggatcaccttcgtgtaggccttctcgttaaaatataatgcagctgactgtaacagtgtatcctcactatttccccgctccgcggctacctgcatttcaatattgccataggtatccatgtaaccggtatcgcgggaataaaagcggaataagaagatcccgcccagcaccgctgcggccataccgattgtgaccaggtactttttaaagcccaccactttccctgtacgccggaaatgttcagcacgttgtgcctccagggtggttttcaactgctgaagccccggatcaggctttaagcggtccgacaaggcagcagtgacctcgcggtattgctgtaccgatgcggacaaagcagcatcttcccggagggcggcttcaaattgcagcagttcatccggctgcatgtcgccttctacgtaacggataatatcttcctggttataagcagccatacactaaattttctgagcctgaatataggataacaatgtagccatgcactccgattttttcttccgcagatacccataggaaacccccatggccgctgcaattttttcctgggcttcaccggtcagcgattgccggagaatttcccggcacttctcccccaaccgttcaaactgtgccaggtagatgcctatccgggcttcctcttgtaccacctgttcggccgcggcaaatacatcttctcccacatcatataaatcatccagtctttttgttaccggctgacggcctcttttttttagttcattcagccatttccttttacagatcaataagaagaacggttcaaagggacaggtaagctgcagctgtttgtactttgcctggcgatatacatctataatggactcctggaaaatatcggctgcatcatcttccgtaccctgatgttgcaggatatggtgtttgatctttcccgcaaaacgctgataaatctcctgcaccagcaacgtatcgttctggagcagaccttcaaggtatcgctggtcggggtgaatactcatctggaagtgattcgcatgggttgacaggaacatgcgctgactaaaagtacatctttctaaaaaaatattccggaaagggggtaacaaaataaaagggctgttgatctactatcaaacaagcaaaaacattactcaacaaaaatatcttttatgaaagcgatcaccttaacctcgatcacctgcctggtagctgccgcactggctatttcttcctgtaaaaagaataacagccaggaaatacctggcccggaaaaaggccaggacgctaaaatgctggccgaattcctggacggtcacgcccgaccatttgaacacttcagtataaatgcagcagcgggcggtgttatcactaccagccagggaacaaaattcaatattcctcccaacgtttttattactgccggcggggcacctgttacgggcgcagtagatatcagtatcaaagagatcagggatgtgagcagtatgatcctgtcggacaaagccactgttactgccgatgggaagatgctggtatcatttggagaatttttcgtgagagccgtccagaacaatcaggaccttggcctgcgaccgaagaatgataccggcaaaggcatcatggtacaggtacccgccagaccggcagataacgtactgaatggcatgaaagaagtgccgatgtggaacggcgacaccaccgtatctgttacccagcacggctttaactacatcaaccagcccgtgaccattaccaccgagcacactatttcgaggggcgtgttatggaaccagatccagagcagttatgcactgttcaattcatccaatggctccatgaacttccggctcgacagccttatccggtgggttaattgcgatggactggctaatatgcctaatcccaaaaccacggtgatggcttatttcactaatcactttaacaatgaaacaggcagcagctacggcggcgaacaacccagcatgctgttcttcaaacccaaaaactataatacactggtaaaattctacaacgttattatgacgcctcccgctggtaaagaaggcttccatagctaccagacctctatccccgtaggactggaaggcaccttcctcgctatcagcgctgtaaatggccagctgtatgcagaacagaaaacagttaccatcggcacaccggcaggcagcgataactattccaccgtaagctttgatctgcaggctgtggatgccgctacgttgttgtcgttaattaacagcatgaattccaaataaccggcctgttatccgtttacaagtactccaaatctgaaggcaataagtcaatcccccggttggcttattgctgcttttatataatatttatttatatttatgttatatgcaacctacagctctcctggcagcactattacttttctttcaaagcgttgtgatggcgcaatcccctgtacctccatcatttccgcaggatacccttcctccggaaattgaagtacaaggtaccgacgacagtatgcacctcgttgcaaagctgcgcccactgcgccagatagccggcgcccccgcatctttctatacatatttctgggaactgggagatggcacgtttagttttagtccaacgccggaactgcactacaaagataccggcacctaccaggtacgcctatacgccaccaataactacgacgatggtaaggcgccgcccaccaaacccaggcccataaaggtgaagaagcctgtaaagaacagcgcctgggcttcccgtttctttcacggaaatgggaatatagagatgaagataaaccggaaccccaaacctggcgaagacttcatggcgcttattggctaccggaatatggccggcgatgcgggcagcggcaccctcctgttgttttataacgagaaacagtttgggcatgctgcatttgatcttacagaaaaaagaagctaccacggggaagacagcagctccctgcaatccttgctggctcaactggaaacgcccggtattgaacccgacgtagcactggcccatggcccccatgccggcttacccgcagtgaacaacgctgctgccaaagccatgttacaggccatgcagggcgcatatagcagtcataccgtattgcacttcagcaatgccggcaaaaccgcagaacaattccttttcctcaacatgcacacgctgccggaaatggtgcaggacaccaatgcaaccgttaccatgaccgccatgatggtgcccgacaacgcgttggcgcaaccggaagtatatgagctggaaatggccgtggtaaattcccacgaccccaaccggctgcaactgcggaaacaccggatcaactatcgttttatgggaaagaaaaaagaactgacctataaaattcaatttcaaaatacgggtaaagggcccgcaaaaagagtggccatcggcatcgccgtgccacggcaactgaacacagaaactatacagctaaaagaagtaagccctgcttgcatcgcctgcgactccgcctatcagtcgcaaagctgtatggataccgtgcggacaaaagacagcatctattttgttttcagaaatatttatctccccggccttcagcaggaaggtgttaccgatcctgattccaccaaaggatttgtgcggtactccattctgtttaaaaagaagcccaaaaagattcctttcagcagcagcgcggccatcatctttgataaaaacgagcccatttataccaaccgcgccactgccaggtttatcaaaggattttcccccgggattattgccggctacacgttttcccctaacagcggcgactatacgctgaaagggccgctacaactcggcgccgtattggcgccttttgcacccgaccgtccttactttcaggtggaagcctttgccggcctgctggaaaaggaatcttccggaacaaccatcatacgcgataaacgggataccaccgtaaacggccaggtgtacctgatcaggggcaggaatgaactcaccaccaccacgcggcagtcgctgcaactggtgccgttacatttccggtataacctcaacaattggatcggtgtaggtattggtgcgatggcgcaaataaatattgctatcaaaactactactgagtcaaaagtatacctgaccggtgtgcagcaacccgacgtggtcaccaacacggtcagtaaaacgctcaaagatgatccgcaatggtttgccagcatcaacgcggcgccctttgccgatatacagataggaaaaataaaaagcggaccggcaattgggttgcgttacctgcggcaggtaaccggtaatacgcccgatcgtttctttgtatacgctatctacaaactgtaataaatcataacttcagccattataccatggctgaagcccgatcatatatcacctacctgaaaaaagtactgctgttactggcggtatccggtctgttgatttcctggcaggaccctgaactggcagtactgaaaaaacaccaggccgccaaccggctggatgagtggatctacacctatattcaatgccctgccgcttcgcctgcagaaaaggccgcacagctgaaaagagctgcagccaatgcctggcgggcgccccggtctaccgatgaaatacaggcatggatggacctgctcattaaccagggctattccctgttgcaaagcggcgatatcatttcctctacagacgcctaccagcaagcctttgaatggggccggcaacacacctccgttactgatcccggcctggtactagaatatatcctgaagccgctgggtaacaattatacgcggctcggcgactacgaacaggcgttgtttattcaccgcatagcgctggaatttgcccgtgagctcaacgatcgtgaggctactgcagccacttacagcaatctcgctaacactgccgccaacatggggcagctggaacaatcgcttcgatactgccaggaaggcctgctgctggcggataagcacagtgctacctatggtttgctgttgtctgagcaggcagatgcctgccagcagttacgccagtttccggccgccaggcaaagtattgcgcaaagtatccgcatcctgcaacagcagcccgccggcaacccggaagccacgcactggctgtttatggcctatcagcaggcaggcgatatttatctcgctgatcccaaaaccgcagcacaatactacttccgtgcgctgtccatgccggaaagccaacgcaccctgcgaaagagggaacaggcccgcctgttcctgcgtatcgcgaagttgcaagcttcgggtaagcaaccggcaaaagcgcttccctggctggatagctgctcaaaaatattactaccgggaaaggatatacgcaaagttactactgaagatgtttatggtgaatacaccctgctggatctcctcttcaccacagcatcggtgtaccagtcgctcgggcaacccgctacagcactgtccttataccgcctgagctttaccgcagaaagggagttgcggcaccagtatatatccccatcggccaaagaggccgctatatcagatagccgttaccgttatgaagccgctattgcactggcctggcgctgctggcaaaccacacaccaggcagcttaccagatggccatcctgcagtttatggaagacagtaagtcgcagttactatgggaagaaatgcagcagcagtccattcattccggcaacgatactatccagaaacgaatccggctgctggagcaggcgcagctctactaccggaaagaagcgctactcggtagtaaaaatgatagcttattgcagcttcgccagcagcgactggcctgggacctggctactttaaggaaaaaagtacggcagacagcacataacggcaatgaattgttttcgcccgacagcctgctgcaccggctggctccccgccagcggatccggacttactttgcaggagagcataccttatacagtatagaatcggatcaccagggtatacggtatgcggatagtacgccgctggaccgtgatgcgatccgctattttaagcagcatttttttggagaagggccgtcggccatggtgaaccatccgaaggcctatcaccaggcagcataccgcctgtatacgcaaatatttgccgggcacccattacaggccggctacagttacctgctgatgccggatggtccgctcaacacactcccaatggacgccctgataacagaccctgtatataaatccgccatcgggcaatggtcctttcttgtgaaacaggcaacggtatcttacgcttattcattgcgcacctggaacctgcagatgcaggcccatagcaatcccgggggcttcagcggtttcttcatttcgcggcagcacgccggattaccggatctgcagggagttatgaaagaaaaagagttgctggcgccggtgataaataacgggcaatggtttgtgaatgaacaggcacacagtcaacagttcaggaatgcgttggagcaatcgggcattgtacatatcagcacgcacgggttcactcaaaaggatagcaccgctgccccgcacctcatgttgtatgatgcgccgttctacttatttgaattgaatggtattgtccgccaccccgccctggtggtgctgagcgcctgtaaaacaggcgacggccgcctggtaaccggggaaggcatccagagtatggcgcatgcttttatggcgggtggcacgcctgcagtggtagccgcttactggaatgtaaacgatgccactgctcccctgctgatgcaacaattttatgagcaactcactatacaacacaatgccgccactgccttgcaacaggccaagctaaactggcttaaagatcccatggtaacggacatgcataaacttccctattactgggccgcattgagcttccaggggaatacggcggcggcagtcctgtcttcttcccgtttctcctggtattggctgcttttattgctgctgataccggctttcctgctggtacgcaaatggattcgttaaggaatcatgaacagtccaccgaattcccctttttttccttaaattcattgaagagagtcttcagtcatatcctgcttttatgtcattactactgaatgttcccaacgcggaaaaagagcatgctgcatctatgggcgcccaatgggatcaggtggcgcgcgcctggtacttaccggaggaccggtacgaccggctcatagaggtggcccggtggataccggaaaagcatcctgccattattctgcccaccgaaataagtattgtgcaggctggcaggacgtgctggaaatgccagcacaataaccgggtaatagcgcttgccggtaattatttttatgagaaagatatgaatgagcgggatgagtcggtatggctggcgcaggatttctttacagtattccagcaggtgtccagcatttcagataacctgcaaacgtttctgaatgattactatccgcgttacaaacgggcgtggtcaaatacactggggagtcattgctggtctaatcattgcgaatcatgcgacagcatccagggcgactggttcctgtttgatgaagcaggcagcgtgtttaatcctactgtaagagaagaggctgcccggctgacgatcaggaactataccctgaaatatgcgcccctgatcgatgcagtttattctctcggagatcatgcacggctcatcaatgaatttgcagaaagagcggatctataatttcacatgtgttttcaggaaaataaaatagcggggatcttcttctgcaaaaatctccttcccttccagcatatacgcccttaacaggtattccagcgattgatcatgctggttcaattcatacaggctttcccccaggcgtaaattcacaaagccgttggcctgtgcatccgggccgtttaaggcgtcataaaagctattggcggcggcctcatagttgcctttaaagtaatacatatccccaatgctggcatacaaccaggtactagcttcccagttccgcgccggttccggcaggagctgcaaagcttcggtaaaccgggcaatggcgccatcaaaatcatctgcatccgccagttcgttgcctgcctcagataaagcttctactttttcgtggatatctgccggcagttcttcctccactacagttgccaggccggaaaatacatgcaggtatttttcatccactccttcaaatacgcgcccggcagacttatgcatagccgtagtaaaatattcttctgctcctttcatatccccgttttcaaaacgggctttacccagcacaaattcacgttcaccatcttctgcacgcgcaggatcgcattgttgtaaggtatttgcccagcggagcatggccggaaaatcttttaatatgaaataggtttctgcaatggcaagggcaatatgatagctctcgtcatacacctctttaggtgctggcagcagttcccaggcttcttccagcttcaatgcatacctggcaggatcattgttttcaaacaacacctctgcttcttcccagatgacttcaatagccgccacaattttctgatcgtgtaattccatatatcccgttttaaaaagtccctgtacaaccggaattgtacagcggccattcagatgatgccgctttcgaaggagcgtatctcacgttgtaatttttcgcctttgtattcttctgcgagctgcaatcttcgcagcccgatctttacatattcttcctgcatttctataccgatgcaattccttcccagctctttagccaccgcgcaggtagtgaaagtaccggagaacgggtccaggattacgtctcccgggttggaactggctttaatgatacgttccagcagggcaacaggtttctgggtgggatgattttcatattcatccatgcggtagcgtacccgtgcaaagtcccatacattgccgggaactttttgcgtgttataggcagccggcgtgcttttccggtagtcgatcagtttcctttttgcccctgttttggcttcaatgagaatatcggctgcattgaaagtgtagttgtttttatcgtttacgcaaaacaggatgggctcatacatggacccaaagtatttcctggcctgtaccccggagctatcatagctccatacgatgcgggagagaatattgattttctgacgcaggtaaatatcaaaataaggcatgaactgggtggcggtcattacataaaagctgccggcaggtttgagtttctttaggcaaaggtccagccactgatagcaccagttaaggtattcttcttccgtatcccatttttcaatatgtccattaaagtttttgccgatattatagggaggatcggcgaagatgagatctacagaatgatccggcaccagcgtttgcagcgcctgcaacgcatctccatgtattattgtatgattgtggttaccgaatacttccatttccttcttttctgccgataaaattagctaaaaaaaggccaggataaagataccctggccttttttagcggaaacctgcatcagaaggtgatccacacgatatatgctttcttgtcatttcccttccgttctatcatcagggtagctaacgacttattgtcatcgctgtacgcgttcatctccagtaagctgaacctggcttcatcttttctgcccggatcaccaaacaggaaggtctttttcaccttgtcgccgtcgcaataggcaattactgtattgaccgcacttaccgcgaccattgttttcttcctacggtagttctccgtgctatccgaaacatttaccgggacatcgttaaaaatgctatagccaacattattcacaaacatgtagtcgtaagaaaggaatccttcattataggtgcctgttttaaagaaaaccctgcggaaattccaatcggtttggggtctgcggtaaataaaataaggacgcaataaagaaccggtatgttgacttttcgcaatggcataactgccgggtgtttccttcccctcatcatcgagccttacaatcccgatatcaccaaagcgggtactataactggtacggttactggtagagggtcttccattgatataggtggtagaagtataatattctgtttttgcttccagctcttcatacatcagcgtgatggaattatcttcattgatccggaaatcctggataacaccataatagggtttcttatatttcaggtgttcctttgcgtagtccgacaataaaggatgatcaacaaaatactttttgcttaccgctaacgcaaacggatcgatgacactcatctgcaataccaggttttcactggtggtatacatcgtgtagggccggcctgcgcttttagcatttatagctgccagcaggtataaattcttattggcgctgttgtacttcagggcaaccataggctccttataatcgtcggtataatccagcagcttgtgttcgaacgccttttcgcctttggcgatgcgggaaatcagtatccgggaatcctttccggaagtttttgtgttatgtgcaaaagtggcaataaatacaaactgatcctggtgcacatacatgcctttaaattccatgtatttaaagccgccgttgggggattcgtaagatgcttcatttatttctttgtgatccgggctgtaatgcgtgactttaatcatttcgttactgccgcgctccagcgagctgaatcccgccacggcatagtactccgagttgggatccttacgtacctgggaatccggcaggtctgaaatcatttcttctttgaccagcttacccgttttaccatcaaaaataaggcggaaaagacaggtcttcctgtgtatggcctgctttataaaaacaacgccctcgccattcatttcatataatcctgcaagggaagcattcttcgtcttctttgccttccatgatcttatccggctattcactgtggaggaggcatgatgctttttgtcgtatacaactacgtcaacacccttttttgcggtaaagtggaagaaaagcgtatttccatttttcatcagcagtaaccggctggcgccatcatcgggttcgtcgaaaggtttactccgggttatttccggcgcctgggccaatagcgttatgggtaacaacaggctgcaaaggcaggccagtaacagatttttaagcataggaataaaataaacagcgcgcaagatagaaatagttattcagccgtgaataacactaaatggggattatattattatattcgtataaatactaatggaagatgagcctgcaaaaacccatttcaataaagattttcctggcgatcttatcctgctttgcctggtttgccctgatcccacagtttttcatcaccatcggcagtaaccaggcgccctggtttgagaatttcatccggtatttcagttatttcaccctgcttaccaatgctatggtagccatttccagcacggtgttgttagtagcgcccaatagcagctggggacgattttttgcacggactaccaccgctaccgctatagcggtgtatattactattgtggcactgatatataacgtgatccttcgccccctctaccaatttgaaggattacaaaaaatattaaatgaagtacaacatgtaatcgtaccggtactatttgttttatattggtgtgtgtttgtgaacaaaagttcccttcaatggaaagacttccttccatggctctggtatcccctggtttatgttttatttgtactgatccgtggctccttctccgatttttacccttatccgtttatcaacttaaatgatttaggtttccgtcaaacattaataaacgccgttggaatgggcgtgctattcaccttaatgtccctggcttttattggtgtcgggaaattatggtcgcgtaaaaaataattattgtcaggggcgggtgctgtagcctcttaatttcgcccggatatatttaccggatgctgtgagctgagcagctgtccagcccccatttgcgggcgcaccgggcaacaggatagaacataactcgttgggcttatcggacacggaccagttaatccagcttacctggttgctttccaggaacgtaaaccacgcctcccattgcgggtagtcgatgtggccgctgccggtagcttccgagccattacactctgttacaaatacaggaatgtttttgctgagcgcataagcacagtcatctctcagccactggccatgtgacgccgcatagaaatgtaccgtgtacataatattactgtagccggttaaaggtgcatctgctacttcgcggatcttctggtcccagtgcgggcaacctacaattataatattatccggatcatatgcgcggataccggcaatcaccgccgctgcataggatttcacctgttcccatgtttgcgttttattaggttcattgatgatttcataaagtatgtgcggatgatgaccatacgtttgcgccatcaatttgaagaaggcgaccgcttcttcctggtgaaatgcttcacaatgccagtcgataattacatagctgcctttggccagcgcggcgtcaattactttcttcagcagtgcaagctgtcgggcacgatcattcagataagcaggcgttgcatcaacgcccatggcggcgcggacaatatctgttttgaaatcatccgtcagccagttcactacgcctgggttccagtactgcggccaccaggtgctccagccgaaactttgtccgcgcagggatatagtattgttacgctggtctttcaggtagcggccggatacatgcaacgcgccataccgccgcaccggtgatcctgccgggagcgtgtctttcggaggcttatcgccggcatccgaccgggccggttttgcacaggcaaaggcgcataaaaagaacacaatgatgtagaaagataacgggagccgtttcatatgctgcataatttatactgctttcttcggtgaatctttccccgactgcttgatataggcagaaggcaatacaccgaattcagctttgaaagattttgtgaaataatgcggggtattaaatcccacttcgtatgatatttctgcaatactcagctggcttttttccagcatcagtgctgctttccgcaggcggatagagcggatgaaatcaaccggtgttttaccggtgagcagcaacatctttttataaagcgataccctgctgatgcaaagatgcctgcttaattctgccacactcaggttggcgttctgcaggttttcttccacatatgccaatgcggcagcgataaatttttcatctacagattggatggagatatccgccacctgcacctccacctgtttggtatatacttttttgatagtggtttgtaatgtaagcaggttccggatctttgacaccagcatttcaaaattgaatggcttacagagatagtcgttggcgcctgtttccagtccctttatctgatattcctcgcctaccaatgcggtgagcaggataatcgggatatgcgaggtgcgcttgtcctgtttgatttttgtgcacagctccaggccattcatttcaggcatacttacatcgctcacaatcagatcgggatgcaatgccagcgccttctgccatccttctttgccattggcagcttccagtaaacagaagtactcctgcaaattatctttcaggtaaaatctgaaatcatcattatcttctaccagcaaaatggtaggtttcttattcttttcccgttgtgtaacggcggtttgctggttctctgtaactacctccccgttttccgccggttctgttttcagcggcagctctactataaagcaactgccgccattggtaatagattctacccggatgctcccctgatgcaattttacaaactccctcgtaatagataaaccaataccactgccctggttgatgagcgaggctggaatatcatgctgatagaaacggtcaaagatcttatctactttttccgggggaataccaatgccggaatccatcacattgatgcggagggttacggtgttgccgctttcatctgccgggagacaattcaggaacacgcctacatgcccacctgccggtgtaaacttgaaagcgttggaaagcaggttgaataaaatcctttctatcttatcatagtcaaaactggtttcaagggaagaaatatcggtatcaaacgcaaacttgatatttttctgttccgcaatatccataaatgaaaaagatacttctttaatgaaacgaataatatcacccgggcgggcatccagcttcagttcatacacttccatcttcctgaaatccagcagttggtttaccaggttcagtaagcgtcttacgttgcgtttgatcatatttacctggacgttctgttctgccagctgcggatctttcagcattttgtcgagtggcgctatgatcagcgacaagggcgtccggaactcgtgacttacattcgtgaggaatttaatctttagccggtccagttcatgcagtcgcctggcttcttccctctcctgctcgcggctccgttgtgcttcctgtttttcctgctcctgtaaaaactgcgtccgtatttttttgatacccctgtatctcaggtaaaataaacccgctaaaaccagcaacacataagtgatgtaggcgacctgagttttccagaaaggtggaaggatacggatattgatcgcgagtactttttcgttccaggtatcatgtacagtggatgttctcactttaaacacatagctgcccggatccacattggtgtaagtggctttgcggattttgttatcaacggctacccagttttcatccagcccttccatcttgtactgataccttactttgtcggggttcaggtaatccagtgcggcaaattctatcgaaaaaaagttctggttataattcagtacaatatttttggcaatggtaatagaaacaggaagaatcaccctgccatttattttttcaccggtatttacggtatgattaaataattggaaatctgtaaataccagttccggtaagatgttgttgatcttaatacttgccggattgaaaatattaaagccgctgcctccgccaaagaccatttctcctttggaggttaccagggaggcatcttcattaaactgctttccctgcaggccatcttttacatcatagttaatgaagttcagcttgtacacctcattttccaccgacactacggcattggaaaggccgttggctgtacttagccaaaggttatgatttttatcctcccggatgccgagtatattattgtctggcaatccatcttcttcccggaacagggaaaactgtttggtattgggattaaaaatgttcagtccctcgcgtgtaccgatacagatatatcccctgctgtcttcgatcatggaaaggatattatcatttgccaggctgttgggattatcattttcatgctggtaatgcacaaacctcccggtctttttctgcaatacgtcaataccgttcgacgtgccgatccagatatccttgcgccggtcttccagcagggtaaaaacgtagtttgaacggatgctgacggaatcttcccttcttaaatgcctgaatatttttgtttccggatcaaaaatatctacgccaccagacagtgttcccacccagatacggtgttcactgtcttccataatttcatagatcctgttatcagacaaactattggggttctgttcatcatgacggtaatgggtaaacgtttttccatcgaagtactcgagtccaccaaggtaggtgcctacccatatatgctgtttatgatctatacaaatacttacaagcacattggtgcttatgctttgcgggttagatttatcgtgtacgtacgccttacaagtacctgtttgcgggttaaaacaagtaagtccgccgccgttactggccagccacaggttgccttttgcgtcttccgcaaatgcgtttatgtcgctgtagttgagtccttccggtttcatgggatcatggctgtacaaagggaatttgaagagatccggataataataattaactccttttttataagtcccaaaccagatcataccggctgcatcgctgtacagcgtggtaatactattttgggaaatactgtttggattacgttcatccattaccaggttctgtacatgaaatcctgatttatcaagcaggttgatgccaccgggatcagtggcaatccacactttgccttgtttatcctgcattaccgcattcacaacatttgcggtgatcctgttttccggggcatctttatagaagtgtttcagcaggttgcctgaagggctgtaatagtaaagcccatcgccgctgccggtaaaaacccagatatcctgctggtggtcgatgtacagctggtacctggtagctttctttttagccagggttgcatacaaaggcatggccctgtataccactttacgggtacgggtgtcaaattgttccacccatccgtcgaggtatgcaatccacaggtcgccgcgatcatccagcgcaatatcagatatggcaatggaatgaagggaggtactatcgtttgcagcaacgcagtaggcttttatttgtttggtgtgttcattaaggatgataatgccatgatcggcatgtaaaaaataaaaatcgccgttggcgcccttcagtattttttctacctggtagccatatacctgcaacgggtgcagcaatttggctacatcatcattgaagctgtctgtttccggatcatagatagaaaagccaagctgtgttctgatccacaggcggttcccgggggcatcataaatctgggtaataaaattatcactgagagaagtggcatcattcagccggtgtttatataccttaaatttagaaccatcaaaccggttcaatccattcaggcttcccatccacaggaatcctttggcatctttgaggatgctggtaattccattatgggacagcccgttatttacatccaggtgcgagaaagcatacggtatatcctgtgcagaaacggacgtgcagtacatccataacaacagcaggtattttatattggtaagtttcatcttataacgcggacgcaattgaaaaaaggtatatccccgctgccggtagtgacagcgggcgatatgaaaatacgattcctctgtttaaaatgtatgctattttcgggttattcaatcaccagcggattttccgactcaatatccattggtgtgataccgtccgtgctgaataccagtgtgccggtagtggccgtggccggtacttttagcaccaggtctgtcaccgatttgctgacaaattccgttactgcagcatcatcgttaccaaaagtgacccgcgttatccagtttacaaaagtgcctttaatggtgatcgtggctcctttggcggcggaagcgggaaccgtggtaatggttaccggcacattgaggttcagtaccgttttggatacaatatcaccttcgggtgctttcagggtaaccactcctttctccgtttcctgcggcaccgtgatgatgatatgatcggccgtttgttctgagaaggccgccgcctctacggtagcgcctttcagcacgatggcggttaccttattaagattggtaccaataaagccgatcttctcgcctggctttgacccggatgggccaaagctcaggagtgttaccttatccgttttaacggcatcgtcgtcgtctttactgcatgacatcagtccggcgatgagcaggagcagccaaagcagttgtttatataaaatagttttcattgaaatgagttgagaacttatgaacacttattttttaatcacttttggcactacgcggaaattatcgaacgacatatcgcagtcgaggtcaccggcgccgctgaatacaatccgggtgtaatacccattgggttgcacggtttgtttggcgtagctggcggtcacttcttcgtagggaattgtcaccgtttgccatacgcctttggtgtcgtagggaggcatccaggagaagtcgccctggccgtcattcttcacacctacacaaaatttaagtgcattattgttgtagggtttcttcgtgttcagttcaaatttcaggttataattttccggtttcaggatcgcttcatccgggatatttttgctgatgggtcccatcgcatctgcaggtccgccggccagctccacccagccccagttgctgatgggttgttttacgcggatatagttaccattgatagcggcagggtcgccggcacccggattggttactacaaaagaggagttccaccaaccggtgaatgggtcgctgctgataaaaatgttcctgttatcgcggaaccagaaatcggaaatggcttccccgaaattggttttaacggtgatttgccctggttgtgcgccgacaggcacccttactctcacttgcttatctgttgtttccactatttcgccaacagcgccaccggtaaaggttaccgttacgggcgcatagaaaaaatcacctgtgatcacggctacatccccggcggccacatattcacaatccatccgggtaaccagtggtttgctgatttttaccgggaaattgtactcgagtttttttccgctgccgaagatgatctttagtttattatctacttctaccgggatctgggaaggtatgcttacgaggataacggtaggcgtaatgtagggttgtgtaagactggctttctgatcgttgaaccagatttccctggcgtctccgaggttctcccctacaatggcaatcagcacaccctgcccggcttctacgagcaaggagtcgctggtagcgggatctgtgagccggacataactgatccgcggctctccgttgttggggagattatctttgctacaggaaatgattcctatacacataatgagcaatactatggagctatatatcttttgcatgagtatattattttttgtaaaaagcgtataggcctacttgttataataatctactgccggtttcttcagattgggcgcctggcttagttctgctgcaggtatcggaatcaggaagttgccatcgttggcaataattttccggaaggatgcccaggatgttttcacacatttccatgatgtaggatcaggcattttatccggcgcggtggcaaacaagcccctgtcctgcgagtttaagatggcgtatgcttttgctttattgtaatagtgaagagctaccaggtcgtaccaggccattccttccatggcaaactcgacgatgcgttcgttaaagatcacatctgcggtaagtggtttttcaaaacggggtaagcctgcgcgggtatgtacggcgttaaaatactccagtgcagtggcgtctgtagtactggcgctgttacccagtaccgcttccgcgtaaatcaggtacatttcagacaaccgcatcatgtaggtatcgttaccatagttttgttgcgccgactgtccgcctacatcggcggccctgccggttacatatttcttgatgcagaggaaattgttatcaccggtgttataagggtaaattaatttaggtgtggtaccatctgcgagcttctctgtaatttccgggtagtatgcgcccggcataaaaaaggtggctttcagtctttggtccagcgttctgccactgatgagcgtatcgccggagttcacgaagccttcgtacttgctgatcatccaccaggtggcgcttttatcgccgccccagccatcgccgttgcacattttgctatcgtagttcagatcggacggagaagcattggaggcgccccagtcgcccggtgcgtatacccattgcagtgagaacatggattctgtgttattgtcataaggaaagaggaagaggtcgtagtaactcctcagcaatgaatatttactttttgtgatgacctgttgagagaagtatttggcgctgtcgaggtccgattgattacgggcgccggaaccgtttgctcctaacccggacctggccaggtaaaagcgggcgagcataccttgtgcggtccactttgtgatccggccttcgcgggctggtacttccggcaggtcttccgccacagcacgcatttcgctgatcacaaatttccatacactttctgcggtatttttccggagagaagtatcggaaatcaacttcaggttatcttcgataatgggcacttctccccagttcattaccaggtatcggtaagccagcgccctcataaaccgcgcttccgcaatagccatttttttagcgttggcagaaacttccggccccgcatatttattgatattggaaatagtgagattggactggccgatcacaataaagaacgaccgccaggacgcgccattggccgtagtattggcggtggtgttaaactccacattgtctttatcattccatgccgaataagcagtacccgccctgaaatcgccgatgctgatagccgaacggccattgtaatcagaccatactttactgtatagcaaagcggtagctgccatcagctgatcatccgttttataaaatcccgcatccacgatagcatctttgggtggacggcgtaaaaattcttttgaacaggctgccagtaaaaacacagataacagcagcgccccgtgatatatattgaatgtaccttttttcataaccagcaattttagaaattaacgcctagggcaaaagtgtagatgcgtgtgagcggataacgtccgaaatcaagtcctatagcctgattcccggagctggactcccttccgacgtaaccacctacttcaggatcgtatccggtataaccggtgagagtagccaggttttgcgcgccaaaagttaaccgggcgcccctgattattttttgctttgccagcagggaagcgggcaagctataagagagggaaacatttttcagccgaaggaaagaaccatcttccacgaacctgtcggtgatccggccgtagttgccgttcggaccactggatattctcgggacatttgttcccggatttgataaggacacattgccgtctttatccgttaccggtttggcatagtccattgcttctatcatcatgttgcggctaagattgatctggttgggattggagttcacccttgccaggtaattatatacatcattgccgtaagtgccggtgattaaaatactcaggtcaaatcctttataagaaaaggtgtttgtaaagccgccaaatactttcggataggggttgccgatataggtttgatcatttacatcaatgatgccatcgggctttccttgcggaccgcttacatctttgaacttcacatctcctacccagatattgtccacattggtgggaagacgctgcccggtgttatctaccggcacggcgcttttattgatttcgtctaccgactggaaaataccttcctggatatagcccaggaacaaccagggcgcctggcccacaacagattgctgcgtccagttatccagccaccaggaagtgcggttcagcacacctgcatctgtattgaactttttgatcgttgttttgaaccccgacagattgagactggattcccatttaaaatcttttgtgcggatgttggtggtgttgatggttacggcccatcctttattctccagggagccgatgtttacggtcggcgctcctactgcaccgatcccgttggtacccatataccagggcagtggaatatccatcaggaggttgtcggtatttttcacataatagtccgcctcgatgctgatcctgttattcaggaagcccatattaataccaatattattggtttgggtagactcccactgcaaccccgggttcgcataccgggatgttaaaaaccctgtaccggttggtgtagcggcggcctgcataggcgcatagataccggcgctccagcccgagttaccggtgataccggtttcaaatctcagtttaaggtcgctgataaaaggtacctggaagaagtgttccctggaaacgcgccatgctgctgaaactgcggagaaggtgccccagatattttcatctccgaagtttgctgatccgtctctcctggcagaagctgacaggatataccggtcatcgtaattataatttattcttccaagataagattccattgcccagtcgccctggccaccggagttggtggcatcggccgcctcacctgcgttcagatccaggatgtcattggtaagaaaccctttcctgccaccggttaaatttttccagttggattcctgcgcctcatggctcaccatcaggttaatattatgttttccaagttgtttggagtattcaatcagctgattccagttccagtaggtacttacattgcttccgttggtaagactggcccggtcgtttaccgcccagccaatagaataggtaggcaggtaattttctgtgttggcgaagccaaaattggtattgaaagtagttctgatgtaaagatcctttatagggtttatgctggcgccgatgccgccgatcaactgccgccttactgccctgttgatattcagattggcaatggcaataggattcaccggggtaaagatattggcgccattggtaagatcgccgcctccccaggaaccgtccatatttttcacggggatctgcggagtgagcatcaaagcgttagatataatattttcctggctggtggtgagattttcctttgtttggttgaagctgagattggcgttcagtgcgatccagttgcggggtttattgtcgaggtttaaccggaacccatacctgttaaagcccgaacccagtgcaataccttcctgcttcatgtattcgccggaaaggtagtaggtagttttatcggtgcctccgctcaggctcagctggtgtttactcatgggagcatttttgaagagttccttttgccagtcggtacctttacccagcagggaagggtctttaaattccccctgggtgttgccgcctgccagtgcgtggtattcatttaccatttgtgcgtattggcgcaggtccatcacttctacatgtggtggcggcgtttgtatattatattggaacatgtagtccattttagtatcgccggctttacctcttttggtggttacgatcagcaccccgttggtggccctggagccatacagcgcggtagcggaaggtccctgcaatacttcaatattttcgatgtcggcggggttaaggccggccagtggattggacgaactggttgacccaaaggagatggacgcgccgggcatctgaacaccatcaattacatacaacggctcgttggtaccattaatagagttcacgccacggatgttcacggagataccgccaccgggctgaccggaattctgagttatatacacgcctgcggagcgtccctgtatggcttgttccagcgtggtatttactgtgcggtccatttctttggaggtaatcgtagtttgtgcgctggtgaggttggcccgtttggccttgccataagccactaccaccagctcgtcgagcttactggtagcggaagtaagtgatatacggataacatcttcctcccctacacggatttccctggtttgataactgagataggtaacgaccaatacatctcctttggcggctgcaatagtgaattctccgtttaaattactaagcgccattgttttggtgccttttaccagcacggttgcaccgggtaatggctgcgattcacctgtaatcactccctttacagtacgggattgactgtaagcacgcagggagcagttgatcattaacaatgaatagcagaggaaaaaacagcatatgggttttaaccttgttagagtttttttcattgaagaatgatttggaggtgaggtaataagtgtttcataacgtttgttttaaacatactgacggtatctggttgatataaaaagtggaattcttaaaatggaaattgttcttgtacaggtcctttttatggcatcatacggtgcatcataaaagtggtataggccaattttacaaatcataacgtctggaattcatgatgaagctatcgttctttcgtaagaatccatatcagctttgataacgattataacacaaatgttaaccagtgctaacaatctttaaatcaaccatttatgtaaaaagtatttaaaaaaatggtagtctgcagggtcagaaaaatactactattgataaataagtattaacaatagtagtatcagggaataaattttccggcgatatttgttattcttttcgatggcttaaccatattttgaaccaacaattaagtttcttatgaaatacactaccctgggaaataccggattgattgtttccagattatcctttggcgccatgacctttggcagcgatccatctatgcctactatatataaggtatcagatgaggaagcgcgtaaaatgattgacacatcgctggctgccggcataaacttctttgatactgccgacgggtatgccggtggccagtcggaagtaatgcttggcaaattgctggccagccgccggcatgaagtggtgattgccaccaaagtaggattccggaatggtgcgcctattacgcagtcggggctttcccgcaggcatatcctttactcctgcgatcagagcctgaagcgcctgggcaccgactacattgatctgtacattgttcaccgggaagacccggtaacaccactcgaagaaaccctggccacactggacgggttggtaaaaagcgggaaggtgcggtacatcgggttctccaactggtcggtatggaaatcggcgcttgcctggcagatgcagcgcgacaataattgggctaccttttgcaatgcccagatgaactacacccttgtgggccgtgatgtggaatacgatgtggtgccgtttatgcaacaggcaggaattggcatgacggtttggggaccactggccggcggattcctgagtggcaaatacacccgggaaaatctgaaagaagaagggaaccgcctttccggctttgatatcattccgttcgacaaagaaaaagggtttgtcctggtagaccggatgaaagaaattgcggcggcacataacgccacggtggcacaaatatcattggcctggctgctcaccaaaccggtagtgtccagcgtactgattggcgcatccaaagtgcagcagctggaagacaacctgaaagctgcgtccattgagctctctgttgcggaagtggaattactggacaatctcacggctccggggccgttatatccgcactggtttaaccataacctggcagatcctcagcatgtggcagcggggttgattaaatgattaagacgaagactttgagactcgtttaaggcgctgaggctggccattacttttggtcagcctcttcatttcttaaccgttcgttccatatctcttccattacttttcctattttcttaaactcttcttctgagaattcatctgttttggcattattgcaccagtaacagcaaagcaccaggttcccttcttcataaggttggaatggattgatcctgtccacctccagtgtttttcctcttgtgatgaaacgtttggtctttattttcttgtggcttctcagtagatcaatttcagcttccgtaatgttacagtagtggcatttcctctctatattattataaatctcactgaacttttctatggagagaaaacagttattttcaaaatgttgtcgtagggattgaagttccggcgggtgattgttataccagtttgtgtatagtttgtccagttccccgatggtaagagattggccttccggtactttctcaacagatattagctggtaacaggaagcatatagatcatataatccaggttctattataagttgtttaatatcgtttacttccggattcgctattgcatgttggaaaaaatagaacaaccggatttctatataattattaaaagcgcgcttgcggatactgttatatctcttgaggatagtgtcctgggatgtcatagtccaatagatatgagttcttatttactttcagccaccgttttgtatttcttctccaaaatattaactaccgcatttttcaaatcatcatacttaaagttatcattaaacccgataccatagtttaaatgcgttcctccctgagaaccacaaagaatatatttcggtcctcccatctctacagaaataggtgaatactccgtttgtatagtgaagtccacatttccaatggaatccagcacataaaaaatctgcttattaaaaatcccttgtttaggcccttcttcatatcgctcaaaagcctggatggatttgcctttccacttaaactgatcaaagcagaacatatcttccatattttctttcagcagtccttgtttgtgggcatcatataaactggccctataaaactttgccttttcataggttttattatgataatacacctggatcagttttgcataagcatgaaagtcggatgaatcggattttatcactgcaagaaaagccgtttccgctttatcatagttgccgcttaaagattcgatctggccgatgttaaaccacgacttcgtatatccctcgcttccatggggaagcttcgatgtattattataaagtgcttccagcgctttcgactcctggtgcagattaaagtatacctggggaaccattaaaaacggacgttcgccgggagctttcttttccgttgccgttttataattttcaagggccgattcatacaggtggaggttgtagtatgcatctcccaatccgctgtaatactctgcagtatctggtttcaatgcaatagccgccttgaagcatttaatcgactgatcaaactgctgcatgtaattcagtgtagatccttttataaaatatgcccggtgatcattcgcatttctatcaatagaaagatccataaatttcaggcagctgtcatcttgctgcttcataaaatacgcatatcctacgtagtataatgctgccgctgacaggtgctcctgtgccggggcatactgcgcgataattgcatcaaattgcttgtcggtggttaatttttgtaatgagggaagagtagtatcctgcgcgaaggaggatactaccaggagactaagcattattgttaagagtatcttgttcatagatagcgctaaatttgagcggatactaatataggcaaaagggttaaaacaatacttcctgcggaattctttgggtcaataaagtgcactctcaaaaaaaaattataaaaagaaaaagttttatttatttttacggcaggagcacatcaattacaacaaaactatacccgatggaaggtggccatgccggcccttctatacctttagaatttattgcgtgagcactgaagttatagtaacccgttccggtagtaaaaccaaagtctaacctaaattacagcagtactatggcgattttatcctgagttaaaagtcaaaatattttatctaaacagctaaatgctaagacggatgtcttaggaatgataacttattgtacaagtctaaatctaaacaacgcctttaggggcggcctatttgcttatatgagaactaaaatccaaaatctgaataagggctactgaggcggcgcttcagaagtacatattcgcttacgagataaaattcaagctgaatttttaaagagatgttttaaaggccggcgcctttaacgtcattcttgcgcgtagtaaatccagtttgaaacaaacctgcatatctcctgatatgtgcggcaggcagggctatgggtatactacagctgcaatcttttctatgtctgagttttctttctatatctaaatctaaattttcatgagaaaaagtttacttgtttttttcctgttgagcatgctgcaaactgttgcagtatttgcacaggaaaaaagaattaccggtaaagttaccaacaccgccgatggaagcggtattcccggcacttcggtagtaatccagggtacatccacgggaacccaaaccgatgcaaatggtaattacagtattaatgtgcctgccggcaaagtgttatcgttccgctccataggctttgcgataaaaaatgttacggtaggcgcctcagatattatcaacgtgacactcgccgtgcaacgtgatgatctgaacgaggtgattgtagtcgcttatggtaatgcaaagaaagaatcgctgacaggttctgtagctgcaattaaggcgaaagacatcgaaaaacgccctgtttccaatgcgctgagtgtgttggaaggtagtgcaggtattcaggttaataacactacaggaacgccgggtgcactgcccagtatccgcatccgcgggtttagttccgtaaacggtgataacactccgctgtatgttatcgatggcgtgcctttttccggcaatgtaacggatatcaatccggcagacatagaatctgtttctgtattgaaagacgctgcagccggcgccttatatggcaacaaggcatctaacggtgttattattatgaccacaaaaagggcttccaaagccagcgatggcaatgtaaacctggttatgaaccaaggcgtatacacccgtggtatcaaagaatacaaagtactgagcgctaacgagtttatggaaaccatgtggaagggttacagaaataacctgatgtctaccaaccctaccggctatccgacgaaagaagcggccggtgcaaaggccaccagcagcttgatttccgactacttatacctgaacatctacaacaaaccagacgaccagctatttgatgccaacggcaaactggttggtgatgccaggataaaatccggctacgccaatgacctgaactggtttgatggtgtggaaagaaccggcttccgccaggaatactcactcaatggtagtgcaagcaataaaaaaagtaatctctactattccgccggatatcttgatgaagacggatatgtgataaataccggttataaaagattcaccggcaggattaacgctgatatacaggcgaaagactggtttaaatacgggtttaatcttgctggttctcatcagaataccagtaatatttccgctacttcaacaagtgcatcttcttatgccaaccctttcatgtatgccaggggcatagcacccatctatcctgtacacttacacgacaaagctaccggtgaactggtgctggatgatgccggtaaggaacaatatgatgatggttctaccagccgcaatcaatttattggccgtcatactacctgggaaaatgaactgaataaagacctggtatatagaaatacagtaaatggccaggtgttcctggactttaaattacctaaagactttacgttcaccgtaaagggcgatctcaacgtccgcaacagcgatacccagacttacgataacgccatcatcggtgatggtgcaggtaaccagggccgcgcctcccgcaccaactaccgctataaaaattacactgcccagcaaatgctgaactggggtaaatcttatggctttcatacagtagatgcgttggtaggtcatgaaaactattacgacaactataactatctgtatggatataaaacgactgaaacgtttgccaatgcaaccgaattagtaaactttaccaacattactgatctcaccgactaccaggtaaactacagatccgagggatacttcgcacgtgcacgctataactacgatgaaaagtatttcctggatggttcattcagaagagatggttcttccaagttctataaagataaccgctggggtaatttctggtcattaggtggtagctggctcttgtctaaagaaaagttctttaccggcctttcccgctatgcggattatgcaaagctccgtgcttcttacggccaggtaggtaacgacgtaagcgccgccacctacgcatacatggcattgtataccattgatcagaataacaatcttgccgcgttatataaaacgcaaaacgaagcactggatctgcaatgggaaacctcttcttctatttctgccgctttggaaacacgtttgttcaacagggctaacttcactgttgagtattttgataaacgttcacaaaacttgttatttgatgtaagcttaccattatctgccggtggtacttctaatacggtagccgagtctgttattacaaaaaacctgggtacggtttccaataaagggtttgagctgtcgttagatgttgatgtaatcaggaagagagattttaaatggaatgttggcgtaaatgccactttcctgaaaaataaaattgtttccttaccggagcaaaaccgggccaatgggattatcaacgggaattataaatacatggaaggacatggcatttatgacttctggacataccagtacgcaggcgtggatcaaatgaccggcagcgctttgtacctggcggataatgaaaacttcgatccgaaagatgtaaatggcgcacactacaaatatcttgtaaatatcaacggcgttgactataccacctacaccacttacgcaaaacgtgattggtcaggcagtgccatcccggatgtttttggcagcttctccaccggccttacctacaaagatctcaccttgtcgggcatcttcacctattccctgggaggtaaagtttatgatgattcctacctggatctgatgactatgtcgggtactgtaggccagatgcataaggatgtactaaaatcatgggatggagttccttccggtatcacagaaacttcttccaaccgtattgaccctaaaggcgttcctgtaatggatttctccaaaagcaattatagcaacgctatgtcaaccaggtttctccagaatggttcttacttcgtagtgaagaatattgctttggcttaccaggtaccttcttctttactacagaaaatagacatcagatctgccagatttactttgagtgttgaaaacctggtgacgcttacaaaactgcaaggcatgaatccgcagcagtcgtttaacggaagaagcctaaacgcttttgtaacgccacgtgtaatatctcttggtgttaatattggtttataattaaaaagaagaaagatgaataagatatataatataggtttgttgttttttgtactgcttgcaggctcttgtaaaaaggattacctggataccgaacctaccagctcaaccggtacttctactgcatttgaatcaacggaaaatgcaaaattagccgttaacggcctggccaaaatgatgacggtgcagtacctgtcttcccagggattcaacggggaaggaaccattaaaatgtactatggcaactaccctggcaacaatttttatgtaaacctgccgggctgggccacgcttatcaatggtactatcaacgaaaatgtaagtagcatttatgactactatccgtggtactactattacaaagtaattggcaatgccaacgccatcattttttacattgatgccgcaaagggatcagaggctgataaaaatttcatcaaagcacaggcgttaacctacagggcttactgctataccatgctggcgcaattatatggtaacagatggagcgattccaataacggcgcaactccgggccttgtactgagaacggacctctccaatggcgacctcgaaaggtcttcgctgggagctacctatagccttatctacagtgacctggataaagcgatcgaattgttcacggccgctggtaaatccaggtcgaagaattttgaaatggatatcaatgtggcgtatgcagtttatgcccgtgcagcactcacacgccaggactatccgaaagcagaggcttttgctgctaaagcccgcaccggatatcctttgatgtctgtagctgactacaaagcaggcttctctactccaaacagcgaatggttatggagcagctatggcgcgtcagatgaaactttatactattactcttaccagtcatacatcgcatacaattccagcgcttctgcagtcagaacttatcctaagtgtatcagcaaagaattgtataataaaatccccgctacggatatccgcaaaaacctgttccttgatcccaaaacagatccttataccactgccacaggcgccgccggcgcagcattgaaagcccgtgcgttccagctgttcccggatatctacagcacgtcaaacatatacgcctatatgcagtttaaagtgaaagcgaatgaccagcccggcgttggcaatgtgaatcacttccgctcttccgaaatgtatctgattgaagcagaagctaaatattaccagaataagccggcagccgaagttcagcaggtactggttgacttaaccaaaaactcgggacgtgacgcaagctacacctgcaccaaaacaggtacagatctgctaaatgaaatcaaaacataccgcgctattgagctgtggggagaaggtttcgattggtttgatatgaaacgttggggagatcctattgtaagacgcgattacgccaacggtggtaactttataacttctttggctattaccatcactcctgaaagtaataataaatggacctggaaagttccgttgaaagaatcagattataatggtgctttagaatagtattcaatcaatcaaaaaaatgggctgcaggtaatttacccgcagcccatttttaattttataatggagaaattagtcggtctcctcacacatcttcaggtaacgccggtgattagccgggtcaatatcaaccttgctgaatagttcctttgccacttcaaatgcagtcagggaagatgacattttttctcccttaaaataataatccttcttatccctggcaaaggccttatataccgggtgtactttaaaagaggcatagtctgctactattgggtcgaggctgtatgtatagtggtaaacctttttcccatcagtgatatacttagatcctgcgtacactttcatacttccgggcttcactttatggatcgggaagatctgataatagagtgtatcgccattcaggagatatccacatagacaataagaaaggggccatgctttacagtatagccccttcccgtggtataccctctatcagagatcaaaccggatcccttgtgccagtggcagatgggtgccgtaattaatggtgttggtttgtcttctcatataaactttccatgcgtcgctgccgctttccctgccaccgccggtttctttttctccgccgaaggcgcctcctatttctgcgccggaagtaccgatgttcacatttgcaatcccgcaatcgctgccggaggcagacaggaagtattccgcctcccggaggttcatggtcataatagcggaagataacccctggggcacctcattctgtatagctactgcctcttctgtggttttgtatttcatgagatatagaatgggggcaaaagtttcggtttgtacgatagggtaaccaggcagtacttcggcaatacagggcttcacgtaacagccgctttcataacctggtccctccattacgccgccttccacaacaaaacggcctccctgctctttacaggctgcaatagcctctaggtaagcatttgcagcatccttatcgattaaaggtcccacatgatttaactcatccaggggattgccaatcctgagctggccgtaggcatgtaccaatagttccgtgaaacgggtgtatatctcttcatggatgatcagccgccgggtggtggtgcagcgctgcccggcagtacccacggcgccaaatacgctgccggtaagtgccatatccaggtcagcatctttagaaattatgatggcattattcccgccaagctccagcaggcaacgtccaaacctggccgctacggcaacacctacatttcttcccatgagcgttgaccccgtggctgatacaagcggtattcttacatccgtggacagcagcctgccggtttcttttccaccattgattaaacaacttactccttccggcacattattacgctttagtattgctgcaataattttctgacaggcaatggcagataccggtgttttctcgctgggcttccacacacatacattcccgcataccattgccagcattgtattccagctccataccgccaccgggaaattaaaagcagatataatacccgtaaccccaagcggatgccattgctcatacatccggtgcatcggacgttcgctgtgcatggtaaggccatataactggcggctcaatcctgtcgcaaactcgcatatgtcaatcatctcctgtacttctcccaaaccttcctgcaaacttttccccatttcaaaacttaccaggctgcccagtgcctgtttcttttggcgaagcgcctcccctatctgccgtactatttcgccgcgttgcggcgcaggtacggtacgccaatacgcaaaggcttttactgcagtattgatcaccgtgtcataatcagtttcatcagccgtcgtaacagtagcaatcagctgcccgtttacaggagaatatgacgcgagagctccgcccctgccgttcagccagttcataccggtgctaacgccggaattgtgcggcattatacctaactcctttagaaattccattattttttattggtttgagatgaatacgtgctttcgaatattttgttggcattggctgcttcaaagccctcccggcgatgttccctttttatggctgccgcatccaggtgccggaaagcaggcaacacgcggcgctccgcgaattctacataagaaccggagatcgcgtgcttttcaccatctgcaaatgctgctgttatcatacccgctacagtggagctttgcagcaaaaggccatccggactttccttgaacttgccgccggcatcattaagcacgaagccatgttgttcaagaaaccggttgaacgctgtaatgtcattatagccaagcttcaggttgtgtacactaatggtaaaatgattgagataataacggttgtaaatagtccatgaagcatattcactttctttcgctaatgttgaaaaatcgctgtaaacaggtagtcgccaaagaccgctgtggagaaaatcatctaccgcagcggcatcgttcagatccagttgcagtacaggatccgccgtaacttcatctgtataatggtgtataatatgttgagcttcgggagaaaggtcttttacccggagctcactgataaagatgcggggcaaagaaggcgctggcggggcataccagtaagcgtcgagtttcttttcagcgaaatagtaataatcccttttgacatatccatggtgcaggaatattttctccagtgattggatgcccaggtggggcacgccaattgtccggaatgcgatgtgatcattttcaatttcgtttgcatgttgtatcagtccttcttccatcatggctgatattactttttccacatccggcacccgttctttataacggcgcatcaggccgtccagtatcaattgcaggttactcatacctgttatattttaagttaaagattggataatacttcatcaagatgatgcaccatatcggcggcgttttctttactgaacaccagtggcggttttattttcaacacattgtataatggtccgtcggtgctgagcagaaaccctctttccttcatttcttccactaccttgttgatctcatccacagcgggttccatagaattcctgtttttcaccatctctgcccccacaaataaaccgtgtcctcttacatcgctgataatggtgtgtttattcattaaaccacgcaagcctttcatgaggtaattgcctgtttccagcgcgtgctgctgcaaatcttcagattgtattacgtccagtactgccctgccggtaaccattgaaacggggttcccaccaaacgtattaaaatactccataccgttgttaaatgcggcggctatttctttggtaaccaccacggcagccagtggatgaccgttgccgataggttttcccaacactacaatatcaggttccacctgctgcagctcaaatccccagaacttctctcctacccgtccgaagcctacctgcacttcatctgcaatgcatacgccacctgcttcacgcacatgccggtatactgcttccaggtaatgatccggtaaagggatttgcccacctacacccaacagtgtttcacagataaaggccgctaccttgcccgggttctccgcaagaatagtttgtacatcctgcgcatatttaacgcctgcttccggatcgttgtaccggtatgctccacggtataaatcgggagagatggctttgtggatataaggcatttgcccggagccgcctttgccatcaaacttgtaagggctcatttccattgcaacagtagacgtgccatgataagcatgatccagcaccaccacatcgttccggcgggtaaaatgacggctcatgcgaatagccagatcgtttgcttcacttcctgaattggtgaagtaacatacggagagctttgaaggcaatgtgcgatggatcgctttggcaaactccaccaggtggtcgctcaggtaacgggtattcgtattcagcgtggcaatctgtttctgcatcgctttcactactaccgggtggcaatgcccaacatggcttacattatttacgcaatcaataaacgtatttcctttgtcgtcgtagaggtattgcaatgcaccttttacaatttttaatggcttgcggtagctgatactcaggttggcgccgatgaatgttttcctttcctgcagcaacggactgtaatcctcgccggcattgatgagcaaggacatgccacaggctttccggaaagtatcggcggctttcagcgggtttatccggatcagttgattcagcagcgaccaggcgtcccgttctgttacaaagtgatggccgttgacagagccgagcgaggcctgccaggccgactgtgttacactgatacaaagcctcgcagccaccaggtaataaataagatctgtttcctgttctgttaacgggaaggcgccgtgatatccctgtatcacccaggaagctgcctgtaaaggatcttccgtgttcagcatcgcataggtacatgcaatagccacattattcaccagtgcggaatacaccatatcgccaaggtctatcaaaccgcttacttcaccgttttgaaccaatacgttataatcgttggcatcgttgtggatgctcgcatgacgaagggagtcgagcaccggcaatacttctgtctcaaaggcaagcaaaaaatatccggccagccttcttttttcatgatcgcggatgcagtgcagcaggcggttagcgcttgcggcagtgctgatatcccaggtgtaatgccggtgcagggcgtcgtgttgaaaatcctgcatcgcttcatctgttttgccgaggaaactgccgagaccaagatagagctccttgtttttgtgcggtacctgcgcccagcatactccttccagccaggagaggatacgcaggtaatattgtttaccatccttgaagatgggcgtaagttcctgccggtttttgttgcggagtatctgctgaaagttccacgccacggcgctcactgaaagatgttccagtatgcggagttgcgcatccaggaaggagtagcgcttttcttcccccgttattttgaggatgaatttacggccggagacatccgttattttataattaaattcatcgtagccctggagtgtttccacttctactgcaagcaggtaattcttttgtaccagttgctttacttcatttgctgtaaattccatgacgatatttatttttcagtatcattaacaagtgtgcggccgaccagctgaaattctttgcattcagccctttaccggtaagcgggtgatagttttcatataccggttcgttggctgtcatgcctgctgcattttccaatagttgcttttcgaatgctgctgccaggctatcatagccgtatttccgtaaaccgcttgtaccaaaggcaaactggtccagccataccggcccgcgccagtatcctttcatcggatcaaaggcaacatgatcggcagccagggtaggcagcggtactttcgtattgaattttgccgggtcttccattttttcctttactcttttagcctgctgcgaggtggctacgccagcccataacgggatccacccttccgggccatccacctgcacacggccattcgccctggtgtcgtagaagtaaccggcatgctcatcgtagaactgtgtgcgtatcagccggagcagcttctccgcttgctgccggtaagtatgttgtttgttatccaggagagatgagagttttgccaggtacaatttctccgcatagaggtaagtattgagatccacactttcctggttcagcgaccaggcgctgttgttgttttgcagcatcaccgcgctgtcgaagcgtacggcattatccattccgctttcccatgctgcggctatgcgggtaccatcggtagcgccgtattcgcagaggccattccggtcgtgatcgcggttagcataccaccattcatgataggcaataagtttaggcagcatttctttgacgaatgatttgtcttttgtatgcagatagatttcccacactgcccaggcggcaagaggaggtttggtatcccgccagttgttttcacgtttatctgcatagatacagtctgccaccatgccgtgatcatcctggtaatcgaacatggaacggacgttgtctttcgccagctgggggaaaaaggtggcgaggcccgcggcctgcttccagctgtcccagctccacacgccataaaagccctggtagtttacagagggaaatacgccgtcgtgcaggatgtctttagcgctgcttcgccagttggtaataagcgtgatgatacatttgactgccagccgtttttttatctctgttaaatgagatgccagggagaaataccgggagagataaccattccatctcgcttcattttttttgagcgctgttttgaagttgtattgaaaaggttgccgcgtttcaccgggataatacgcctgcacctgtgtttgttcataacttccgccgggttgtatcactacattcttccaaagcgctttataagtaaagctgtccgcctgcaatgcagtgtccttggggaatacggttacaaaaccatttacccgcagggtggaggcctccgcagtcatcctcttttttgtttgcccatagtattccacatccagcatacggggatagcgggagctgttggtaatttttgtgtacaacaacgcttcgcggctggaagcaaagaggagctgctggcatatcaccaggccggcgatttcaaattgctgctgtaacagcccgggataaaacttaatgttggctttcgctgccggcaggttaagcggtacaccgttttcacggacagctaatcttgagaaagagccggaaagccattctccctgcatatccatcaacaaaggacccataaaggcgccgttgttttctttccccgagggcagtgcataggcatgccatgcacccatatcgctgaatacattggcctcgatactttcaccggcgggaggcgccgtccgcaaatccaatacatcaggataacggtagcgctgcgcagtagctgcctgcacggtgagcaatagtaatatccatattctcatctgcttcattttatagcgggacgtagcgtaaaagagtaactgtaatcctggtaaggcagcaaatattctgcgtgtggggtggcgccccagctgttgtcgccgcctacgcccatttgtttataatcgatattccaccataccaggtcttcgttcgtcatagagccaccgtggttgttctccgctgcgtagcggtcaaattcaagatggtccatattgaaatgcaatacgcctgtgctgatatgcggctgaccctgtgcggtcaatcccacgccgtttttgttggtcagggttatccagcgcacatccgttctgtagccgctttcctgtgcacgcggataaggatggaaaagctgatcggcgttcatgctgtatatatcaacagctgcagcagtttgccggtcggcataattatcaaaagggccgcggcccagccacttcacctgatcgaatgctccatgcaggatcatgcgcataccgaatcgcggaagctccggcatgggatctctcccggatttcattgctacgctgatgtttattactccatctcccgttactatatacgctgctttatacactgcttttaccgcaggcagatagtgccaggtgcggatgattacctgtcgtttatttgtggtgtctattttcagggaatcaagccgggctgtttgcaatacatctttccatacggcgcagcggatctgctgactgttaccgatgtcattatccgtggcagcgcgccagaaatgcggctcgaggggcgacttcatcattgcctgctgctgccagttataagcgctcagccagccagtttcccggctgaatgccacttcaaaatcaaccccggcaatttttatttgcgatggttcttctttaaccgatattgctttagtgcttgcaggagcgggcatttcagccagtgccacaggcaacgggaactgctcccatgccgcgaggtagtgtgcaggcaccagtggcgcatcgtgccacgtcctcatttctatcgtaacaaaatattccgtaccgggcttcgctttcagcaccggcaaaggcagtgtaatgatcttttctttatggggcgccacggaaccggcattcagttcacctttggcgatcgtttccccgtttgacctgataacccagttgaaataaaactgatccaggtctgtaaaatcgaggcggttaataatgcggatactgtttgccgacaacggcacaggctcaaagcctgccggctgtattacttttttaaattcaaacgcctgtggatgcggcgtgcgatcggctgcaaacaacccgtcagcacaataactcgtatcactggtaagacctacattacccatatcccggccataggcccagatatcccttcctgctttatctttctttttaaaagtctgatcagaaaaatcccagataaaaccgccctgcaattgcgggtaacgatacatcaggtcccagtactctttcaggttaccaccgccgttgcccatcatgtgcgcatattcgcaaagaataaacggacggctgcgccactctctcacatatcccagcagcacactggtggatttatacatcgggcacacgatgtctgtaaattcattatctcctgccgcttcatattgaaccgggcgggtattgtcttttgatttaagataccggtaggtagcttcaaagttttcaccaaagccgctttcatttcccaacgaccatgtaataatggagcaatgattcttgttggtttcaaacattctccgggtgcggtgcagataggcttctttccattgcggtttatcggataatgttttcagcggatgaaacgacatgccatcgcattcaatattggcttcgtctaccacgtaaataccgtattcgtcgcaaagccggtaccattccgggctgttgggataatgactggcacgtaccgcattgatgttatactgcttcatcagccgtatatcttccatcatattttcctgcgtaatcaccttcccggtgtacatgttgtgttcgtgccggtttacgcctttgatctttaccgccacgccgtttatcagcaatagcccgttccgtatctctatcgtccggaagcctgtttcatgcgcaatacattccaccagcttgccatttttatcgaattgggaaatgagtagtttataaagatggggatgctctgcattccagctttttacattacgcagcgtagcatcaaagtgataatctgcagtaccgttcaatatttgctgttgttgtataacgatgcttcccttgtcatccagcagttttatttgcaaacgcccgtgctgtgctgtagaatttagttgtacgtccaggctaaagataccgttggtgtaagtgctgtccagtcctgcttttacaaagaaatcgcgtacagctattttaggttgtgcaatcagctgcacgcttcgttctattccgcttagcttccacatatcctgcccttccaggtaggtggcgtcgctaaaacggaatacctgtacggaaatggtgttctctcctttccgtaaataatgggtgatatcaaattcggcggcagttttactgtctttgctaaagcctaagtaccggccattgatccagcaataaaaaaaggaatttacggcgccgaagcggaggattatattcctgccggcccattccgcgggaatggtaaagctcctccggtaggagccggtgggattgtcgttctccggtggatacggcggatttacgggaataggatattccacatccgtgaaaataaatttatcgaaaccttccgtttgccagtgcgcgggcactttaatattcttccagttgctcacgtcataatggtccgcaaaaaagctatcggggcttgctgcgggtgatgcatcgagcctgaatttccaggtgccatccagcgaaagcaggaatggggacggggaacccgacatggcagcggcctccgagatggcgggtataaaccatgcccgcggcgccagggcgttttctgtttgtatctccgggtgctgccagggctgtggatgctgttgggaactggcagtaaaaatattgagccataacaaccaaacaatcatcaatccggtgctgtatttcattaagttccttgcttatcttgaaaaaaaattaccggccggcatacaatggcacaccggcccggttgtttagtacaaattgttttgcttcaggagcgggtttacgttgatctctttcagcggtatagggtagcggatgtgtttatcttctacatagttggctgcagcagctttaccatggtttgtcagcagggcttttatcggttgtttggcggtagcgccacggccccagcgtaccaggtcgaaccagcggataccaaattccattgccagttctaccggtctttcgtgatttcggatctgctcccgcagctgttctttattcagactgcctgctgcaattggtttcgcgtgactgcggttacgcacttcattcacgaggtcaatagctgctgccgttcccccattttcattcgttgcctctgccagcatcagcagcacatctgcataacggatcagggagatgttcgttcctacataagaaccgcccctgtcgttagggtatgcatatttattgaagaaggcggggtgggaaagattgcctgccacatctgcgtagggcacgaggttggcgggaatgttgagatcccacatttttgacgctggatcgttgaaaaagatagtaccatataccctgtcgctataaccacctgttgcggttttatctttcatcagtgtagtcaccagccagtcagaaggataaaagagttcccagccatcaagcgcataaggcctcacttcaaaattgaaaggatgtctttcatcagacacggaacgatcgccactgaattgcacttcaaagatggattcagggccattttcctttgtgccgttgaagttgtcgatataatttgtattgagggtgtactgcccgtaaatctctctgaattttgcttctgccgctgtccatttttcctggaagagatatgtttttgccaacagcgctttagcggcgccttttgttgcacgacctttatatgcatccggataagcggttggcagcacggcttctgcttctgtcagatctttttcaatttgtgcccaaacgtctgcagcgggggactgcggcgcttgaagcctggtaagatctttttcaaatttcaataccagcggcacattttcaaaaccatttaccagtatgaaataattataggcgcggaggaatttagcttctgcaacaatttcatttctttctttctccgtcatagcggtaatgcctggtactttttcgatcacctggttagcacggccaattcctgcataacaggtagcccagagattccagggaccgccttcatctgcactgtttacaaatgcagccagattttttccataaggctcatttttattattatctatatcatcagccttataggagagcgtgatatatatttcctcaaagaaagtccacatggagccgtcgtgtccctgtaaagccgcatagctggcggtaattccctgcaaagcatgctgccgggtggtccagaaagtattttctgtgaggttttgtttatcgtccagttccaggtatttatcggagcacgcagtgaagagcgcaacggaaaagaagaagagaacggctattggtagtttcatgattgtcagtttaaaatttcagattagaatccaacgttaaggccgaatacaaaagagcggctcagcgggtagtagccacggtctaccccacggccaaagatgccggtgttggagaggtccggatcaaagcctgtatactttgtaaaggtgagcaggttgtaggcgccggcataaacccgtaagcggtcgatgtgtacttttgccgtgagttgctgcggaagtgtgtaacccagctgtaggtttcgcaggcgtacaaaagaagcgtcttccaggaagtagtcggacacacggaggttttcgttttcatctgtattggaaagacgatataccgaagcatcaggattggaggggctccaggcgttcagcaggtctgcagagcgatagaagcggtacaggaacatctttgcgccgttgtacatcttctggccctgtttgccgttgaagaacaccatcaggtcgaagtttttgtaactggcgttgaaagtaataccgaagtcgaggttaggaagaccgttacccatcagctgtttatcattatcgtctaatgcgccgtcggcatttgtatccacgaaacgaaggtcgccgggtttggcattgggttgcagcggatcgccggatttattgacgtgtgcatccacatccgcctgcgatctgaagatgccgtctgttttataaagataaaatgatgccagcgcctctcctttcttggtgagcgtggtaccgcggttgttaaaatcaacatatccgtcggcaatcactccttcgtcataccccaaccggatgatcttattccggctgtgtgaaatatttgcagttatatcccagtaaaatgcattggacgcagggcggcggtaggtagccgttacttcccatcctttattttccatatccgcgatattggtgagcggcaatgctgtgataccggatgatgcagggataggcgtttcggccagcatatcagatgttctggaactaaagtaatcgaaactgccgctcacagcaccttttaagaaactaaaattcaaccctgcattgagggtagctgtttgttcccatttgatgttgttattagccaatgtagctgcaatggcgccgacatatacctgctgactgagcgcggaacccaaaggatagttcaggtagggactggagcctgtcaggaatatcttggcgaggtactgaaagttgctcacgttctgattccccacggtaccatagctgatacgcggctttagttctgatatccacgggatattgaaaaaggattccttatgcatgttccagcctgcagagaaagagtagaaagtaccgtaacggttcagagggccgaatttagaagagccgtcacggcggaggcttccctggagaaaatatttatcgtcataattatagcttgcgcggccaaagtaggattgcagcgtgctggaaaaattccagccgccggcgcggataaaatctcctttaccgtcgatgatcaggcccgacagtgattcgatcagcggactgctcaaatgattgcctgcgccggtggtaccctggctcacagacttttcacgggagaagccgtacatgcctttaatattgtgcttgcccagttgtttttcgtaattcaggagatgggtaaacacggtgaactcattccggccacggctctcggagcggctcggattttccaccagcgcctgtgcgccaaagtcgtaaggatctgtttgcgtaaactcgtaggtgtttacaatattacggcccagggtaaagttgtaagagaaccctttccagagttgcaggtctgcagccatattgaactgcaggtgatcatctattgttttgccgttgctcagcattctttcacctaccgggttgccggagcccagctctgtttcgggtttggcataaccgttcaccgaagcagggtcgtagatgcgtttatgtgggagcgtgttataaacgttcataatgggagaaaatcctgcatttccatcaccgttcacatctccaaaattcttattgtcaaaacgggtataagcgataatgggacttaatttgaggcgattgttgagtagtttgatctctgtattcagccggatgttatctcttttagagccggaattaatgatggacccggaatgtccccagtgtcctaacgacaggcggtaagcaattttctctgaagcgcctgccacatcaacatcatatttctgttccacgccttgtttggtgaaagcgctgagccagtcggagttagcgtatttattatcatcctgcacataaatgggaggtgtttcgccgtcattggcataggcttctctcaccaccttattcatgggaactttctccagcaggtcaatattattattcagcttgtgcagggatgcgtatgaattgaaggtgatacgcggttcacccgttttcccttttttggtggtgatgatgataacacccccggccgcccgggcgccataaatggtagcggcagaagcatctttaaggatgcttactgattcgatatcattggggttgatatcatatgcatatcccaggggaataccatccactacataaagggggttgtcgttgttgatactgttgaggccccgcaccagcactacgggattggccgcaggattgcctgtaccggcacttacgatcacgccggccgcttgtccctgcagcatggtaccgatgttaccggagggttgtttggcgagattttttgtatttacggaagatatggccgctgtcacatctccttttttctgagttccatagccgatcaccagtacttcatccagtcctttcacactttcttccagggctactaccagttctttggcgctggtcagtttaatttctttggcggtaaatcccatcgccgaaataaccagggtagcattttcaggtacggttagtgtaaagacgcccttgtctgaggtggccgttccgttagccgtgttttttaccacgacgctggcgcccggaatagggttgcctgcggcgtctttaattctccccttcagggtccagttaacggatgctgtttgagcgattgccgttaacccggtaaataaaaggaataataatattccgttcctccgtaatagtttccacatacgcattttggtttttagatcttttttttaaaaagtataacatggatcgtccggatgctgcagcataggtacctgctttcaaacgtgaaatcggcagcaacggatcagggaagtaatgtaggcaggaaagatgggcacaggagagttgtaagcctctatatgagccttacaggcacctctacatgacctctacaagagagacaggtagttgataattaattggttagaaattcttcagaaaatcagacaggttgtctttgtgttccaggttgaatgctttacggaggcggtagcgagccatttcaactgattttacagagatattattcaatgaagcgatgtctttgatagagagatttaaccggatttgtgcacaaaggcggcgttcattttctgtaaggcccggatatttttgaaggagattaaagaagaagtctttatggatttcatttaccgagagattaaaatcctgggcatctttattatgatcgaggtcatgctggaatttatggaccaggcggttgaaacgggtgatattctcatttctggcgtcgttatggatatcaaggctggtcagttcatcaataaaattccggatcatttcattacgctgggaaatgtatagcgcatagtttttgaggtcgttatcgcggaattccagtttaccattcagggcttccttttccatcagggcgccatcaagctcctgtttgatcagggcacgtttaacctcttccagttctttctcctttttctgcttttgtttcatcttgctgtaaaacagcaaccagataataataaggagtaccacccctgctgccagcgcattccgttgaaacgcccgaagttccttctgcgccaccagtgtgatgatgcgggtttcgttctcttttgcctcccgttgcagcttaagcgccgaaatagcttcactcttgcttttggaaaggatctggtttcggaccctggtatattcctgcagttcggtgaaagccttccggtattctcccagctcctggtataacaatactgaattggtaaggttatccagcagcttctccttctttgtattggagttcgattggttgatcagtacccttgcatcccggaggagggtttccgcctgcggatattccttcagcataatgcgggagtaagccatctggttcagcacctccgcatgcgacaatacttctgcagggttaatgattgccattgcctggttaaaatcagcgatggccacctggtacttcccttgttcattccagcaaataccgcggttactcaacgctgtggcaatcatcccttccagatgattttgctttgcgatggcgagcgtgctatcaaaatacaggcgggccgtttcaaaatcatctttcatcaggtaaaccagtcccagtgcattcatagacaccgccagccggtggggatcgccgctttttttatataatgtgtgcgcctgctggtggtactgaagagagaagtgagcgttctccgtatcataaaagacccagcccaggtttgtaaagcaccgggcaatagcgctatcatttccccactccaggcagagatccagtgcattataggcgtaattgagcgcctggtcgtattgatcgttatagagatatccctcggaaaggttgaggagagaggccgcctggagcggcttgttcttttctttcagggaaagcaggtaagcctcattggccagtaccagtgccacattggtggaatcctggttgtaatgggccgccagcatattgagcgccgtaatcctttccggcgtggtcatgtttttatttgccagcagttgattcaggctatccgcattgagctgggcattggcagtaatgcacgtacagtagcaggctgcaagaaggagtagcaatttcatcattcagtcatcattttggcgtgttcgggcgccgatccgtggatttgtggattgtaaaatacggattataggtatgcgaaaagcgggaaggcaatacaatttataattaaccatccgtctaaaacaggaaacagtaatatccggggagaatgcagggcatgtagaaattacattgcggaataagtatcattggaaatcatgttcagcccggacagaaaagacagcagacacaacacaatcatcataatttaaattacagtgctattagccaggcggcaatgcaataaagcaaagccgcctgtacttagtaaaaattggacgtggaaaatattatagttccacttttcgggtaaaataatctaacagaatagccggtatggcctttcaaaatttactcaagcgttgcctgcacgatcttttcaatatcaaattttcgcatttgcataaacgcctgggctgctttaccggccttattgggatcggtcatcaatttccccagaatagtaggtattacctgccaggaaacaccaaatttatcttttaaccatccacacctgctttcttcgccgctttcggttaattttccccaatagtgatctatttcttcctgtgtgttgcaatgaatcgttaaggaaacgccctcgttaaaggcaaatttgtgagcatgtgcactttccattagcataaacttctgcccggctaaggttatcacggcatgctttacttttccctctatatcgggctgttcctgttgagagtaacggagtatcccatctgttgctgaatcctggaatatggaactataatgctgtatggcctcttccacacgaccatactgatccccgacgaacattaaaaagggcgtaatcttttgacccaccgcggctactgttcccagggtaacctgccatgaaatgccaaaccggtcgctcacccagccgtatttttcactccagggatacttatccaatggcatcattataaaaccgtcgctggataatccttcccagatatcctttagttcttcttctgtttcacagatgtaatacattgaaatggatggattgggtctgaacataggccccccatctaacagcgtaatatgctgtccggctatctctatttcggtgacaacaggcgactgcattactattttggcgccgggaattaatttgcaatacaaagcggcggcttcttttgcctggttatcgaaccataagcaaggcgtgattagttctttcatacatttaaattttgtgtaaagatgaaccagccaccaaacatctccttgtacaaaaccgacattattttttctttagcccaaactgcaggtattcattgggagtggttgctgtaaattccttaaaagaacggatataatggctctgatcaaaataaccattggcatatgccacgtcggtcaatttatgaaactggccggactttaactggtaaaaagccatctggaactggcagatccgcctgtattcgctggccgttatacctacatattttttaaagatccgttgaaatgttctttcggtgagactaagctcctgcagcatttgtgccaatacatcggcttccgggttttccaatattttatcggtcgcataccggatgatcctgcattcccgctggttggctgtaacctgggaaagaataaactggtgtagcacctccactttctcggctgttgatggagcataggctagttgaatggtcaatgccattgccttttgtggattccaacgattcagcccgatggcttcattttttaactgctgtgcagatagcttaaaaacaggccctatggcaaatggtttgaagaaaaatgcgatcagggtagcattcccccattcggcccatctttctgaaggaacggtctttccgaacagcgacaggcgactttcctgatgctgtgttgtacacaataaagccggcatgccgttggtaaatatgggcaagtcatccggctcagggggatcggcactatcaaggattaagacggcttggacagtgtcttttagggctgggtctagtttattataccattgttgcatatgaatttacactaggcttaatcaaaaaaaggtatttattccccggaagaaacactctctaattaaaaatatgaaaaatgtagcgaatctgttgaaacgtcacatataaaagcaataaagccgcacaatggcggccttattgctgtcttcacgttgctattaaaccactggcggtgtcaacttcacctgccagaagattttgttttacgcgcatttgatttttgcgacgtcgtcttttctatgtgcttaaagagtaatcagtcttattccaatgtgttcttccatttggcagtacggcccgtaaaccatacagggagatccggattattagaaggactaataattgaccaaccttccggatcggaagcctgaacgctaccaggataagtcattctttctttccacttgtatctttcatacattgaagcaggatttgtacccaggtatttaattaacctgcgggcagcggtatacggcacttcaaagttcaacatattataatgcaactgaagctgattaaaaattgcctgaactttttgagtgcttgacatcgcatcaaatttctgtgctgctacctctgcataaacacttgcgttatattccattgcgggcctggcgctgattctcgaatcgtccatcgttgttggcatagccggcaaggttgtcttagaatattgatttgagttattcagttcataccaatatttgcaggataagataatggcattcttatagtgatcgcgcgcggcaccattcagttgaccaaaacctcttactgctgcctctgccaatgaaagctccgtttcaaccgcatgaatggttggatattttaacgcaaagttaaattgtgggcgtacattgtactccgcaaccaggttgtttgcagtgcctacgttccaaccattgtcatcgtagttggccactctgctgcgaagcgtatttaacaggaacgcctcacgtttactcagatctgctttagatgctgcgtccaacgcgatcgactggctattatttacgccgtaataaaaggttgtttttgaaatatcggtcaggataggatcgttgatgtaaaggccacgcaaaattttatttaagtaactattcttatcagtattgccatcccattttgtatcaacacccaggtatctgccactccagtctggagcgaagatataagaaacgcgcgggtcaacagtaccatccaataaacctgttgcagaattatcaccactgaaataatataacgcttgtccgttcaccaccttactgctcatggtcggctggcagtacatcacgtcctgcaggaattttttccctgcacggcaatcatccgctctttccctgaaagcacgtgtaatacccagttcgttacaaatacgattaagtgcaatcactgctatgtcagctacaccagctacatcgttatagtcggtcagtaggggtttgccttgcaactccgtaagcacctgcttcgtaatagcaggcaaaacttcgcttacattcatcgcacaacgcaaccttaatgaattaatatacttacgccatttcaaaatatttccgccaaaaatgatatcctgctggttaaatgatgcctgctcggtagacgtaagtgtcagcgtcgtcaacacttcttcggcggccttaaaatcactgattatcttcggatagatgtccgattggccaaggtattttgctttaacgccatcaagcccacccgcagaacctgtttctatgtagggaatcttatcgtacatgtcggttgctctttggtaggcataaccttttaaaacatgcattaaggtgatatacaggctatctaaattggtccgtttagcttgcggtgtgttgttgtattcacgttgagcccagagtattggtgtgatccattgtgtattaacaaagttgaaaacagattcgttaaaaccacccgtaccccagtcgtgctcaacatctgcgagcgtgtaggaacttccttcggtagttgtattataaatctgaacggcatttgccataatcctgtttccacttctcacctggtggtaaacagaaccgtaatcaccactaagaaagaatccctgggttagctgagaagtgaagaatccggcaataacgcttactcccgacttatcagccatgtctttcgaatatccgtcaggattttgatatgagtcttccaggctcttcttgcacgcgacagaagataataacaacgtaagcaagaaaaaagatcttaattgtatatatttcatcttagttgtttttaaaatttagttttgatagaaatacctattgaacgttgtgagggtaatgcagttgttccataggaacccacgccccagcctgttccgttagttgattcaggtactgaatttggtgcatctttgtagaggtaacccacattgttcgcaaaaactgatattatcagactgctcatatggatcttttgaggaatctttggattcaaagtataatcgatggccacattacgcagggctacgtaatcgcttttaaagatcctgtcttcagggaaaaagccatttgaaaaataagaatcgtaataataattatcagcagaaaccacttttgtgttcgttttgccatcagtactaacaccatccaatattacaccgtcgtgaaaggtggatccgccattagggtttgtgcctgcaactttcttagaattggcatctaaataataagcagatcctccatgcgcctcatctctatatttcaatgtttcgtttagcgcaccggctgccatcatataagtttcagagcctgacaggaaagtggcgccaaactggtagtctatatttgcaataaggcgaatatttttgtatgcaaaagaagtgaaaaaccctcctgttacatcaggaattgttttgccgattaactttgctgtgctcgtataatcataagccgagccagcagcatttacaactctttttccattgtttggatcacttggatcatttggattattgtaggtgtaggttgacttagtcaggtaaagctgaccatattcctgacccacattagccactgcattcactgcgccgaacgcgttccacagggtgagagattgtagtttgccatccagtttttccacataagttttgccatgtgcaaacattaagtttacatcccactcaaaatcttttgttaaaattggttttgttttaatagccagttcccatcctttgttcatcacgttaccagcattcatacgaacatttttaacacccattcccggaggagctgctaccgccatgatctggtcgtagatatttgatttgtaataagagaagtccactccaattctcctgttatggaacagataggtttcaaaacctacttcaaattcacgtttacgctcaggttttagatttggattgccgttggcatccattggaggaagatcggatggaggagtaagcacatatccaccacctgtttgagatgtagcatagttcacgttgctgaaatagcgtggacccggacggcccacatcggcccatgacgcccttactttggcataatcaaacaccgccggtaatttcaggctttcgctaaagatccatgctgcacttataccaggatagaaataactattctgatttggaggcaagatagatgaccagtcttgtctggcctgggcttctatataaacctggtttctccatgccaactgtgcagatcccaataaactgtataacatatcctcaccatttgtaaactggtattgaggctgcactcctaatggtaaattattaaaagaaaagtaattaggaataaccagctgtccataaccattcacagatgcaccttttccttctgtgtaattttttctgattactccacctacaaaaccagacaaatcaaaatcactatttattttggtgttgaagttaagcatgccctggccataggtatttttgtatatgttggttacatcactatacatgaaaccactattagggcctaataactgtggatccaacaatttccctttatactcattcctctccgtgctataatctatgccccccattaatgtggcactaaatatattggtgagttttatatcggcagataaagactggatattgtgcaatcttgtaaaaatagatttattctggagctgatcccaaagatagcctaccactcccttcctaccgttggagattaaatttctctggcttgggttggcaaagtaattatatccatctggcgttagtaaatgtgactttaacaagcctacgttgatatcagcgctatatgcccctatctctgcctgctgaccttctccattcattgtactcaggttggcagcattcaggtttctggaaataaaaaagttgccggtatatttaagggtaatgttattatttaacttataggacgagttaaggctaaaagtatttttgtcataatcagaacctggtctgatgggggtcatacttaagttagtgtatgaaaaacgaatctgtccctgatcattcccgccacttaaagccacattagttgtgttctgatgccccgtttggtaaagatcgttatagatatttttggattgagcctgccatggtctttctactccgtcccaccacaaaagtttcacgcttgggtcgaattttggtccaaatgcagctgcgccaaaaccatctcccaatgtagttgccaacgctctttttccatttgcatcaatatagtatccctcagcgtcattcctggagttgctagggctggagccagttccatattcattttgcaacttaggaaggaacgctgcgcggtcccatgaagttgtgaaagaagccgccactcccagtcctttccctttggtgccgcttttggtagtaatcagcacaacaccattggcaccttcactaccgtatagtactgatgctttagctcctttcaaaatttccatggaagcaatgtcatcagggttgatatcgttaatacctgttccgttgtcgcgatcagtagcaccgaaacccatttgcgtattctgatcgtgaatgggaacaccatctactacaataagtggacgcgttgatgaattttggtcaaaagataccgcattacgaatgttgattttcattccagcggaggggccggctgctgtagctgcaacctgcacgccaggcgcggcaccgtagagtgcttgtaaagcattggtaggtgtaccgctggccataatcctgtcattatcaattttggatacggcataacctaacgctttagattgttttttgatacccaaggcagtaacaactacttcttcagtactctgaacactggctactagcgttatctgcatagaagatgtagcctgcaattcctgggttacaaagccaacataagaaataaccagttttgcatctggttttacattgatagtaaagctaccacccttgctggtcggcacccaattggatgtacctttttcgctcacggtagctccttcaagaacattgccggttgcgtccttgatggtacctgaaaccgtcatttttccctgcccataggcaaacatgcttcctatgcaaaagagcataaaaagcaaaagagatcttttggttgactgcatcgttttttagtttttataattgaatagaactgattttggtatagtattacgaatggaaatcttctatgttgttggctgtttgtatcttccacatcaatcagtgccagactgctaatttctatatcgaacagaccaccctgctgataacactgatggtagatagagttggcggagatagtattttttgatgcattaaggttaaacccgttttcccgggaaggtcaccattggttggttataagacagtaattagtcgccatatacaatgtatgtaacattgtatatggtactatatgtaccattctcgccatgacaaagggtgctcagctttgtttaaaattttagcactataacccgtagggccgttacccattcttccacgcagtttcaatccttgctgctgacaatggctggatttatataggtgtcattgttcagtattcattcttttggttcatacttttctgcgaaagcagtagctattgtgctctttcatagcacaaaaaacaatgcttagtcatcctgatttattaaggcaatatgatcctgtttgaaagacatcactattgttcaccaacgctgtttgatgatagaaacattttaacgcatatgcttacgaataacaaattgattgataaaaaagtctggttatttagtggaactctcgtcgactgttaaaagaaatctaatctttccaattgttgctgatgttgattgaatttacagtttaaggaaatacattgttgtagggacaaaatatgctaatcggtcattagttaaacgttttagctaccaataatgaatctttgttttctttgctctaatgctcttttttcgtctttctcaaacctatgtaaactttttcaagtcgcgcaattttttaacaacttttttaggaaaaggtcaagatagaattgttttttatcaaaatagaatcattagtgtagttagcttatccacttaaataaggaaagttggataatgaacaagacccggaaagattccaagctggcttgtctggaaaaaataaccaaaattgatcctagtgttaatgaaattatcacttgtcgttggggaaaagcgcttgacggaactcagcagtggatgaatgggaatgggaatgataaataaaatttgataacgattatctccagtagttgcattttatgcaactactgactaaattgcctttacctcttcaaagcccaagctcaattgttcaattaactgataacattcttccaaagaagtatcaaaatattccagcataatcaacgccattctcccagaaccctcttcagcatttacttttaggatattataaacgcggtcatttagatgctgactcctatctgtaatcttacgaatttcccggcccataaccctcgccgcaataaaaagtaattcaacactctcctcctcaaagaggtcatggtgatgctcccatatagcatcccgatgcatatcgaagaaattattcagaatatcgctaatgtctttgatgtcgtcccggcgcgcctccggcctatcatcccaggctatcaattttaataatacaatgcctggcaaagtacagactttaaaatgatgtccctcacctatttctatttccggcagatcctggtcgtatacttccttaaacccttctacgtgtatgttggtatatccattgcctttaacggtaacctggcggtgttcatcttcaattgcccaaaaggcaataggtccacttcagttccatctttccagattatcacgaaagcattaccactatatgaggtaaatccctgtacattaataagatactcctttagctcttcgtatacgcctttatcgttaataaatacagcaaagtcaatatcccctgtagtacgtctgggagtgattttattaatgccgctcatccacacgtcccttgataccgctcctaccaggtaatagtcaattccaaatttcgatagcacattttccaaagctcctaacaaatctcctaaacttggatgttgccggatctgatcaaaatttatcctgtaagtactcatcgtaaattttttgagcggtttcaatacatcgcctatcacctgtgttaactaaatcaacatacacaagcaaaggagggactgtactatcattggcgttatcttgccaaaatttctgaaatacttttacattgccatttgcatcagaaacaagacgataatgtctgattatatcagctcgtttttccaatgtatataaagtatactcgcccggatgtaagaaattagtgagcaggtcagcggcaggttctccgccccaccatgtcttatcttccttaagagaaagttttttccaatgattacgatcttcttctgttaagaatcgaaaagtcgcaaccaataaggatggctttagcttttccttgtaggcgatcatccatttgtttaacaactcctttctattatttaaaaagtaactgttcttatctttcgggagcaaaaagccttgtttctttaaatcactaatgatcacattaatgttgccgaagcccactcctgtttttaatgctatttcccgataagtttcatttaccaggtcttcattgattaagaaatgaaacaccaacttaagtcctgttttagtgaatgcccggcccgctttttccgtttcagggggaatcactttttgtccatccagccagagcaacaaatcgccctcattgaaataaatattaccattagtttccaggtagccaatatcttccttccttagctcctctttcagttttggagagatgtattcagccatgacaataaggggatgatggctctcgttttgccttagtaaatagggtaattggtggttgcgtagctccttttttatcgtcacaaatgcgtgatattgctttttattatgcttaaaagctactttcccgtcaagatctttaggtgcattgggctcccatttcatcttgatgttagtctgcttttctaaagctacaatagcattttgagcgattatttcagtttccatgtttacattttttaactgtttacgaatcgtaaacaataaaataatataaacaaatatagacaatcaccttctgtttacaaaaaataaatgtttacgaatcgtgaacatcagctaaaacgtaaacaaggcttaatattcggaaactccgaatttcttagcttggcgagctttcatcatcacttcctcaactattcccattttggaagtagttaacgattcggaaattccgaacagttcaattaactcttaaagaccctctggtaagatattcatgtttctatacaattaccaccttaggaacccaatgagctggtagacattaaagccttatccgcaatcacccggataagtcagcgtaccttattccggcttataaaaaacgataacgagtttccacggctccgcattgaccgtagccttttctttcaccggcaaacagtaatgaattatatcatcaccaaattcgggaacaaatgagagggaagttgcgtaaaaaattttcggctaaatcgtttactacattgagtttggaaagaaaatggaaatagagaaaagtatgagccccctacttcccgatacagaaaatataattggttggttcaaaaatagttgcgatccgaagttaatcatagattcgcccatcgtgtccatagatcatgatttgaacgatctattcataatttcacgtactttcatccccaacctcaaccttaaaatatgcgatcatcaaccgacctctgcctattgtgccgcacggcacctgcggataaaacaaattcccacatccttccacgcttcatttctacgaattttcttcaggaaccaggtaaaccgagaaaaggcttcgaattgggcaccgaacacatagatggcaagagacctaagaccgtacaagactcgccgaaggaagattatatcttatgctctgattgcgaacattatttttccattatcgaaggcctagctgcagataccttcaaaaattggcgcactcatctggccggaaggtctttcacggaaattccaattacgccaccacatctatcagtagtagaatgtggggctaacattgccatgtattcaagactgctggtctattccatgttctggagagctagtatttcctcgcatgacgtgtttagaggatataaactcgaaggcaggctggaggagtcgcttcggggcaacctacattctgtaaaggcggaaaacagagcgaatgtcattgccaagatcaacgcaacagacataatactacacccatatacggcattgacaagccgagattttaaagacagtacagctaacagcatcgcagcaataaacgatcagatccctgcttctttaaacgtagatcagtttggatttctgcttttccctgattccgcctccattactcctgaaatcatagctccgctttccaatattgttgcggttgaccataaaattgcattaattggtgcagatctatggcactccatcatggtagagcgtctaatgaaagaagtggtaaagcgaggctggaaatgaaaataaaatcataacaaatgaagataataatcttagcaaaaagttattgcatcaatgatgccatcattcgcaatcaatataaacaattgacctatttacaatagttctaatgtccagataatcatcataactcaagcttccaaatttcgacaatcaggttacgcattatttcctgtctttcagcaactgtgtccatattccattcatcaaacgtcttcaatttagtagatgcgaagccattaaataacgtttgttcaccgattcttatttgagaaaaagtacgggtcaataagatattggagttgagataagcatttttctttacatcaaaccattgattggttgaaatatcattggaaaaattaaggctttgattgatgggtgcttccaacagcgtaagattgcccaaacggtaaactgtgttgggataatcgtatggttgcgtgtatctatcagctggaatattttctcctgtttgaggcaatatatgttctaattgctgagcttgataaaaagaatagttagctactgggaaattaacttttattcttatgaagttttccagttttcctaaaatgtattttatcctgtacagtggattcagatctccttggcctttagaggcaaattgtgaattgaacttggtttgttgatctgaaagttcttttcgaaaatcgtcttgcaaaaatgactttaattgttcacctgtatttattgccctcaactttaccgcccaattagcaaatttctcttcataagattttgtcaggattctgtttattgaatagtaaaaaacaaggctttcgatatttcttgccagttgattaatgatgttgttatcaatattatcctttaaggccattagcaacacaagatgttgccttgaagttttcttactgaggtaaccaataccagtaatacttggatatacattatcagcatccctgccgttggtggcctttatgaatattgaatatttggttgccgcagatttaagctcattggcgaaccctactgggtcagacttgtatttgatgttagctttgccttcatcagaaatcatccacttatagatttcatcttctcgaataatccccttatggtaacgcgccatgagaaagtaacggagaaaacgaagcggcttatccccctcaccactttcatcaatgcttttcaacattactttccatgtttgcttaatgggctcaaaatcgtcatccttcgcatggctgaataatagattcttcaataaatccatagcattcaagcccactcccctttcattaatggtctcaaatatcttcaaagcactgctgaggttatcaggcttaattattaccatttcgacattggcaagaaaataactgataaagtttattaatatgccatcatcatttacctttaactccttcaagaagtccgatattgttgaataggcttccatcatctttttaatagaaggagtttttatatcagtaaactctttttctccaatcaacctattcaaataatctttactctcagcatattgtaatgataatctaggtgtgtgcttacgactgctaatatcatacttataaagtagctcccttacaacctttaaaagctcatctctaaccgtccttaaatcatcatcacacatatccaattgttgcaatgaataccttatagcacaaagagaaatcacaatagtagtaagtctttgctgtccatcaactacatcaaaagcaccatcttcacgttttactataatggtagaccctataaagtaatttgattgctttcctgagttaggattaaactcatcgataatatcttggaagaactgcgccacatgaatatcagcctgccaaacatactctctttgataatcgggaacaacaaaaaaataatctttgatactttcgattgattttacttctgctttaatctccataaaactagttattccagttgttgattaattctactaatctccccactttacacaaaaataatagaaacattaactatcgccttcgatagtttaacctatctaatcttaatttcattgttagctaaatcatacatatagccgactatttcccctgaaattatcaagtcaatagctttctcaataatttccaatggtgcaatgaaccattcccttggtgtataacgattcccagctctatcgaaaacatcgatattcaaacacgctcgaccgaaaaaattatgtaatagaagttccaatttctgcggattcaagttgtaacatttaaccgtcattacgatgcttacttctgccataaggtaggtcggttccaatgcggcatttttaattctatcttcaacttcgatcttagaaaaaccaattttatataaatcatggatacttttaatctcaggattctcactcttggatttgagtatgtatatatatcccgtttcgaggtcgtcaactgtaattggggtaagcgcttctaataattcatcatctttgagcgtaacccttctcccatctttataaagctctgctgccaatgatcttaataacatgtcagattcagtcccattttcaaaaacacatctcaatctcgcattcgttttgccattctccaattcacgccgaccaatctctgcaatgtataatagaatcccttttaacacataaaatcgccctttctcaatctgttgttcatttttaaaaggatacaatttgcggattcctttttttagttctgcctggcactcaataaataaatcagaaaattgttcaaaatcgacacattgtattcttctgccaatatattctggcatagtggtgaccttaggaatatttttaagctcgtgaaggctgtctgccgtatcatccgctaagaggccgaggacatcatcctccaaaatatcggctaaagacgttacatttctttgttcaaattttagcagttcaaatcgatcatagttaagcaaaatctgctttttagccgaattctcgcggatagacttcaatcttgtaaacaattgatgctcctgaaccccatttccttgctggggctccctcccatatttctcaaaaaaagagttaatctccaaaaaggaattgattagcctttcttcctctggcattatggatgaaccagaaggcttaatatttaaaagccctaaagggtcattattgaatatttccagcagcttttttttatccttatccattatctgccttccgcttttgttctttcaaaaaaatgattccttctgccattcttctttctaagggatcagtagactgaagaataggctccttcttaaacgtttttacgaaatcgttaatcttcggccaaagtattaaggcttcttccaatgtcatttgaattcttgtagcttcaatcacatcttgaatgactttcagtacttttggcgtaacatcctttgatataatctcaaacgctttttgaaatggattaattctatctatcaaatcaatatgcaagtcatctatatttataaactggcctgccatccttataaaacgtttatcgcccacctcctttatttcccctgttttaacaactgaatcaattactacatgttgtctaacttcctcaacttctccttcagttaattcagggtatttcgtttttataattttggggattaaaactttgttgatcacttctggatcgacattaccgggtatcgcctttagtatcacatcactttgaagaattgtcgccttcaaatcattcaggtcagattctactatatctttaactcttttagaagtcggtgttttaaaacctctgatttttatttctccttcttcggctttgtcatcgtcagaaagttttgttttgaatttaaaactaggagccaacacttgttccattaacaaggatgctgtaatagctttaagcatattatttactgactgcctcaccagatcgtctgttgcatcaggctgtgcaatgaggttggtaaattgtgcatggcttttgttgctactatctctcgtacatcggccaataatctgaataatttctgttaaagaacctctatatccaatagtcaaagcatgttcacaaaaaggccagtcaaaaccttctttagccattcctaaagcaattatcaaatctaaatcatctactgttttaatacttctgagataatcaactactttttctcgatcttttggattatcatttactaaatctgcaattttcaatacctttccatcattagccctctttagatgaattattcctgtgtcggcatctactttagtaatgtctccaagggtatccagtattgtgtctacttcgccttgcttatccttggtagactcaccagaatttacatttggaatatgcaatattgttttcttgtcagtatctaaaatatcaagaatggcagaagtatatttaccctgataaaaatgatacccaatacccaatgatttcaaataggtatagccattaagttgttcatagtaattatacgtcactttagtgaatttagcttcctcttcagccaaaagaacaggcacactatcaccacgaaaataagagcctgtcattgctacaatgtgagccgatgaattttgcataatacttcttaacaactcacctaaccgactgtccccatctgctgagacatgatgaaattcatcaagagctaatattatgttattgaatttcgactcgtctaattcttcaaatgcaaaacgcaatgttgcatgagtacaaatcaaaataggttcttcattgtctagaaagtttttaaacgcttgtaccttacttttgcttccatccattcctggtgtgcaaaggttgtattcgtcattcggctcccaattagcaaaaaatccagaattcttcagatcagttttgccaaaagagcctccaatagatttctcaggtacggctacaatcactttctttaacccttgatttattagtttatccaacgctaaaaacattaacgctcttgattttcctgatgcaggaggagctttcaatagaaggtactgtgcatccctcgcctgatatgccttttcttgcatctcacgcatgcctaacgagttaatatttgagcttctccctgtctgggcatattttacatgaattatatcaggcataattatttcctcttcttttttatcgcagtttcaaacaaagtttctttcttgttttcggaatttatcatctgctgatagagcttaaacaaataggccagtcgttcctcgtcagtttcaaatggcttacttctatagcaacgttctacagcaagatcaagttgatgatgagcttcacgaagccccgctggcatttcatcaggattataaagctgcgctaatgttttttcagaatgcttttctcgttcttctaacacattatacatatgtctttccaattcttgtttttgattgttgttgatttgagggaacggaaaagtattgtatccaagggatgaagaatatcttattcgagtttctaagctaccgcatactgcttttatccaaattgtatgaattgaggaagttactattgaaaaaatatagtttggagcttcgtatattgcctgcgcagaggcgtagattaccggccccttgtctacgaaatcaattggtatatattttctttgctctgaagtaacacagggtattacaattgagggcttattgatatatctgttctcggcaaagcgatgagggaaagccgctagtttctgcgttggaatttttgtgcttttcagcctcatgattttaacaccttcgaggcgatttcttataaattcgatctctgatacttttccagcatcttcatcaggaatatacaaacaccatcggttgattttgtcaattatttcttgtgcacctatgaatttttttaaatacggcatcagactaccattttttgaaatacgcttaaattcggcctcatcaattatcagatggcctccatcagccggaatactacctttaatcattttagggaatccacttatcgaatttgacattctgctaattattaaattcgggccatcaactatataagggtttatattacttactatttttcttaacccctgattaaaaagatatttcggtctattattaatattccttacacctattattaaaacagaaacacctgcattcgatttcgcattattttcccatttaaagctctgatgagcaaaatatatttccaatttccaattcaacagaacagtattccaagtcacactaacttgatcaccttgagaaattgaattcgttgttacaaatgcatatgaagaattgtatccaagtatatagtttgatgctttgtaaaaccagcatgcgatatagtcaagggttttatagttttgtatgtgacccagcacaaaactaacatcatccttatgttcttttttttgatttcttgtacccagataggggggatttcctaaaatataaatctcatctcttccttttttaggacaaacggtttgccagtcaatttgtgttgcatttccgcgaataatgttacctgtctctttaagaggaagggctggcttagttcttccgaattctttgaagaattcttgattcatttgatgttccgctaaccaaagagagagtatcgccacctcatgggcaaagtcatctaactcaataccataaaaatttcccaagctaatatttgaaagcgcaaggctatttattattttaaatattttcatttctaatcggcgtaactctttgtaagcgataattaaaaaattaccgcttccacaggcaggatcaaaaattttaatactccaaatacgattaagtaaggcgttaagctttttcggagtatttttagatatttccagttcttcttgcaattcatctaaaaaaagtggcccaattactttcattatgttaggcacactggtgtaatgcatacctagcccttcacgatgttctggagtaataaccgcctgaatcatgctaccaaaaatatcaggattgatcgcgctccaatctagtttaccactttcgataagtatttgacggctacgtcttgtaaaaattggggcacgatgtttatttttgaaaagtcctccatttacataaggaaatgcttcttgataggcagacaagttccgtcgcttatcgtagtcagtattcattacatcgaataacccttcaagataaacacttaggtcgctcccatcttcttgagtgtggctttctatagcagtagtaaactgcgctttttcaaaaatatctgtatcctcagcgaaaaaacaaaatagtagacgggaaagaaagacattaagattatgaacttcttcatgtgtgctagttatattatccttttttatttcatcatataactttgccattcgttcggcagcctttacatcggcaggattctcactttggcgttgggccttttccatgcctgcccacggcagaaaaaaatcaaaatgttttgcaatttcagtaatagggatgtctaacgtatgaaaggttctacgatcaattgccaacaatgttttaaagtcagtgaccactataaaacgcggatcatgctttattcttaaatcattttctttaataccagcaatcacttcatgtatatcttcatcttgtacagatttaaaaaatacttttttcttccatgccacttctccaatggcttttgaaagatttaatccaccatgttgcaagcgagtaatactagctttgggatgaccatacgctagaagcaaatcgtaaataaatgattcgttattaagggagcttactagctgctgtaaattactttctatttgagctaaattcattaatactaatctttcacaaattaaaatgacatacttttatacgctggatgacgtccttttcatactgaaagaatgatactatagaccaggaagcgcacaatacattcttatatgggcctagcaattaccatcaacaaaaatcaacttatctattgcaataaggattgcaaaatgatctgaaaagtacatcttcaaacttatcaacatctaaagtgaaataaggagaaggctttctcatcaatgtacttgtgataaatcatactttcatttaaaccacttatactatcaacatttcttacttgtatattctctcaaataatgaaacgttctctaacgttcttactctctttccaggaaacaggatgccccgaatctttataagcgatcccccttccccatgtgcatgccaggcagtttcataatctacagaatttagttctaccctcgcattaacaatctctgaatctattaataaagccaacatcacttctcctgaacgtctgccatctcccccttcattcccgtttaaactttctacagttccaaaaaatgtatcttccaattcttttccaattggattaagataactctttatttcctctagtttaggcttaaattcatatggaaattttatagccctaggtaaattcaaagggggcaatttcgtcatgtatgccctactccaattaaaaatcaattcaaacggcaattctctttcatcatcaaaaagatttatcaatgcatcacaaaaattataactgatgctcggcctagaagaagacacttgtgcctctattaattgatcaatactgtcagcctcaattgcatttaacagttccttagaagtataattcatcaattcaaaagcacgcctactcagtggtttaacaacctcgtcgtcaaacaacgtcaaggatgagcttctttcaagttcaactgggcaagatatctttaaaataaaactcccttcttctgtatgtctaaacttggtcttccttaacagctcatttgcttcgttcctaaataaacgcttatgaagtaatgaaggatgtactacggagctaccagctgttaaaatcaattgtttagtcgcgtcaattgctttaactgtttcctggaatgacaacgcattgactattttagattcagagaaatacctcaaattcaaaacatcgtcatttacctcccttatatcctctaatattttaaactctgattgattactaaagtcccctaattttctgatagcaattaatgccatattctgaaaatctggatttgaactatctgtaggaaagattaactgtttataatccttattggggctatttaatacaaacaatccatcttttagaccttcacgtactaattcccacccgtaactaaatgcgtagtctctaatttgtattgatgatatatctatcacttttctcatgatggaacagtgtacgttggtatatttccttgcccaatttcttgacaaattgcaacaagactatctggcgttagcaaattagtctttggaatatagattgtctgactaacctgattggtagaggccggtgcattatataagcaaatccaatatgctgcattccttaaaattaactcatctatggaacatgataaccattcattatccgaatttgggaggagaagaactactagtaatctatgcggttcgcctctattagaacgcaacttatcatattgatctattcctcgaaaagaatacgaaaaatgagttgaagtttcggactgaatattagtcgtcgctttgagttgaattctcaacgaaacgtctgtacggtaggtattcggtataggtgcaaaataatcaaccaatgcatctgttccataattatccccatgtctattttcaactttgcaattcattccagccttacttgcaaccgcatgtaaatacgcataacttaattcagattctacatttaatgaggataggggcataattacagggattttttagaataaaactcactaaattctacatttagggtatcaaggatcttaattagagttgtaaatgatgggtttgatgctccttcctcaagcttctgcacataacttacagacaattctgaggcataagcgaaatttctaatacttaatttcttcgccttacgcaatttcttcagccttttgccaaactcttttaatatttcctcctccttaatttcatccattcatgaaatttcaactaaatccgaaaatattttgtacctctatagaggtacaataagaaaattaccctatctttacgaagtgaaagattatcaaatctttccataaaatgctaaattggcgattccatttaatataaaatgaatcgtctcgcaaatgccttggtccccgaaacgaccaaattccagaccaacaaggcaacggcgaagctcacgtcataaaggcgcgtgggctcgcgttgctttggtctttaggcgcttggtcgtgccaggggacggtaacgttgagtcctgcgccttttttatgctcacgcagcaggctccaattaaacacactgaaatggctttggtggttaatacccactacaatcttatcatgtctatttgaaattggaagctatgagtagatacattacaaccggcacactggagaacataacccattttcaacttttcaaagtaggtgacgaaacagggctgaactacatatacaataacctgtacaagtcgatcttctattacgccaggcgcataattgaggactcttttgttataaactccatcctccaggatgcctttctccgagcctgggatttcagaacacgaatgaccagcatgctccaccttttccgattcatccggctacatgtccggtgggggtgcttcgaatacctcagaaagaaggtcaataaattccattgcagctttatgcaccttgaatttcttgagaatacccattatgcctcctttaacccggagcaagaggcagaatatagccatctgtcagggaaggatcttgaacacttggaaagaatagaagaggccattccatatctaccagcccacaggcaaaccatcataaggctctatatgctctatggcctcaactataaagaaatagcgaaacggtttgcggctccatatcagcatattacaacagaaattcaggaaagcatcgaatccctaaaatcgatgctgctggtacttccgcaaaagcaagccactattagaagaagccatcacgataactatacagcacacttaacaccagaacaagcccagatatataaactacggcatcaggacaaatacagctttgacaggatttctcaggaaacgaacaggccattagccgatgtagtaaatcaatacgtttcagccaatcaaaccttacaaaagattcgcaaacatggaaacaagaaaaatcattgttacgcgtagaatccagttacttatcaatagtgatgatgaccaggtaagacatgcaacctgggaaacgttgtggcaatggcaacatttctgtttccgcgcagccaatcagatatctacccatcactttattcaggaccagataaaggaactcttctacctgaaggatgaaacaaaagtcaaactaactgatgtccacaaagatccggacgggatattaaccacctccaaaaccaatactacttatcagttcctcagcaaacgatataaacaggaaatgccaatggcaatactagggtgtctaaataatacccttgtatccacatacaacaaggaaaaagaagcatactggaaaggggatagatcattgaggaactataagcgtagtatcccaataccgataccagcgaaggctttactcaacataagttccattgaaaaaagtagaaactatactttttcaatctatgggcttcattttagaacctatttcggaaaagatctggatgataagtatagtatgtggaaaagggctatagaaggagattacaaactatgcgataactctctgcaattaaatggtagtaagatttacctactggctgttttccagtttgataagctggtggggaatctaaagccagaggtggtagcagaggcgtctctttctatggaaatcccggtggttgtaaaaatcaataggtatcaatatagaataggcacaaaagaagactttctttatcgcaggatggcgatccaggaagcgatccggcgctgtcagaaatcatgtggctttaacaggactaaaaatgggaaagcgcgaatgcgccaaaaggagaataccttccgcgatgcagaaaaaaagtatatcaactataaactccatgtttacagtaaacgcctaatagacctttgtataaaacatcaggcagctactcttattctggtggatcagcaggaaacagaagaactggcaaaagaagaaaaatttgttgttcgaaactggaactatggcggattacgacaaaagataacctataaggccaataaagccgggattaatataattgtagaatagccctggctaacaaaatatttgagggtgcttgtacacccgtggagtgaggcttcatgtgtactcactaaatatctttccttttatggtatccatataaggggtgtatacaattacatggttcgcggctcatcctgcaaccgtaccaggaaagctgaaagctatatacaacagagtcagtactctacaaacaatcaaaccattttattattcaattaacctccttcaattatggaaaatagtaacccgctaatcaattcttctgaaatagaagatgactacagtcaacggccattccggcttaacaaacaagaaatcaataacccacaattggtaattactgatttctgggaaagatattcccttcaaagctttagaaaacatctatggaatggatttattaaaaatctgcttatgggtaacattgatccattaggaacagcagaactatacatagacatggaaagaatgattgaagttacttttctgcttagaaatcaggttaccgataatacaccagaaaacaaataacttccaggaccaggcatatccaggattataaataattacattaacaacatattaactttcatctaatacaatatcagcatggtaatcattggtgatcttcatggaggttatccggaaatactttacaagatcaaaaaattcggagtggagaaaacgtcctttatacaggttggcgactgggggcttggctttcagcataaggagcttgacagaaaagcattatctcaaattgataaatttcttagggagaaggaaaatattctgtacatattgagaggcaatcatgataataagtggttctgggatcatagggatactttcaatcttcgaaacgtcaaactggtacaggattatgaagtacttgaaatagaagatcaacgggttatttttattggtggaggtatatccattgaccggttaagcagaacgcccggtaaagactactggccggacgaagaaatccggtttgatgagcctttgctacaatcagcatgcgctcaaggtattgacatagctatttcgcatgtagcccccaaagaaacatggccttacacctttgaccctatcgttcttaattttattgttaaggagatggccgccggcaaagacctggctactgatcgggaaaacgaacgacagataatgagccagatctacttacatcttaaagctgccggatgtcgggaatggtactatggtcattatcatgaatcccatatggaagaaagagacggattaattttcaggtgcgttgcaatccaagaaatgtatgacacaaaataatctaacacagatatattggttggaaggcttcagtggagttgctcacggcaaacatgtcatttctattgaagacctaccggaatttcttaaaaaatgtaatgaaaccgggctgcaggtggtgggtttaaaaatcggcgacccggttcaacgtctggaatgtattcttcacgccaacgatagctatattcagcaatttggtaagacagcacaggaaacctggtatttcaggccgtagcaactactgattcatgctacctgctttcttcctcaattccctcgcagactgttcttgttcagttgccagtcgtagcatttccaacctgtcatttttcaattgctcctgatgcagcacactatcccgcaggacagaattacaataatataggctatcggtagtaattaataattgttgaatagacttattccccagcaatttcaggaagcggtattttgtatctgatgctttatactgcttcagattatcagctgtattataccacgccatactcaggaccgcaacaactaccaccagagctatcgctataaaaataacctttgacaaatgatgatgatggataagattctcggtccggggagttttcatgatccggatattttcagataaagcagcagttagcgtgacgacttcttctttaggtaaggaatgtcgaatgaaagtaccgtgcatttccttccatatttcgacaatcttaccggagctatcggggatagtctttactttttcatccaagtcctgcagtgatttttcttgcttgtctaacttggcagcaagtgtttctataatctgatgcatgatttaatattttaaagatgtcaaagagatgggccttttttctttcttctcctttttctatcaaatgcctcctgggtcaattcatacggaataaaattaccagtcatctcaggttgtaataaccattcaataaagtttgccaaattttgaatagccaacgtcaggggagaactggtaggatactggagccgatcattatccgtatagtgaatatttttcccggattgtcttcgggagagtgattcgatattcttttgctcaagttgcttattcgccagttcctttttcagggataaaatcttctcaatttttgaaagggagaagccgacgtcgcttcctttaatctttaccttctttccatcaataaaagaaatacctcgacctttaatcactgtataacccaatgcgcgcatagctttttcaaaagcaggataatcattcacgtccctcaaagtattccggatgtgatctttcaatttcatctttctttgatcctgccggggaattaattgctggtctttcgataaaaaagctttgggactcaatacttgtgtcaatcctagtttctgttcctgcttccggcaaaaagcagccattcgtctatagctgttactatcactggcggctttaccatcaagccctaccctgtttactacaatatgaaaatgttgctcacgggtatctttatgaaaaaccattaggtactgatgatctgcgacattgaactcctttaccaatgcttcccccaactcaatcagctgatctttggtcagatggtcaccttctgccagtctgatagaaagatgaaatgcgggcttttccactcttttactcaggcgggctacatctctaaactgttcagccatctcatacttatctccgaaacaattattaaaggcaagtatttccgctctatccttatgctgaacaccatctcttaaagacatttccattttctgatcttcggacaactctcttttatcttccagtacataactgataagatgataaaaagaacttccggttattactgtgccgatcacctgagataatttttaatctccgcggcaattccctttagcaccggcaccagatttttgaggtccacccgctccagcattgacaagtcttcattcttattacgctttttggctacctggttgatgttcgcggctatatgattaagtgttccggatagcgccaatacttccgcagggaatactttaacctgctgatcaaccttaccatttacagacatctgcctgatatactctgatatattaaggtttaattcctttgccttttgggcaatgaccaacttttcaaaagctgaacatttgaatgtcaggataatatttttcctgacttcttttaatggacgccctcctttattcccccgctgcttatcattctgcgtcataattcagttcattttatttttttgaatccgcctgtaagcggatgaaaaaacccgcccacaaatgcgatagcatgcggtgggtcagaagttttggtattaccaaaacatagctggctataccgaacctcaagacccatatgctcctacccgcatggttttcctatgctataatttgtcgtctgatttgggagaagctatctttttaccttccccttcaggcccgtttttcttgggtccgggcttagttaatttgttctgaggtggtaactccatctcaaaaatcatggggttatctatcccgtatttatagatattctttttcaagtccatccaaagttgaatgttataatccgccaattctatcagttcatcacgggttaacctgaagggattatgcacagatgcgagggaattactttccgaaactccatcgttgcaggcaagtatattggggcgatacccttcgccaagttccaatgatttccctatagccatgctatttccaaataacttaatctgcttaccagaacttaattgcagtgtttttcttttgaagtctgccataatttgagatttttaatacttgaataattactcccgagaggagtgggttacagtgaaacaaaaaaggatcatcccctttttctgatgttaacctgggcgtagctttctgaggttgtcttgtgggcgtttggtggtttccgcagggttagaatggatgaggaattgatttaagtctttgtagttcccatatatgtaactgcaatcccggtatttcttatccagagataacgcctgatgcgtttgggtaatacctgctttgtctctatccaaatacagatgaatagtctgatacccctccattaattcccgactctttttgaagaaggacaaagaatttagtaccaggtaattcgtcaccggcagatttttcccctgaatgatcaccaggaaagatagaaagctgaagaagccttcatatacggatacttcagatgcaccgttatcaataaacgtagttgccttggggctggaactccctttgaaataaggattgcgcaattcatacccaccggcatcatttttaaaaccgatagcgtaataatcctttccgtaaagagagtaccggacttcccggcaaaactgctcggcaagttgcaggggaataccgcgcacttctaaatagtagagcagggccggtgaagtaatcggcgcatcccctatcacccggatctttttttcttcactggaaaaatggggagctggcctcgctggtggaagctgagagataacctggtgccggtgaaaggaaagaaaagattgcagcttctccagaacttcaggaatagtacaatggtaaaacaacattccaaagtctacaatacttcctccctgaccaattccaaagtcataaaacagattcaatctgcggttaaccttaaaggaggcagtattctcttcccggaatggagataagtaccaataatcctgactttggatcttctggggctgatagccgagggatgccaggtaatcaaccatgtcgatccgctttgcctcggcaatggggaaatcatttgttgccataaaatggtttgagatgggttaaagggttaatcttccggttcgggtttctggttcatggatcgaatccgcttaatgtcttcctccagctcagacagataaaacaccttcttacgctcaccaaggtcatggcggcggatcagggacatttgcacgaacttccggagcgtgggcgccgaaacacctataattttacaagcctgccggatgttcagcggtgtttctgataaacctttggataggttactctcctggaggcaggacttaacgatactttcaataaagagccttgcttgctcgatactgaaaccaataaattgcatttgctcactcatatctcttcactattgattcaaagcaaatatgaacgcaaaaaatgccggttttaggcaaataccggaaaaaagatgcaaaatccggactttatttgtaggagggagattacttattttcttttattggcggctaactcattcttaatcaagtgaattatggaagacatatcactctccagttttttggcgcttttgacgtctaatcttgcccatacttacctcggaaaaaccggcaaatggacttccatttgcattgaataaccgaactttcttttcaattacctgccaggaaacgataagcccctttgcttccttcaatgcctggaagatgatttttagcgactgattgttgaaattcttctttttaatcagttccaattccgggctatcttcattactaaatatcttacgaaaggtagcaacatcataagggacatgaaagtaagggttgaaggtggtatataaaaaatcgatcacctcgttgcaagtttccggagagagatcttcatttaatttcagataattataactgctggcttccctttcccgcttccccgttgtgggtgtagtctcttgtttgggaggcgggacagcagattctttattgggatctgttatttgctctttccctatcttctcttgtagattttgcaaatagtcgaataaaatagtcctttgttccttatcattttcaactatcttcaaaaaatcaacattcttctgaaagttagatttcttcaatagcgcccatttttgtttgttatctgcgtcttccaaatcatattgatatgcctgaggatattttacaagaagttgtttcaagtatgccaaattctcattatcgaaatgccggtttgccaactctgttaatattcctatgcgcagaatagattcttcaaaattgaagtatagatatcggctgcaccaatcaaaatgggcaattaggctttcaaaactcaaaggaaatgggcatgctaaaaaggaaatacagaaatgattatatcgagcatggttagccagtttatcaaagtcaattgcccagcgtgtagatttggattggtcattgtaaggaatttcacgaacaaaaatggtcgtttcaactacccttacaattaaaggaacatcctttacttgattaaggttggtcatgtcctgccttttttaacacttatcaataaatttttattaatagcggactgatggattaaaatttttactaacctgccccgtctccttcatatggttaattaaatagctaaactcttcatctgtaacctgaaatcccgcattatcaaatagatcatatgctgggatatacttttgaattaagcttacaattttttcaccataaatagttgtcggttttaacttagctatttctgcactaaatctgtccgcagataaaattagttttagcattggatcaaatacaaacatcttatcatgtggaggttgcattaatggacgaataacaaatcgtaaatactcttcaaaagtattgggcttttttaataaatatttcgcataagcttttctcgtattgctttgatcttttacaagtaaaaaatgatccataaccttgttggaaaactcaggatcgctatttaaataatgaataaatccatcagaaataatcttttctaattttggttttgaaaacccagacccaatagaccgctccttaattaagtaatcagcgataatcgctttattatactcaggcaaagattcgtcatttaatattttcattataacatcaacatactcttcatcactatcataaagactatctccatcctccgccaaattttgtttaacgatatttaataagaaattctgaaacccacccacttttataaaagctgttacgaacttttgaaactcatctttattcctattgataccatacgtttctaatatggcagcaagttctctataatcattgaaagcccatttgttcagaaactgattaaggtcttcttggtcaccgttaatagctagtgtaaattctttataggaaattgaattaaataactgaaaagaaaagtataaccaaaaatgctcagtgctgactaatgttctaggcgatctatttgcacgatcttcaaaaaggtactcaagaaccttctgcaattcagtaagctcactctcgtcaatgaaactcgcgttcttctccttataagctgtccacttttcagtatcaaattgaaatttaaatggcggatcagctgagacttttacaaattctcggttagaaacatttatatatatatcaaatcttttaacttgtaataatgccaaaataaaataatcaataacatctaattcatccattataaaactgaaattcaattttataatgttagtgaatcgctttaggtcacgcatgttatcaatcataccttctaaaaagtgctcaggtcgtttcagaggagttatcgactgggcaatattaccataagccaaattattcaaggcgtgatcaattttatctttataatcttgctttaaactatcgtactgcaataaacttttgaactcaacaacatatatacttttctgtattttcggaagaggtattattagttgaaagacttttttcaaatactcctcctcctttgaaagtaaatttattcttctcagtacttgaataacatagtttggatccagcgctacaataaaaaaagtattggagaaatttgcagtattacgaataagctttaaaacatttagtatctcaatagcattaagtctatcaatgtcatcaataaaaacaatgatcctcttccctgtttgctgaatgccctcatttatagaattataagtttcagaaatggattcatctggtataacttcattaataagtgtatctaacaatcggaaatagatttcctttccaggttgaaaaagtttttttgaataagactttagtttatttccaatggatttattatattttttaagtgaagaagaaagcgtcacaaaaaaatcctcgatcaagctatctgtactacttgttttccaaacattaaaattgataattagattatctgaatttaatttcagttgattttccaatctatttaaaaaatcagtcttaccggccccccactcagcaaaaattcctatagagaaagaatttttagaagtagtgctgtttatcacgctggctacctgatcggcataccctgatcgacttaatgaatcattttctgaatctggacaatcctcaattaatgatatctcattttggattttaagtggtcttttatatgatttataattactccataatagcaaaagactaaataatactaaatcagtatagtataatatcggcaatccccaattttgaaacgaaaaaaatacataattgtcattgaaccggataataaaaaaatatattaataatatagttattatattaaagaagccattgcctggagggattaatccattctttattttatcaaatagcttaaaaatcccatagataaaaaaaacactaataattacattaagtacgtgcccctggtccaaataggtaaaaactttagaaacaactaagttgtctccaacttcaatgacataccttttcatcactagtgtaattactaagacgaataggcatttgattaattgcgagtatttaaatgactttctatattctgaccaattatacgccttatagggatttttcatagagaaaatattgtctatgtctttaagataagtatttctttgataataattactagcctctcaatgcatttgcctgtaaatacctattaacataatcatccactgaaaaagcagcaccatcaccctgtctcttcacccactccaatatctccgacttcttaaacttatacagcttccccatcttaaaaaaaggtatctcccttttggaacacttaccataaataacattcacatccatccgcagcagatccgccacctccttagccgacataatattctcgtgggcatgcgattgaaaagcccccttcgacaagtcgagtaattcagacaacatacttttgatctgctggatatcgctctccatccgatccaacctctgctcaataggcgataaactcatgtggggttaatttaaatgtttattaatagccttgctggctgctttagccctattcgtgtccggcaccttcgcatagatctgtgtagtcttcacatgcttatgattcagcattttgctgacaacataaatatcttcacccttttctataaggtcagttgcatacttatgccgccagttatggaacttggctttatcttttaaacccacgctggcaaaccattcctgcaaccttgtacgggtgcgggaataattgagatccggaaatattagcctatcctcttcctgcttctctcctaatatatcaaccgcttgttgactaatataatgcttgaaagaccgttccggcttggggtctataatatacacgtaccaggtacacaatgcttcagagaaatgcaaatcactccatttcagtattttaatagcactaaaccggaagccactcagcaacgcaaaaatggaagaccggaaaacagtatcatcatcaatgggattctccaataataacctcagctcttcatcatcaatgatctgccggaaggtatctacgttactgattcgcggtacacgcaaagtatagtcttccggtagatacttatctaagaaagcactctgaataatgagaataaatttatcatagtaagaagcagccgaattctgagccagcttcgcttttgaagactttagagaattagtcgttaacagatactctttgaacttcttcaggaatatttcatcgatgttccggaatttaaaatgctctcccatccatcgtttcagatacttgatggctgtttcatgatgcgttgtatcaactccttcccgctgttttccacggatgaaattcaacgcatacacgtagaaatcggcatccagtgcatctttgttatacaagccattagcatccagcatcagggctttcattcgtttgagatagattttctcagcaatctcgttatacagtttgttttcctgtttctccagtggagtaacaggattagcgtgtagatgcaggttaaggaactcacggcgggtgtattgtttagcctgtggattccatacaggcgggtaatagtctatataaagactgagcttcccactcttcagcttcttatttctcagcgctcctctcatatattcccgtatttggtggttaaataatctatcacggtttgccggtgaaaaagaagactacgccctactttcagcttggggaaatcttcatcttttatcaaccggaataaagtacgttcgctgatgctggtaagggaggatagcgccttaatatctatcaggtcacccaatggttttgaggctggggtatcaaccaacctggatctagaaagaagttgagtgtttgtttctgactctactttctgtacacgttctttcttctcacgtaatttataattgcgccgggcgcaggtaagcgaacagaatttggttactgtcttttgggcgatgaacacttctccgcaatgctcacaaatcttctttatccttaaatgactactcattttttagaagttgaaattggaactgttgggaggctactgtctggggatgaactaaactgtctattactgccttatactgtcaattactgccattatttctctatttccccatgtacatttgtacctccgtatcttattactaatttagaggtttatggatcaacaacaaaataaaacaaaggaaaaatcaggcatcctgtcaagatgcaacactgataagcattacgttaggcaaataaagaaaagtagatgtaaataaaagaaagggcttactttccgatacaaaacttactgaaaatataatccagcctgtcctcatttgtcacctcacccgttatctctcccagataatgcaaacaaagccggatatccagtgccagcaagtctcccggcagaccgtcgtccattccctgttttacatcctgtaatgatttcagcacttcctgcagcgcggcgtgatggcgggcattggtgatgatggtatcttctgtgttgacatcgcctgccagtaccttatgtaccagtgcatctttcagctcctggatgtgtgcatgattctttgctgagataaaaagtatttcaggtataccggtgaatttggcgcggatggctgcttcaccggtgatatctgttttgtttcctaccaggagatagttaacgttttgtgattcaaaagcagtaatctgattacgtatatccgtttcagagagttcattcacatcaaagagataaacgactacaccggcctcgcgtattttctccattgttttctgcacaccaatgctttcaatggtatccaggctttcgcggataccggcagtatctataaggcggaagaggatgccatcaatgttgagtatttcctcgatggtatcgcgggtagtgccggcgatatcgctgacgatggcgcggttctcattgagaagcgtattcagtaatgttgatttgccggcattgggtttacctactatggcggtattcacaccatttttgataacatttcccatccggaaggagtcgatgaggtgcttcactactccggtggcattagtaacaagggtatataagccgctacgatcggcaaattccacgtcttcctggctgaagtccagttcaagttcgatcagggcggaaaaggtaattaattgctcacgcagggcatgtaattccttggagaagccaccacgcatttgttgcatggcagtttgatgggaggcggcagaattactggctatcagatcggccacagattcggcctgggtaagatccagtttaccgttcaggaatgcccgctgggtaaattcacctggcttcgccagccgtgcacctgctttaatggtggcatcaataatttgttgttggatatagggagaaccatgacaggatatctcaatcacatcttcgccggtataagaacgggggcctttatacaggctcaccactacctcgtcgatgatgtgaccattggaaacgatgttaccaaaatgcagggtatgactggcttgttgcaggagatccttaccagggaatagtccgttacagatcgcataggtatcggggccgctcagccgtattaccgcaatagcgccgaggcccggggctgttgctaccgctacaatcgtatcatcaaatcctgttaatttacccagcataccgtatttagtttatgaatattcccaaagggcacaaatttacggacaatcggggctatcaccaattcctgaaaatcaaaggtcccgttccaactatgttgaaacgggacctttgaaaattatattgatacagtactactcctgcaaagtaaagcggatagggaggttgaactgtacagaaacctggcggccattttgcttaccagctttccacttaggcatggttttcaccacacgcacagcttcttcttccaggccaccaccttttgcggcgcctactgtttttacatctttaatatttccttcagaatctactacgaactgaacgaatactgtaccggagataccattttcctgcgcaacgcgtgggtaacggatatttttgctcaggtatttggccagtgcttcttctccacccgggaaggttggaggttgctctacgaaagtgaagatttcttcttttgcaggagcaggaggcgggcctactacaccggtacctttactatcttccagtaatcccggatcaactccgtttggatcaccgtctacagttttagtactgatggctttatccttaatatcctcatgtttcggaggttcctcatccggtggtacttcattatccttcttaataacaggaggagtgaactgtactgacggttttaccggtggtggcggcgcaggcggtggaggtggcggaggtggcgttttcggatcatccggtaacttcacatcctccatcttaatttcctgtatcaccggcttcttcgtgttttcaccctcagaagctttaacccactgtgatatcatgtacgttgcaaagaatattacaaacaatgacgcggttcccaaaatggcattccgcacacgcttattatactgtctccgcaaatcgtacgccccataatccttgttcctgccgtcaaacaggatatcaagaaaatcggactttaagactttagcagaatccattgttgttgttttatgatggatgcaaaaaaataattagttatttagccggcggagttgcaggagtgctactaggtacaccgttagctgtttctgtagactgtatccattttttatcctggtcactgatatctacggttgcataacgttgaatcctgttgatggccatttcatcaagaatatctacgaaattcttgtaattagcctgatcatcagctttaataatcactacaacatcttctggttcaccttttgcatttctcagtttggcaacctcatccctctttctgataatctcatctctgattcctccggtattggcaaatgatgttgccttgaagaagtcaggattagcagaggcattcgggtcttgtgccaaaccttcgtaatagtaaacacgattatcttttccgagtaaaatggtcagggccgtactttcttttactttgttctggtccttctcattttcggtatcctttggcatgatcaagtccattgttttgggcttggacatggtagtggtaagcatgaagaaggtaatcaggagaaaacctaagtctaccatcggtgtcatatctacacgggtagattgtttcttggatttcgtcccaccgtgtttcttgccaccgccactactactggtatccatttctgccatagtagccaattttttttagttcttaaatcaacagccttccaggtcaggaagtaattactgccgtttacttcttaggtgcatttgcctcttcccaggcagcagtacctttaggtgcttcttccaggttagtaaccaggttcagcttctgaatatgcttctttttgaaggtatccaggatttccttgatctttggataaggagtctggttgtctgctttgatacagtacttcagcttcgcaatgcttccgccttgtgctgcaacaccatattcgatccaggcacctaactcattattagcagaatctgtaggaattcccttgtccaggcctgattttttacgttcgtcctcagagagggagaggtattgtttcaggtctttgataggtgctcctacactggctccggttacaaagcttttaatttctttatcgtccaggcccagtttgtactgcgtgttcagatcttctatcagcttctttcttttgggctgaccatccatgctgaaaaacactctgccatccttatccactgtgaataacaacacatcggaatcaggtaaaagggtggtgtttatagaggatggggtaactactgttaccggttcatccggtttaaacttagtcgccagcataaagaaagttaacagcaggaaagccacatcacacattgctgtcatgtcaatggccgtgcttttccttggcattttaactttaggcatctttactctgttttatggtttactttaaatagattcaaaaccgctcaaattccacaaaataatctcagattatttgtggtttgctgcgaagctctgagttaaagtaaagccagattcgtcaatagcgtaagtgatgctatcaatattggtagtaaagtagttgtacattacgatcgcaatagcggatgtaccgatacccagtgcggtgttaatcaacgcctcagagatacctaacgccagctgtgcagaatccggagcaccaccagaagacattgcagagaacgccttgatcatacccaatactgtaccgaacagacccaacagggttgctacagacgcaatggtagacaggaacaccaggttcttttccatcattggcagttccagtgcagtggtttcttcaatttcatttttgatggtcaggatcttctgttctgtatccagatcagcattggtaaccatttctttgtactttttcagaccagctttcagtacatttcctacagagcctttctgtttgtcacactcagccagtgctgcgtctacatttttgttagccaggtggtactgtactttacgtaccagctcagaaccgctgaatttaccttttgcttttgacaggtacaggaagcgctcgatcacgaaagtcagacacaccagtaatacggaaatcaataccggtactaccaatcctcctttgtaaacagtaccaaaccatttaccgatacctgaatctataggatgtccatcgggattattaccctggaaattggctggattacctaatacaaaaaagaaaaacaggaatcctatcactaagcagataggcacagccaacgtcgcgaacaggttggatgactttttaggttgatgagaagaagccttagctgtagctgcagtcacagttgttttagtctcagccatgttgattgaaattttagtgttaaaaattaaactattgtttgttagaagtttctgtccctttagaatgcccctcagcacccaatttactgttttaatcagtgattcgcaaagttatacggttggtccaaaaaaacaagtgcagcccaaaaaaacccacaaaaattaaccttcacacgtaaaagccccatcacagggcttttagaccactcatttttttagagcaaacacttacataagcgaataaaccaatattgcagttctcacaactgattgttactgtcccaattcttgaaatcgtttgatttttttcaaagttggacgcacaatttaagaaaaaattcaaatgttccaacagaaatctcacaattctgccaacttatttatttccgcgccagtaaacactttcaggccacgctaatagcatttagcaatacaacatccatattttgcccgccccataacttgaaattcaatgccgcagcggcaatcaacttctcccctgctatctctgccatatgaaattattatttgctataataataaatacttacataaaaaaagttgccaccgcaactattgtttcaacgcctaccattcaattttgcttctttttttccattcctacagtcattactgcgcttatggattttcctgataagttaatacttaaaatacttacttgcaaaggtttttaaaaaaacataacaactaatcaaaaaccaatttattaaatcgtaatgatcaaaccaattcatcacaaactgataatagccatggcaggcgcactttgcctgggtactacagtttatcaacctgccagcgcacagcgaaaaaaacaatcgcgtaacgccaccccaactactcctgctcctgctaaagattctaccgggaaacctcccatgatcaagccaggaccaaagccaggacccaaaccctttgccgaagtaattactgataaagcccaggctgattccggcctgtttaacatctacaaactggatgaccgcttcttttttgaaatccctgattccctgctcggaagagacgtactggtggtaaacaggatctcaaaatcagctgcaggtctccgcgccatgatgatgggcttcagtggcgatatcatcggcgaaaatgtgatccgctttgaaaaaggccccaacaatcgcatcttccttaaaaatatctcctacgccgacgtttcaaaagattctacccaacctatgttcacctctgtgagcaactccaacctgcaacccatcgttgcagcgtttgacgtaaaggcggcatctaaaaacgggaaaggtacagttatcgacctcacagaatacatcagcggggataacgagatcctgttcttcgacggccagattaaaaacatgctcaaaatcggtggtgttcagcctgataaatcttacatctctgatgtgaaatcctatccgatgaataccgaaatcaaaaccgtaaaaacatacagcaaatccggcggaccgggtggcccgggtatgcccccatcccagggcggcaatgctaccgtggagttaaacagctctatggtgttgcttcccgcagtgcccatgcaaccacgctattttgatccccgcgtaggctacttcaccaccagcgtaaccgacttcgatgcggatccgcaaggcgtgaaaagactccagatgatcacccgctggcgcctggaaccaaaacctgaagacatggagaaatataaacgcggtgaactggtggaaccagttaaacccatcgtgttctatattgaccctgcaacgcccgtaaaatggcgtaaatacctgatcatgggtgtgaacgactggcagtctgccttcgaacaggcgggctttaaaaacgctattattgcgaaaatggcgcctactccccaggaagattccacctggtctattgaagatgccagattctctgctatcgtttacaaaccttcagatgtacccaatgcgagcggtcctcacgtacacgatccccgctccggtgaaattatcgaaagtcatatcaactggtaccacaacgtgatgcatttgctgcgtaactggtattttgtacaggcgtctcccaacgatccccgcgcccgtaacatgcagttcagcgatgaactgatgggtgaactgatccgctttgtatcttcccacgaagtgggccatacactcggtttgcgccataacttcggctccagctccacttacccggttgaaaaactgcgtgataaggaatgggtgaaaaagaacggccatgcagcgtctatcatggactacgcccgttttaactacatagcgcaacctggcgacggcatcaccggcgctgatctctatccccgcattaactactacgataaatgggcaatcgaatggggctataaactgctgccacaggccaaatcaccggaagcagaaacgcctatcctcaataaaatgacggtggaaaagctgaaggataagaaattctggttcggtacagaaatgaacccggacgatccaagatcccaaaacgaagatctgggcgacaatgccatgattgccagtacatacggcataaaaaacctccagtatattatgcctaacctccttagctggacaaaggtggataacgaaggttatgcaaacctgtctgaattgtataaagaagtagccggtcagtttagccgttacatgggtcatgtggctaaaaacgtaggtggtatttacgaaacaccaaaaaccgtagaacaagccggtggggtgtatgaatacgtacccgaagcaacccagaaagaagcgatacagttcctgaacaagcaactgtttaccactccgaagtggctgattaaccaggatttactgagccgcataggcagcgatggcgtttccctgattaattcccgccaaacacctgttctggacaggctgatgagtaccaataccatcaataaactgattgccggtgaagctgcactgggagcaaaggcttattcacctgttgatatgctgaacgatctgaaaaaatccatcttctcagaactttatacacatcaaccgatagacgtataccgcagaaacctgcaacgcgactatgtggataacctttctgacctggtagccccagctgcccccgccaatccaatgatgggtggttatgcacctccgagtgctgccagatcagatgctgcaggcattggccgtgcccagctgaccgccctgagaacagagctgcgtgctgctgcaggcagtggcgacagcatgacccgcaatcatctccaggagctgattgcccgtatcaataaggcactggatccgaaataacgaatgcgcatacacgaaaatatctgcacccttcccggtaactccaggaagggtgccttcgttttatagatgttcaaaagcctataaattattgcggaaaatgcttaatatcgctgcattattaacttagaagcctcaaaagtgaaagatcggactaacaaaatcacgatatacgatatcgcgcataagctgaatctgtcggcatctactgtttcacgtgcattgcaaaacaatccgctcattaacctggaaacacgtgaaaaagtacaagccgcagctacagagatgggctacgtacctaactggattgcttccagtttgcgcaagaaacggtcgaacattctcggccttatcgtaccccgaacttccatgtactttcagagtacggctatcagcggtattcagcatgaggcacataaatatggattcagcattgtaattggccagtcggatgaaaccgtggcgatggagaaggaattagtacatactttttattctcttcgtgtagatggattactggcagttgcttccatgttcaccaccaattttgatcatttcagtccgtttatcaagaacaatattccactggtattttatgaccgtgtgcctaccgattttcagggctacactattaccggagatgatttcagaggcggtttcctggccaccgaacacctgatcaaacaaggttgcaaacgtattgcccacttctccggagtgctcacctgtaacctttaccagcaaaggctttcaggatacaaagaggcattggcacaatataatattcctttcgacgaagagctggtttatatccatgatctgacgatggactcggcgactattgctgcacaacaattgtttgatgcacagaaaatgcccgatggtatgtttgcagccaatgacagttcagcggtggcttttatccgtgaagcgaggaacaggaatattgcggttcccgggcaaatcaaagtagtgggatattccaatgatctgtcttcccgtattatttctccttctttaactaccattgaacaatcggggtataatatggggcagaaagccgtggaaacaatcgttcagctgatcaaccacgaagagacagtgaaagtgacaaaaaattacgtattcccggtggagttaatcaagcgggaatctaccggaatataattttaatactaaaactgataacctacaacttttatgaaatcttccatttatgtagcattattatgtactgccgcagttgccgtatcctcttgtaacaagcgtatttatgtgcctaaccaggtaaatgtgccgttgttgaaagagaagtatgaattcaaaggcagcgttacacctaccaatctgcagaccgcttttgcaattactgataatatagccatcatggccaatggccagtacctgtgggggtttaattatgccgatccgaccaatagttacgatgaagacggcttattccgggataacaatacccgcggaggattgatagaaggggccgttggcttcttcaagcctattggcgtcagtaaaaaagcagtttttgatgtatatgcgggttatggcagcggcaatttcaaaacattgactggcaactacaaatccgataatgatggtactggtaacattaacctgaacgactatgtcataaaaaaccgtttcagcaaagtatttatacaaccaagcttcgggctttcccatcgtgtggtggaagcagccttcagcagtcgcttttccctgataaacttttacgacagtaatattggcgtaaaggcatttgaaaataatgaacaggagcagacgaaatttatgcgtatccacgacaaatccgtggtgttctatgagccggcattcacagtgcgggtgggttataaatacgtaaagtttcaggcacagttacagttttcaacaccgataaacagtaatagtttttacgacgataccgacgaccataatttcaatgagtatttccagccggtgaattttaatatgggtgttgcgataaatctggcgaagtggtataatcgtacgaatagataagtgattccaggaagtgatataaaaaagaaagccttagtgtttgaaacactaaggctttcttttaataagtatggcagctacctactctcccgcatgatattgcagtaccatcggccatgaggggcttaacttctctgttcggaatgggaagaggtgaacaccctcggcataaccaccataagatctttagcctgtttgagcaggcaattatatgatgaagttctgaacgaactgtgaatcgtatttgagtctcttaaagagataacctataacagcttttctggatagaatttaaataaagaagcctcggtgtttgtacaccaaggcttctcttaataagtatggcagctacctactctcccgcatgatattgcagtaccatcggccatgaggggcttaacttctctgttcggaatgggaagaggtgaacaccctcggcataacc

SEQ ID NO: 11 - DNA, 288237 bp, Chitinophaga pinensis
  source 1..288237: mol_type = genomic DNA
tgctaaagcaagctgacattaactatttattctcttaaaaaacacctgatcatcataatgattattaggccatcttttggctaaaacaaagaagctgtctcaattaattatgagacagcttctttttattttttcttcgctcgtttccgaagctcattcacctgtgcagtgatggtttcaaagaggatatcggtaagccgttttacagccggggagggcgtttttttacggatgagcataaacacggcaacatcaggtagtgctggcaaaccactggtctttgtgagtgctacacagcctgcaggcagtcccatttctgtgcggatggtgatacccaatccggcctgggctgcagcccacatccctgctacgctgctgctggtgagcgccggccgccacgtacgtttagctttttccagcgctgccagccccgcactgcggaacaggcatggcgcttcaaacagcagcagcggcaacggccgcagctgcgcgatgtgcttttgcgtgttaccaatccatcgtataggtacatgccctatcaggatggcatcatctggtatatcttttccaaaggaaagtaccacatccagtttaccgcgttgcagctgctgttgcagcaccgcctgccggtcgatcgtcacctccacttccatgtgcggatgtacagcggcaaaccgtgccagcaccaccggaagaccactttccgcaaagtctgccggcaatcccagttttaccttccctgctatatgcgtggccgttagggcattgatcgcctgctggttaacatccagcagttgccgggcatatcccagcaatatttcgccggcaggagtgagctgccagcctcgtccctgcctgataaataactgttggccggtaatttcctccagccgctgcatctgcaaacttacagccgattgcgacctcgctacctggtcggccgcccgcgcaaaactatccagatccactgccagcacaaaagtacggagcaggtccatctccaggaggtctgttatcatagtttagttttattaaagtataatgttaaatgtttcaatattgcaaatgtataaaaccatagtaaatttgattcatgaaaaacaaattactgatcatgagcatgctaactaccggggcagcggccgcacaaatgccaactgcccgcaaaacattgttgcagcaggacctgactggcctgactgtagaaacagtaaagatggaccaggccactttggcgccggagcagcctactatcatcataaataaataagccatgccttttgtacagatctacctgggaaaacatctttcccaacaaaataaaaaagatatttccctcgctgttcatcagagtctcgtggatatcttcagtattcctgtaacggattatttccaggtgatccatgccatggaacccggcgatattctttacccggaaagctactttgaggtgccgcacaccgaaaacctgctctttatccgtatcaccgccagggccggcagaacaccggatatgaaacaggcgctgtatgaaaagatagccagccgtatagcagccgctacaccagtaagtgcagatgacgttatcatcatcttcgtggaaaatgacctggcggattggtctttcggccgcggtattgcgcagatggtgaagaaatagcaatatcgccggttttaatttcctgcaaccatttaaccggcaaagcaaatttatcggtaaattgggcgcaggtatggacactgttacaacagaaaaacaattgccgcgctggcagcttttcctgctttccttcaaagaagcatacaaggcactgcaggccagcgatccgctgcggatggcgggtgccactgccttttttaccacttttgccttaccagctatcctgatcattattatccagttgttacgtattattttccggatacaacatgccggtcagcgtcttatgatccagctggaaggaatgtttggaaaggaaacaaccgaagccatcctgggaacactgagagccttccggagcattgcgcagaactggatcatcgccattgccggctttattttcctgttgtttgtggccactacgctcttcaaaattattaaaggctcgctgaatgaactgtggaaaataagattgatccataaaagcagttttggagaaattatggtatcccggctgaaagcagtattggtgatcgttttcgcaggagttttgtttatcatcgacctggtggcggaaactgcgcgcatctttcttggaaagtatatagacctgtatctgcctgccctgggcagttattataacagcacgctcaactatgttatttctgtgatcattgttaccatctggtttttcctggtgttccatttcctgccggacggccgcccgcgatggagggtagggattaccggcgcactggtaaccagcatcctgtttaacatcgggaaaatggtgttgaaagtaatgctcacctacagcagtattaacagcatttatggggcttctgcgtctactgtgctggtgctgttgtttatgttttattcttccctgatcttttatttcggcgcctgctttacctatgcctggggcgctcttaccggcagacccgtggagccattgcattacgccggcaggtttgaaattactcctgcggaagactaatctcctcaatggataacaaagcaccctgaatagataaataagtattataaaaatgatcttttatagagatagatttgctgattgtataaagtaatttttaagcagaattccacctatgggcgacacaatttctttaaaggaaaaaatagggtatggctttggagatatggcttcttccatgttctggaagttgtttggtatgtacctgttgtttttttatacagatgtgatgggcatcgctgctgctgctgtaggcactatgttcctgattacccgtatatgggatactttctttgacccggtagtaggtactttgtctgacagaacccattccaggtgggggaagttcagaccctacattttatatatggcagtgccttttggcgttataggcgtacttactttcactacgccggattacggcgccaccggcaaactggtatacgcttacattacctattccgccatgatgatgatctattccctgattaacgtgccttacgcatcgttactgggagtgatctctgccgacggaaaggaaaggaatacgctggcctctttcaggatggcctttgcttttggtggcagtcttattgcgctggcgttgatagagccgctggtaaatttttttagtaaagccggaggagaaaataacctgcaaatgggctggcagctgggcgtggcagtgatcgccgtaatttgtgtgatcttatttctgctatgctttgcctgggtaaaagaaagagtgcagcctataaaagaggagcagtcgtcactgaaagaagacgtaaaggatctctggaaaaataagccctggtggatattgctgggagcgggtattgccgcactgatcttcaactctatccgcgacggcgccaccctgtactatttcaaatattatatacagaatgcgcaggcttttaaactgggcagtgtcagcattacctattccacgctgtaccttgtactaggccaggcggcaaatatagcaggcgtaatcctggcttctcccattggtaataaaataggtaagaagaatacttacctgggcgctatgctgatagcttctatcctgagtatcgggttttactggctgggccgcggacaactcaccctgatctttatattccagttcctgattagtatttgcgcaggtattattttcccattgttatggtcgatgtacgcagatatcgcggactattccgagtggaaaaacggtcgccgtgccactggcctgatcttctcttcctcgtcgatgtcgcagaagtttggctggacgatcggcggagcgctcaccggctggctgctgggcgcctttggttttaaagccaacgaagtacaggccgatgctgcacaaaacggcatactgttaatgcttagttttttaccggccatcgggtcggtattgtctatcatatttatcgccatgtacccgctctctgaagagcgcatcgctactatctctgctgaactggaacaaagaaggaaataatgcaacaggaattaaagacatcactggaaaaagaacttaccgccatcctggactactggatgaaatatacgccggacgaaacatatggcggcttccttggcaagctgggaaatgataatgttcccataccgggagcggcaaagggtgcggtattaaatgcccgcatcctgtggacatttgcagccgcctacaacactactcgcaacccggcctacctggcaatagcagatcgtgcataccggtattttaatacacactttattgatcctgcttacgggggcgtatactggacggtagactataccggccagccggccgaaacaaagaaacaggtatatgccattgcatttgccctttacgcatacagtgaatactacaaagcggcgccacacccggaggtactgtctaccgccatttccctgtacaacaacatagaacagcacagttatgatccggttcatgatggttactttgaagcattcacacgggagtggcaggaaatagtggatctgcgtctcagtgcaaaagatgccaatgaaaagaaaaccatgaatacccacctgcatgtagtggaagcgtatgcgaatctatacaccgtttggccggacgagaaactacgtatacaaatacaacggttattgcaggtatttcacgataagatcatcgataaaaaaagcgggcatctgcatttgttttttgatgaacaatggcaggtaaaaggtaatcatgtatcatacggacatgacattgaagccagctggctcctgctggaagcagcagaaattatcggcgatcccacactcactgaacaataccgcaaactggccctggtgatcaccaatgccaccctgcagggcggcatagataaggatggtggcctctggtacgaatatgagacctcccggcgccacatgaatacagagaaacactggtggccacaagccgaagcgctggtgggctttatcaacgcctggcaactgcaaccacatggccgttacctgcaacacgcacaaaacacctggaactttataacgcaacacatcatcgacaaaaccaacggcgaatggttctggggcgtgtacgcggattacagcatcatcccggaagacaaagccggactatggaaatgcccttaccacaatgcgcgggcgtgcatggaaggaataaagcggttatgcgaaggttgtcttggctcaggattacgctgattatactgattaccttgattttactttttgggattttataaaggattttagttgattttgggagatataagcgaaaatatccgcttatatctcccaaaatcctttacaaaatccaaaaagtaaaatcaaggtaatcagtataatcagcgtaatcctgagccaagacaaccttcgcacaccaatacagaattcgcattttttaatttgtaattagcaattactccttataggtttccccagcataactattttatatatcttgaagcatatgaactgcaagatatattccacgctgcaagctgcatttttattgggcgcccttacgttatcggcgcaatctgatgtaacggtacggttcagtgaaccagcccggcatttcacggcatctgccccgttgggaaatgggcgtatgggagctatggtatttggcaacaccaacagggaacggattgtattaaacgaaatatcgatgtgggctggcggtgtgcaggatgccgacagcaaagaagcaggcaattacctgccacagataaggacattactgctggaagggaaaaatattgaagcgcagaaaatgctgcagcaatattttgtgtgcaaaggccccggaagcagtggtggcgccaatgtgaagtttggttgctatcaaaccctgggcgacctttttatccagtggaaagataccacgtcggcggtaagcaactaccagcggcaactaaggctggatagcgccatcagcgccgtaagctgggaaaagaacggggttacttttaaggaagaagtactggtatcagctccagggcaggtggccgtagtacgcctcagcgccagcaaacctggcagtctttctttcagtaccggcttataccggaaggaacgcgccgccctgaaagtggtaaacggcaacctggaaatgagcggtacgctcaatggcggcaacaacgaccccggtgttcagtatgcagccgtactgaaagtaatacccaaaggcggtacccgtacacaaagcaatgaccagatcatcattaccggcgctactgaatgtttattactggtagccgcccgtaccaatatgaactggccggaggtggaaacaccaggtccggccccgctgccgaaaacgctggcagatatcaataaagccaccacatcttcctggcaggcgttattacagtcgcacgtaaaggactatacgtcgttctttaaccgttgtcgtatatcctttaccgataacagcaatgatgaggtgaagaccctcgctaccatcgaccggctgcaacgcctgcacgatggtaaaaaggacgcttccctggcctccctgtattttaatttcggacggtacctgctgatcagctcctcccgcaatggcggcatgccggccaacttacaggggctttgggcagaagaataccagacaccatggaacgccgattatcatctcaacattaatgtacagatgaactattggccggcagaagtaacaaacctgtcggattgccaccagccactgtttacactggccaggcaaatggcgaaatacggtcagcgcaccgcccgcacctactataaagcagatggctgggtggcgcatgtgatcaacaacccatggggctttacttctcccggtgaaggggccgactggggttctacgttaaccggtggcgcctgggtagctacccatctctggaaacattaccagtataccaacgataaaaaattcctgaaagaaatatacccggtactgaaaggcgccgctgttttttataaagatatcctgatcacagaaccatcgcatcagtggctggtgactgcgccatccaactcgccggaaaatgcgtacatcctgcccaacgggcagcagggacaaacctgcatgggaccaaccatggatatgcagatcggaagggatttactcaaagccaaccaggaagcggcccgcatcctgcaaacggataaaggctgggcagatacgctgcagggagtactggccaaactggcgccaaaccaggtgagccccagtaccggcggtgtgcaggaatggctggaagattataaagaagcagatccgcatcaccggcacgtatcaccattgtatggtttgtatccgtatgacgaaattacaccgtgggatacaccggaattagctgcggcagcagaaaaaacactgcttagaagaggcgatggtggcaccggctggtcgcgcgcctggaaaattgctttctgggcccgcttaggcaacggtaatcacgcctataccatgttgcaggaattattggcgcctgccgccgctaccagcgaaatcagtatgcgctccggggcaggtacttacgccaacctgttctgctcacatccgccgttccagattgatggtaacttaggcgccgtggccggtatcgcggaaatgctgctgcaaagccatgggggcgataacgtaatccgcctgctacccgccctgccggataaggaggaatttgctgccggccaggtaaagggactttgcgctatcaatggttttgtagtggatttcagctggaaaaataaaacagtgcaggaactcaacctgctctccaataccggtgcggagtgccgcctgttgctgccggaaagcgctgtggtaaaggatcgaagcggagcagtgataccgcatcagtatagtaacggcgtattgcgcttcgctacaaagaaaggaatgaagtatcatatagcagtataaagtggcggagttttgtcttactcagtctaacctgagtaagacaaaaaaatcgcatctttacctttcataacaacccatatggaagatctgaaacaagtggctgcaaaggcagcgttggattatataaaacccggcaataccatcgggctgggtgcaggcagtaccattgcacacctggtgaactacctgaaaacggaggaaacgttatttaaaagcattaccacggttacctcttcctttaacacacagcaactactgcaggaacacggattcaacactaaacaaccaggagacgtatcccggctggatatttattttgacggatgcgatcagtttgatcatcagctgaatgccctgaagagcggtggtggtattcatacacgggaaaaattgctggccgcaatggcagataaattcatccttatcggcgatggctccaaatacgtagcgcagttgtacactacttttcccgtagtgatagaagtgatcccggaagcagttccctttgtgctgaagcagctgaagaaaatattttcactagctaacccggtgatccggcttagtaataaaaaagatggggcagtgattaccgagaatggcaacatgcttgttgatatctggttccgttccttcccgccattagacagcctcaattatcgtttaaaggacattccgggtattctcgaaacatcgcttttctataatatggcgcatgctgccatcatagcgggaaagaagggagtagaaattattcagaaagaccctgcttacctgatctgaaactctttcgtacctgcggttacatgataacgtaaccctttaccggtgttttctgtaattaccggtttatcgttttcatatattttttgtgtgggtgagatgtgaaaaaagatgtctgcaccggcatttgcgggcactgtcacacggtaggtgatggccgtaccgtttcttttccaggaagaaaccacggttccgtaagggctgtcatgacttccttcaaaatgatccaggccttctacgaaattaggagataacaggatgtttttaaacccgggcgcattttcatccggcttaataccagcgagtcccttgtacagccaggcgcctatttcaccaaacatgatgtgattgcgcgaaagatctgaagaggcattgatatcccagttttcgaagagggtagtagcgccgttcatgatccaccagccccacgatggaaaagtgcgttgcgcggccagtttccaggctacatctgcatagccgttttcgctcagcgcattcaggatacttttggtgcccagcaaacccacgtcgaggtgaaagttatctgcggccactctctttgcgagattggcggctaccttgcttttcatggcatcgggcactaatccccagtacagggcaacgctttgctctgtttgtacgccttctccatagataccggtttcacggttcaggtatttggcattaaaagcggttttgatcttctctgccagtgcgctgtatttactatggtctgatgttctgccaaacaatttcgccgctttggccaggatcagcgcgtcggcatagtagtaagccgaggatgtgaattccacgggtgattttgattttaccggcacccagtcgccgaggccccaggtggttagtccggacggactaatcgccgtgatccggtccacataacggcgcatgttatcataggaggccgagagcagtgtagtatctccgtaaaacaggtagatgttccacggaatgatggcgatggtgctggtccagtccgggccattgccccattcatatccccagccgccggtgggaatgatagagggcagcaccccgttgggctgctgctcgtcgcggtggtctgccagccatttttcatagatggtgatgccatcgtaactatacaacccggtttcaatggcaatctgtgcatctcctgtccagccgttcttttcgcgctgcgggcaatccgttggataaccgaacaggttggagagataggcattattggtggccgtgaataatttattgatcatggtatcggagccatgaatgtggcctgccggaggtacattgctgtgcatgaaatagccggtgagactttccttattgagctgtaccggtttactgctggtcacttccacatattgaaagcctttatagttgaagcggggcataaaggtttcttctcctttgccgccgaggataaaaatatctgtctggaaaggatcggtgtcatctgtagggcgataatgcactataatattggagaggtctacaaatccttttttatccagttgctcgccgtgcttcagcttaatgatagtaccggctgcaccgcttacgcggatcttacttacgccggcaatatttctgcccaggtcatatatccaggtgctgtcgttgggatgggtaacggcggcagcaggaatttcctccacattttcgatgggatataattgttgcgatacaatgttttgggaaggcgcggcacggtaaataacctctttccatttgttgtcgtcgaaattaacggtgttccatcctggttgttctttgcgggcgtcataatgttctgcggtataaatgctgttaaatacgataggtcccaatgccgttttccagtctttcccagaggtaacagtttccacggtgccatcagtataggttacccgcagatcgaggcagaatgccggccggccgcgccacggcgcttcatgaaagttccatacggcggtggactggtgattataccagccattaccaagcattacgccgatggcgtttttaccggattgcagcagggaggtaacatcgtaggtaacgtatagcgtgcggcgatcgaagcgggtgtacatgggatcgaggcgatggttgcctgctttttccccgttgatatacagttcatacaggcctgctacggcgatataggcgcgggcagactttatggatttcgtagcggtgaaaatttttctgaagttggcggcgggtttcaggcgggtgtcctcaccgtcgctgatccaggcgcctttccagttgctttgctgcaacatgcctgtttcaaaccaggagcggcggggagtggattttacgccgtctttatcccatatttccacgctccagtagtagcgggtaaatggttgcagcggtttcccggagtagctggtaagtatatctgcgcggttaattttgccggaagtccacaacgggtgggtgtccagggtcagtgaatcggtggatatgcggatctggtaggccgtttggcgcgcgcccgggcgcgcatcttccagttgccacgacagccgcggatgagcagcgtctacaccgagcggcattaccaggtgttcgcatttcagatgggaagcttcacaggtagtggcttttgcaccggcgtacaccgttgatactgcacaccataaaattaaaagatacagaaatagtttccggaatgttgaatacatgctaaacgcttgattattttgccaacaagataaagtaagccgtacttttttttaattgttttatgtaaatggaaaaaagatagatcgatctgtctattttgtactatctttgttccatgaagaagaaaacaggagatccaaagcagcgtttgctggatactgccactgcacttttctataaccagggatatcacgccacaggcattaaccaggtgattgaggaagctggtgtggcgagagccagtttgtacctgcattatgaatcgaaggaatctttgctcctggcgtttttacatcagcgtcatatcgactggatggccgggctgaaaagctttacagacgaggccggcaagccgaaggataaaattgcggcagcgtttgacttcctgtttgataataatgaaagggagcatttcaggggctgcgcctttttgaatatcctgtcggaaactacggagaaggacacagcggtgttgacggtcatacaggatcataaaaaagatctgcgtgcttttttaggtgagatcctcaccaatgagaagcaattggtaaaggatcatgtatacctgttgtttgaatccgcgatcgtggaaagtcagctttaccggaaccagtggccggtgcaggaagcgaggaaaatggcattgggattgttgtaatgcggaccacgtgcatatttcatctctataaatttaaagatgcccggcatcttttttttaatcttttaaaatagacagatcgatctatctgtaatattatactgatcacttttaaacaattatctcatggaacagaaattcccccttcctccatttacgcatgaaaccgccctgcaaaaagtgcagatggcagaagacgcctggaacagccgtgatccgcaaaaggtatcactggtatacacgcccgacaccgtatggcgcaaccgcgaccagtttatcaacggccgggaagaagtagtggcctttcttacaaagaaatggcagcgggagctggactaccgcctgaaaaaagaactctggagctttacagataaccacattgccgtatgctttgagtatgaatggcatgatcatgccggtaactggttccggtcgtacggcaatgagctgtgggagtttaatgccgatggattcatgcaacgcaggctggctgccataaacgatgtgcctattaaaagcagcgaacggaaattccgtgaaccggaagatttaatactggcctgttaaagagatgtgattattatggttacccgggaaatcataataatcactactaatcatagtgtgaattttgtaacttcgctgaatgaacaaaacagaaacactccaggagttttacgaacataagttccaggcagtacctgataagttacagcaggatataggtcactttaatgtattccggctggaggactgcattgtagacggcgcttcaacggtgaaatacagccgccgtgacttttacaaggtaagcctgctaaggggagccaacctttatcactatgcagataaaaccattgaagtaaaaggcagcaccctgattttctttaacccgcaggtcccttacggatgggagcccctgacgaacgacatcagcggctatttctgcatattccgggagtccttttttacaggcgccacccgtggcaacatccacgacctgcccatgatgatgccggggggtattccttcttatatactgacaaaggcccaggacaaagaagtatcacagctctttaaaaagatgctcacagaaatcaatacggactacgtttataaatacgacctgctgcgtagctaccttacagaaatcatccactacgccttaaagatgcagccctccgaaaccctgtaccagcacgcagatgcgaagtcgcgtatcacggcggtatttaccgacctgctggagcggcaattccctattgaatcgccggcacagcggtttgcattgcgttctgccaacgatttcgcaaaacagttgtctgtgcacgtgaatcacctgaaccgggccatccgcgaaaccacaggaaaaaccaccacggcgcacattgcagagcgcgtaacggcagaagcaaaggctttattaaagcatactaactggaatgtggcagaaatcagctatgcccttggatttgaggaacctgctcacttcagcaactttttcaaaaaacaaaccagtatccctcccggcgctttccgcgttgtttgatttttgcaattattggtttgaatagcgtaacacgcagcagcattccctgttctacttttgtgttaacaaaaaacacaagatcatggacaacaaaaaagtatggtttgtaaccggcgcctccaaaggattaggccgctccctcgtaaaacaattattaaacaaaggatataaagtagccgccacctcacgtagtatcgacgacctgcgcaaaattgcaacggacgcggatttcctgcccctggccgttgaccttaataatgaaaatagcatacaggcagcagtaaaggaaactatcagccgtttcggtcgcatcgacgtactggtgaacaacgccgggtacggacaattaggcagcattgaagagctgtcggatgcagaatcacgaagcaattttgatgtgaatgtatttggcctcctgaatgtaacccgcagtatcctgccacaaatgagaacgcaacagtccgggcacatcatcaacatttcctctatcgctggtcttaccggtagcttccccggcttcggtatctattgcgctaccaagttcgcggtaaacggtttatctgaatcgttggcggttgaagtgaaaccttttggcatctctgtaaccatcgtttcccctggttatttcagaaccgatttcctctcttccggctccctgggcctgcctgtgaaccaactggccgcatacgagtcggttcgtgctgcccagcacgcgcatcaggaggagattaacggcaaccagccaggtgatcccgaaaaagcagtagccgccattatcgacgtagccgctgcagacaatgcaccgctgcatctcttcctcggagaagacgcctacaatctcgcgtatcaaaaaatagccacgttggaagctgacctggagcagtggaaggatgtgacggtgggaacggcgattgtgtaggatggatcgcagcgtattttgtcttggctcaggattacgctgattatactgattaactggatttttacttttttgattttataaaggattaagggagatagcagcggatattcgctcttatctcccttaattattattttaagaaaatcaaaaaaatctaaaaaaatccaaaagtaaaaatccagttaatcagtataatcagcgtaatcctgagccaagacaaaatacgctgcgatcccccgcactaagtcaacgtgacattaaagtccgcccccagctcgagcctcccttcgcgctcctccgtgctgccaggaacctggagcccttttattttggcggttttgcctttggtcagcaggtccgcaatgtgtttgtcggttaattttttgcccagtatttcgaacggaagtttgaagccgcattctttaaaattggcgcagccataggcggtgttgccttttttgagcggatgcgttttgcatttcgggcattgcatttccgctatcactacggcctttttgggcttaggttcctttttgggtttctctttttcttccggtacaggcggcggatcaggggcaatggtgatgaacttgtagctggatgtttttacttctttggtaaggtcaactaccatctggatcagttcatctttgaaggtgtccatcgcgtactcgcctttttctatgaggcgtagtttacgttcccactgaccggttagttcggcgcttttcagcagctctgtttgtatggtgtcaatgagatccatgccggtttgggtggcatagatatttttctttttcttctcgatatattttctgcggaacagggtttcgatgatattggcgcgggtggaaggccggccgatgccattgtctttcagcaattccctcatttcctcatcatctacctgcttgccggcagtttccattgctcgcagcaaggtcgcttctgtaaaggctttgggcggagaggttttgccctggtggatgcgtggggtatgtggcccgctttcacccacttcaaagtgagggagtattttctcttcttcttccccttcctttttctcttttacatcgttggcatatacttctttccatcccggttctataatctgtttaccggttactttgaaaggtacctgtcctactttaccgagtacggtggtattggagatcttacattccgggtagaaagcggcaataaagcggcgggctaccaggtcgtagatccttttttcttccaggggaagaccaccgggatgctgaccggtcggtatgatggcatggtgatctgttacttttttatcgtcgaaaacagtctttagctttgggataggagcagccagcagcggtgcggtgagcgcgttgtagggcgtcatatcctgcaggataccggcaattttcgggtgcaggtcttccgagagataagtggtatccaccctggggtaggtagtcagctttttctcgtaaaggttctgaatatatttgagcgtatcatctgcagagaagccgaattttttattggcttccacctgcagggcggtgaggtcaaacaggcgcgggttgccttcttttccgtctttcttttcgaaggaagtcacctcaaacgggtgttctttgagataggcgagccctttggcggctttatccggtgttttcaggcggtcgatggccgcggtgaattctgtttcccggtaaatggttttcagttcccagtagtcttccgacacaaaggcattgatttccttttgccgctgcacaatcatggccagggtaggtgtttgcacccttccgatggacagtaccaccttaccctgcgcgaattttttagtgaacagccgggtggcgttcatgcccaggagccagtcgccgatagcgcgtgcgctgcctgcggcgtacaggttgttatattgctcggatgctttcaggttttgaaagccatcgcggatagcctccactgtcagagatgaaatccagagccttttaatgggggcggcgcatttcgctttcagcagcacccagcgctggattagttctccttcctgcccggcatccccgcaatttatcacttcttcacacgcctgcaccaggctttctataattttaaactgtttttgtacacctgaattttcaattagtttgataccgaagctgggagggatcatgggcagatcttccagtcgccagaacttccattgctcgtaataatcgtgcggctccttgagggtacagaaatgtccgaaagtccaggttacctggtagccattgccctcatagtagccatctttgcgttgtttcgcaccgatcacttctgcaatatcccttgccacgcttggtttttcagcaatgcaaactttcatattcgtttaaaattgggtaacaaatgtcggataaaaagttgtaaatgaaagaaggttaaaatacgccaaaaatcttaaaataatcaagtacacactttaacttttagtctgcaaaaatacctgttattttaaggaagatttgaaactaacatcttttccttatgcgctttcctgcccttgtattatcgtgtgccttatcgcttcccgctgtagcacaataccctgcatcttttgacggaagcttcgaaagtaaaaaaccgggaggcgctttgcctgacgggtgggtcgactggggcggtaaataccgactggccgtcgacgacagcatctattacgaaggacatggagcattgcgcattacaccatttgaaaaaagagggatgaatgattatggttgtaccgtgatacgtataccggttacttttgccgggaaaaccatttcgctcaaaggctacctgaagctggatgcagttaccgatggctatgccggcctgtttatgcgggtagacgataaatcgggtgccgtatacaaaatggataatatgcagaagcggcggctgcagggaactaccggctggcagcaatacaacattaccctttccctcccgtccggtggcggcacagtatacgccggcgccattaatcacagcaatggtaacgtatgggcggataacctggaagtattgattgatggcaaaccattgaaggaagcaccaccgctccacgtgtataaagccgacagtgatcatgcgtttgacaaaggctcgggtatcagtatttccagtcttaccccgctgcaggcaacacacctggaagtacttggaaaggtttggggcttcctgaaatattatcatcctgcgataatggccggggagtacaactgggactatgaattattccggatcttaccggcagtattgagcagtaccagcgaaacggccaggaatgaggtcctgcttcggtggaccaaccagcttacggcgccgcaggagttccggcgtatgcacaccggtaaaatggtgattaaattcacccctgatctcgactggatttcagatgagaaaacattaggtacggcattatcggcagccctgaagacagtggccgccatgaaccgcgatgatgccagttattacctcggactggagcctgctggtaatccggcatttaaaaatgagcaggcctataacaccatggcctatcctgacgccggtttccgcctgctggcattataccgctactggaatatcatacagtattggtttccttataagcacctgatcaccgaaggctggaataataaactggcggagtatataccggcaatgattaacgcggcagatactgcggcataccaaactgcgctgctgcggctgattgcaggtatccacgattcgcatgccggtatatatggcgccaatgtggtgattcgcaatacagacaggtttagaacgttgccactgcgggcacggtttgtggaaaacaaggcggtgctggtgaaagtgggtgatgaaaaatacggattgcaggttggtgatgtgattaccgctgttaataaagagccggtgacggctatggtacaacgattattgccgcttgcttctgcttccaactatgccacgcaactgaacaggattgaacggatcctgtttcaaacgcaggacagtaccctgcagctggaatacgaaagagagggtaagatcagcagtgtaacgctcgctaccactacttataaacaagccatcatagcgggcgaccgcccatctgtttcctggaagatgatcggggaagacgtaggatatgtatatcccggttattttaagaatacacaaatggattcggtaggtgaagcttttaaaaacaccaaaggaatggtgatagatatgcgttcttatcccgcagacaacctcctggcttcacttgtgaagtatgtgctgccgtcgcctgtaccttttgccaagtttactgttggcagtgtacagcagccagggttgtttggcgtgacaggtgaaatgaaggccggcgcaaagaacaaagattattacagaggcaagatagttatcctggtggatgccaccacgcaaagcaacgccgagtttgtaaccatggcgctccggctggcgccgcgtgctgtggtgctgggcagtactaccgccggtgcagatggaaatgtttcttatttcgcacttcccggtggcgtgcaaacgctcatcaccggcattggcgtgtactatcctgatggacgggaaacgcaacgggtggggattgtaccggatattgtaatggagccaacggtgaagggtatacgtgaaaacagggacgagctgctggacaaggccctggctattatcagggaataagttacttttttggtaaagaatatttctttgctactttattatatttcttcaggtacttccggtcttttttaacgcctacggctgttacaataccggaagtttctgcttttacccaatagttgaaaatgaacttttcccggtcgcggataaagaacatccgggtgggccgttgattgcggtttttcaggaagaggttggccaggaacgtttccaggttagccatgaaaccctgccgcgtggaatcctttttattcagcacctgtacgttcaggttgtgataataaaaattcatggcgccaagtgtagcgtatttatttccggaccattgtgagaagatcgtatccgcataaccgcgtcttacttttacagctgccatcgggatggctacggcattaaaatctttcaggtccattggagcaagatagctttctgctgtaaagccggaaagggaatctccataggattcatgataggaaaagtaacggataggattttccaggagcctgccggtagcctgtaccaggaggctgtcggcgttgccgtaggtgttgccgaaatgggtgatcagggcgttgatatccgtaatgggtacggctgaccatttgttcgtggacttcgacgattcattgaccgttaccgcagattgttgtaccacaatggaatctacccggagcgcaaatggaatggtatgaattaattttgtgggcatccatttttcaatgccgtgttcaaacggaattcgtttatccctcgccgttgtcagctgtgtattgtccaccgtaattttacggatcgcaatggtggtgtcgccgggttggtgatgcatattgataccgctgatctgcaatgcatctcctttcactgtaatgtaatcgcgttgccagtgggcagtccggaaagtttcctctgccgaaaggttgggcgtcacttcaaagttacgcacctgaaatgtttgggtggccggatccagtttaaagttctccgcgttgacatgaacctgtttattgcgatagtgcaatccgccgtcacggagcgtggtattgttgatgaatgaggtccactttattttatgaccctggctccaggagaaggatgcatctttaaacatgcccgataatttttgtaataccagttcaagcgtatcggcctggtgcagggagaactgtgcctcctgccaggcgaggtccacacctgagcggagcgacaggtgaccggacttctccttatgcaacgaacctttactgagttgcagggatagctgcggaacggaagcagttgtaccggtatgactgtaggagagcgccgataactgtatgttcatatcgccatattgtaacaggtgttgactgccggtatttacttccagttggttccccgttagccaggcctgtgtttccaggtgggtggtgtcgtgttctttgatgctggtatgcgaaacagcggcattgcccgtagccagtttactaatggctatcctgctgaagtcagtgttatggatgttggtttgtatatcgagagaaggggtggttattttagtatgcccgttactgttatgcagtgtggctgcggcatcggtaatgtacgtataaccgttgctgttaaaccgcacgttgccaatggtagcatccatttttttactgtgatggctgatgtggttaagctggcctgtggcggatgcccaggtaaagaagtgctgccgggtgcgcatatctttcaaagctattttatccgcattaaaactactgtgttcaccggcgccttcgctgttgaactgcaccttgcctatatccagccgggcaacccgtattaccggcaaatcctttgcaggaccttcttttttagcgccattgtgacgtgcctgtatatcgatggccccgatccttaacacatctacctgtatatcctttgattgctgaaatacgtcccagtcgaatacttcccagtaaagatcccttgccgctatgcgggtgccgttttccagtgccacggccactttcgtggctttgttatgccggtgtgtaccatcgaaactgtagttatccatggtgatattagctttatcggatattacattcacctgcagaatatgcaggttaggcatggaatgtttgatatccaccagcgaatcgctgagcaggaagttatgcagcaggatatcggtgttcaggttttttaccatcagcgttacctttgatttgccggtggaagtaaaattgatattgccatctactatccggaaggtgttcacctgtatcagttcactgaggccatgcagcgtttggtagaaggccggcattttaatagcggtgctgtctataggaactttgcctttaacccgtttctttgctttggtaagaaaggtaatacccggttgatagagcactgcgctggtggcttttaaacgctttctcagcaggtgttccaggcttacgttgttgagccgcagggaaggagcgcggaatgttaatcctttgccggaatggttcatcggcgtggggctgtattccacgttgttaaagatcacatcgttccgttgcaggataaattcgtccacactgagctggaacatgctgtcgagcgaatagaactttattttatcgaggttgagtgcgatgctgtcggcggtgatggctggtgtggaatcatgtgcaatattgaggttataaatattcaggttggtacgtttggtggtgccggtagacacatttccacgaagcagcagttcgccgtcttttacttcgatgtaccggaagttcattcgtttgaacagggtattgggcaggctgtccagcgctatctttttatctttggtgctcaccttcttgccagggagtttcaatactgggcggatacatacaagcgtatcaatcagtaattcttcccgcatataaatagcgggaagatgccgggcgttaaagtagaacttatctgcctgcagcgacatttccccttttgtggcagtggcggcactgaagatggtcgccgagtcgagttcaaaaatctgttttttaccggagaagtgcagccgcctgaagctgatagtattcctgccatccgggaggatccagtgttggcggtcgaatgagaagtccacatcatcagatccaagaatatgattatcggagttggtaaccttggagaagttgaggatagagaaattaaaatgatcgacgtgcaggggtggcggcccatttaccttgctgtataccagggaaccgttttgcaggtgaacgatgcgggcatttacatattgcagggtttgttccaggtgctgtactaaagatgaaagctggaatccttcctggcgggagccgcgcgccacatgttcatggataatgagcgcagggctgatcacggagaggctgtcgaccagcagttttttatgcaatatcagcgcgcgccaggattgtatggaaagatacaccctgggaatggacacatcgaaatgagcggccacgttaacggtgtctttcccggtgagccgtgcgccgctgattacaatatttcttttgaaaagggagaagtcaatatcatccgcgtcgaacctataggcgttcccggattctttgctgacgatgtattgtatgatgtttacgaacttatgttctacaagataatataacagcacaccaatggctatcctgaggatgagcaggaccaccaatactttcagccatatttttgctttgggcgatatcttcatattcctggtatgcgaatgatctgattacaaacagccgggccttgtatatgttcatttttcaggaaaccaattttgcgatggcaaaagctgctgctgcagcaagcacacctatcatggttactttcagggctccctgcacgggaggttgaccggttactttacttttaaaatagccaaatacaaacaggcagatgatggtgagcgcagtggaacctatcaaaccgcgttgaggcgtgtccgtgaaaagataagccgatagtggcagcagtcctcctacaaaataggaggcgccgatggtgagcgcgctttgccgcgccctgtttgggttgggtgcttccagtcccagttcaaatttcatcatgaagttcacccatttggttttgtctttcgacagttcagtggcaatcaggtgttgtacttcgggactgaggccatattccgcaaacacttccttcacttcttccatttctttgtcgggtacagtttccacttctgtatattctcttcttaattcgctttcatagtgttccagttctgttttcccggcgaggtatccgccgaggcccatggcgatacagccggctacgatttcggcgataccagcagtgaggatgatgttgttgctgctcacggcgccgctgagtcctgcggccagggcaaagggcacggttaatccgtcgctcatgccaatgaccatgtctgtgataaaatctgagctttttaagtgttcttcctggtgcatctttttccgggttttagggggcttcgcgttataaatataagtgctttatcgtattttgtctgaacaatgtaagggatcatcacctttaatcaaaataggaaagttatggcaaacgggattgtatgttttggtgaaatgctctgggatattttaccggagaaagaattacccggtggcgcggtgatgaatgtagcttaccacctgcagaagctgggagagcaggtgtcgctggtatcccgtgtgggacgcgatgcccgcgggcaggggttgctggacatgctgcaccggtatgggctggataccagcctggttcagaccgatgaacagcaggaaacggggaaagtatatgcggatatgactgatccgcataatgtgcattatgatatcgtatacccggcggcgtgggattttattgattacacaccggcattggcggcgcggctaaaggatacggctacacgttattttatattcggaagtctttgttcgcgcgacaaggtatcgttgcatacgttgcagcaggcattgaaggaggaagtggtgaaggtgctggatattaatttaagggagccgcattatacgcaggcgcatgtggaatggttactggcggagtgtgatatcctgaagctgaatacggatgaactggcgctgatcagcggatggtatcatccttatgtggataaggagcaggccgtgcgtatgttatcggagcgttttgggattgcgactatcgtggtaacgatgggcggtgagggtgcgttgttgtttatgaatgatattttttatgtggaacctggtattgtggtgaaggtggcagataccatcggaagcggggacgcgttcctggcggggttcctgcatagtgtgatccgtgggcgtgcggcgcgggagtgcctggtgtttgccaatgccctcggagcgctggtggcatcttatgcgggaggtgcaccggactatgaggtgaatgatattttaaagcagaggaaatagcttccacccggaagttaattcccctgccagattgttatttgcgggtgtatttgatttccatgtcttttgtttctttcccgtcggttaaccggtacatttccatggtgtgatggtctttatcctgccattttaatacctggcgtacgttgtgttctttgccggtggcagggtccaggcctttgccggtaaattcaagtccatcgccggatttgaggggttcaccttccatcaccatgatgccggtgcccatgttatccacccaggtggaaaagtattttttctttgcattgtcgtacgccatggtactaatgccttcgaagtccatgcccatcatgttggcagtgtaacggccttcacaatagcggccgccgaggatcatcttgtaagtggcggtgccggttgatttgctgggcggtgcatccggtttttcccagaaggtcatgtcggctgtccattcgccatcggtttctgccattttctggtgtgcggggcctggtgtcatgtagtctgcccacgctttcatcatggcggcagagtcttgctgggcaaaggttgcggagttaattaacaggcataacgcagctgttaacaggtaaattgttttcatgatttgcagctgtttaagagatgttcgtaatggggtgaaattacagtccaacaaggtaagatatttattgctttccgcgatcgcatgcgtgttacacctcgtaaatagccaggatttcccctacctttgatcctgaaaaagaattttcccctttatgcaaacaaccatcttggatgtgtcaggaaataaggcgcagccactggccatagatgcagccatttcctttgaaccatttatcgcctatctcaggcagcggatccacgaagaacccaccgtgaaagcccggttgtataaagaagcgctggccgcgtttgaagcatcggatattggccggcgggatattcccctggaagaaacccctcagtattccggcctgctggaatatgtatatgcctgcctttctccggccatgagcccggaatatcagctggcctggggactcagcttcccgttccttcccactactttttatggtacagaccttatctatcaactgctggcaaataattcgccggagtataattacgaagtaacccgcacaccggcagattaccaccgggagcgcctgcagctggtgtattcactgatcctgcaacggctgtataatttccaggcgccggtaaaaacggagcaacaccatgcaggagtaaatacagctaccggtttgctgcaatattatgcggtggccatcagcaccgactttgttgacgtgacggcgaagggtgagctgccggacattgactttgtgcagttgtatacgcattttagtgaaggcggtggtgaagagatactggaagatatgttgccgctggacctgttcagcttccgtggattttgtgtgatcaccgtaacagatgtaacggcggagaaagcggtggagaatattgccggtatgcggttatcgcgtactacattgattgatgaacagaattacgaacgggtgatcttatcgcttaaatcgctggtgcgtgacagcaggattgaattcgacctgtttcctttcctgcgcgtaaatgataatcccgtatatagttttgaaaaaggtggaacgggtgtattgtttgccgtgtggggtgaaagccgcctgtcgccggaagaattcagcaggaatgcgaaagcctttatgtcgaaaccacttttctttttttccggggatatcgtaaaagaaacgcgggaagaatattccttcctggaacatttccgtcagcagggggtaaagtcgctggctattatgcccattttccatatgggtgaaccggtgggggcatttgcggcacatacctggagcgatcatagttttgacgagaaaacgctgtcgctgctggaacctgccataggcgcaataggccagctactacagatctatatagacgaatttaacggggagatagagcaggtgatcaaagagaaatttacttccatacaaccggccgtgcagtggaaatttaatgaggcagcctggcattacctgtacagggtgaaaaagaaccggccggctgtcatcaccaatatattgtttaaagaagtataccctttgtatggcgccattgatatccggaattctactatagaaagaaataaggccatcatcgctgacctggacagtcatttaagcatccttgccaataccctggacttgctgcgcaagtaccagcagaatgacctgctgcaggaaatgatctatcatagccagcggtggcagcaggccctgttgcatcaacagctgagcccttccgatgaaaacgcgctgaacaggttcctggaagaggaatcggtgaattacctgcaacatattgcggcgcaatatcctgatacccgcgaaacgattaacacctgcctgcaaagcatggcgggtaatgtgaataaagatgcgctggaaacatctatgcagctgatcacccaggcggcaaacaactacctggagtcagagaaagccaagttgcaggattcttatccctgttattttgaaaagttcagaacggatggcgtggagtatgatatttacattggtcagtctattgcaccggcacggcctttcaatcatttccatctcaaaaacctccggttatggcagttatcttccatggtagccatcaccaaactaacccactcgctgatcgcccaaatggagaaggagttgtttaccacccagcttatttttgtgcataaccatcctatcgatatcagcttccgggcagatgaacggaagtttgatgtggagggcgcgtataatatccgttaccagatgatcaagaagcggattgataaagtacatatccggaataccgaagaacggttaacccagcccgataaaattgcgttgatctattccgacaaagacgacgtagatgattatctgccgtttatccgctatttacaggaaaccggtgtgctgcagccggagctggaggaactggaactggaagacctgcagggcctcagcggtttgaaagcgctgcgcctgggcgtggtggtggaagacgcgaaataaaatattatctttctcaaaaataatttgcattcccgttaatagtatactaagtttgtagactaataaatcagcgcgggggtagtacctctcaaccgcggtaagcagctcatgaagaaaaaagattacgatgtaatagtggtagggtccggacccaatggcttatctgccgccatcaggctgcaacagcaaggggtatcggtattactgctggaagcaaaggacgtcattggcgggggcatgcgtactgccgagcttacgttgccggggttttaccacgacgtatgttctgcggtgcacccgatggcgatggggtctccttttttttccaaattgccgctggcagattacggtttggagttcgcctattccccgctggaagcggcccacccgtttgacgatggtactgcagccttcctggcccgctcgctggacgataccgcccgtgcgctgggagcagatgaaaaagtgtaccgggaactgataaaaccggtggccgacaattgggaggcggtggcggaagatagcctgggacccttttcgtttccgcggcatccattgatcatggcccgttttgggttgaatgcgctgcgctcagcatcggctgttgccaacaggttttccactacggcagccaggggcttatgggccggcatgacggcacactccatacaacccttaaccaatgtggcttctgcggccatcggcatcgtattgtcggcggtaggccaccgctatggatggccggttcccaaaggcggttcacaggccattggcaatgccctggcccaatactttgtttcgttaggcggaaaaattcaaacaggcgtgcacgttagttcactgtcgcaattgccgtcgcatcacgcagtggtgtttgatctcacgccaaaacaactgctcactattgccggtgatcagttttcaccattctataaacggcagctgtcgcgctatcgttacggtccgggcgtgtttaaaatggactgggcgctgagcggtcccattccttttacagcgccggaatgcaggcaggccatcacggtacacctgggaggcacctttgaggaaattgctttctcggagcaacaggcatacgatggtaagatctgtaaggcgccttttgtattgttatcgcagcaaagcctgtttgatgaaagggcgcccgccggaaagcatacagcatgggcgtattgtcacgtgcccaacggcagcgatgcggatatgacccagatcattgagcagcagatagaacgctttgcaccgggattccgcgacctgatcctggcaaaacataccatgaatgcacaacagatggaaatatataatccaaactatgtaggcggcgatatcaacggcggcatcatcgacatcaggcagttgtacacgcgccctgcctgccgcatttcaccttaccggacttctgcccaaggaatctatatctgttcctctgccacaccgccggggggcggcgttcatggcatgtgcggctaccatgctgccaacactgtgctgaaagattttttttaaaccgtcactatcttaatgaataaatatgcctggagttaagtcttatttacaggaagattgggccattgtcgtactagggttcctgatcatcctgctttcgctggccggagtacatgttgctttaccggattacaaatggagcaccgccggtgaccttaccacgaaggtgctgaccggcgccaactttttaaagatcggcgcacagtttatttacgtgttgctggtggccctgctcgggtcctttcttaccggcagatcactaaaaaataccctgctggtattcccggcagtgtttatattaaccacattggcgctgattgtagcgggtaatgccgcgttgaatgaactgggactggaagcggtaattttcagcctcatcatcgggttgctgatcggtaacctgtttaaactgcctgcctggttccgggaatcccttacgtcggagttttttgtgaagatagggctggtattgctcggcaccaccgttattttttcagatgtgctgaaagccggttcccttggactgatacaggcattggtggtcgttatttctgtttggtatttttcctattgggtatgtaagcaactgaaaatagataaagagctgaccatgatgttgtccagcgcggtgtctatttgcggggtgtctgccgccatcgctacttccggcgctattaaaggcgattcaaagaagttatcgctggtgatctcactggtattgatcaccgccatcccgatgatgatctttatgccgatgattgcccatcatttccagttccccgaagaagtaacaggggcctggctgggcggtagtatagatactaccggggcagtggtagcatccggatcgctggtaggtgaaactgcactgaagatcagcaccattgtgaagttttcgcagaatgtgttactgggtattgccgcttttgcgatttccgtatactggacgtataccaaacatccgaatgcggccgataaggagcaaaagcccacgctgaaagtgatctgggacaggtttccaaaatttgtgatcggctttatcatcgcgtcgctggtattctcctttttgttgtcgcccgctgctattgcgccggtgaaaggatcgctgaaaagtttacagggactgtggtttgcgctggcatttaccagtatcgggctggaaacaaatttcaaggacctgatcggcacagaaagcaggaaaccggtatatgcattcctgatagcccaaacgtttaacgtaattgttacactgatactggcttacctgctgttttcctgaaccggctgattactttttttagtattttgccggtatatgaaatacctgaatccctttgctttcctggagaagatgaatggcggacccgtatcaacggaggatactgctgcgatatcccttctccggaaaaaaatgatggcagagctggaattatcggaagaaaaggtattacgggcaggagcgcaatggttcagcaaaaacaacctgctgcttttttttgatgaactgcagtcgcccggcaaattacacttacatcaacagatcagggatgataacgtcctgttggttttcctggaaacaggtaagctgacaggattttttaatcataacccgctttacaatacgcctgccttcctcacttttatagcgccgttttatgagcccgtgtttaccactgcggtactcgatagcctgaaacaacagcaggcgccggtagtagagcaactgtatgcgaacccgctgctaatggacggcgaacaccagcaccggagttatgataaaatattccgggcattacaggaatcctataaaatactggaagcagcagaacaacgcaggacggcggatccccgctcggggtggaaggacgcagcgccgtatgtgaatttgcaacaggtacaggtgttgaatgcattgccggaaattttccaggagttcagaaacgactctggtatcctcatgatcaacttcgcactggcgctggatggtacccgtgaaaataaaaaagcgctggaaatcctgtatgccgtaaaagcgttgaaatgcggcgcgtatgtgagagaagaaacagtcaaatatttacagcaactggaagaaaaagctgccagccgcaaatcattgctgggcaggtttttcgggagagagtataaaacgaaacaacaacgccggaaactgctccgcgatactttgctgaaaggagggattgcgctggtaattattacggccatcatcatcggtgcgcgctttgaacaggaacaggtaccccgtataaaggtccgggaaagtgcgaacagcatttttaccggcgcccgcacatcgctgactatgcagtatcttttatcacagttactgatggacaatgaaaagcgtgcgaagaagctattggaaggtaccaggctgccagttcctgccacaggcgcagatgtgtatggcgccgattttatgaaagccgtacggatgcagggagattacggcgccggctttgtgcgtccgccttttggccggtcgaggaagtgggcgccggaagacagctcccggaacgatgccgcgcaccggcaaagtatgcaggtaattaaccgccaggatggagcgctgattacaatggtgcaaacgcccgactctttttactcgtgttacatagcgccgttcgacagcgcctttgtgcccctgccgctttccataagcagggtatacttttatgccggcacaggctgggacccggaatggaaggcggagtatgcaatggactacgtaccatcttatcgtgctaaaggtttttttcttatgcctgtttatgatgcgctctcattcctgaaaacctcctgcctgcagctcaacctggatagcagctactggcagcactccaaccgttatatcccggtagaagttttcttatccgaaaagaaccaactgcaacagcaactgcaactccggcagctgaccaataatttcaacggcgtagacctgattccgatggagtagccgcttttttatttattttgctttcttatgaaatatgtgaatccccttagtttcctggaagccgttcatggtggacccgtagataccgggaacagtgctgcgttatcccttctccggaaaaaaatgctggcagaactggaactgtccgatgataagcaacttaaagtaaatgattgggtattcaataagcaccagctcctgcagttttttgaccagctgtcggcaggcaatgagctgcgctatcatgcgcagatcgccgccgaccccgtactgctgcatttcctggaaacgggtgatatcaccggccggtttgccaataacccgctttacgaagaacatgcgtttctgaaatttatctctccttattatgaaccgctgtttacaaatgcggtactggatagtttgaaacatcagcggctgcaaaatacctcccatctttttgccaatccctggctgctggatggggaacatactactaccagttatgggcggatattccgttatctgagagtgctggaagaacaggtgaaaattgttattactaagctcagagcggcggaggtgattccatggaaagagttatcagtttttgctaacattacgctcatacagcaactaaatgtgctgccgcgtgagtttcatgagtttagaagtgactatggtatttgtttaataaacctgggcctggctacctaccgggatgattttaaaaatggaatgtctgcacttgaactcgtgggaaagctgcatactacgacctatgtacaggaggaaaaggagcgttggagactgaagatgaaaggctacaggaaagagcagcgggcaaacagatcgcttgcgcagtgggtaggacattttataggcccgcttaaaccgcgatggataagtgaggaaggtgcaggaacgttaattcttctcatatcggctttagtgtttttcagcatgatgtccaggataataacaaagaagccacagccgaaggcaactaccgaggtcgtgtattttactcatgaccccacttatcaacctgtaaaatatctcctggctaatttacaaatggacgcggcatatacgttgaacaagtatgctggtaaaatgccggaaacaggcgacgatgtatacggccctgatttaatggcggcgttgaaagtacccttcaggaaaaccaccgataccactgtatcggagacggcggaagagcagctgacggatagtaagccgggaggaacggagtccactccgaaagcaaaatcggctccgcggcaaagcctgcatctctataaccggttaatagccccggcaatcgccatgattcagacaccggacagtttttattcctgctatatcgcccctggcgacagtgcttttgtgccgttacagctcacgattaaccagctgtacgtatatgttggacaaaactgggatggaagtatggaggcaaggggagcaatggacgatatccgtgcttaccgggtcaaaggtttttttattctgccttataaaaattccaaagacttcctcaaagaaagcagccttattttcaaactggatcccaattactgggccacttccaaccggaatatccctattgaaatcgggctcacagacagtaccagtctccacttcaacctgctggaaaataatgccgcaggcatagagctggaaatcgccaattagccgatcccggttcctttcagctgatcggcttcttttttggtatccggcatgaggttgtacagttgattcaccgctactttcagttcttcataatttttccgttccagcgctctttctccgatttccttgaaacgggcagctgtttgcgggtcagtataatcttctgtacttacattggcatagtaataatacgcattgatccaggtttcgggtttattgcgtcttatttcccaggtgaggtcattcagctcatcaatttttgctttgattgcatagtagctttgtgaagaaagacaggcgctttcatcggcaatgaccttttcaaaacggagcatgcgggcgctgtcttcttcttcccggatattatacaaacaatattctttccgtttaaaatagagttcggtaatttccacgatcagctggtctttcccggtgctgtcgaggtgttgcgcgagtttacgtttcttttcttccagctgatatttttcatcggtcacatcgtctgtgctgagcagttccaggcggttgctgatatgatcaagatccaccatgatatcttgtaccgtggcagccagttcatattgctggcttctcctgaatgattttattttttcagatgcactcaggcgcagctgccggatatcgtcgagcagtttaccagtgtttattttcctgaccatcgggttgaatacttcggagaattcctgttcgttcatgagcaatactgctttcacggacaggtccctgctttcgctgatctgcaaagtaatttccacatcggagccttttacaaggtcggtgatgaggtctgtgctttttatttcaatcatgccgagagggatacaactgcccgggatggcatagcgactgccttccagtacgttgatcagcaggctgtcctggctggtgcgcaggatggttttcatcacttctttgatgattgttttcctcagcgggaggatggcgttcttttcaaagataagttccagcttggtcgtattattttccaggtcatctatttcaatgcagatatcgttgggcagtggctgaccatgaatgttgaacttgccctgggaaatagcgatcaccggtgcctgtaccggcagttcgttgtgggcggcatcgaataccaggatattaaatgcgttgctggtattttcagccagcagcaacatttcggatatgcgttcctgcagcggtttgatgccgctgtcgtagccgccgtcggtacgcacaatgcgatagcttagtccggctacaggaccggttacgatggcagtgaaatattcttctttatcggcagtgtttttctggtaggcagttttaaaccggatgtccggtatgcctgctgccaaaggtttgctggctgcggatttggacggggtaattgttttggtaccggcataccatgctgcgcctgcggctacagcagtggtaggatctacgctgcaattaaccgggatgcccagttgtgcggtaaccaggttttttaccagcgggatgtaggtactgccgccgatcatcactacttctttgatatcggcagcggtgaggtggttacggtcgatgatcctttttaccagatcaacggaatattgtatgcggtcgtatataacggtttcaaattgttcgcgggtgatggtgagataaatatcctgtgtctgtccgccggcatcagtgatctcgaattctatttctgcagaagaactggcggtgagctgcacttttacttcttctgcctttttaagcaggatatgatacagggtattgtatttaccgcgtgcgctgcgcatctcgttgagcaggtcggggaaggcgtgttgttgttgcagggcagggatcaccagttgctctatgatggcgatgtcgaagtcaacgccgccaagatagttatctccttcatgatcggtaacacgcatttcaccatccacaattttcacgagggccacgtcgaaagtgccaccgccaagatcatacaccagccattggccctgcagggaggtagcgttggcctgtttgttggcaaaagccaggctggcggcaatgggctcctgcaacagcagtacttcactgaagcccgcatcgttgccggctttcttggtagcgttcgactggatcgtgtcaaaagaagcggggatcgtgatgatcactgcttccggtttttcaccggtatagataaagtttttgagttcgcggagtaccagggcagagagttctaccggtgttttaaaatcgctggtattgggcacaaaaaaagattccgatgttcccatttttcttttgaaagaagaaaatacattttccggatctttctctattagttcacgggctttgtcgccaacaatgatcctgtctttccggaaggccaccaccgaaggcagtgtttctttctggccaaacgggtttttgaagatttccacggcgccgttctggaacctggcgatcagggagttggtggtgcccaggtcgataccgaaattaatttggttgttcataggtttattttgcggcggcaatgactacccctttttgtaaaatggacttttgtcccccggcagtataatatacaacaggtttgatcacatttactatttccatgtccggcgacatatcaccggtgatactggcttcgtaatccacccgtgtttcccggtacggttcacccaatggattaagaatggtatatccggcttcttcaaaatgctgtttgatccggtctatattacgttgcagggatagcagctccggtttggtacttgttttcttgtccagttcaaaaacctggttaatgatccggatatgcagggtagatagtgggtccattattcaaatgctggtctaagcaaatatatggataatttaatctgtttacaggggcggtcaaggaaaacgtttcctatgtatggcatcggctttgatgagaggaagttcctgctgaataactatattctaaaagtagtaacctgatatatggaaacaacaacatatcccggaagccctttcccgttgggcgccacctgggacggccagggcgtaaactttgcgttgtatgcagaaaatgctacccgggtggagctgtgcctgtttaatgatcctgcaggaagcgcatacgatactgtccgtctttcggaccgcagcagtaatgtatggcatgtctatctccctggtgcgaagcctggtcttttatacggctaccgggtacatggcccgtatgaaccggcagaaggacaccgctttaaccccaataagctgctgatagatccctatgcgaaagcggtgagcggaactatcaactggcataattcgctgttcggatatgaaccggggcatccggatgaagacctgagctacagtgaaacagacagcgcaccttttgttcccaaaagtgtggtgatagatcaacagtttaactggggcggtgacaagccgcctaaaactccttatcagcaaagcattatttatgaaacgcatgtaaagggtttcaccaaactgcatcccggtattccggatgaaatacgcggcacttacaggggcatggcgcatccggccaccattgattatataaagcagctgggcgttaccgcggtggagttgatgccggtacatcattttgtggccgaccgttacctggtagataaaggattaacgaattactggggatataacagcattggtttttttgcgccggatgcacgatatgccgcttccggctgttgtggtgaacaggtcacggaatttaaggagatggtaaaagcgctgcatgccgccggtattgaggtaatactggacgtggtatacaaccacaccgccgagggcaatcacctgggacccaccctttccttcaaaggcgtggacaacgcggtgtattaccgccttacagaagataaaaggtattacatggattataccggtaccggcaatacgttgaatgcacggttgccgaatgtactgcgcctgatcatggacagcctgcgttactggattacagacatgcatgtggatggttttcgcttcgacctggcagctacgctggcgcgtgagctgcatgaagtagaccggctcagcgccttcttcgacatcatccaccaggacccggttatttcacaggtaaagcttattgcggaaccctgggatgtgggcgaaggcggctaccaggtaggtaagtttccgcccggctgggcagagtggaacggcaaataccgcgacagtatccgtgattactggcggggagccgacagcacgctcgcggaatttgcttcccggatcaccggcagtgcggatctttataaagaagattatcgccgccccactgccagcgttaatttcattaccgcgcatgatggattcaccttgcacgacctggtatcttataatgagaaacataatgaagccaacggggaagacaataaagacggagaaagtcataaccgctcctggaactgcggcaatgaaggaccctcgcatgatccgctggtgaatacattacgactccggcaaaaaagaaacttcatcgccaccctgttcttatcacaaggcgttccgatgttgctggccggcgacgaagcaggaagaacacagcagggaaacaataatgcctattgccaggataatgaagtgagctggctgaactgggcaggcatagatgaagaactacttgcctttacaaaaaagatgattgcgcttcgccggcagcacccggtattctgccgcaagcgctggttccggggcgagccggtggagagtgtgggcgtagaggatatcgcctggttcctgccggaaggtacgcctatgtctgaagagcactgggataccgactttgcccgttccctgggtgtttatctcaatggactcagtttacgcacccgcgatgaaaaaggaaacaaaatcctggacgacagcttttatatcatctttaacgcacatcatgatgaactgggttttcagctaccgccggcagcatatggcgaccgctggaagatggtggtgaacactgccaccaatgaggaaggcgatgaatataccgccggcagccagttgatggcagcgggcagatcgcttattttattaatgaaggaagaagataaatcagcctgataccatttccagcagggcaaccgggaagcgatccaataatgccagcggaagcttcccgttttctgttgttatcctttctcccgtaaatatattacgccattgctgtggcatattgttatccagcaccaaccaccgctggcccatattattatccgcatttaatagcggcgctattaccaggcagatatcctgttcatgttgccgggcataggctatcagcggatcctggtcgccgctgagcgggagatagtcgccttgctgaaaaagtgcagcatgtgctttcctgaattgtaaagctttggcagcaacaaataatttctcccaggcaaagtggcggttttccttcagcagttttattaacgcggccggatcatcttcttccagctgctgcatcagtgacagcatattgatgcggttgagataatttaccgggcggcggttatcgggatctacaaagctgaagtcccacagttcgcagccctggtagatatccggtatgcccggcgccgtaattttcagcagcagctggctgagtgaatatataggcgcatgctggttgatcttttccataaaaatgcggaggctttccaggaagccatgatccggggaaaacaaccgttggataaaatgcaggcagctgttttcataagcttcgtccggcgcagtccagttgctgtgttcttttgattcgcgcagcgctttgatgagataatcggaaagccgtgtgataaaatcttctccgggatcattgttttcaggaaagcctgcgatgatggattggtagatgaagtattcatcattttgcgccggtgcggtttcttcgcggaaaatgctgttcatggcatgccattgctgtacctgctgaatccaaaggtcgggaagcagggtgagtacatttaagcggatgcgcgcatcttcgccacgtttggtgtcgtgcgtggcagtagcattcagtgatcccggaaataattcctgccgtttgatactgcgttcgtgaaaagtcgccggtgtgcatttataacctgcgggtgaatctcctacttcgttgtgcgaaagcagggcattatacacataaaatacggtgtcttccacgccctttgcggtgagcgggccggtaaactgcatcagtctttttaaaaactttaaagcaacagcaggtttttcgaaatcttcctcccaccaggagcggatcagggtaaactcctctgttaatgcaggcacacgttgtgcggcagcggtaagcgcttcttcaagaatatgtatgtcgttttcaggcagtggccatatttcaggataaacacggtatacaggcatgcataccatccataatcccagcgccgctttcagcttctggcggtcggtgttttttggcgccagctggtattggaacaacaggtgcaccaggttatcccattcggcgctgagttgtgtttgcaggatcattgtttttttattctgcaccagctgacggtatttggcgagtccggggaacagggcccggtaaaagcggctgatcttttcatcgccccagtgattggtgagcaggtgatttacatccgacaaaaattcatagccggtggcgccatccaggtgccagttctccggcaatgactctccttctgccaggatcttttctgctataatgtaacagttgtccccaaagcgttcgcggagcctgcgtacatacatagccggttccatcaggccgtcgatatgatcgatgcgtagtccctggataagaccttcctggtatagctcgtgcaggaatttgtgccaggtgtcaaatacctgtttgtcttccatccgcagggtgaggagtccatttacggtaaagaagcggcggtagttgatccgttgctccacttcgcgccagtaggtaaaaagatagtattgttgttccagcaacagggtgagcagcgcttcgtggttgttcacctgttccaggaatgtgttgagtatggttgtttgcagcaaaccggtaaacagccgttgcttctgtgcagaccaatcttccggcgataatggcagccggctgttttgtttgagggtaagcaggcattcgtatatctgcggatgtaaatcgtcgaaggcatcgaggagaatatcataggcggtagccgacagcgggaattgcagtccgccggtatcgaatttaaaaccttccgtatcagctgtaaaggcgatctgtttttcagtgatggcctgcggcaatggccggtcgaggaaaggaaccatcagccggccgtggagttgcggatcgcggtactcccaatcgatatcaaagaaatgataccagggggaggaagggcctctttccaatgtatccatcagccaggcattgccgggatgcagcgccatgtgattgggtacaatgtcctgtatccaggtcatgccgcgttgtttgagtgcagcgctgatcctgcggaggtcgtccagtgtgccaatggcagggttgatgcggtggggatgaatgccatcgtatccgtgtaaactgccgggtactgcatcgaatatgggagatgcataaatggtggtgatgcccagttgttgcaggtagtcgagtatttcttccaggtgtgcaaaggtaaatgcatcattgaactgtatgcggtacgtggaaagagggtaagtagtatcagttttcataagcaattatttcataaacaacagcagataaaggtggtattaccagttggttttcgttttcagctggaggtaatgtacctggtccgttgaaccgcgtactggcagaatcaaatatctgccgcagtttgccgtgggtggtgtagggtactgtttgcgtattggaatcgaaattaaatatgatcagcagcgtatcagcgttcatgcggcgctccagtatcagcaggcgttcattttctgcacgatgcacacgggtgccttcccgggcggtgttgtaaagagccggttgttgtttacgcagcgccagcaatgctttatagcagttgagcagggccgtgttgttatcaccagtggtattccagcttaatttacttcgctgaaaagtagcagcgtcctgtggatcgggcgcttcgccggcgtgtgcaaattcccgctgccgtccttcctttactgccttcatgagtgcggggtctgtatgagaggtgaaaaacaggaacggatttttttctccatattcttctcccataaataataagggaataaagggagataatatgacggtggcagcagccagtttgagcgcttcaaacggaaccagtgacgacagccgttcacccagcatcctgttgccggtttggtcgtggttttgtgaaaaaacaacgaactggtggaacgggttaccggaaggttccctgccgaatttccttttgcggtgaacggaatactggccggtataaacgtaggcgttttcaaaggagcgggcgagatgtgacacggcgccaaagtcttcgtaatatccttgctgctcaccggttaggaggctatgcaaggcatgatggaattcatccacccactgcgcatcaaggccgtaacctcctgctgatgcggagttgataaagcgtggatcgttgaggtctatttcaccgatcagcactttccgcttgccggtgcgctcctgcaggtcttttacggctgccgacagctcttctgtgaaatgcacagcgctgttgtcggagaacgcgtgcaccgcatcgagacggaggccatcgatatgaaactcctccagccacattaaggcgttttgtatataaaagttacggacgccatcgcaccaggggccgtcgaagttaacggcatcgccccagggtgttttatacttatcggtgaaccagggcgcgaagtcggagaagtagttgccttccgggccctggtgattatataccacatccaggatcacagcgatgtccaatgcatgggctgcattaacaagcgttttcagttcatccggtgtgccatagctgttgtgtaccgcgaacggatatacgccgtcgtatccccagttgcggttacccggaaattgcgcgatgggcattatttcaatggctgtaatgccaagttctttcaggtaatgcaggtgttggatgatgccccggaagttgcctccggcagagaatgtgcctgtatgtatttcatagatgatcattttttcggggtcaataccggtccagtgatcatctgtaaatgtgaacgacgtttcaggaataacggatgggccgtgtacgccttccggctgccagcgggaagccgggtcggggcgttgcagctggttatccagcaggtaggtgtaccgtgttccggggcgtatgtccgttagcgttagttcccaatatccttccgctgaacgttccattggtaagaggcggtcgtgcagttgcaacgccacttccttacggaaaggcgcccacagccggaaggtggtagctccatctgcgttggtgaatattcctgccaaatcgtatctgttcataaaattaccggttatacagctgtgtccatttttttaatcttgtgatggtctttttgtcgaactgccccggcagcattcgccatgcccaatgttgcccttctgctgcgggtttgttcattctggcggcagcgccgagcccaagtacatcctgcatgggcagtatggcattggccgcaacagaagcatatatcatgcgggcaggcaggaggtgttttttctttttaccgggcgtaatgccggcgtattgtttcaggcgattgcatgcagccggcgatgcctcttcttctatccatccggcaatggtattgttatcgtgtgtgccggtatatgcgtagcagttttgcggatagtgatgggggatatgcacacttacgggcatatcatcgccgaaggcgaactgtaatactttcatacctggtaaccggaactggtcccggaggtctgtcaccgctttatcgatgtcgccgaggtcttctgctacaaaaggattgccgggaaaagtgctgatcatggctttcagcaggtcgccacccggacctggttgccattcgccggtttttgcagtgggcgccgtggcgggcacctgccagaaagcggcaaaggcgcggaagtggtcgagccggagaaggtcgaaccaatgcatgttccgtttaatcctttgcatccaccagtcgtagccggtacttttaagttgtggccagtgatagatgggcatattccaccgttgcccgttttcgttaaaataatccggcggtacgcccgctacgctggtcatgttacctttatcgtccagcaggaaaagttcgcggtggctccatacatctgctgccgcgtggctgatataaaaaggcaggtctccgaacaattgaatgttccgctggtggcaatatgttttcagttgctgccactgccggtcgaagatgaactgccaccactgttcctttaaactgatggcggcgtattcagtgctgagacgggcatctttcttacggtcgggcgcatcccattcctgccagggtttgccgccgtatttgacagacagcgctttgtgcgtggcataacttttcagccatgctgcctcacgattgcagaaggcgtcaaagtcggccgctattgcaggataaacgccgttgctgtaatttaaccaggccgattccaggatggccattttataccgcgcggccacattgaaatccaccgtatctgccgaaggcaaagtaaattttaccaacatctctttatccagcaatccgtcttccatcagcaattccgggctgatcagcaaaatgtttcccgccatagcggataacgcactgtacggggatgcattggaaatatcaacaggatttacaggcagcacctgccatatctgctggccactgttgtgcagctggtcagcaaacttccgtgcagcaggccccatatctcctattccaaaagggccgggcaatgaagtaatatgcaggagtatccctgccttccttgctatattgccggaaggttgtaacgccatatgttgtatttaaaataacggatcaggcagataatcgacggggcgcttcctgtgttgtttgatttccgtgcatcatttcctttatcagtgaagccacgttgctcagcaccggaacaggttctgagataactgtcctgctgtaatccttttcaaagatgattttcagtgcatctcttaaacaataaatatcagactgcttgggcaaacagtccgagaagccatgcgtgctgaggttatcaaggggtagctgctctgcggccgctgcaaaatgtatcacaggtacagtggccagcctttttaacctgcggatttgctgaataaacaaggcagcatgtgcaactggtacccccgaactaataaatatataatcggggacgaaaccgggttgtagtttcagataggcaagcgcctcaaaggtgttgtcctggcaaacacaggcctggttaactttcagcaggtctaaggacaggtaaaactggatgcgttgatctgctttttcttcaacgagaaggctggtaattttctttttcatacgacacaatattgggatctggttacattttaatccggaaacaaatcaggtgccggatgatgatatgattataaaatggctgtggtggccggttatcgggatctgtctttttttataagtggggataatatcactcaattgtgtaataatgccgcagtgggtaaacagcctgaaggatttgttacaggctcatctggcgcggttatcacgcaggcttcgcttttattaacggttacttttggcataagaattactattaagaaagtatgcgaacatcaacggttaaaaagaaaagatcttctcccccggcaaaggccggcaaggtgtccggaaaactgcaaacactattccggaagtatggttttacagatgcaccggagaagcctttccccaaaacagtgaagcctatgctggcaacgctggtagaccagccccccggtggagaaggctggctgtacgaagtcaaatgggatggttaccgtgctgttgccttatgtaaaaatggtgacgtaaacctgatatcaaggaataacaaatcttttaatgataaattttatcctgttcaccaggcattgctgcagttgaataaaaatgcagtgattgatggtgaaatttgtgtactcaatgaaaagggaatcgctcattttggcgcgctgcaaaactggcggagcgaggcggatggggaactgatctattatatttttgacctgttatggtacgacggaaaggatcttaccggcttgccgcttaccagcagaagggggctgctggaggcccttatcccgggaacagacatcattcgttacagcgaatcttttagtacgtccgccactgatctcctggcagctacaaagaaaatgggaatggaagggattatggcgaagaaagcagacagtttttatatccaggacaggagcagggactggctaaaaataaaatccaataaaaggcacgaagtagtgatcggcgggtttactaataacgaaggttctcccaaagcattcagctccctgctggtaggcgtgtatgaaaacgggaagctgcggtataccggtaaaatcggcaccgggtttaataccaggcagcagcaagaattgatgcagcgctttcagccattgaaaataaagaaatgtccttttatagaaacgcctgatgtaaaccagccttcccgcttccggccaaacccgccggtggcaaccgctacctggttgaagcccgaattggtttgtgaagtgagctatgcagaaatcacgggcgacggcgtcatgcggcatccaagctttgaaggcatgcggaccgacaagccagccaaggctgttaccgccgaagaacccgctgaattagtggatatactccctcaaaaagaaaagacgaaaaccgtgcggttaaccaaaccggttggtacgcgcagccgcaaatcgttgttgaatccaacagaggcaacacaggtaaaacaggtgagccagcatcagttgaagttcagtaaccttggaaaaaaattctggcctaaagaaggatacactaaacgggatatgctgaattactattaccagatggcgccttacatccttccttatcttcaacaccgcccccagtcgcttaaccgttttcccaatggtatagaaggtaaaagtttttatcagaaagatgtgaccgctgtagcgcctgaatgggtcaaacaatttccctaccgcaccagcgaaggggaagacaaaaatttcctggtagtagaagatgaagccagtttactctggatggctaaccttggagccattgaaatgaatccctggaacagcaccattcataacccggataatcccgactggtgtctgattgacctggatcccgataagggtaatactttcgcgcaggtgattcaaactgcgcaggtggtgcatgaggtactggagggattaggaattaaaagttatcctaaaacttccggctctacgggcattcacatttatattcccctgaacgcaaaatattcctatgatcagtgccagcttttcggaaagctggttgccaccaaagcacaggagcagttgccaacgtttaccagtattgagcggatgacccgcaaccggaagggaaagatctacatcgattatttgcagaaccggcccaaggctacgcttgccgcaccttattcattgcggcccaagccaggagccacggtttccatgcccctgtattgggaggaagtgcggaaaggattaaagatgaccgattttaccattgagaacgcattggcacgtgtcaaatcggaaggggatctttttaaaccggtattgggaagggggattaatctggaacggttgctgaaaaaattttaggtgacgcggatagcccgtgtttccctattttagcaattcatttccacaatccatgttatgaaagagcgttccttcttcatcaatgcaacaggcattcagcaaaatacatttgacgctattgtgatcggctcggggatcagcggcgggtgggctgcgaaagagttatgtgaacagggattaaaaacgctggtgctcgagcggggaaaaaatgtggagcatgtaaaagattatccgactgcgactaaagcgccgtgggaatttaagcatcgcgggcaaatgacgaaggagtttttacaggagaatcctttgatctcaaagactgcggggtttggagaagatactgcacatttttttatcaaagataaagatcatccttacatacaggaaaagccatttgattggatacgcggctaccaggtaggagggaagtcgctcacctggggacgtgcctgccagcgttggagtgactttgaatttacggcccccgagcggtatggatatggccccggctggcccattaattatgaaacggttgcgccctggtattcgcatgttgaaaagttcattggcgtatgcggtacccgagatggcattgaagccatgccggatggcgaatttctgccgccatttgatcttaactgcgcagaagcagcgatacagcaaaagatccatgcaaattacaaagaccgtcaccttgtacatgcaaggtgggcgcatcttaccgagccgaaagaaatacatttccagcagggccgtgtaaaatgccaggccaggaatttatgtatgcggggatgtcctttcggcggctacttcagctccgtttcctctacactgccgtgggcaaagaaaaccgggaaccttacgatacggcctttttctgttgtgcattccatcatttacgacgaacaaaaaggcaaagccacgggtgtgcgggtaattgataccaacacaaaacaggtcaccgatttttttgcacggatcatttttgtaaatgcctcggcgctgaacagcaacctggtgttgctcaactctaccagccgtcgtttccctgacggtcttggtaacgacagcgggttgctgggtaagtatgtagcgtttcataattacagggcgtcggtgagtgccggtatagaaggaatggatgatcaatactactatgggcgtaatcctacggagcctatcattgccaactaccggaacctgcaccgccaggacactgattatgtaggtgggttcaccacttttatgggcgcgcatcgcgggcggggaaacggggagggcataggcgctgcgtgtaaggaagcattatccgaaccgggcgcctggagcacttatatgtatatgcagggagaaactattcagaaagcaaccaacctggtgagattaagtaccgatcaaaaggatcagtggggcataccattgttggtgatgtctgttgattatgatgataacgacgaaaagatgatccgtgacttcctgacgcaaagtgcagagatgctggagaaggcaggttgtaaaaatattcagcagcatgataacaagcaggccccgggtctggacatacacgaaatgggaggttgccgcatggggaaagatgcccgtacttcgttgctgaacgaatggaaccagctgcatcattgtaaaaatgtatttgtaacagatggcgctgccatggcgagtaccggcaatcaaagcccttcgcttttatatatggcgctcacggcaagggctgcgagctatgcggtgagtgaaatgaagaagggaaatttgtaacaaccgtttttttattgagggtttgtcggaatttatagttatattaatatagaaaatataaaaagatgaaaattgccgcctcaaaaatacttccttccattaacgaattagcggagactttaaagcaaaagttttccgacaggtattcatatgaactatttgatttcggtaacaagcaaagtatttttgtggagaagtctgcttttgtatcgatccaggtaacaagagaagaaaatgaaattatgatagagagaattgcaaaaccatctattttcacggcggttttctttttagtggatcttattgttacgggtagcggcaatgtattgtaccggctttcgccattccattcagaacagcaaaaactcgaacaggaattaagtgcctttttaaaaaaggaatataattagtcagcacttctttctgcttttccttcccatataaattcaaaaattaccttttatttcgtcaggctatcccgatgaacgcagaatacaggctatgatttgtcaatcgctgggtacctaccagtgttttaccaatcatagcctgtgttgtttttcggcgggtaaaaaggggagatagtgcatggggagtgcatgcttagtgcatgaggagtgcatggggagtgcatgcgaacagtattagtactgtatggatgatccatggtatacccatggatgaggcaactcagaagtatcggtgaagtagtcacggcacgaccgggaagcgtgtttttagctactgtgtccctggttcacggccaggtccaggcgaaccatatagccctccattttcccgcccccgtctttttgttttgtttttccggaattagatattatcttaaagctgttcctttttccacataaacttaccagacgttatgaaaacttggttgctactccttttagccgttgtcttctccccgtttttgcaatcgaatgcacagtcgttgcctgccatcggcatctgttcttctttttccaacgacagtctcgctgctgccaacgggtttactttcatggaagaaaccgtgcggaagatcctttcacctgcactgagcgaggcccagttcagggaacagctgcatgccatccgcagcagtaaatgcaagatccagagttgtaacgtatttattcccggaaccatgaaactaaccggcaacgaagtagacgaagctaaagtgctggggtatgtggactccgtgatgcaacgggcaaaaatcgccggaataaagatcattgtactgggcagcggggaagccaggaaaataccggagggcgcagaccgggccaaatgtaaacaacaattcattcaactgtgccgtaaaatggcagtggtggcgggaaaatataacgtgaccattgctatggaaaacctcaattccaccgagactaattttgtgaataccctgtcagaaggcaatgagattgttaccgccatacaacatcctaacttccggcttacggcagatatctatcatatgcttaaagagcatgaatctcctgccagcatcgaaaatgccaaagcagtactggtacattgccatatcgcggaaagggataaacgtacacctcccggtgtagccggcgacgatttccggccctattttgccgccctgcataaaatcggatataccggtcatattatgatggaatgccgctgggacgaccctgctacgcagtacaaaccagccttcgactacctcgaaggacaactgaaagaagcttacgccaaataaacaacacactataaaaaacgcctttatatgtctgaatcaaaaaaaacaagacgggaattcctgcaacagtcgttactggcaggagccggcctcacgatcagtgctatgggaatgcccgccagcagctacgcccgcatcatgggcgccaacgaccgtgtaaatgtgggactggtaggattctccgatcgcgcacgccaggccctgttgccatctttctttaataacaacaaggaactgaacttcgacctggtggctgtatctgatatatggaaccgccgcagggacgaaggaaaggctttcctgcagcagaaaaccgggcataatgtacaggcctgtatgaataacgatgagctgtacaatatcaaaggactggatgcggtattcatcgcctccgccgattttcagcatgcttatcataccattgaagcagtaaaaaacaagtgcgacgtatacagtgaaaaacctttcgcggaaacaatggaagatgcccgcagtgctctcaaagccgtgaaagactcgggccgcattatgcaggtgggtacacagcgccgcagtggtccaagctatcatgcagccgccaactttatccagcagggaaaatttggtcccattacgatggtggaaatgacctggaacgttaaccagccaggccgctggcgccgcccggacctggtaaattccattaaagaatcagataccgactggaaacgcttcctggcaggtcgcccgcaggatagctgggacccgcgcaaatatctcgaataccgcctcttctggccctactcttccggtatcttcggacagtggatgacacaccagatagacaccgtgcattggttcagcggattgaaacatccacgcagcgcggtcgccaacggcggcatttatatgtggaaagacggccgtaaaaatccggataccctcaccgcagttttcgactacggtccggagaatgatcctaccaacggtttccaggtaatgtacagcagccgtttccacaactccgccggcggtaccaaagaaatttattactccaatggtggcactattgatatgtctaccaacaaaataagcgctaccggtggtctcacagaaagagaagcccaggaaatggggatgcacgccaacctgctgacgcctcaaacgctcagcaatgacgaagctgccaccaccagcgccaacaccggcggcgacccgctcaccaacgcgcatgtacgcaactggatgacatcggtacgtgaacgtaagcaacccaatgcgccgatcgaagcagcctactcacattctattgcactcatcatgggtaatgcggcctaccgcaccggcatgaaagccacctttgatgaagccacccaggaagtaatggtgggaggtaaagtatttaaaatgtaaaacacgaggcggagggaagacattccctccgctttaataatcagtttgtcccccattagtccgcgcgttaccccattgttgaaaaaagacgggaatactttgtattttggatcagcgaagtaattgcaaggtatagcaacatgaacatgaaaatttttaacacattgctgcccattgcagcaggatttaccctgttaaccgcacccgtagcggcacagcaaaagaaaacaccccctcccaatattgtttttattctggccgacgacctgggttatggcgacctgagtgcatatggtcaacgaaaattcaatacgccccatatcgatcagctggcaaagcagggcatgcggtttacacaattctatgcaggtacatcggtatgcgcaccctcccgtgcgtcgctggttaccggcctgcatacaggtcatacttttatccgcggcaataaagaaatacagcccgaaggacaacagcctatagccgacaccgttatcacgctaatggaagtactgaaaaaagccgggtatacttccggcatctttggtaagtggggactgggcccggtaggctcggaaggtgatccgatgaagcaagggtcagaccggttttatggctataactgccagcgcgaatcgcaccgctttttcccgacacacctgtgggacaacgataccaaagtggtactggaacaaaacggccggctggagcacatgaacacttatgcgccggatctcatccagcagcaggcactccgcttcctggatgataataaaaacaaacctttttttttatacctcacctacaccctgccacatgcagagctgcaggtgccggatgatagcctcttccggcattttaaaggcaagtttgaagagaagccctataaaggcaacgactacggtcctaacgccaccgtgcccggttacgcttcacagcaatatccgcatgctacctttgccaccatggttaccaggttggataattatgtaggagaggtgatggcgcgcttaaaagaactgggcctggataaaaataccctggtaatttttacgagcgacaacggtccgcataaagaaggcggcgccgatccggcattcttcaacagcagcggaggtttccgcggtgttaaacgcgacctgtacgaaggcggtatccgtgaaccatttattgcacgctggcccggcaacatcaaagccggcagcaccaacagcttccagggcgctttctgggacatcatgcccacactggcgcaactcaccaacgcacccgcagtactctatacagatggcgtgtcactactacccaccctcaccggtaaaaaaggacagcaaccacataactatctctactgggaattccatgaagacggcggccgccaggccgtgcggcagggaaattggaaagccgtgcgcctccacgccgcacaacaccccgatggagccgtggaattatacgacctttccaccgaccccggagaaacaaagaacatagccgccgcccatcccgatattacgcgcaaactggccgcctacatgcgcgaagcgcatgtggagacggcgttgtatcctttccaggagaagtaagcgaattttgtcttggctcaggattacgctgattttgctgattacctggatttttacttttggattttttaaagatttttagattttttttaataataattaagggagatagcagcgatatatccgctgctatctcccttaatcctttaaaaaatccaaaagtaaaaatccaggtaatcagcaaaatcagcgtaatcctgagccaagacaaaatccgcgctactagctccgatccaccagtttgttcattgcttcactatacctttccccggtgttgggatacttccgcagtaagtcttccaggttttgcagatcagcaggtgttaaactcacgtctactgcgccggcgttatcgaggaggtattttcttcttttggtgcccggaatcgggatgatattttcgccctgtgctaatacccatgccagtgccagttgagcaggggtacagtttttaccggcagccagttccgcaaatccggcggccagcaggcggttgttttccgcatgttcgccctggtagcgggggagagatttccggaagtcgttgtcagcaagattggatatatcgaggtcgttggtaacgaggccccgcgcaagcggactgaatggcacaaagctgatgcccatctctttgcaggccggcaggatctctttctccacatcccttgttaacaaagagtattcactctgtaatgcgctgatggggtgaacggcatgcgctttacgcaggctggtaacagaagcttcagagaggccgaggtagcgtacctttccttccttcaccaggtctgccatggcgcctaccatttcttccaccggcacattcggatcgatgcggtgggcataatataaatcaatcacatccgtttgtaatctttttaagctggcttccacggctttcttcatgtacgcgggtgaaccatcgaactgcacggcgccgggcgaagcaggcgaagaagtgaatccaaatttggtggccaggaatattttgctgcggttaggcttcaatactttcgcaatcagctcttcatttttaccggcagcatacacatccgcggtgtcccagaaattgatcccgatttccagggctttttccagcgtggcaatggattccacgtcgtccggtgtgccataggcatggctcattcccatgcagcccagtccaatggctgacaattgtacgtctgttgttccgagtgttctgtacttcatataatgtaatttcgggttgctgtaatacaatgaggcaaagataggcggcgtaatacttgtatagttgtaattatgacagtattaattgtgcaaatcaaagataccccctgcacgaaaggtaccgaatattcgtatttttaagacccattatgaaccacgataaacaacatcagttagttaccgcattcagcgttaccgatatcaccgactggttttgcgatgatatccggttaacgcataccgtttcccgttacacaaagcccgataaaatccgtgccagcaacgataccgatgtggtacgcctccattttggtatgaaaggcgattatgctttttcgtataaacaactggaccgttcttttgacctcatcggcgggcatcataatattatgtattcaaatggctttgagatcgaaataatgcccaaagccactgagatagaaacattcgggatccagttctccaaaaaacaattcctggaatttaccgaaaacgggaatgaacacctgcaacggttttgtgaagccgtgctgagtggaaaaagcgtattgctgtctgaaaactggggccctattgacgcgggtattcaacaggtaatcagccagatactgaactgccgttttacgggtcagctgaaaaaattattcctcctgtcaaagagtattgaattgctggtgctatcggccgaagcatataattacaccgcgaagaaagacatctttataaaaaataaaacagataaagaaaagatcattgctgtcagagacctgatcaacgaccggcttagtaacccgcctggcctcagtgaaatagcgcaactcgtaggactgaacgaatataaactcaaacgcggttttaaagaaacatttaattccacggtgttcgattatctcaccgggcaacgcctggagctggctaaccagtacctgcagggaacacagaaaacatccgctgaaatagcctatgagctgggctattccacgccccagcattttaataatgcttttaaaaagaagttcggggtcactcccaattccgttagaattaatccgtaaaatgcaatcgggcggaacagccgttgcttaatattgtactatcaaaaacaatgtattatggacaagcagttaaaactttcggaaagtaccagtatcaacgcgcccgtttcaaaagtatgggccgccatcactgataagaccctgatcaaacaatatttttttggaacagatgttaccagcgactggaaagtgggcagtcctgtgatctggtccggtgaatgggaaggacaacactacgaagaaaaaggcgaagtactggcgatggagccggacaaaaaactatctttcacctatctgagttccggcaaagaagataaaccggaaaactattccgtcatcgtttataccctgaacagcaacggtaacggcgctaccggctttaccatcacccaggaaaattttgaaaaccaggaagcctgcgatcattcgcgcgacaactggcggcaggtgctggccggcctgaagaaggtcgcagagagcgtgtgatgcggattttgtcttggctcaggattacgctgattatactgattacctggattttattcttttggattttataaaggattaagggagatagaagcggatatattcgctcttatctcccttaattattattttaagaaaatctaaaaatctaaaaaaatccaaaagtaaaaatccaggtaatcagtataatcagcgtaatcctgagccaagacaaaatccgcatgaacaatccgcggacttccgttgttctaatatcctgacaactccgccaaacaatctaaaggtattacgtatgaaaatcttaagtactttaatcattgtattatttgtttgcatatcctccattgcccagaaaccacgtgtgatcatcctggctaccggcggcactattgccggggaaggcgcttctgccgacagggcggcttacacggcaggtaaggtgcctattgcatctttactgaaagcggtgccgggtattgagaaaattgctgacattaccggcgaacaggtagcgaatgtaggcagccaggatatgaccattgatatctggatgaagctgaataaacggatcaatgaaatatatgcgaacaacgaagccgatggtattgtgatcacgcacggtaccgatacgcaggaagaaacggcgtatttcctgaacctcaccgaacgttcggataagccggtggtgctcaccggctccatgcggccttctaccgctatcagcgcggatggccccaaaaatttatttgatgccgttaccgtggctgccagtcccaaatctgcgggtcggggtgtactgctggtatttaatgaaagcattttcgacggccgtgatgtatcaaaaggaaatacaaccaaagtagatgccttctatgcgcccaacctgggaccattgggccaggtgtacgatggcagggtggcctattaccagaacgccatgcggaaagcaaataaagcaaccccttttgatattgccggcgttacctcactgcccaaagtaggcatcgcctatatgtatgcagatgcagacccggtagccattaataattttgtaaaagacggctacaagggaattattattgcaggtgtgggcaacggtaatttcaacaaagccttttacaacgctatcgacgaagccataaagaaaggcgtggtggtagtgcgttccagtcatgttggctccggacgcgttacgcaatacgatgaagtagacgacaaagcgctgggtaccattgtgagtgatgacctcaacccgcagaaagccaggatcctcctgatgctcggacttaccaaaacaaccaataaggatatgttgcagagttactttttcacctattgacccgaaaacatcattttatgggactgtcgtatatcaaaactaccgtggcagaacaacgtgcgctgcagaaattaagcccttttgaactgaaggatacgctgatttcactggcacagaacaccgcacagaagagtattgaagtaatgctgaatgcaggacgtggtaatccaaactggaccgccgccacaccacgggaagccttcttcctgctggggcaattcggtattgcagaatgccgtcgtaatatgcccgaagagcatggatttaccggtgtgccggagaaaagcggtattgccgatcgtttcaagagttttctggccctgcataaaaatgcgcctggcgcagcgctgctgcaacaggcctatttatacggacaaaacgtacaccagtttaacgacgatgcctttgtatttgaactggcggaaagcgtgatcggcaatgaatacccggtgcccggccgcatgctggcgcacatggaaccaattgtgcatgattatattgttcaggagatgtgcgggggggaaaagcagaaaggcaaattcgacctgtttgccgtagaaggcggcaccgcggcgatgtgttatattttcgattcactgatgcagaataaactgctgaaacagggatcaaagattgcattgatggtgcctgtttttacgccttacctggaaataccggaactggaccggtaccagtttgaagtggtgtatatcaacgcaaagggcgaaaccaaagaaggccggcatacctggcagtacccggatgaagaactggaaaaattaaaggatcccggcatcaaagtattgttttgcgtaaaccccagcaatccgccatcaagggcgctggcgcctgatgcgctggataagctgtcaaagattgtaaagaaagataacccccatttgatgattgtaacggatgatgtatatggcacgtttgtgaacgggttccagtcgttgctggcaaaaattccctacaacaccatttgcgtatactccttctccaaatattttggttgtaccggctggcgtttaggcgtgatcgctattcatgaagataatatctttgatgaacagattgccgctttaccggctactgcaaaaaaagatctggcaaagcggtatagtaccactaccttgcacccggaaaaaatgaagttcattgaccgcatggtggccgacagccgccaggtggcgctgaaccatacggcgggattgtcgttgccgcagcaaacgcaaatgactttattcagcctgtttgcgttgctcgacaaagaaaacaattataaacaggtagcgcaaacgctggtgcataaacggctgaagctattgtgggataagctggaacaacagcagctggaagatccgcttaataccggttattattctgaaatagatattgcatcctgggcatcgaaaatttatggagatgatttcctgaaatggttgcagaaaaaaatgcagcccaccgacattcttttccggctggcagaaaaaacagcgatcgtattactgaatggtggcggttttgcgggccccgaatggtcggtaagggtatcactggccaatttacctaccgatgcttatacattgataggagagagcctcactgaaattatgcacgaatatgtgagcgcatataaagaagaaaccggtaaaaagtagctttttttcataatgatagatgtacggcaggtggcattgcaagggctgcctgctgttttttttatgatttggtaataagcggggaattggtcaacttagcaggtatgaaagcacccaaaaacgcatggcgtatatggctgttatgcctcctggcattttgcagtgtatctgtacacgcgcaacattatgttcccacagacgctggttccaaagtacagtttaccattatcaatcacctggtttttacgtctacggtgaatggctatttcaaaggattaaaagggagtatccgttttgatccgcgtgatctgaagtcgtcgtcaataaacgctaccgtggatgtaaataccatcagcaccggtattggtaagcgcgacagggacctgctggaggagaaatattttaatgcggcaaaatacccggtgatgaagatcgtttcttccgccattgcagccacagacaaaccctctacgtaccagctcactgcggcgcttaccatcaagggaattactcggaccatcacctttccgtttacagcagtagtatctgcggaagcggcgcagctgaccggtaagtttactattaaccggaaggacttccaggtggggccggataatgccatcgatgataagctcacagtaacgctgaatgtacaggcaaaaaaacagtaacggtgatacgccgtgtgcccgtacccgggtatcatcgttaccggcagccgttacaatggttgcgaaaaatggtgggcggagatacggaatccctgccggtgatacagccggtgcgcaggatacagcccgtgtccggagtccagctgtacagaacgcaatccttcacttttcgccagcgcttttatatgatccagcaacagggcagcataaccccggccctggtattcaggaaggcaggccagatcatctatataaattgttttcccggtaaatagcttgttcatatgacggaagcctgcaaaggccgccactttggaaggatcttcttctgccgtgatatacacaatttcatacttttcagattgcatttctttcagctggggtaacagctgttcccgttccaggaagggacggagaaaaagaatgacttcactgcaggcctgcaggtcggcttcactgcgggcagtttttacagacaccatatcgcttggtttaaatgggcttattgaggaatgcgccgggtggtaatcccgatacggtcccacgcgttaataatattcaccgccatgatcagctgggcagtaccattcaggccaaatgcggcaagcgctttttcataggtttcatcagtaagacctttttcgctgatgagcgtaatttcttccgtcatagccaggataatcctttcttcttcggtgaattgcggtgattcacgccatacggggagcagcagcaaccgctgcgtggtttcacctaaattaagcgcatccttgctatgtttatttacacaaaaggcgcagccattaatctgagaggcacgtattcttatcagctcatgatggagcggggcaatgccggtagtagcgagatatttttccagtccgagcatagcggcgtaggcgcctggttccgtttcgttcatcaaaaatctggttgtcatcgtcaattgttttgtattaaaaatgatccacaaatttaccatcaactggagtatcttagtagtccactttgtaattgttaagtagtccagatgctgccatttaaaacgctcatacaaacagataaaacgctgaaattgccggtgtaccagcaaattgccaaccggctcatcgggcttatccaggaagggatcctgaaacccgggctgttcctgccgggcagccgggtattggcgttgcagctggaggtgcaccggaaaacggtgattgcggcttatgatgagctggtgagccaggactggctggtggcaatgccgcgcaagggtgtgatggtggcggctaatttgccggtgatgaagcccaggacctaccgggacgctgcctctccctatgaggatgcagcagcctttccatttcacgaggttcctaccatcacattggcaggtgtgccgccggctgccggtacgctgatcatcaacgatggtttcccggatgcgcggttggcgccgctggccgactgggtaaaggaatgccgctcggtgattgaaagtccccggtatgccaagctgctgatgtatggtggcgctaccgggctggaatcgctgcggaagcagatgctggagtacctttctgatacacgcggattaaacatcagtatgccgcacatcatgattacccgtggtgcgcaaatggctatctacctggctgccgcgttgctcattaaaaaagatgacctggtaattgttggtagtccgaactatttttttgcagacctctgtttcgaacagctcggcgcaaagctgctgcgggtgccggtagatgaagaaggtattgatgtggatatgattgaacaactttgcagcaagcgaaaaataaagatgctgtacctggttacgcatcatcaccatcctaccacggttacgctgagcgcagcgcggcgaatgaagctgctggctgtgatccggaaatacaaactgcctgtgatagaagatgattacgactatgatttccactacagctcggcgcccattttaccgctagccagtgcagatcatggaggtaacgtcatttacatcgggtcgtttaccaaatcgctgggactatctatccgaatcgggtttatgattgctcctgcggatttcattgaggccgccgccaacctgcgccggctgatggacctgcgcggggataatctttctgagcaggcattggccaacctgcttgcggatggtaccatagagcggcatcttaaaaaatcaaataaaatttataaagaaagacgggacctgctttgtcatttactgagcaccaaactcggcgacgcagtaaagtttacggttccttccggcggaatggctatctggttgcgcttctccaaaaaatacccgctcaaaaaaatcgctgcaaaggcagcggaactcggcctgcacatgacaagcggcgggcaataccactatggcgctgcatcgcagaatgcgctacgcttcggcttcgcttccctcaacaataaagaaattgctgcggtggtggcggtgctcgaagaggtgtgcgaattttgtcttggctcaggattacgctgattatactgattacccggatttttacttttggattttataaaggattaagggagatataagcggatatatttgcttatatctcccttaattattatttaataaaatctaaaaaatcccaaaaaaatcaaaaaagtaaaaatccgggtaatcagtataatcagcgtaatcctgagccaagacaaaattcgcttactggtcgaagaactgcctggtgcggttaagccggagatctttcagcaggctggctttggcgctgatcgtaaagctgaactgccggtaggtaccgaagggaatgaggttgatggagagattgaagtcgtgcagatcccgcgagatatacatgttggtgtaggcgatttccatgttggtaaaatcgaagccgctgttcaggccaatcttccatttgggcgtgagactgaagtcgccgttaaaacttacatattgcgtgatacgtttcactacgcccccggagtcggggatgatggtgttggtatacgataggctataagaaagatctatgcgccaggggatatcgaagtccacgtattcaccgggattgttgcgtatttgcgccagctggcgttgttgcgcggcaaaggcggcgtcgccaccctggacgttttggagggaatccattgtttgttctttggcggcgccctttttatctttcgattggaaggaggtgctcatggaaatgctggcgttggttaaacgacccaggctgatttttccctgctgccacacgtatttatcgatgcggcggccgcgggcatctacctggtaggggtcgagattgccgctggcggagatgttcagtttatcgaacaggttggtacgggcgtataagctgaaagtcgacaacttaaaggagtcggccaccaggttgtagctgccgttgatgccaaaaccatccagtagttttattttcttttcatggcgcccggtcgtatcttttttcgagaatactttcatctccaggttattatccagtccgaagttaatacctccaaaagcaccaggggaaggtaccccgatgatggctccgtcgaagtcggataccatttgtttatcgccttccttgttgtattgcagctcatggtaatattgactggaaaggtccgggcggtagctcacactcatggtgggccgcatcacatggcggatggctttgatcttcgagtttttgttaaaggtgtacataccgtacatggcagtagacagtgacatgctggcgctgatgtcgcgggcactgtaaaatccgggaatgtaggtggtatcaatagcgccacccgcggtatccgatccaaggttctttttattgggatcccatttgcggacgaatttcttggtataccagtattctgtatagttaatccctggtgataacgtaaaggtttttttaaacaccgggatagagaatgagatcgggatattgtgctgcatgccggtttgcatggcgtcaaacatggcttgtttaccaaacagggaatccttgaagttagcctggttgcgcaggatagtattatatgagatcccgatcttttcgtaccactttggtgtgcccaccatttcctttggctggaaaggatagatcgtgttcaccgtgaaagtggcgtccgggaaggagatagacacatcacgggtgctcaggttctgggagtggttcaaccccatggtgaggttgtagggcttcccctgccaggttttggagaacgtaatagacgacccgatgttattatttacacgtgtgttgtaatcatacacgttgtacttgttataggaagaggtgccaaagttcacggcagcgccgaaatttacaccggggcgtgctttgctgtccatgctatggttccaggtgacccggaaatctttggaggtactgaactctgatttcacttccggatcgccgaagcgggtgttggcaaagtcgaagttaaagccgccgttgtatttatagcgtttccggtaagtgggactggctttgatgccccagctgccgtacgagtagaggtctatccgcgtggtgaggtcgaagttgtcgcccaggccgaggtagtacccgccgttttccaggcctatccctttctgttgattcaccacgtactgcggcggcagtatcccggagcgctgaccgtgggtgatggggaaaatggcgaagggtatatacagcggtgtgggtatgccttcaatttccaggttagccgggccggagatcaccagtttatcggggatcacttttattttgcgggcgcggaattggaagtgtggggtatcgagatcgcaggtggtaaaagtatttttaaaaccgaagatggtattgtccggcatccgtttggattgctggctggtgataaatccttctccgtataccgacctggtattataaatttttgctttccgggaggtaatattaaactgcatggtatcagattcgaagctctggccgttgtctgtcattacggggcggccaatggctttgccggcggtgtcggtcattttggtggcttccaccatcccgttttcctggtcgaagctgatacgctccgcggtgatgttggtttctttatatttggtatcgccgctaccgtacaggagtatacgttttttgggtatctgcattacgatagagtctttcgccttgtaatggataggagcatccatgctatcgggtgaggcgatgggcaaagtatcggcagggaggctgtccaatgcatccggtgaaacaatgagggccgtatgaggtacgcctgcggcaataagaataagggcaatcagtaaaaccgaaagtagctggcaaagtattttcatgtatgcaattggatggcatccgtggagcgaaaatagtaccggaatggttacgtttgcttcgtgtaactggttacaaaaaggatagtgacggggaacatttaagcaaaagggaatgcagatcagccgggatggctgtgagagatattttggaagctgttggtggaaagtggaaggggttgatactttaacattttattttgtaaaggatcgcgcggattttgtcttggctcaggattacgctgattttactgattacctggatttttacttttttgattttttttggattgtttgattttcttaaaatgataattaagggagataaaagcgaatatccgcttctatctcccttaatcctttataaatcaaaaaagtaaaaatccaggtaatcagtaaaatcagcgtaatcctgagccaagacaaaatccgctgcgatcaccctaataaaataatcctcgtaataaatttttcttgtcgtccagtggtggctttgatgccaggaacgcagacatttgctggctgctcagcactgtggcaagttttgttttaaagtcgttgaacagggcgggctgctgctgcctgtaaacgctgaggtcttgtttgtttgccagcgccaatgttcttttggcgtcgaggtagttcaggattattttatttacctgtggtttttgtgtatcggttactgaaatgtttttcaggtagatcatgctataatcggtattggcccttgtttgattatagccttgttttacctggttcaccggcgacaggttactctgttgggcctgcgctaatttgccgcccagtagagttataacagctatgaagaatatctttttcatctgataaaatttaaataataaaattactggtggttccatgttatccatcccagggcatcgccggcagttaccatatccatggtagttccatctgctttacgaacaatgtaaaaacctgcggagttagcgaaataagggggtgctgttttcccggtattaaaaacattgttggtagcgataatgcttggcggattcacgatcggatcgccgccgtcgagcatttcgaaagtgaggcggccgccgctctgtaaataggggtatgccactccgcctgcaaacaggtaaggataaccgttggtggctcctacgaagaagggcgacaacacatcatagaaatcgccaccacctgcgtctaccaggccggggtagtatacataccggtaataggtacggccgggaaaggttagtccccggatattgtaagcatcatccactccgctgatatggaagcccggaacggtgagccaggggttatcgaggccttcgttgtagaaagccagtgcaacgcctggttccggcgatatgggcgccagtgccggcgaaatggtagccggcgtaccgttgacgctcgcgctgatagtacgcgtaccagggttccagacgaggttgtcgagggatttgaccgtgagtccgccgatggtaacgggttcctgcagtatgatgctgtgcggtgcaaactggcagcccacattggtaatgttttgactgccggctgttttaatatcaaatgatctgccgccaacaccgggagttatttcgaagacaacgccaccggtattcacccgcttgaaatattcgaggattttattgaaggtgctgtaagaaccgaatccattggtattaaacaaggtttgctcggcttgtgtggcttttaccatcaccgcttccgcctgattcaggttacctttcaaacggatggtgtcgcccagttccgctgcggcaacgttatctgcaaaagcaaattcaaaatcggttccccatccgaaccctgatccaaagggactgttagatatagcggcatccggatcgcagggcagatgaacatagctgtaggtatcaaagatcagcgtaggacgctggttagctttgatgcggtagccggtattgttaaaaacagtggcagctcccatgttaaaatccgacaacatcgatacctggctgtttttgtcgaatttcatatagtaggagaacaccgctttaggcccgttgcgggtaacgccgccattggtggaggtaccgttggtgaattgggtaaccacccatccatagggagcgtctgtaagtttttgctgataggtggccagggcctgtgctatccttacatctgttggtatcccgtcaatattaaggtcagatttcctgtcgcacgcagagagcatcactgccaggccgaggaaataatatatccatatctttttcataaataataattcagggtgatcaacaattattgataataggcggccagtgctctgcggcatttgcgttgcagggcgtaaaagtcgatggaccacgaccgggcgaaataatccactaccgctgcttcttttgctttgatggcctcatacccgggtgttcccggaccatctgtctgatcggccagtattttctcatagtcatcatacccatcgttgccattgtcggcgcctatcagcagggaagcgaccatttccacgaaatcttcgttggggtccgactctgcataagcggtaataaatccgtccatccgcgcttcctgatcggcgatattataccagttgccggtgtatcgtggtgtgatctgtttaaatgaaggaggaaccacgatattctgattcaggatatgaccaaactcatggtgcatggtatgtcccatccgtttcagcgtattggaatcttttgcctgcgccgtgaagttattaaactcgaacagcaccatggaagtgccgccttccgcctggccgagaatgatggaaccgttgctcaggtattgtgcggaccctgccactttaaacgttttcggcaggtatcttctcaggaaaacgttgctgccggtttgttcgttgtaaggtctgaaagtaacggccagcaaagcttttaatgccgggatcattttctctgcctttggcggcacaatttcgtaaggaaagtccagctggccgggcagccatttatagtaaacggcgatgttataaggtaccgtgaggctatcatgtataaaaatatcttccggtgtgttggcggtagagtcgccgccaagtccaaccgggggagtggtgaggctcaccttctctttcttacaggcgcttcccattagtagtagcaggaagatgccggtgattatctgtagtttcattggtttcattttaaaaggtttacaacagatgaattatctcgggttcaatgccataccgtcgttaactgcttccggcggtagttgtaacaatcttcgtttatcgccgggcgccagtgtcgtgttaaaattaggcgagccggtatgtactaccgggatatcaagccggaggatatcgaaccagcgtagaccttcctgcatgtaagtaacccttttcatatagagtgtagtttcaatcatggatgcgtcctgcggcaggccatagaacgacatcatttttgcgatggtgacgttgtgccgggatggactgtagccagaaatatttttgctcacccaggtattcatatccgtaacagcggcggtgtaattctttaagcggatattcgcttcaatcctgttcagcagtacttcatccatgctgaggagcgacatcacagtaacatccgacttaaatttcgggaagttaaaatactgcgggccggagccatatatagacatcgccaggttgccgccggtcacattgtccgacaggaaatattcctggttaatttcggtgcctatgccatagcggtagctgtagtagttatcaggatattttgtgccgggcgcttcctgcagtaaaatattagcaggattggatgcgtggttgtagtataccaccatgtcatcgtacgacatgccatagaatgcgtcctggtcacggatcaggttagccgggttgacgctgccaaaaacagcggtggcatgtgcaaccactttggcataatcccttttgaatagataaaaccttgcggcgaaagcatttgcagcctggcgcgtgaaatggtatttaggcgcattggcatacagctcatctttcagcaggggtaaaccagtggtgaggtcactttcaattttctggtataccgccgctacattgctcctgtcgtatttattgaaaacggaggtgctgatggtggtcatgtagggcacacccggatcgttggcggcagtggccgggttatatgctttggcaaacagggttaccagcataaagtgtgcataggctctgcataccagggcttctcctttttgcgcggaataattcgctgagtccgggccgttgcagtaagacaatgcctggttagccaccgcaatagcggcatagcaggaatcccagtaggcaatgggcccatcggcagaaatatcatctgcatcctggtatttaaaagtttgcgtattgatctggaaagtttgcggatcaatacctacgccggtgttgcctttgtcttccacattatcgctcagcgcttcacaaaacaacatgtaactcgcatgcggataggcggtcgtgagcagctgggttacctgctccggtgaggtgatcaccgtcctgttatcgggcagtgtttcgaggtacttcttacagccgggtaatgttagtacagcggcaaataagcctatatagatcagtagttttttcataatgaatactttttggattagaggcttactttcagtgaaacggttacctgtttgttgacaggcattgctaccccgccggtattataaaattccgggtcctgcccatgcaggcgttcgtcggcgtagataagccataagttgtttcctgtagccgtgagtgatccgccttttaatcctatgcggcccagcaatggcgcggggatctggtaactgagggtcactgattttaatcttacaaatccaccatctgctatgcggtcgctggaaaaattatagttattatatggataggctgtatttgacagcagatctgtttgtgtatagatgtctgccacagaggggatattggttttcttctcatctccgggtaaactccatcttcctttaaattcatttggcagcgagttaaaatcggtgtaatcggtagtgtataccggtgtaagcctgatcttatttcctgcctggtaagtaatgagtgcgctgagggagaaatccttataccggaaggtgttgctccagccgccggtaatggtcggatcggcggggccttcgtacttcaggtatttcacattatgactttgcaggtacacgccggacgataccgtgccggtgtcgttgataaagcgtgccacgccggtgtatgggtccagtcctgcgttttgcagggagaacagtccgcgtacagggtagccttccagtgcgccgccaccttcacccaccaggtcgaagatgaccgggttgtttctggcattggtgataagggtattattataactgaagatgaacgtactcgtaaggcctacatttttttgcgcgatgattttgccggtaagggctacatccacgccatgtgatttcatatcggcatagttggcgaattgatttacctgtccgcctacgccggaagttttaataagaccgatcaggtcaaaactttttctccggtagtagtcgaaggtaagtccgagtctttcatcaaaaaatcccatatccgctccgaggtccagttcatattttttctcccaggtaagatccgagttttcgagcgcctgtatgaggatggctgtttgctgatctacgagatatggccgggcggtaacaaaggaccgcaggatagcggtggtattggtagcggcgccggtgctggcgttcaggccatagctggctttgagcatcaggtgactgaccgcggaagagtttttaaggaatgcttcctggtccacattccagttaccggcaacggtccaggtaggcagccagcgtgcactgggagagctgccaagcctgttggaaccatcttcacggacggtggcctgcagggtgtatttacttttataggtataactggcattggcgtaaaaggcgatgaaccggtcgaagtcgttgctcacaccatagtaggtttggtttttctctgtcatttttttgatgaagagataatctacaaacggtgttccgccgctgttgtattgataacccacgcctacgttgttggacgtctggcggtcggcatattttacttcctggccaaccagtgcggatacctggtgttcatcgtcgttgaacgactggttatagttgaactggttacggaacgtatagtttttcagttccacatcatttctccggtaaaatcctccgtagggcagtactactacagccgggtcgttggggaagtcggggtttttgtagagaaatggattccgctgattgatgatgctgttgccattggcgcggtaggaattggcttcattggagttttcatttgatttatgctccgcacttgtccgtgcataacggatggcgccggtaaaatcataattaaagtggggactgaatttataattcaggttaccctgtaatctgaaatcgatgacgttaaggtctgtaaaattattcctggtttcttcaatgatgttgaagggggcaaagtttcgcgtaaagtattcgagttgaccgttttcatcgtacgccctgagtgccctgctggtgctgagtgcgtaggagaaaggattgatatcgaagtccctggtataggtgccctgtactttgtcagatacgcggtcttctgtgcctggtgcgcgttgctggcgtacgttaccgttgatctggaggccgtagcttagcttattattaggtgtatagttggcgcgcatattcaccgtatatcgcttcacgttgtctgcaatggtccatccggcgtcgttatagaagctggtggaaagatacagttgtgatttttcgttgccggtggacaggctcagtgagtgttcctgggtgagggaattacggaacaggatatcgaaccagtcggtgtttgcgttggcatattgcatgagccattgctgccgtgcttccggggtgttcagtaccgaaaatttatcgctgccatcgggatattggagcaggcgccccagttttccgtagatgcccgacgtacgttcgttgatctgttcggaatactggagcagttgtttacgttccagttcagcatataccgacatctggtcggcggagttcatgatatcgtagttttcgtaggagggtttcagttgtacgccgaagttgccggtatacgccactgccgccctgcctgccttaccttttttggtggtgataacgattacgccgttcatggcgcgggcgccatagagcgcggtagccgccgcatctttcaggatatcgaacgtttcaatatcgttagcattcagtccggctacggcagaccccaggagcgtattgatattaccgctggtgagctgttcgttggaaacgtttacaatatcttccagtaccacgccgtctaccacccacagtggcttgttttcaccggagatagaagtagcgccgcggatacgcactttaggcgcagaaccgaatgtaccggaaacgttttgcacgcttaccccggcagcacggccctccagcatacggcttacgtcctgtacgccgtctattttcacattatcccctttgagggtaacggcagcgccggcaaatttcttacggtcgatattctggaaaccggttactactacgcctcccagttctgttacatcttcttcgagggaaattaccaggttgttggtggctcttacttcgcgggttttatagcccacggcagatatcacgagcgtggcgccatccggtacttcgaggtcaaatgcacctgcggtgttggtaatagcgcccctcgtagtgccttttacttttaccgaggcgccgggtagtggttctcctttgttgttgcggatgattccgtgcacaggtgccgcagctttgacggtttgccgcagtacgccgggagggagtttttccagggaatccctggcgcttgcctgcaaagaaagcgcgagcagaaaaagggacagtagcttcatagttaacagcgatttaattgaatataatccgggcaatgtagggtagggaaacgcacccagctttctacatcttttggttgaatgcatatgaggcaataagggtttaatattacattctggttgatatcactatcgcttcccggcagtattgatgatggctccgacttgataaataaagcaaaaacttaccgggtatcttatcttcttcagtactttatcatagtgtataaggctaatttaactaaaattattataccatcaggagcaaaaaaacaggaacggttaatttcgtcccggcaacggttgcgcattttgccgtaaacgatttttgctgtattttgccccttcttatgaaactaatcccattattccaacatcatgcatgataatgaattatggtactcctataaagaaggagatgtaaaagccctggaaggattatatgaattgtattattccccgctcacgaactacggatttaaatttacgcccgataatgtatgcatagaagaaagcatgcaggatcttttcctgaagctatggcaaaacagggagcgtattgaaagtccggcagtggtgaaacagtacatgtatctttctttccggcgtatcctgcttcggaagctggattataatccttcgcggcatgaggaagagctgagtggagaacatattccttttcaactggaacttatcggcgggcatccgatggtgaggaaagagcgtatggaggaacttactgccaaagtagatatgttgctctctattcttactaaccggcaacgggaggcggtattcctgaaatactatgaggatctttcttacgaagagatcgctgacattatgcacatgaatgtagtgggcgcctacaagctgatatatagtgcgctcgaaagtttgcgcgaacagtttggcgacttcactttactcctgatcctttacgttttaaaacgggcctgagaattgaaactaatggataaaaaaggaagtgtcacttttttatttttggtcgttcggtgttgttatcttttttaaaacttagtgctgggtacattgtaagttgttgatattcaatatgttttttatttttcgttgatttgaattataattgcataaatgatctcagatgaaatcagacaaaaacttcaaaatatcattagaggagatgtcctcgaagggcaagaagatcattgcacaacaatcagaaatctccttgtccaaagctttggctcaagtccgactgttaaaggagaattcgaaagtcgctcaattctcaaagaaaagcaggctaccttcctaaaaactcacgttgaaaaaaatggtggatggctaacagccctaccaaagggaagtcaatatttaacccacggaggtgaagccaaaatttatcttgcttcagatcaaagacatgtaatcaaaattaatgatgctgtttattacgctacctggttggagtattttaatagtctggtaatccataatatactgtttcctaataccgcctatgagttgattggtattacctctaataaagatgcaccgttactcgctgtcctcaaacagccatttgttgaaggggagcaagcagacctgacagcaatcagggaacatctcacctacaatggttttctaaacaccaggcgacaggattatttcaatgaagagtttgggttgatattagaagacatgcatgatgaaaacgttatcgcaaagaacgacgtacttttttttattgatactgttttttacattatggcgaaataatttgtgaataaaaggctgcccttttgaaaagggactaaaaaagtatcttgaaacaaaaaaggtaatcggccatacggaatctggttttaaaaacttcatacaaatcaaataaaaaggggcagttcataaatcatgaaccgccccattccttttaagacagcttttttatgttaagctgttttgcagaaagcaatatgatcatgtacctgtggtattttctggtagccgttggtaagacctaattgcagatccagccagagaatatacgcgcagggttccattccggcggtagagaataccaggctgttgttatggtattccgctgctgctggtggtggtccgccgtggaaggacgccgggagtaccgggttgccttcaaagcggatggtgaatgcctcgatgtgcgggtgggcaatggtgtattgcgcggtaacggtagtggtgatgcctccgcaaccatggccgctgccggtagtttccccgatttccagcatggctgccgcgaggatattttcatcgccggtatagccccatcccgggtgtcttctttgtttataattcacattggacacgactattttctccaaggtgttgatagcggtgagtgtagtagtgccaacttttcttgcttcgaagataattttgaaagtatggatgcctgccctttgcgtaggtggtacggcgttgccggctacgagcacagcgggggcggtgagatcgaaattatcccttgcgaaggtggtgccggcggcattgagtgccagctgggaagtgttgaggatagccagtacaccattagtaggggtgaagataccagtggttaagttattgccgcgtggtaccgggatccacacttctccggcgccgttgatggccggggtaacaatgactgcgtcgtgcgtccaggtggtggggccggtttgtttcagcagttcaccgatcttgaatggcagcagggcgctgagtacctgtgtggcgctgagttcgtagctggtgtcggcgttgatgatgcggaagcggtattccatttcattggagttggtgccgctgggcagggtgccgttaagatcaagcgcaccgtagaaagaaagacgcggcacatctgtagtataaccctgtgcatcaaactgggcgccggtggggcctatgtcgtaggcgcctactctttcaaagagggcgggtacttcattattaggtgtgatatcatccggtacgcagagttctatgcagaagcaggggccgcggttggtacggtcggcgcgatggcccacgctgcggtcttctttcagcaatacggcgcccgatacgggttcggtgatgctgaaatagagatcgggtcctgccggccattccacattgagccagggcgacagcagcgtttggctgaagtcggccatggtataatctatccggaaatgcccggtggcatcggtgagctgactgccgagcgggtcgtcctggagccagtctacatcaaaagcggctacgcgcaggccttcgaggggtttctgggttttacagttgatcacgcggccgcaaatgacccatgcatcgtatttcgcgcggatgagacaccaccagcggttggggattacatattcccaggaggcgaagaaatcattttcctgtccgcgccaccgtggttggagggtagtgatatgaaactgcagggtaggcagtttgcccgggtaaggtttggggcgtggcacattgccgcattcgaagtcgatctcgaaggcttcgccttcatatttactttcccttccaagagaaaaggcgaagttgccttccgcatcggtgagggcttctgccagcaggttgccggctttctttttggcttcttctgcagatacttcatggaaggtttccttctctgcagcagtagcctgcaggacaacttcccgggaaacggcggcccggtaaagccggatcttaacattggcaatggcttctatgcaatatttatcgcacaggaggccctttaaattgcctttgaactggtagctcatgacattattttttggggttattttaaatcggaagcaggtgcttttggggtgttcttcactagaattttttggggactgtttgtgctgttataatggcccctgcttctttaacaaatctccacctaaattccttcgttatcaagaggataagtgcgggaaatgccaaatgcgtatatatcgcgcggtggcgggaatgcgctgataaatggaaaggtattttgggcatccgggataaaagcgcttattttgccggttaggtttggtagagcaacatgaaagaagatagcagcaattattccctgtatgatgaggaggatttggtgacagctttccaggtgagtgaggatatgcgtgcgtttgaagaaatctataaaagattctggttcaaactatacagcgctgctgtgaagcgcacaagttcccagcacgaggcggaagagctgatccagaccatttttgagcggttgtggaccaaccggcgcaaggtggtgatccataatataggcgcttacctggctgtttcgctcagaaatagcctgcacgattcccagcgcaggaagatgacggcagaaaaatacatggaaacactggacaccgatccattggtaaatacaacggaagaagatgtaaacagggagcttctcctgaaagacatcgaaaaaacgttgcgggagctgccggagaaaacccaggccgttttccggttgagccgttttgaaaataagtcggtccgcgaaatagcaggcaacctcgatctcaccgaaaaggccgtggaatatcatatcacaaaggctataaaactgctgcggcagcggctccgcggctatatgtcttccttcctgtaaaattctttaaattttttttaggggtttaattcagttatgcgtcaatgtaatcagataaactgattccatgagccaatatgaattcgatgacctgcttgaaaaatatctttcggggcaatgcaccccgcaggaggaaaaactggtattggcctggtaccgttcatttatcaacgaaagtgaaatagagatatctgcagaagaaaagcagcgcattgaaagccggatctggtccaatgtaactgccactgttggcagtggggaaccggaaacaccggtagtgcggatgtggccccggcaggtagcgcggttagctattgcgggctgcctcgtactggccgttacaggcgcctggtattggtggtcgcagcaacggaccattacgccaaggaacatatttacgcaggagcctatcccgggaggatacgtatccgttttcaatgaaacggacaacaaccgggaagtggtactgagtgacggatcggaggtgaggctggaaccgggaagcatagtgtattatccgcctgcattcagtggtcatacaagagatgtgtacctcagcggaaacgcatttttccggatagcgcacgatgccagcaggcattttatcgtacacaccagcgaaggagtgctggcagaggtattgggaaccagtttttatgtgagccacgacaaagtaagtcataaagtagaagtagccgtggtaaccgggaaagtatctgtttatgaacggaagaaaaagaatgatactttatttacagcatctgccaacagcattattattacacccaaccagaaggttacatataaaacagaaaataaccagttcaccacctcgctggtagatgatccaaagccggtaacagcagcggaaaagcagcccacgttcagttatgaagatgcttcgctggaagaggtattaaaggctttggaggatacttatgccattaccattgaaacagataacgggcaattcagccgttgtcattttacaggagatatcacgaaacaacatctatacgagaagctggacattatttgccaatctgttcaggcttcatatgaagtaaagggtaccaccatttatataaaagggaaaggatgtaattaatgaacatactataaaagtcactaaaacaaaaaaactggtaatgtggggcattaccagtttagtaaaattaaccgtttgccgcggttaaaatgcgctatgtccgcaaactttcaattaacgaaacaaagccacacaagttatgaaaaaaaagcgattcgctgccgtaatctactacgttatgagattaactgctgttcaacttattcttgcttccgttttttcactgtcgctgtacgccaataaggtgaactcacagtctgtgctggaaaaaccgatctccatttcggcagagcaaacttccgtgaggaagctgctgaaccagatccggacccagacgggcgtgaatttcacctatagcagcgatatggtggatgtaaaccggaaggtatccgtagagctgaaatccagacagctgaaggagttttttgatgatattttaaagcctatgggcatcgactttaaggtgatcgacagccagcagatcctgctgttcctcacacctgccgatggccgtcagaatatagtggtaaccggtgtggtaaacggtgaagacggtttaccggtgcccggcgctaccgtgagagtaaaaggcagcaccacaggcaccaccacctccccggatggtaaattcacccttccggtccccgacaaacaggcggtactggtgatttcgtttattggttatcaaccgcaggaagtggtggtaggagaacaaacgcacatcaccgtaaagctgaccgcagaaaacagtaagctgaatgaagtggtggtagtgggttatggcacccagcggaagaaagatattactggtgcagtatctgttgtgaaagcagacgcttttgaaagcagaccgattgtaagcgccgcagcaggcttacagggccaggccgccggtgtaaccgttaccgcgccttccggcaaacccggtgcaggactgaacgtgagcatccgtggtaatacctccctgaatgccagcaataacccactgtttgtagtagacggggtgattgtgccaaacattgatttcctgaatccgagcgatattgaaagtttctctgtgctgaaagatgcgtcttccgccgctatctatggcgccagcggagcgaatggcgtggtgctcgttaccactaaaaaaggaaccagccagtcgaaagtatttgtaaacgcctataccggcatgtccaatttcgctaagaaaatggatgtactaaatacagctcaatatcaaacgctgatgggcgaactgggcatcaccgatcccaataacctgaacaccgactggcagaaagaaacatttaaaaccggccgtgagcagaatatccaggtaggtgtttccggtggtaccgagaaaggacattactatgtgtccggcggttaccagaaacaaaaaggagtggtggcgccggcagattatgaccgttattctgtaagggccaacatcgataataaagtgaaagactggctgacactggcctccaacctgtcgttcaacagatccgtttacgtagatgtgccggataacagcggcgtagcgagaggaggcaccatcctgtcggccttaacatcaccgccaaccatcggtatttataacgcagatggcacctatacatctaacccaaataacaaaagctggcagaatcctatcgcctatgcttttgcaccacagcagaaagccatcaacaaccgtttcctgggaaatgtaagtgcggacttcaccatcctgccggaactgcatttccgttctaacctcggtgcggaatcggaaggctaccggtatgattatttcctggacccttattctactgattacggcgcgaaggaaaaaattggttatggtaaatcccagtcgatcgaacgttttgtatggttatgggaaaacaccgtgagctataacaaacagtttggcaaacacaatgtgggtgctatggttggtcataccatgcaggaatctgattataatttcaccgatgatattgccaaaggatataccagtgataagatacctacgctgacaggttccactatccgtgaaaaacaggaagtaacgaaaagtcaatggggcaaacgttcttacctgggccgcctgaattatggctatgccgataaatacctgttcaccgctaccatgcgatatgatggctcatcgaggtttgcacccgatgcacgttacggatggttcccgtctgtatcagcagcatggcgtatttccaatgaagacttcttcagcaaagacggtatcgtaaatgacctgaaaatccgtgcaggctggggtaaaaccggaaacgacggtatcggcgattacgactggcgccggctgttcagcagcaatggcaccggtggtttgaacttcaccaacctgccaaagaacgacctgacctgggagaaaactacccagagcaacgtgggtgtggacctgagtatcctgaacagccgcatcaatattaccgctgatgcctatatcaagaaaacgaatgacctgttggtggatatccagccacccgccagttccggctttggtacccaacgttacaatgtgggcagcatagaaaataaaggagtagaactgagtgtgaatgcactgatcatcgataaagaagtgaaatggaatgccaatggtaatatttccatgaaccgcaataaggtcttgaacctcggtcctacaccaagtttaggttatggagatgtgtatgaaagaggtaacgctatccgcgtagaaccgggtcatcccctcggtgcattttatggttacgtagcacagggcgttgatcctgctaccggtaacatgatttacgcagacctggatggcgacaagaagttgtctgatggtgaccgcacctggatcggcaatgcacaacccgactttatctatggtttcacaaatagcatcagttacaaaggctttgacctgaatcttttcttccagggtatccagggcaacgagatattcaacgccactcgtatggaactggaaggtttgtacgactccaagaaccagagtaccgcagtattgcgccgctggaaacaggcaggggatgttacagatatcccaaaagctgaaaaaggaaataccatcaacagtgcatcatcttcccgcttcgtggaaaacggttcttacctgcgcctgaaatcagctacgctgagctataaattttcaaatgacctgttgaaacatatcggcgttggccgtttgaatgtgtacgtgacaggacaaaacctgctgacatttaccaggtacaaaggactggatccggaggtgagcaaggatgcagccaacggtccggctatgggtatcgattatggaacctatccacaatcacgcgcctttatctttggtttgaatgctgagttttagtcttaacaattaattattccaagtatgaaacaattcacttcttatatagctaccggttttctcagcgtgtctttgttgtcatcctgcacaaaggatctgctggacaagaagccaatttcccagtcggaaactgccactgcagagtcgctgctgctgggcgcctacgataatatgtatgatgagtactacacctccgatttcctgaccaacggagatgtgtctgcagataatggttatgcaggtggtgacaacgcggcaaacttttccattgataagttcaccgttaattccatcaacggtaacgtgaaaagagactggaaatacctgtacaccgatataaaaaactgtaacctgatcctcagcatcacccccaccacggatgataaaggattaacacctgaacgccgcgaggagatcatgggagaggcatctttcctgcgcgcatggcattacttcaacctgatcagaagctggaaggaaatcccgatcatcactgctattccaacagacctgcaaagtatgtacgtggctaaaaagcctgcggaagaagtatatgcgctgatcattcaggacctggaatatgcattgacccgtgtccgtgataatccgcctgcaggtaacaaagggattgtggcgaaaggagccgtaaatgctttgctggcaaaagtatatgcacagaaacccaatcccgactggaacaaagtagctgcctactgtgatgccgtaaccgccggtggttacgacctggtgccggattttgctaccctgtttaccgtagcaggaaagaataatattgagtccatctgggaaacacaatttgatggtgttttacaccagaactgggtaacgggtatgaatacaccgtttatgtggggcgactggaaaaaattcaatattccttcgcatacaatcgtagctgcctttgatgcggaaggcgacgcggtgcggaaagcggccagcattaaatttgtgaatgtttcctggacggacgactattggaaacaaccggtcccggtgatctataaatacaacgacgccgatggtaaaagcaatacttaccgcctgcgttatgccgacatcctgttgctgaaagcggaagcgttaacagagctgaacaagctggataacactgccaacggcgcgcaatactacatcaataaaatcaggcatcgtgcaaagctgggcgacaccccggccaaaacacaggcagcactgcgcctggcagtggaaaaggaaagacagctggaactggcgtttgaaggccatcgctggtatgatttgctccgcactaaccgcgccatcccggtaatgaatgcacagaaagatggcaatggcaacaacctgaactacaacgtaactacggataaattatacttccctatttcgcaggacgaaatagacagcaatcctaacattaataagtaagtgcaattataaaaatgaaaacggaacaggagcctggataacaccaggctctttgtttaaataccctttcatatgcaaaaaatatttcgccctatattatttgccggcggccttgcgctggcactcttcgcctgctccggcagtaaaggcattacacaacccttaacaccggtagacaccagtggtgctaacggcgccacagttaactggtgggttaccaccggggatcagcaaagcctgttgaaacctggaaacgggcagccggtattcagtagccccaacgccaacggttatacgactattgaagtggacagcagcacagctttccaggaagtagatggctttggctatactcttaccggcggcagcgcgcagctgatcaatgccatgaatgccaccgcgaagcagcaactgttgcaggagctgtttggtaataccgctaacagcattggcatcagttacctgcgcatcagcataggcgcctctgatctgaatgccacgccttttacctataatgatgtaccggcaggacagaccgatttatcattgacgcatttttcactggaggcagatatgtccgcaggcacaggtttgatccctttgctgaaagaaatactgctgatcaatccgcagctgaaaatactcgcaacgccatggagcccaccggtatggatgaaggacaatgcttcttttaaaggaggcgtcctgcaaataaagtattacgaagtgtatgcacaatacctggtgaaatacctgcagcagatgaaagcagccggtattactattgatgccatcacaccacaaaatgaaccattgaatcccgacaataatcccagtctgaaaatggtggcggaagcgcagcgcgactttatcaaaaacaacctggggccggcctttgcggcggcgggaatcgccaccaaaattattatatacgatcacaactgcgatcacccggattatccgctgaccatcctcgccgacgcagcggccgcgaagtttgtgcatggcagtgcctttcacctctatgctggcgacatcagcgcgttatctactgttcatgctgcggcgcctgataaggccttgtattttaccgagcaatggaccagtgctaccggcggtttcgacggcgacctgaaatggcatataaaaaatgtgatcatcgggagcatgcgtaattatagtcgtactgcgctggaatggaacctggccaacgatcctaattacggtccgcatacccccggcggctgcaccgaatgcaaaggtgcgcttaccgtcagcggcagcaatgttacgcggaatgtggcctactatatcattgcacatgcatccaaatttgtacctgcgggttccgtacggattagcagcaacaatggcgggaatttatacagtgtggcctttaaacgcccagatggaaaaaaggcgctgattgtattgaatgataataatgcagctgcttcttttaacctgaagtaccaggggaagcaggtggtgcctgttttacctgcaggcagtgtggctacttttgtgtggtaatttttttttcggagttatgaaagatgatcagtttttactggtcatcttttttttgttaatcattttcttttaacctgttctttacggatgttttgtattggaaagatacatttgttggcatattgtttaacccataagaacctggtgaaaggcgggagctattggatctgcgccgggcggcggtcgaactgtttgaaatttactaagggatgtcattaaattgaatgaatgaatttggagaggtatgaatgtactgctgattctcaattcagtagttttacgtttgatagcataggtccgaacggaaccattagaaaggttataaattatgagcagattcctggtattttttacctgatggttctgctgtaaggaatttggcatttggtgactggaacgaagtggaggaaagaattgatgatggcattgtttctaataataatgacagggataaagtgcttgcaaccgttgcctccacaattatttcgtttacagaaaagcatggaaaaatacctgtctatgcagagggcagttctccggcgaaaaccagactatatcaaatggggatcaatgcccatctggatacaattaaatcattgttttggatttatggccgcattgaaggagaatgggaagtatttgagtcaggggttaattttgaggcatttctggtaattcggaaatagtcttatttttgttgataacaaatgtttgattatgtttttaaagtatgtaagaaagaagaaaaatataccttcaaatatcagggtttgtaatgctatgagggattacagcaaagaagacttttttatcaaaaaattggaagccgcaagaattgccattattaaatgggggcttcccaaagaattatacgttaaataatgcaactttcttcagattagagcatattcctacctgtgtccatttccgaacaccccctgtcttaaatccggacaaattatatttttaatacattcaattccgcctgattctaatacccctcgtcactggcattttcttcgcagtcatgtgcgcggtcccgtgagatagatatctttcaaaatccaatttcctgctgatgtttaaaaactatctcaaaattgcctggcgcaatctctggagaaataaagttttttcttttatcaatgtaatgggcctcactattggtcttactgcctgctttttcattttcctgtatgtacattttgaacttagctatgataagtttcatagtaagggagaccgtatctaccgcgttatctgtgacataaaaacgcccagcgaaatgataaaaagcggaagtacgccatggacgtttgggccgaacatgcagcacgactttccggaggtagaagcatttacgcggctaaaccgcgctaatttgctggtgaagaaaggtaacctgagtttccaggaagagcattccatgtttgcggattcgtcgatcttccgggtatttgatttcaaacttatttatggtaacccggctacagcgctgagagatgtgaacgctgtggtgcttagtaaaacagctgctaagaaatatttcgggaatacagatccggtaggacaaaccgtgcagctcaccggcgagctggtaccggtcacggtcaccggcgtgatggaagacatgccacagaattcgctgatcaaagcagatatgctggtgtcgatgtcttttttggtgagtagaaatccgcgcctcgatgactcgtggggcaatttcggcgcaactactttcctgctgctgaaacctaatacagacgctgctgcgcttgcggcaaagttcccggattttatagagcggcataatggcgacgagagaagaaaggccaaaatgctctataccgttttactgcaaccgctggagcagatctacctgcattccgaccggtcctcttttgagaatggcagtatcacgaatgtgtacattttttccgttattgccatttttatattgtttattgcctgtattaacttcatcaatcttaccactgcgaggtcggtagagcgggcgaaagagattggtgtacgtaaagtagtaggcgccacccgtgcggagctaatccggcagtttatcggagaatgcgtgttgttatgtttaatggcatttgtattcactattatattgtttgcagtattgctgccatcctttaacctgctggcgggtaaaacgatcagcaccggtttgtttgccaatgcctggtacatcggggcattgctggcggcagccatagggataggtttgctggcgggtgtatacccggcgctggtgctgtcgtcctttaaaccggtaacggtattgaagggccggttctctaccggtaccagaggcattttcctccgcaaaggactggtggtaacacaatttgctatttccattgcactgatcacaggcactattgtggtgtacctgcaaatgcattatatacacagtaaagacctgggctttaacaaagaccaggtgctggtgatcgatacacatggcgacccggcgaaacatactttcaggacatctattgaagatattccaaaagtaaattccgttaccatttcatcaggtatccccggcggggaaaccaatggcgcttactcagaaattcagaacaaacaaggcgatatgcaggtggccaacctggacctgtattccgtggattataattttttgcagcaatataaaatgaagatagttgccggacgcgggttttcccgcgactatggcagcgactctgcccatgccctggtgatcaacgaagcagccgcaaagctgtttggctacgccactcccgatgaagctattggcaggggctaccggcaatggggccatgaaggcactattataggtgtggtaaaggattttcatttccgctcactgcagcaggatattaagccgcttaccatccggatggagccgcaggattgcgaagtggtgtctgtgaatgtagccccaggtgatctgtcaggtaccatcgccgctattgaacggaagtggaaaacgctgatccctaaccggcctttcagttattatttcctggacgaattcttcgacaggcaataccgcgccgaagaacgttttggtaaactctttttcgacttcgccctgctggcgattattatttcttgtcttggtttactaggactggcttcttacagcgccatacaacgtacccgcgaaataggcatccgcaaagtaatgggagcatctgttacagatatcgtgaacctgttgtcaaaagaatttcttaaactggtattaatctcctttgttatagccacaccggtagcctggtattttatgcacaaatggctgcaggagtttgcctaccggatcagtattggttggtgggtattcgccgtatcgggcatcattgcaggtatcattgccattggcacaatcagctaccaggcgctgaaagccgcgttggcagacccggtgaaaagcatgcgggcagaatagcgtccccataccggcagttccggaaaacttttatcatcttatcatgagcgccctgctcctaggaaattaacgcgtttggaaatgccccctgaaggcaaaacaaaggcgaagaaaattgccattattttcgatggtgcacagccaattataatttgtattttgttccttgccgacgcattttttctgaaaaaatgcgtcggccccaatgatcagtccggcgttttgaaagaaaacagtccggagtagctaaaattccacttaattgcaaaaactcatgcgaaggaacaaacacactatagccgtttgcgttatagcattgctaacatcgctgcctgcattggcgcagcgcacagaactgaaactcaggtacgacaagccttcgggcaaaatatgggaagccgcattaccggtgggcaatggtcgcctggccgctatggtgtatggcaatcccggaagcgaactgatacggctaaacgaaaatacggtttggagcggaagtcccaaccgcaacgataacccccatgcactggctgcactgccggaaatcaggcaactgatcttcgatggtaaaatgaaagaggccagcgagatggcggcaaaaaatatccagtcagaaaaaatcaacggcatgtgctatcagccggtgggagacctggaactggtttttcccggtcatgagcagtacgccggttatgcgcgggaactggatctgcaaacagcggtaaccgctaccagctacacggtaaacggcgtaaagtataccaggcaggtatttgcttctataccggatcaggcgataattattcagcttactgccagtaagcccggcagtattacttttaacgccggcatgaagagccagcaaaaatcgaatgtagttaccagcgggaataatgaactggtgttatccggtatcagcggagacagagaaggcgtaccgggaaaagtgaaattccagtcgcaggtaaggtttaaaaccagcggtggtaaagcctccgccaatggtagcgccattagtgttgccggcgctgatgcggtaaccatctatgtgtctgttgccaccaactttgtaaactacgccgacattagcggcgatgaagtaaagcgcaccacggcgtatatgtcgaaggtatggccaaagaatttcgcaggtctgctgaaagatcatatagcggcttaccagcacttttttaaccgcgtacaactggatttaggaactaccgattctatcaaaaatacaacagatatccggttaagggatttcaggaacggcaacgatccgcagctggtaacattgtatttccagtttggcaggtacctgctgatagctgcttctcaaccaggtggccagccggcaaacctgcagggcatctggaacccgctcatgaacccaccctggggaagtaagtatacgatcaacatcaatacagaaatgaattactggcctgcggaagaaacaaacctttctgaaatgcatgagccactgatagaaatggtgaaggacctatctgttaccgggcgggaaacggcaaaagtgatgtatggcgccggcggatgggtagcgcatcataacactgacctgtggcgtataacaggcccggtagacgggatttattctgctatgtggccaatgggaggcgcctggttaagccggcacacatgggaaaggtatttgtttaacggggacaagaaatatctgcaaacagtatatcccgcattgaaaggcgcggcgcagttttacctggactttctggtagaagagccggtgcataagtggctggtggtatcgccttccatgtcgccggaaaatagcccgaaagcctaccccggcatatccatcgcggcaggcgccaccatggataatcaactggtatttgatctgtttaccaataccatccatgctgctgaaatcttacaaactgataaagtgctggtggaaaaaatgaaagccgcccggaaacgcttaccgcctatgcaggtgggccagcataaccagttgcaggaatggttgcaggacctggataatccggacgacaagcaccgtcacgtgtcgcatttatttggcttgtatcctgccaaccagatctctccctaccgcacgcctgttttgttcagcgctgcacgtacttcgctgctgcaacgtggtgatgtgtccacgggctggtcgatgggctggaaggtaaacctctgggcgcgtttgctggatggcaatcatgcctggaagctgatcaaagaccagcttaccccggtggacgtaagtaatgtaaagtatggtggcggcggtacttaccccaatctttttgatgcgcatcctcctttccagatcgacgggaactatggctgcaccgcagggatctgtgaaatgctgctgcaaagccaggatggcgccatccacctgttgccggcgcttccggacgattggaagaacgggcgtgtgagcggcctgcgtgcaaggggaggttttgaaatccgggagatggtatgggaaaatggtcagctcagtaaaatcaccatccgttccacgctgggtggcaattgccgtctccgcgtacccaatgcgctccgggaaaacggacagttgaaagcagccggtggtgatcaaaccaatcctttctttgaagtaacaccaacagctccggccctggtgagtgaaaaagctaaggtagaagaactgccgttgccccagacaatattatacgacctggatacacaggcaggaaagacgtatacttttgtaaagcaatagataattaatatactttgtacaggtaaagaccggtgggagcttctttcaccggtctttcctgtttgttgacatatggttttgaaaaaaaagtttactttcggggtatagcgccagagatcattcagcgcgccagcaatcagaccaactatcttattatttataagcgtcatttactaccggatttggaaaataacacggaatcactggatgtgcaattgattcttcggctacaggcgggagatgagacggcgtttcgtgaggtatttgaccggtttaatcagaaaatatacggcctggcctgtcatttcctgaaaaataaagagcagggaaaggaagtggtacaggaaacgatgcttcggttttgggaacaccggttaaagctgagtacagattatgccctggcgccttatgtttataccattgcccggcgggtcactttaaatatgttgcggcaggcggccagtagccgtgctgcttccatgaaactctggcaatctgttcctgcttaccacaacgatacagaggaagccatactgggggcagatctcgaaagggttaccgtgcagatattgaatattttgcctccccggcaacaggaaattttccgtctgagcaggtttgaagggctctcttatgaagaaatagccgtccgtatgaacatctccacccatactgtcaaataccatatgatggctgcgctgaaagtattgcgtacccactttaatgaagccgaaattgtttttggcttcctggcattctccctgttattttaaaaaaatattttttttgactacccgatagcccccctctgcgtgtattgcactataccggcttttttctgcccgggataaattgtatttcacgtggatgaacatcgtatacatcttttgctgacaaaactggcaggcaacaccatcaatgaacaggaatttgaagaattgatgttgctgttgcggcaggctgaatccgatgatgcggttcagtcgccattcgacaaaacctggtcgggacttacgcccgcctcgcagctgtcacctgtagaagcccaatcactttatgaccagattaaagagaacccccgtttttcggaggatgttcccgttttgaaaccccgtcgctggcttgcgtatgccgcggggatactggtgttgatcggagcaggtgtagcggcctggctgctcaccaaacctgccggacaacctgctttggtgtatgaagaagtattggcgcccgcaggcaagcgggtacgactggtactggaagacagcacggaagtatggctgaataacggcagtaaactgaagtacccggttgcctttactggtaacacccgggaattatatattgagggagaagcctgttttgacgttacccgcagggatcagcagccgtttattgtgcatagtggtgatgtagcggtgaaagtactgggaacagtgttcaatatacaagcctatcagcagtcgcagttggcggtaacggtggttagcggaaaagtgagtgtggcagcaggaactacctcattaggcatcttatatcccaaccaaaaactggagtatgaagcggcaagccggcaggcgaaagttgttacggtgaatgcagcatcattgctggcctggaaaaagggggagcttatcatggataatgtaacaatggagcaggctgccgccatcattgggcggtggtataatgtacaggtggaactggggaatgacgccatccgcaactgccgtttttctctttcttttttacacggggagaatatcggggaagtgatgaaaatgatctgtgagctcaacgggtgttcctggaagatgagcggcagcaacattattatcagtggaaagggatgttaacacggtttatttattcatcactataatcatgtaccatgaaaaaattccacttcaattagcccgtatagcggcaaaggaattacgttatgaaatcagtttaaaaaagtatcgccgtggaggcaaccacgacgatacctgaaaaattggttacaggtacaggcaagtaccggtaaccggatggtttttaaactcagtatgtcaaccgattaaaaccaaacaaatctatgattttttcagtaagtaagggacggatgcgcccttatgagcgtcttatcctgaacaaaacaatcctttggattatgagatgttccacgataacactggccatagtgcttttttgctgtcagctattgatggctggcagaacaaacggccaggatatccaccagacaaaaattgcactgggtatttcgggcaaaagcctggaggccacgttaaaagaaattgagcagcgaacagatttccgctttggttacagggccgcagaactaagccgtaccggcgaggtgaacctgcccgccggtacgcggacggttgccgccacgctggatctcctgctggcaaaaacaaatctcacctaccggcaaaacgaccgctatatttttattgtgcctaaaccggctcctcccaaaacggtcatacaggaaaaacgtatatccggaacagttacctccgccagaggcgagttgcttccgggggtaaatgtgcggctgaaaggcacctccacaggtgctaataccgatgcagaaggccgttttaatatccctgccggcaacaatgaaaatgctatcctcgtattttcatttatcgggtatgttacaaaagaagtacctgttgccgggcaatcccatatcgatgtacagttgaaagaaggctccactgcactgggagaggttattgtagtagggtatggcacgcaacagaaagccactaccaccgccgcagtatccacggtgaaaggaaaggattttgcacaaaagccggtggtcaatcttaccaataacctcgtagggcgggcgcctggtattatcgcagaccagggcagtggcgaacctggccaggatggctcccgccttcgcatcaggggtacctccacgttaggtaacgccaatcctctgctggtagtagatggtatttaccgtgatttttcccggctggaccctgcttctattgagtccatcaccatcctgaaagacgcggcagcagtggcgccctatggcctggccggcgctaatggtgtaatactggtgactaccaaaaaaggtaaaaccggcgtacctaccttgtcctataacggctatgttggtatccaaaatccaacgcgtatgccccaaatggttaattcatgggagtatgcactattaagtaatgaagctaacgcgaacagcggattaagtcctgcttttactcctgaggaagtagcacaatataaaaaaactgttaccggcgccgcagatgcggatcccgacaaatatcccaacagcagcgggctccgggacgtaatacaaagaaatgcattgctcactaatcacaatgtgcagctctccggtggaacagaaaagatccggtattacatgggattaggttacaccaaccaggatgggcagttttctaccaccaacctgaaaaaatataacgtgttggccaacctggaagtgcaggctaccagcactacccgcgtaggactatcgctgagtggctgggtagaagaccagcagtactccggttatgccgatccttacaatggcgatgccaacaatcgctacgctgctgccggcgggggaattatgtaccaggcattcagaacaccgcctacatctgccatttattacagcaacggcctgtggggtagttatattacgaactccctggtaggcaccattaaccacagcggttatgtgaaaaatgagaatacacagatcatgaccaccttttcagtagaacagcagttgcctttcgtgaagggcctcagcattaaaggagtggccagctatgatccctatactacctataccaaggtatggcaaacaccgataccaacctacagcgtaaacttcagtactaacccttacgaatatacgcaacggctgataggccctgcaaagccgtcgctccagctgagcaacagccagaataaagcgtttacctaccaggggcatatcaactatcacaacacgtttggtgcgcacgatgttactttcctcggtgtagcggaatcgcggatacagaaaggctggaatgtagatgccagcaggaggaattaccctatagatattgatgaactggaccgtggcggcgtagccaacggcgatatcagtaatggcggttcttcttcagaacagcggcaggtgggttatgtatacaggttgagctacggttatgcgggcaagtatctggcggaagtatccggcaggtatgatggtcattattattttgcccccggccgcaaatacggattctttcccgcgttttcactgggctggaacataggccaggagaactttataaaagaccattacagctggatcaatttactgaagatccgggcttcctatggcgaatccggtaatcttgcaggaggtccgttccagtatatgagcggttacgccgtttataataatgcagctgtattaggtaatgcacttactacagggatctatgaaaccatccagggaaatgcctttatcacctgggagcgggcaaagaaaacagatataggggtagatggaattttgtgggatggcgccctcacattcggggtggattatttttatgaaaagcgttcgaacatgctggtgccgcctacggtaactgtaccagcggagtatggaacaggactgtctgaattaaatgccgctgttatgagtaaccacgggattgagctgagcctgggtacttcgcatactttttccaatgggttaaagctggatgtcaatggcaactttacttatgcgcaaaataagctgttgcagatatttgaatcggatgccacttttaataatcccaatcgtcgccgcaccggccgggccaacggtacccagttcggattaaaggcgctgggctactataaaccggatgattttaatgcggacggaacgttgaaagcgggcattgcctccctggccaatgcaccggtgaagccgggagatctcaggtatgcagatctgagtggcccggatggtaaagccgatggtgtgatagatgataatgatgaaaccgtgatcggtcgccccaacggcgtgccgcaaatgatcttcggcttatcgcctgccatatcctggaaaggcttcgacctgaacttcctgttacagggtgccgcgcagatcagtttaccggtgggcggtaacctggtatatcctttcgatcagcagggttctgccagcaagttatattatgataaccactggacgcctgccaacccggatgcattatatccgcgtgctaccaatcagccggtggcctacaacacccggttctcttcctggtgggtgagagatgcatcttatctgaaactgagaagcgcggaatttggttataccctgccgtcttccctcaccaaacgctggtatatgcagcaactgcgcgtatatgtgtccgggcagaacttatggacatggacgccaaacatgaaggaaatgattgatccggaagcccgttcttctaacggacagtattacttccagcaacaggtattttcattcggactgaacgtaaccttttaacatccaaaccgccaacagccatgttcaagataaaacaataccctttattactgattgctacgctcctgtttatttcctgtaaaaaggatttcctggatgtacaggcacgcgatagggtgggagatgatgccgtatgggcatctaccaataatgccgacctctttctcaacgatatttataaccagttgccggatctcaataatgaaacggaacacctggaacaatatacagataactcagatgtaggcgttacctggatggccggttacagcagtatccgggtggctaatattacgccctccaacctgccccgcggaccgtgggacatgtggtactggggtaaagaaagtaacaatgacacccgcaccgggaactatgagaaaatccggaaatgcaatctctttattacaaaagtaggtgcgtccgcattaccggaagattataaaaaagaaagaattgcagaagcccgttttctgagggccatgtactatcactggttatggatggcttatggcggcgtacccattatcaccaatgtgctggataatcttacccagggagatgatatttatgtgcctagaagtacggctaaacaaacgttcgggttcatcgataaagaactgggagaaattgcagacatcctgcccgaaaaacagtccgaacccggccgtgccaccaaaggtgcagcacttaccctgaaaggctggtgtgaattgttttatgccagcccgctacgtaattcaggagatgtggccaatccaggcggtgatcttgaaagatggaaactggctgcgaaaaccaataagcaggtaatagatcttggcgtgtatgatctttatcccgacttccgtaacctgttcctccgggtgggcaacaatagcacagaatccatttttgccaggcagtatatggaaggaaaaggcgggcagctggaaggtaaggaaggacctaccattgtaaacggtgtgcagcaggcctggggcaattttcagcccacacaggaactggtagatgaattttcgatggccaacggtaaagcgatctatgagccaggttccggttataacccgcaacaaccatatgtgggaagggaaaaaaggttttaccagaccatcctctttaatggttcgccctggcagggagatacgcttcgcatggtagtggggcttggacggaaaacagctaacgaaatcgatctcgggtataccagcgatgttacccataccggctactatgcctgcaagcggctggacgaaaagattgtgggaagtgataaccgcgccaacagcacatcttaccagaactatatgtttttccgctttggagaagtattactcagtttcgcagaagcagaaaatgaagtgaatggtcctacagcggaagtgctggcggcagtaaacagggtgcgtacacgcgccggcaacctgcctacaatagaagctacttacggaaccgtgaacaaacaacagatgagggatattatccgccgggagcgcagggtggaacttgcgtttgaagacaggcgctggtgggatgtgctgcgctggaaaattgcagaccgtttgatggatggttcaacaggcgtgttaaaccggcctgaaaaaggcattgtcataacgggaacgactacccttacttatacgccttcaaatgtgagcaaccgcttgttcctgccaaaaatgtacctcatgcctgttccgcagcatgtactggaccgcaaccctgcaatccgtgcccagagcggcggggaagacaactggcagaacgggcagaatccagggtattgatttttgcactcacctcctttaattccgattttatgaacagattatccagctatatttttttcctgctcatcacaggcgttattgtttttaccgcctgtaagaaggatcattccgctacgccaactgtatacatgcccaacgcattgggtgtggtaaaggtaacgtttgagatggcagatacgccttacatagtacctgtgagcgccgttattaccggctcggaatatgccacggtagtcaatgcggtagccggcaacgatattgtagtacactttaaggcagccccggcaaaggtggatttctttaatgaacagaatggcactgattaccgtgtattaccggaaggcagctacgaaatgcccgctgttgctactattacgaaaggcgcttctattaccgcagcaacaggactgaaaatttatgccaaagggaaaatagaccctttccaggattatatgatccctgtcagcattgaaaacattgaaggagccagcgccagcgcttaccagcaaactacttactatgtggtaaatgctaccgcagacctgaacagcatggtgccttatgatcaggctaaatggacaatcgcaggcttttctacggaagaaccggcggaaggtggtggcaacgggctggccgcaagagcgatagacaacgacccgtctaccttctggaattccaaatggtctggtggagaacccggccctccccattattttatagtggatatgggagaagaaaaagcggtacatggcatcggcatcatggaccgttattttgaaggcagctggcaaaccgatggccacggccagccacaggatataactgtttccgttagtgcggataatgccgcctggacagacgtagctgtattaaaagatataccgcacgatcccggccagccctggtacaaatattttgtatctacgctgaaacaggcacggtacgtgaagttcaccgtaacaaaggtatacggcacttccagtaccaacattgcggaggtacaggtgttttaatgcaggcaccacatttcttccacttattttatcacaacagatcacatttcttatatgagaaatagcccgacttttgccttgtttattgccactatgctggcagttgttaccgcctgcggtaaaaagaatactgttgaagttcccgtaacgccgccaccaggaacagataccaccatactaaaaactggtgtgcttcatcaaaagggaacagcgctcacggcattgtgcgtgattcctgccagctcactcaccgcggaacaaaaagtgttgatcgccagcctccagggtgtagtcgcaaaaacttccggtgaacaaatatatatagatgaaggaggcgcttcttctgtatggaaaaattatctcgctgaaaaatataaaataaggatcactaactatacgtcgtgggcggaactgctccgtcatttcgctcctaaagtgagcggctatgtgctgtataatcgcgttaaaaatatcaggtccctcagcgctgccaattccctgtgtggccccctgaatgccattgcagtggatgccagcctggaaacggcggtgatcactgccggtattaaaacaaaaaaagcggatatgcgtgcccgtgatgagaagtgggtgtgggaacattatcctgcaacattcagccggtcgttggccgcagaacagaaccctgctattgatcaccatctccgggattacattacgctcaccaattcgtttactttttacgacggggaaacaccctggcgtgccgatgtgttaaagtcgcttcaacccgaagccttttgttttggatacgggaaggaagagttttcaatggtggccaatgcagcagctgccggcgtggtaatgttgccaaccgatctggcagccaacctggcgccgctgagcagcatatacgatgaaacgccgttaaaacaaccggcccgcactacaccggcagcagaacaaaatgtacactatgttgctttcctgctgagcgatggggataacgtgggctacgatctgtggagtatgcagcagtattttagtcacccgctgagaggtacgttcaacatgggctataccattagtccttccctggcagacctggcgcccgcggccatgcgctggtattatgaaaaggcagccaatacagataaaggcagggatttctttgtagccgggccaagtggaagcggatatacgtttcccagtaaaatgccggcagctgcactcgatcaataccttcgccgcctgaatacttttatggagaaatccgatctgaatattgtgaacatcctggatcagggtgcgctggaaagaatggacctgtgggataaatatcttgcgcaacctaacatagatgctttattatataccggttacggggaagcgcccggtggcagcatccgcttttccgccaatggtaaacccattatagaagcgggtgataacctgtgggcaggcttagaggaagaagccactgtgatcagcaatatcaatgcaagaccagcagacccgcatagccgttcgggttatacactggtatttgtacacacctggacaaaagacatgtcggccataaacacagtaatcgccggactaaacaaaaatgtgcgggtagtaaccccggacgcttttgtgcaactggtacgtaaaaacctgggcacgaaataacggctgcgtgatgttgtaagcgcgtatgttgtcttactcaggattacgctgattatactgattcaggggatttgatcacttttgattttaaaagattcggggagatttaagcggatgtattcgcttaaatctccccgaatcttttaaaatcctttataaaatccaaaaagtaaaatcaagcaaatcagtataatcagcgtaatcctgagtaagacaacatacgctcaaagcaccagctgccggtgcaaccgcatcagcgtatcttccgcattggcgctgcaaaaaccgggatgtaccctcgatgtttgcaccacgctgctgcgcgtggcagttagccagcggaagcggctggcaatatccagtgccccgatcgggccgcctgctttgctgccgttggaaatttccacaaaggcatccaggtaggggcggatggtattgacatctgtttcaggagaaagtgcgtgtaatttttcttcgtttaatgtatatactgcccgtaaaaatttttgttgcctgcaatagaggataacaccaacattcagaaactcttcccgctctacgcttggcaccacccgtattacagcgtattcatataagtgattgtcttgcatgttgtgcttcttttacaaaaatgccggagtggctgatccggtttgttaaaaattcaaaatatacctggcgtctttcttccggtgtaacatcgttgctgtcgtcgctgcgcagccattcttcgggaatgatgtttacaacggcgcgtatccgttccggtgtgaggatcaggttgaaggcagcatctacttgttccagttcacttgcctgtggcagcagcacatgatcctttacctgtacaaagggacggagggactgttcctgccagttttgccaggagtgatgaaaatagagcgaggccccgtgatcaataagccatagttcattgcgccacatgagcatgttggtgttgcgggcagtacggtctacattggtcaggaggcagtcgagccacacgatcttcgatgcagttaaagcatcgatggtatttaccgtagggtcgtatgtggtggcgccggataaatagtgcagggcaagattgaggcccacgctttttttcaggaggtcctgtatttcctcgtcgggttctgtacggccaaaggcggcgtcgagatgggcaaatacaagttccggtattttcagtttgagtatcctggccagttcaccgcctattagttcagcgatgagcgcttttacgccttgtccggcgcctctgaacttcagggcatacaggaatccgtcgtctgcttcggcgatggccggcagcgaacccccttcacgtaacggcgttacgtagcgggttacattcaccgttcttagctgaagttgaatatcgtctatcatctgataatctggttatcgttttctaatatgagtctatagtcaaacaaagtaaccaaatatcaggcacttttgccacaggcttttatatagcggttacgctttgcagctcctttcccataaaagccgcataggcagcagctgcggtgtctactgctgttttcttgccgggggaaaccagttgtgtggtaagggcaatatgccggttcccttctttccggttccagataccaccaatttttccattgatcactactacgggcttaaagatgccataaccggcggtggattgatgttcggccgggaggatatcgctgcggtctttgtaggccacggcgtattcatcgtaccagggcaggagcaaggtagagggagtggtgcgtttagtcagtggtgtgccgccggtaaaccaataggcctggccgttgacgaccgtatgagtgagctgtgctttgttgagctgcagtcctgttttgatatcggatatatttaacccgctccaccactggaagtcctggatagtagcaggtcccctgctgctgaagtagcacagggtgaggcgggcgatggcttcctcccggccgggcgccgcggtggcgggtacacggtcggcaagcaaggcataggtgaattgttttccctgccttgggccgctgcagataagtccatccagctccgcatccatcaggagaaatccgagccggatatcatcggtgttgatctttgctttggcgagcagcggaagcagggctgtgcggggaaggtaggtatgatcgctgagcgctttggtaataatggcgctgctgcgtttcaggtctttgtcggagatgcccagttttacatgcagccgtttattaaaggcttttattttaggcgctgtcagttgcagcatccagcggatgtcttccggcgccacaaagtgccaggtagggcgcagtacatgagtgcgcaggatctttccttcgttaaaatccttttcaatggaggcgtcggtgctgcctttaatacggttcccgatggcccatttggcgcctgcataatcctgcgcctggatgcagcccatccagcgtaccaggtcggcaggccgggtaaaccgggaatggaggagctgctgctgatgcagccggtgttgtatgatctgcaagctgttcatatctcaaaattaccggtggggtgtgacaacggtatgtcagttgagaaaacgggtcaggaaacttttttcagcatctcccgcaaacggtcttttaccagggttttaagggaagctggtgaaataatgtctgcctggtcagcgaaggtgatataccagcgggaaaatgcttgtatacagggcgcttcaaactccatgcgggtgtgggttttgcctgctttctcgctgttaaagccataattatatttctgttccgtaagatacctggccatatcgttatgcacgttgatcactaccgggaacgactgcccgttatttttaggtttgtttgccaggtattccgtcagggagatgtgttcctggtgaaatggccggccggtatcttttaccgaaagcatccgctctgttctgaaaggatgatattttttggaggtggtacaaaaggcgatggcattccagctgccgttttcccggaaaataccaatgggctctatgtccctttcgttaacaccggtttcggtggcataccggatatgcagcactttcttttcacccactgccctgatgagcaggggaagggtgtcgttgagcaggtgattatgttcagataccttatgtttaacggcaatattttcttccaggtcttccagcacttttttctgtgcattacgcagtacagcttttactttgaacatcgcgcctttaaagcgttcgctgttttgcaggtcggcatggtgttccagcattttttccgccatcaggaaggcaatcacttcttcttcggtaaacattaccggcggcaggcgatagccttccataatggaatatcccagtcctttttcgccgataacaggcaccccggcctgttccagggatcgtacatcgcggtacaccgtacgcaggctcacatcaaagcggtcggcaatttcctgggccagcaccagttttttggattgcaggtgaatgagaatagcggttaatcggtcgaagcggttcattgttggaatcagttgtaggttgaagtaactaaattactgatttcccgggatatcgtttttgcgccgtgaatactacctttgccggcacagataatagcttaaagttatgatgaaacgtttgtttgttgtggtatgcctcctggccggatgggtaaccgcctgttttgcacagtcggatgagtacctgaaaaagaagaatgtccccgataccattttacaaaaccgcaccctgttactggcaggtacttttaatgcacagaaagcgctgctgcaactgttccccggaaaatattacaatctcaccaaagatagttaccggaatgagctgatcaactgggaatgcaaaacctgtaaacccaaaccttacccggatgtaaatgaagacggcaaccctgtatttccttaccccgaaggcgtggccacccgcctgatcaatgaaatggattttaaagacgccacaggcttacagtataaggtgatcagttttaaccattcggtatttgatgaagaaggtttccagacttcgcgtttcaccggcggactcctcggccttgccaagtttgtactcaccgacgagggctggaaactaaggatgtttcaaccggctatccaggcgtacggcgctttttctaagtgccccacgccaaagccactgctgataggcgatgatcagtatgcgtttatgattaaacatagcaacggacctgcaggtggtccatactatggcgattatttcctggttgccgggatcaatggcggctatcagcaggtaatggctgctcacaacgcagaacgaacagaagtcggagcggaggaagggttatccagctggagcagtgagtatacggtgccggcgggcgataaaaagtacttccgcgatattgtaatcacctttaagggaaccgctactgccacggataccgacgggcttccggatgaagtgaaaagcctgctgaaaggcaaaaagaaaatacggtttacggccgtgaaaagatatgtatacatgggcagcaaaggctatcagctgcagctgccggtgaaggctacgttaatcaactgatgccgtttccagggcaggcaatttcaggctgcgccctgtgatttttttccggtgcatggcgccccataccgttaatgaatggagcacatctcccagggtgtcactgtaatcggtcagctcatactccataagttgactgccggctactggtatttttctcacaaaaccattcagctccagctctttcagttcattcgacaatacctttgccgaaataccttccactaaacgctgcagttcattaaaccgcctgcggtgatctatcatagccacaatgatcttcagtttccacttgccgccaatggcatacatggcgtctcccactgctgcgagcgaggcagcacatacttctgctgaaggatgatgtcttttatccatttgcatatattttaacttccctgggttagcagtaaccaaaggtaagtagttttcgaaataaattcgcggaggttgtcttgagcactgattacgctgattttaaggattggatcaggttggattttaaaaagattcggggagaagtaagcgaagatcgcggcgaattttgtctttctcaggattacgctgattttactgattttactttttggattttttttgattttaaaggatcagggagatataagcggatatattcgctcgtatctccctgaatattttaataaaatccagaaaatcaaaaaagtaaaaatccgggtaatcagtaaaatcagcgtaatcagtgctcaagacaacctccgcgtgttatttactcagcgcatcgaagtcctcgtcagagagcgtgatcgatcctgctttaaggttttcttccaggtgggcaatgcttttggtgccaggtatcagcaggatgttgctggcgcgtttcagcagccaggccagtgcaatctgcgcggtagtggcgttgtggcgggcagcaattttgctgatcttttcttccagggtatgcggaccggaagccagcgggtaccagggaataaacgcaatgcctctttcagtggtataatccagtacggattcccattggcggttaccgaggttatacaggttttgtacagacacaacaggtactaccttttctgcctgctcgatctgttcaatagttacttcagacagccccacatgtttaattttaccggcttttactgctgctactaccggcgccagggtttcttccaccgggatgttaggatcaatgcggtgcaactgccagagatctattatgtccgtcttcagatttttgaggctgttgtcgatgtctttggcaatccattccgggcggccatcaggtacccactggttggggccggggcgctgaaagccacctttggtagcgataatgaggcctttttgatagggatgcagcgcatccgcaatgaggcgttcattggtccccggaccataagccgccgcagtgtcaataaagttcacaccggaagctaccgcttgttgtaataccttaatggcattgggacggttggctgcatcgccaaatacgccgttgccggttaattgcatagcgccgtaacccacacggttaatattgaattcgcctcctaaaagaaaggtggcggcgggagatatttgtgttttttccatttttttatgatttgctggatcaaaggtaggggtaacggctgatccggaaattgtgaaaataacaggaagagttgtataaatcaaagaatgaggggacgggatattaattttttttcacagttttaagctgggcatgcagataatctgccaccatcttagcaattgaaggtagtcctttctttaaccaggtctttttcaatgaagattctttagccattttactacttcgttatcttccagtttaacaagtaaagtaggtttaatcattccgtcatacaggcaaataaccttaaatgtattgctatagttgttgatgtgttccagatttttctcataaacgcccttaatggtccttgcatctacagcatgtccaccttctttcactcttagcctcactctttgctcacaatcttttattttatcgagacataggtagttaagttgaatttgatagcctttgttttcaaaacggtctatgtacttcgagtaatcaggatgggataagggcgtttccaaaacaaagtggtgatttgcaagaatggcttcgtccattttagaaatcaaaaaatcttccatcatttgtgcggagcggtttttgatctggtctggtgacattccatctttctccagttgtttttcaatatttgtccgcgttaagtccctgtcgaaaggtaaaacgccttcaaatagtgaaggtaacatggattcaatgtgtgtggacttacctgctccgtttggcccggaaatgactagtagtgttggcttagagtaatccattttctctccggtactgttgcctgatggtattagattccagatctgataaacgacgcacaagccgcgtttctatttcagcaccaatagtataaacttcttgaatttcaatatgaccatctgcatattcataaaaaccttgtccctccggtagtttatcagagagcatcaggaatggcaggttattgctaaaatttctttttcttattttttcaatagtagcagtaaattttctatcctgcaaagcaatttcagattcaatatttgtcatatggataatgctaaattactgtgtaaacatactaaaatgcaagctgaaatccaattttgaatgccgtttataaagtgttgataattagttgcttgcaagggaatgttattcgcctttttttgtctgtattatcttcgggtttccatcttatccgtcaacgcatgaataaacgctatcaggtccttaatctccgcttcccggagattaagcggcgtggaagaaagcgtttgataaggatcagtcattcccactccattgccgccgccggcattataaaattccattactttttcaagatcccggaatgcgccattatgcatgtagggggcggtcatagcgctgttgcgtacagtgggcgttttgaaggcgcgctgataataagcaatggggaaaaattcaaacctgccggcatccgtatcgcgtcgtggatgctggagatcatcattagcgggcatgccgaggttttcaaattccgtgaactggtataagggtggtgtgaggccgttgaacagcggggcaaagtgacaggtagcgcattgcgctttcccggtgaataagttgaaaccccggatctgcgcgggtgtcatggcgtttttgttgccggcaaaatattcatccattgcgctgttcataggagcgagggtgcttaggtaagcagcaatggcggtggccaggtgaggcatggtaacagcgacgctgtcttccgggaaggcggccgcaaaggcttcgcggtaatgcgcgctgtcttttaaccggctgacgatcacggcaggatggccgttcatttcctgcgggttgctgatcacggtgagtatttgttttgataaggtacccgctcttccatcccagaactgcgcatattggaatgcggtataggtaaggcccggcgcatttcttcttaccatggttttattatccagcgtcctgctggtgcggagtccatcgctgaagtataattccgggcggtgacaggtaccacaatggcgggtgttgttcccggagagtgccttttcgaagaatagtcgttttcccaatgccttttcattttccgtatatacggcgccgttagtaaaagctttgaggtctatggcgtttttactgaaaaggtttggagcgttatagttcagcgcgctgcgggtgtgctggtccagttgtaaagcgcgtatcagtgcgccggtgctctcctgcaggggcaaaccgcaggcggtgaggaattccagccggttaaagtcatcgaaacccggatgcgtttccaggtattgtatacaaaaggtgaggtaatgggctacggattttgtttcgggagaagagctgctgagccagggttccatcactgcctggatagttcgcatcgattgcgcggtttctgcaatgcctgtttttaattccggtgcatcgtaaccggtgatgcctcctgcgtataggcgtaccagttcgagccgtatgctttccataatggctttgtcgctggtagtaaactggtagagcagcgacgtaagatcggcggcggcagtacggattaccagcgcttctgttaccagttcttttttccgggagaaaggttctttctcaaacaacagtaccgctatctgctgtaaccctgatggcgcctggtactccatgtacggttcatctatttccgttttggccgggcggttatacaccatggaagaagagaagaaaaagtaatcaagaaaaaactcgatccttttgtattgtaaccggcatttttttagcgcttctttagcggctattaggctggccggatcatctttatcaattgcctgtatggcctgttccagttccagggaagccgccgaaaatccgttggcgccctccctgaaaatggcaatagtatgggtaacaccgcggtcatccgtggatggtgtaaagctataagctaccagcaggctgaataacagccagatgaccttatttcgatacatatacggtgaaagtatcttttacattattgtatgcatccaccacggtatattttgtggtggaagccgtgggagttacggtaatactccgtgtagtgtctttacggttattccatttataagtaccaatgaacgacgcggttaatgttgctgcttcgccttttttgatacggatattggtattccggtttacatttttcatcatggtaaactggtcgcgggtggtgccatctgcgcagatccatttcaggtcgaggcggttgtcctgtatttcaagaatgctggagccgccgtgttctgcgtctgcaaaatacatggcattatgcgggtaaacggtttgtttgcctcccagcttaccggcggagccgctcactacgtatacagtaccggtggtatggatgctgtccttgatgtatggtgcagaattgctgccgccatcgtaccggccggaagaattgctcacgttatgtttgataggatcaaagctgttagccgggccgtagtgccccttgatcatcctggatctttcgtaatcatgactatgcccgttcaataccaggtctaccccgttgcgctccaggatccggataaagttttcccggatgtgtaccagctcatcttcttcatcggaattatgggagcccatggtatacggcggatggtgccagtaggcaataacccagcctttatttttattttcggcgaggtctttctttatccaggtaacctgcggaccggtggtgtcgtacaggcggtaggcgctgtcttctttgccgtagctgtccagcgacaggaagtgaatgttcccgatatcaaaggaatagaacgaagccgagtgggaaggtgatccgccggattctccttcagatggcatggagaagttctggtagtagtttgtttggtgcgactgctgcgcggcagcggcggagatatcggtatcatggtagtcatgattgccgggcgccgggaacaggggatatttcttcagcaggtcatctttataaacattaaaaaacttgctttgatattccgcatcggtgccgttgggataagcattatcgcctaataatatccatgcattcaggtaattgctgccgatgtattttaccagttgttcctttaccagttgctggttgggagagccgtcgccgcaatcgcccaatgctgcaatgcggtacaggtctgttttaccggcttcgggcagggtcataaagtaattgtctgtgttgccctgcaatacctccttatagccgccaatggaataatagtagcgggtgttgggctgcaggtgggtaagcaatactttatgttctgttaccaggttggcatcgtctgcctgctgatccagcttatccggagcggtgccgtatttcacacggctgcgggcagatgcatcggtgcgccagcggatcagcatctgctgtgtacctgctgcctgcaggtaaggaccacggatcagctttgcagcgatggggtcttttttaacagcagcatcctgtgcctgcaccgggcctaaaccggccaacaggcacagcgaagcgagaaagatagatttcatatatgggacactatttttttgttggcgctgattccagctctttaccggcgatatcttcccagcgataataatggaaggtccggtcgtcgctcatcactacaaataatccatgtttgaaagtattgttcagtggcacatttaccatatcagagccatcgctgtggctggcgcttactttcactgttttcagcaacgtatgtgttgttcctgctctgttgaagatatgaaatttgttggcaccctggtcagataccaggatatatcctttggtgggagacgttttataaatggagatgccttcatgatcttctgtaaaaccggtggtaccgaaaactgttaattcttcattacctttttcgggatcagcataatattgccgtacgccgtactgttcatccgaataataaacataaccggcttcgttatctaccgcaatagcttctatttcctttttgccactgtagtggccaaacttacgtaccagcgtggcttttatttttcctgcaccgttatcagagatacggtattgccataaataggtcccatcctgcggaccggttttgcggcctgctataacatagtgttcgttcttcttattagtgtaaacagctacgcccataagatcacggaactgtgtgccggtttcaccttcaaatgccgggatgccgccatcatcgatgggctgcatgtctggtaatgaatagaagcggagtttatgcgtgatgcgttccgtggtaacggcatagtctatacgttttccgttgaggagcaatccgtatgcaatgtctacattattggggcgttgcaggttggctactacctgtttgatcttcccttcgaggtcaaacacatacagggcgccctgggccgatttatcggtacctatcaccaggctctgggcgggattctgtgggtttacccagatcgccggatcatctgaatcaaactttacagcttcggtgataaccgccggctgaataatagcagtatccgtatatacctgcccgttagcccggctcgccggtcttgcgcaggcaagaaaacacagcagtccgggtagaactgctgcggaaaataatatattgcgtgtagtcattactgtgagatcgctgttttagtttttagtgccaaatgcaccaataaaagacgaaggagcgggagaagcgtaattattcccattcagctccagaccgttcgggaaattacgggtaaaagcagtggtacccttgcccagcgcgggtgaaccggcctgtaaatgaaagtcccagctggtgttaaagtcagggctatccattggtgtgttcagcggataacttacaaatttcggatcattctcaccggctttggtactaataacgtcgttggcgccgctaacaatatctttcgcaggctggaactgatctacggtagtttgattaaatccgtaataaagattgttgctgatcaccgagcgactgtcctctacttttttagtatctctcttaataccaaaacgtgtgttggcaaacaggttattgtgcagttccacgaatactgtggcctctacccaaacggagccgccttttacagtaggtcttctccagccggtgttgagcatggtgttgttataggcaatcacgtgcgcctgtggcgtgcgctcaccggaattggataacttaagggcgttggtattggtagagtagaagagattataacttacatccgcgatgcagccggatttgatgttaataccctctccgccggtaataccggtagtatagaatttattattggagaagataatcttaccgccttcaatgtaggtgcagtcttcattaaaattgcggaagatacagttattaacaaccagcttgccattcacattactgtaccatagcgcgggcagcgcttcgccgctcacagctttatacaaacccagttttacagaggtagatgattcggtggtaacagcaccgccgtattcaaggatggtattgtctaacaatagctctgcacaggatttagccgcaaggataccgccccattgtttaccaaacttgcggctgtcggtgcggtagttttcttcaatggtaaaccgcaccggttgttcaggtgtccccatggaatacaggtttccttttacaattacttcgggtttcacgagggtatccataattaccagcacgccttcttcaatcaccagcgttttgccttcaggaacggtgatatcgccggaaacacgttgaatactgcctttgggccagatgccccatacatcgccgtgaacagtgccggagccaatgatgccttcgctgaggtctacatcgctgtttgcttttttacagccggcgacaatagtcagtatcaatgcagcgtaaaagagaatatttttatatttcatgagatgaatattttagaatgagtttataacttgtaacgtacgccgagcaggtaggtttgtttataatattctttcctgatcagggtttcattggcctttccctgtccgggcatactggtattggcaggatctgttcctttgataaatatttctgttggagtgttcagcaggttacctgctttaacgaagatgctgaagttgtttctgaaccttttttctacagaaagatccatttgtataaatcctttctgccacagatcattatcgatgtactgggaaacagtgttgatacgcggaccggtgtaagcgccggccagctgtgcatcccatccatgctgaatgtctttgtacagcacggaaaggttaccgatgtgttccgactgtccgtataaagggcgggtctgatccacagcgatggtctcaacatcgcctttgtcatcccggatcctcaggcttttagaagtggtgatagaagaatgtgtataagtgtagttcgctttgaatcctatcttactgaaaaatttgatataatctatttccaggccgtagttacgggcggtaccaaaattaccggcagaataatactgatcctgcgggcgggtggcatctgcgcggatggtattttcaatcgggtcctggatccttttgtagaatacacctaccagcaattggtcggagcgtttcgggaacagttcataacgcaggtcgaagttgtccgcgatagcgcgcttcaggtccggattaccgcgttcctggtagtcttccagtataattttggaaggaacaatttcaaagaagccgggacggttcagtgagcggaagtaggaaccgcgtaagttctggtgtttagataactcgtacttcaggttcaggctcggcaatacatcggtatatacctggctgcccgtggggcggtcttctccctgtggaaagaacatatgataaccctggtcggtatgttctatgcgtgcgccaccggttatttccagttcagctacttcgaatttaaacatgccatatccggacgtcgttttttcggatgcgtcgtaagtaagcgggttgcctactgcgcctccgggattctggatctcccatacaatgtctgtatagctggtaaaatctttgccatatactgcattgatattcgcaggtcggaaggtatagttgttaaagaaactgctgcgttgtttgtcgcggtacaggccacctgcggagaaatctactttggtcccggctatcctggcagtgtacgtaagatcgaggtagcccgcgagatcattgtctgtattacgttcccagcgacgggaggtaccgttgttttcaatagtggtgcgtgtgtcctggaagttgttccttaccccgtttaatgcgatggtagtattgtccggcacttcatttttggcagaagaaaacacggcagaccactgcagctttaatttacccggaataatatggtgatcgccatgcagggtggaattgtagatctgctgcgtggttttcctggaacggttttcaaacgtcagctgtgcatttccggctgcaggatcaaacacgccatcagaaaagttggtggtaataccttcccttgtctggaaactttgcaggttcatgtaggcgttgtaaagcgacagcttattattttcattaaacacatagtcgattttcccgtgaacaccactgcgctgctgttgttcgctgtactgcctgttttgcatactggtaagtacagagtaatgccccgtatccatatcattcttatagaatgtgctggtagtaccgcgataggtgttctggaaactgccggcgaggatcacacccagtttattgtgcaggaaacgctggccaacagataatcctgctaccaggttgggagcgaagcttttgtttttataatcaagtgtaccagtggcaaaatctgcgggagtggcattatagcttttaccgtgcgcttcgtaaggtgatttggattgtatgttgccggcgtcaaaggaagtaaagcctttatccagcaccatctggctgtagccggtggctacgttggcgttgagcgacagtttcccgggggcgtctttcattaccatgttcactacgccgcctacggcgtcagcctccatgttgggggttaaggatttatatacctcgaggcggtccagcaattccgacgggaagatgtccagcggcacgtagcggtatttattatccgggctgggtattttcaccccgttgataagtgtgtagttatatcttttgtccataccacggagaatggcgtattgcccgtcgccattgctgctgcgttctatggagataccggaaacgcgctggatcacgttggccacagtgaggtcgggcgatacttctattgcctgaccggatacaacgttcatcacctggacggatttctgttccagtttgcgggcggtgttttcagaggaggctttggtgccgccggcaattactacttcactcaggtttttgctgctgcgttcactgaggtagatgttgagcgcggggttgtcactttcctgtacggtaacttcttttgttaatgttttgtaggtaagatgggaaatgtgcagggtgaatgttcctgcggtgatttttttaaattcaaaggaaccatcaagacccgtgagggctaccagtttggtttggtccattacaacggtgacgcctaccagcggttcgcccgttttctgatcgtacacatgtcctttcagactgccggcgctggcaaatgtgacgctcagcagcagacataaaagcgttgttaaaagtgtcttcatcttttggtgaatttgatgccgttcgtgttagtggcgaatggcatcgcaaatgtgggctgctccaaaaaaaaatgcaagaaagcagcgtaagcaaaacgtaaacagcgttaacaacaccgtaaacaaagcgtgatcagcgtatacaaacaggatgtaagttgttggtagttaggtgtttatttgtaacaggaatcgccattaccattatgttaccgcaacgttaccggaaggttatgcatcacaggctttgcacaaaagtgttgagcgtatcgccttccggaatgtttaattttttccggagacggtatcttgccacccgtaaactgtcgggtgaaataccaagaatggtagccatatcttttgagtccatattcattttatggagcgccagtaatttgatatcgttgttggtaagatcgctgtgcaacgcattgagtttatcaaaaaatacctggtgtacctgttcaaagatgccggtgaattctttccattgtttctcgtgattgacggtctggttaattttcagcaccagttgctgcagttgttttttctggtcgcgtttatcttcctgtaccatctctgagagggtattccgcagttcatccaggaactggttccgttggatcacgtccagcgtatgagtggccagctgcctgcttttcagttccagctggtctttctgcacgcggtttatttcggcattccgttcagatacggtctgggcctggctgatcttcagcttctggcgggaaatggtgagcaggcaaaggaggatgagtaacactactacaatgactaccgccgtgtaaatgatgcggtttattttatggctgttttccagctggaggatttcgtcattctttttattggtatcgtacaggatctggaggaaattcatctgctggttgttttgggcagagtaaatgtcgagcaggcatttgcggctgtactccatataataaaaggcgctgtcgttccgtccgaggagattaaacgctttggcaatgtctttacaggccgcggcttcctggtacttgttattggtttgctgtgccagagcgagtgctgccttggaatagggcaggctgttttttacatcgccggttttccggagcacatcacctatattatttaatacttctatgccggctatccgttcgtggcttgcctcaaagagttgcagggccatgcggaaggaggagagggcggtatcgtatttttcgaggtcttcataaatggtgcccaggttttcgtagatgccggccatgccgaacgtgtcgcgtgcgcgctggtattgtgtcagcgccagttcctggaaataccgggcgctgtcgtattgttgctgtttttcgtagtagtgaccaatgtggccataggtggcggcaatgccggcgggatcatttacctgccggtatagctgaagggctttatcgtactgcattttggcgcccggcttattaatattgcgataatagagctggcccatatcattgagtacagccgcttcggcggctttatggccggtggcggtaaaaagagtggccgcctgctggtagtattccagtgatttggcgtagtgccccagggtaaagcagatttttcccatctggcggaggcatttgccggcagtggcttcatctttgttactgatagctgcatcgtgcattttgcgcagggcaagaaaggcggcatccggtgattcctggctcagctttcctgcggctgccagctgcatttgcagggtgtcctgtgcagcggtggcagttaccgggaagacagataagcatactacgataaactgaagaaaacgtttcatttgtaatgacagcacgtattaattaagtgtaatcaatccgcaaagaatgttttttagtgttaactgtatgttaccaaacgggctgccgctgacataaaaatgcttgcttaccgatactattttatatattattgtgccgccggttacattttttgacccataaattagttccagttaaatattgattatgaaaaagagaatcttagttaccatgctgctggcgggaggaattggcgccgccaatgcccaggagaaagcaaaacctgaagatacagaagtatataccccggtgccgccggaggtaaaacccggaaaaaaatgtggtgaagcgccttcggatgcgatcatcctgttcgatggcagcaacctggatcagtgggtaatgaccgacgaccgggagaaacctgcagaatggctggtgaacaaaggcattctgacggtgaacaaaaagtcaggaaatattgaaacaaagaagtcctttaagaactaccagttacatatcgagtggcgcgttcccgccaatatcaccggtactggtcagggcaggggcaacagcggcgttttcctcgcctccattggtaaaggggatgccggttatgaattgcaggtgctggactcctataacaataaaacgtataccaatggccaggccggcagcatttacaagcagtccgtgccactggctaaccctaccctgaagccaggggagtggaatacgtatgatgtaatctggacagcgcccgtatttggtgcagatggcgcgttggtatctcccgcaaaagtaaccgtaacttttaacggcgtagtggtacagaatggctatgagctgaaaggccctacccaatacattggtcaggcatcttaccgccaggcgcatggcgccagcccaatcaagctgcaggcccatggcgataagagtgagccgctcagcttccggaatatctgggtaagagaattacagtaacaaaaacgaatttacaggagagggctgccggaaacgacagcccttttttatttttttctccccgttccatcattttctttacttttaatacaacgacgttatgtaaaactattccactttatccggttccatggagcacgtaaacattgaaaagaaattgttgcaaagggctgccgaaggccatgaggaggcgtttacccaactctttttcctgtacaggcataagttgtacagcttcctgctgcgcttaacggaatctcccgaaatgacggaagacgtaatacaggacgtattcctgaaattgtggaaggaccgtgaaaacctggtgaacattgaacagtttggcgggtatgtttaccggatggcccaacaccaggcactgaatgcgttccgccggatggcgaaagaaacactgatcctggctgaactcaccaggacgatcaacgatgccgcccccgccgatgccgcggataacctgagtgtccgcgaggtgagggaaaagttacaatacgcgctggatcatcttcccccaaaacaaaaactggtgtataccctcagccgggaacagggactgaaacatgaagaaattgcccgtcagcttaatatttccccgtctaccgttaataatcatatgattgccgccctgcgcaccatccgccagcagctgggcccgcacctgcattccattaccggcgcttcctgcctcctgatgatcatcgatggcttctgctgaaaaaatattttcagggacactagttatatccttccgcccgggtgtctataatacgacagattccgcattaatgtaaaaacaccgcatgacttcagcaaggatcagctacctggcagcacgctattttgataatacctgtacaccggcagaaaagctggagctggcggcatggatcgaccggcaaacggatgataccgtgctggaagccgtattgggagaagcctgggcatcgcatgtgccgctgatcatgatgccggatgaaatgtcggaccgcattgtgtcagccatgtttggccgtgcgccggaggtacccgtgatgcaggcgcgtacccgctattataaaatatggtgggcagctgccagtatccttgtactgggtggcataggcgtatgggcatggcagcatcagcggtcgccatcgccggtagcagaaagcaaacaacaacgatataaaaatgaagtgatgccgggcagcaaccgcgccatgctcaccctggccgatgggagcgtgattgcgctggacagcgccggcaacggactattgggccggcagggcgccgtaaagatcatcaaacaggccaacggtgaactggcttatgtgggcaacggcaacggcgaggccatgtataataccatgaccaccccgcggggcggtcagtaccaccttaccttgccggatggcacacaggtttggttgaacgccgcttctgcgattacttatcccgccgcatttaccggtaaggaaagaaaagtaacagtaaaaggggaagcctatttcgaggtaaccgccaatgccaatatgcctttccgggtagccgccggcaacaccgctataacggtactgggcacacgatttaacgtaaatgcctatacggaggaaccggctgtccgcaccacgctggtagatggtgccgtaagcgtaacagccggcagcaacagcaccgtactccgcccgcgcatgcaggcgagggtaggcaaagatgaagtattacacgttactgaaaatatagataccgatgaaatcatcgcctggaaaaacgggttcttccagtttaccgacgcagatatgcctgccgtaatgcggcaaatagagaagtggtacgatgttaaagtaacttatgaaggagctgttcctgaaaagagctttggcggtggtatgcaacgctctttgcccttaacggaagtgttgggaatactggaagaaaatggggtgaaatttaagatagaggggaaaaatattattgtattgaaataaaaaaccacgttactgattcactattaaacttagaaacacaaattccactgcataagctcctgtagtttatgtatcctcacctgttatgcataataaagccggaaacgctgataacatttccggcggcgtctggataacagaaacaaaaaagtcggcgaagactccttattcattcaaccaaacaatgcaaatgtatgcaaattaattgtatcgctctttgcagccggacagctgttgctattacccggagcgttatttcccggacaggcagcagggtttcccggcatcgcacgctatgctcaaccaaaatgctgttagctatgaagttaacgattgtgttcacattactgctcctgaacgtaagtgccacgggcctttcgcaaacggtcagtttttccggtaagtcggtatcactcaaagcagtttttgccgccatcaaaaaacaaacgggatacgtggtgttctacgacaaccagctgctgcaaaacagcaagccggtgaccctctccgtggaagacgcgccgctggcggtattgctgaatgctgccctgaaagaccaggggatgacttttaccatcctggacagaactatttcagtaaggaagcagcggccgccgctcacacttccgcccctcctgaaattgatgatcccgcaaatgaccatcaccggccgggttaccgacgattccaatacaccgctgcccggcgttacggtattgcagaaaggaaccagcaacgccgttgtgaccagcgaaacgggcgaataccggctttccaatatcagcgatggcgccgtgatcgttttttcctacatcgggtttaataaagaagagatcaccgtgaatggacagtataagctggacgttcgccttaccaaagccgccaacaccgcactcgacgaactggtggtaatcggctatggcaccatgaagaaaagtgacctcaccggcgctgtgtctaccgtgaaaggcgatgccatcgcttcccgcaaaaccacgcaggtatcgcaggcactccagggcgctgtgccgggcgtaatggttacccgcaccaacaacgcaccaggcgccgtggcgcagatccgcgtaagagggatcaccaccatttctgatgccggcgccacaccgctcatcatcctcgatggcgtacccatagatgatatcaactccatcaacccaaatgatatcgataatatttcggtattgaaagacgccgcctctgcttctatttatggctccagggccgccgccggcgtgatcctggtcaccaccaaacgcgcaaagagcgggcagctggacctgaactacagctatgaatacggggtggaaaagcctaccaaattgccggattatgccaatgccgtacgctatatgcaacttaccaatgagctgcggtggaacgataatggtaataacgccaacgaatatcctacctataccaaagatattgtagataactacgccacattgcatgcacaaaatccggatcaatacccggatactgattttagaggcatgatcctcaacaacagcgcaccccgcgaaacccatgcactcagcattgccggcgccgggaaggcactgcgctccagggtttcactggtatatgataaaatcggcgcactgtacgacgaccgctcgtacgaccgcctcaccacacgtatcaataacgacatcgtcatcaataaatacctcaccgccagcgtggatgtgaattacaaacgcaccatcgttaaacagcccatcgttgacccgatgtacaagatgggtatcatgccgcctatttacgcggccatgtggtccgacggccgcattggcgctggaaaagacggcgcgaacatatacgtgcaaacaaaatacggcggctttaacaacaactggtttaatcaacttggcggaaaggtaggtatcgattttacgcccatagaaggattgaaaatttccggtgtcgtatctccttttattaacttcgataaaggaaagaaatttacccggaaagtgccgtatacgtctttcaacaatcccaacatcatttcgggatatattgaaggcgctacggaaaccaaactggaagaagtccgcaacgataactaccgctataccacccagtttattgccaattatagtaaacagatcaaagaccacagcttcagcctgatgggcggatatgaattttataaggcattcaatgaagatctgggcgcttcccgcggccaatatatcctcagcaactatccctacctcaacctgggaccactggagttccgcgacaacagcggcggcgcatatgaaaatgcttaccgctcctggtttggaagggttacttatagctataaagacaaatacctgttccagggaaatatccgctatgatgcgtcttcccgttttgctgcaggctaccgctggggttctttcccctctttttctgccggctgggtaatatcagaagagaaatttatgaaatccaccgcgccctggttatcctttgcaaagctccgtgcttcctggggttcgctgggtaacgaacgtatcggtaactacccttaccaggcattgctgcgctttgaaaataactccctgttctataaaggcaacaacgccgtatccgcgcaatctgccgcacagtggcaatatgcgatccgtgatatttcctgggaaaccacccactcatgggatctcggcgctgatgtaaatttcctcaataacaggttacgtttcaccggtgattattttaagaagacaacagacgatatcctgctggagctggaaatccctgattacattggcttcgacaatccttaccagaataccggtaaaatgtttacaaccggctgggaagcgcaactgggctggagcgatcgcatcggtgatttcacttatagtgtatccgtgaacgtagcagactttgtatcaaaaatgggcgacctgggtggtacacagttcgtgggagattctatcaaaaaacaaggcagtgaatttaacgaatggtatggctatttatctgatgggatttaccagacacaagacgaagtggataaatcggcgaagctcaacgccaatgtgaggcccggcgatatccgctaccgcgatgtgagcggtccgaatggcgtacccgatggcaaaatatcccctgaatacgaccgcgtattactgggtggttcgttgccccgctaccaatatggcatcaatttgcaaggtgggttccgcaactgggatctgggtatcgtattccagggcgtaggcaaacaaaactccaggcttactgtggatatggtacggcccctcatggaaaatttcggcaatttcccggctatcctcgatggcaattcctggagcaaatacaatacgccggaacagaacaaagcagtccggtatccgcgttacagcaatacttccgcaggcaataactacgccatgtccgatttctggctgatcaacggcgcctatttccgcctgaaaaatatcagtgtggggtattccatgcctaacgactgggtaaagaagatccgcatacaaggtgttcgtatatacggcagcgttagcgatcttttatcggtgcataatttcccgaaaggctgggatcctgaacaaccttcgctgggctatcctattaccaccagttatgttattggcgcatctgttaaattctaaattccacgaacatgaagcaacttattctcatagccggcatcacttgttttttcttcagcgcctgcggcagcctggatctgaacccgctgtccgacggctccagtgaaacctggaattccaatgcggaagaaattgaaatgtcgctcaacggattgtataaaatcaatttctggatgaaggacgacgatgagtggaccgacgactggatctaccgcgacgttactaccgctattaccggcgctaccatcaatgggcaaactgattttgtaaagaagtggtggacagatacctacaaagccgttgcccgcgccaacaacatcctgcaaagcatttcccgcgccgataaggtgttgtcggccgaccagatcaacaactacaccgcagaggcccgctttgtaagagcgtgtatgtattcccgtttgttatcgcattacggcaatattatttacaccgattccatgctcgatatcgaccaggcattgcagctgaagcaaacggacaaagccacggtgctgaaaaagatctatgaagattttgatgccgctgccgctaccttgaaaaccacttacggtacatcggaattgaaacgtgccaccaaaggcgctgccctggccatgaaagcgcgtattgccctgtatatgggcgactgggcggttgcacgtgacgccgctaaagcatgtatcgatctcgatgtatataaattgcacgataattttggtaacttgttcctgtcgaagacaaaaaactccaccgaaacagtttttggcctgccaagatccgtgaccttaaaagttactttcgacgattgccagaattatgtatcgcgtaacgccggtggctgggctgccaaagatccgtcatgggatctcttttgcagttttttatgtaaagatggattaccggtagatgaatcccctttatttaatccccgccgcccgtttgataatcgtgatccgcgctgtgccgccaccatcgtggagtttcagacaccgcacctgggatatatttttcagccgcacccggactccgtgaaagtaagatccgtatcagacaataaatacgtagaaaataaagacacccgcaccattgcacagtacgcatcgttcaacgggttgttatggaaaaagggaattgacggcgactggctcctcaactcctggaaatcagaaccggataatatcgtgatccgttttgcagatgtattgctgatatatgcagaagccaaaacagagctgggagaaacagatcagctggtgcgcgatgctattaacaaagtaagggcgcgcgcctatggtaccgtgtacaccaataccagcgagtatcctgcggtgactacggcagatcagtctgccctgcgtaaaattatccgtacggaaagaagaatggagtttgcgctggaaggcatccgctatatggatatcatccgctggaagctggcagaaaaagtgctgaacaaagcaaactatggtttgctggaacccgcggacctgcgcacaaaaatagtgcagcctggattatggttcttcccgcaaacgccggctatcgatgaagatggtatagcagattttaccgcgatgtataatgccggtctggtaaaacagatcaccgtgcgaaagtttgatgccacgcgccagtacctgtggcctattccatctacagaagtattgaccagtcacctcacccagaacccaaattattaagccagcacatgacacaaagaaatagattggcagcagtattaatgaccatcggtatattgggagctgcctgtaaaagtgaaaaagccgcggcgccgcgatcgttcagcggtatttacccgcaactggcgatgtataacaaggaaggagaatgcggtaccggtgcagtagtgccctgggcggggaaactgtgggtaattacttacggcccgcacctgccttttggttcatctgataaactgtatgaaataacccccgacctgaaacaggtggtacgcagcgaaagcattggcggcacaccagccaaccgcatgatccacccggaaagccaccagttgttcatagggccatatgcgattggagaaaacggccaggtgcgcgtcatcccttacacggcaatgcccgggcggcataccggtaacgccaggcatcttacagatcccgccggcaaaatttactatggcactatggaagaaggtttttatgaagtagatgtaaaaacccttcagcctactttattatatgaagatggaaatgtaaaaaacgaaaaaggcgcagacactaccgccaactcaccttccgccttgttgccgggagcgcatggtaaaggcctgtattcggggcagggcgtaatgatctattccaacaacggggaacccggacccaaagcattgacccagtttgatattgaagccgggtcgttatcggaatggaacgggaaggactggaaagtggtgcgccggaaccagttcacggaaatcaccggcccgggcggtatctccggaaataaaaatccggccacagatcccatatgggcaacgggctgggatcataaatcggtgttactcggattgcgcgaccagggcaaatggagctttttccggttgccaaaggccagtcacagctacgacggcgcacatggctggaacaccgaatggccgcgtatccgcgatatcggcgccaacaataaaccggattacctcatgaccatgcacggcctgttctggcatttccccggacagttttctaccgggcatactgcgggtatccgtccccgtagtgcctacctgaaagtgatcggcgacttcacccgctggcaggatcaactggtgtttggttgtgacgacgccgcacaaaaagaatttctcaacaagcgtaccgccaaaggaagtattgaaggacccggacaatcaaattccaatctctggtttacctccctgcaacaacccgatgcgctgggacctaataccgccgaaggcgccgtatggctgaatgaagccgtaacaccctctcagccttccgagcctttcctttttgccggctggcctcaccgcagcgcgcgcatcacccacaacagcaaacgtgccgtggagttcacgctggaaacagataaaggcgacggcaactggagcgttgcgcaaaaagtaaccgtagcacccgggcaaaccggtgacattattttcccggaaaatatgccgggagaatggatccgcatcactgccgcacaaccggtagttgccaccgcgcatttcttttatgctgccaatgatgcccgcaaaacagccccggcggctattttcagcggactaagcaaagtaaccgatgccgtttccaacggcggattattatatggtttaggtaacgatcgccgcgcacttggcatactggcacagtcgtataaaaatggcgacgctacagtggaaggctattacgagctggatgctaatatggacctggtaaaaaaagacgatcctaaaacggcggactttatccggcagaaattcgccatcccgcaacaggcggtgacggtggaagccggcgctgtattgattgtagacgacaaaggccgcagatggcggttgccattaggcaacgaagccttcgccgggcttaccgggaaagccgccctgcgcatttgccgcgaggtgtcaacagaaagggacctgtttaattgtatgggcaccttctatgaattgcctgcggaaaacgccgacggctacgcgaaaatacgaccggtagcatcgcatcctttccggatcaacgactacgccgcttaccgtggtatgctggtaatgacaggcattgctcccggtaccaaagccggcgaacatatcgttgtatcggaagataaaaaagcgatggtatgggcaggcgctatcgatgatctctggcagctgggccggccggtgggccgcggcggtccgtggaaagatgaggcggtggaagcaggcaaggcatcagatccttacctgattggtttttattcacagcggcagctgcagttatcgcatgatgctgccgcgccggttgaatttaccctggacatcgacccggtgggcaatggcgcctggatgaagtataaaaccgttaccgttgccccgggagaaacgctgaactggcagttccccgatggcttcgaagcaagatggatccgttttaccagcaataaaaactgccacgctactgcatggctggaatataaataaggagcggcatgaaatatacagtggtctgtttactgatgtggtgttgccaggtagccaacgggaaaaatcccgtagataccggcgccgtgaaagacgtgctgggtaaccgctcgctgttaccggtggcggctttctataaaacatatcgtatcagtgacactgcagcttatgagctgcagctggcgctggaccgggataacaggccactgtactattatcggcatatttttacgccggtttgttatacgggagaatgtaaaccggtatacatcaacctttactgggacctgctgggcaattatatccgttatgatctgcccggaaaggaagtattaacaaagctggatcacaaagaatttaaacgcgacgattatgaaaagctgcaggacatactggcccggcccaattcgttgctggctgatctggctatcaccgacctcattgtaccgggaacggaaagtctcagcgattcggtggatgcccgcaccggcgctacgctgaaaaccattaaaaatgaagtgatttccggcgccgtgtacacctgttataccttgtggcatatcgcacacggtaccgtgacagatgaaatcgcccgtattacagatacctatatcaatcccgcactgctgcatcgttttctgtcttcctccaatcacgcttatcagtataaagcacttgaaaaggtgatggataaaaacgggaggataatgccgggttttgaaaatgatatccgtactttgattaatggcaaaaatatttttattgccaggtatactttgcaacaggtacatcccggttttatcagcggcgtcaaggcacagtcgtggttgtgggatacttacactaaaagcgtgtacccgttacagttaaccatgctgcgtaaactggccaccgtgccgctgagcgatgcaatggcaaagcaactcgcgaatgcgggcagcagcgccaatgaggaacagttccatttaatactggccgcattacaggccacgccccatttgccggatgcagcgatacagctgctggcaaaccagttaaaaaacaccgatgccacacgggcagccgctatccatgcgttgctgctacaacagcagccggtgaatcattccgtaaaaattaagatgcatgaatatgaacaaacgcttcatccaactgaaaaatagctggctcaccatcctgttgttgtgtatatgtacaccctggctgcaggcgcaacagcgggtatttgtagaaacagaatcctttacagaaaaaggcggctgggtaatcgaccagcagtcgtttcccgtaatgggctcctcctacctgatggcgcacggcatgggccgcccggtaaaagatgcggtgactaccgttaatttcccggagaaaggtacttatcatttatgggtgcgcacaaaagactgggcgcccttcccgaagggaccaggaaaattccaggtggtagtgaatgatgcaccggtgaaaacggtgtttggggaaagcggcaacgacaaatggaaatggtacgacggcggcgagatcaccgtggctgccggcgccacaaaaatagccttgcgcgacctcaccggttttaatggccgttgtgatgccctgatgtttaccaccgggaaatttaccccgccggatgacgcggccgcactgagtgcattacggcgtaaccttttgcatttaacagcggcgccaaaagaagcaggcccgtttgatctcgtggtagtaggtggcggcattgccggcacctgtgccgctatatccgcttcccgcatgggtttgaaagtagcgttgatacaagacagacccgtacttggcggtaacaacagctcggaaatacgggtgcacctgatgggcgatatcgacaaaaattactatcccaagctgggtcgcattgtaagggaaatggataacggcgatcccggtaacggtaaccccgatgcaaaagaatatggcgatgcccgtaaaatagccatcgttaaagcagaaaaaaatcttaccctgttcctcaatacctatgtattcaaagtagaaaaagagaaagatcatattgtagcggttaccggccgtgatattgcgagcaaccaggaaacacgttttaccggcacttatttctctgattgtaccggcgatggcacgataggttatcttgccggcgccgccttcaggatgggccgggaaagcaaagaagaaacaggcgaatcgctcgccgcagagaagccagatagctttacacttggcacttctaacttgtgggcctccctgccaacagacagcgttactgctttccctgccaccccctgggcattgcagttttcagacgaatatcatattgatgcgtctaaggcggactgggaatgggaaaccggttttggtaatttcaataccatcacggaagccgaacaaatccgcgatcataacctgcgcgcaatttatggtaactggtcctatcttaaaaacagcaagcccgaaaaatatggcaaacagcaactggcctgggtagcctatatcggcggtaagcgtgaatcccggaggatcatcggcgatcatgtgctcacccagatggatatccaggaaggcaaaatgtacccggatggcgctgtcaccgccacctggaccatcgacctgcatttcccggatcctgtcaacaaaaaatattttgaaggacaggaattttttgccggcaccaaacatatcagggtggccccgtataccattccgtaccgttgtttatattctaaaaatatcagcaacctgtttatggcaggacggaatatcagcaccacgcatgtagcctttggcagtacccgcgtaatgcgcacctgtggtatgatgggagaagtagtaggctttgccgcctatgtggccaataaataccacggcagcccgagaagtgtatacaccgatcatctccccgaactgatggacctgcttaaaaattaaacatgtacgccgtttatatcctgctgctgttgcataccgccgttgccccttccatgatacacctggaaggcagcgcgcagggcactacctggcatattcaatatgcggatgcgcagcagcgggatttcacgccgcagataacacaaatcttagcagacatcgaccagtgcctgtctgtttaccggaaagactccgagatctctttatttaaccgcgctacctcccttgaattccagctgccttatttttacccggtattaaaaaaatccgccgagatatacgccgctaccggcggcgctttcgaccctactgtcatgccgctcacagccgcttaccggcagggcaaaagaacacataccccgtggtgggaaaaggccgattccctgttgcaatatgtaggcttttccaatatccgttttgatgaaaccggcgtgcgcaaattaaaggaaggcgtaagcctcgatttcgacggcattgcgcaaggctatagtgtggatgttttagccgcattactggatcgcaacagcatcagcgactacatggtagagataggcggggaagtgcgctgtaaagggcttaaaaacggcaattcgtggaccgttggcatcgataacccattgcatcccgatcagcaactggctaccatacggctgcataacaggtccgctaccacggcaggcaattaccgcgatcactatgagcaaaacggtactgtatccgggcatatcattcatcccaaaaccggctactccacacccgattcgctgttgagcgttacggtgttttctgaagatgctattaccgcagacggatatgataccgcttttatggtaatgggagtagaggcaacgaaacagttcctggcgcaacggaaagatctggatgcatacctggtgtatgtggatgcgcagggcggggtaaaggtgtggatgacggaaggggtggggagaatggtggagtgagagagagactgttccgaagattaacccaaaaagctgtcgttattgatggctttttgttttgaatttaattaattgcatagtactgatttgcgatatctgtgtatatttaattaaactaaatattcagctgttttatactttgtataacccccggggaatttcctcttatcagttaattaactacgcatattgcttcccattttgtaataattaatgatgcttcagccgcaatacagttgcttttaagtcgggtcatttattcttttaattgatgatttttatcaattaattgacaaataaaataaatttacataactttatgagagttctacatactgcatcgggcaaatataaagaggctcgtataactttactacgaaaagtggagttaacaggcgccacaaagaagagatttgattttgattgggaaagggaagtagaatttgaaacctataaaatcacatttatcaatgatgattatattcttggactgatgtctgtttaaattaattcttcagagcgtagatgtgaaataagatttgttggaattgtcacgggagaatagaggtgattttaaggtgtatgataggctggcaggttgtttgattgcttttgcatgcaaactgtcatttaaagaagggtttaatggttttgtttctttgatacctaagacggtattaatttctcattatatgaggaaatattttttttctccaatgggagcacagctctatgtagacggtgaaatttctattactctcattacagattatttggaaaacgattaattatgaagaagaataagaaaataggtgaagaactatctgtggataacatttatcctcacggcctttccaaagaagaaaaaactgctgcagatagagaaatggcagcgtttcgtatgcagcagtggaataaaatgaccccagccgatcacctcagagcagacttattgcaagttaagtaccagatggaaagcgtaattgaatcactggaataccagggctcattgcacttcggctatttcctttctgcctatatccgggccgtgcaaaagaagcaaaaggaattcgccgcggagatcagtatcgatgaaacccgtttaagccgtattattcataataaagaatttcctaatgatgagttgtttatcaggctggagctgcactcaaacaatacaatacccgcactcagctggtttttgctggcggagaaaggcaaggcgtataatatcagtacaaataaagaattaaggaaaaaagagaagaaaaatgtgcataagacgattgcaaaaatataagttacaaatacttcctaattacctcattcttacacaccagccatataaaataaaaaagttgcaggacctgcctgcaactttttttaatagatatctcttaatatcctgggttctgcacaatcttcgggttacggtctatcacatcctgcggtaccgggttcaggtacatttttgaggtaaacacatgcgggtggttcaacggcacaatttcgtatttccatacccctgagttgttattgggcaccgtattcgtgatcttcatggcgtgtttatccacattcatcaccgtgctcacggttttccagcgaatgatgtcataaaagcgtttgttctcaaaacagagctccacgcgtctttcatgataaatagcagctcgcatctctgcctgagataatcctggcgccaggttgggcaacccagctcttttgcggatctggttaatggcattgtatacagtggcatcggggcctgcggattcattttgcgcttcggcatatcccagtaatacttctgcatagcggtagtagataaagttggcgccgcttactgcgccaccgccgggccgcaccagtggattgagccgctttttaaaataatagccggtattgcttacgtcatcggtaccaaaatcaatctggtttttggaaggacgtactttatcaatgcgggtgtatatggtgtcgcctttatccatccagttcattttatagggcgcgccgtcatatacgatccagtcgtaaaaacgcttctcgcggcctatgtaagggtgttgcggatcatagccggaagtgggatcagtaatgggtttgccattggccatattgaactggtctaccagttcctgggtagggttgtagttgccccaggtataataagcgccattgatccacaccgggccgccatattgttcaaaggaagatcccatagtgttggctactacctggcgatcccacactacttccgaatgatactcattggcttcgtaccagatagcggaaggttcgggaaacagttcgtatgatttaccgttgccataaaggtcgatgaactgtttgaaagtagcggcggccttactccagcgctgcgcatcgaagttattgtaaccggctactttgtgcgggtcgttgcctgcggcaggttgtgcggcgttgaaagcaggactggcggcatataattccacccatccttttaaggccagcgcagcgcccagtgtagcacggccagcatctgcgtcgcccttgttgtatttagccggcaggtaaccatctttggcaatggaatccagttgcgtggtgatgaagtccgttgtttccgcaaaagtactcctgggcgtgtaaatggcggcgctgtccatggtgcgcctgtcggcgggcacggtaataataggcaatccgccgatgtgcatccacaattcgctataaaaaaaggcgcggataaaacgggcttcatcgagccgtttgttcagccactcgggcgagaagttagcagcgttattacgcacctccgtaatgaaggtgttgcatttgcggatattagtgaagatggttgtccagttggtgagatcgccggaacccgtgatgcctccccaaatagtatagtcgttggaggaaggttccacaatgccctgtttccagttgtaggaagtgtaataaaagccggcgtcgttgtcgtcggtgaagttatccaggttttccggctggttccagtagttcggtaatgcgctgtaaatatcgttcaggaaaagatcggcattcccttctgtactccattgggtttcatcggtgagcttcgacttgtcggtattttccaggaattcttttttgcacgacaggatactgagcagcagtataacggcgggcaacagatgtatgaagcggatcataatatttttatttaacaggatgaatctaaaaggtgacattgagtccaaacacaaataccttctggttaggatacgctgtttccaggtcggtgtagcctacttccggatccatgaatttcattttgctgaaggtgagcaggttctgcccggagaaataacaacggacactctgcatcttcatagcttttgaaatattgagaggaagggtgtatcccagcacggcagtttttaagcggagataacccgttttcatcatccagaaatcggagttctgtgtattattagcgtagggcgactggttcgcacgcggatactttgcattgggcgtggccggtgtccagtggtcgttgtagtattcataagctgaattactgttgttgttgttaaacggcaccgtctggaaaccacggatgttaaggctggccagcgcagatccctggaaaaacaggctgaggtcaaatcctttccaggaagcgctgggcgtgaaaccgtaggtgatgaaaggatacacggggttgccgattactgtttcatcataggaatctattttaccatcgggtttaccaccgggaccgcctatatctgcatagcggatgtcgccgggatgtagcacgccaaactgggtaacgttgtagccatcgtcactgttgatgataccatcgctgtttttatcatctccctgggagaacaatcccagcgcatgatagccgaactgcgtgccggtgggccggcctgttctgctgcgattgggattatcatgtgtggcagcagtttcaaacacctggatcattttattcttcgcatagctgaaattgccgttcaggtttacttgcaggccattgttgaaacggtggctggtacccgcggaaatatcgataccacggttttccataataccctggttttcgtcggagaggcccaggccatattcaaccggcaccgttactgccggcggcagcagcatacccgttcttctttcatgaaaataatctacttccagtgtaagtaaacctttccataaagtagcgtctataccgatatctgttttagtagatatttcccaggtgatattgggattggcttccctgctgatgttggaaccctgtaccatattgccgttgccataagcataggcgttaccgtataaattataaccgttcaggtactggaacgcagatccggccaggttacccgattttccccaggagcccctgagtttaagatagttcagcacagagggacgatccttcataaatttttcttcggagataatccatcctgcggagaaagcagggaaataaccccagcgtttgccaggcgcaaaataatagtgaccatcgtaccggccggctgcttcaaaaagatatttttgatcgtagatgtaacctacgcggtatacaaaaccaagttgactaccggtaatagtagagccattgttatcaaaatcatttttgttggaactgcccattcccagctcgtcgatgtttaccgcaaaattattccgccgggcagagaagccggtagagtcattcttgcgggcttcggctaccagcagtcctgtgaagtcgtgcttgccaaagctgttatgatagttcaggaatccctggtaagtatagaactggttctttgaatactcctggttcagccaggtgtaaggtgcagcgctaccttccgaagtggatatctgtttcgtatatgagtaggggttagtggaggtattctgcgaataaaagtaaaacggcgtatgccatcctttcacggtgaagtcgttaggatcatagctgaaagtacctttaatactaagccctttaatgaaaggcagttgctgttccacggcgagggtggtcagcagggaagtagcattgcggtgggaataacctgctttcaggatacctaccggcgtattgcctgcaaactcgccccacaggccattactgtaatacatgttggtgatggggatcagtttatatgcactacggaacagttgcccgggtgtagtggcagcatctacactgttggtattttcaatggcgccaataagcgacagtgataccgtggtggtggacgtggcgctcacttccatgtttacattataatcgtaacgtttgtagttgatcgggtcaaacataccatcctgtttaaggaaaccaataccggcatagtaccgcaccactttggtgccgccactgagttgcaggttatagttttgaatcggcgcacgcatgcgcacgaggtctttggtattgctgatgggatatttgtcgggatctttggcgttcaggtctgcatacgtgttgatcagctcttcggagaatggctgctgtgcgccacccgggttttcattcatataggcttcattacgcaggcgcatatagtcctgcgcattcagcattttaggataataagtgggcgtttgccaaccgtaataagcgttgagcgataacgacggcatacctgtttgtccgcgtttggtggtgatgaggattactccattagcgccacccaatccgtaaggggctactgcggcggcatctttcaataccgtcacggaggcgatggagctgggcgcaatctcgttgatgttgttgcggatgataccatccactactatcaacggtgagttgttaccagtggtggcaatacccctgatgtgaatatcaggattatccctgccaggctggccgccattgggacgcatgctgataccggaaacatttcccgccagcgaattggagatattggttaccggcgattttgccagctccttaccctgtactgctgccacggcggcggtggaggaagttttcttctgtgtgccgtaacccaccaccactacttcatttaatccgctggcactttctttcaggatgatgttgataggatcggcggtgcttaccacttcggtttgttcataacctacgtagctgaataccagcgtaacgccggcggcagcctgcagttcaaaacgaccgtgttcattggtcatggtaccaatattggtaccttttacttttacggaaacaccaatcagcggatcgccgtgttcattttttacaatgccgcttaatttggcggcgatgatatttccggatgcaattacaatagcgttgtcgttcagtacagtgtaacgaagcgtagtaccggaaagggtttcagtgagcagctgctctacggtggcattttctgcgtgaatggataccggcggtttctccggtaaaatatcgtcgttgtagatcagccggtagcggcttttttgttgaatagctttcagcactgttttaatgctgactttctccagggagatactgatcttttcctgggtggcggaggtggcgtataccggcgtgataccggttagcagcaaggccaggatgagtataccaggcagcctgccatgcagacttttaataaaagtccataggaacattatcttcataacatggaatgtaaagagggtgaacgaaagttaaaagaacgggtttgtaatgtttttatgtcatagcatttatttttgaagatgataaatacggtatcaattactgatgcggacgtccttcccgttgatccggaaattaaagggccgcgatagctgcagcattttcagtgtctcgtctattgattctgtatcgatgatgccggaaaaccggagttgttgcagttgggcagattcaaagtgtatagtaaccccgtaccactggtgcattttcaccgccagttcaccaaaggtttcgttgtcaaataccagtttattattcagccaggatatttcgcggagctgtccgctgctatctttctccaggtgtttttgctgcaagacaggcgccagccgggttgcagggaccattagtttttcttcaggttgcatcaccacagtttttccgccaaacgataccgcaatttttccgcggaccagcgtagtggacacggcgctgtcgcccgtataggctttcacgttaaacgcggtgccgagtacacggatgtttactttccccgcatgaataataaaaggaacgccttcgcttttggcgatatcaaaaaaggcttcaccggtaagtgtaatttcccgctgttgctggccaaagctgtttttttcgtaagaaagctgcgtgttgctgttgagccatacgatggagccatcgggaagtatcaccttcgattttccgccgggagcggagctgagttgttgcaccgcaggggccgtggtgcgcgtaaaatgccacagcgtccaggctgctgtcagcactgctgctgccgctgccatcgctaccagtttgcgtatattgttgcggggaagttgcgggttcacggtttcccatatacgttctttactgtgctgcatatcagtcacttcctgcatgggcgactgccagatggtggcagcaagttcctgcgaagcggcagcctccggatcatctttcagcaatgtttccagttctgacagttcttcacgtgaaatatcgccgctgaactgtttaccgagtaatatccatatacggtcgttgctcatagtactattgaaaatggttgacgaagggcacttcggggtataagacaaccggaaggagataatacccccaagagggcaggaattttttttgagaaagattactggtcgcccggaagcggcgtagtgaggaaggactttattttagtgagttttttcagcgcgatgcctacctggttttctaccgtttttatggagatgttgagcagcatggctacttccctgtatttgagctcatcttcttttactagtttaaagatgaggcggcactgcgggggaagttcgctgatggccgtattaatatgccgcatcatttcattgctgatcagttgcgcttcgggatttatttcatattccagtaaataggcttcatcgagatgcagcgtttttttatgggcatatttacggagatagttaagcgcgatgttacgggtggctgcatagagataccacttcaggttgcttacctggtgaaggcttttcctttttttccatacggcaataaacacatctgcaactatttcttccgccatttccctggaatgaacaatcgccagggctaattgaagtaatggcgcgcaaaagtcatcgtacaattctttaaatgcctgtgtatcaccggtgtatattttgttttgcaattcggggatatcttcgcgcatgatagtaaaaatacccaaattatgtaaaaatgcaagtgtataatattaagtgtccggatgacatatagcttacccttgaagggtttttcaccgggaataatcaatatatataacagacaggataatatactataagaaatatcttctttaatcctgtttctttgaatatcatgctgttatccaccggtgaaaataaaacgtccgggtacggatttttttttctaaattaattatggtgaaaacactcatttgtactactcccggtaattttgaatatggtttgcaggcaatgccccaggtgcaggctgggcatgctattatccgcatccgcaaaatagggatctgcggcaccgatctgcacgcttttgaaggtacccagccttattttaattatccccgcatcctcgggcatgagctggctggtgaaattgtagacctggacggcataacatctaccagctttcacataggggaactggtaaccgttattccatatgaaaactgcggcgtttgtattgcctgccgcaacggcaaacccaattgctgcgaaaatatcgcggtattaggggtgcataaagacggcggcatggcagagtacctgtcggtgccggaacgcctgctggtacatggcaatggcctcaccgccgaacagctggcactggtggaaccgttgtcggtaagcgcacatggcatccgccgcgcagccgtccaacccggtgagttcgtactggtaatgggtgcaggtcccatcggcctggccgccatggaatttgcccgcattgccggcgcacaggtaattgccaccgacatccaggataaacggctgcagtttgcacagcaagcgctgggcattccttttacgattaatgccgctgcagacgtagccacgcagctgcgcaatattaccggcggcgatatgccggtagtagtaatagacgccaccggtaaccagaaagccattaacaacggcatttattacctggcacatggcggccggtatgtactcatcgggttgcagaaagacctgctccagttttcccatccggaatttcataaaagggaaaccaccctgatgagcagccgcaacgctacccgcgaagattttgaacaggtgatccgctgtatcagagaaggacaggtgcatccggataaatacattacccaccgggtgaaattcggcgacgtaaaaaccgcctttcccacctggctggatccccgtaacggagtgataaaggcgatcatagatatctgatcccttaaccgatatcaaaaacagttgacgatgatgaaatcatggctcttgttgctgctcctgggtactacccataccattgttgcgcaatctgtttcattgcaacacctgctatgtgaataccaggataatcccatgggcatagatgccccgcaccccgcgctcagctggcaactgcgaagtaaaggcaccaacatccggcaaaccgcctaccgcgtactggtagcggataatcccgctgcactggataaaaaccgcggacgcatctgggattcaaaaaaggtgccgtcggatcagtcggtgcaggtactttacaacggcaaaccactgctgcccgctactacctactactggaaagtaatggtatgggatcagcagggaaagccgtcggcatggagtgaaacggcgcagtggcatacgggcctgttttcgccgcacgactggcagcaggcgcaatggatcggttatgagaaaatgccggatactgcacgcatcgttcccgctattaccaacgacaacgccccaaaataccggtaccggaaagacatactacccctgctgagaaaggaattcaatatcgccaaaccactgcaaaaggccactgtttatatcagcggactgggtcagtttgatcttcatctcaacggaaaaaaaacaggcgatcatttcctcgatcccggctggacaaaatatgatcaacatgccctctatgttacctttgatgtaacggaacaactacacaccggtaccaatgcactcggtgtaatgcttggcaacggcttcttttatgtgcccggtgaaagataccgtaaactcaccggcgcgttcggctacccgcaactcatttgcaggctgcatctgcaatacaatgatggcaccacggaaaatattatcagcgatactacctggaaagcaacacccggccctgtaactttttccagcatctacggcggagaagattataacgccacattggaacaaccaggatgggacaccccttccttcgacgatgcgtcctggcggcctgccgtaacggtaaccggcccgccgcagctggaagcgcaaaccgccgctcccctgaaaatattcgaccgctttacgccgcttaaaataacacaaaccggtactaacacctgggtgtacgatatggggcaaaatgcgtctgctattcctgccatctccctgaaagggaaaaaaggaatggtggtacgtatcacgccggcagaactgatcacggaaaagggcctggcagatcaatctgccgtaggcagcccggtattttttaattatactttaaagggaacgggtgcagaatcctggcagccgcagtttatgtactatggtttccgctatatccaaatcgacggcgccgtgcctgccggcaaaagcaatcctgcaggattgccggaaatacaaacactgtatagcctgcatacccgcaacgcagcgcccaccatcgggcaattcagctgctccaatgaattgtttaataaaacctttaagctgatcgactgggccatccgcagtaacacagcaagcgtgtttaccgattgcccgcaccgcgaaaaactgggatggctggaagaagcacacctggtaggcagttctatccgttataattacgacattgccacactttgccgcaaagtagtgcgcgatatgatccatgcacaaaccgcagatggcctgatccccgacatcgcaccggagtatgtgcaatttgatgacggcttccgcgactcaccggaatggggcagcaacggcatcatcctgccctggtacatgtatcaatggtacggcgataaatcggtactggaagaaagttacccgatgatgacccgctacgtaaactatctctcgcaaaaatcaaatcatcatattctgtcacacggcctgggcgactggtacgacatcggcccgaaattccccggcgaatcccagctcacgccaaagggtataacggctacggctatatactattatgatctcagcatcctgtcgaaagtagccaccgtactaggaaaaacggcagacgcacaaaagtacgaagcgcaaagcgaagccgtaaagcaggcttataaccgcgccttcttcaacgacagcaccaaacaatatgctacgggcagtcaaaccgccaacgctatgtcggtatacatgcagctaacagatccccgttataaagccggcgtagtggaaaacatcgtggcggatatccgtcagcataacaacagtatcactgccggcgatatcggttaccgctacctgctccgcgtgctcgacgacgaaggccgctcagatgtaatctttgatatgaacagtcgcagcgatgttcccggttacgggctgcaactcgccaaaggcgccactgcgctcaccgaatcgtggcaggcctaccgcgatgcttccaacaatcattttatgctgggccacctgatggaatggttttacagcggccttgccggtatccgcccggtgcccggcagtgttgccttccacgatattgtgatccgcccggaacctgtgggggatgttaccttcgccaaagccagctacctttctccctatggggaaattgtgagcgactggaagaaggaagacaacacgtttaccctgcgggtgcggatacctgccaattgccgcgctactatttatgcacccgcagaatccacttcagatgttaccgtaaacggagtagccgtagcgatagagaaggggtataaagaagggcgatacatcatggaaaccggttccggggagtatttgctgcatgtggtgaaccggcggccggtgacgtcgtcggcggggagttatgcggggaggtaatttatgtgatggtaccttctgcctgatgggagtgtattattatttgcacgtgtggcacgcggcaaggatactaaccccaatcgttatgaatgaagcatcactccaggtaatcctcaggaatttaccggcatttctgcagcggctgaataaaaagcataaggctccccggccagcgggcatactgggaaaaacggatattgcctaccttgaagccgtgcagggaaaccagcggcaacagcaggaacaaatttccttttacctgatactggcatacagccattatgcgctgggcgaaccacagatggctgttcattattttgagcgggcttttatcttatctgatgactatttcccccagggcgatatattggcaaaagtttacctggatgcattgcacgccgtggcagcgcaaacgggcgatctttctttgttgaataatggtttggagtgggcgggaaaatttgagttcattacgtttaatgtgcataaggagctggcagcaatttactaccaggcaaaagactatcacactgccgccgctctctggagccaacacctgcaaaatgtccccgactgtgtaactacctgtcaccacctggtcaaagtgttatcggaccagcgtcgctatgaagcggcgatagcggtgtttaagcatgcaccggcgtctgtgcagcaggtatctttcttacagctcctggtggggcattgttataaagaaaccggggaatacgccgaggcggaaaagctgtataaagccgccatgtccactcccggcagcgaccaatgccagcctatgtgcgcactggcggagttgtatgcggaaagtcttacggattaccagctggcgcatacctggtaccagcaggcagtagatcagaaggggagcagctatgatttgttgcatgcaaaaatttcttacctgcgtttcctggtagaccagggagaaacgtccattgcggtttccctgttgttgtttatggagcaacagctcaattacaattatctccgcctgccggcccgcgatttgaaccgggtagcctggtgcctgtatatactgaatacccggatggatctggctgcgaagttcgcccgccgggctgttgacctggatccgcatgtaatggatcatgtacacagcctggtagctatattaatccgtttaagggagtgggaaaaagtgacgccgcatgtgcgtcactggctgaagttctccgatgatgaagccgtgaaagcctcctggagggattacagcctggtgttccaggataccattatgcaggatcaacaggccactatggaagcgctgttatatgataaaacatctcattgctggcgtgctatccggtgcgcattgtataaaacgtcggagtatggggaaacggtggctattcccgatgatatttatcctgttgcagatcagttatacaaacaatttattttcagggatatgccgcgcatattcccggagtagggagggggaaaagcccggtaaaattgttttaccgggccattttttttaagacaggaacaaatcccgctgcagcttgccgcccggcactaccgcatatttatcgaagttggtgatccccatcgctttcagcacatcttcatcaatcaatgtatttcctgtgtacgacgagggctgttgcaatatatattctacggcgtcggcaataatttccggggtacggcttttgttgatcagcgagtcgcctcccagcaggttttttactgccgcggtagcaatggtggtggcaggccatagtgcgttggaggcaatgttgtatttctccagttcattggcccagcctaaggccagcatgctcatattgtatttgctgatggtataggctacgtgtggtccaaaccatcttgggtcgaggttcaccggtggcgacagcgtaaggatatgcgggttatttccttttttcaggtaggggaggcagtgttgtgttacgaggaaggtgccgcgtacgttgatattgtacataaggtcgaaacgtttggcgggtgtttcttctgtattggtgagctggatggccgatgcgttgttgatcactacatcaattccaccgaatttttctacaccctgttgcacggcggcggctatctgtgcttcttccctaatatctacctgtacggcgagtgctttaccgccggcagcttctacttcagcagctgcggagtagatggttcctcccagtcttggatcttcttccacgcttttagctgcaatgataatattggctccccggctggcgaggcgcagcgcaatggctttgcctatgccgcggcttgcgccggtaataaagatggtacgttgctgaaatgacataacccttgcttttagcggtgagaaagaaaaaggaatttaaggaatctttctctgacggcaaaaagcaagggttattttgagggacaagtgattgccggatcaggattgatccggcatactaatggggatattcaatctcttcattgactacttcgaatgatagcgatggaacagttaaaataggattcaaacagggtagtgaattcgtctgcattgttcattgctatggaagtacaaattttttcagggggatcgggagacgtgatgacagtgccatatgcctggatcatctggcgttggaagtggaagtgttccggcgtcataaaaaagctattaacgaaggcttctctcaattcctgtgtgccgaggtccagcagtactgccattttagccatggaaaacttttcgttggtgacattcaccaggtatttaatggatgcctctaatttttcagatacatataacgggaacacccgcatgggctcatcctccagtttatcctgcgccgcaaaattgaaatacagctccaggcagcaccggtgcatgaatatttccgcctgtttgcctacaaacttacagttgcagatggcatcaataaggtctgtacatgccaggttgatatgatacggctctgcgttgataggcgcactgccttttttggatgttttcttaactattgccgccagttccgggtattccagtgccagctccttcaaatcttctggtgtgatattaatatggaagctgaacatattatcccaaggattcatgggtgctttatgcgcgctgggttccagcttgaataaggtcatttcccttttggccatcatatacggcccctggtcggtgagctctgctactatttcgccaccagccataaagtgcagggccagcagctcaatttttgtataaggaaccagcataatgggatgttccttattgaatacttcatgcgtacggagtgtgaaccggccaaactttatcgtttggctgatgatatccacatagtcatcacttctgaaatagattttagcagccggcatggccaggtgctgatattccgggggtaaactttcaatagagatgaaatcctggtcatcttcatcgattcttaaaggtatacgcgggagattactgggcgctttcataacattattttttttgtgaaagtggtgtaaaaatgtctgttattgttttgcctgctgaccgggctgattgaagtgttttataggatagcaacaaactatttcaatctggcctattcagttttgtatcttaatatttttctttcgtcttttttaaggttaatcatatatagtacacatgcgaggttccctacgtactatgaatatgaaaaaataatttatttgacattttgagtgtgattttgagaaaaaatgggtcactaataagaatattagcgaccgacacatgagtgcgtaaggggtgtaaaccatccacccacttacaccgcgtagagtttaattactttgtggccaggtagggagaccggctttcattttttgaagggtttcggcgtagactttttcgtctggcgtacctttctttaattttagtgctttttcttcccacggtatagcttcattggatctatttgttttatgaagaagatgagcatatgtatcgaatgcctcaggtgattggtcccatttttcaattgcatatttcatgacatcaattgcaaaatccaaagtctttgggtcgttgcaatgttcgaaaatgagccatgaaaagttattaatatcatattctggtcgttccaatgctaacttaaaatatagcgtgtagtattttgcataaatattccaatctttatggcttgactccacgccgtagtataacattcgtttgccaagtactaattcttcaccaactttaccatatctacttgtcactcgttgctctatggtctcccaatcagggtttgttttataaggagctatttcctctgcgtcgattattgattttactttacttattgccgcagtttcccagaggaacgaatctactttcctgggttgctctatgaaaagttgaaaacctctatctttactggtctttgttattcttctaataaaagttaagttatccttggaaaaaggattcgtcaaaatgctgatataattgttccctattatggtagttgttgattgatcttttttgcgtatggatattagtataagtcttcttagaaaagcagaatctcttcccccttttttataatcatcaattagtgactcatagcgactatcattgtcgtttatattcatattcgttgcaataacgaaacttggatctattgcaaatcctttggtttgttttaccagttcttggttgatggctctcaattctgtaacaggaatcttaattatctctctgtcataggtaagtaggccattctcctctccctcaacatcaaaaggttgggtataaatggaagcgcttagaccagcgacctccaatttcttaagctcacttgtcatatggatatacttagtttttagttcttccggagtgacttgtatatagccccagccctgcatatcgtcccattcatgaccaggaacaggtacacccacaccaccaaattcaccaattacacgagccttattgggcaagggaggagcatttattggatctggatatgaatgcacatccgtcatatcactaccaatccacggatcatcagcaggtgcacgaagttgattgtttacataaagcaattcgccagaatgtccgttgattatcctgcttggatcatatttttttacccattctgttagccttttttgatcatatgccccccatcgctcattaaatagaacccatgtaataatgctgggatggtcatgtaattgatctattgtttcctgtgtttctttttcaaaaatagaatcatagcctttggggtatccatgaggtggatttacaaagtcttgccaaactagcataccaattttatctgcgtggtagtaccatctctctggttcaacttttatatgttttcgtatggtgttaaaacctaacgattttatggttttaatatcaaatgctaatgcctcatccgttggggcggtatataatccttcaggccagaatccttggtcgagaatcccaaggttatacgtatacttattatttaaaaaaatacgatctgcacctttttcatccttttgaatgtttatttttctcattccgaaatagctctctacctcatcaattattttatttttctttatgagttttacagtaagatcatacaggaatggatcgtcgggagaccataatttagccttaggtattgtaagtgtataatttccctgattattggttattggaaatttttggatgcttactactttgtcatttgctgatgtagtaatttcaagccctgtattttctattttcccttttgttgtgatgcttagagctaaagtacttttgtctatatctggagtagtttttatatttgctatatacatagctggaacagtttccaaccataccgtttgccagataccacttgatgaagtataatatatattcgtcggattaagaacttgttttccatgaggattgggccccttgtcactgggatcgaatacttttactaaaatttcgttgttgtctggttttagtaaatcggtaatgtcaaacgagaaactttgatagcctcctgtatgcgttccgatttgttttttgtttataaagattgttgcttgccagtctacggcgccaaaatttaatataatacggtcgttaccttttatggccggtttttggattattttcctgtaccataaacgcatctcaggaaatagttttttttgtacacctgaaagggcagattcgacaggatagggtaccaatattcttccttcaaaattggcaggcaaagttgttgttgagtctgtaatggagtattcccaaagtccatttaagttctgccattttcgacgtttaagtaaaggcctaggatattctttcaatacattattcgggttcacttcttttgcccacctagtttgcatgtggataggagacatttgatagctagtagatatgggtgttttatcctgagtatagcagggtgaagagattaaaatcaggagtccggctataaaatttttttttctcatcagtcaataatttatccagaaattgtaagtatgtgaatacaatctatttttaaattttaagtatactacacgggtggcatattaatatcctgtattttgagatagatttccatttgtaagtatatcgtttgatggaatagggaacaattcccagtttagattccatgatcctcctttcaatggagtcacattcctcattacggtatccacaatatgaatcctcttcatatctagccacctatgtccccattctgtaaatagctctacctgcctctcatgataaatgctggagagtaatgcagatttttgatttaattttgattcatctagccaagctcttatacgaatgatatttaagtcagcacgtgaaccggcgatcttgttttgttgtgctcgtgcttctgctcttataagatattgttctcctagacggaatattgtattgtactctgttaacggagcattaagagcgccagatttgtacttgaatacaaagtgatagggtatgccagtaattaatacagaatcaatccataacgtttttcttcggtcattggcttcaaagctatttaatagttgtgggctgagatatactggcctagatgaagatggtccactacgtggaagtatataaactttagcatcctccgtgtttgaagcaaaattgactggttgtaattgccaaattgcttcgcgactattcattaggaatgtattgttcaaagagtctaaattgtataatgttgtattgtttatgatttcagtggattctatttccgcatttacccagtcgtttgtatataaataacttctcgctaatagtgcggtagcggcccatttatttggtctaatacgttcaatacttttttttagtagagtaccatcgacataatcattagaaagcaaaattttggcatctttaagatctgatataatttgcatccatacttgcgatattggggcacgcggtaaggtactatttacagcataattggaagttgtcactaatggaatatcgccgtatagatttactaaataaaaattgcaaaatgctcttatgaattttgcttctcctaatagttgctgtctaaccccaggtgttagcgaaaaggagttatttagcctctcaattgataaatttgcaatatatatttcgttatagatattggcccaaaaatctattcgtgaggtaatggtagccagattgttttgatagtatgctctcaatcgtacatctttggcaccagcatatagagttagctcatctccagctagtcctgttattaatccaattgctgatagatcatttcccgttatgctattcatactaattctagaataaatgcctgttaaaacggctgacgctgtgagattattagtgtatacgttatctgcagttatgctggtggttggcgcattgacttcgatcaatttttgacaactcgtttgagttataatgatcattatatgggctgaaaggagaaataaaaatgtcgttttgttaatgggatttagcattgaatacatcttcttgtattttatggtgaggatagattagagtgttatttgtgctcctatagtaactgttcttaatggtgggagcgataatccgctttcaggattgaatcctttatagtttgtgaccgtaaggatattttgagcatttagaaacacttttgcattaataatatgtagaattctgttcaaatggtcagggaattgccatgaaatagagatgtttctgaggctaataaaggatgcgtctgttagaatagcactgctatactttatgtaatctaagttctcgtaatgctccgcgctataaggctgtatttgggctttgtcaccagtcttttgccaacgatttagaacggtagttgattggttaccggcgcctccattgaatgtacctggataagcgatgtttcttaaaccataagtaacatcgtctatagttgttcttttcgcaaacattaagaagatatccatggtaaatcctttataattaaagctattttgcaagccaccatataattttggatccgtatttagtgcaacagttttatcaattggatctgaagggcttatcgttatatttccctttgtatctatgaattgatagacgcctgtggtgtcatttaatcctgcataattataatatgcgatagtcgataggggctttccaatatatatcgaattgtttttgtctcttccgtagtatgaacgcaactgattctttggaatcgttatgttaaaatttgaagtccaatagaaatgatccttttttatattggttgtggtgagtgataattcccaaccggtgttttgtattacagctggaaaattgcgggttattccggtaaagccagtaatgcttggtagacgtgcttgtgttaactgattattggagcgattttgattgtaatttacagtaagtagaatcctatcttttgaaagaccaagttccatcccaatttgaagtttcctagttttctcccattgcaggtatggattcgttattctgctaggagaaagtccaattatattttgatacgcatttcctgtcacataaagtggctgatatatgtccatgaatctataatcacctatttgatcatttccagtgctaccaaagctacctcttagttttccaaagcttaaaaatgggattttagattgtatgaaaggttcttgggagaagatccaggctgcacccacagccccgaaattatgaaattgattttctggtccaaatcgagaactaccgtcacgtcttgatgtaagattaagtatgtatttatcgagccaattataagtgactctactatatatggcgttatatttgtatacggcgttgatgctacttcctgttaagcttgtggcggaacttaaatcctccattacaagttcattgctgaacccaagtgctaagacattttgttggtcgctattttgttgtgttagtgagctgccaattagaatgtttaagatgcctttatttatcttcgttttgtattctatttgtggctctacgatccaggaactaattttattctttataaaaactgatgcatttgaaatatctggttgatactccggctggtaaattgaattcgggcttttggttatttcatcagttaatagattgttaaaaccaaaactacttttaattatcaaaccaggaagcaattcataactaagaacagcgttcccaattagatttgatgttttgttggtactgtttagtgctgtcgaagcaaatggatttgctgaaaaagaactggctccagtcgcagttggcatccagttgatagttccgtctgaattatatggcttaggggcattgggagctaatgtgatcgcgcttgtagtcaagtcatttaaaggcaatttattgtcatcgaaaataaaggaaccagtgaactgaattttgaatttttgattgagagaattaccgcttaaatttaagtgaagcgacgcttttgtgtcagagaaagagcctggatagacagttgtctctctatggtatcctcctcccaatagaaattgagttaaagcattacctccggatatatttaattgcgcgtcagtatattgcgcggattttccaatgagttctttttgccaatttacattgcgcattgtatcccaagtcccatttagatcgtagtcaaatggagaaatggtgttaccgtcattttttattgcttctcgtctcatcgcaagataatcttcagtatctaagaggtctattctttttgacacttttgcccatccactttgaaacataatatttattcttgtaggaccagattttccttttttggttgttatcaacactgctccgtttgcagctctggatccatatattgctgtggcgtctgcgtcttttagtatttcaatactttcaatatcggcggagtttaagtaacttaaaggattgcccgaaacaccgtttacacctgatccaccagttatagtattataaataggaagcaattgggatacatatggcaccccatcaacaacatagaaaggatcattgccgcttgagatgctatttactccctggatacgaacagttactcctgatccaggtaatccatttgattgttgtatataaatgccggggacacgtccttggagggcatttaatgggttgccaactggttgtctttctatgtcagttgctttcaaactacttatgtttcctgtatttaatctcttagttgtactcccataagcaatgacaaccttttcatcaagtagatttgtgtatgtattgagttgaactaagatattattcttaataattacgatttcttttgattcaaatccaatagaagttattacaataacacttcctttgtcaactttaggtagccggaatgttccatcagagtttgaaatcgtaccttgattattactctttagctttatcgacaccccaggtattggattaccatccttgtctagtattttaccaatcaattgaaatgtgtttggtattgtatcaaatttatttatcgataaatttgatctttctctaagaatatgaatttcgttattgtttagagtgaagaagagattttctttatcaattaacaaaaaggtcattacttctcttatgtccgcctgcttgaagttaactgtaacttttttttgttcatttaggaatgtctcgtgaacattattatatatcttaattccagtttgtttttgaattttcttaaatgccttttcaagagggatattattggctgataacgtcactttagatatttgacgttctccttcgcccattgtcgaggttgaataacaaataccggttagtattgcgattatcaagggaagttttgatgtcaacactcctaaatgcattttagtcatacagtatagtttgataccaggtttggaatttgctcttgtattaaatattacacgcaaattgttatagtcgtactattcaggccagtcatatttgtattgaaagtatattttttaatataatatattctaaaggcagatagtactttagatattaactcgtgtatagagtatgctatattgtttggagttcactttagacaaacaggtcattttaatccaatatcatatatgccgtatgcgggctgcaattatatcacattgtcaagtgctaatttaactaggtttattccattaattcatttagtgtgaaacccgcttattatatattattaatcagtaaatagaaaaatgtttatatgagaggaattttcttagctatagtttttgttttttcttcactaattaattatggacagactgttccgttagaaaagaaggatcatccttcctctaatgataaacttgtcatagattctatggcctataataagtggacttttgtcgatggcgcaaagatcactgatgatggtaagtttatgtcctattttattagaaacgatatcaagtttaacgacattacaattttgaaagaatgcaaaggtagttgggaaattagaattcaaggtattagaagcattcaatttacaggagatagtaggatggctttctttgtttttaatgacaccttatgcatgataaaattggggcattcttactttgagaagataccttttgtcaaatctgttaaggtaccttccgtaaagaatggggaatggatcgcgtacggaaatgcttcacagaaatcggtagtgctgcgtaatcttaaaagtggcgatacaagaccttttgattcggtaaggaactatttctttagtgaggacgggaaagtattgatcctagagagtattgaaagggatagtagtggtttttcagaagcattgcgggtggtacaggtaatggatggtggtattatgaggatatggaaaggaaaagggctatctaagttagtattaaattcatctgctactcaattagcgtttatgctctcagatgaaaatgggaaaggtaagtctataatgtattataagaagggcgccttgtcaccaacgttcgtggttgatgtcgactcgattggaggtgacaggtcgtttgttataaatagtttgtcaggtttaagtaaggatggtaaatacgttttctttacggtaaaaaaaatcgagaatatagatgtaagtagaatgacaaactcgacagtgcatgtttggagttatttggatgagaagctacagtcggctcaaattgtggatggcaaagaaactgctgaatttttgtttgcagtgagcttggtggataagagtattattcagatcggtcatgagaatgaatggattttaaacaagagtttagatgataatacgtttttagtgcagcatatgtcaggagatgctgatagttacgaatggaaatggaataccgctgctcagatttcttattacgtgaggtctattcagagaaatactaacactcttctgaggcctaaaggcgtggtaactattaatttgtcggatgagggccgatttgtggtttactatgatagtgattcggcaagctattttagttatgaaatgtcgactggaatatatcgtaatataactgcaggtttggatgtctcctggattaattcgttcaaggaagatttaattaagactccgagaggtattttaggttggttggagagagattctgcgatattaatttatgataagtatgatatttggatgattgatccactgggaaagaatccttctgtaaatctaactaacggttatgggttgaagcatggtattatttattatatgggactctctacctttccaggagctgcttatacagccaaggatacattaattctgaatgcactggatatatatagtaagaagaacgggtttttcaaaaaaataataggcagtaagggggatccggaaaaattaacaatgggggactgtatttaccaattaattgataatccctatgttgagaataatggtgttgctcctattaaagcaagaaatgcaaataaatacattgtcatgcgaatgagggctgcggagtcccccaattatttcttcacttcagattttagatcctttatttctcaaagtgcaattcgtcctgagaagtcgtataattggtacacgacagaattacatagttggaaaaaagcggatggttcttcaattcaaggggtattatataaacctgataattttaaccccagtttgaaatatccagttatattttattactatgaaaaaaaatcttttggactaaatgcgtatttaattcctgagaatatatccggttgctgtaatatgaatatacccactttcgttagtaatggctatttggttttcactccagatattgactatactattggcgatccgatgcaaggcacatatgatgcagttgtttccgcggcgaactatttgtcaactttgccttttgttgacgcccagaaaatgggaattggaggttgtagttttggtggtatacaaactaattatttagttacacatactagtctgtttgcagcggcctattcttcctcctcgatgtcggatatgattagtgcctatggggatgttccaggtagatatattagtttacagaattattttgaggctggccagggtagaatgggggggactctatggcaaaaacctgagcagtatattaaaaactcttcaattttcaacgctgataaggtaactactccattattactgatgcacactagtgatgacggcattagctcattttctcaggcgattgaattgtttactgccttacgtcgtctaggaaagaaggtgtggctactagagtataccgatgctaatcacgggatactgggagaggctgctcaggactttagtatacgcttatcccaatttttcgatcactatttaaagggcaaagctgccccgaaatggatgacaaagggtgtgcctgcaaaaaacagggagaaagaagatccatataaattggatctaaatataaagactcctggaaatgggttgttaattgatttgcatagataaaatttgaaactataatcaagatgtatcgacataaacttttcaactttcggccgatgatattaggctttgagatcttgattgtgaagctttaaaaggagtagacgccaatttttttgaatgttgtgcgtttatatgagggggccctaatagtgatgttattaagttggcttgctaaaaaaaaagtttgtgaggacttagaagtcagtattgaagacgaagtatgaattgattttaattttaattattggaacgaagtctatttatttgtgaatactaggactacggttgacagagcaaataaacattttgaactggattttaaatctgttttaaggggaaggcgctgctgccgcgccattccccttaccccatcccggcacgggtttcaaacaatggctacgttttagattgtagtcgttctctaagtatttcgtagggtgttttgcccttcagtgcagcattaggtctatggcagttatagaaattctcccactcctgtaatttcttattgatgtcgatgtcatctgtgtagtcaagcagttggtaaaactcttgttgatcggtcaaatgggaccgttctacttttccgtttaaatgtggactagctttccttatatacacatgttgaatgcctaaatcttcgcaatgccaatgaaattgcgcctgaaattcatgcccgttatcggtttgaatagtatgaatccggaatggaaatttgttccgtatgtagtctacaaattgaattgcgcaactctgattatgtttactatatattttcagagcccgagctcttgttgcgtcatcaatcgccgtatattggaagcgcttaacttccttcccagaggacttatcagtaaaagataaaaatttaacatcgacctggattctatgtcccggcacctgtttttcgtatcttttaaattgttccatggatcttttccgctgattttgcggcaatttattaagcccatttcttttaagaacattatatactcctgcaggagaaacagcaatatcatggtaacgtttcatataccatgatattcgtaattgtcccaaatgataggtggttcttaagtgtataatctgagcttcaatatcagctgcaatacctagcttcggattttcaggacagggtttactattaactaaggcgctttctccttcactttcatagtctttcttccatttatagtaggtttccctggatataccaaagtatcgacaggtttttgatacattccctgacgcttggccatgttgaattattctaagctttctacgaatatctgatagttcttttggactcatatatagacatttgattgacaagataaaaactgtcaaacaaagtcatgatttccattatttatttattcttgcctaagaaataggaaaatccaatagtgaagaagcgctccaatacattagtgctaatatcttcaatatagttgtcttgaatgatgcgattataacttatattttgttttagtacatcaaacccttggatttttataagtccttgtctgttattaaatattgatttgctaatcgaggcatttaacattagtggactcccattgtacccctccattcgtccagttgtccatgcaactataagattagagttcaaatttattccgtatgggagatttagacggttcgcaaatgataggccaccactaacataattttccttaagctccttattgttattatagcttagattgttatagtttatgcttcctgttattgcgcattcgtaagttttccgagtatagcggaaacttatcacttgagttagggatgtttgattacttatagattcctttccatttacaacacttagagatctttttaggctgccttttgtgtttagattaacgccaaagtgttgcttcttgaatggtaggtagttattaatgtttagttcaagaagatagttgccatttaaattgactggtttagtagcttgacggccaatggaatcaaagaatgagagattgactatctgattgattatgaattttccacttgtagcaatggtgagtgttctcaatgtggaaatgttaatagagttatagttgaattgcaaatcgtggaaagtgatgggttttaacattggatttccacgttttatatttaaagggtcgctataatctggagtttgctgtaactgagatgcttgcgggaattcgatactttttctatataaaaactttaattttcgattattcctcggtatgaagttgatggttgcttctggtagtaaggcaagaacattagtcgaataaatgttacttacactattgtctttattctccatactgaagtatagtgcagctagggatacagagtagtcaaatttttcttttttaaccagccaatttaacttggcgtaatggtgaattggaacagtgacgaatatattgcttagactgtcatttgctttatcatatagttttgtcatattattgtagtctaatattgttttatttaatgaaccttttacccgatcttcaccaatcataaaacttatggctccatagttgtgtatgggttcagtataagtagccatgacaaatagttgttcgttttgggtgttgataatagaacgttgatcaagtgtgtctgatatagtttctcggctatttggatagtagagggtgtttgatatgttgtatccaatctgctttgatacgcttttactataacttatactaatattaaggagacgtctgtttttattaaatttcttttcatagtttagacctgtaaacgctgttatggtattattttcgtccatagtcttaaaagttccgttgcctagtacttgagcataattccctagtgaattaaatctattagcgaagttattatctgttttaaaaagtgtgagttgatttgagatagttatattttgtagactgtcaatttggtattctatttgtgttgttagtgcttgatttctatctttattattgctgcttgatttctgttgaattagcaaacttgtatcgcttattatattttttcttgcactgttccgttgagtttcgcttatattgttattcgctatatagtttgcacttatagtcgtattcttgttgattctgttactatagttcccagccccattccaattctcttgaatgcccccaacactagtcgttttggtctctatagcaccgttagtgttgtcgccgttacctagcaatagaagctgctcttcacctttgaatcgactaagacttagcttggtggagaatcggttggccgttccgtaagcgcctgaaatctctccagagattaaattttgtttgcttttcttaattgtaagattaattactttatctggttgattggaactcgaaccattaaaatcttgtctgtttgttttcctatctattagttggaccctatcgattaagtctgcttgcaaattcttactaataattctattgtcaccaccactgaaaatgggtcggccgtttatcataatgcttttcacaggctctccattcacactaattgtaccgtctttgtcgatctgtacaccaggtaataatctaaatagatcctcgaccaatgcattgtctcgggtttcaaaataatttgcattatattccattgtatcccttgcaattcgtagaggtattctagtttctacaatcttaacttctgttaatgttagccctgttcgttttattccaattgtccctatgtttataagagtgtcagtggatgaggcatgcaatggatataataatttttcgtatccaataaatgatacgagcagtataaagttcgtaggtgtaaggctgtcaattataaaaaatccctctttattagtgaatgataggcctgctttggaggaatccttagcgtacagaaatgttattgttgcagacgacaggttgtcttgtgtctccttgtcagttatgcgacctttaattactaattgatgagatttttgcgccgaagaatgtgaggttgacacaactattaataatagcattattaactgcttcataatggggatttccaatatcatgtaagatgaatattttgaacgcatctgtattgcagtatttatatggatctttgtttgtcgtttagaggagacgaattttttaagaaaaatgtttcgctgtatggagatggcagtggttggatttaattttgatttgactaatgataggtaggtagctctatcgtaattcaatttagttgcactattgttagttatgagtaattgaattgaaccctcaaataaatcataccatgtcagtaataacttctttttttacaatccggatggagaaaatgaaatgccaattccctgctagaatttatcttgaattgtagtgctttgccctgttgtctagccctctttttttttctatgaactccgttgtattatatgtatacaggtgaatacggaattagctcaaactatatttgtgccggcactctattaattatctttttaatcattgtacctccgtttgccttttaggtctacttaaattgaaaattgatgttggttttgcaataaggtctagtttctatgtaactaaagtggttatctttcacttatatttaagtgaaagaactgcgaattataagtgaagatttacaatacatttatgtgtcctccgcattaaaatggtttaggacatgatttagaaattatgtggaggtaacattctagccgatgttaaatgtttttgtatcgcctgatgatatttgtagggaattgttgtaataaattatatcgaaaatgttagttaatagtgtaagcacaagggaaagacaaatgaatggcaatgtcgatgctaggtttcaacttagtttgtttgagtatattttcaaacatcccacaaataggtggtttgctagaattgctatccctattgttattgtccagttcattgttttcaagttcttttatccatttgcgggatttataaatggagactcttatatatatattgagacagcataccataattttactgtaaatacttaccccattgggtattctaaatttcttaggttaataagcgtttttactcattcagatttagcggttgttgggctgcaatatctacttttgcaatgtgcgagcctcggacttgtatttaccatgttttatttttatgaaccatctagatttgcaaagatttctttgttcgtattcatgttggttaatcctgtctacctttatcttgcgaattacatttcaagtgatgctttctttctttcattaagtctaatttggtttactttgttaatttggataatgaatagacctactaataggttaatcattataaattcacttgttctttttgtggcattcaccgtacggtataatgcactgttttatcctgctgttggagtgatatcgctactattaactaggagaagaatgataatgaatattgttggattctgtataagtcttctccttataggattttttatacaagtcacaagcgtaaagtataaaacaattagcggatttagacaatttacgccatttaccggatggcagatggcaaataatgcgttatatgcatacagatatgtcgacagcgcggatcggagagatgtacctgtatctctccgtatgttggataatatggttcgacactattttgattccagtagagatatacggacgcatccatcagaagcattgattgcgagcactgtttacatgtgggatcctaattcaccactttccaagtatatggaaagtcagtttaagaatgattccgcggcatctgcgttaaagaagtgggcaactcttgcaccaataatgaaagagtacggttcgtttttgattaaatcttatccttatgagtttgccaagtattatttagtcccaaatgctataaaatactatgcgccaccagttgaatttcttgatcattatagtactggcgtagatagcgttaatcaaactgcaaaggtttggtttgactataaaagcactaaactgaaatgtcattttaaggattttaaggtaaatacattggatttctatcccgttttagtaggtactatgaatgttgttcttgtaatgagtacaataagttttatattattaggaggttataagcaacattttcaattgaaaagagggctaatacttgtggtgactttatggacaattaattttggttttagtgtttttgcatcgcccatagctcttaggtttcagttgttccctattctggtctcattgtcgtatacttttttgttggttgactatttagtgaaagcagctaagagtatatctgtcgtacaggaagaatatttgacagagactgcaaagccggaaagtcttactatatagcactatatcgatttgagtaatttaagtaattattatgaaacgaatgtatgttattgttgcagcgatgcttctggtagggctatctttatatatgggtctctttagaatggggggatattcactgatagatattcggaaaagaggttatgcgaaatcagttataactggacgagagggcgagttattgccaagtataagtatactactttctgacagtataactaagatcaatctttcgtcaattcccaagggaaggcctacagtgctgttctatttcagcccctattgcccttattgtcagtctgaaatggatactattataaataatgtaaagaagcttaaacatattcaattttatttagtaactccttacagccatagagaaatgaaattgttttataataagaatcatctcgaaagatatgagaacattatagttgggttggactatgatattcggttttctgaatactttagaatagcacaggtaccctttattgccatttatgataagggtaaaagattgaatgccggttttttcggcggagtggcgtctgatcagctaagacaagttagtcaagaataaatttttgcgcaaaataggccgattgaatacttgcaagagaaatcgaccaaagaatggcgaagccgaaaaccattataaacgagtaggcatttttcataaaaagcaaagtttagctttttgattttaaaaagcatctatcattatgaaacaagcaaaattcgcgttaacagctgttgctcttctcgcagttataggtggtgcattagcattcaaagctaataggcaattgaagactttctattcacttggtaccactgtgattcagggtgaagaagttgcaggttgcgttattcctgtacaattgttacgtactccggcagctgcaggagcaatcactccatactcatcaacatttaactctgctaccacaacttgtacagttagagttaatgttaatgattaattgagaaatgatctatgaagattatttgcattaatgatttgattagatctcttagttatgtttattaactaataatttacaagagccgtcttattgtttgcgaaaacaatgagatggctcttctgcggtaatagtgttcggattttagtaagcaatgataaggcagatgtaataatctctatgagggtttaaattcggggttgagttgcgcggactgattaaagcatactaagtgttaacccgtgcatttttcgtcttactagggaattgtttgcaatgaaagctttatacgagttaggtgtacccgtataaagatcgacagcgtcgagcccttttatttaattagcttaactcgatcaaccattgattagtaccacagccgtacaaagtgtcgttggatagttgaccgtacttgaataagaggtgtagaatcctcctggatttggtgttagatataatagttgagttacgacgcatccattaatttgttctcctccgatagtcgtagttcctagtgagtaaaaggctcttagttgcctattggctttgaacgcgagagttcctccgattatggagaatgtaatcaaaacggttaatgcaaatttggcttttttcatggcaatatatttttattatcttgatagattttactttattgaaactctgttaaaatataatttgttgctgatttttagcgtatgttgttgtgtattatacgtagtgtgtttcgctatttttgttatcctcttaccactaaagaaaatagtaggaaatttttagtgaaaagattgaatgatgacgattaatattttcttttgtttcgttatcctttttattgaatagttgatacctttttttgtttttccacgtggagtccgggtgaatagatatacttatagttgaaaggatttggaatcggtgttacgattccagttttgtgaggcctggtgagatgatcccttcaatattgctaagttcatccaaggtttaaagacttttgttatgtgctaattgttgtaatttcatatcgattgcaatttctaggttattattggtaggggctgtatttacatatttaaagacgagatgggccataaatgataaagtttcggggataattgtgagggttatcattgtggctgacattattttttttcataaataataaaatttataaggagaggagaatattttcttgctattgtatctttaccgggcttgttaaatgaatgtagtcacataaatatatgttttttgcctgcgattgtttctccgtagttgatgctaaattccatctccccgtttacctgctggtaaaaggcgatacccagagccaggaaaacggcttggtactgttacctgttacagtagtctgtaagtggagttccggggtggcagaaccacctatcggaatttcttcgctggtagagacactatttacaaatgtttccgcttcgaagtccacttctgcgccgcctaccaggattttaaaatgcgtggcgccggcagggcttgccattaggtcaatcggattgaatacaggcaggtctactttgagcgtacctgcaacacgatctattgcggcagtataaggagcgaacagtgttacgcctaaacgtgaattgctgttgaattcaaagcttttcagtaactctgcttcgccgtcaattacgttgcgttgtcctctcacattcacggtgtccgcctggatcactttcatcatttcccggcataactgtgaggatgtatagctgtctttaatattcattaccagtgtacggaatgcagtgagaagcatcttgtaggctttacctgctctgccaaattccgccgggttttctcgcgttctggcaaacgcgggatctgttgcgatccggttggcgctaataccgcctttctctctggctagatatccttcttttgatttgtagaaggtaatgttgccaatcgtgccttgaagtgggataatcctattttgtttggccatttttatagatttaaaaataaagaatagggcttttggtagccagcccttttaagcttacacctgcgcaggatgtagtaaatggcattcacttatgctaaactaatgtcgtatttttactcaaaaaaatttccattcacattgatatgaattgtatcacattgatatgtgttttattggaagagagtggaaattgagagcaaagaaagaagagaaagaaaaaaatagataagcagttgcttaggagctactccccgttttactccccatttacttcccggggaataaaatgtaaatcagtcaccaatagcttatctttataaagtggtatatggtaattcactgccagctttaggggtttttgactatattatcatcattaattcatattctgaatttgcaaacttgcttctgcaaattgaatgtagttctaaggttttaagagagttttttatctgtgaactagagtatgaatgtgtcgattatgaatcaagtatgtcctagggtatttgaatagcaccactgtataggggattttatcgatgttttggagtaaagtatctgtgtttcaatgatgagttattagctatttatgactctgcaagtgcaggtagttgtaggagcattaaaagtacttgaatatggagtgacaaagccaccagggttgggtgttaggtttagatcgactggtacaacacatcctttggttccttgtccatttattgtagtggatccaagtgagtaaaatgttctgaggagcttattggctttgaatgccaatattccgcaaaatgtagaaatgactataactaaagttaataggaattttgcttttttcatagggatataattttattgatgtagtaataatattctagcattaaggagagtattgtgcttatttttctaatcgatgaattgatttgctgtaaatataggtttcttagctgcattaatttctcagcgattgacactttttcccgccacactcagaaaacataacaataccttaaaccacctccccaacaaaatcccctattttcgccccgttgctcaaacctctgccatgctgcatgctcatgatgatatagcgcttatccgtaccggtgatccaaaagcattcgaaaggtgtttcaatcagcactggcccgccctttatgccttcgcgctgaaaatcctcggcaataaagacgatgctaaggacgtagtgcagggcgtatacatctccctgtggtcacggaaagagaagctgaacctgaacggtccgctggaaaactatctccaccaggccgtccgctttcagtctattaaaaaactaaaggaaatcatgaaccggccggaggagctggaccgcgtgcaggaatatatcatgccggtgttaaacgatatctgggaaaagatggaaacggccgatgtatttaaagaaatagataaccagctaaccaccttacccgaaaaaacgcgggaaatattcctgctgagtcgccggcatcatctatccatcacggaaatcgccgggaaattaaatctctccgaaaaaacagtaagaaaccagctgcacatagcattgaaggctttaagacaccatatcgcagctgccctgatcctcgcggaaataatgagttaataattccttaacgtacttcttcgggacaagcacctcctttgaaggaacatatctatagaagaatgttccggatgaatatcacacagtttaaaaaattggtcagcaactacctgtcgggcaatgccacccgcagcgaagctgcattgctgaacacttacctcgataaggcctgggaggaaaaacaggtgccggacgatgtggagctgcagcgcctggaagtatggaataacctggaaagggaaattgcgccgccacggataaaggtatggcggtacgcagctacggtactaattctcatagccgccggggccacttacacctaccgcctcgccttgcaggactggctggatccggttcccatgcaaagcatcaccgcattgaaataccagataaaaaaggtaatcctgccggatagctccgtagccatcctcaatggaggtaccacgctcacctatccccaatacttccgtggtaaacaaagaaatattacggtgaacggggaagcattcttcgacgtcaccccgcaaaccgcgcccttcatcatcaccggcccgcatgtaagcgtaaaggtattgggcaccagcttcgtagtggcagacagtaccagtatcgaaaaaccaaaggtaagcgtgaaaacgggcagggtagcggttaccgccggtacggcggtacagcagctcacggaaaacgaggaactggtttatgacaaggaaaccatctatatctataaacaaacggaagtaaacaccgggtggaccagcaaaaagctgttgttcaatgaatcagcgctgaacgatgttttcagggagatagaaatgctgtacggcgtaaaaataaaaactactccaggtatcagcgacctgaaattcaccggcgcattcgaggaaaccgacagcatgaacgatatcctgaaagtgatatccctgtcgtaccggctaactattcataaaaacaaaaacggcgtcatcgtaatcaggtagcagctcgcacagcggaaatgctaacaaccatcagcgtacagctgctggtaacggatcttctttttttaaatcacaaacgaatgaaggaaaaaattttacacggatgtatgtggatcctgctctgctttaccttgccggcaacggcgcaggaaagcttcctgcagaaaaagatcagcatcagtttcaggaatgagcccatcgcaaaatgtttcatgactgtgcagcagaagggcggcgttaccttcttctacaatcctgccgatatgaaagcggtggataaaaaatatacggccgatctcaataataaaaccgtagcagaagtgatcacctggttattgcagaataccgggctggaatttgaagcagtagatggcaggaaggtagtggtacgcaaaatcatcgtcaaacaatcaacagccccccgcaaacgcaccatcagcggcatcatcacggatgctgccaaaaacacgcccatcgcccgcgcggaaatcatggcccaaagcaccggcagcgtggtaatggccgatgaatccggccgcttctccgtggaagtgaaagatacctcggatgtgctggtgatctattatgtaggctatgctaccaaaatgatcaaagccggcagcgcaccggtgttatcagtacaactgaaagccgacagcaaaacactgagcggcgtaacagtagatgcccgtcggcgctccaatacggaagtaatgctgctgaacgaccgtaaaaactcggccatgatctccgatgggatctctgcccagaacatcgaaaaaacagccagcattaccaccacccaggccctgcaacgggtatcgggcgtaacagttacagacgataaatatgtagccatccgcggcctgggcgaccgctccgtgatcggccagctcaatggcatccgcctggcttcttccgatcccgacaggagcgcgattccgctggacctggtacccgccggcctgctggataatatcactatctacaaaaccaccacctccgataaacctgctgatgccgctgccggtatcgtggaactcaaaacaaagtcggtacccgaccgggaaatgctcaccatcaccgtgcaaaccggcatgaactcacaaaccggcagcaaagtgaacagcttctataacagcgacatgggcttcctcgggcaaaaggtaaagtcaaaaggattatccccggaattccgggagctgtccaaacagtacccaaacggcttaggcgatatccagcgtaaaatcgccaacagccgcaacgatccggccctgctggcagaagccaaccgcgtcagcggtatcatgcacggcttcgatcccgtgctcaccacaaagtataaatcggccccgctgaaccagatctatgcggttacttacggtaacagctatacggtatttaagaaacaccaggtaggattaatagccggcgccaattattataaccgcaccaacgatatctacgacggccagctcacccagtacagcgtataccagggcgtgttaacaggcaacagcgcattgtacagtccccgcgtaattcctaactacattactcccaacaatatcaatctggggaagtatttaaattataaggaaaacaccggcacacaaacactcaactatggatttttgggtggactcacttatcgcttcagcccgcagcacgaaataagtatgcagtacctgggcagccggggtgcggaaacacgcgccagcaacctgcacggcgcctacgagtacaccggcctgccaggcaaggtgtataacctcgtgtattccttacgtcaaagctatcgtacactcaatacctttaacttacagggcgagcataagctcacaatgaaagaatactctccgaagctgagttataacctcgctacctcttcgtcttcacaggatgatccggattaccgctttgtaaacctggccgactatcgcgtaaacggtggcagcagccatccgggtgcagtggatgtgccgggcggtacaccgcctattgtggcttcccccagtttgtattccctggtatcaggatatgtaaacggatatggcccctatggtatcatccaggccgatcccaatggacgccgtttccgccagctccgggaaaataattacaactataaagcggatctcaccctgccttttaaagtatttaataaaaaacaggaatttaaaaccggggtaaactacctgcatcggagaagaagcttttcagagaatgtactctatctcccgggttccaattatgctgtcaatggcgcactaccgctgtatgaagtaaatggtcagctggatcagctggtaggatatgatcgtatcggtatccgcccgccttcttcctataacgaagaaggtgccccccgcaatggcggcttcctgtataatatccagaaatcccccaataactataaaggctactatgaaacccgcgcgttttatggtatgctggacctgcatctcacggaacagttgcgcttcacgggcggcgtacgttttgaaatgacggatatccaggctgcagtagatacatccaatgtattcctggatccctctattactgctacagatgccggcggtaacaaaataaacctggtatataccgaaccaaattctatctataaaacagattatgaacctttctactctgctaaccttacctatacactgaataagaacatgaacttccggttgggctacaacactactttggcccggccggagctgagggaactcaccaacgtatttgattttgatcctttccagtttgcactggtggtgggtaatcccaacctgaaaaaccagcaaaccaccaactacgattttcgctgggaatggttccccgcaccgggtgaggtattgtctgcttcggttttttataaggagatagataaccagttaacaaaggtgtttaaacaaaattcatccggactggaagcacggttccccgaatttcctgccatcgaatttcagaatgatcctaacaaaggtcgtgtgtatggaatagaactggaagtagtaaagaacctgggtatcctgacggcagccatgaagaatttgtcattgggatcaaacctgctgctggcacaaagtgaaattaagaaaactaaggagagactggaatcctcccgtgccatcgatcgccgcgcaccggccaacagcccgctgtttgaacaggcgccgtattcagtgaatatattcctgaactacaacaacacaaaatcaggtactgatttcacagccacttttaacatggtaggagagcggctcatccaggtaaacctcgatggtacgccggatctgtattccagacccaacccggtactggatttcgtgttttcccagcggctgctgaaacgtctgcagttaaaagggtatgcaaaaaatatactcgacaggccagtggaagaagtatatgccaatcctggcacaggaggtaatttttacggaaagaaatatgtacgcagaagtttttaccgcggaacagaatttatgctgggcctgacttttaacctgtaaaaatttgaatgatgaaaatgaaaattacttacatactcatagcagtggtattgatgatgagcgcctgcagcaaaaaactcgactacagctacgataaccgcatggtgcaatacccgatggctgcctccggcatccgcctggtcaatttgttaggcgctacagaattgtcggtgaacggacaacgcctcaccagctacctgcagcccgataacgaaggatactatggtgccaatgaaacacgcggtacagcatactttccggaaacaggccgtttagggctaacctatagcattccccgggagcaggtgaaagccagcggctgggtagatagtatcctgttcagcagcttgtctgtcaggaacttggtgccgcagcccagacccttccgcgcaaaaaatgatgaggcacatccgaacgattattactttgtacgtttcagacccaatccggatggtttccaggactctttgttcgtgatcccacggggtatatcaccggcggcagatccggttgcatttaaggtgcgtttgctgaatctcagctcctccattacgggtagcattcctccgggtattttccgcaccgggcctatgtcgctcacgctggccgatggtaccggcgtgccggggcttagcaacgtagctcccggccaatattctgattatgtggaaataccctatggcacctaccagttcaaagtattgaataacgaaggaaaagaagtaccagccagtggaagcatgtataatctcctgaacccggttaccggcaccctgatggatataaacggtacgcccggcatcggaggtggtaaagatacctggctcacctacgcaccactgaaaacgtttcagcccggaggcatttataccatcgtggtatccagtacctacgacgccaacatcccaaccggtaatcctaacggggaaacttacaaatcagaaaataacaccttccgcattattgcagatattcctgaaccggtgaacattacctatgcccgtttacagggcgtaaatgtagccgcaggtaaaaacattaactggcaggtagacggacagcccctgggaggcacattggcctttgccaaacaaaccagctacagccgctatataacgggtacgcatatggtaaaagcactggatgaaaaaggacaggtattggccgaaagtaatctcgccatgcaacccgccgataattttactgcctggctgtatacccgtaaagatggtagcaccgcaattactttttctgccaataacctcagtggaaaatactatggtggtactgctacagatgatggtacctacggtatgttgaaaaatgtatatccttttgggatccgcttcatgaatttttgcccggacctggaagaagtcacttttacacagagcaacggacaaccgtttattgcaatctccacattggcgtttcaacatatttattttggaaaagcagtaaccgatcttccctatgtgatgcaaatggtcaatttctcgcaaccggtaatggcctatgcctcgatgcccggtattgcccccggcgattggctgcgcaatattgcgccgctgaaaagccgtgattttattgcccgcccggaattatataaaacaccggaaataccacagagcgaaccaggtatttataccgtagtactactgggcagcaccgctcccaatgccacggaaaaagcccggatgattattgtgaaacataacaattgagtagtcttatgaataataaatactttttactgacactactactggccgcgctgtttttcagcagctgccgcaaaacggactatgtggtattggataatcccgcctacctgcgggtattcaactgccttgaatttaccaccagtcttgataacaaagatgcgccacaaccattcctcgccttcctggtagaccccgtgatggatgataacggggtacctgtcagcgcagccatcacaggcgattttctggggctgcgcgccgactgggcaagaccttatcccgacgccgccagcaatgtattgtggcaaaaagaatatcccggtactaaaagagtactggccgctcctattgtgaatggatatgacctttcgagctgggcgcaggtgccttcaggtaagcatcatattgttttccgtacccggccgctgaacaacgtgccatactttgaactggataaaatggaacggggcgttacgctgattgataccaccatagacctgagcgcgggggaagtatatacgatgcatgcactgataaaagaatataccagccagcagccatttatgtacctgcgtaaggaaatatttccgaaacaacccttcgctgattccacagtatatgtgaacttctataacctcagcgcagtcaatttctatgagaaagcgcccagtactttgccaaatgaagacctgtccaacaccaagctgagtgacaccatgaacgtttattactcgcttaataaactggcgccaaatggagctcccgtggccctgccgggttacaaaggcatacctatgggacggatcatccattccctggaacctaaggtaatgccttattacagcttccctttatttgcagacaccagcagcaataaaatctttacaggcaatatgagtcagctgttcggattttacgctgccggttttaccccggaaaacctgggctacccgggcttcataccggtaggcgtttactccgccattattatgggcgactatggcgaatcaaacagaagtgcctatctgcccttcaaggtaaaatgcgatctgcgtacaggcctggtggtgagtatccattccggtaccaataatccccgttcatttgctacagtgaatacggtggagtatatcaaccggaagatgtatgtaactaccatccagcgcaagtttgcaccacccgtttattaacgtctttatcatttcgatatgctgaatatttctatcataaaacagttcatggcagtatcgctgctgctggcgttcgtaacgggctgccggaaagatgacctcattccgcccattgacagaactactacaccacgcgcaatgggcgcatttattgaaaacaattatgacctgagcattttaactgctgccctgaaaaaagcaggtctgctggatacattgaatcagggtggaccctttaccttttttgcaccggataacgcagcatttaatagaatgggtgttacaggtcctggagatgttgctaaaatggatgcagatagtctgcggtctatgctccgttatcacatcatccgtaaccgttactttaccaccactatcccacagcaaatggataacaggtatcttacgctttccggagaagaaatatatatatccaccttgaagacagttactatgttaccagacaacgacatgtttgtaaatggtgcgctgatcctcaaggaaagtaaaaggaatatcgccctggcgaacggtgtgctacatattctcgccaagccgctgaagcgcacccagggcaccgtacaggactatatcgccgcagataccagcttaactttatttgctgccgccatgaagcaattcaatttatgggacggtctcaaaacaaataaaccattaacggttttcgcaccggccaatagcgccttcctgaaatacggacttacggcagaaaggattgccagcatgaaaccagccgattataaggccatcacctttgctatttacccgatagagatgagacctatgcatatcttttgtaccgatggttatctgctttcaggtacttctacagtaggcgacggcggcatcaaagccggcggatattccatcgcacccgggtattcgtataatagttactacggcacagaaacttcttccataagtattttgaaaaagaaagcagccgactggtacccgagcgaagacggcccctccaatgtaaactacctgaatggactcacaaatgcagatcatacatgcagcaacggcattgttcacgtaatagatgaccttttcctgaacccggatttaatgaagcaataaaaatgaaacagatgacatcaaaaatatctttgctcttattactgctcctggcttttgctgcctgccgcaaacaggacattgaaccggaaccggtcggtgaacccgtgccgcatgaatcaggacccgataaaacatggcagcagcaactggccgcttcttcgtacacccgtttccgtgaagcatggcagcgctccggtatggatcagaaaataaaagaggatggcgcaggttttcataccctcattgtacccaccgataaagctttcgatgaagccggctggacattggaaaaaataaaggcaacagatgcagctgtactggatgagttgttgtcctattatataatgtctgtccgcctgttgccggaaaatattaccgccgtcaaaggcagcacgccggcagcaacgctgtcatcccgctctttcgccgacagggaaaactggtacaaggattacgtggatttccagttcctggctaaatccggcgatagcctgatcgtcaatgggatggccctcggcaaatggggacaacaactggaaggcactaatggagtaatatatcccattgatcacctgatcagcaaaccacaacaatccatgtgggaatacctgcaaagccagccgcgtttcagcctgtatgtggctgcattacttgtcaacgatagcctgtaccagtccgtctggatgaatagttcactgccgctgctgaaatcgtccacctcactggtacagtttaccctgttcgcacccaacaacgatgcatttataaaaaatggttttcataatgcagatgatattctgcaatactgtctccgttcctggccactgccgcctgccgactatgatgaaaatatgtattggcagcaaccggtaactactatggattctatactgctggcatgcggacctgaaatatccaacgccgcccagctaaatggaatagaggcccgtgtaggaccggttttttttagcaacgacctcacgctgaatgctaccaatctcagcggactaacactatacaaaggagagccttataataacccgccaacacggatcagtttgtcatttattaacaacaacggtcagcccggcgtcagaagaataggtaccagctatccttacaccagtttaaagagcagggatataagagtgatcaatggtgttgttcacgaagtaggagatctgtttaaacaataattttaaaaagcagccaaatgaaaaaattcacttatacaggtttgctgatactcttattgtcagcctgtacaaaggataaagataacacagcaggttcggatgaaatcaatcgcctgacctacatcatcgacgataatagatttaacttctcttcttttaatacggcattgggcagaaccggttaccgtaaagtgctggcgcaagccgggccttatacggtcatggtaccggataacaacgcatttgtaaaagccggatatgcaactaaccaacaggtactgacccaaagtgcggccattctcaataacctggtgtcctatcacattgtaaacggtacctgggagttgaataaactgccttatcagtttaatcaggaaatatcggcgattaccggcgcaaaaatgtttgttacacactggatcaaaggcgaagataccgtgttgacgattaatggcagccccgtcctcgcgtacaacctgcccgccagtaacggtatgatacaggtacttgataatgtgttgcaaccattggtataccaaacactgtcagatgcaattgcgacagataccagtcttacttttctaaatgtagcgttgcaacaggcgggtatgaaaacactgatctccggtagcgccacctatactttttttgcgccttccaattcggcattccgcagcgcaggctttccttctatagatagtatcaataaaacagatgcaagaatattacgcgatctgttggaataccacctgtttgcaggccggaagtttatctacgattatatccttaccaccggcagctctgatcaaacggaacaagcgatgaagaacggtaataacgtaggtatttcactcgtaaaagacgagacagatgtgaaatacataggcatcaccataaagggagccggcaacaaagtaccggcagtggtgaccagagaaaatctcatggccggcaacggcgtactccacatcatagaccaggtactaaaagaaaatcagtagtgatgaagaaaattttatacatagcttacttgttcaccgtactgctggctaccagccccttggcatacgcacaggaaacaaacggcacactaagcggaaagatcaccagcgataaaaacgaaccgctcatcggcgttacggtactggctatccacgagccttcgggtacaaagtatggtgcaatcaccaccgccgatggccgctattatttacccggcctgcgtatcggcggtccttactcggtgagcatcaccatgatgggcatgcaaccgcagaaaagggaacagctgaatatccgtcttggggagcccgtacaactcaacatcataatggccgttgctggtaaagatctttctgcagtaaccatcaaaggcacaaagaaaggcgcctccgccaacaccaccggcgcagggcaaaacatcagccgcacacagctggcaaacatgcctaccatttcccgcagcctccaggatatgactaaaatggttccgcagggtagccgcgacaactcctttgcaggtaccaacttccgctataacaacgtaaccatcgatggcgccatcaacaacgatgccattggcttcagcccctctgcaggcggcattaccggcagctccggtatgcccggctccagtacccgcaccaacgcagtatcgctggatgcgatcgaagacatgcaggtatacctggcgcccttcgatgtgaagatcgggaacttcaccggcggcagcatcaacgctgttacacgcagcggtaccaataccgtaacaggatcggtttacggctttggccgcaatgcagccctcaccggtaaaggccccaacggcaaaatgaacagcgacttctatgattaccaggcaggcgtccggctcggatttccgctcataaaaaataaactgttcttttttaccaacgaagaaattacttcccgccaggaccccgcccagttgcttgcagggcaaccggaaacggcgcagatcctcagcgtcaaagatgcggacgatatccgcaacgcaacgctgagccgctatggccaggactttgatccgggtactgccggtaattacacggcctactcccgctcgcagaagttctttaaccgcatcgactggaacatcaacgataaacaccaactctccttccgcaataataccattctatctaaagccatgaacatggaccgggatcaacaggatttccggttcagcagcatggcctatcaacaggtgaataaccagagctccaccgtgatggaagtgaagtcacggttcaataaccgctggtccaacagtttcatcgcaggattcagcgtagtacacgataagcgcaaccccggttcagatccgtcactgccacaggtgcagatcaccggccgcacacccggcactactatctatctcggtacagaccgggaggcgagcatcttcgatatgaaacaacgtaccatcgaaatctccgataaccttaccttcagaaaaggaaaacataccatattactcggcacccacaatgaactgtatcatatcgattatggctttgtgaatagctggaatgggagagtggattacctgagtattgaagattatcttaacaacaatccttaccgtgttcgtggcagttacaactataccaataacagccgcgaatacatcctcgcgcacccggaagcgcagtttaatataaacatgcacagcgtatacgcacaggatgaaatacaggtaacagacaagttgaaggtgatccccggtatacgtgccgattatacctggctgccagagaaacccgccctgagtgataaaacacagaacgcctataccgatggttcttttggtaacacctacgcctatacgccgctgaaccgcatcaataatggctacctgggcaaagtacagttgtcgccccgccttggcttccgctacgattggaaaaacgatcaaagccttatcctccgcggtggtactggcctgttcaccggccgcatcccttttgcctggatcgcctatgcctattataacaacggcatcaactacggctcctttgatcagaaagcagatacaaaagtatttgtgcccggcagcgatccgctgcaacccaatcctaacggtatcgcgcagtttattgagcaaaatggcgcacagatgaacaaccggaatgcaggtaaaacacaggtagatgtaattgataataacttcgtgatgccgcaggtatggcgcagcagcctgggactggattatgtgagcccggcaggatttaaatacaccgtggaagcgatgtacaccaaaaccctgaaagatgtgctgtttcagcaggtgaacatcaaggatgatccaaagtattatccctatgataaagaccggcagcaacccatttacagcggcactacagacccgcatttctctaacgcttatttgctgagcaatacaaagaaaggctaccgctacagtttcaccggcagcgtcaaccgcagcttcccttcaggtctccaggcgtcgctggcatatacctacggcggttccaaagatatctccaacggtatccgtaattctatggaaagcaactggcagctgaaccaggcgctcagtcccaataatcccggactggcatggtccaactttgacgtgcgtcaccgtatagtcggtaacgttacttaccacaaagcctggagcaatagctgggtaagtaccattactatatttgccaccgcgcaatccggcagtccttttacctacggtgtggttaacaacagcatccagggattaccgcaacaggtaagcttgttatatattccttatgcagatgaagccattaattacttccgcgggaaaggcatttctgcggaacagcaggcagctgcttttaacgcttatatagatggcgataaatacctgcgcggccgtcgcgggcagttcacagagcgtaatgccggtcgcacgccatggaatgtgcaggcagatctgcactttgcacaggagtatcattttggcggaaagcagttcatcacttttactgcggatgtagtgaatctgacgcacctgatcaacagcaactggggcacggtatatttctctcccaatacatttaactccactgccagcaccggcttaacaccggtattcccggcagggcaaaaccccggcggatacccggtgtatactttcgaaaatccgggtaagccttactccgttgatttcctcaactccagggcgcaggtgcagctgggattaagatattctttttaatcaatgttaatcatccaacaatgaaatatgctttatacctgctgccggtaattttgttactggtggcaggctgcaaaaaagaccgggataatagcacggtggcaatgaatgtaaaaacgttctggcctaatagtggaaatgcgggtaccattgttaccctgcagggacagggactcaccaaagatgtacaggtaagctttaacggtacggaagccagggtactggatgcacgcgattccgtgctgatagtgctggcgccggataatggcagcaccggttcacttgctgtaaagtccggcgaccgtaaaatggaacttggcacctacacttaccaggcactgagcctgcatggtatcagtccggctaacggtcccgcaggtacgaatatttctatccgtggcgcgggcttcagcagcatggaagcgccggcaaaggtaaccatcaatggaaaggacgcactgatcaccggtgcatccgatacgttactggtagcggctgtgccggaaggtgcaggcagcggcaaggtagtggtaatggtagatggaaaagaagtaagcggacctgatttctctttccaggtcatcagcagcattaaaccgctgaagggtggtagcggtacggcggtaaccattaacggggaagggtttaataccctggccgccggcaacagcgttacgtttaatggtaaagcggcggcggttataagcgctgctgccggcaaactggtggtgacagcgccggaaggcgtagctacaggaccggtagtcgtaagcatcaacgggcagaaaactattggccaggtatttaccgtggttcccaaaccggtaatcagaacggttacgcccctgagcgcgccggcgggtgctgctgtggatattgcaggcgattacttcagcacgttccccgatgaagtaacggtgtcctttaacgggcatgccgctattgttactgctacaactgataggagcataagcgtaaaggtacctgccggagcaggcgccgggaaaatacaactcatcgtgaacgggcagcaatcggaaggaccgctgtttaaagaacagtcgctgggcattttacaattattaccggataacggtctcgcaggtacggaagtaaccataaaagggattggcttcagtgccaacgcggcagagaacatcgttaccttcaatggggtagtggtgccggtaactgcagccaccgacagtacgctgcgtgtagtcgctcccgttggcgttagcaccggcgcgctgaaagtaaaagtaggcacgctggatgccacaggcccggtattccgcagggcaggagtgatcacggttgcaggcggcccgtcgcaaacccttttcgatgatccgaaaggcatagcagtggattcccgcgggaatatattcgtgctggatctgaacgtgataaagaaagtaacggccagcggggcggtgagcatttttgcagggaaagcagatggctccgcagggaatgtggatggcaacggaacagccgcggcattcaattacccggtggcttgcgtaatagatgcgcaggataatctctatgtatgtgatcagaataacagatgcatccgtaaaattacgccggccggcaatgtaactacgtttgcccgtgtggcatttacgcctattggtgtgggtattgataaaaacggaacagtgtacataggcgcacaatacgcaggtgtataccgccttgatggcgccggcaatgccagcccgctggcgccgaatgtatatcagagcgcaccgggtacactggtaatagataatagcggaaccctgttttttggcggcgattcggataacccgtttgtttcaaaaattacaggtggcgttaaaacgctgtatgccggcggccagtatggctacggcgatggatcgcttaccggcgcacaattcagcattatctccggcatggcccgcaacgcggtaaccggcgaaatgtacgtggcagataataatgccatccggttaatcgccaacgaccaggtaacacgcatcaccggctggaaaggcggtagtaacccggtatcaggaaacgacgacggaacattgaaccaggccacctttaacagcattaatggtatttgtacagataaggaagggaatatttatgtagtagagcggtttggaaaggcagtaagaaaaattatcctgcagtaatttttttagaaaaaaaaaaaaggggctgaccagttaacctggccagccccttcgttatgaataagtgttacggctttagtagccaggattctgtttcatgtttggattacgttctacttccgcgtttggcagcgggaataccactgcatcatcattccactcctgtgcatctacaccgccgtgggcaggaattgcacggtgtgttctcaggaagtcgaattcgccatgtccttcgaaagccagttctattctgcgttcggtgaggatatcgttgatcagtgccgcctgtgttaacggggccagtaccttagccttggcccttgtcctgatggcattcagcagggtgatagcttcgggattagctacgccgggagttaacctggccaatgcttctgctttggtgagcatcacttctgccaggcgtacaacgggcacccaggcatctacggtgctggcgccaaaaaacttcttggtataaaatgcggtggtatcgccaccactgatggtataagtaaacagtggtttcgcccgcagatcggtgaaacgatcgaaattggggagcgtcaggtaggtctggctgatggtgatatcacccctgcctgaactgccataatgctggccgatggcgttattggtattcgggttatcaccggagctcatggctacagagaaaatgcgttccagggaagtctggtagtttccggaagaccatacatcagcaggcgtggcgtcgaggtcgtaaccaaaggacgacagcagtacgctgtctgcatagtcacgggctttggcccagttgccttcatacaggtagatgcgggaaagcagtgcatgggcggcgcctttggtggcacggctgcggtcattgtaatcatcaccggtggtaacaggaagtacggctgctgcttcagtgagatctttgatcatctggtcataaacttccttcaccgtgttgcggggaactttattcttcggatcaatggcttcgccaccatcctttgcagcggtgagtatcaacggcacgcccatatgtccggcatcagcctggtaagtataggtttgtgcataggtatttaccaggaagaagtacgtgagggcacggataaattttgcctctgcgtaatagcctgctgctacctctgcgccaactacactttcatgatctttcaggttctgcgaaaaataattgctttcaaaaatggttctatatccgcccgaccagcagttgaacgcatacacattgttggaaagcatattaaaagtaggtacgttaccaaaataagaggagatatttacatccactgatctcacgtccgagtagatcagtacgcggccccccaggaattctccgttctgcagggcatcgtacataccgatggcggacttttcaattctttccggtgtgctgaaggcttcctccggcgtcagtttggaaaaggggatctggtcatttactttggagcaggaaaacagcatcgaagatgctatcgctactgcgccaatggccaaacctatgcttgtttttttccgggagttcggtttatattttaattccataattcagtttttttaatcgctaacaattagaatccaacatttaagcccagcatgaatattcttggtaaaggcatacccctgttatctgttccgtagttgatattgctatcacggttggtattgatttcaggatcggcgcctgtatatttggtaatgataaaggcattttgaacgagggcgtaaacgcgcaggctgttcaaaccgattttatctttgatgccagggaaagtataaccgaggctgatttcacgacctctcaggaaatcgcctttttccatccagcgggtggatgcctggttggttggcgcgtcagagagtaccagcttgggaacatccgtgtttttattttcgggagtccatctgtttttgatttcctgcaggttgttctggaaatagttgctcatcagggcagccctggtggaattgtatacatagttaccgccactgtactgaagcaggatactcaggtcaatgcctttgtagttgaaagtgttattgaaaccaccataccaggttgggtaaccggatttatcctggtactgcgcgtcagagcctgtaacagcgctcattggcttggtaccgtccggagaagtccatttcctggcagtaggtacgttaggatctaagttgtacatcaccagttcgcctttggcgttgtagtacattggattaccattgtccgggtttacgccgccccattcgatcagcttgaacacgccgagggttttgccaacgctgacacggttgtttcctttgatgatatcagatccatcagcagtggccgtcaccctgtttttaataatggtgaagttaatgctggaattccagctaaagtccctggtagtaatgttctgggtatttaatgtcaattccagtcccttattccacatggtaccgatgttggtagtgaggatagaacccaccgtaccggtaacagggtcccacggagtacccacggtagccaggataggtgcatccaggatcaggtggtcgatattactgtggaagtagtcggccacaaaagtgatcttatttttcagcagggtaacgtctacgcctatatccagtttctttgatttttcccactgcaggttgggatcaccaatctgtgaaacgccaaatccgttgatatcgccatattgtccgccgccatacagggaacggaatgcgtatgcacggatgttggagttacccaccatgccatagctggccctgagtttcaggtcgctgatcagggaaatattatctttgaagaagccttcttcagaaattctccatcccacagatacaccagggaaataaccacggcggttgttggagccaaagtcggaataagcatctgctctcagggttgcatcaaagtagtatttcgatccgtagttataacctaccttaccgaagtaagactcaaacgagttggcaacgcggccaccaccggtataactgttttcagaaccggcaaataaaccgtcatagatttctttaaaataagaatctgccaggttaccctgtccggtgtataactgtttctgttcagtatgttgggattcctgacctatggtagcactgatgaaatgcaggttgttgatagatttcgtataggtggcgaagttagaccagttccacaggttctggcggaagaggttttcctgcaccaggccattgttgcctaatcccaaacctgcctgtaatggtccgctgtactggtcttcaaagttctgcaccaggtcaacgccaaaccgggaagttattttcaaaccggcgataggctcaatttctatataagcgctggataatacgcgggtggcggtattatcatttcttccaaactgtaagttggacagcgggtggaagaaacggttcagtttattggtcgtaatgttattaccatctgccagatccccgttgctggatttgatatacaggttgccgtttttgtcatacaccggtacgttcggcatcgcattgtatgcagagaaggtggaacctgcgaggtatccgtcggacaatacgccgttattcaaagacttggagctgtataaagagatacctgatttcaaccattttttaggggttacatccaggttcatacggatgctacctctgcgtaaacggttaacaagcaccataccctgctgatcggcatattcaccggatgcataaaatttcgctttctccgtgccgccggcgagtgataactggtgattctggataacgcccgtgcggaacacttcatccagccaatccgttctgtctggtttgccatcgccgtttatgtcaacgtcttttgccaggatgggagtaacgccgcctgttttagtagcgttctttgctttttcattctggataatagtgaagtcatcgccgttcagcagttttggtaatctcacggctttgctcatacccacgtatccgttgtaatttacattgatagtaccgttttttcctcttttggtggtaatgataattacaccggcagcagcgcgggaaccatacaatgcactggcagcggcatctttcagcacatccaccgattcaatgtcgttgggattgatgtctgcaagcggattgtaacgggtaccgttaccactgttgaaaacgttcaggttagtgagggagtttaccgggataccatccactattaccagtggctgcgagctgttggtaatggagttaatacccctgatgcggatgtttacgttatcgcccagtacaccggagttggtactgatgttcacaccggcagcgcggccagttaacgcctggtcaaagctggtggcagggcggttattgacaagtccggctgatacatgactcacagaagaagtcacatcttttcttttgagctctccataaccggttacaagtatttcattcagtactttattgctgccggataaggcaacactaatgttttggcggttgccgggtttctcttctttcgtttcatagccaacaaaagaaaacagtaagatggtattggcatctgcctggatggtaaatttaccgtcggcgcctgatacaacgcctgttttggtacccttgatgattacagatacgccaggcaggtcctgtccatcctgtgcgtctgttaccttaccagtaatcgttcgggtctgggcataggaatgcaccacaccgatggctagtaaaagccatagtagtaaaccttttttcatacggtttcaatttggtttagatatataagaaaatgttgcgggcgggcggccttgtgtcagattttggtttaattcatcgggttattgccaatcgcagtcgcctgccttgttcatagttatacagattttggtttaaagatgaagtcaatttattctgatggatcaactattattttctataggaatctaaagcctggtaaggcttatagcattgtgctaattttgttgtttacagatcatgcttccccggacggactaaatccggggcacaaatttgctatataaaaggctaaatgcaggatccgcttgtagttggcaacactacaaccaatgatacctatgcttccagaactagttggaattaaaatacgtcctcaataagcaaatagtaataacaaaaaacaatcagtacagcatgttcaaattttggttatagggtccatgtcaggttacagcgggtcaaggctgaaaacacaacaggatgattctcattagcggcataaaaatatactgtttttcgcacaaaaacaatattccccgggatgtttattttgaaatataattacttacctccagcaggttgccgtcggggtccctgaaatagatagatcggatcctgccggtagcgccggtcctttctacgattccgccttccaggatgtttattttcagcgtcgttaattccaccaggatttcttccaccggcgtatctgcaacaaagcatagatccgccgatcccacagtgggtgcaagcgctttgggatctatttccctgcctttttcatgcaggttgatcttctggtgcccgaaacgcagcgccttgcggtcatcaccaaaggtgatcacttccatgcccagcaccgtttcataaaaacgacaggtccctgatatatcttttactgtcagcaccaaatgatctaaccggttaatgaccatatgaatgtgttttattaatagcgggaagaaatcggtaaaaacgatggatcaataataagaaaaaaaatactatcacataccttacccggatgaagggttgcaaaggtaacccgatatatcccggatttccactaacttaccatatacccattaatgatcaggttcatggataagcaacgctctcccaataaactcgccacgttttttaagaaactgggcccgggattaattaccggcgccagcgatgatgatccatccggtattgctacgtattcgcaggccggcgcacaattcgggttggcaacgttatggacgtcgttactcaccttcccgctgatggcggctatccagggcatgtgtgcccgcattgggctggtcaccagccagggcctgacggttactttaaagaagaactatcccaggccggtgctttacctcatgttattatttagttttccggccatcacactgaacataggtgcagatatccagggcatgggagcggtgtgccatatgatcttccccgcagtaccggtatccgttttttgtgtaggcgtcaccgcgataatgatgttcgtgatcatccgcttctcttatgaaaaaattgccatgatcctgaagtggctctgcatgtcgctgctgctgtatattttagtgccctttatgataaagcaaaactggggcgatatcgcaaggcatacttttattcccaccattcagtacaataaagatttcttctctatcattgtcgccatactgggtaccactatttcaccttacctttttttctggcaaaccacgatggaggcggaagaccaggcacataacggcaaaggaattgtggtagataaaagagtgttgagtgaaatgaaaacagatgtaaacacgggaatgttgttctcaaatattgtgatgttctttattatcctcacggcgggcagcgtgctgtttcccgccggcgtgaaacagatagataccgtagaccaggcagccaaagcgctggagccgctggccggaaaactgacctacctgatttttgctacgggcgtattgggaacggggctgctggccatcccggtactggcaggttcccagtcgtacatgcttgcagaaacgctcgggtgggaggcggggctggataagaagttctcccaggctaaaccgttttatatctctatcatcatttcgctgatcgttggcttatcgctcgacttcctcggcgtgagtcctattaaagcgctgctgtacacggccattgcctacggccttaccgccccggtaatgattgtgatgatcatacatatcggtaacaataagaagatcatgaaagagcacacgaattcgaagttatccaatattctcggcggactcacactattactgatgactgccgccgcagtggctatgatctggttcctgttctgagtttatcatttttccacgtaaagaatttttaagcatcctcaacaaatgaatattttcaggaagatacttaccggcgccggcatcgttttttctttcactgttgccgcacaggaacgcatacacgtaaatagtttcggacttaaacctaataccttcacagatgccactaccagggtacagcaggccattgccgcctgtaaggataagcccggcgcggtattggaatttgctcccggccgttatgacttttacccggatagcgccgtgaagaaagtatattttatttccaacacctccagtgaaacagaagtgccggacaaaacaaaaaccatcggattgttttttgaaaactttaaagaccttgttatcgaaggtaatggagcagaatttgtttttcatggaaagatgaccacctgggtttttgaccggtgcgagaacattaccatgcgtcatgtgaccatagatacggaacgaccttccatgtcggaaatgacgctgaaaacggtgacgccggaaatggtggtcgcggccatacatcccgattccaaatataccatcattgatggacgcctcgaatggcatggtcccaggtggggcatgaacatattccatgcagtgctggcggataccgccaagggtatatacacttattcctcctggacgccgttcctgaaaagcagggccgccaccattgcgcctaacacggtacagtttaccggcgatttttccggcttcaaaggtgagccgggaaacgtgtttaccgtgagggatggcatccgcgaccaggcgggcgcctttatccggcattgccgcaatgtgcagctggatcatatcaacatgcgttacatgcacggcctcggcatcgtatcgcagttctctgaagagcttcactacagccatatacagatcatgccggatgaaaaaagcggccgcgtaatggccacttttgcagatggcatgcatttctccggctgcaaaggaaacatcactattacggattcgcattttaaaggcctgcacgacgatccggtgaatgtacacggcacgcacctggtgatcacggaaaaagtggcgccacgggtactgaaattgcggttcatgcatcatcaaacgtatgggttccaggctttctttgccggggacagtatcactttcgtacatgcggctacgttacaggggtatgcaaacggccgcatcaccgctgcccgtatgatcagtgaaagagagatggaagtaacgctcagcggcgatgtacccgaagggatcattgccggcgactgcctcgaaaacatcacgtgggtaccgtcgctcaccgtacgtaactgcgtgtttgaagctgtgaatacaagagggctgctggtaaccacccgtaagaaagtggtgatagaacataaccggttctacagaacaggtatgcatgccatcctcattgccgatgatgccgccagctggtttgaatccgagccggtacaggatgtgctgatcagcggtaacacctttgaaggttgcgggtataacctggcgcctgataacaattatgtgattgcgatagcgccggaaaatcatcagctgctgaaaggttttatggtgcatcgtaacatccggataaccgataatgaatttcgtatctacgactacccggtgttaacagcccgcagcacgggcaacttatcgtttattcgtaaccgtatttcctggatgaaggactatttgccacagggcgcagaacggccagctttccggcttactggttgcgagggcgtaaaggtaactggaaatgaatggcaggtgccttttaagccgcttgtgttgctgcaaagcatgacggccaaagccatcaaaacagatctgccggtaacagtaaagccatagttattttacggtccggaaaccctggttgctgaaggaagcacgctggtgaacgcggccaatatctaccgagttaaagaaggagcaggatcgttggctgcaccaccacgatccgccgcgggcatgtgccagggtagggctttcgccgggctttatgtggccggaacagaattcaaaaacgttgccatacatatcatataggccccaggcattgggttggaagctgccaacaggcgccgtatacacgtatccgtctgaactatcggcctgcaggtgatcctttccgtgccagatattggcatagcggccaatgagcgcttttttatctccaaaaaaataagtggtgcgggcgcctgcacgggaagcaatttcccattcttccagcgtaggaagccttacacctgcccagctgcagtatgcctgcgcatccttataactgatacaggtaaccgggtgctccatcttgttttcaataccgccggcacgtacgccgttggggaagcgccagcaggcagtggaatcgttgctccattcaaactcgcgtaaccctggtgcaaataccagcgcatcgtgccgttgttctgcatcagttatataaccggtggctgctacaaatgcagcaaactgccggttagtagtttcatatattgcaatgttaaaactatcgacgcttacttgtctttcggggttaagtgtatgtagatgcccacctatatggtagctgccggcgggtaccaatacgtacccaccgggcgtttgtgcagagccggcatagccactcagcaacagcaacgcggtactaaccttttttaggaagcccattgtaaaatgcagtagcccgttcaatgatcaatgcttcgttggcactattgaaattcaggtatgcctggtaactggttggttcatcggcatacaactttttgtaggaagcagaagataagaaaggtgcgtattcgttattcttcatcaatatcatcagcagggtaagtatatcatgatctttatgatcgcggttataagtgctgatcagcaaagggatcatttcccggccattgatgtcgatgatcgcttttttatagttaacaccgatgcggttactgcgctgtatggaagcgctcattaacgcgatagccgagtcgcggttagcggtcatgaaattcgactgccgctggctccagctgtattcgccgaatgcatccggcaattgcgcaaagatctttttatgttcatctggcaccggcggcatggcatcacagttctggctatacgattccgcatgaatgaggtgataagtaagcttttcgcgcatggataacgccatgtattccttttggggcaacggggtgttctcgtcttcatcatgaccggctttcgcaatcagcgccagcactttctccaaaccatccggcggccggcttattttcaggcggtactcgtgataagcctggctttctttgctgggctccacccatgtttcatcttcctgggcaaaacaaacgctgtaagcaaatacagataaaagaactgctaccatctttttcatgcaaactcaaaatttatgggaagataaagcaggcgggggtatttgccaaatgcggattttgtctttctcaggattacgctgattttacggattagctggatttttacttttggatttttttgattttattaagatataattaagggagataaagcgagtatatccgcttatatctccccaaatcctttataaaatccaaaagtaaaaatccagctaatccgtaaaatcagcgtaatcctgagaaagacaaaatccgcgtacatgaaaaaaatatgaataccctataggatttgtagactataacatatatttttgcccctgtcaatgaaaaagtacaagaccaacatcacttccggctgataagagctaacacactaatataaataactgaatgaaaaagcgatcacttttcatgtatggcatcgccatgctgttaacgtttgctgcggcagcgcagcaagtactgaaaacagccggccaggtaagatccggtaaaggcgaaaaattgccgggcatcaatatccaggtaaaacattccggtaaaggaaccgtaacggatgcagaggggcgtttcgcgctcaccgtggcgcccggggatacgctgctggtttccggcatcgggtataagaaactggaggtgccggtgaatggaaaatcacagctggatctggggctcaccgacgatgaaaccgctctcggcgaagtagtggtggtgggctatggcacccaaaagaaaagtgaccttaccaattccgtggcgcaaattaaaggcgccgatattacccgtcgcccggtatccaatatccagcaggcattacaaggattggcgcccggcgttacggtgctcgacaggggcggcgctcccggcgtatccaacgctaccatccgtgtaagaggaattaccactttcaatatcaacagcagcagtaccagcgggtacgacctgggcaaaaatgatgcgctggtaattatagacggaatagaacaacggatgcaggatatcaaccccgaagatattgaatccctctctgtgctgaaagacgccgcttccactgccatctatggatcccgcgctaccaacggcgtaatcctcatcaccacgaaaagaggcaaatcagggaaattaaccgtgaactacaacgggtactacgcctggcagaaaagtgtaaacaaaccgcaaatgatggacatcgaatcctatatgcgggaacaggtagtagcctacaccaacgccggagtggcggtgccggcgcggttctcagaggaatccatccagcagtatgtaaatgcaacggatcgctataaataccccatgcccaacacctggttcaacaccatgctcaaaacatcaccacagcaaagtcatgtgctgtcgctgtccggaggcaacgaagtggtgaaaacccggatgagcgtacgttaccaggaccagcaggggatcgtggaaaattacagcgacaagctcagtgaagtacgcatgaatgccgactacagcccgctcaatagccgcgtgcatgttgccggcgatatcaattaccgcaataattccaataccaaaccaactgtagaacccttcaacaatatgttccacggctcgctgtgggcggtacccaaatatcccgacggtacctatggcctcagcacacagggcaacaaccccctgatgtttgatgaaatcggtggcttgtcgaaacaggggatcgattattttcttggtaatgtcaggggagatgtggacctgctgccgggactccgtttctcctcacaattcggtacccgggtgatgtatacacaacagaagaactttaccaattcttacaccaacaccgataaaaataccaacatcaccaaaacggtggccaacaacagtttaacagaagtgcgtaataccttgcgggaatatacctggaataacctccttacctacgaacactcgtttggtaaacatgatctgaaagcgttggccggttattcacagatagataataaacaaaccttcctcagcgcctaccgcgaaaggttttataataacgatatcacctccataggtcagggtgcaaatgatggcactaaaagcaatagtggcagcgatgcggaatacggactgcgttcttattttggcaggatcaactacgcctatgccggcaaatacctcctggaggtaaatggccgctacgatggatcttcccgcttcgcagatggcaaacgttacagcttcttcccatccttttctgcgggatggcgtatctccaaagaacagttctttgcgccgctgctgcccattgtaaacgatctgaaactgagaggttcctatgggaaaacgggtaaccagtcggtggacctgtacagttattacgacgcactcactgccaccagttacaccttcaacggtgtgccggtaccaggctaccgccaaaccacactggctaataccgacctcggctgggaaagtaccacgcagctggatctcggtctggatgcggccttcctcgacaggcgactgaacataactgctgattactaccgtaaacttacttccgatatcctgctgaacctggatattcctgcaaccgtaggcttgaacgcaccgccgcagaatgccggggctgtagaaaataaaggggtggaaatagcggtgaactacaacagcaaacaaaacggccatctccggtataccatcggcgccaatttcagctataatgaaaataaggtaacagacctgaaaggcaccggcccgtatattaccggttcggatattgatccccgttatattatcaaaaaaggattgccgatcaacacgctttggggataccagacagatggcctgttccagaccgcggaagaaatcagtaagtatcccacgctggcatccaatactcaacccggtgatgtgaaatatgtagaccgtaacaacgatggtaaaatagatgccaacgatatgacgaacatcggcctgtcatttccgaaatacactttcggactgaacgcagggcttcagtacaaggaatttgaactgaatatcctgatccagggcgcggcaaaagtggatacccgcttatccggcgcattggccgaaatggggaaccaggaaggatttacgcacgagatctatgcgaacaattactggacgccgcagcacaccgatgcccgttttccacgtcccattaagtacgatctgcgtaacgtagctacatccgacagactggtaatcgacggctcatatatccgcctgaaaaatatccagctgtcgtatcacctacctgaatatattaccaaaaaagcgctgatcagcaggtccacggtatatgtatctgctactaacctgttcacaatttccaaactgaatgaatggaacctcgatccggaagcagaatcaggcagagcggtatactatccgcaaacatccctgttcaccgttggacttaatctgcagttttaatgttgcaaaaacgaattgttatgaactcaatccataaaagtatttatcttttcctgatcgtcctgctggcctcctgcaataaagacctgctggataccgcgcctacagaccgcctcgcagtggatgtattctggaatacagaagctgacgccaaactcgcagtaaacgcgctgtatctcgatctcgacagtaccaacatcctgtcactggatgcgctcaccgatatcgggcacaccaaccagaactttgatgtgcaggcctatattgaactgggtacctacgatcaatccagcgccaaagtatacggtgaatggaagaatgcgtataaaggcattcatgctgccaactatttcctggaaaatgtagataaggtaacttcctccacgccagcgctgatcaaccagttcaagggagaagcaaaaacactccgcgcttaccagtatattaaactggcgggtttatatggagatgtgccgctggttaccacctctattaccctggaacaggcgcggaccctgcaaagaacaccggtcgcccagatctacgatttcatcgataaggaactaacggaatcggcggcactgttacctgctgcttacgccaatgcagccgataaaggacgtattgcccgcggcgcagcctgggcgctgaaagcccgcgccgacttgttcgctggccgctatcagctcgctgccgatgcagcaacggaagtaaacggtcttggctacacgctgtatgactcctaccagaaattattcagctatgcggcagaaaataacaaagaagtgatcctcgataaacagtttatcaaagataactaccccaataacgtgttcagcatgatggcgccctacagccaaaagaacgggaacagctcctatgtgcccaccaaagtattggcggatacctaccagatgtccgacggaaaagatatccacgcgccgggcagtacttttgatgaagatcatccctacgataacagggacccgcgcctcagatacagcctgtttgtagatggcgatgtgctgccctccggtaccgtatttcatcccgcgcctaacagtggtacagcagatgccattggcagcacttacatcgcatccaccaccgggtacaacctgaaaaaatacatcaacccggaagactatgccaatccggcaaacagtggtattaacatgatcctgctgcgttatgcggaagtattgcttacttatgcagaagccaaaatagaactgaatcagctggaccagagcgtgtacaacgccattaataccgttcgccggcgggcagatgtaaatatgcccgctttgcctgcaggtcttacccaaagccagctgcgcgatgcggtgcggtatgaacgtacggtggaactggcctttgaaggactgcgtctctacgatatccgccgctggaaaacagcggagaaagtaatgacaggccccgtgtatggtattacatggaataacaatggtcagcgtacggtcgtgcaggtagtgtcatttaaccgtgcatttgataaatcgagacactacctttggccggtgccgcagaaagagcgcgacctggaccctgcactgtcacaaaatccaaactggtaattattatttatgaagcgatatatctattgtttactggcaggactttcctttggcaccgtgcctgccgtgtatgcacagcagcggcctaatatcatttttgtattaactgatgacatgggatacagcgatctcggttgttacggcaacccgcagatccgtacgcctttcctggatcatgtggcggagcagggcgtaaagtcaaccggttatatggttacctctccttcctgtacaccctccagggtaagcctgttaacaggtcgctatccaacccgctcacagcttaacttcccgatccctccgggctataagatcggtctgccggatgaagatgtgaccattgctgaaatgctgaaaggagtaggatataatacctgcatgataggcaagtggcacctgggtgatatccagccttacaatttccccgtagcacagggctttgatcattactttggtttattgtatagccacgactaccgcttcccctacgtaaaaacggatacagtgctgaagatttaccgcgacagaacacctgaaatcttccgtccggcagatacttcccttacggagttatatacaaaagaggcgattaaatacgtgaagcaacagcgaaaaaacaaacctttcttcctgtacctggcgcataacatgccacatctgccggtggccgcctctaagaagttcaggggacagtcgcccggtggtttgtatggcgatgtgattgaagagatagacgccaacctcgcagacctctggaaagcagtagagcaacaggggctcgcggataatactatttttattttcagcagtgataacggtccctggatagatttcccggcgcgcatgtcggcagataatgtgatcaagccctgggacgttggcagcaccggtattttccgtggaaagaaaggagaaacttatgaaggtggtcaccgcgttccgttcattgtgtactggaaaaaccatgtaccggttcacaaaactattacagatgcatttaccagtatggacgtactgcctacgctggcagcctgggtaaatgcaccgcttcctgccggcaggaagctagatggcgaatccgtactggatctgctcaccggtaaaaaagagcacatcgctcattcacctatttattacgtaaacaatggtacaccggaagcgatccgtgtgggcgactggaaactgcgcagaatcaccgatcctaagacaggcactaaaaacatagagctgtttaaccttgggtccgatgtacgggaacgtaccaacgtagcacaggagtatcctgataaagtgagcgcattggcgcagttgttggaccagtacaatggtaatacagcgaattgatcttgctataataaaaaagcagcgaaggctttcttcgctgctttaattccttgcaaattacaggtcacggcgccatcatcagctgcatggcctttttgtgctccagttcccggtgatgacggaaaacgctttttgttacaaaatgcccaagcgccaggcccacccatacatcgctgctccagtgccggttttcatacaggcgggtggcgccggtgaggccggcaatgccataggatacccagggtacccatggatgatcttttccatacagctccgcaaaagcggtggctactgtcatcacggtgaggctatgtccggaggggaatgaggtatgctttttatccttactgaaaggagggtcaaagttaaacggggaatcgtagtaggtgggacgtccgcgtcttatcacacttttaagcgtggcataaatggcggtggaaatgatcagggatttggcggccatcagcccgccgtgttccaggttgcggtcctttgcaatcactcccactacatacataccggctacaatgtacggggaataggcattgccaaagggttctatctggtcggttacgctggtaacaaaattcgactggtgacgtacaaaaaactgttttacgccgtaatcccctcccagcaggatgccggtcacaccggtaattacgcccagccggatgtaatcctttttctcccaatgggcgggccgcgctaccgtatatttcaggtcctgccagatacttcccaggtaggcgccgtttatgcggtaccgtattaaggtatcgctggcgttgatcaccgggcggatgctgtcagccaccacgggcaggctgctgtccgattgcgcctgtatatggggagaaaaaataaccagtaaaagaaatgtaagcctgaatcccatctgtttaaatactttggagcgagcacgaaagtagtatttttagggagaagcagcgcgggaattgttaactttacgatcacattaatcaacaattatgagaaactgtttcctcgcacttttcctgctttttgccacccgcagtgccattgcacaacgggttgcaccagatgagatttctacctccaagggaaatcttactatccagcccattaaccatgccgacctgctattgtcggtggcaggcaaaaccatgtatgtggaccctgctggtggtgccgaaccgcataaaggattggcagcgccggatatcattttggtaacggatattcatggtgaccattttgacccagctaccatcaacgcggttaaaacggcgcatactatcattgttgccccggaagtagtaacagctaaactggaagggataccagccgcgcagatcgtgaccctgaaaaacggggagtccaaaacagtagccggaatttccatccatgccatccccatgtacaacctgcccgaaagcgccaccgctatgcacaccaaaggcaggggcaacggttatgtgttgaaggtaggaggcaagtcggtttatatctccggcgacacccagggtattccggaaatgagggcgctgaaaaatattgatgtggctttcgtttgcatgaacctgccatatacgatggatgtaactgaagccgcagatgcagtgctggcctttgcgccaaaaattgtgtacccttatcactaccgtggtaaaggcggactggcggatgtgaataagttcaaaagcctggtagatgcaggtaacaaaggaattgaagtaaggttgcgcgactggtacgcgaaataacaacgcaatttattgctggaagaatagcccgaatgctggtgtaaaatccttaaatttagtatttacaccagcatttaatttcagcagcacatgacagaaaacaatatcatttgcccgggctgtaaactacatcttgcgtaccagcaatttgccccttcagaaagatataatgcatccggtgaatgcctggatctcttcaatcagctcgccgaccgcacctttgcttttcagcacccggattttcatcatcagttgtctgtagatgcctacggcgcccaacatgccggtggcgtgagccggaacatcatcaccgcctacgcgttgatagggctgtatctggcgctggaaaaaaattacaccgggcggcaggtacaacatgtgcacagcattatcccgcagcaatcatgggagaagctggaacctcccgctaccaccggcgccctcaccgttaaggatgtactcaaagcaaccactgaggaggaactatatgccgccatgaaaaaatgggcacaggcagtatgggatagctggagcgcacaccattcctttattaaagaaaagaccgcccattacatttaaaagaccaggaacgggatatttgtatagttttgcggcttgttatgcaactatcttcttttcccgaactgattattgtaccggtggcggtcatcgccattgcggtgctatgtgtaataaaacgtaagcttaccccgggcggtggcgtaatggcagcggcagtggcgctgctggtagcagcaggcgccggctacggcggactattattgctcggtgcattttttatcatgggcgtaatcgccacctcacataaaaaggatctgaaaatttttcccggagaaaatcatcccgggcaacgcacggccggccaggtatttgccaatggcggagtagctgctttcatggcattgctggcactcatgcatcccgacatcgacgatatgtaccagatgatgctggccgccagcctggctgctgccactgccgatacactgtcgtccgaactgggaatggtatacggccgcaacttttataatatcctcacctttaaaaaagatacccggggactggatggcgtaatcagcctggaaggtaccctgctgggcgccgcaggcgcaggtatcctcgctttgctgtacggtatcagctttggtatggacgaaaccgtatggtttgtagccatcgcgggtatcgccggtaacctggcagactccctgctgggcgccaccctggagcgaaaacatattattggtaatgatgcggtgaacttcagcaatacgttgtttggtgcaattacggcgatggtgctgtacctgttgtaacgttatccccctgtaccccggacggcgcaccggtaaactgcggtccgggtattaatacgatagaagaagaacaattcccgaccattgctcccgatggcagcctgtacttttccagtaaaggatggaaaggtatgggaggattcgatattttccatacttccgggagtaaagcccaatggagtataccggaaaacctccgctatccgaccaattctgcaggagacgatttttattttgtagccgcagctaacggaaacacctatttcgcctccaaccgcaccggcggcaaaggaagtgatgatatttattccattactccacctcccatatatacgctcacccaattaccgccggcactcgtgatcccattcaccggtacggtatgcccaggcgcctgtattgatatctacaacaaacaacggcaagtcggctggtgctttaccggggaggccggcagggaaattaacctgacactggaaaaagataccgactatgaaatccgtctctattatccggggggcagacgcgtggaaaccattgagtttaatacacgcggtatgaaagacgcagaagtgcggagaaaagatatctgtaaataaaaagaagcacgaatgacagctttttttctatttttacgacatcaatcaaaataccgatctctccgcgcctagatttttatggaatgcaccagttagaagatgagaaggaattgctccggaaggtagccgacgccgatcaggaggcattcagtatactttatgaacattatgccaggcatgtgtatggactcgccctgcgcctgatgaaatcaccggagatcgcacaggatcttacccaggaagtttttgtaagaatatgggtaaaaaggtcacaactgttcactgtacagcaattcagaccctggctcaataccatcacccgcaacatggcgatggattacctgcgaaaaaaagtagcggctccggagcaggaagaatacctgaccagtttttttaccgatacaacaccttctatagaagaacaactggcgctgaaacagctggaaggagccattttacaggccgtagaccaactttcccctcaactaaaaaccgcttttatgctaagccgttttcagggtttaacccatacggaaatcgcacaacgcatgaatatttcacccattacctctaaaagtcacctggtaagggcactggccattattcgcaaatacctggaggaaaacttcccggaaatagcactggtagcccttttatacctgacgccattattttctgcttttttttaagaaagtatgcattacccccgggatgtatttacgtctatagtagcaaggggtaataacaacatcaaccattattattttaatgcatgcaacctgccgataacgaatttgatgaactgttccgcaagtacacggaagataccatgacaccggaagagttccggcgatggcgggtgatgctgctggatgaacgtaacaccgtcaggctggaaagtttgctggcagcactggccgaaaccgatcattcggcattcgggcaggatgcccccctgaaggaaatgtatgccaatattatacgggtcactccactaaaagcaaccggtaaaacaccacgccgcttaaattaccggcagtatgcatggtgggcagcggcggcatcgctgctgttactcgtggctaccggtattttgcgctggcagcaaccatccggtaaacaacagctggcaacgaaatacgatgtggcgcctggtggcagtaaagccgtattaaaactggccgatggctccgtgataacactcgacagcgtagccaaacggcaaatacagctgggcaatgccactgcccagcaggtaaacggccagctgaattatgcgccttcctccggtggagaagcggccggcataaatgtactcacaacgccccgtggaggccagttccaggtagtactgcccgatggcaccagagtatggctgaacgccgcctcttcacttagttatcccactgcctttactggcaaagaacggctggtggaagtgagcggggaagcctactttgaagtggcaaaggacgcacacaaacccttccgggtaaagatcagcaaccagaaaaactatattgatgtactgggaacccactttaatgtaaatgcctaccccgatgaagcagccatccgttccaccttgctggaagggcgtatccgcttcagcgctgcgcaggcggtggtattatcgccgggccagcaggctgttttaacggccggcacacaaacgccgcaagtggtgaatggagtagataccagcgctgtaatggcgtggcgcagcggcctgtttaattttgaaggacaacacctccgcgaggtaatgcggcaactggccagatggtataacatcgaggtggtgtacgaccaggaagtgccggatgtggtgttcggcggcaaaatagtgcggaatgtaagcctcacacaattactgaaaatattgaccgatgccggcattcacttcagactggagccgggaggaaaattgatcatacaacctaaataaaccaatcattaaaaaacgaaaaccgaaagtgcttggacccacttccggttagtagttcagtcgttttaaattttccgtaagagaatctattatcaaccaaaccaaatgcaatttatgcaaaaaaatgcttattgtggccacctgtcatggtggaggcatcgttacattaccaaaatcttgttcgtaatgaggcttacctttttactgctgactattacttttctaagtgtgcatgcgtcaactttttcacaaagtgttacactttcagggaaagatctttccctgaagaaaatttttactgctattgaacagcaaacaggctatgtagttttctacaacagtgaattgctgaaaacagcgaaaccagtcacggtgacagcggaagatatgccattgacggccttcctggaagcggcttttaaagatcagctgttgaattatacgatcaccggaaaagtgattacgttcgcggaaaagccaccaccactggaaggaaagctgcctttcatcacaagcacttttattgaagtgaacggtaaagtactgaatgctgccacgaaagaaccaatcatatcggcatctgtaaaaataaaaggaaagaacaggggagcgattaccgatggagaaggcaacttccgcctgaacgccgagcccggcaatgtgctgatcatcacctccctgcaatatgaaacacaggaagtgaagatcattcccaaccaacccttcctcacggtaatgatgaaccccggtgtatctaaactggatgaaacggtagtaacggcttttggtatagaaaaaagttcgaaagaagtaggctatagcgtagccaaagtgagcggggcagatatcaaccgcgccaattccggcaacctgctacaggggctggctggtaaagtatccggtttaaatatcgctatacaaagcgccgacatgaacccgcagatgcgggtgctgatccgtggtatccgctctttcagtaccaccagcaacaaccagccgttgttcatcctcaatggcacgccgttatcttttgggtcggacattaactccgccgccatgatcatggactttatcaataacatcaaccctgcggatattgaaaatgtaaccgtgctgaaaggcgccaacggtacggctttatacggaccggaaggtgtgaatggcgtgatcatcatcaccacaaaaaaaggacaaaaaggcaaacctactatcaatttccgcaacagcgtaaatttttcccgcctcgatttccggaatgacaacagtaagcaaagacgcttcggtaccggtagcggcctggtagacgacaaaggaaacggtatttacagcagcctggataaaagcggctggggccccgcctacgacggccggctggtacccatcggaagagccgatgaaaacggcgactaccagatggtaacctactccgataaaaaggatgcaaggcgcttcttcaacgtaggtcgcaccatccagaataatttatccatctcccagtcagatgctatctccgatttctatctcggcctcaacgctgtcaatcaaacaggcatgataccgggcgataaacaggacggcgtaaacctcttcttcagcgcggggcgtaaactgggcaaactgaatgtgcaactgaacctcaattactcccgtaccaccgctgataaaggtcctacgttcgacgatatgctgagcacacctacttatatccctatcctcagttacaaaaattatgagaacaataagtgggcagatataaaccactactggaatgataacgacgtaatgagtccgtatcagcaagcggcagaccgtagaaagaaaagtaccgataacgcattggtgacgggtttgatactaaccgcaaaggtgctgccgtggctaacggtaacagacaaacccagcgtggtgtatgatggcttctacgaaaaaaccgtttcacagccaatgaacttttctgattttgccaaacaatatggcggctataaccgcttccgcgaccggcttacgcagttgggagaggaatcccgatccaataccacgcttaacaacgacctgctgatcacggcattaaaccacgcaggcaattttaatttccgcactacgttagggagctctgtaaaagaaaattattataagaaagtttccggtagtggtaatcccatcatcccggtattcaacctcgcgttttcccgcgatctgccatatggcgccgaggaatcattgctcacccgcaactattccttttttggtacgtcaggcattggctacaaagataaagtgtttgtggaactgatggcacgcaacgactgggattccaagcgcgcaaaagccggcaggggaaaagatctctacgtgggcggtaatacttccgtgatcctgaatgaagttatttcttccctgaaaaattatacctggttatcccgtctgcagttacgagccgcggtaaacaccacggccaatatgaacattgaaccttaccagtctgaacggaccctttcaatggcctattctaacggcttcccttatcccggcacatccgatgaaggcgtaattgcttataactatatgcagggtaatcccaatccttttctgaaaccggaaaagatcctcagccaggaatacggcgtcagcgcaggcttttggaagaacagagtcgcgttggacttcacctggtatacccaacggaataatggtgtgatcatgaaagtaaagatcccgtggctgagcggtggcagcaccatcgataacctgggcatcatgcgcaactatggctgggaagccgatctgaaactggaccccatcattaaaaccaggagcggatttactttcagtgcagatatacgtgtagccatgaacgataataaagtgatctctatcagcgatgcctatgatggattgttcccgctgagaactccttattacggaagcatgtacggagtggtggcccgtaccgggcagcgtgcatttgaataccaggtgtatgatttgaaaaaagatgcagaaggcagggtgatagtaaataaagaaaccggtatgccggacgcggacattaataaccccatctacggtggacgcaccttacccaaatattccgggggaatgaacctgaactttgcctttaaaggatttacgctggccgtactgggagaattcaataccggcgctatgcactactctgaccttatgcaatacgatgtgcagtatgggttcagcgtgctcactgtgtacaacgaccgtaaaccatttatctatccgaattccgtgtacgacgatggtaccgggaaactggtccctaacacagatgtatatacgaaaagtgctaaccaggaattatacagtcacttccagaacgcttctgccagctacctgaccaaagccgacttcttcaaaatacgcgaagtggtgataggatacgaaaggttcttcaaaacaaaaacaattaaaaaactcaatttaagtgtatacggtagaaacgtgtttaacttctacacaaagaaaaacaaaacgggggatccgcaattgatcaaaggtcctggcgacagagggtaccgtaccattcccgacaacctttccggatctgcgtccggtgtttctaccgttccgggtgtggcacaatacggcgtaatcactaccgtgagtttttaacaacaaaaaattaaactgatgcgcaaaagatatcacattttagcgggagccttactaactgccgccacctttatggcaggttgtaaaaaaggctggatagacattaactacaatccgctgcagcttacagaaaacaatgccacaccggacctcatgttacccgatatgttgttcaacagtatttccggcgtggagaatcagctggaagcacaatggatgggctattggacatatgcggagtatgccaccggcgtcactgaacttacctattaccagttaaatgacggttctttcggaaccagttcccccgatccgaccattctcctttgggaagccaatgccaggttgcatgaccagccctattacataggaattgcgaaagcgatccgggcgctgcaatggagccgcgcggtagataacaataacaatatgccctatagcgaggccaataataccagtatccggaaacctaagtatgataccggggagttcatttatgaagacctgatgacgcagctggattcggctatcatcctcatccgcgatgctccgcaggacaaagcgctccgtatctccattgcagatattatgttccatggcgaaaaacaaaagtggttccggtttatcaataccctcaaactgcgcatgctgatacatcaggcgaataagcccggcagggaaaattatatcaaaggtgaaatagcaaagattaccgcacaaggctccggtttcctgaacagtggagaagatgccagtgtaaatccaggctttaccgatgtgaaaccttccaagtactacgctaaatattcgcagtatgatgtgtatgtccgctattatgggttagcgggtaataaatctattcccaactggcagattgcatccgcaaatgtaaccgccatgaatatgctgaaagagaaccgcgatccccgtcttggtttcttttactcgcctgcccgtgttccgctgcctgccaatgcaccggaaccattcgcacaacccggtccgcaggaatacaggggcaataaatttggcctgccggtagatgaacagcagtttccttataaccgcacggagtatgtatcgcaggtgggcggtgtacgcactttccgtacggccgtatcgcctttgtcaaccggcattataaaaggctatgacatgccctgctggattatcaccagtatagaaagtgcgttcctccaggcagaagccattcagcggggctggttgcccggtgatcccgaaacagcctataagaatgcggtaaaggaatccttccggtggcttaatgtaggtggcaacaccacggtgccttccctgtcggacgatgctttcaatacctggtacaatgcggaaacagctgccgccaatccaaaggtgagctgggccgccgcgccggataaatacaaactgctgatgttccagaaatacatggcctttaatggtattgaaccttttgaagcatgggtggactatcgccgcaacggcgccttcccggacattccattgtcttacgatccggccaggataggtaataccatgccgatccggtgcccttacccgctatcagaaatggtgcagaataaggaaaacctcctggcgcagggacctatcgacatcttcaccagcaaaatctggtggatgccataatcatctttttaaaaaaataacagttatcatgataaaattttgttgcagcattgcagcatgggggatgctattgtctgtatttaccggcagcatagctcatgcacaacaaaccggtgagtcagtgccgatggacccggaagtaacaataggtaaactccctaacgggtttacctattatatccggaaaaataccacaccggaaaaaagagcggtaatgtacctggtaaacaaagccgggtctatcctggaaacagacgaacaacgcgggctggcgcatttcctggagcacatggcgtttaacggcactacccattatcccaaaaatgaactggtaaattatcttcagaagtcgggtgtgcgctttggcgctgacctcaacgcttacacgggtttcgatgagacagtataccaattgcccgtatctacggaagataaaaccgttttccgtaatgccatgcagatcatgcgcgactgggcacaggaactcacgctcagcgatgaagaaatagataatgaaagaggcgtgatcctggaagaaaaaagacaacatctgggctccgcacaacgcatacaggataaagtgatgccactgtcggtgaatcaatcgctgtacgcctcccgtctcccgataggcacggaagaagtactgaaaaatttcggacatgaacaaatccgtgctttttataaagactggtaccggcccgacctgcaggcgctgataatagtgggagatgtaaatgtggcgcagatagagaagtcgatccgcgctatgttctccgatttgcgctcacccgcgcagccgaaggaacgtaagtacaccaccatcccgctcaccgggaaaaaccagttcctggtggtaacagatccggaagtggctaccacgcggctggaactctccatcaaacaacagggtaacgtcattaaaacaaaaacagatttcagcaataccctcatccaatcgttgttcaatagcatggtcagcgatcgtttaaatgaggtggcacggcaaaaaaatgcgccattcctcagtggcagcgcaggattcagcaaaatgatggccaatatcagcggacttagcggcagggtagtactcaaacccggtgaaacggaaaaaggcgtcaaagcatggtggacagaattgcaacggataaagcaatatggcttcaccgcgggtgaattgcaacgggcgaaaacatcgttcctcagcagtatttccctgagctacaaggaacgggacaaaaccccgtcggaatcatatgtaaaagaatatgtaaggcacttcctggaaggcgaagcaagtccgggtaacgcatatgaaacagccctgtataaagccagcgccgatacacttacgctgccgggctttaatgctgctatacaatcttactttaaggataccgaccgcgatcttatcctcgttgccaacgataaacagaaagactcccttccttcggaaaccatggtactgcaatggatgaacgaagccgcctcagcgcccatcgcggcttatgaggataaaaaagtattgcgcaccacgttgctggacaacgcgccgcaacccggcgtgattaccagcgaggaagtgatcaaagacctgggcattacttcactggaattcagtaacgggataaaagtattgctgaaaccaaccacctttaaaaaagatgaaatcttatttaatggtttcaaccctggaggcttatcacaggtaagcgacgctgatttttataacgccagcatcgccgcttcactcgtaagcgccagcggcgtatcggatatgacccaggcggaattacgcaaattgctcaccgggaaaaatgtatcagtggcgccattcatcagcgaaacatcagaaggcatttccggcggttccgcggatgaagacctggaaactgcgctgcaactggtatacctgtattttaccagtccgcgtaaagaccccgtgatgttcagcaatatgacagaacaggcgcggttgtcgtacgccaatgcaaacaaagcgccgcggcaactttacagcgataccctcagcgctgtaatggccaattaccacttccgtaagatgcagatgccggagcaacaactgaacctgcttgatgcagatcaggcactggctatctataaaaaccgttttgcagatgccgccggctttaccttcaccttcgtggggaattttaatacggatagcatcaaaccgttgctggccaggtacctgggatcgttgcctgctttacatcgccgggaggaagtgaaggatcttcagctgaattatccgcagggcagggtagtgaaaaaagtgatagccggtaaagaaccgcaggcaattgttacccttgctttcagtggttcatttccgtatgatgttagcaccagcgaccagatgaaagcactggcaggcgtactcaatattcgtcttacagaacggctccgcgaacaggaagccggcgtatacagcgttaacgtaaatgccaatacccgcaaggtcccttccggggaatatatgtttggcattaattttatttgcgatccacgcaacgtggaatccctgatcctcagcgttaacagtgaaatcatgaaactgaaaacaacgggggtggcagacgacgatgtgataaaatataaggcaggctataaaagcagtgtggagagagcgtttaaagaaaacggcttctggctgaattatattacttccgccctgtttaacggggatcctttacaacaaccggatataaaagcccggctccagaaaatcaccccggaaactttacagcaaacggctgtaaaatattttaacaatgctaactatatccgcgccatactggtgccggaaagtaattaaataaacgtgaaagcactatacgccgggatcgcatttttccttgccggatatttcgtaaccgtctcctgcgccacggcgcaggggcggactacggacagcctgccggcaaccaaaaccgatacagcccatcccaaaatcattggacttaaagcggtggagataaccgttgccaaaccgccttttacacttcgtaacgataccctggaatttgatgcttcggccatcaggctggctgcaaatgccagcgtattgcagctgctgaaaaagctgcccggtgtggtgataggcagtgatggcagtattactgtaaacggaaaacccgtgacaaagatcaaagtagatggcagggaattttttggagataataaagaggccgctaccaaatacctgcctgcagacatcattgataagatagaagtaaccgacaccaaagacgttgccgcccaacgttcccttgcagtgaaagccccggcggaagatgttaccgttaacctcgtccttaaaaaagataaaaataccggcatcatgggaaacatcactgccggtgcgggtagccatcgccgttatcttgcagatggaatgatcagctccatgcgcaatcctacgcgcatcagtgtgatggcggcggcaaagaatgttacagatgaaacgggcggcgctataatgatgtcgccatccggtatggtcggtggcggaggaggattaccggaatacaacaacggcagtatcaacatcaacacaaaaccaggtaaaaagctcacactggatgtgaactataattataacaataccaaaaataaccagaccaccatcaccgaccggctcaatttattaccggataacagcttccataatcaaaccaatagtgatgctgtagccgggaacagtcagcatcagctgtatacgaatcttgtttatgaaaaagattcactcaccacctggaccttcaggagtaacgcgggtatagggaaaagcagcaataatttacaaatgtattccctgtcggaaacctccggcggaactttactgaacacactctcttcccggagtaacggggaagcacatacgggtaatggcggcagcgaaatcaatttcaataaaaccagccgaaaccgcaggctcaaccttaataccacctggaagtttgacgccggcagtaaaaaggaaaacgaatacaataattcagttaataacttttatacagataatagtgttagtcaccgtgattctgtaaatcagtatatcagctctgctgaaaccagttttaataataattttacatttaatttatcggcgtccttaggacatggttttgtggcggcgttggactatacgctgggtaccatgtacaacaggcagctccgggaagtatttaaagaagatcccgtgtccggcaaatacggcatgcgggacagcgctttgtccggcagtagtagaaataccagttttacccatacaccatctgtgcagctggcctggaaaaatgatcgcctgagcatagcgctgaacaccggtatgcggatcctgcaacaggaaaaccgcctgttgtggctggattccgtgattaagatccatcagcagcaatttgcgcctaacctgcaactgaattattccctcagcaaatacgggcgattgttcaccaactattccatttcttcttccgctccttcggcagagcagttgtcgcccgtagtagataacaccaacccgttgttcatgaaggtcggcaaccctttgctgaaaggcgtctttacccaaaacgttgcgctgatgttttacatttatcagccggtgaaagggtttagtttcaatctcggcgccaacgggacagtggtccgtaatgaaattgtggcggatcagcggtatgattccctgggccgacaaatcagtacctttcagaacgtgaatggtacgtggagaatgatggtacatggaaatatcaatcttcagaaaaaaaagaacagctggacatttaacaatggccttaacgtgagtatgaaccggaacaggagtattggcctggtggcgggtgaggaaaatatctccaacgggtggaccgccggcgccggtgtttatttttccgttatttacaaagagtggctgacaatatcgcccgctgtaaacgtagatgtgaataataccgtttattcgctgcctggtattgacaatgttaactataccacacaacgttttaacctgcaatggcagctgattcctgttaagcgcctggagttgtcgggcgatatggcgtacaattataattcgcaggtaacggcgccggatcaacgccgttattttatttgtaacagtgccgtagcttacagttttggaaagaaggagcagctgaaactaaaatgcaggataaatgatctttttaataacaacaccaatatttctaacataacaacagctacctataccgaaacaaagcaggtaaatgctttacaacgttatgtcatgatcactttccagtatttttttggcaagatggggccgcagtaagaatattctttgaagggttcctgcacagggctatctttgaaaaataactattattttcaggagcatgaaattgctgacagatagtatccttcaacatgtaccgctgcgcgatgccgatattaaacgtattcccggctattttgaaccggtgcgaacccgccgccggcagttcctgttgcgggaaggcgacgtttgccgctacgaattttttgtgctgaaaggttgttgccgccagtatgaaaaagatgccaccggcaaagaaaatgtgttgcagttcagcgtggaaggctggtggatcacggacctcgacagcatgctatccggtcagccatcccggtttaacattgatgtgctggaaggaggcgaggtgctgcgcatcacccggcagcaactggaacaactatttaacgatatcccggcagtggagcggtattaccgcattatttcccagcgaggctacatcgcgttgcaacgtcgtatcttgtcgctgcagaagcctgccatagagcggtaccgtgggtttgtaagctgctaccctttcctcgaaacacggctgccccagcaccaggtagcggcttacctgggcattacgcccgaatcgttgagccgtttacgtcgaaaaatagcaaaggagccgttttaaatttcttatcatttgtcattgttttggcgcagcgaagtgtacaactttgtgctaaagttttatatatgaccacacacccggtattggcgcctgttacactggcgcagcaatttgttaagaacagggtggtgctggcgcctatgagtcgcgccagcgctacattgcagggcattcccacagcagccatgcacgcttactacgaacgttttgccctcggcggttttgggatcattatcaccgagggattatataccgatgcagtagccagccaggcatatccgcatcagccaggactggtcacatcacagcaggtggccggttggcaggagctggcggtcaaagtaaaaacacctggcagcttatttattgcacagctgatgcatgccggcgctttatcgcagcatttgccgaacacgctggcgccttccgtggtaacgccgctgggccgcaagctgcgctcctatggtggcggcgacggtcccttcccggttccggctgccatgacgcgcaatgatattgccatcgcagtggcaggatatgccgccgcggcggttaatgccgtagccgccggtttcgatggaatagaagtgcatgccgccaatggttacctgccggatcagtttttaacggagtataccaatctgcggaatgatgagtatggcgggtctgttgagaaccgcttccgtattatcgcggaaatcattaccgctatcaggcaggcagtgcccccgcattttattatcgggttgcgcctgtcggaaggaaaagtgaacaacttcacctatcgctggcccgatggcgctattacagcagcagcactacttgaagaagtaagaaaggtatctccggattatatccatatttcaggggaaggcagcacctgggaaaaactgggcgcttatgaacatggggaaacgctcacgggtatggctaaacgcattgtgcagcggccggtaattgccaacggcggtatggaagaactggccgtggctggaagggccttaacggaaggacatgcggatcttatttcgctgggaaaggcggcactcgccaatccaaactggccggcacgtgtggccgcaggagagccgttcactccttttgagcggggaatggcggagccttttccgccggtacagtaaaatccgggagcagcgggttattcacctctccataaaaatttatttaggaagcggcccgttattcgccattattcagcatctccatttcgaggagcttactgccgcctgcaaaatctgcagcagcatccgggcataataccattcccagggagttcatcatcctttgggcaaccaggtcgatatcttcggtagtggtggcgagaaacggcgcctggcttttcagccgctggattaacgcatttttctgggtaacagaaatgtctaccagcttgttaattctttctacagccgctttatatagttcgtcgtaataaaaaagcatgttcatgtcaacaggttattttgtatggctcaaatgtagcccatcgcctataatcctggctatatgaaaatattatgacctataattaataattataaatggatctggccattttgatgaaacgtttgttgaggtcgctggtttcgcctttacgttgaatgaagtaaaaactgcgttctatccgcaggccttcaaaggaaaggatcgttaattcgccgtgttgcagctctttagcaatggagcgggtagagaggaatcctacgcaaccggattccaggaggaaattcttcagcgcctcggtgcctcccagcctgacctttattttcaggtcgttgagccggatcctgcttttctgtagccccttcttgagcgcttccagggtgccgctgccacgttcgcggatagctacaggcatctgcaggatatctttcagcgcgtagttctttttacgggcaagaggattgtcgcggctgcataccgctacgatctggtctttcagaaatgactggtaggtaatattgctgagttgtcctttttcttcggtaacgcctatattaatttctttgtcgagcagtgcctgcaatacaatttcactgttccggttgagcagggaaatatccaccagggggtattcgcggtgaaaggccgacattactttgggtagtatatacagcgcagcagtggtactggcgcccaggttaagcatgccggtggcctgctgctggtcgtggatcacggaaatgtcgaactcagtttcctgttgtatatgacgtacggtaagcaggcggttgtacagcagctgaccagcttctgtcaactctatctgcaaaccttttctttcaaataatttggttttatactgttcttccaaccctttgatatgtgtgcttactgccggctgggaaataaacaatgcctggctggcctttgaaaagcttttctgatgggccacttccataaagatctggtgtcggttagatagcatgtgcgcaaatttatggagcgtataaaatttctctccggcggataaaacggaccttgtctttataatccgttatcctgttattcatgatttccactttttctatccagttatgatgaaggtcgtaggtaaattcataccggtacacggttctttccacagcatcggtggtggtaaccctgtcggatattttcgcggtaagatgtccctgctcattatactggcaaataatggtttccactgcctggttgctgtcaaaaccatcagcgtcctcgaatttgtattcttccagtagctgctgccggctgttgtacttacttttggtgatttcctgcaaggcaccaaaagagtagtagcgggtaatttctatccggcagccgtcgtcatcagtgctggtgttggtttcccattgctcgttgtacggatcttcttctacaggcagtgggtcgttgttttccagttgttcaagcacgttgcctgcttcatcgtaccgggtgtaaaaggtatcttccccatagtattcggtacattctttcagcgccccgttttcaaagtagcggtttttgtagatgggcccctttgctgcggaggtcagcgctttttccagcaggttcccctgttcatcgaaagtataggtaagggttttatccagttggtgggtggaggtataatcctcccatctgagcaataatcctttttcatcgaaaaaagagagttcatacccgtaatatttgccatcggggtctgtggtagcatatttcatttgctgtaccggcccggtcagctcagtatctgccaatgtttgtttcatggtacctaaagttattggaaacaaaataaacttccactatttaagtacttatttctgcatgatattttttggagtggtgttttccaggtatttttttccgggagagatggaagtgcggtaatccccgtaaagccaggcagccctcacgggagctgcctggcggaaggaggggttatttgtcgaacgtcatgttttcaaacttatccagttttgccatgattccccatccataaaagtcgttggccagggcgatcagtatttcattgtcgccagctaccagcggaagggagaaagacgcattatccacggtgcagcggccatccggttgtttcatcagcgggtaggagtagaggtttttgtctacgtacacaaatttatcgttcacaaatacccatacttcgtcgctgaagccgaggtgcagttgtcgtgtttgcgctacagcagaacggatatttgttttcagccacacgatgcgccgggcgcggttttcagcgccgccaaatttgcgggttacgttgatcagtccccgcctttcggcgcggatggtttcccatggtgtttcttttccgggtatccatgctttgctgaaatcaatttgatcaggggtagccattggctgggtgatttgccaggtgcggaggtaggcggcgtcattgttggtaatgtcgatgccttcaccgggaggcagtccttccgtttgatccggtttcaccaccaggttggcaatgaccgcctgcccgtcgaatgcaaggccgccatgccaggtattgctttccagtcgcggcacttccagcaccggccgggaggtatcgttcacgtacacccgcatttgcctgccggaaataaccagcttcacatggttccagtcgtctttggaaatccaggcggcagcctggtactggtccagcatatcccagaggttaacgccatcgatatgcggtgcatactgcaccgcatcgcctttaccggaagaaggcgtacggaaataaaagcattcgttctctttccggctggcgcgcctgaaataaaacgatgtgaaagtagaaacaggttgcacgtcgtattcgatggtgccgtttgtaaagtcaaggtttttcagcactacggtgtcgttccggttcaacagcttcatcgccggtaccgatttatacgtgataaactctaccgtgccgggttgaaacgaccagtgtccggcttccagggggaccttgataatatcctgactgccggggtggccggttttctttttttgtgctgctgcgcataatggaagcaataggaataagcacgcggtgcggatttttgtcatgaccagtgttttaaatttaaatgctgcagcaaatctgaataataactaatttcagggcgaatcattggcgcatcaagtgtgtgcaaatccgtgcaagcttgtaatagactaccaggaaatgaataatagttttgagattaattacatacgaaagtgccttgagctggcagaagcccggttgaaccgtggtgacgccagcgagtggacaagctatgattttgaaaaactaagtgccgccatagaagaagctacgggggtgatattgagcgttactaccctgaaacggctgtggggaaaactgaagtacaccaatatgcccgccaccactacgctgaataccctggcacaatttgccgggtatgccgactggcgggagtttaaacgtcttgccaccttgctgcctggggatattacgactgcggcaaccagccctgaagcgatggttgagtcgttgccagttgatgatgccacatctttaaatatggccacgggggaaactcctgtcagtcagacagtatccggttatacaacaggccatggcatgaccactgccagcactcattcacccgcagcaacgccaccaaaacgcagtaaatggacttactggctgctcgccctggtaccaataggaattctcgtatatgccttactgttatccaataccaaaccaggcaaactaattgatacaactgcattttcgttcagctccaataaagtagttatggatggagtgcctaattctgttattttcagctataatgctgccgcagcagggaaggattctgtgttcattgcgcaaacctgggatatcaggcggaaaatgccggtatctgccaaagaaaaaacatacactgctatttattatgagccgggttatttcaaggcgaaactgatggtgggtaaacagatcgtaaaagaacacgaactgatgatcagctccggtggctggctggctatggtagaacaagagcccggcacaccactgtatttccggaagaatgaagtcataaaaggaaacggcctggaagtgaatgaagcattgttgtcggcatatcacgttccgctgcaacctgttcctcccgccatacgcttttataatgtacagccccttggcgacctgcaaacggatcactttacttttgaaaccacgctgaagagcggttttcaactgggcaccgctgcctgtcagcgggtggaggtgttgctcctgtgtaaaaatgatttgatctccatcccgttgtgcgcgccaggatgcgtgggagacctgtcgctgtttgccgccggcgttgccctcaacagccggaacaccgacctctcgaaatttggcgccgacctggcaaaatgggtaaaactccgtgtagtggcgaaagaccagcacctgcagttttttgtgaacgacagcgctgctgcggagctcacgttttccaatccgccttccggcatcgtcggtgtgcaataccggttcaatggcactggcgcagtaaaggatacccgctttacgaaagatagcaccgtgattgaattacaataatagctgctgcctatccatctctctgaaaacaattactgctgctttattcctaaaaagctttatttttctctggaacatattcccgttatgaaaagtaagttatggtttctcagcagcctcctttactgtttatgcaccaaggcgcagttgccggagcgtttacaggttaccccggatggtcattatcttcaatatgccaacgggcaaccctttttctggttgggcgataccggctgggaattgtttcaccggctggataccgcggaaattaaatactacctcgataaccgtgcccgcaaaggctttaccgtaatccaggcagtagtgctggcggaatttgatggtcttcgcaaacccaaccgctatggacaactgccgttgctgaatgaaaaccctgccactcccaacaacgcttatttcacgttaatagacagcaccatcagctgggcaatgcagcgaggaatgtacatagggctgctgcctgcctggggcgataaggtgacaaagttatggggcgaaggccctgtggtgtttgataccactaacgcttacgtatatgggaaatggataggcaacaggtatcgtaatcataaaaacatcatctggatacttggtggtgatcgcccggcggttaacgacagcggcgactggcgacccatctggcgggcaatggcaagaggtataaaggaaggcactgccgggcaatgcatcattgcttatcatccttccggaggagctaactccacgtcgcaatggctgcagcaggaaaactggctggatatcaacatgttccagagcggtcatggcagcggccatgatgtagcatgctgggagctggtacagagggaccggcaatctttaccggccaaacctacccttgacgccgaacctaattatgaagaccatcccgtgaatccctggcctaaatggaatcccgacaatggttatttcagggactacgatgtgcgtaagcaattgtaccgttctgtatttgccggcgcatgcggcgtcacctacggtcatcatgcggtgtggcaatttatgagtgcgcgggaggaagccgttaactatcctgatcggggctggatgaatgcactggaccggcccggtgctttccaggcgggttatcttcgcaggctcatagccatacatggcgcactaaaccgcgtaccggaccgcttcctgatcttgtcgggtcagggggaaggaggaggtcatatggaagctttccgggatgcggcgggtacttacctgatggtatatctgcccataggaaaatcgctgcaggtgaacactgctgtgataaaatccgcgcggttaaattgttggtggtttaatccgcggaatgcggaaagaacaagcatcggagttgtgaaacaaagctccgctgttacatttgtgcccccggctaccggcgtgggcgatgattgggtgttggtggtagaggcgcacccgtaacaaaaagccggttggcaaaagcatgctccaaccggtggtgttattacttttcattggctttcagcacttccacataatgaggattgtacataatgcccagtacgttgccgaaaggatcaattacggaggcggtaacaaatccatttccccgttctgtaacgggttctaaaacagtagcccccagttgcagcaatttttccaaccccgcctgtatatcgtctacatgccagtaaataatagcaccgccgggtccgctgcccagcgattttggcgcatacttactgtcgataatacccagttcatgctggtagtcgcccaggcggaactctgcatagccgggcctttcaaagtaaggaggaataccggttaactccgtataccatttttttgccgcctcgtgatctgctgcataaaagctcagcgtggcaaatcctcttaaaatgtttgtgttgctcatttggtttgttttaggatgaaatttttattgtctgatgtaaaagtagcaggcgggtatgacaaccctatgtcaacagcaaaaaagaaaggcagaatatttctgaatatagttataaattttaaatatctatttttatgtcctaatctgtatattatgaaaaaggtggcctatgaccctaatggtggaaaactgtggataaggatagatatgaccggcatttactttattacttacatctaccagatgtgggcggctaccgccgatgaacatcctatactaacaaagcccctccggcaaaacagcaatgagctgccccaaccggattactatcttattcaaaacgattataaacccggtgaaccattaatcaatttcgacaaaagagtactggatatttctttcagggtaagaaagtacgaggacgacaatggttataaattaagggtaagcgtattgcagggcgatgattttaatacagccaaagtaataggcagcagccagattggctatggcactactgctactttaggtaccgatgttaccggcaaacaggaagatattttactgcagttgatcgtaaaacaggattgattacccctatttaaaatacatgtatgtcagcacggaaaataattttcattctgttatctcttatttctttccggacatctgcgcagtttaaaacagacagtaccgagcattacctgttaaacttttctgtgccggatatgccggcgtttaaagcgctgggagcagatccttccaacctgctgcgtccttcggatattcaaaagtttgcgctcagcttatcgccattttattcaaacggccagggcgttatcccgcgtaatttcgccgtggaattttccccggggaaactggccagcaaaaactggacgctggaagattatggcaaaaggaagttctggtataactcctccttcagcatcggggcaatcgttgattcaggaaatgtatcctccaaactggctgtaggctaccggttttctattgtgagaaagaaagatgacctgttactgaatgccgcaaaaagaagggcggtttttctggcacaacagcaggcgcagctggcgctccgggaatttaaaaataactggatcattattgtgcataaagaagtgccacctgcagagcgcgcgcaatatggagccgagcatgacaaagaattctgggatttcgcggaaaacaaagcagaagaatatctcagggaaaacccagatacaaccttgcaggccagctacgacgcctttaaaaaaggatacgacaccgataaaaagaaatattatgcggcagtagatgacctgatagagcaatttaaaagcgaaaattggaacgctacccgcctggatggcgccattgcgtgggtagggcaatcccgcgattcattgattaaaaacgccggcttcacctccttcaatacctgggtcacctgggcactgggcatcgggaaaagcagccagctgctgctgggtggtagtttcagcttaccccgctctgaatttaaagacagtacattcgtcaacgcaacagtgaatgtccgctattacctggggacctccggtttcaggggatttgcggaaacacagtttaaatatcagaactatgataacctggacaaatccctgctgttcaattttggaactgaattcagggttgctaaaagtatatggattgtggccgaagcaggcattgataactacctgaaagagaaagaccctttcagtgcttttatagcgagcattaatttgcggtatggatttaaccaggtgatgaagtaggaggggaaatcaactaactccttcggggtgggattaagagaaggcttttatccctttactgtgcttgaatacactagacgcaaaaaaaccaccacaatcatttttcatcgaacattgattacattcttcgtgaaagatatttttccagtcggaaatagatttttttgagaactgccagatctcacggggtgtagtgcaaagttgtgagttataaagggaggtggtcataccaaaatccgataaataagtcatcgcttccgtaagttcttttccatattcaatcggatcaatccaaagtttatccaggttatacggcgtgtatccctgatgctccaatcccataaaggccacatgttctgcgaacggtagatttttataaataaacttcgccaatttaagaagccggggtaacgtctgtttatgtagaacaattcttaattctattctgacatttcttctggcaaggttatataacccttgaacggtctgatcaaatgcacctttggcttgtacaatataatcatgttgcgcatggtaatccgagtatattggtatgccaagcatgagtctcttaaaagacatatctccaagtttgtcggccatgttaggccatgcaaatgatctcccattggttaagcagtgtacttcggtatccggcagctgcgtttgtatttgtgccaggagcttaaaaaacttatcaccggagagggttggttcacctcccgtaatgcctaattccatgcaatctttcgggattaatggaattgtttgagtatggatattgtataagtaatctgtatcgtccttatcccggggaggctgagaacacattaaacagttgctgttgcatctttccgtaaacaataggaaattgtgtggggaatttattctatataaagtagaaatcacgccatccgtattgacgacgacgatatctccttcgcataagtgagaaacatcagggattgaatatacacttggtttatcaaataaactgactttttgattgcttgagaggattactttataatgttggagatgcattgggatgttctcatttgcaatcaaaacttccccctttgtgtcagagccaaaagttactctgcccactattggcgcattaatttcagatggaataccttttgtttttaatagcattagcttctacctgttatccagtttctgaatattttttctatttccttattatcatccattaactcaatcaaataccgcattatttccatatttctctggcaaaaagaacttgttggtctgtggccgtataaatcgccctgtgtagtgtgattgaaaacaggatcagctccacaataggtctggaaggcgcactcagaacaacctggcagtgattcattggtcattacatcactaagtgccagggctttttctccgtaaaagatttcttcgtatgtattttctcctaactgcccaagttggaatgtaaaatcattcatttccgcgagcattctggactcgtccgaggcatacactgccccatcataattaaacacaataacgctattaataagtccggcgggagattgaagatcgacatatccgacgggaaatggagttagcattttctttaaaatgatacttgcatagtcttctctgataaaatagccgtctatattatattgaataattctggtcagcgcttttttgtaaaattccaggaattttcctgtctcatatttattcttgtccttgcttctggtcgcaaaaccatatgggcttataggcctcaggaaaatgtttttaaatcctaatctgacatattcatccactatttcatgcggatattccaacgacagcttagtagtggtaactaatgctgaaatatgttctgcccctataatctgcctgcatttttcaatgccatcaactgcaagctgatggctgttggcatttggcttgtgtctgtttttgttgtgtataaatgcagggccatcaagcgaagtcgatattaaaattccgttttcatggcagtattgaagcatttcatctgtcagtggagcaagattagtgcagattacataagtaacctctttatgatgcttctctgcctcgacttttgttttttcaacagcatatattatgctttcaaaggctaataatgcctcaccaccttgaaactccattgtcacgtgtgggttaggtgatttcatcatcatagctataccagcgtcaatatgagggatactcatatcatatttgcttttatcggaagtaactcttgatacctggcagtagtgacaggtatgttcgcatctcaggctgattacaaaaatatgtagtgatgtaaaaaaatcaagaaatgacttttttgtacggtagcgggtcgcaagaacatcaatgagatttggaacggaattccccgaaataaagaaattggctgttaaatcggcgtatagctcctggtcctcactatttccggcttttatttcccgcgccacgatcctggctgttgtacctgcgggtactaccagaaagtccccaatttcatttacaatcacttcttttttattggaaatacggtggaatctgaatggaagtaaagtatattctggtattgacgtggtataagcttcaaattctttaaatttcctgcttacccttgttgttaccggtgttgatttcatggttgtatggattgggggctgaagcctacggggtcacttatctccgacatgggtattgtctcattttcataatatgcgaaagctttagcgataataagctccctgatcgtttttgtttcatctgttatacactgccgtagcttgaaatctatgagatcctgctttagttttactattatggttttccagtcaacaggttccgcgttatagagaggagttagtattattttatactggagaggatctgtctttataatatctacttcaaaggcattagtataccagtagagacatttaaacaaaacaacttcagggtatagctcggtagcaaccgtaaaagagagcgtgttattatcttgtagaaatttcattcgctttatttcttagtacattaagtgttttagcgtctactttaccatcaggccttaattcattttcttgctgaaaatgaataataattgcttctgtttgtagtccaaaatatccggttataaacatgtctttttttaaggtcattaatatcctttgcagcacttctacatcctttccttcgcatcctttgaatagtacccgatctcccaattttagactggaggaatctgctacatgtacagcatctgtagttctgtttgaaggtgaaatacgtgccgcacccgggttatagaaaggagtcgcaccagaactttttccggtagagtttgttccgggagtacttttcacagtacctcctgaggttgaatgccctgaagaggaggacgacgcaggaacatatacaggtgtaggggatggcgtatagctactgccagagctataagacgaggaataatgcgaactgtgagagctatgcgaggaatgagaacggtgtgagctatgcgaactatgcatggaaacaaggctattcgatggatccattatattgagtttcagcactagtttaggtttcaatacatttttatgcgtgttctcaacagggatgtttttatcattttcaatttcgtggttagtgttattgggaacctcggctttggtgtgggaaaatacacttaacgcggctgttaccacagcaaggcttttcttagccagattttggaagccaaatttattgttgatcattaggatgttttttgtggtctaattatctggaattatagggatgttagatataggttcaaacacgcagaatggtcaaattttttgaggataagctttaaagcagaatactaaggtatataaatttgttcaaattggctaattggattatttattgtgttttaatatatgattgcttggctcactatttacttctccgcttattcctcttcaccagtaaaaagcatccatacaaaaacaccacccatgctgggatcagttctaccggcagtttcatccctgttatccacatcaggatcaggatgcccaccaggaacaccaggcaaatgtaattggacaccgggtaaataaaggaaggaaattttgtcaggatctgcgcttcccgtttgctctttttgaatttaagatgcactacggtgatcatcagccagttaatgatcaatgaagataccaccagcgacatcagtacttccagcgctttttcagggatcaccttatttaccacaatacaaatagcagcaaataaaccggataccaggattgcttttacaggtacatggtttttatttagctgagataagaaagcgggtgcattgccttgcttcgacaagccatacaacattctgctgttactgtatacgcaactgttgtaaacggaaagtgccgctgttaaaacaatcagatttaacacatttgcaatcaggctggtgaaatagatggttttacccaaaaaggaaaaccggaatccttttaagctttgaaataccattacaaacgggctgctgtctgtagtaatacttttccatggcgataaagaaaacaggatcacaagtgcgccaacataaaagatcaggatacggtaaatcacctggttggtagccttggggattgttttttccggctggtctgcttctgcagcagtgataccaatcagttcaagcccaccaaaggaaaacatgatcagggcaatggctgcaaacaatccctggaaaccacctttaccatcggcatgcaataatccacgcgggaaaaatccgccatcgttccagagattccggatgctggcctgtgagccgccacttccgcttatcagcaaataaattccaaaaacgatcatggcaatgatagccactacttttatgatggaaaaccaaaactctgcttctccgtatacttttacagagctcaggtttaacgcattaatagcaatgaagaaaaaaagactggaagaccataacgggatctccggccaccagaaatgtacatacacgccaatagcagtcagctccgacatgctcaccaggatataaaggatccagtaattccacccggaagaaaagccggcaaatgagccccagtatttataggcaaaatgactaaaactacctgataccggttcttccactaccatttcgcccagctggcgcataataaagaaagcaataataccggccagggcatagcccaaaataacagaaggccccgccagcaccgccgccgggcctatgcccaggaataaacctgttccgatggcgccgcccaacgcaatcagctggatatgcctgttctgtaatccccttttaaggtttttttcgtttgctgagtccaatgtttatagtgctggataaggctgcaagttgaggtaatttcggcaaaattgaaactttgatttatttgctccgcagatgcctgtttcagcagtacggatcatactttgagtgttctgtctgatataacaggtacaatggggtagatgtactccatgggttttacgtcaggcttttccggcgacgaactttgtgttcgagtaagattccccatggcacagttatcgataccaaatctgctgaaaaacaaacccgcagatcatgctacctcatcaaaacccaataatccggcataaattcactgccgatcccaccgcactggtccacaatgatactatatacctgtacaccggccacgacgaagcgccggtaggcacggaagcctatgtaatgaatgagtggctctgcttctcatccaacaacctcacggaatggacggaacatcctgtaccattaaaagcaaccgatttttcatggggcagcggcaacgcttacgcctcaaaagtaatagcgcacaataataaattttattggtatgtagccaccgcccacgctactattaagggatcagccattggtgtggcagaggccacacatccggagggtccgtttaaagatgcccgcggatcagcgctggttacccttgatatgctgccagcgggtgtgcacgaaaaagccaatctcgatccaacggtgatgatagacgacaacgggcaggcatatattttctggggtaatgggaaatgcttttatgcaaagctgaaatccaatctcacggaactggatggaccgattaaaacactggacctgccaggatttgaggaaggcgcgcacctgcataaacgcaatggctggtactacctgtcctatggttacgggatgccggaaagagtggcttatgccatgagccgcagcatggaagggccgtgggaatttaaggggatattaaatgagctggcaggaaattgcgaaactaacagacctgcgatattggattttaacggcaggtcttattttatttatcacaacgggggactgaaaaacgggggcagccaccggcgctcagtgtgcatcgactacctctactacaatccggatgataccatgaagcgggtggtgatgacctccgaaggcgtacagatggcatattaaatgcaatgcctgttattatgaaaacaatatgcaccttactcatcatcaacttattcgtcatggctacagctactgcgcaggataccgcccgctatatcaaaaccagtaccggctacctcatggtattaaggcagggagatgatatttttaagcaactggaggcctttgcagaaaaggaaaagattccctccgccagtttcaccggcttcggatttgtgaacgccacctttgggtattttaacagggaaacgaaaaagtacgagcccaaagaattcagtaatatggaactgtccggcctgaacgggtctattgcgtggcagaaagggaaagtgtcactgcatacgcatggcacggttacggataaagattttaacgccttcggcggacatatgttaggtggcaccgttggcaccggatcgctggagatcactgttatagtgcatccgcagcaactggaacgcgtgtttgaagaaccactgggcgccaacgtgctgagcctggaaaagaaataatcaactatagtgaaatgctgcttttaccagagcttcattgctttctgcaatagcgccggatgggtcgagtaaggtatcttcaaatcctattctcaggtcgtaacctttatacttggctactttcaggagttcccagcaggtactgtcgaaaccatgcaataccaccgtttgatgtggctgcctgccggtcaggttgtcttcaatggccttcaccgttgccagcgctgcgttgaggtcctgctcctgtggttcaattaacaggcggaaacattcgttcaataatccgctgccgctgaaatccgctgctgcctgcgcggaattaagtcccgcttccaccccgatcttcttgtccagtatggcctgtacaatacgttcaaaaccggcttcatgcccattcacagatacaaagttgggtagttcttcccactcactgatataggcgagccgctgatcgatatccggtaccatccaggcgccggtactgatgcccacaggaatttcgggcacggcggcctttactgcttttacctgttcatttacaaagagtggctccagggtttctttaccgttgcggtcacgtacatggaaatggatggcatcagcgccggcgagaacggcgcttttagcggcttccaccaattcatctgtcgtaaccggaacattcggatggtctgctttggacctggaaccatttaatgctgcttttataaacatacttcctggcttttttcaggtcactgcataaatgatacctgtatcgtaatcatcagcttttccggcattaacggccaaaagcatgggatgctgtgttgtggaacaggttgagcagattgcaggattttttccctgaagtgggtattgggctgtggcagggttcgtcctctttcgtcattatttttaacctgccggttgcgtttttttattatagctttagccggaaaaaagcctccaatgaccgggaatattctgatacaatcgctgaaagatattacagaccaggagattagcattaacaagtttatcggaacgcagaataaggaggatttttacaagaaagccccacaccgccgggatgaccattacctgtttatctttcaaaaaaaaggcagaagtacggtcatgatagattttaaggaagtagcgttaatcgaaagcgcggtattatgtgtactgccaggacaaattcattatggcgttacggcaaacagtgacaccgaagcctggctgattacgttggatactaattttgtagaagaagattaccggagaatttttgatgattactattttcagaatgcacccatcaccatatccgctttagaaagtattccgctggatgatagcattgaattgctggcatccatagtgcgcaaccgccatccgttggattttatgccacaggtaatacattcgttgatcagcgcttgtgttgggatgttcgcttctgcctatcgccggcaggaaaatagggaggtccctttatcacgcacacatcttttaacacagcaatttaaacggttgcttttgcaacagtttaaaacacataaaactacttccgcttacgctacctcattaaatataacccctgcatacctgaatgatgccgtaaaacaaacaacaggacttaccgtaagtttctggatacaacaaactatcatcatggaagcaaaaagactattgtacgctaccaatgcatccgttaaagaaatagccagccagttggggtttactgaccatgcttactttacccgctatttttcccatgcagaagggcagtcgccattgcaattccggcgcaattgccgcaaataatccaatggttccctttatctatccattttacccgggtgcagctgtcgctaactttgcaggaaaataacagatgggtaatcatatcatttttacggttggaataatatgcctcttatggcttttatataggacgataaaattcatttatccttatatccgtcgctcggatcttgaaaaatacaggaagccgggcgcctttgcgctggtcaccggcgcaaccgacgggatcgggaaagccattgccgtggcactggcagggaaaggctttaatatcgttttacatggccggaacgaagcaaaattacaggcggtgaaaatggacatcgaaagggatcacccgcagtgcaaggtagtgttgctgttacatgatggtagcagggaaagccgggtaaatgtggaagaaattgagcatttgcccataacagtactggtgaataatgtaggaataggaccgatgaatgcactggctgatttttccgccggggaaattgatgaaacaattacgctcaacatggccttcccttcacagctaacccgtagcttgctgccacaactgggaaaacccgggcttatattaaatgtttcttcgtatgcgggcttgtttccaccaccttatttagcggtttatgcaggctcaaaggcatataacaatgccttttccatttcgctggcgcgtgaattagaaaatgtggaagtgatttcattgataaccggtagtgtaaacaccgggacaaataaaaagcccgtcacctttatgcggccggccgcggccacctatgcaaagcacgtgctggccattgtgggttgtggcagaaaaagtattatgccttattggcctcatgccatacaaacttttctgatatcgctgctgcctgaaaagctcatcgacagcgcaactaagaacgccatgcagcgggaactgcaacatcctgaacgttaatatagccggaagggattcactaaatcccctccggctatatcttcttaaaaaataattacttcgctgctacaacaggtttttcaaatccgtctttcttcgctttctccgccatcgtattcattcttttttctgtatcagggtgggaagagaataattgtgagcctttctttttatcaccgctgctttcctgtgatgccttccacaatttttcgaaagccatagacatgccccagggattgagcttggccgctttcagaaattcgtaaccgtagttatcagcctggctttcctggttgcgggaataggcagaattagcaaccgcttctcccaactcgccgagctgtgaatcgctcagggtgccggcagcgccgccctgtgaagaaacaccgtctttcagcgcggaggtcatcagcgctgttttgaacgcatctttggaatccttgttttttacatgcccgatttcatggcctattacgcccattacttcgtcgtctgtcatggtttgtaataacccggcgcatacacgcacactgccatctgcacaggcaaaggcgttgatatcccttaccaggtacactttgaagttaagattcatgccttcgtagccggtaacatggtcggttagctttttcaggcgctgggccatcggatcatctgagggtgcaacggggttgtgctcatccatccactggatatactctttggtatacctgatcacatcgtcatctgtgagggtggctgctttcactgctttggcgccggcgcccagtgtttttgtgtttaatttcaattgagcatttgaggctaacgcaaatgacatcgtcaaagcgcatacgaaaccgaatcgtgcgtaaacagacataataaaggtttttattgttgaaaagggttaaatactaatgattgcattcaaggctacggcgcgaagataaatattgttatgatctcttacaaacaattttagccccgtaaaaggagtgtttttaaaatatattaatatcagggagacgaggtaagtgtatggtgagtgcatgaggagtccatgagaagtgcatgaagagtgcatggatagtccatgacatacgcagggctgaggcattgatgaagcatcagggaaataaccgggatattggaccccaatacatccgaatcgataataacattaaccggatctgatcttcacttatctttgccctcacttaattgatcttttgaaatttttaagatgataaacatatatcgtaaaacagcgttaatcgaagcagtatcttacctgatattattgtttgtggccatgcccatgaaatacattttctctgttcctgaaccggtaaagtacttcgggtggctgcatggcgtattatttatcctgtttattgtactcctgctttcctgctggattaagtacaggtggagtatcatgagggtggccggcttcttcgtgggatcgctcctgccgtttgtgccgtttatatttgaaaagaagctgaaggaagaatacggcgcctgaggaggcccggttccagtggctccaaaccggcataatcatctttacccggtaaaatttaaaaataatgggtaagaaagtaaagtcaattcctgtaaatccatttgctcctgcattggaccccggagttgtcgtgggaaagatatcgtccggcagtttgctgtcctaccaggcggcccacaggccgcacaggcatgatggccattttttcctgttggtggaaaaaggaacggcgcatatcgaaattgacctggaaaagtatcatatcaagacatctcatgtgttgtatgtccatcctaaccaggtgcaccgggttgtaaaatccgggaaaacagacctttacctgctggggatcactaacgaaaacctgacttcccagaacctggagttgctggagcaaattgttcctgcacaacctttgccactaaccaaaagtagcttttcaattgtaagccaggcaataaggctatgtataaatatttttgaaagaaaacaggataagttatacccatctttgcttaaaggcgcctgcaatacactggtagccctgattatttcgcaatacctggagcaatcggcttcaaccggcaaactttcacgcttcgatactattacaaaagcatttaagttattactggagcgcgatttcgccggggtcaaacggccttccgattatgcgaccgcattaaatatttccaccccttacctgaatgaatgtgtccggaatgccaccggctttcccgtttcataccatatccagcaacgcgttatactggaggcaaaacgcctgatttgccattccggcaagtctgttaaagaaattgccaccgaactggggtacaacgactatgcctacttttcacgattttttacaaaagtaacgggaatgacggcgatagctttccggaaaaaaaacctcgaatagtccaacaactacgcttgtattgccattgttgccggcagaaatatagccttgctttgcaggttataataaactgtgtaaaatgccaagaacagcaaaatggttaggcgacgcaatggaaggcttgctgggatccaggtttccattaatgaaagtgatggaaacaaattatatcaatccgaacataaaaaagatacggtttaaagggaatctttcagggatgaatttccagttaggctatgccgttataatcagggtaagtgatacggaatacagaaattactcggtatcattcagcgatgttgaaaatggtatcctggaaatcatttttcacctgcacggtgctgcaccaggatgtctttttatggatcgcctaaccgctggtgaccaggtaagggtcagcatgccaagagggcaaaagcaatatgatccggcagtggaaaagcagttgttgtttggcgatgaaacatcgttgggcctggcggtgtcttttcaaccttacctgaaaaagaacaatcacgagtttcagttttattttgaactggatgaagcaaacgaacaggtaccccggctgttggggttggagaactacacagtatttcctaaaaacaatcacttcaggaatgagcagtggataaacgacctggcggtttttaacgctggcgattggctcacggctaactacattcttaccggaaatgtaaaatcagttcaaacctttagaagagtgttgaaaaataacaatatcagcggcagaatatttacggctggtttctggctggaagggaaaacgggtttgtaatgccagtacatttactaccgggaggctgtttcccgctgctacattaaaaatgttttcttaaaaaaataagtactaaatggcggtaactgttccattgcgtgtctactctaaaagccgttaccacgcaatgcagctaccacgtataaaaaacacacgccggtttttcaccggtttactttgcagtttctccctcgccaccacagcgcagcaaaaagaattggtggcctacgccaatactttacagggcaccaattcggagttctcgctcagtaatggcaacacccatccttccacggcgctgccttttggtatgcatgcctggtctgcccaaacaggcaaaaacggcgacggctggaagtaccagtacaaagccactaccatccgcggcttccagcaaacgcaccagtgcagcccctgggtgggcgattacgccgtattcagcctgatgccggtaacaggtaaactggcagtaggagaagaggagcgcgctacagctttcagtcatgtggatgaagtagcccgccccgactactacaaggtaactttcgccaataacatcaccacggaattatcacctactgaaagaggcgcacacctgcgtttttctttccccgcgaagaaacccgcctatattgtactggatggctataatgccctgagtggcgtgcaaatatttccggcagaaagaaaaattacgggatacgtcaccaacgggcgctttatccccaaaggcttccgtaactattttgtgatcgtgttcgaccagcctttcgaagccagcggcacctgggaaaataccaacaaccggatctttgccgatacgttgtcggccgaagggaaaggcgtaggcgcatttgttcgctttaagaatggtgcggtggtacaggccagggtcgcttcttcctatatcagcgccgcacaggcggaactcacctggcaacaggaactcaaacccttcaccaggctggaacaaacaaaagcggcggccgccaaaatatggaacacgctctttgccagggtacgggtggaaggcggaacggaaaaagacaaagccactttttattcctgccttttccgcgccaatcttttttcacataccttttttgaatacaacagcaaaggagcaccttattatttcagtccgtacgatggaaagatacataacgggtatatgtacaccgacaacggcttctgggatacctttcgcgcgcagttcccgctaaacaccatcctgcaccccaccatggaaggccgctacatgcaggcgctgctggatgcgcagcaacaatgcggctggctccctgcctggtcgttccccggcgaaacaggcggcatgctcggcaatcacgccatctctctgctggcagacgcatgggtgaaagggatccgcaccttcgatcccaaacaagcgctggacgcctattatcatgaagccatgaacaaaggcccctggggcggcgccaacggccgcgccggttggaaagaatactatcagctgggatatgtcagcttccccgaatcacagggcagcacctcgcaaacattggaatatgcatacgacgatttctgcggctatcaactagccaagctgactggcaacaatttttatcagtacgtttttggccgcaccatgtataattataaaaatcagtacgacagcctctccgggtttatgcgcggccgtaaactggatggcaactggcaggaaaactttgatccgtatgaatggggtggtccctacacagaagggaatgcctggcactggcaatggtccgtatttcatgatgtacaaggcctgattaacctgatgggaggaaatacgcccttcatcacaaaactggactccgttttcagcgcccccaataaagtgaacgtgggcgcttacaaacaaacgatccacgaaatgacggaaatggtaaacgccaacatgggccagtatgcacacggtaatcagccggtgcaacatatgatctatctctataactatgccggccagccctggaaaacacaggcgcatgtgcggaaagtaatggaccaactttacaatgcaggagaaaacgggtatcccggggatgaagaccaggggcagatgtcctcctggtacgtaatgagcgctatgggcttttacagcgtgtgcccaggcacggatcaatacgtgatcggaagtccgctgttcccgaaagtgacaataacacttgaaaacgggaagcagtttgtggtgcaagcccataacaacagcccggagaatgtatatatccagtcggcggttctcaacggtaaaccgtggccgcacaactggctccggcatgcagatatcgttaatggcggtgtgctgctgctggaaatgggtaataaaccggctgtcaaccggggcattgccgatgccgacaaacctttctcgctgagcagccggtgaaaatacggctgccgatattttcgtaccgacatgaagaatttcgtactgaaacgattaaattagcccgtagttcgaattcatgtcgatgcgaaaagatttttccacgtatacagatgaagagttgttcctgtttgtaaaacagggacacaaggaagcgtttgaggatgtgtacaggcgcttctggcaggagttactggatgccgcctaccggcgtgtaaaagtacaggaagcggccatggagctggtgcaaagcctgctggtagacctctacctgaaaagggaaaccatttctcttaacacatcgctccgcaattacctgcatacatcactgaaaaaccggatactgaataccatccgttcacaattggtgcgcaacacctatcagcagcatgtactgaatgatagcggtctttatcagtcagacgccgccagcacgctgcaattaaaagaactgcagcggcatatagatgaatcctgcgccagcatgcccgaaaaatgcagggaagtattttacctgagcaggagagagcagttgtcgtaccagcacatcgcccggcaaatgaatatttcggtgaacaccgtagagaaacatatggtgaaagccctgaaaatattacgcgctcacctgaaacaatatcattacatcctgttctggtgcctggtatcgctgttgctgctgtggagtgcaaatgtcaaactattttgaatcgtgatggcggtaagccatttttcaggtgtctaatgttagagagactatggatatgaacaacacccggttaaaagaattattggataaatacctggacggtacagccactgatgttgaaatcagtgaggtggacaattggtacaggtctttcgaaaatgatccggccttcactgcgcaattcagcccggagcaacgcaccgcgctggagcagctgatcttcctgcgcatcagccgccaggtggaagctgcggagccacgggttagctaccggtctgttcgttggtgggccgcagccgccgcggtggctttgctcattaccgcaggcgccttcttcctgacccggaaacaaccggttcagcagggaatgcccattgcaagtgtgacagcacaaaccggtaaaaaaggcatcaagaaggtcagcctgccggatagcagcattgtatggctgaatatagatagtaaactccggtatgaagaaacaaaaggccgggagatctggctggaaggggaaggctactttgaagtagcgcccaaacaaggcgctcccttcctggtgcatgcgggcacgcttcatatcaatgtacttggtaccagctttaacatcgacgcctacacgccggatgcaaaagtaacggtaacagtagccagcggaaaggtcgccattggaaacagtcagcgcaaccatgccacgctgggggccaatcagcaggtcatataccatgctgcggaagatcagctggaaacaagcaacatcgctgcggcagacgtcagcgcctggacacagggtcagctgatatttaagaaagcgctgttccgcgatattgcacaaaaactggaacgccgttacgacgtacgtatccggtttgccagcgaacaaattgccagctcattgctcaccgcccggttcgatgccaacgtaccgtttaaaaacgtactgggcatgttgtgtgatatttatgggtttagctaccggcaaacgccgggcaaaaacgaatacctggtttacaaaaaaagtcaaccaactaaataatccggaaggatcagccatgtggcgtgataatttcaagttatgaaagtgaaaacagcggagtgcgtgcacatgacgcccaggtggcttgcctgcctggtgctggcattgtgttgcctgtacccgccgcggatgatggcccaatccggaacaacaacagagctgaaacaaaccacggtagatatacatgttgtgaatgaaacactcgataaagtgtttgaacaggtggaagcctccaccacattccggtttgtatataacccgtcggaaattgcaaaaagtggaaaagtaacgatcaataaaaagaatattccggtggaacaggtgctgaaattattgccatccgtattgcaatatgaactgcgtggaaggaacctcctcatcacccggaaggaagcgccgccactgaaccaggcttcggtattaacaggaaaggtgacggataccaacggcaaccccttgccgggtgtatatgtcataaagaaaggttcgccgccacgtatcgtaacagagccggatggctccttcagcatacatgccgatccgggggataccctgcgcttcagccttcccggcttcggcgaacaggaagttcccgtggaacgcgccaatatgctctatgtttccatgctggcgaaatattcatcactcaaagaagtagtggtgatcggttacggcacttccagcaaggagaaacttaccacagcggtaggcaccgtgagcggcgatgtattaaaggaacgtgctaccaccatgaacctcatgcagggactggcagggaaagtagccggtgtcagcgtgatgatgaactccgggaaacccggcggtaatcctatcgtaaaaatcaggggcaccggttccatcaacgcgtacaacggtccgctgtatgtggtagacggcattgtgggcgcagatcccctgatccttgatccgaatattgtggcttcggtggatgtgctcaaagatgcggctgcctccgccatttacggtgcaagaggatctaacggcgtgatcgtgatcaccacccggaaaggcacaaaaagcagcccggctatttcattccgcaacaccctcagctttggctcactggcccgcaaagtacagctgatgaatgcagaagaagcactggagatgtttaagcgggagtatgaatacctgcctggccgcaccgcgccgcatctcgatcctacccgccagtttccgcggaaggatgaactttttaatgcagacggttcgcctaaatatcatacagactggcaggaggaagcaagccgcctggcagtgtcccacgaacattcattgtcactgtctgccggaaaggatggcttctccgccctggtcaacctgtcttacaacgaccagcagggaatcctgatcaacagctactcccggcagatcaatggctttatcaacctcggctgggacgtcacaaaatggttgcacgtacaggcggtcatcaacagcggggcagccaaacagaataatgtcgacatcaatacattcggattaaatgccgtacgccagatatatgaatttctgcccttcctgccggtacgctatgcagatggcacgtattcgcgcaaaggagattatcctggtgcagaggattctgaaaacccggtgagacttatgcaggaagtaaagtcggtggccggccgcacgtatacgatgggcaacctgattaccaccattcggctgaacagcaaactgcatatcacagcgggtttgagcggacaaacaggcgccacctacaacctgtattattccggccgggatatccgcggatattcggatacgcaacagggagtagccacacgggcaaatggtaattccggctcctggacttcggaagattacctgacctggaacaaccagtttggcaaacataaagttactgccgtggcaggcgccagctggtactatttcgggaacatgaacacgcaggcaggaagcgaaggcttcttcgatgatttcttttcgtataacagcctgcaaacaggactggtaccgcaacggccgcagtcgggaacaagcaatacagcaatgaactcgtattatatgcggttcaactacgactacgacagccgttacctgctgggattttctttccgtgcagatggatcttcgcgcttcggagccaataatgtgtatggatacttcccaagtttctcgggcgcgtggcggttgtcgtcggaacctttcctccgggatgtgcgcagcattaacgacctgaagatacgtggcagctacggcatcgtaggcaatgcggatatcggcgattatgtaacgcaggacaggctgcggagcggccaggtggcattcaatggccaggcggcgcccgcagttatgctggaagcattgggtaacaaaaatcttaaatgggaaaaagcccatcagctgaatatcggggtcgatgtttcactgctggacaacaggatacaatttaccggcgacgtttataaccgcgtaacaaaagatctgctgtattaccggctgatgccggctaccaccggctatgagggcgtgtttgacaatatcggttctatccgcaacaggggtgttgaactgtcgcttgttaccaacaacatccggcgcaaacaattctcctggaacacttccctgatctattccatgaaccgctccctcgtactggaactgaatggcgatatcatgtatccctggggtggccgcatcatggaaggacggccgttgaatgaattttatggctaccgccgcctgggtacctggggtacagaggaagcaacggaagctgctgcctatggcaaaaagcctggcgatctgaaatacgcagacgggaataataataaagtgaaagatgccaacgaccggacggtacttggtaacggtatgcccgattttgaagcaagcctgagtaacacgtttacctataaaaatttttcgctgttggtagatgtgcaaacgatctatggccacagcctggcaaactttaccaggatgctcatggaaaacgcagcacccaccatcaacagctaccgcagcctgctcaatgcctggacgccggaacaacagggcggcatgaacccggcgctgcggctgccgcaggatggactcgataatgagatggatagttattacatagaaaaaggaacattcctgcgcattcgtaatatcgcactggcctataggctaaaggaagactggctcgcacggtatcatataaagtcagctgccatcagcgtcagcgcagaaaactatttcctgttcacaaagtataaaggatatgatccggaagcatcttcattcgatggcgactttaaccagggagtggatatgtatcaatacccgaaagcaaaaacgctggcgttcacattaaatgttacattctgaataaaggaattgaaatatgaaacaactggtgctgttggggatgatcatattgattacttcctgcaacaaattcctggaagaggaaccctcgggttctctcagcctcacacactactacaaaacacctgaacaggtgagcgctgcggtaaacggtacctacgacggcctcgctactcccttcgtggctaatataggcgtagccgttagcccggtgtattcactggaatatatcacagggtatagccgccggccacggccatcaggttttgaagatgaccagttcctgcggttagaccggctcgataatgcaaactcaaaattacagggatggtggaacgctacttattacccggtggaaaactgcaacagcgtgattgaaaacgtaagcgtaacactggtggtagatgaattaaccaagcagcgttacctcggtgaagcgcatttcctgcgggcatggtattacttccaggcagtacggctttttggcgacattcccctgaaactcaccaccacaaaagatattaatgatgtaagaatccgccgctcgccgaaagcagccgtgtatgaacagattgtgaaggaccttaccgtagcagaaaatgccggtctaccctggacggatcagagcgggcatgtaagcctgggcgccgtaaaatctttgctggcaaaagtatacatcaccatggccggttatccgttgcagaaaggaatgccttattaccagaaggcctatgacaaggcgatggaagtaatcgacagccaccagttttccctgtttgagcaatacagcgatctgcgtaaccccgcggtgcaaaatacccgggagcatatttttatgctgcagcgccatcctacggtggcggtgagcaacattcactgggcctatcttccatatcccggtcagccggtttctatacaacccgcctatggtggggccatggcgccagcgcccgcgttttatgattcgtatgcagcagacgacggacgtaaacaggaaaaggctttcttctatacgaaatacccgcgttatggcaacccggccgaaaccatctttttctccgaaccttatatcttcaaattctgggatgaggaagcagaaaaaaccggccgctcaggggctaactttcccctgatacgttacgcggatattttgcttttatgtgcagaagcaaaaagtgtaatcgacggtggcactacatccgatgcagcggctatcgacgcctggtattcggtacgccaccgggcattcccggcagcgcctaagcctgctgctttaacaacagatgatattctcagggaaagatattgggaactgtgttttgaattccagacctggtacgatatgttgcgcacccgcaaagcctttgatgtggcgcgcggccgtatgaccaacctcgtcggatacaaagcacccaaccacctgcggagcttcgaagaaactgattttcaatttccattaccattagctgaagttcagaaaaacccggacttggccctttaacaacagcatgaaacgaatgactatttgcctggcggttttactcaccgctgcggcacaggaatcttttgcccagcagccttattttattgatggctatcatggcggcgtttacgggcactatcccgtaggatacacccggtttataaacagccagctgcaggcaaaccctaactggaaaattaacctggaaatagaaccggaaacctgggatatggtgaagacccgtgaaccggaagcatatacggttttccaacaattatttgccgatcaatccaacaacggccgcatagaatatgtgaacccggcatatggtcagagttatctctacaccagctccggtgaaagtatgatccgccagttcagctatggcatacaaaaagtaagggaacattttcccggcgcccggttcactacttattcaagtgaagaaccctgctttaccagcgccctgccacaggtactccgctcgttcggatttaaatatgcatccctgaaaaatccgaatacctgctggggaggctacacccgcgcatttggcggagagttggttaactggcagggccccgatggcagccggctgctaaccgtgccgcgatatagttcggaagccttattacccaattctacctggcaaactactgcctggaacaacagcaaagaatatttagcatccgcacgggccgccggcatcgccaatcccgtgggcatgtgcctgcaggatgccggctggcgcaacggcccctggctgaaagataatgcacagtatgaaacgtggcggaattatatcggcagcgtggccggcaaaacaaatgtgccctcatggcgctttagccaggaagacatccaggtaagcctggtatggggtgcgcaggtattacagcgtattgcacagcaggtgagagcagcagaaaataaactgataacagcagaaaaatatgccgccattgccacgctatatgatcatgttgcatggccgcagcaacaactggataccgcctggaaatcactgctgctggcccagcatcacgactgctggatcgtgccttacaatggcagcaaaggtgatacctggatcgataaggtacaacactggacagataacaccatcgccgtaagtgacagtatcttgcaacaaaataataacggcgctgcttttatacgcgtgttgaataccacggcacgccgccgcgaagaatggattgatttaccgggtggcaattggaaagtaacagacagtaaaggaagacaggtgcaaacagcgcagggagctgttaaagtttccgtgccgccaatgggattcagcgtttacaggttgcagcaaataacaggtacagaaaaagatacccgtccggaaacaggacgctatctgctggaaacagacttataccgcgtagaaatagaccccgccaaaggcggcgttatcaccagcctggtagttaaagccaccggcaaagaaatggtagacacaaaaagcaatcgcgggttcaatgaactcaggggatacttttaccaggaaggcgcctggcgctccagcatggatacggcagcggttatccgcattactgaaaataacaaagcccgcatgtcggcggaaatcaacggttttattgccggtcacccatttacacaacagcttacacttaccaacggtcagcgaagaatagatatgaaagtaaccataaactggaagggcaatcccggcataggcgcttattctcaggctaacaactatagtacggaagcatatcacaaagcattttataacgatagctgcaaactgcaggtactgttcccgcttgcgctctcttcacaaaaactcagtaaagatgcaccgtttgatgtaacggacagccggctggaaaatactttcttcagcagctgggatagcattaaaaataatgtcatcctccactgggcggatgtaaccgatggcaacgcaggactggccctgtttaccgatcatactaccagttatgtgcatggaaaggattatccgctgggtcttacgttgcaatatgcgggcagggcgctctggggacgtaattatgatattaccggccctacagaagtgaattatgccatcgttccgcataaaggcaattgggaaacgggcgccatccccaatgaggaagcacgctggtgcgaaccattgcaggtattgcctgccaccggtggaaaagatttttccctgctggcagtagcggatgatcattggcaggtatccgccctgcagattgatggaaaagatttgcttatcaggttgtacaatgcgggtggaaataacggtcagcagcaactgtctttcaacggtaaagcggcgcaggctgttatagaacaactggatggacaggcagtggaaaccctgcaacaacggcaggctgcgggcaaaacaatcatccgcctggcgataccacgtttcggtatccgcaccatccggctgaaaaatgtaattgtaaataactaaaccacaatatgaaaaagttcgtgtattccatcgggttatgcctcgccaccttgttcacgcaggcacaggtaaaaccctttcaacaaaatgaccgcgtgatttttgtaggcaacagtatcaccgaagcaggagcctatgtctcgtatatttatctctactacatgacccatttccccggcaaaaaactggtgatcctcaacggtggcattggcggcgacaaagcatcggatatataccgccgcctggattatgatatcctggctaaaaagcccacggtactggtgctcacattcggtatgaacgacaccggctactttgaatttaacagcagcgatgctgctaaaaccgccgctgaacggattgacgcgtcccgcagcagttatcagcaaatagaacaacggctgctcaaactgccggctatacaaaaagtaatgatgtcgtcgccgccatacgatgaaaccgcgaagataccagggaattattttcccggtaaacaacaggccatgctggaaataataaagttccaggagcaagcggcacagaaaaataactggccttttacagacctgttccggcctatgaaagcgctgaatgaacaactgcagcaaaaggattccacttttaccatgattggccccgacaggatccatcccggtaatgcaggacacctggtaatggcttccctcttcctgaaaagccagggactgaacggcaaacctgtggcagcagtaaggattaacgcgagcgctggtaaattgcaacaggcggtgaattgtaatatcagccagctgacagcttccggtaataaagtaagtttcggctacctggccgcatcactgccctttcccatagatacggtgtcccgcatatggggcaataaccagaaacaatctgatgcattgaactggattccttttacagaagattttaaccgggaaatgttacaggtagatggattgtcgtcaggagattatacactgctgatagacggttacgctatgggcaaatggtccgctaccgcattcgccgaaggcatcaaccttgccacgctgccggaaacgccgcaacacaaacaggcgtattccattatgcagctcaatctccgccgtgcagagctggaaggccatttgcgcagttactactgggtacagggtaacttttttgataaaaagcatttattattgcacgataacgccgcagcactggacagtgtgcgcaccgccgcaaaaacagatggtatgctgcgcttccacgaaggaaattatgaaacagccatgtacaaagaactgcgtacggcctggctgaatgagatcgataccatcgttaaactgatttataccatcaacaaaccggtgcttcataaaattgagatcgttaaaatttaaagatgaaaatcactgcttctatattcgtttccgcactctttctggttgcaacggttggtaaggcccaggggcccgctgcttacgtaaatcctttcatcggcgccagtaccagtgaagatgccgccggcagttaccacggcctcggcaaaacttttcccggtgcagccacgcctttcggcatggtgcagctcagccccaataccattaccggtggcgacaacggctcaggatacagttatgaacataccaccatagaaggctttgcctttacgcaaatgagcggcatcggctggtatggagatcttggcaacttcctcgtgatgcccgccaccggccccctgcaaactgccgccggcagccggcaacatccggaagaagggtatcgttctacctactcaaaaaaagaagaaaaggctaccgcagggtactactccgttctgctcacagaaaataatatcaaagcggaaatgaccgccgctccgcacagcggcatcatgcgctttacatttcccgccaatcagcaatcacgcctacaaatcgacctggcccgccgggtaggcggtacctccacctggcaggaagtgaaagtgatcaacgacagcaccatcgcagggtacatgcagtgcacaccggaaggcggcggctggggaaacggcgatggtaaaggtaattacacagtatacttttacgcacaattcagtaaaccactttcaaaatacggcgtctggagtgcagacatccccgacggatggtcgcgtaaacgggaagacattgaaagcgcccgctaccagcaacagatcgcaaaagcaacggtgatacccggcactaaagagaaagcaggtaaacatctcggcttctatacagaatttgctacaacagaaaaggaagctgtattgatgaaagcaggcatttccttcgttagcatcgatggcgccaggaataacctggaaacagagatcaaagactggaattttgatggtatcaggcagcaaaccttcaactcctggaacaaagcgctgggaaaaataacggtagcaggaggctcggaagaggagaagaaaatattctatacagccctgtatcataccatgatagacccgcgcaatttttctgatgcggatggaaaatatatcgggggagatggaaaagttcacgccgtgaaaaactttaccaaacgcaccatcttcagcggatgggacgtattccgcagccagatgcccctccaaagcatcatcaatccccgcgtagtaaacgacatggtgaattcactggtcaccctggcagatgaaagcggcaaccaatacctggaacgctgggaattcctgaacgcctacagcggttgcatgatcggcaatcccgccgtatcggtgatggcagatgcttgggcaaaaggaatacgtggctttgatatcagtaaaggctatgccttcgccaaaaactccgtagagaaattcgggaacggcagcaaaggatattccaccggcggactaagtgtgtcgctcacgctggaatacgcgtacttcgactggtgcctcggcaaactggccggcgcactcggcaaaaaggacgatgcgaaaaaatacctggcccgtggcgccaattataaaaatgtatttgacaccgccaaagcatggttccgcccgcgcaacgacgatggcagctggcaaccctggccggaacagggccgcatgcaacagggatatggcactattgaaagcagtccttatcagcagggctggtttgttccgcacgatgtgcccggcatggtagctcttatgggtggaaaagaaaaggtattggaagatctgaccgtattctttgataaagttccgcaaaacatgatgtggaacgattattacaaccatgccaacgaaccggttcatcacgttccgtttttattcaaccgcctgggcgccccctggcttacccagaaatggacccgcgaaatctgcgcccgcgcttatcataattctgtggaaggactggtaggtaatgaagatgtagggcagatgtctgcctggtatgtactggccgccagcggactgcatccggtatgccccggaagtacccggtatgagatcaccagcccggtgtttgataacattagcatcgccctggatccggcttacgccaaaggcaaacagtttactatcagcgcccgcaataattcgcctgccaaccgctacatccagcgcgcctggttaaacggcaaaccatacgcccactgttatatcaaccacgccgatatcaccgccggcggcacactggtactggaaatgggtaaccagccggcaaaaaactggggaattaaataaaaattaatggaagaatggcggtagggtctttttaaggtgtcataccatagggacaaaccgtaaccaatcaaaaaagatcccgcatcataggccactgtagaagactgcttttacagaacaggcgatgtcatgccacgtatgtaaatttttatcaccaaaagctggatgctaacacgtattaacgttatgaaaatgaaatttgcgttcactgctcctgtatgcctgtgcataggaatttttaccctcgcttcctgcggtaaaaagaacttcctggatcagacggaaacgactaacctgaacgagcaaacggtatttgccgacagcgcccgcaccgtcgctttcctcaccaacatttatgtcgacattggctttgcggaaaacgctacccgctttggcaacggcggcctcgatgcctcctgcgatgaagcggaaccacagaaatctgccacggtgaccacctccattcaatttgccaccggtaccgtcaatccttctatcatcagcgccgacgcctggaacctgccctataccaatatccgcagggtaaaccagctgctgaagcacctgcccggctcacccattccgtcgtttatccgcaacgtgatggccgcggaagcacgcttcctgagagcatggtattatgccgatctgctgaaacattatggaggtgttccgctgctgggcgactctgtgtataaggtggaagataagatccccgcggtgcgcaactcctataaagagtgcgtggactacatcatatctgaatgcgatgcagccgccgccgtattaccactcgtgcggattcgcgaagattacggccgcgccagcggaggcgctgctatggcgctgaaagcaagagtgctgctgtatgccgccagcccgctcttcaatggtggcggtatcaatccgcaggaggcgcctacagggtaccccgacaatgttccgggacgctggaagctcgccgccgatgccgctgctgccgtaatgaacaccgctgcttattctttgaatgaagataataccactgctcccggttatggcttttataaattatttacccttcgggtgaacccggaatatatcttcgccaggatgcagggcggcaaccgtgaactcgaaagcgcctggcaaccaccatcgcggaacggcgcccagggaggcttcccctaccagggatttgtggatgcttttggtatggcaaacggtaaacctattaccgatccttcatcaggctacaacgcagccgatccatacagcaatcgtgatccacgactggcctattccgtcatccgcgaccaaacgccactgatacaaaacaccggcctgaaagaaccggtcaatatctttctcggccccgatggcaaaggcgtaagccaggatgcggtacatgccggaacacccaccggttactacaccaataaaatgctcgatgaaaatattgccgccaactttatacacggctcgcaacgctgtttcccgctgatgcgctatgcagaaatcctgctaaacttcgcggaagcacaaaacgaatatgcaggcccggtgcaggaagtatacaatgcggtggaactggtacgtaaacgcgcaggactatcgccgtatgaattgccggcagcacttacaaaagaacaaatgagagaggccattcacgcggaaaggagagtggaactggcatttgaaggccaccgcttctgggatgtaagaagatggaagatcgccccgcaaacagaaaataaacaaatgaccggcatggaagtgaaacgcaacggcgcgaacgttacctataccatcttccccgtacgcaaacacaatttccgcgaagccatgtacctgtgggccatcccgcagggagaaaccgcgaaatcgcctgagttaaaacaaaatccatcctggtaaaaagcaacattatgaaatcaagattccagatatgtttactgatgccaatactggtactcatcatcaactcctgtcaccgcagtgaaatactggtgcccgagccggtgaaagatattgcaggcgaatggcgcatcgttaaagcagtgcgcaatggcgtggatatcactacactaacggactttacaaagttcaggatacgcttcaccgccgatcttcaatataccattgaaaatccattgcctttcgtggtcagtaaaaacggcagctacgcactggatgatcccaaatatcctttccggatcagcttcagtcaaacgggcgtcagcagcccggtcagcaccaccttcacttacccggtggtaaacggaaaacggaacatcaacttttcgttcagtcccggctgtaccgctaacacatacgactacacactcgaaagattgcatccctgatccaacacaacataacacgttatgaaaaaatatacatacggtatcatcctgttcctcttactgctggctggttgcgtattcctcgacggcgtggacgagccctctgctgctaaagcaggagagaacatcaccatcaccatgcataaccggatcgatgtagccgacggcggccgcaccggcgtaagactgatcattggtttcctggcgcctaaaaactgggcggcagcagccaattcaacgattacctataccaccacttcctatggcaacggtaaaatggtgccggtgccttcgtctgttctcgtcggcggcctgtcatggccggcggcactgaaaaacaggttcggcatgggcggcaactatatgacagacaatctcgaatgggtagtgttctggacagatcaggcctataatgtaccacaaggcgtaaaagataagatcgatgttaccatggtgatcaaaccaggtccggaaaatgtacagtttaaaaccggctatttccttggcaccagcagcgatggactcagcgatgtattcggttccaacaatgtatacaaaagcatgttcaaagattgcttctccatcacggatggtcagggcgatctcatcgacttctgcaatccgcagatagcggcagtaagccccggtgttgccaccgacaatgacttcctcaccctgagcttcgacccggatgtagtgtctacagcgctcaatggcgtaagcaacatttatctctgcgcaaaaggatataccagcgatggacatatcctcgaagcctgcacgcaaacggaaagctcaaaactgaaaagctataccggtaataaatctgctatcaccatctggccccgcgcatattttaacatgcaggaaggacaaacgctggagaagatcgaatacttttttacagatgctaccggcacggtgaaagtaggatttagcaataccactgccccttttgtgtacaccttcaaatgtcaataacaatggctcacagctacatcaataaatatatttcagcccttgcctgttgtgtacttgcggtttgcgcgaatgcacaggcacagcaaaccggtatcatctccggccggctgatagataactatggccagccacttgcaggggcggccatctctgtaaaaaataccggcgacactgccagcagcaataccaacggcgcattcagtatccatgcggccctgaacagcacgctggttatccaatatcccggttacaaggcaatagaacaaaaaatacacgataccaccgcgctcacactgcgcatggacgaactatttatccctttaccccaacgtattcccgtactctatggagaagcctccccgaaaagttcggtaggcgccatcggtacggtatacaccaatcaattgtctaccacaccggctaccttgtttgcctacgcattaccaggccgtttggcaggattgtatacccagcaggtaagcggcttccggaacccgggcacgggtaacaacttcgatgtagatatctttatcgggaacattccccggccaggcgcatcggaacccaatgataatacagaaatgaatctgtcgttgcgcgggcaggtaccggtaacaatagtagacggaatacagcgggatgtgttttccatcgatcctgaaaatatagaatcgatttcagtgctgaaagatggattgtctaccatcatgctcggtcagcgcagctcccgcggggtattactggtcaccaccaaacgcgcccgcgccggcaaaccacgcgtatcctttactgcacaaacaggcatccagcaatctctcagccagccaaagcctttgccggcatggcagtatgcttacctgctgaatgaagccctgcagaacgatggcaaagcgccgctgtacaaggaatccgactttatcgccttccgcgatcatacaaaaccttacaccaacccggacgtaaattggtataacaccatcctgcgcgataacgctcctatgtcccgctacaacctcaacatcaacggcggcggtaatgtagcccggtattccgtgtcactgaattataccggtcaacagggtatattcaaaacttcttctgataataactataacaccaacgcaggattaaagcgttacctgatcaataccgacgtagacattgacgttacacgaaacttcaatgtaggcatgcaactctttggccgcctgcaggaaggaacgcaaccgggcgccggaactaacaacatattgggaaacctcctcggaacaccgaacggcgcttatcccgtttacaatcccaacggcagctggggcggtaccagtaacctcaccagcaacctcctgtcgcaaaccattaacagcggctatatacaggataacagcaaagatgtgatggcaaatgtaaatttgcagtataatcttggcgactggctgcccggcctgtccttaaaaggaaaaggtaacctgtctatacaatcagccaatgcaatagaccgcagtaaaagtgacctggtataccgcgtatcgataacagatgaagacacgctgtataccaaagcaggcaacgcagtggcgcagcagaataatttcatttccgtttttaatgcgcagtatttctttggacaggcatcactgaactacgaccggcagtttggtccgcatggcgtgaatgccgtagtgctggccgatacgaggcaaaccatctttaactatgatctgcccggtaaatctaccaacatatcaggtaaagtagcttacaactacgcaggtaaatatttcatagagggcgccctcaacaggagcggctataaccgctatctgccgggtaaacaatatggcactttcttcgccggcggcatcggctgggacctcgcacaggaaaactttctcaaagaaaacaacgattggttaaaccagctgaaactaagaggtacctatgcacataccggcaacggtatcgataattccggctattatatctggcgccaggactttagcgaagataatggcattggcggcggcatatactcccaggggacagcgagatccgcaggttccggctttaaggagaatggcctggccaatgtgaatatctcctgggaaaccgcgcggaaaatggatgtaggaatggacctgtcactcttcaataacaggttgcaggtaaccgccgattattatcacgaccgctacgaaaatctcctgcagatacgcggaaaaagtatcgccctctccggcgccgcctatcccccggaaaacatcggtattaacctctaccagggcggagaacttacggtaacctaccagggcaggataaaggattttaactatttcgttactgccaatggaagtatcgaaggcaccaaagtggtgtttatggatgaacagcgccgcgactacgactggaacaaaagaacaggacagccggtaggcatgcgcttcggttatatagcagatggcttttttgcatcagcagaagaagcggccggcagcgctaccatcgccggttataaaccactggcaggcgacatacgctacaaagacctgaacggcgacggcgtcattaaccagtttgatgaagcgcctatcggtacgcataagcctcgtatttattatggcgttaacatcggtttttcctggaaaggaatagaagccagcgcattgttacagggtgtgggtaacagaattaactatgtagataattttgccaccgaagcaggtttccagtttcagaacttcacctacggtcaggcttatgaacagatcaccggccgttggacaccggaaacagcgggtaccgctacctatccgcgtttgactgccgacgcgaacaacaactacaataaattcagctcttctttttgggtacgtaatggtaattacttccggctgaaaaatataaatgttgcttacaatctcccttaccgctggacaagccgcgtgaggctgggcagcgtaaaggtatttgccaatgcacagaatctgtttacacatgctgcatacgatttcgttgaccccgaagtaggagtgggagcctatcccatccagcgggtactgaacaccggtatcaacataaaattctagtcagccatctaaacaacgcaccatgaaacatttccgcatattgatcttcctggccggctgtatgacagtcatcatcagctgcagaaaagattacgaagttattccactcgaaaaagtaaccatcgagtatgtatttgaccaggatgattcactgggtacctatgccaacaaatttctcaacagcatctattccaaacttcccggtggctacaaccgtgtaggcggcgatttgctcgatgcagcctcagatgatgccatctccggcctggtaggtacctccgcggtatcacaacttgccacaggtgcattcacctcttatgcacccatcacagacgaatcgccctggaacaattgctacgccgctatccgcgctgccagtctttttgtttccaatatcgacgtgtcgcccgtaaaggaaaaattacccaacggcgcctctatccgttacgcatggaaagcagaagcccgttttatcagggcgctgttttattttgaactgctgaaacgctatggcggtataccgcttatgggagataaagtaagagagctgggagatgatgtgcagataccgcgcagttctttcgcagattgcgtaaactatattgtaaacgaatgcaacgccatcaaagacagcctgcgtcctaatcccattgtagcgccggagttgaacagccaccgtgccaccaggggcgctgcactggctttaaaagcaagggtgttgctgtatgcagccagtcccttgttcaacgggcaaaatatcgaggccggtaatccgctgacaggttacagcagttatgataaagcacgctggaagctggcagcagatgccgcccgggaactgatcaatgaaaagactttcgcgctggtacccaatttcaaagatgtattcatcacccaaaacaacagtgaggttatcttcttccgccaggggggaaacactacggaaattgaaagtaccaacggaccggtaggttttgccgcggtagcaagagggcgcaccaatcccacccaggaactggtggatgccttccctaccaatgccgggctggcgatcaccgatcctgcatcaggctacaactccaatgaaccctatgcccgccgcgatccacgcctggccatgagtatcctgtacaatggcgcccgctggctgaataccgaactgcaaacatttcagggcggtcagcaccggcccggcggcgcagaacccggtacgaaaacatcttactatatgcgcaagttcatgggcaactttgaaaatgccacacagtacagcaatacaagccacgactggatcatcctgcgctacacggaagtattgctcaattttgccgaagcagaaaatgaatccaacggccccactgcggaagtataccaggtgctgaaagacctgcgcgcccgtgctgggattgcagccggcgataacggcatgtatggtctgaaggaaaatatgacagcagatgaaatgcgcaatgtagtgcgtaacgaaagaaggatagaactggcctttgaagaacaccgcttctgggatatccgccgctggaaaattgcgcagcaggtatatggaaaggcactgcatggtatgaacatcatcaaggaaggacctgcctttagctataacctggcggaagtatttaaaccggtgtttattgcgcccaaaatgtatttgtatcccattccatacgatgaagtggtgaagaacgataacatgcgccaaaatccgggctggtaaagtcatattccttacaagaaatttaactgactgaagatgaaaaatattatactgtttctcctgctgctggttgctgcaccatttgtggcaacagcccagcaaaaaaatataagtggtacggtaaaagacgtaaatggggtactgcccggcgcttccatttcggaaaaaggcgtgcccaccaacggcgtgatagctgatgccaacggccggttcaaactcgccctgaaaggcagttcccacaccctgatcgtaaaactgatcgggttttccgcgcaggaagttgacatagccggtcgcgatgcgattgacgtagtgctgcaatcttccacccagggcattgatgaagtagtggtggtaggctttaacaccgccaaacgtatcaccagcaccggcgctgtaagtgccattaccggcgctgaaatcaggaacgtacctaccgctaatgtgcagaatgccttgatggggaaactgccgggattcgtttctcagcaacgctccggacagccgggaaaggatgcttccgatttctttatccgtggcgttagctcgctgaacagcgatggaaataaaccgctgatcattgtagatgacatcgaatattcctatgatcagctgcaacagatcaacgtgaatgaaatcgaaagtatctctatcctgaaagatgcgtccaccacggcaatatatggtatcaaaggcgccaacggcgtactggtggtggccacccgccgcggtaaggtgggacttccgcaggtaaacctccgcgtggaatcaggccagcagtcgccggtgaaaacaccaaagtttttgaactcctatgatgcggccacccttgtaaatgaagcgtacaaaaacgatggactggcgccgaaatttacctcccaggacctggaacttttccgcagcggcgccgatccttacggacacccggatatcaactggtatgatgcggtattcaaaaaacacgcttaccaggccaataccaacgtggatatttccggcggtacagaagctgtgaaatattttatctccggcggattcctcacccagaacggcctggtaaaagacttctctgatcccaggaatgaagtgaataccaactacttcttccgcaggtataatttccgctccaacctcgatatgcgcgctaccaaaacgttaaccatgcggctcaatcttaccacccgtttcggtgatattaaccagccccggtcggccaacgtggtatcagaagtatacaactttgaaaaaatacatccctactccgcgcctttaatgaaccccaacgggagctacgcctatgccgtggatacaaaggacgcattgcctacgctcaatgcacggctggctaacggtggctacagccgcactaaaagaacggactttgatgtgctgtacgacatcacgcaacagctggacttcctgacgaaggggctgtcgctcacaggccgtattgcatacggtggcatcgaacagtatgcaagaaatttattccgcgaagcagaaccgccatcatattattataacccggcggatcagtcgtacaccctcgatccccgcggcaactaccgcctgcagaaataccgggtaacaggtaacacagacctctacagccggaatgtgaatacacaggctttcctcagctataaccgtattttcggtgatcatacactcaatgggttggcgctgtataacaggcaaagctatacgtcgaaggcagatattcctgccaacttcaggggcttttccttcaaggcaggctacaactataaacagaaatacctgctcgatttcaacggcgcctacaatggctccgacaggttccaggcaaagaaacgcaacggcttctttcctgccgtgggcgtaggttggagtatttcggaagaaccattcttcaaacgtaacaacagctttgtaagccttctgaaagtgcgtggatcatacggtgtagtaggttctgatgttacgtcaggtaaccgttacctgtaccgccaggaatatctcaatggcggcggttattcttttggggagaatgatacgcaatccggctccatctacgaaggcgatcttggcaacatggacgtaagctgggaaaaagcaaaaaaagcagacgtaggggtcgatgtaaatctctttaaagacaaactatcttttacggtagattatttccacgatatccgcttcgatcagctggtacggaaaggctctgtgcccaacatgattggaattggctacagtcctaccaacgtggccagaaccagtaaccagggcttcgacgggcagatcaactaccgggggaatatccgccaggtaaattttaataccagccttgtattccagtatttcaaaaataaagtactgtttaaagacgaagcgcaacccgcctatccctggctgcgggaaacgggactgccaatcgatcagccattcggatacacctttatcggtttctacacaccggaagatatccagaagatccaggccaatacacacgataaacccgctgcaccactcagtgaatatcctatacaggcaggcgatctcaaatacaaagatatcaacggcgatggcgtgatcgataacaacgaccaggggcccattggaaaacccaacctggccagcactgtattgggacttaccctcggcgccaattacaaaggcttcagtattaacctgctgttccagggctccttcggatacagcttcagcgtagtaggcaccggtattgaaactttccagagccagttccagcctattcaccagcagagatggacgctggaaaatgctgataaggcgcagttcccgcggctcacgagcaaccctaccacggtaaacagtgcgcgtacgtatatgtcggatttctggttgatagatgcgcgctatgtgcggctgaaaacagtggacctgggctatcagctgcccagccgctggctgccgggccggttgaataatacacgtgtgtacctgagcgcgtataacctgcttacgtggaccaactacgataagtaccagcaggatcccgaagtagccagcaactccgccggggatgcctacatcaatcagcgcgtgatcaacctgggtctccaaatcagctttaaataatatcttatgaacaaaatgctattgctattgattaccggcggcatttttacttcctgtgtgaagaacccgctgagtgattatcaaagccaggaacgcgccatcatttccttccggttacccgaaggccaggtgggtacttcagagatcataaacggaacagattccgccaccgttacggtatgggtagaagatgatgtggacctgagtgccgtgagccctttggtgatggtatccaaaaacgcgactgtgctgcccgcgccgggagtgaaggtggattttgctgccaataacaatcgttatgcttaccgcgtcacttccgaatccggggagcagaagtactggtacgtacgcatcatgaaaaagacaacagctgccggtccgcgtttgcaactgctgccaaacaatggccagtggaacccggcagtaagagtatacagcgatcttgattacaacgattatcttacccgctaccagggctggaacggtggcgacggctgctattcggtgttactgccggatggccgcctgctatggtcattccaggatagtttcttcgggcaggtaagtgcggaccgtaaccgcaccaataacgtaatgctgcgcaacgcagcacacctgcaactggatacttctttgcaaagctttgtgcaacttaaccctggttcagggagtgccagtcaaacctggatcaaatacggcaatgcacctgaagaccaggactggtactggcccggcgccggacaggtatataataacaaagtacagatgctgttaagtcatgtgaagaaaaccggcagcggcacctgggattttgcacacgtaagcacagacctcgccatcttcgatttgccctccatgcagctgaaccagttgatccaggataaggatacactcagtaactacagcgctggcagcatgaaagcacccgatggctatacgtatatgtacagtacggaaaatggttttctcacctcttctatgtacgtggcccgcgcagcaaatcatgatcttaacggcgcctgggaatattacaacggaaccggatggagtactacaccggtgaaatacaatgtttgtaatgacatcagccagccgaacgttttttataaaaatggtaaatattacctcgtatcgcagcaaattattttcggactggatatctatattcttgaatcaactacgccggtagggccgtggacgaataaacgcacactgtaccatatcccggatcaatacagcgtaggtttcatcagttataattcatttgtgcaccatgcactaagcagggaaggggagctggtgatttcttacaatatcaatcccactgatttttccaccaacttcaacagtcccggtagtgccgacaggtacaggccgtattttgtacgggtattcaattggcaatagcaaataatcatgttcaacaaaggaaaaaaattgctggccctgctgatgatctcagggctggcaatgaaagcacaggaaaagacgttcagcttaaacagcagtaataaagccgtacactggaaagtaaaagcagcggaagcaggccaggagcctggtctccatgccccggactataacgaccataattgggtgaacggcgtggtgccgggtacagtatttggcgcatttgtagcagctggattggagaaagatcccaacttcggagataatatttaccaggtagataaaacaaaatatgaccgcgatttctggtaccgggccacgtttacgcctgcacgtaatactgctgaaaagcagtggctgaatttcgaaggcgtgaaccgtaaagcggaagtatacctgaatggtcagcgtattggcgcgctggatggttttatggaccgcggcaaatttgatgtaacggatatattgagatatgaccggccaaatgtactcctgttattagtgcattggccaggtacgcctattgtgaattattccagtcctacctacatttcaagcgccagctgggattggatgccttatgtgcccggccttaacatgggcgttacggacgatgtatatcttggcagctccggccaggtgacgattgcagatccctggatccgcactgctttaccggattcatcgcgcgcaaagctcagcatcagtatggacctggataatcattcggccggcatacaggaaggagaagtatccggtattatccagccaggcaatatccgtttctctaaaaaaataaaactacccgcaggacaatcggagcaggtaatgtttcatccggagatagcacatccgcagttgtggtggcccaatggctatggcagtcagccgctgtacacctgtcagctgcagtttgtatccggtggaaaatcatccgacagcaaacaggttactttcggcgtaaagcaatacagctacgatacgcttggcggcgtgctgcacatcagcgtaaatggcaaacgcatatttataaaaggcgggaactggggcatgtctgaatacatgctgcgctgccgcggcgaagcatacaatacgagggtgcggttgcataaggaaatgaactttaacatgatccgcaactggataggcagtgtaaccgatgaagagttttatgatgcctgcgataagtatggcatgcttgtatgggacgatttctggctgaactcacatcctaatctgccaaaagatgttttcgcctttaacaggaacgccgtggagaaaatcaaacgccttcgtaatcatcccagcatcgcggtttggtgcggcgacaacgaagggtatcctttaccgccactgaatggctggttaaaggaagatgtgagcgcctacgatggcaacgaccgcctttaccaggctaattcccactcggacgggttaaccggcagcggcccctgggccaatttcatgcccgcctggtacttcacaaaataccccggtggctttggaggaacacccggatggggaatgcgcacagaaataggcaccgccgttttcacctctttcgaaagctttaaaaaatttatgccggacagcagttggtggccgcgtaacaaaatgtgggatctgcacttcttcggtccctctgccgcaaacgcaggccccgaccggtacgacgacgccattaataaaagttatggcaaagccaccggcatcgaagattattgccgcaaagcgcagctgttaaatatagaaaccaacaaggcattatacgaaggctggttgcaccatatgtggaacgatgcctccggtgtaatgacctggatgagccaaagcgcctatccaagcctggtgtggcaaacctacgactattactacgacctcaccggtgcatactggggcgttaaaaaagcctgtgagccattgcatattcaatggagtgcggcagataattccgtaaaagtgatcaacactacattggaacaatacaatggtttacaggcggaagccatcgtttacaatatggatggaacgccggcgccaaccttcggccggaaagcaaccgtagatgcagcttccaatacagccacaccctgtttcgatcttaacttcaatatcgataaccttgcttttaaaaaatcagcagtagcatcttcgtcatcaccggaaagcgccggcgccggggccgtagcggatggcagcaccggttcaagatggagcagcaactacaccgacaatgaatgggtatatgtggacctggatgccgtacaggaaatcagcagcgtgatgctgcattgggaaagcgctcatgcccgtgcctatagcctccaggtgtccgccgatgcaaaatcctggcaggatgtgtacgccacagatactggcagcgggggaattgaaaccatccctattaaacccgtaaaagcgcgttacgtacgtatgcttggccgtaaacgcgccacagaatggggctattcgctgtatgacatggaggtgtacggcaaacgcagcaaagcgttgacggatgtacagttcatccgcttgttgctgaaagatggacagggcagattacagtctgaaaatttctactggagaagcagtcgaatggcagattataccgcgctggatcaactgccccgggtgcaattgaaaacttcctccaaactggaacagcatggcgacagtacccgcgttattgctaccatcacaaatccctcatctgcccccgcctttgcagtacatgtgcagctgttaagggcagacaacaacgaacgcgtgttgcccgccatcatgaatgataactattttacgttgttaaaaggagagcagaagcgggtggagataatgtttaaaaaagaattattgaaagatggaaaatataaactcctggtgactccctataatcattaatacgctggtattattggatagaaaagcctttgcctggtcaggtaaaggctttttttatgggggtatttatatatcgattataacatatgtatgctgaatctacggtgctttctttaatttagtggcagaaaatgagcgaatttgataagggataactcctatagtgacctggaactgataactatgctgaagagaggggatgtgacagcgttcgatctgctttatgcccgtcattggtccggtatgtaccaggcggcatattacctgttgcgcgaccagggcgcctgtatggacatcatacaggacatttttgcatggttgtgggagaagcgggagcaactggatatacaggcggtgccatcctatctgcgaagcgctgtcaggtttaaggtggctaattatatccgctccggtaaggtgagagaggagttctatacggaactggcggggttgtctttaccggaaacaccgggtccgcaggactttatggagctgagcgacctgaagtcgattatcgggcaggtgatccgcagtttgccggaaaagtgccgcgagatatttctcctgagcagggacgggcaactgacgaatcaacagattgcagacttattgaatatttccataaaaacagtcgaggcacagaaaacaatagcactgaaacgtatccgcgcagcagtagatcctcacctgctcgccttgttattactcccggtgatgacccattaccattaagatacccggctcaaaaaaaaaatttgagactcttttaagggtatgtccttttacaattgcctatgtatatgacaggttacgcatgacacgagaagaggcaatattattaacagaaaaagttatatccggcacagctacggatgaagagctgctgcaatacaaccagctgttcaatgcttttcagcaacaggaaggctgggatgaacacctgctgggcaataaacagctgctggaggatgcgatccgcctgcgtttacagcctgtactcgaccgcaggcccaaagggaaagtggtccggtggtacaggtgggccgcagcagcaacagtaacgctggtactgggtaccggctattatttctatcagcaacagcggcaacaaccgctggcgccccaggcggtccgttttaagaatgatattttggcgccggccggtaatcatgccgtacttacattgggtaatggtcaacagatcctgctggatacagcgagcaatggcacgcttgccatgcagggacaaaccagcgtttccaaaaacgcgaatggccagatcgtttataacagcgctggtaacgacgttagttttaatactatccaggttccaaatggaagcaaggcgctcgcgattgtactgggcgacggcaccaaagtctggatagatgcaggttctacacttacctatccggctgcattcagtggcggtaaacgcgaagtatccgcaacgggacaggtttattttgaagttgcgcaaaacagcaaccagcctttcattgtaaaatccagcaccaataaaaccaccattgaagtattgggaaccgctttcaatctccgttccttccgggatgaagaaaaaatgaaggtcacccttgtcagcggtaccgtaaaagtaaataccgccgccgcttcacagttgctgcatccgggcgaacaggcggcaacagcagggagtgctatacaactggtcaccaacgccgatctgcagcaggtaactgcctggaaggaaggattatttgtttttaatggcgctgacatcgccaccataatgtcagagctgcaacgatattataatgtagacgtcgactttcagaccgatgttaaagatgcttttgtcgcgagaattccgagggatgtccccgtatctcagttgctgaacttgttggagatgaccgatctcgttcatttcaaaattgaaggacggaaaattactgtgataaaatagtacatacaccagctcaatcgtccgatcgggtaaggcaggccaccttaccggcgggagaaatgttgccagattttagtttatccgcacagcggtattgttcatcaaaaatcaaccagaagctatgcttgtaaaaaagctgatgagcgctttatgcctttcgaaatcaggagagaaaaagccaggtgccaactacctcaggacttatttactcatgggatgcctgctattggccacccagactttcgcgcagaaagtatctatgaacatgaaatcaggttccctggaaaaagcgttccgggaaattgaaaaacaaacgggatacagctttatttatgggaagaaccaactcagccaggcagcgcccgtaaacattgatgtaaaagatcaggagctggcagatgtgctgaaattacttttcaataaccaaccattcgcttattccctgtcgggaaaattcattgctatcagggtgaaaaaagccccgggcactgaaataaaaccggcagatgacggcattactatccgcgggaaaataacagatgagaaaggaaatcccattcctgcggtatctgtggtgattcccggcactcctttcggcgcaatgacgaatgaaaacggagagtatgtcatcaacagggctccggcggaagcacagctggtagtatcctatctttcctttgaaacacaacgtatcgccgttaaaggccgtacagccatcaacgttgttttaaaggagcaggtaaatgcattaactgaaacagtagtgatcgggtatggaactactactaaaagattgaataccggttcggtgagcagcattacggcaaaggatatcgaaacgcaacctatctccaatccactggccgctctacccggacgtatcccgggtgtacagatcacccagcagaatggcttgccgggtagcgctgccgtggtacagatcaggggccagggctctttgaactcaggcacccttcctttatatgtgattgatggcgttcctttcaccaattacaacggctcttttcctcctacggataacctcaactcctttggtgccagtggcgccaacggtggtatcagccctttcagtatgatcaacccggatgatattgaacggatggatatcctgaaagatgctgatgcaacggccatctacggcgccaggggcgctaacggcgtgatcctcatcaccacgaagaaaggcaaatccggcaaaacaagggtgaacctcaatgcctatacaggatcgggaaaagtaaaccacttcatccctatgatgaacacacagcaatacctggacctgagaaaagaggcctttaaaaatgatggcctcacaccaaatacagcgaatgcgccggaattaaccgtatgggaccagcatgcttacaccgactggcagaaactcctggtaggaggaacggccagatccaccgatgcacaggcgtctgtttcaggaggggataccaaaacgcattttatgttcagcggcggatatcataaggaaactactgtgtaccccggtaacttcaacagccagcgcctcactggccgtttatctgttgaccatacctctgccaacaataaattttatgcggctttcacaaccaactattccaacgataaaaccgttctgccggcatcagatgttatttccctgtacaacctgccacctaacatgcctttgtacgacagcaccggcaaacttgcatggactggtcgttacgataacccgcttgcgctcctgcaacgccgctataccaatacaacaactaacctgatgacaaacgccaacctgcgttataccatcattaaaaatctcaacttcaaagtaaatcttggttataccaataccaccctggatcaggtgaatccactgccggcatctacgcagaatccggtcaacaatccgcagtcgtccgccacttttgcgaacacacggtcgcagaattacatcgtggagccaacccttgattacagtatagatatgaagcagggcagactgaacctgttggtaggaagttcgtatcagcggaccctcacttccggtcagagtgtagacggccggaattacagcaacgaagccttgttggggtccctggttggtgcaggtactattgtgctgaactccagcaactacttcgattaccgttacgcatctttgtttggccgtatcaattacgattaccaacaaaaatatttgttgaatgtaaccttccgccgtgacgcttcctccaggtttggaccggataatatcctggctaatttcggcgcagtgggcgctgcctggttgttctctgaagaagattttattaaagacgcacttccctggcttagtctcggtaagctgagagccagctacggtaccactggtaatgaccagatcaataactacatctacctgcctttgttgtcatccgcaggtacttaccagggggcttccgcactgctccggggaacgctgccgaacccgggtgtgaaatgggaaaccacccgcaagctggagtttggcctggagctgggcgccctgaacgacaggatcgcatttaccggtagttactaccgtaaccgctccgccgatcaactcctgtcagccgcactggctacacagtcgggatacaacagctatactgtaaatgtaccagccctggtacaaaacagtggggtggaactggagctgaataccctcaatcttaaaacatggaatttcggctggaggtcatctgtcaacgtaaccttctaccaaaataaactggtggaatttccagggattgagaaatccttttatgccagcagctatcttgtagggcagcctattgaccttgtcagaaaatatatttacaccgggtatgatcctaatacaggaatcccgcagtatgtggatgtgaacaaagatggaagtgttgattttaacaatgaccgtcagatcatcaaaccaggtacgcctttcttcggaggattgaacaatagtttcagctataagaactgggacctgagctttttcctgcaatataaccacaggaagggagctaccaatactttcgatatacccattggcagcagcacaaataaccagaacacatctttgctcgacaggtggcgtcaaccaggcgataaagccgcctacccggcagctacttctacttccggcacgcctatctatctcggctatacgccgtattacagttctaccgcatggtggggagatgcaagctatctgaaactgagatctgcttctctttcctattcattcccgagggcatggattacaaaagcaaagatcagtaacctgaaagtatatgcagaaggacagaacctgtttacctgggcgaagaataaatacatctacgatcccgaaacgagtgtttcaggaggtcctccgggattgggtaccggtatgattgccatgccgccgttgaggaccattgtatttggtattaactgttcattctaaaatctgaattcgatgtcttgcttcaaaataaataaaaaggtaaccgcagcaatattactgacaggaattgctttttcttcctgcaaaaaactggtggaaattggtccgcctacaacgcaggtgggccttgaccaggcctttgcatccgatgcaactgccaccagcgcagtgctgggggtttataatgccagctttacacgggatgtacttttccctttgagtgaaatgccgggactttctgccaatgaactgcagaacaatatttccagtcccgctttcgatgagtttaaaacaaacagcatcaccatcaccaacagcgtgattaacttcgtactctggggatattcttactccaccattgcacaggccaatgccatgatggatggtatttcccgcagcactaccttgtctgctcccgtgaagaaccagttactgggagaaaccaaagtatggagagccttcatcaatatgtaccaggtaaatatgtttggcgacgtgccaatgccggttacagacgatccgctggcaaatgccacactggcgcgtactccggcagcgcaggtatgggagcagatcataaaggatcttacagaggcacaaagtatactcacagatgcataccccgccacactgagaaccaggattaaccggcaaacggcgaacgccctgctggcaagggcttacctgtaccagaagcaatgggccaatgcagaatctgccgccagcaccgtgatcaactccggtatttacagtctgaataaagacctgaacactaccttcagtaataccagcaatgaagtgatatggcaactggctacgcttaccggcttatccacctatactaccaacaggagtgccaatggaggcagctatgcagcagcaacaggttccgttccggcagtaacgctaacggatacactttataattcactggaagcaggcgataaacggaaaaccagctgggtagcagcaaccgatatcgggggcaccaattataaagtgatcacaaaatataaattgcgggtgctcgccgctggtaccaccaccggcaatgagtttaacgtgatgctgcgcctggctgaacagtacctgataagagcagaagcgcgcgcccaacagggcaacctcaccggcgccattgccgacgtggataccatccgcgctaaagcagggctcccaatgctggataataacatcacccagcccagcctgctgctggccatcgaaaatgaaagaaaagcggaattattcggagaatggggacaccggtggtttgaccttaaacgcacacctggaatttccagcggaggtaaaacccgtgcagatgaggtgataggcggcatgcgccctgccacctggacaagcaccgacatactctatccaattcccgatgcacagcgtgttgctaacccggcattaactcaaaacccgggatatacaaactaatcataaaccaaccatgcacaatatgaaaaaagtactcccgattttgctgagtggtagtctccttaccgccgccctgcaatcaaacggacaggcaaaagttagccaggactccctgatgagatattatacgcagctcgctaaaggcagtgatgccgataaagcactgctggcgactaaactatatgcgctcaccaaaagtaaaaaggaatccgactggcttacggcatccggtttcttttaccagctgaagcaggtaaatgtctctgactctatccggcaggcagctgaaaaaaaattccctgctggtatcaccgtccgcgataagcaggtacaacctatctacgacgaaaatgacccggtgaaaaaagaagcgctctataaagcatggatgaagaaattcccgcagggcaaactggacaacgatctgatcgtttatgactatgcccgcaatagtgtgggcattgcctatgcgaacgccgataatttgccaaaagcactggaatatgccaacagtatagaatcccctttctggaaagggcaggggtgggcaggaactgctgaacgcattattaaaaaaggacacaccgcggaagcaaaagtgttgctgaaaaaagccgttgatgatgcctgggaattcagaacgacccgtaagaatgaaatggcagccggctttgcagcgatgggctatccaggctatctgagtacctatgcacagctgctttacaacgataaagaatatgactccgcactggtgtaccttaaacgcgcagaagaggcagaaacacctgtgagaccacaggtaaacgagatgtatgcaaaagtgttcctggcaaaaggagaatataaagaagtactcaaacgcatgactgaaattgcggcacagggcaaactgaacgacaacaataaagaactgttggctaccgcctatgccaaagtacgtggtgataacaacctgcagggatatatagactcactgaaaagcgggctggataaaaaaatgcaggaagaattcgccaaacagatcatcacagaaccggctcctggcttcaccctgaaagatgtagatgggaataccgtgtcactggcagattacaaaggaaaaaccattgtactggacttctgggccacctggtgcggcccctgtaaggcctcatttcctgcaatgaaaaaggcaatggacaagtacaaaagcgatccgaatgtgaaattcctgttcgtgcatacctgggaaaaagaagcagatgcaaccgcgaacgcgaagaaatatgttaccggcaataactttccttttgaagtattgatggacctcaaagatcctgcaaccggtgtaaacaaagtagtagagagctataaagtgaatggcattcctaccaagtttgttatcgatggcaaaggtaacatccgtttccgtttcacgggcttcagcggcggcgacgatgccgcggtggcagaagtatcagccatgatcaccctggcgaatcaacaataacagaacagttactttaaataaaataaaacagcggagtggcatcacttcgctgtttttattttattactgaaatgagtattgatgaaaacacataatatccttgtgtaaaatttgttaacaaaaggttacggaaaattgatatattcatagtcaaccaaaatcaactgctgctatgagaaatccagttcttaccggatgccttatcctgttatgcctgttcaccagtctaataacctatgcacaggtaaccactgccaccctgagcggcaccatccaaagtaaggaaggcaaaccattagccggtgccaccgtgaaaatcgaataccgggaagccggtatcagtaaagtaatcatcacccagaataatggctccttccaggtgcctaatctgagggtaggggggccctacaaagtgacggctactttcgtgggctattcagaaaaatcggaagagaacatcttcctggaactgggacaaaacactgccctggacttacagctggaactcagctctgctaacctgtcgggcatcacggttaccggccgctccaaaattttcgataaccagcgtaccggcgcctcttctaatatcagttcgcgtcagttgcgtcaattgccaaccatctcccgctctgcggatgattttacccggctgacgccctccgcgtccgcaacgatcaacggtacctctttcgccggccgcaatgggcaatacaataactattcgctcgatggcgccgtattcaataacccatttggcctggatgcacctacacccggcggacaaacaggcgctcaacccatttccctggatgccatcgaccagatccaggtgaacctggcgccctacgatgtaacccaggcgggcttcaccggcgccggcgttaatactgttaccaaatcaggtaccaatactttcggcggcaccgtgtacggtttttaccgcaaccagggcatgaccggcaaaaaagtggacggcaacaaaatcgccgtaccggatctcacacagctgcaggccggctttgcagtaggaggcgccattgttaaaaacaaacttttctatttcgccaactttgaaacagaacaaagagacgacgctgccagcagctacgtggcccgaaccgccagcaacggcgacaacaataacacttcccgcgtgctggaatcggacctgatagctgtaagcgatatcctgcgggacaagttcaactatgaaaccggtccctggcaaggttttaatctcaagcaaaaaaattataaatggttagcaaaactcgattgggtgatcaacgaaaatcatagcctgtcttttacctacaatggcctgcaggcaactaaagaaaaacctgcgcaccccaacgccatccgcgaccgtggtcccgattaccagactttacaattcagaaattccggctatgagatcgaaaacagattgcaatctttcggcgcggagttgaaatccagtttcggcaaccgctacgccaataagctgagggccgtgtataccaccttcaaggacaaacggacgcctttctcggaaccctttcctgtactgaatatcaccaagtacggtaccatgtacatcgtggccgggcatgagccattttctatcaacaaccggttgaaccaggatgccttccaggtaacagacaatttcaacatcatccttcccagacataccattaccgttggagggtcttatgagtcctttaaattcgggaattcgtttaacctcaccggttatggcgctacccttttcagcgacgcggatatccaggttttcaaagacagtgttccggccagcggcaaatatgtttttggtgcatacccgctggatgtggatgtagcggcagcaagagccgcaggcgccgctgataaatggaactggtattatatcactgttgcacagttatcaacgtatctgcaggatgagtggaaagccaccgaaaacctgcgcgttaccttcggcctccggatggatattccgctttatatgaattcctcctttcaatcgccggatggcaaaaaaacttctcccaccattcccaataacgatgacctcaccctcttcgatgaacatggagaacgggttacgaacggccagggaaaacaactggacaatacccggcttccttcctccaaacccctgttctccccgaggatcggtttcaactgggatgtgaaagccgacaagagcctgcagctgagaggcggttccggtctctttaccggccgtttcccgtttgtatggattggtaaccagatcggcaaccccacctccggtttttattgcgccaccgaccgcgattttaaatggccgcagatctggcgcaccaatatcggtgccgatatcagggccggactgggaactattttcagcgtagatgtagcctattctaaagatgtaaatgccatgatggtaaggaactataagctgggtacgcccacaggctccttgaacagcggcatcggtgatacgcgaagtgtatacaaagacaccgacaaaggagccgtgaatgcgtatattttcaccaatacaaaaacaggcgatcagttcaacaccagcttcaccgttcaaaaaacgttcgccaataacctgtttttatacggcgcctataattacctcgtgtcgcgcgatgcaagctccatttccgcagaaatcagcggcgacgcattcgaccggaatcccattctcaataatgccaacgaagccaggaatacaccttccctttatggaaatacccaccgcttcgtagtggccgccagcaaaaagttcaactacggaaaaggtaaatatgcaacaaccgtttccctcttcggtaactggagcagtggtaaccgctttgcctatatttatggaggagacatcaacaacgacggcactaccagcaacgacctgctttacgttcccaagaacagcgaaatcgacttaatgcagttcgcaccgcttactgacgtaaacggggtagtacagaatgccgcagcccagaaagcggcgtataaagcattcatcgaacaagatcattacctccggagccggagaggtatgtacacagaaaaatatgcaggagtaagcccctggttcagccaggtggatatgcgcgtattacaggatttttattttaagagcggagaaaaaatccggactgttcaaatcagcctggatgtagttaacctcggtaacctgatcagcagcaaatggggcgtccggaagtatgccagcaactcaggttatttccagccaatatctgtaaccggcgtaaccaatggcgtgcctacttaccagttcgatccttctttgaaagaaacgtttattgccagtccggatttgttaagccgctggcaaacccagctgggattgcggtttatattttagcgaagtaaaattggcgtgaatcatcaaatagcattttcaagtatttaagcaaaaagaagaagctgtctcataattaattgagacagcttctttgttttagccaaaagatggcctaataatcattatgatgatcaggtgttttttaagagaataaatagttaatgtcagcttgctttagcaagc

SEQ ID NO: 12 - DNA, 265188 bp, Chitinophaga pinensis
  source 1..265188: mol_type = genomic DNA
acattcgagaatatatagaatattataataacgatagaatcaaattaaaactaaatggcttgagtccaatacaatatcgaactcaagccgcctaatcaaaaaagtctaaactttggggagcagtacatattttcgcttttatctcccttaattattattaaaaaatcaaagaaatctaaaaaaaatccaaaagtaaaaatccaggtaatcagtaaaatcagcgtaatcctgagccaagacaacatccgcgttatcttacgcggaactgctgcgacaacacgaagttgtctgaactctttcctatattgatcgtatacgtgcctttgtatagcttccacgcgtgttgctgcaaatcccatttctgcaactctgctgctggcagtgccaattctacgatttcttctccgcctttgtttacacgaacacgtttaaatgctttcaattccttcaccggcatgcgttccatatccggataggtgatgtaggcctgtactacttcgtcgccatcaaaggcgccggtatttttaacggctacggatacacggatagtgtctttgctgcggtattcttttgcgggcgttgcgtgccaggcataatcaaatttcgtatagctgaggccgtagccaaaaggatatgctgatttacctttaaaataacggtaagtacggttcttcatgctgtagtccttatagtcgggcaagtcctgcagggattgataaaatgtaacaggcaaccgccctgcgggcgaatattttccaaagatgatatctgcgagggcattaccaccctgttctcccgggtaccacgccaggatcactgcatctgcatagggagcaatggcagatacgtctactgcactgccggcagtaattaccgcaatgatgggcttcttatgcgcttcccttaattttttcatgaacagaatctgggagcggggcaggctcagcgtatttttatcgccgccggacgaggacaggaaagcgtcaccttcttctccttccagcagaggcgttaagccgatcaccgctaccgttacatcgcagttctgcgaagcccagataccaccaaaatgcagggtatctgtaaagtcgcatccctggtcgtattgcatggccatacccggacctgcagccctggccaggccagcggcaaaagtgaccatgttacccgatacaccatgatagttgcccatcagtgcttccaatgatgcggaattggagccggtcaccagcatggaagcatatttatccggacttaagggtaatacaccgtcatttttaagcaataccatgctttccctggccgcttcacgggccagttgggcgtgatagccgttatttacactatctgcgccatatccgttataaggactttccgcgggcgcatccagtaatcccagctttatgcgcgtacgcagtgtggcactcagggcactgtctacattcgcgctggttaaccagcccttatcaatggctttcatcacatcgtcctgtaaaatattggcgcaatcgagatttacgcctgctttcacggcggctgccgccacttcctcgcgggtgggaatggctttatgacgcagccagatatcgtccagtgcccagcaatcggtaacaacctgtccgccaaatttccattcatgccgcaggatatcctgtaacaacgtattaccggtgcagcaaggctcgttatttacgcggttataagcgcacatgatcgattctactttgccgtccaccagttttttaaacgcatagagataggtttcccgcaggtctttttcgtcgatgatggcattaaagctatgccggtcggcttccggtccgctatgaacggcgaaatgtttggcacaggccgccgttttcagcatgccgggcacatctccctgtaatccctgcacaaaggcgcccgccatggtagcagtgagataaggatcttctccatatgtttcctgaccgcggccccagcggggatcacggaagatattgatgttaggcgtccagaaattaagccccatatattgcacatgccggtgttgctgcacggccaggttatacttagcacgggcttctgtagaaatggtactggctacttcctttgccagtggcgcattaaaggtagccgacaaccctatcgcctgcggaaatacggtagcttctccacccctggcaataccgtgcaacgcctcattccaccagttatacgcggggatttgcaaccggtctatcgccgggctgttatatcccagcaacgatatcttttcagacaaggtaagggtatgcagcaggtcgttcacccggtcattcaacggcgcatccgcccgtttgaacaatgccggctgctgtgcaactgcgtttgatgtaaataaaagtaaagaaccaaaaatgaaaaactgttttctccacatgctaaacctgatttttttctataagatgatccacctctgcgcaagttatcatataaaaaacataatcgcatgccgccacgccaccaatggtttattttgtttattatcgtgaagaaattaataaaatagtatgactaaatgggagaatatcagggccgattacccggtatgcgataactgtacttatttttttaccaacggcggcggcccggtaagtaccccctttgtacaaaaggcgacagcgcttttcacggaactcagtgaaaaaggccgcggggtaatgcccggctgggatcaccaggccgacgaagccaaaggcctcatcggtgaaatgatccgcgcaaaggccagtgaaattgctttcatcaccagtacctcacaggccatgatcctcctgtacgggatgtttccaaaacactatgaaatcatcaccatgcgggatgaatttcccagcagctttgtgggctggatgcataacggtcataccgttcatttagtagacagtgatgaccgtaaccagatctccatagcagatattgcggctaaaatcacaccggacacccgtatcctcatcaccagccacgtgatgttcagaaccggcttccgtcaacacctgaaagccatcggcgaactatgcaaacagcatcagctgatccacattgtagacgccacgcaatcattcggcgtaaacgatattgatgtacaggaatgtaatatcgatatcctcatctttcacgcgtacaaatgggtaactgccggctatggcaccggcgctatgtatgtatcacggaaaatactggatcaatacccgccgcaggtgatgagctggtataatgtagagtatgaaatagcagatttccagtcggtaaaggactacacgaacttcactcctaaaaaaaccgccaccgcatttgaacccggcacgccgccgtttgtaaatatattactattgggagaagcactaaaatgccttcatcgtataggcattagtgatatagaggcgtatgtcggagagttaattacctacctggcgcaacaggcttcggcacacggtatccggctgctgtctgactatccgccggaacacctttctgccatacaactgctggaaattacgccggcgcaaaatgaaaaagttgaaaagaataatatccaggcgcgatataaaaataacatcctgacggtagcccttaacttctacaacaacaaagccgatatcgacaaattatttgccgcgctggccggggcttagagcgagttttgtcttggctcaggattacgctgattatactgattacctggatttttacttttggatttttttgatttttttaagatataactaagggagataacagcgaatatatccgcttctatctcccttaatcctttataaaatccaaaagtaaaaatccaggtaatcagtataatcagcgtaatcctgagccaggacaatttccgcgttagaaattgaaattatccgggtccggtcctaccctttcgccacggtccagtgcatcaatcttcagcacatcttctttactgatctcgaaattgaacagctgcgcgttggaaatcaccctgtcctggcggatgcttttaggaatggttaccacatccttttgcaggtcccatcttaataccaattgtgctaccgacactttatatttctccgcgagttctttcagcaatggcacgtcaaatgctttaccctgcatcaatgggctccaggcttcaaactgcacgttgtttttctgacagaaatccagcagggacggctgtaccaggtaaggatgaaattccagctggtctaccataggtattacctttgcgctttggaagagatcttccagttggtgttgcaggaaattactgacgccaatggcttttacgcggccatctgcatatagcttttccagtgcacgccaggtttccttatacttacctttcaccggccagtgtatcaggtacagatcaagatagtctgttttcagttttccaagggaggtatcaaatgctttcagggtactgtcgtagccctgatccgcattccatacttttgtggtcaggaagatatcctttctatcggtggcatttttttcaatggcaatacccactccttcttcattaccataaatagcagcagtatctatatgccggtagccggcatccagtgcataagtcactgaatcgatcacttcctgtccttcctttgttttaaaaacacccaatccgaaataaggcatctgtacgccattcgataattgtaccgtaccgttaatgtctgtaatattcatataatgaagattttattttactggttaaatgccgggaagccggtgaggcaaaattacgacgaaacaacatcgggccaccagtatatatgagagatatttttgtacaattaagagaaaaaggacctgctggcgctcttccctcagattagttttttcaataaaaaccacctatctttgcggtgcaattttaaaagtatatgaacaactatctcacatatcaggcatgcagttacgcaactaccgttatcagagcggtaattgcaagtacccgcattgtcttaattcaagacggggaggcaaatccatcccggatatgagaggttaatatataactcctgaaatctttttcaagggcctcttcatccgaagaggcttttttatttgcttcccccaatatcttcaacagtttctttagcaaagaataattcaacatgaacaccaacaggaaatttattattaaagcatcaatgtcatttacgcggctggtccggtaatgcagacttcctgttgcataaagcaaaggccgctcattaccagatgaacggccttttttaattcctttttaaataagaatatatgaaacgcttagcggattttagaaatataggtatcatggcacatgtcgatgcaggtaaaacaacgctcactgaacgcatgctttacttcaccggcttcacacataaacttggcaacgtagacgaaggcaacactgtgatggatagtgatccacaggaagaaaagagaggtattaccatttcttccgcagcgatcaccacctattggcaataccaggatcatacctggcagatcaatattattgatacgcccggccacgtcgacttcaccgctgaagtggaacggtccttacgggtgctggatggcgccgtagccgtgttctgcgcccgctccggtgtgcagccacagtcggaaacagtatggcatcaggcgaatcattataatattccccgcattgcgttcatcaataaaatggacaggcagggcgccgatttccggcgcgtagtaagcgatatacgccaacggctaaacgccaatgcgctgcccgtacagctacccattggtgcggaagatgacttctccggggtaatagaccttatcaccatgaaagcgctcgtatggaacaccgcagacggtaaaacatatgaaacgctggatatcccgtcggccctgctgaacgaagcgctggaagcacgtaattatttactggaagaattatccctgctggatgaatctttactgaataaatataccactgttcccaacagtatccttccggaagatatttacgccgcactgcgcggcgctaccatccgcctggaagcggtacccgtattggccggtgccgcttataaaaacaaaggtatacaacccctgctcgatgcagtggctacctacctccctgctccgtcagacatcggcgatgtaaaagccgccgatccagaaacggaagcaacggtgatgatcccggttagtgaaaacacgccgctcgctgcccttgcgtttaagatcataacagacgattacgtagggaagttaacgttagtgcgggtatatgcaggcgtattacacagtggcgatacactctggaacagtcgcaccggccgcaaggtcaggatcagccgcctcatgcgtatcatgtccgataaatatgaaacagtggaagaaataggcgccggcgatatcggtgcggtagtaggactgaaagatgtaaaaacaggcgactccctttcgcatccggatcacccggtattgctggaaaaaatcagcttcccggaacccatgatcggctatgcgattgaggcgaaatctgccaaggacaacgacaaactcggcgatgccttaaacaggttgctggaagaagatcctacgctcaccgtaacagtggataacgctaccggccaaacgattttgaaaggcatgggcgaacttcacctggaagtagtgctggaaaagctggcaacgcaatatcatctcgacatcaacaaaggacaaccgcagattgcgtataaagaaatatttacgcaggccattacccatcgtgaagtgtataagaaacaaaatggtggctccggcaactttgcggacatccagtttgaactatcacccggcgatgaacaggcaaccgggctggaatttatcaacgaaatcaaaggcggtgctattccaaaagaattcattcctgcgatcagtaaagggttcgagtccgccatgaacaatggcgccctggcgggctacccggtgaagtccatgcgcgtgcgattgctggatggttccatccataacaacgactcccacgccctggattttgaacatgcagccatcaccggtttcaaaagcgtagctgccaaagcagttccccgcttgttggaaccctggatgaaagtagaagtaaccatgccggaagaatttaccggtaccctcacaggcgatctgaacagacgccgcggtgtgatcaaacaaatggagatgaatggagccgtgcaaaccatcaccgctatggtgccgttgtccgaattattcggttatataacggtactgcgtacactctcttcgggaagggccgcggcatcgctgacattcgacagctaccagaccgttcctggtaatattaccagccatctgctggtgaaataaatgaaaatggtgaaggacaatccttcaccattattttatgcgagaaaaccatttcctattgcaacacctcacgatcgctgtgaacatcctggtaaaatttctttaccagccggctatctggcagggagtttaacacagcgataaaccatttgccgtctttcttcaccaccttgcccttataataaccgaccgacatcaactggatctgcccggtggtaaggtctgtccagaggttactggcatacatcgttacccgcaccgtatcatttgtgccgggataaaactgcatattggagataaggtgcctcgactggtaatgcgtattccggatactcagcaccagggaatccattttagcggtccagttttgttttccttttagctttaccccatcaatttccccgcggatgttatcatccataaactccacacatttatccaggtgaccgttgtcgaaatgctcacagaagccataaatcactttttcaatctgttgttgttcccggtatcccaggtcgcggatatggccaacgtccggggtaacggcagcggtgctgtcggcggtaattttttcttcgggagatgtgtggcaggaaaagaggcctatggtgctaagaacaagcgcagtggcaaacgggaaaaatctggacatctgataaattttatgatataacaaaacaaacgcataattagttttattatatcataaaattttcggtctataacggacacttctggtgataatcaattaattcaatcggcgtgttggccagttcaatgcctttataataggcttcaatctcatctaatacggcttccacttcttccacggttttcatggtcaccagccgggtgcggaactgtttgatatcaggtaaccctttcaggtaattggcgtagcagccgcgcatttcgttgattccctgcacagggcctttccattccaccgacaggcggaggtgtttcttacttacggcaatacgttcttccagggtggggccagccataatctcgccggtattcacataatgtttgatctcccggaacaaccatggatagccaattactgcacggccgatcataataccatctacgccgtaacggtttttatattccagcgctttctgcgggctattaatatctccattaccaaaaataggaatatgtatacgggggttattttttactttaccgatgagggtccagtcggcttcgcccttatacatctggcaacgggtacggccgtggatagccagggctttgatgcccacgtcctgcagccgctctgctacctcttcaatattctttgagtcgtcgtcccatcccagccgggttttcaccgtaacaggcagcttagtggcctttacgcaggcttcagtgagccgtaccatcaggtccaggtcctttagtacaccggcgccggcgcctcttccggctaccttcttcaccggacacccaaaattgatatccagcagatccgggttggtaacatccacgatcctggcagccatcgccaggctatcctcatccccgccaaagatctgtatccccaccgggcgttcatattcaaaaatatcgagcttcttcctgcacttcatagcatcacggatcaacccttcactggaaataaattccgtgtacatcaggtcagcgcccgcatccttgcacaccgcccggaaaggaggatcactcacatcctccataggagccagcagcaaaggaaaatcaggaagcgttatgttatcaatctttaccaaaatctatatctttttgcagaagccgcaaagataaagaattattacgcggattttgtctttctcgctgattacgctgattatactgattactttgatttgatcactttggattttaaaggattttggggagatataagcgatatattccgcttctatctcccgaaatcctttaaaatccccaaataaaatccaggtaatcagtataatcagcgtaatcagcgagaaagacaaactccgcttttccgcttctatctcccaaatcctttaaaatccaaagtgatcaaatcaaagtaatcagtataatcaacgtaatcagcgagaaagacaacatccgctttaattcgctaaatttacttacttttcgttggtataatctttggccccgcatcctaaatctttccgtatgcaaaaatttgacgccatagtaatcggatcaggtcaggggggaaatccgctggcaaaaaaaatggaagaaaaaggctggaaaaccgcgctcattgaacaacgctatctcggtggcacctgcatcaacgatggctgcacacctaccaaagcaatgatcgcctgcgcaaaagtagcacataccgtttttcatagtaaagactggggcattcacagccacggattcatggtggatctgccgtttattgtagcgcggaaaaacaatatcgtaacggaattccgcggaggaacagccaaaggattacaatcagataatgtaaacatcttcatgggaacagccgccttcaccgggcataaaacaattacggtgaccggctacaaaggagaagaagatatactaactgccgatcacattttcatcaataccggcaccaagccgtttattccccctataccgggcctggctgaggtaccctatcttacctccaccaccctgctcgatgaagtaacggttccgaaagaactgatcattctcggcggcagctacatcgccctggaaatgggacaactctatcagcgtttaggcagtcacgttactataatagaatccgcttctcaactggtatcaaaagaagatgccgacgtggcggcggtaataaaaaaaatgctggaatcggaaaacatgcagatccataccggtacacaggtaacgcacgtatccctcaatgggaaaaggatcagcatagacattaccaccggtaatgataaagatactataacgggcacgcatatactgattgcaaccgggcgcacgccacaaaccgcggcactgcagctccaacaaacaaatgtacttacagatgaaaaagggtttatacaggtaaacgaccgcctggaaacttcccaaccgggcatctatgccctcggcgatgtaaagggaggccctgcatttacacatatctcctacaacgatcatctcattatttataagaacatttttgaaaatgcaaacatcagtataaaagaccggcagataccttactgtatgttcaccgacccgcaactgggacgtatcggcatcactgaaaatgaagcgcggaaagaaggtatcccgtttaaaacagcatgcctgagtatggacaaagttgccagggccatagaaacggggcaaacaagaggttttatgaaagcactggtacatgaacacaccggtaaaatcctgggagccgctgtaataggcaccgaaggcggcgaaatcatgtccatcctgcagatggccatgctgggcggtgtcactgccacgcagatacgtgaaatggtgtttgcccatccgctctatgcagaatcattaaacaatctctttatgaccctggagaaacctgctccataatgagcaattttttccacaatctgatatataccgaatgatcaaactgtcgaatgtttccaaatattttggtcctggaaagaaagcagtcgatgatatttcctttgaagtaaaggaaggggaaacactggtactgctgggcaccagcggctgcggcaaaaccactaccctccgcatgatcaaccgcttactggaagccgacagcggccagatatttattaacgggaaagaaatacaggagctgtctcctgaaatactccggcgtaacatcggctatgtattacagaacaccgggttgttcccgcattacaccgtgagcgacaacatcggcctcgtaccctccctgctgaagtgggataaaaaacgtattcacgatcgcaccaccacgctgatggataaactccgtttacctgccgccacctacgcggaagtatatccgcagcagctcagtggcggacaacaacaacgtgttggcctggcccgcgcactggcggcagatccgccggtactcctcatggatgaaccctttggcgcactggatccgcttacacgcatcagtgtccggaaggaatttaaatcgctcgatgagatcagccacagaaccattatcctggtaacacatgatgtggaggaagcctttgaactgggccaccggatctgtctcatgaacgaaggacgtatccagcaactcggcacacctgcggaactgatcttccatccggccaacgattttgtaaggtcattcctcgatccgcagcgactgcagctggagctgaagtccctgcagataaaagacctgtggcaatggttgccatcttccactgctgctgcaaacgggcaattaaccgcctccagcacctgctgggacgccctggaagccattacgcaacagccggtagccgtaacatacgaacaggaacaaaaaataattgacgggaatggacttatggcggcaatagctgcctacaaaaattaacgcaacggcatggaagcaaccgaaaccttatttgaatttgtacaacaacaatccggtaaactgctggagcaaaccctcacgcacaccgggcttacctttatatctgtgctgctggccgtagccataggcgtacccgccggcattttcatcacccgtaaaaaaagactggcagcacctgtgctgggcttcgccggcgtaatgcaaaccattccaagcatcgccctgctggggttcatgatcccgctgctgggcattggccccaaacccgctatagtagccctgtttctttatgcactgcttcccattatccgtaatacctacaccggtatcagcggcgtagatcccaatgtaacagaagcagctaccggtatgggaatgagccgcaggcaaatgctgatgaaagtacaattgccactggccatgcccgttatactggccggtatccgcaccgcaacagtgatcaatgtaggcgtagccaccctggctgcctacatcgccgcaggcggactcggggaatttatcttcggcggcatcgcactcaacaacaccaatatgatgctggcgggagccatacccgcagctttactggcattgctgttcgactggctcctgtcgctgctccagcacatcaatatccggaaagcccgtaaaacattatacgcactgccttttatcttcctgcttctctcctctttctatcttttgcccgatacctacagcggtaaaatgctggccggattcacccccgaatttatgggcagaaaagacggtaacctcgggctaaaatccgtatacggcctgcatatccgtaccctcgtcatcagcgacatgatcatgtataaagccgcctacgaaaaaaagctggacgttataagcggaagcagcacagacggcagggtaaaggcttttgacctggttgtactggaagatgataaacatatttttccgccctattatgcagcccctattgtacgggaagaaaccctgcaacaatacccggaactggaaccggcactcaacctgctggttggtacaattaatgatagtatcatgacggaattgaactaccgggtggactatcttaaacaaaatccggaaaaggtggcaaaggattttcttgttgccaggcaactctggaaaccagccggcaacggcgctaaaggcactatccgcatcggctcgaaaatttttggcgacggttatatcctcgccgccatgtacaagatgctgatcgaaggtcataccggtcttgctgcagtcaccaaaacaggactcggcggtacaaagattgtgttcgacgcattggtaaacgaccagatagatatgtacccggaatacaccggcaccggtttgctcgtattactccaggcgccgcaacaggtcacagacagcattatcggcgacagccagaaagtttacgactatgtaagcgcagcatttgaaaaacaatatcgtatcaaatggctgcaacccatcggatttaataatacctacgcattaatgatgcagagagccgcagcaaaagaacggcacatccgcagcatttctgattttacaaaatatgtgaatcaacagtaagcacctgtaattatgttactgaaagaacaatatgaaacagtacggcggagaagcgaaaaaatttgcgccccgctaaaaacggaagactatgtagtgcaacctattgtggatgtaagtccgcctaaatggcacctgggccacaccacctggttttttgaaacatttatcctgcttcctaacgctaaaggttacacggtttttgatcctcaatataattatgttttcaacagctactatgaatccgttggcgcacgggtgatccgcaccaatcgcggtaacctgagccgcccggcagtggaagatatcatgcgctaccggaagtatgtggatgaagccatgacagattttttgaaagaagaactgtccccggagctgcaggagctgtttattctcggactgaaccacgaggagcagcaccaggaattactgtacacggatattaaatatatcctcgggcataatcccctgttccctgcctacgatattcatcataaagatatacccatagtgaacaatcccggcgatacctggttaaatatacgtgccggcgtatatgatatcggctttgcaggggacggattctgttttgataatgaactgggcaggcataccgtatatttgcaggattataaaatcagtaccacgctggtcaccaacacggaatacctggactttatccaggccggtggctaccaggatttccgctactggcacgcggaaggatgggactgggtaaaaaataaccaggtaaccaccccgatgtattggtacaacatcgacgggaaatggatgcattatacctggcaggggcttcagccaatcatgccggatgcacctgttacgcatatcagctactacgaagcggctgcatatgccgcctggaaaggacaacggctaccaacagagtttgagtgggaagtagccgcaccgcaactggcatggggccaacggtgggaatggtgcgaaagcgcttatctcccctaccccggctttgcaaaggcgcccggcgccatcggtgaatataatggaaaattcatgatcaatcagatggtactgcgtggtggctctgaagtaacttcgcccaaccatagccgtatcacttaccgtaattttttccatccttcactgagatggcaatttaccgggataagattggcaggatgattgagacaacgttgtgaaatgatccggatctccggaaaatagcttcgctgctttccgtgaatccaagttcagaacatcaaaaaataattatgactgtaattcctaatgtacttgcgccatgcaagcgcaaaccggccaccgatatattttatcacgacgtggtgcagggcctcactgcaccccagaaatacctggacccgaaatatttctatgatgcggcaggagatgccctctttcagcagatcatgcagtgccatgaatattacctgaccggatgcgaaatggaaattctccgcgaacagtctgcgcaaatagtacaggcgttacagttatacgccggcgattttgatgtggtggaactgggtgcaggcgacgctaccaaatccgttcacttgctgcaacagctgatcaataacggcgtcgattatacgtatttccccatcgacatttccgccaacgtgatcacgcaactggaaaagaacctgcccgcgcaggtacccggcctgcaattgcatggcttaaacggggaatatttccatatgctgcagcaggccaataaggtgaccgccaaaaagaaagtattgcttttcatgggcgccaacatcggcaacttcagcgtgagcgccgcccgtagcttctgccagcagctgcggcaatatatgcagcccggcgatctgctgctgacaggcttcgatctcaaaaaacatccgcaggtaatcctgaatgcatataacgactccgccggcatcacccgcgcgtttaacttcaacctcttacaccgtatcaacagggaactgtatgcagattttgacacctcaaaatttgaacacttccctacctacgatccggttaccggcgcctgcaaaagttatctcatcagcctggaaaaccaacaggtgcacatcggggaggatacgaccgtaaattttgcagaaaatgaatccatttatatggagatctcacagaagtacagcctggaagaaacagaccagctggccgcctatgcaggcttcaggccggtggcccggttcttcgaccgcaaacactggttcaccgattgtttatggaaatgtatttaatgccaggcattcagcattcttctgacagctacaatctcaccggtgtgataactggtgtgatccagcaacaatacggcttcccggaataagtgctgcccggtgccatgcggaaaaggcgcaaacagatcatcgctctgttccagcaggtcaataaaggcatgcaggtccttatccacctgctccacgctgtgcttccatgcggcatcgtccttcggagcagtttcctccggccagtaggcctttggccactcaatttccttatagtccgggttcctggagaaatcgaggatatcatattgcgtaatcctgatatgctccaccaattgccagatgctgtaaggcataccggcaggtaccacccccctcagatcagctggcagcttttttaccgaatcgctgaaagtgacgtgtgcattgggtttaagcaacatgtccttcagcgatttaactaacgtagcagtattcataaaatagtaattttatttgtcggggttcaaagatcaaaaaagaaagacatctcatcaaaaaatactccaataatcatggccccggcatttgtgaatcaattgttaatctcgttatcttattaataattctttaaccattctgacaacatttggtattgattaacgggatgaggatgcttccatactatcattgtattgaaataaccaaaatcctcgcatggcaaaatactacgcattatcgttaaccgtactgctgataggaatgcatttcacgctttccgcacaaagagaaataaaaggccatgcgtatgataaagatacccgtaaaccactgacaggagcaaatgtactgctcttcaccgcagaaagatccattcttaaagcacagggcatcacgaatgaatccggcgactttatcctcaaaaaaataccacagggaaattatgtgatcacgatcagtttcatgggatacgatgccgctacctcgctcatcatgatatcagaaaagtcagccaaggtattccaggtagaccttcgcttttccggtcttcagcgtaacccgatcaaactaaacagcgttaacgtaaaagtaaataaatcggcattcaccatacgaaaagatactgttgaattttctgcgggcgatttccagacaaccgaaaatgcttctgtaagaagcctgctcaataaactccccggcatcaccattgatgccgatgggaacctgtctttccagggcaccgctatcaaaaccatcctggtaaatggcagaccgcttttccaggatggcaatagtgcaacaggcgacaccaaaaaaataacgcagaacctgctggcggatattgtcgataaaatacaggtcatcgacagaaaaagaatagatggtatggtggaaggtggtaaaaatgaaaaggtcatcaatatcaccgttaaaaaagaatataagaaaggattcaatggcactgccggcgcaggctatggaactgacaaacggtataacgccgccgccaacgttaatatgttcagggataccaggcaggcggtggtgatgggatatatcaataatgtcaattcctcccgcggccctgcttccaccgatgaaaacctgagcaggggagaaagtatgatgggcggcctctccaggaaaaataatgtcagcgcgaatcttggtaccgatatctccaaaaaaataaaactcaacgccaacttcctccatcaaagccaaaacgtcaataacagccagcagcaacagcgcgacaacgtacttccggacagtaacttccgctacaacaacaacaatacctcgggaagcactgccaacatgaatatcctctttaccaacctgagcatccaggtcgatgaaaaaaatcttgtctccatagatatgtcggccaacacacaacataacactttccgctccttcaatcaatacgtttcaacaggcgggaaaagcaatgacacgatcaactttggcaacaccaataacctggaaacaagaaggaataatgttatcaacctcaccacccaatataaccatcagttcagtcccaaagccggcagtgtaagcatatccttcaatattgatcagaacaatacaaaagatgaacagcagaataccaccctgaatactttcgccgccacaaacctggcagacaccatcaaccagcaggtaaatgcaaaaataaatgtcaggcggctgatggccaggtttaactaccaatatccactgctcacttccatgtacctgaacgtatcctataaaataaccaacaacctcacaaaaaataaccaggacgctttcgatttcgataatgaaaagaaaggatatgatcttgttaaccaggacctgacctaccggttcaaaaacaagatcaatgagcagtcggttggtgcaggactctttcttaataaaacaaaaatacagggccagttaaatattgcctataacttcacagattcaaaaagcaacaacttcaccgccggcaatgagttcctgcaaaggattcattacctgtctcccaacctgtcccttttctataaaatagataactacaaaagcctggacctgagggtaaacagggaaacccgcatccctcctcccaacgtgtatctgccggtagtatctacccggaacccgctgtatgtgcaactcggcaacccggatctgaaaccgtctatttataactctgccgccatcggctaccgttccttcagcgtgaaaggccttacgttcagtaccaaccttggcgctgatttgccaaataatgccatgacacaatccatctactccgactctgccggccggcaaatcaataaaccagtaaatgtggatggaaattttagttttaaccaggacttttcaataggtaaaagattcagtaaacccgccttaacacttaactattcattgtcctattatttcagccggaataattcgtttatcaaccaggtcaaaagccgcactactgatctgagtatcacacaaatgctgaacggctcctggatgtacaaaaaaacgctggaactggaaggatttgtaagcatgctgtatatcagcagcgtttactccatccagaacaacaaacattccgactacctcatgtacaatgtatcactcaccgccaacgtttttctccctgccaacctcagcatcggcagcgcagccctgtatttcaataataccagtcagcatcagcaatttgtagtcctcaacagctggatcgccaaagcctttggaaaagacaaaagcttccaggcaaaactctacgcctatgatctcacaaaacaaaatcaatcgctgctcaccatgcaatcccccacctacatagaacagcagcggaacaccgttctcacccaatacttcatgctaagcctctcctggttcttcggcaaaaaaccagcggcgaagcctgcggtgtaagcatcgccttcggcgatggaaattgtcttggagcaggattacgctgattttactgattagttggattttaacttttggatttttttagatttttagattaatataataattaagggagataaaagcgaatatccgcttctatctcccttaatcctttataaaatccaaaagtaaaaatccagctaatcagtaaaatcagcgtaatcctgagaaagacaaccttcgcttaattcgctggtttttccagtaatttgaagaactgatccaactgtggcagtattacgatcctcgttctgcggttggctgctttgccttcagcggtgtcgttggaagcgataggcaggtattcgcttctgcccgcagcggtcatgcgtgctggcggaatgttatactggttctgcagaatacgtactacggaagtagctctcttcacactcagatcccagttgtccagcaatatattcggacggtaaggcacgttatcagtatgaccttctaccatgaattcaatatccggctgggcaatcagcactttggccactttacccagtacttccttggctctttcattgatttcgtaactaccgcttttaaacagcagcttatcggagatatctatatataccacccctttgtccactttaatattgatgtctttatcatccatatttccaatggcgcctttcaggttcatcaccagctgcatgttcagcgagtctttacgggcaatagctgattggagatctttaatataagcatccttggcgccaatattatccagggatttcttgatgctttctgcctgggcgccggaaattacggacaactccttcaggtgatccagcatctgggtattgttggttttcagttgctgctgttgctccgttaaatttgtcactttttctttgtacgatgcagcggcacgggcggcatcttcttcgcaggttctcagcttaccgtaggtagcgcggtaaagactatcaagttgcgcattcctggcctgtgattcccttaatttacgaggggcagaacaggatgcaaaaatggttactaaagctaccggcaaggctagttgtgctattttcataaaattacactttttaataatctaaagaataagtatatataaatagtggggtatacaatggaaagcaacccctgtatagcaaatagcaggccgaagcccccttcagtccgttagaacccggttagaatccagcgtggtattagatgttgacacgcataaaaaaaataaagccgtcatcctaaacaagctttattcataaaaaaaagctaatgttttccaatatctaagtaacttgtccggcagagtatacgctgtatctattttctattaattgctgaaatgtatgagaaaggtggtttcttcgggtcaaccaacaataaaggaaattgcaaaaaggctgaacatctctgtatccacggtatcaagggcgttacatgatcatcacagtataggtttaagaactaaaaccagggtaaaagaactggcggccgaactgaattatgaacgcaaccagacagctatctatttccagcagggtaaaacatttacaatcggtatccttttacccgagctgtcggaggcattctttgccagcgctatcagcggtatcgaagacacggcatacagcaataactacacggtactgctgggacaatcacacgatgatgaagcccgtgaaaaacagatcatccagagcatgaaacagcaccgggtggacggctgcattgtttctatcggaaaaaataccagcaattacgaacactttgaaatgctgcaacaggcaaggattccggtggttttcttcgaccgcattcccaaccttcctgatatgcacgcggtttcctgcaacctggaatccggcaccgtacaggcagtggatttcctgctgaaacagggccaccgcgtaattggtatgatcaacggccccgaaacaatggtggccagcaaggaacgtgctaccggctacatcagggcactgcagaaacaccgccttaaatacgatcccaaaatgatcgtcaacgccgacctcaccgccgcaggcacagaacaagccatgcagtacctcctgtcgctcaaaagaaaagtaacggccgtcgttactttcaatgactatgtagccatggatgccgtacagtatgccctgaaacaaaaattggaaataaataaggatataacttttgtatcttacgccaatacaccggtaagcgggtatacagcctttccccctgctgcatctgtggagcagttcccttatgaacagggccaggcggctactaatatgttattatcactcctgaacggagaacatgccttgaatgattttcaacgcactgtcatggagtcgcaactggtgatacatcaccgctgaggcattatcttatcgataaccttgccacagtagttgaccgtggcaggttattcgacttcattgttcgctgtctataattgctgcttttccagcttagttcactttctgattaattgctacaacgattctacatgatttttttggcattccatgtacgcaaacgcttgcgttatccgcgcaagcgtttgcgtaaagcctgttttcgcttgttttagctattgttgcaccacccacctgttcaccgtgtttaacggcccttccaatacaatcttgtaaaatgaggatggaagcgattttacgctgatgctggcgccttcttttgatacaggcacctctcccagcagcttatattcatcgtgcccgccggttttataatgattagttgtcgtaacccatatttttacgcttccctttttatcataagctttccatcccagttgcaactgatccttcactaagctggcagtaggctgcgccagtgaaatagcgcctgtcagcggcacgccatccagttcacgcgcattctccttaggaatagagatattcataaaccgcgcaatggaaggcaggatatctacaatacccggttgcgccgttttaaagtaaggattcaatccttttgcattggtaacaatccaggtagtccgctcacgatccgattgcccgccgtggccatgtccgccatgcgcatcacgaccgtgatccgtggtaatatagatctgccagtcttcgttgaaatttgcacgcctgtattccatcgcatcccagatcttacccaccatgtcatccgtcatccgcacggcagtatccagccgctcaccggtaccataacgatgccccatgtcatcgctgtattccaggtatacccaggtcatatcaggcgcatcgcttcttacaaaatctgccgccttattcaccaccgtttcatcaataagatgaatataccagctgtctttatcatgcggaaaccgcacggtatcaagctccagtccatccaccgcgtggtcaatatgcaggttgcctgtttgcgctaatccatctcccaccagtttggtacggttatccagccaggtggaaaaaatagccgtcttcttttcaggataagccgatttaaaaaaccggaaaatgctgggataagcataattctgcgcggcaatatcattgtcccatacattatgtttattcacccaggtgctggtaagcaaactgttgtaacccaccgctgaaatagtaggcgtctgcgaataaccattcttctctcctcccacgtaagcacgacaatacccgccttcctttgctatgcgcttcaggtttggagtgggctgcgactcaatcacatctgccggaataccatccgcaataataaataacactttgtgtttcttctgctgtgccgctaaagtggtaactgttaagaggctcatagcgaggaataaatacttcatcgttgactgtttaagattagctgatcgcaattagcataaaataataaagcgaagataacagcgaatattaatttttcgctatgatcttcgctttaaaaagaaatctaaaaaactatttcagatggacgtcaaaatagtcggtgatcttctgcatcaggtgaaccctgtcttttcccaatacattatgtaaatgccccggatatacgaaataatctacctgtacttcattatctacacaggctttcaggaaatccagcgaatgctgccaaactaccacatcatcgttggtgccgtggatcagcatcagtttaccctgcaggttttttgttttggtaagcaggttggaattggcataaccttccgggttttcctgcggcgtatccatatagcgctcggtatacataatttcatacatgctccagtcgatcaccggcccgccggctactcctgcctggaacacgcccggatgacgcagcatcagcgatgtggtcataaaaccaccaaagctccagccatgtacacccatcttctgctgattaatatacggcagcgacttcaggtaagccacgccctgtaactgatcattcatttccacagtaccaagctgccggaaagtggcctgttcaaaagcctttccacggttatcactgccgcggccatccatcgtaaaaattacgtagccatgttgcgccatgtattcataccaaaggttaccgctgtagggataagtgttacggatcaactgcacattaggcccattatagaggtatacaattaccgggtaggttttggtagaatcaaagttcaccggcaggatcagtttaccgtataaaggcgtgccgtcatccgctttcagtgtcacctgcctgatttgcggacgctgaaagtctttcagcggatcggtggcggtgataatattttgttcaaatttaccggcggtggcagttacccccgctacatacggagtggtaccggaactgtaagcatccagcacatagctgccatcggcgctggcctgtgcatcgtgccagcccgcagctttatcgagtgcggaaagcgttgctgtttgctgcttgtaattaatcttatacaaatgtttctccatcgggctttctttggaagccgtgaagatgatttcatttttcttcggaataaaacccgttagttcattcaccacccaatcaccggtggtaatttcccgcagttgttctcctttggtattatagagatataaatggttatagccacttttttcgctccaccagataaactgatcggttgtgccgggaacaaaagttaacggatgggtaggatgtacgtatttagcatctgtttcttcaaacagtgtttttaccagttccccggtagccgcactgtattggttcagccataaatgattctgttcgcggttcagcagcactacataaacagattgctggtcaggcgcccaggtaacacatgtgagataatgatctgcaggcccgccggttttcaggaaaatagttttttgggtagatggctgataaatacccagcgttacttcatgtgatttaccacccgccatcgggtatttgatattggtattatgcgcgggcgttaccgaccagtcgataaccgggtaatcatttaccatgcgctgatccatgcggtaaaatgccagctgatcacctttgggagagaagaaaatacctttgtcgatgccaaattcctcacggtgaacgctttttccattcacaatattgatatcggcgtcgttggtaactgcctgtacatggccatcgtcggtacggataaacaggttattgttttcggtccaggcaacctggccgctttggttgttcaccgtcacattctctgcttctttgggtaattcgcaccactggctgaattgcatgatgccattttgcagttgacctttatacagcgtgttaccgatagaaaaccaggcactggtagaagacatccagtgcagcggtggcacaccgcgtaaaggtttggaagaaaataactgttcattgagccgtgaaagtgtcagcagggtatctgttttgccggcgggtagtgctaccttgatccaggcgtaattatctttttccgatagtatcctggtgtaggcgttttcaccaggcacccattcaaactgttttaagcgctccggtgccagttgctgccgaagcccgttagtggcttccgccatggtatactgacgttgctggccataggtatattgcagcccacccgtcatccatcctgtcaaaagcaataggaaagctttcttcatccttctttttggggagctaaattaaggttttacccgttacgcgctcacaagatgttttttaacccattccctttcttcgggcaacaggtagtcggcccgtttctctgtaatccaggaaaatgttttcttcacatctgtctttgcagttctgaaacggaacaggaattccatgcccagcatcaggtctgtaaagccgttcttcaccgtttctatcgtcatccgggcgctgctgcgtctttttgataacaactcggtaatgcgggcggtcaccgcctggatcgcattctcatcagcgtacttataaatggcttccatcgcttcaaatttgagttgtccacgcataaggcagcgtgtataaaacatggcttccttctctttttcaatgtcagcgatagcggcgaaagccaggctttttacatcctggcggtgatattccaggagcctgcgcagtgcaggcacacttttctgcgtacctactttatgcagcagcagggtgatataatagatatcgtattcgtttacggtgcgcttcagcaggttcagggcccagtcttccaccgaagggtggcgggtacctctgagcgccagcagcgcagagcggcggatattattattgagtgaaagcgtgttattaaacaacggttccaggttaatatagcctggtatggcgagtccccgttccaggtcctgctgcatcgcagtgatcatatcggcatcctgttccattttaagccggtccaaaagaaaacggatcacttcggggtcgttggtattcctggaaagctgggtgataataaaacaggcggcgcggcgcttatctttgtcgggctcctgctcaatgtattgataaagtaggggtatataagcgtgattagcgagttgttctgcttcgcggagggcctgccagctggtcgtctggccattatgcaattgttctgagcggtcgcatatccgtgctacgaggttagaaagatagtcaatcatcagtagttattttgatctgctacccctgcattttcaattatcataccaacctgaacagccgtccgaaaagtagggggccgctccccttcaacaattaacagttttatgttacatttgcccctgtattttcggaccggttatagaacgtaaagcatgcacatactactcaagaacgtaaagatcatagcgccttcctcacccttacacgggcagcaaaaagacatttctattcagaatggcatcattcagcaggttggtaacaacctcgaagatgcccgggcaacggtcatttcaggtgataacctgcatgtttccgctggctggatggatgttttcgcacatttctgcgaccccggacaggaacacaaagaggatctgcaaagcggtatcaaagctgccgccaccggcgggtacacaaccgtaatggtggtacccaacacccagcccgccctgcataccaaaccgcaaatcgaatacgtactgagcagaacccgtcattcggccgccacggtgttgccaattggcgctgctacgaaaaaccttgagggtaccggcctcgcggaaatgtacgaaatgcagcaggcaggcgctgtagccttctccgatggcctcaagccattgcagtcgcccggcctcatgctcaaagcgctgcaatacatcaaagcattcgacggcacccttatacagctgccggatgaccagagcatttcttcgcatggactcatgcacgaaggcatttactccacccagctgggaatgcccggaaagcccgcactggcagaagaactcatcattcaacgcgacctggagctggcgaaatatgccgactcccgcatccactttaccggtatcagcacccgtaaatcagtggagctgatcgccgccgccaaagcagcaggaatcaaagttacctgctcggtaacaccttaccacctgtctttaaccgatgctcaactcatcaactacgatacccatctgaaggtaaatccgccgctgcgcagcgctgacgatgtgaaagccctgcaggaagccgttttacatggcaccatagattgcattgctactcatcacacgccgcaggactgggatgccaaacaggtagagtttgaatatgccaaaaatggcatgatcggcctggaaagcgccttcggcgtaataaggcaatacctgcctcagctgccgctggaacagctgattaacatgctcaccatccacccgcggaaaatattcggtttgccacagccggccctgcaggaaggcgccgccgccaacctcacgatctttgatccggaagccagctggcagtttaccaaagcccatatcgcttcccggtccaaaaattcagcgtatattggcgaacaactgaaggggaaagtacatgccacagtgaatggacccgtatttcatataaataattaacctatatgcagaaaagttctaacccaggcctgttatggggcgtagtgggaggcgtatctctggtattcctgaacgtgattacttacatcgccggcccatctgtattgtttgcatggtggaacagcatgttgcaactggctgtatttatcgttattgcaatattcgccggcctggaagccaggaaacaacagggagggtatattagttttaaagaagtactgaaacctgtgttcacggcgtttattatcggaactgccatcattaccgtgtaccagtatatcctgtataagtatattgatccaacactggtagatgcactgaaagaaaacctgctggagtctacagaaaagtggatgcacaaattcaaagcgccgcaggatgaaattgataagcaactcgatgaattaagtaaaaccgacttcaatgttggtattaaaaaatcattcctggacttcctgaaaggaattatattctattttgcagtgtcagcgattatttcgctgatcttacgcaggaaaccggctgaaagaccactttaataatactattctattaagatgaacatatccgtaatcgttcctttaaaaaacgaagaagaatccttgccggaactcgcggcatggattgaaagagtgatggacacacaccatttcacctacgaggtatggatggtagacgatggcagcacagacgactcctgggccgttatacaacaactggctgcgcagaaccccctcataaaagggatcaagttccagcgcaactacggcaaatccgcagccctcaatgaaggcttcagcgcggcacagggcgatgtggtgattaccatggatgccgatctccaggatagtcccgatgaaataccagaactctaccgcatgatcgtggaagaaggcttcgacctcgtgagcggctggaaaaagaaacgttacgataatgcttttaccaaaaaccttccttcaaaattatataactacaccactacccgcatgagcggcgtgaaactgcacgacatgaactgcggtctgaaagcctatcgcaaaaaagtagtgaagtccatagaagtatacggggaaatgcaccgctatattccggttatcgccaaatggaacggcttccgcaaaataggggaaaaagtagtggaacaccgcgcccgcaaatatggcgttaccaaattcggactggaacgttttatcaacggcttcctggatctggccaccatcatgtttatcggcaaattcggcaaacgccccatgcacctcttcggcgcactgggctccctctccttcttcgtagggtttgtgatagctgcctatctcgcactggcaaagatattctttgataaagtaaacatgacagacaggcccctgttctatttcgggctgctttgtatgatcatcggttcccagctattcctcaccggttttatcggggaactggtaacacgcaacgccacggaacgtaattcatacctcgtggaagagcggatggaccataccagtaatgttacggatgaagagttgcagttagcacaccaacacaaccgcagacgctgatccgctcattcattatcgttatctgaatctatggctgacaaaaagaaaatacttattttaggtacagcctaccccttccggggtgggctggctgcttataacgagcgactcgcagaagaactccagcaaacggatgaggtggaaatatggacctttaccatacaataccccaaattctttttccccggaaaaagccagttctctaccgaccccgctccggcgcatctgcgcatcaaaagattgatcaactccgttaatccgctgaactggttaataacaggccgcaagatccggaaaatgaacccggacatcatcatcaccaaatactggctacccatcatgggcccggcattaggctccctcctgcggttaggcaaaagaaaacacaccaaagttattgccgtactggataacgtagtaccgcacgaaaaaaggcccggtgatgtagcttttacaaaatatttcctgaaaccggtagatgcctttgtagccatgagccaatcggtactcaacgacctgcgggtatttgagcccgtgaaaaaagcctcgctcattccgcatcctatctacgacaactacggcgccctgatatcgaaagaagatgcgcgcgcccagctgaaactgaacccgggcaaaaaatatatcctcttctttggcttcatccgccagtataaaggactcgatctgctgttgcaggcaatggcggatgaaagactgaaaaaactggatgttcacgccatcgttgccggcgaatattatgaagatgcagccccctacctggaactgctgaataaattgcaattgggcgaccgcgtgctgatgcacaccgatttcattccgaacgaagccgttaaaaactatttctgcgccgccgacctggtggtacaaccctataaaagcgctacccagagcggcatttcacagatcgcctatcacttcgaaaaaccgatggtggtaacaaatgtaggcggactcgtggaaatggtgccggatggcgtagtaggattccaggccgaaccggaaccagcctctattgcagctgccatcgaaaaatatttcgtggaaaaccgcgaagctgatatggtggaagccctccgcaaagagaaactgcaatattcgtgggcacggctggcaaaagaaattcatacgctggcaacagatcgctgatgaatatgccggtgatagacacagcggcatcataattgttgactacatggccagcaaattaaacctgacaactagcatgatttacagaagtaaagcacctttacgtataggccttgccggtggtggcacagatgtaagtccgtattcggacttatacggtggcgccattctcaacgctaccatctccttatatgcgcgcgcatccatagaacccctccagaacggacaagtggtttttgattgcgccgacagaagggaaaccgctacttatgatgccgtataccctttaccgttagacggaaaactggatatcctgaaaggcgttattaaccgtgtgcaaaaagattatggctccttaccatctgctggttttaaactcaccacctttgtagatgcaccggccggctccggcctcggtacctcctccaccctcgtggtggccgtactgggcgcattcgcggaatggatgaaattaccgctgggggaatatgacatggcgcacctcgcttattctattgaacgcgaggacctgaaccaggccggcggtaaacaagaccaatacgcggctacctttggcggcgtaaacttcatggagttttaccagggcgacaaagtaattgtaaacccgctgcgtattaaagaagtaaatcttcacgaactggaaaataacctggtattgttctatacatctaccagccgcttatcttccactatcatctccgaacaacaaaaaaatgtaaccgataaaaaagatgcttccattgaagccatgcaccaactgaaagaacaggcggtgatgatgaaagaagcattactgcggggaaccatcgataaaatcggtgaaatcctgaactacggttttgaaaataaaaagaagatggcccatggcatcaccaatccccagctcgatgaaatttacgaagctgcccgcaaagccggcgccagcggtggtaaaatttccggcgccggtggcggcggattcatgatcttctattgtccgaaaaatacccgcttcgccgtagtagacgcactaagcggttttggcggagatgtaaaacgctatacctttaccaatcacggtattcaaacgtggagcatttaagggcacaacaaatcaaaaatatctgctgatgaaacaattcattgccaataagatccgggaaagcatcgctgtaaaagaggccatctgccaggatgaaccgttgttaaataccatcaaactggtagcagaagccattacccacagcctgcaaaccgatcataaaatccttttctgcggaaacggcggcagcgccgcagacgcccaacacctggccgcagaattctccggccggttttataaagatcgcatgcccctgtatgcagaggcactgcattgcaatacttcttacatcactgcggtaggcaacgactacggctacgatcaggtatatgcccgcatcctgaaaggcataggccgccccggagatatactggtaggcatttctacctccggtaactccgctaatatccttgaagccataaaggtggcaaaggaacagggtatgattgtagtaagcatgaccggcgccaccggcggcaaaatgaaagaaggcagcgactacctgatcaacatcccctccggcgatacgccccgcatccaggaagcacatatcaccgtgggacatattatttgcgaaatagtggaaaacaacctgtttggcgcatgacgagagaatgtatcgtactcgccgggggactcggcacccgcctcagaagcgtagtggccgataagcctaaatgcatggcccccctcggtgaacgcccttttttatattacctgctgcaatacctgcataaacagggcattaaccacgcggtactgtcgctcggctacttgtctgaacaggtcataaactggtgcaacagcataacactcccgctgcgtgtatcctttaccgtagaaacggagccgctgggaaccggcggtggcatcatcaatgccctgtctgccgtgaaaggcaatgagatcttcattattaacggcgatacctattttgatgtggacctcgcagcgtttaataattttcaccaggcgcatcaaagcccactgtcactggcgctgaaaccaatgaaacagttcgaccgctacggcagtatccagctggatgaacatcagcagatcaccaggttccatgaaaaaaaatattgtgaagaaggactgatcaatggtggcatctaccgcacttctgccggtttcctgcaaagcctggccctgccggagaaattttcttttgagaaagaagtactggagcccggcgcacaggcaggaaaattatatggcttcatcagcgacacctatttcattgatatcggtatcccggacgattacgaagcagcaaaaaaagtattggtatcatgaccctattcctcgacagagacggtgtaatcaacgatgaaatccacgatggatacgtgctccggccggatatgtttcacttcagtgaaggtgtactggctgcaatgcccatcctcgccagccgtttcaaacgcatcattgtaatcaccaaccaacgctgtatcggccgcggattgctcactacagcaggcttacaggaaattcatacacaaatgcagcaacagattgagctgcacggcggtaaaatcgatggtatctatttctgcccggatgtagacagcagcagtccatgccgtaaacccgccaccggcatgggtattcaggcaaaacaggacttcccggatattgatttcagctcctccgtcatggtaggcaacacccttagtgatatgcagttcgggaaaagcctgggcatgcaaaccatctttatcccgtctacccgtccggaaataccctttcctcacccgctgatcgatcagcgatatcaaaacctgctgcagtttgcacaggcggtacaataattctaagccgtaaccgtataatagatatggcaaaaaaaacactactgtcactgctcttcgtctttacctcgctgctcaccctggcgcagcggccggatgccgcagggctgaaacagttaatgcataaccaggataccctgcaggtgctcagtcaggatatcttcaacggaaaaggcgacgaaggccggcaacgggctacagaagccttcattccgttgctggtaagaacactgaaaacaaaatactccttccgttttccgttcgattccctgaaaaccatctctattcaatatccgcaggatagcgccttccgtattttcacctgggcactggaacgcgaaaatggcttctaccggcatttcggggccatccagatgaatactcccgatggacagctaaagctcttccccctgtttgatgcctcggattatatgaccaacaccgataccatcggcgataataaatcctggtatggctgcctctattacaatattgtgcaccgccattatttcaacaaagaatattataccctctttggctgggatgccaacaatccccgcagccagaagaaaatagtggaaatgctcaccttccagaatggtacacctgtattgggcggcccgttttttagttttgcggaagatagcacacccaaacccacacgcaaccgctttatcattgaatataaaaaagaaagcaccgccacgctcaactataacaaggaactggacatgatcgtattcgaccacctcatatccgaaaccaatgagcccatgaagaaattcacttacgtaaccgatatggactacgaaggcttcaaatggcaggccggcaaatggatgcacgttaacaagatctttcatgacgccatcccgctcggaaaaggcgctcctaccccgcaaccactggatcagaaaaagaaaagtatgacccagcctaagtcggcagaagatttccagcaggaatcacccaggaaacccgcatcaaagaagaaacaataaaacattcacatggcagcaacggacaacgaatcaacatacatcagggctatcaggctattcaataccaatgaaacagattgttcctttgaaaccggtaagatcccaaccaggaacaaaatcgatgcgaactatttcttttgccagacaggaaccggtgagctggaacatattccccaccccgccccgcggcggcaatttgtgataacgctgaaaggtaggctccaatttaccgtcaccaacggcgatacctttatccttgaacccggcattatcctcatcgctgaagacgtgaacggccccggccatacctgggaggtaaccgacggcaatgaatgggaacggatctacatccctgtggacggggaaagcaatactggcttcctcgccgatcccagctaatactggtcttaaaaaaaatgcgctttttttctttaaaagaacaatcattctcttatatttgcatttaaaagagcgaacattcatttatcatctacactgcaatgcaacttaatcacttaaacctcagcgtcaaagatgtaccggcaacccgggcattatttgaaacctactttgattttatctgcgccgacccaaaactaaacgataccctgtctgttttaaatggccccgacgggtttatcctggtattgatgaaccaacgcatgaatgagaaaggaaataacacctacccggatacttttcacataggattttatctggaagataaagccgcagtaactgccacctgggagcgactgcaaagcggaggtatcgtactggaccaggttccgcagatcatgcgtaagaactttggcttttactttactttcgacaccttcatgatcgaagtaaccacccccatcaaagattaaaaacaattttatgcaatccgaaatagaccaaaagctgcccatcggctggtacctgaaagaagccgattgtctcatcactaatttcaccaatgccgcctttgaatcctttggcatcaacaggtttcactggcaggtattgaaaaatataaatacgcacggaaagatctccaaagacctgtattaccaccaggtaagccgcttcctcaccgttgcagagctggacgaaatactggaaacattgctctcacgcaactggatccaacatgctgatgatctttattcctttacagataccggcaaacaggagtacgctgccatcgacgcgctccaaatgaaaaacagggaaaaagtaatggaaggcatcacgccggaagaacatcttacggcgatcaacttcctggaaaagatgatcaaaaacctgggcggcaaaatataatcatcttacaaaaacaaaaaagcggatagcattttactgctacccgcttctatattttctgcaacaggtggttagaataattctccctgcccgcctgccggtccttcttcattcggatcaggatcttcgtcctcagacaacaactccgcactaatcaggtcatcccctgcaatccttgttcccactgctttccagccggtaacctccacaaattcagaaagatcaatttcctcctcttccggactgcgtttcttgcctgttttcagcaatacaattggctgggtatgcgttgttaccatttccaggtaattattcgcgccctccttaatgaaattgaatttattgtttagcgtctgcgtttcaatccggaaacgtttcacattaaactgcttcttatccgcatcaaagtaaatagcggttaccgttttttccgggttgaacttctcaatgtacactacatcattcgactcgtaacggttggtgagatcgtagttcgtgagctcataagtaccgtttttaaaggcaacaaagatcttgtcttccccttcaaaagcaccaatgtacacgccacgttcctctgtattcaaacgaccggtttctgtatcataccagatcttttgtccggccagtgtagacactcctttctccttgaacttcacaccacggatcgggtatttggttaccacgttccccatggagttacgtcccttgatcgcaatggtttcaaagaacaggtcgaactccttgttacgtgcgctgcagttcggactcagcttgatggtcaccacttctgcttccccgttaggattcgaagagaaataatgcactttggagttcttctcccctttatgcgccaggtcgtattccttatcgcgggtaacacccgttacattgaaacgtttggcatagctcactcccgtcttaccttctacatagatcatgttgtaagtagtacgctcgtcattcttacggaaaatgtccacatgaatgatatccttgcccacaaaggttttatccgctactttggtcaccagcattttaccatcccggcggaatacaatgatgctgtccaggtcagaacaatctgccacaaactcatctttcttcagggaagtaccaatgaaaccatccgcccggttcacatatattttagtgttggcaatagccacctgcgctacctggatgttgtcgaacgttttaattaccgttttacgttcccggcctttaccatacttcttcagcaggttgtcgtagtaagcaacggtataatcggtgaggttcgccaggttgttcttcacctctttgatttccgcttcaatacccttgatctgttcattcagttcattgatatccaaacggtaaatacggcgtacaggcttttccgttaatttcacaatatcctcgcgggtgatttcgcgtttcagttgcttcttatacggtgtaaatcctttatcaatagcattcagtacggtttcccagtccttatgcttttgttccagctccttgtaaattcctttttcaaagaagagtttttccagggaggtatagtgccatttctcctgcagttccgccagtttgatttccagctcctgcttcagcaggtctttggtataatccgcggaagatttcagcagatcggaagccgtgaggaactgtggcttatcatttacgatcacgcaggcattcggcgaaatagaaatttcacaatcggtgaatgcgtacaacgcatcgatcgtaatatccggtgaaatacccggcgccagctgcacttcaatttccacttccgcagccgtgttatccactactttcttgatcttgatcttaccattgtcgttcgcctttacaatagactccatcagctgcgtggtagtaataccataaggcacatccttgatcagcagcgtctttttgtccttctcttcaatatgtgcgcgtactcttactttaccaccgcgtttgccatcattgtaactggcaatatccaccatgccaccggtaatgaaatcggggaacagttcaaactttttaccacggaggtatttgatcgaagcgtctataagctcaatgaaattgtgtggtaatattttggtagataaaccaaccgcgataccttccgctccctgtgccaacagcagcgggaacttcatcggtaatgccagtggctcatttttacggccgtcgtagctaagctgccaggaagtagttttaggattaaatgctacgtccagcgcaaacttcgacaggcgcgcctcaatatacctggctgctgctgcatcatcaccggttcttacatcgccccagttaccctgggtatcaatcagcaggtctttctgtccgaggttaacaatggcatcactgatagaagcatccccgtgcgggtgatactgcatcgtttgcccgatcacgttggccaccttattataacggccatcgtccatttctctcatggcgtgcaggatacgacgctgtacgggcttcagcccatcttccatgctgggcaccgcccgctccaggattacataagaggcgtaatccaggaaccagctctcatacatgcctccaacgtggatgacattgtgcagagattcgtctgatgttttattttccatgtccatgtataatacacttacggttttacgttaatcattttttcaaaatcctcccgccagatacgtacactgtctttttgtacatcctccagggagttcagttctataaagcaacaatctgtaatggccaccagctgatgccatacattcacaggtacttctacccttgccggcgccgttacctccgttgttactatttcatggcctcccagcgcacaccagtgaatggctgccttgccggtgaacaggtatagcacctccgggttcttatggtcgcttttaccttcgtgataatgctgcccgctgctgctgcccgcattccggtagcaaaccaggaaatcacccgtacggttgcagttccagaaataaccgctgccgcggtcatcagctcccatcaattccagtggcgttacggttatcatacagtagttgttggattttcagtagtttctcccggctgtttcacttcaaaatcacggatcgttttcagatcgcccctgctttccagtttgccttcgcggatcagctctttcagccgccagcccaggaactggtccatcacagggtatttcagtttaccggttacctgctgcactacccgccatgctttcacaaactcttttccactctgcgccagtaactccttgtcgtaaaacagggtaggctctcctttgatcttctttccgccttccagtaaacggatacctgcgttctcattcatcaggcgatgccactcatcgccatccagctcgtattctgccagtgaaataggacgcgccagcttctttgccttcaggaattcctttggcagtatctggtgcagatgggtaggataaaacaccgctcccttttcattaaggaaaggcaggttgttgaggtaaataatatggatgcgtcccgcaaaatcatacagctggcttaccagccaatagtacccgcatacatcgcgggcgttttgcccggcccatatccatacttcctgttcggggtcttcctttaattgcgctttcagggatttaaaaagatcggcatcatcgggatcgccggtcacttcttctgccgccggttcttccccggctgccggagctaccggttcaatacccgccagctgctgccagaactggcgacggccggcacggccctctttggtgtccaggataaataatggtccaacggacaggtcatcttcaaaacagcggatctctccgctcattttctcatccatcgcaatcgcctctcccaacaccggaaccgaagactgaccaaaaacaatgtgtattaagcccatatgcctttctatactgtttcttctactaaatccttttcataccgcaggttgttgatgataaactcctggcgggtctgggtatttttacccatatagtattccagtaacttctggacatgaatatctttcgataaaatgatcggctcaatacggatatcttccccgataaaacggccaaattcatccggagaaatttctcccaatcctttaaagcgggtaatctccggcttgttgcccagtttctttactgccttctgtttctcatcttcattatagcagtaaatagtttgctgcttgttacgtacgcggaacaacggcgtttccaggatatatacgtgaccattctttaccaggtcagggaaaaattgcaggaagaaagtcaacagcagcaaacggatgtgcatcccgtccacatcggcatcggtagccaccacaatgttattgtagcgcaatccttccaggccgtcctcaatattcaacgcatgctgcaacaggttgaactcctcgttctcatatactacctttttggtaagaccaaaactgttcagcggcttaccacgcaaactaaataccgcctgcgtttccacgttgcgcgatttggtgatggaaccactggcagaatctccctctgtaataaagatggtggaatccagccggcgggcttcctgttctgccttatctttcccggtaagctcatcattcaggtgcaaacggcaatcgcgcagcttcttgttgtgaaggttcgctttcttcgctctttcattcgccagtttcttgataccggccagctccttacgctcacgttcactttgctcaatacgtttcttcaacgcatctgcaattgccgggttacggtgcaggtaatcatcgaggtgcttggcgaggaattccagtacaaacgcctttacagacggcccgttttcaaaaacaacctgtgaacccagcttggttttcgtttgcgattcaaataccggctcctgtacgcggatggataccgccgcacaaatagaagcccggatatcggtagcctcataatctttcttatagaagtcgcgtaccgtttttacaaacgcctcccggaaagccgccaggtgcgtaccaccctgggtggtatgctgaccattcacgaaagaataatactcttccccgtattggctttcatgggtaatcgctacttcaatatcttctcccttcaggtgaatgatcgggtaacgcagatcttcttcattcgttttacgctgcagcaaatccagcaaaccattctttgaaatgtatttcttgccgttgaagctaatggtaagacccgcattcaaaaagcaataattccagatctggttctccaggaattccggtataaaacggtagtttttaaatacagtatcgtccggtgtaaacgtaaccagggtaccattgggttccgttgtcgccgtttctttatgctcttttattaaaacccctctctcaaactcagcggttttcatccgtccgtcacggatcgactgcaccttgaaatagctggacaaagcattcactgcctttgtacccaccccattcaaacctactgatttctgaaaggctttactgtcgtactttgcgccggtattaatcttactcactacatctaccacctttcccaaaggaataccccggccaaaatcgcggatggtgacatgatgctccgttaccttgatatcgacctgtttaccaaaacccatggtatgctcgtcaatacagttatccgttacctctttaagcaggatgtaaataccatcatccatactcgacccatctcccagtttaccgatatacataccaggccggaggcggatatgctcccgccagtccagcgaccgtatggagtcttccgtataggaagcaaatagatctttgttatccgttttgtccgtgtttgccataatatattataatttcctaaatactattgtttcgtaggtcgcaccctattttgcaaggatactaaatcttttagcaaaatctgattgctggcaaaaataaaggattcagggaatcatcccaagtataagttatacactatgcttacattatttattaccaatgtattaagactgttaaattttatatttccgggagataatgaacagttttgggggttttcgggaagtatcacatgaaaatggtataaaaaaaactaatgtgaatggatccttatatcagatatttctttatatttacataagtcaacaattttgagatatcctaacctatgtccctatgaaaatactatttctaatcctgcttactgcagtttttctggtagcgcttgtagctacctacttcattaaaaaagaagaggataacagcatcggaaataaattccttcgccttatccggaaatttgattcatggcaaatgatgcgatgatcaattttacctgctttaccaacaaatggctttcatacaatattcacaactggtcacatcagcctggcaatagccatcagggagtattatgtcttaactatattacctattaaccgtaaatccctatcccatgaaaaccggtctgttatttaaactcgcctgtctgttgattgctgctgtagtattatctgtgcacctggtgttcaaacctaaagccggacaccggtgaaaaacattcagggattttattgcttccacgggaaacaataaaatccctgaattactgattatctgttataatatttatttacggcatccgtacggctgcgcacgtgcaacttttcataaatattatgtacatgccgtcttaccgtttcaatactgataaataagttgctggcaatttccttgtacaaatagcctttcgacaactgatccaggatttctttttcacgcgtagtcaatgcttccagtgccggattaggtttagcctgcttctggaaaaatgctaccactctcctcgctatctgcgaactcatcggggaaccaccatcatacaaatcacggatggcttcgagtaattcacccggagatgttttcttaagaatataaccactcgcacccgcctccagcgccataaaaattttatcatcatcttcatacaccgtcagcatcataaactgcatatcaggatgctcgcgctttaactgcgcaatacattcaataccattcatgccacccggcaggttaaaatccatcaacaccacattaggcatcagctgagggatttgctccacggcagtttccgcattattgaatgtccctacacaggcataaccgtcagaaccattaatcagcaattccatagccgtgcggatatcatgattatcttctactatcgcaatagtgatagtgtccatgttatcctgggacttcttttttgagtataccgtcatgtttaaaaggaattataacacttaaatgttattaaaaacaaatgtatgttaatttagtgggatatcgagaaaaactattgttccattattcgaactgatatccgcatttccgccaaccgatatcatccttttctggatattttttaatccgtttccaaacaatcttaccttttcctggtcaaacccttttccattgtccttaatcatgatcgtcatgtttttatgcatcttcacttccacaattacctccgttgccttcgcatgtttcactacattatgcaacgactctttcactgccaggtaaatattccttcgcgtgccaccactcagcttaatatttggaatagtttccggaatataaaactggtgcgtgatatgtgcatgctccaaaaactcggccgcaaaacttctcatataagcaatcaggttagccagcgaatcattggaggagctcatcgcccagatgatctcactcatcttatccaccatctctcccgccgtttcagaaatccgctctacttcccgcgtctgcgaaggatcctggattttccgcttcgccacttcactcagcaaccggatagtagataaccccgaaccaagatcatcgtgcatatcgctggaaatacgcgcccgctcctggtctaccgcctgctctttctccagcttcagtttctcatgccgtatcttataatcaagatatagcgtagagaaataataagcaattcccagcagtaataacaacagtaaaaaccggaaccacagcgactgccagaaaggaattttgattacaatttccagcgtggtaggaaccgtactccagatatcatcattattggaggccctcaacttaaaaacataactgccgggatgcaggttggtgtaacgcgccatcctgaaagtacccgcctgcacccaatcctcatccgctccttccagcttatactgtaccttgttctttaatggattggtatactccagcggcacaaattcgatagcaatagtattctgattatacggcaattctattttcttcagcaatgaaatggccgtgtcagattcataaggcttgtccagcacctccatccggcggatgatcactttggcattggataaattgtcccggaaattcttcgggtaaaatccattcaccccacggatgccgccaaaaaataattggccgtcgatggacttataaaacgcaccggtattgaactcattcgactgcaacccatcttcataattataagtagtgatttcacctgtcagcgggttgatctgtgataaccctttattatggctcacccagatcctgtctttatcatccagcaacacaccatacatataatcattgatcagcttgggattatcataactgttgtaatgctgcttaatgcgccctgtatcatccaggatgaataatcctttattggtagccaccagcaactctttatgcgcatttttattgatggatttcaccgtagtgccgggcgcaaggaatacgtttttccagcgggaatcagctactcgctttatatataacgccgatttcgtacccacgtactggttacccaggtaatcttcataaaaagcggttagtacttcatccgaaaaattatgcactaccgctacttcgtatcctttctcggtattatcaaacatcagcagatagccgccataattgaaatacaattgtccgttggtacgcttaaacaggaaagggaatggcgccagctgcgtcggtaaacccaacgccgttacttttccggtaagatccaggaaagacttggtttctacattgaacaggccgatgtgcatccccgcaaagtgcagccagagctgctctgcattctcccggcaaatagcgcccaggtcgttgccgggaaattttccgggatataattcattggaaatacgctccaggaattttccaccatcttcataaatattcaatccgtccctcatcagccccacgtacaattttccatcatcgtgcttgtacacggcctgcaccatgttatgtgtgatataaggcgaacggtaaaggttaaatacttttttatgcggggaatacttcttcaatccatcgccatcggtgcctacccacatgttatcagcaacatcccggtaaagccacgacacatcgttgaacgaccgcgtttcaaaagtattaaagctcacaatatgccgcacaatttcattacgcgcaatactgtatatcagcacaccatcgcttccgcctatccatacattgccgtactgatccagctcagataccgcaggaataaacggttcccctttttcattcttcacatcaaaaaccaggtcgctgaatttgttacgctgcttgttaaagagcgtaatatgacctgcactgatgatgatcatggagtctttattcagattgcgcagcaacggcttatcgcccacaccgggcaggcaataggtggagatgcggagatttttgatgttcagggaaaaaagctctccctggtcgccgttcatccagatggtattcccgtctttcatcactacagaaggcaatatccctctttgtacaaactgcggcggatacaaaatgatgcggcgcgtggcgtaagtcgtattatccagtacatagatacctttcatcggacgccatacccacaaggtgttggtggccgtatcttctcccaggatcacaaatttcacattattatcacgttctgcggcatttacgatagtagtatcttccagcagcttactgaagttgttcttatatttatcgtacacgctgatcccgttgttatgggccagcaataactgggaacggctgtctttataaaaagaaaatcctttatatcctttcagatcaaaacggttgattaccgcgcggttgccggtagatccgcgggctaccagctctcccctgccttcgcctgccttgtaaagggaactgggtttataccggtattcattaaaggtatacccgtcaaaacggttgatgccgtcgcgggtggcaatccacataaatccctggtcatcccgggtgatatcgaataccgtgctctgagaaaggccttcattaacgctatagctgtcaaaaatgtatggtttgtcctgcgcatgcagcatcccggagaagagtccccatatacagcataggatgaacatttttaagcgatgcggttgatgcactggaatattgttaatgtgtaagcaggttaggtaatctgcaaatatataaatctgtgtcacactttgtagcaattttgtaattttcttcccgttaacagattgggaataaacgaaatactcttatgaatacagtcaacacagcagccggcctgccaggcttaaacacaggacagtggccatttatcacccgtaaacaaagggtgctccgccgcctgttgctgctgggatgttatactttaatatttgcttttcgcccggctgccgcccaggacacggcggccggttaccatataaacatactaacagctactccggttcaaagtatccgcggactgagcgtggtaacagacaaagtggtttgggcctccggcaccggcggtaaggtgggtaacagcaccgatggcggtaagcattggaaatggaccacggttaccggctgcgacagctgcgactggcgttcactgtatgcctttgatgcccgtaaagccattgtattgaatgccggtgcaccggcattgatttttttaacggaagatggcggcaattcctggaagcaggtattctacgataacaggccgggcattttctttgatgccatgcagttttttaatgaacaggaaggcatcgctatcggcgatccgatcgacgggaaatttactgtcatacggacacataacggcggccgcagctggaaagctgatcccacgcccgctttgccggccgctgcagaaggggaagccatctttgctgccagcggcaccagcatggtgctgttgccggggaagaacgtttactttgccaccggcggccaggtagcccggctttttaaaagcgcggataacggaaaagcctacacgattccgctgatacagggcagcagcaccaccggcgtgttttccatcgccttccgcgacgcggccaccgggatagctgtgggtggcgactataagcaggacactgcgcggaaaggaaactgcatgctcaccaccaacggcggcctgagctgggaagcacccgcagtacctcccggcggataccgctcctgcgtagcctggatcagtccccggctgcttatcgctaccggtacttccggcacggatatttcagaagatggcggtcagcactggaaaaaaatcgggaaaggctttaatgtagcagccaaagcaagaaaaggaacaaccgtatatgtagcaggaaaagatatcggtgtactggcaaaacgttgatcagggccaccgccaataaaaaggtgctcctggaaaggtgcacccactaaaataggttaaagcaaaaagtaaatttattgatatgaagttaataagtaatttatttacttgttaggattttttgcgaagctgccaatttagagggtaaacgcccaaaaaggagcatctaacgcaaaaggactatcactactctgatttttttatgtaatttaagacctcggtaacgcattaccgcgcatccagaaaaagagattatgcaagttgaaacctcgtcaagtaaatacggcgccaaacactatcccgatggtatcagggattggaaaaaagaaggaaattatttttgtttttatactaccgaaacaattctcgaagtaagggtaattgccgacaagatcctccgcttcagatatgctgcggaaggctcttttcaacgggacttctcctacgccaccagcgatacgctggaagaatcaccaatcgcttttggtataaaagaatgggaagaaacttttgagatctatacagatgaattaaaggtatttattgcgcgggataacctccgtatcaccatttcagacaaggaaggaagagtgatcaaccaggatgaaatgggttatcactggcaacactacctgctcaaaggaggtaaaatccagtattgcagcaagttagtgcaggaaggggaatgcttctacggacttggcgacaagcccactgaactgaatctccggggcaaacgcctggaaaactacggaacagatgcctatggctatcagaaagataccgacccgctgtaccggaacattcctttctattatggcctgcaccatggcatcggctacggcattttcttcgataataccttccgcaccatctttgattttggtaaagaaagggaagatgcctgcagtttctgggcccgcggcggcgaaatgaactactattttatttatggtcccgacctgctggaagtggccgaatcttatacaaaaatcaccggtacccccgaactcccgccactatgggcgttgggataccaccagtgccgctggagctactaccccgatacccgcgtaaaagaaatcgcgaaggaattccgcaaacggaagatcccctgcgatgttatttacctcgatatcgattatatggacggtttccgctgctttacctggaataaggaatggttccctgatcccgcagggttgatcaaagaactggccgccgaaggttttaaagtagtagtgatcatcgatcccggcattaaggtagatgccgactacgccgtataccaggaaggcatcaaaaacaactacttctgcaaacgcgccgatggcgccctgatggaaggagacgtttggccgggcaaatgtgtgttccccgactacaccaaccccgaagtacgggagtggtggagcagcctgttcaaaagcctggccgaaaccggcgttcgcggcgtatggaacgatatgaacgaacccgccgtatttgaaatgggctccttcccggaagatgtgcgccacgactacgacggcgaagaggtgagtcaccgcaaggcgcataacgtatatggccacctgatgagcaaagccaccgcagccggtatgaaaaaatacctgatgcccaaccgctccttcctcattacccgctcctgttacgcaggcgcacaacgctggtcttccgtatggaccggcgataacgtatccagctgggaacacctgtggctggccagcgtgcaatgccagcgtttagccgtttccggtatttcatttaccggcagcgatatcggcggcttcatcggtgaacccgatggcgaactgtacacccgctggattcagctggctgttttccacccgctcatgcgaacccactccgccagcaatgaaacaggctttaaccaggaaccctggagcttcggaccggaatacgaaaaagtggtgactaagtttattacattaagatataaactgctcccctacctgtacactaccttctggcaatacgccacccacggtacgcccatgctgcgcccactggcttttgtggcgcaaacagatgtcgccacacacaactgttcgcacgagtttatgttcggcgactccctgctcatcagccatgtaagcgaaaaaggtatgcaggaaaaagcagtataccttcccgccggaaactggtattatttctggaacgatcagaaatacgcaggcgcaaaagaaattaaggtaaaaactcccctcgacgaaatacccctgtttgtaaaagcaggcgctgtattaccggaattcccggaaatgcagtacacccagcaaacaccggttacggaaatgttgctgcacgtttatttcggagatacagaagtaaaaagcgtgttgtacgaagatgccggcgatcactatggctataaaaacggacaatataacgtgatccgcttcaagcaacgttctaccgcgcaacaattctatcttaaaaaacaattttatatcaattacgaaacaacctataaaaatcaccggatcattgtgcatggccttcccttcaaacccactacactgcttgtagatggacaagccaccgccatacgcccggaaaacatactggcagataataccgtgtcatttgttgtaccaagaagctttgaagaaatatcaatgaagtagaaagatatctaaagtggtaagaaaaaaagaaaggcacttcagatagagatctcgcgccggtttcataacctatgccaactttagaactataaaagtagatgctaaatatcattgtacaaaatgttcagcggcgataaacgcacaatgaacaaaatgaataagttgttaacgttgaattaagagttcctgaatcagaaatcaaagtaaatagcttatagatctaatctgaataaggattacagcttaaaaaatcaatttagcaatgcttacaaaaatcgtaaaggctcaaagatgataaatcacctttgagcctttcttacgttgatgatcattgtttatgcttaataaaaaatagacaaaaagaaaatagaagtcaatgcacaaaacactaaaaagataaaaacagctctgaaaaggatttccatcctgtcagtagtatattctattccgtgtaattcctgaggattctccgcgtggttgatagtaaggcttttcatacaaacaaattaaaaggattctcaataaaaaaattattggtgacttacgggttctataagatcacatcctattgatgaaattacataaaaaaaagctaaaacggacaaatctttttgttcattttagcttccacgctgttcatttttgtcagcccttctttttgtgcttgccggtattttcatgcggcaactgcaacggagctttctttactgcaggcgcggccacctcggtactgtcgcccaactcatcagcactaacggtttccccccgcttgtaatactccttcaccatcttcccggtttcttcatcatatagcttccataccccgttacgaacggaattacccaaccttacaatctctgtcggcgtttcggcattcgtcaccggatctatgatcatgatcgtatcccgctgtccttcaatttcagtagccaggaaagccccttcctcactgagcttcccgttaggaaaataatacttgcagtaaccatccagcacattgtttttataagtttcttccgccagtaaattaccaatggcagaagtctttttccaaacgccttccttccggccgtttttgtaaacgccttcccaggtataccctggctctcccctcacttctcccacttcctccacccaacgcccttgcttacggttttgcgcatcacgctggttcaccttcgcctgggcaatcgccatactgcaaacactcaataataacaggtataaaaacaacagtttcttcatagatattactttgtcacaagttaaatattttacgcgcgcgaattttgtctttctcgctgattatactgattactttgattttacttttggattttataaaggattaaatgaaaaatccggaaagatataagcgaattttgtctttctcgctgattacgctgattatactgattttaaggattttatttttttagattttataaatgattttaataaaaattcggagagacataagcggttatcttcgcttacatctccccgaatcttttaaaatcaaaaagtgatcaaatcagcgtaatcagtgtaatcagtttaatcctgagtaagacaacctacgctgctgctatttatgcagctggatattcccgatccgcgtgtctttcccgcgcgctacctttacgccggtaacggtggtgtccttataaccgttggaggcatttacaaaaacgttccagtcgtcgcccactttcaaaccacgtaccttatactcaccgcttctccatggcagtgcatataaagtatcgctgctgctgttgtaaatagaaatcaccgggtaggcatcccatggggttaccttaccggaaatactgcccattttaagaatggtgaatacattaatgtagggtttgaggatgaattttccgttccatgttctgataatagagcgttgtacatcaaagtccagccacaactgcaggttatccgcgctcagctcatcccactcgttgtgacgcactctcacaatgatcttcgattgaccggagatcgatttcaccgggtaagtaacaccgtccttcaccagcgagttctggtcgccaatagtaatacggatacgttccattgttcctttcgctaccacgccgccggccagcagggtatcagctccgtttcttaaagttagcaggtcataaacactagggttaatatccaatgaatcccacaactggcaggtatcccgcccactgttccggtcgtggtcacggtcctcatcccaccagcaacggtcccggtcggaccagttgtcgtcatccgttttaccgcaggtatccaccagtacttctacgctgcggatatccagtaatactttgtcgaagtaacccggatcatctgataaataaagacttaccttttgtttattgtccggaataggcgtggtggaagcggagttatcctttttacaggctcccgctaatgtaacagcagccaacactgccatcaccaaaccatgccccggtttgcggagaaagtttttcataaaaagaacggttttatgtaactaaataaaaatatggacgaattgatctggttgaaacactgataccacataaaacgtaccaccatcaccgcttattgcaacagggatcagattgctaatagacgatggaaataagagaaggtttaatttggggcggattttgtctttctcgctgattacgctgattatactgatttaggggatttgatcacgttggatttttaaggatttgcggagatgtaagcgtaggttgtcttactcaggattaaacggattatattgatttaggggatttgatcacgttggatttttaaggatttgcggagatgtaagcgtaggttgtcttactcaggattaaacggattatactgatttaggggatttgatcacgttggatttttaaggatttgcggagatgtgagcgtaggttgtcttactcaggattaaagggattatattgatttagcggatttgatcacgttggattaaaaagattttgggaagataaagcaggtatatccgcttgtatcttcccaaatcctttataaaatccaaaaagtaaaatcaaagtaatcaatataatcagcgtaatcagtgagaaagacaaaatccgctcacatctccgcaaatccttaaaaatccaacgtgatcaaatccccttaatcaatataatcagcgtaatcctgagtaagacaacctccgcgctatcgcagcttcaatatagtcgcacccaaaggaggcaagctcaaagaaatcgtatagtccctgccgttatacgtctgcttaacggtgcggataacaccggtgttcaccacaccactgccgtaatacttcggggcatcgctgttcattacttcttcccactctcccgctacgggaagtcccaccaggtagttttcccggactaccggcgtcatgttcaataccaccagcagaatatcgccggctgcttttcctttccgcacataggccagcacacagttatcataatcgtttaccgtgatccattcaaatcctgcggcatcaaactgctgctcgtataaagcggtagaagcggcgtaaaattcgttgatatcttttacaaaagcctttaaaccctgatgggtaggatgtttcatcaggtgccagtcgagctccccgcggtagttccactccgatgtttgcccgaattcatcacccataaacagcaacttggtgccgggatgggtatacatataactatatagcaaccggagattggcaaattgctgccagtcgtcaccaggcattttatacagcatgggcgacttcccgtgtaccacttcatcatgactcagcggcagcataaagttctctccgaacgcatacaccaggctgaaggtcagatcgttctggtaccacttccggtggataggatcctttttaaaataatcgatcgtatcattcatccaccccatcatccatttcataccaaagcccagcccacccataaaagtaggtctggatacgccatagtgggaggtagaatcttccgcaatggtttgcacatcggggaacagggcatatatcgtttcgttcagcttcttcagaaaactgatggcttccaggttctcatgaccacccacttcattcggttcccatgcgcctctctccctggaataatccaggtggatcatcgatgctactgcatctacacggatggcatctacatggaaccggtcgaaccagaaaacggcattactcagtaaaaacgatcgcacctcgttccgtgcatagttgaatatataactgttccagtcagggtgataacccttacgcatatccgcatattcatacacatgcgatccgtcgaagcggaacagtccatgcgcatcatatgggaaatgtgagggcacccagtcaagtatcacaccaataccggccaggtggaaggcttccaccatctccataaaatcctgtggcgtgccatacctggaagtaggtgcaaagtaaccagtgatctggtatccccaggaaccatcaaaaggatgctccataacgggcattaattccacatgggtaaatcccatttcctttacatacggcaccagcatatcggctatttcctggtaggaatatacgcgctccggatcagagggatcggggcggcgccaggaaccgaggtgtacctcgtatacggcaaaaggactgtcgagtgcattgtttttccggcgatgatccatccacttcttgtcatcccattcataatcaagcgggtataccaccgatgctgttttaggacgtacctcccagtgattggcgtatggatctcccttgatcagctcttccccgctgttggaacggataaagtatttatagagggagccaggctttacaccgggtgcaaaaccttcccagatgccggagctatcccaccgggggtaaagcgtatgggtgtaatgatcccatccgttaaaatcccccattactgctacaaatgccgcgtccggtgcccaaacggcaaagtacgttccatgggcgccttccacctccatcgcatgggcgccaaacttttcgtatagccggtaatgtgagcctgcctggaaaagcgttatatcactggaagaaaaaagagtaaatggttctacgtactgtaaagcgcgatttgtatctccggtcataataacgtgtgaattgggtgtcttgattaacaagatagtttaaatttgggaaaatgacctatacaatgaaacagatatttacataaaaagaaaaaggtgcccgatggacaccttttctctttttatattgctattccgttttgcggattagtattttttcttgtacggaggtttgccaccgctgccgaaagactcacgtctgtcgccaccgctgcggctaccgcccgtgcggctgccaccttctgcactccagcttcttttacgcggaccatcttcacgacgcgggccacgatcgcctgcgccggcaccggtgcggggacgtctgtcgccatcctgggacatttctatcctcacgctgcggccgttatattccactttcttgaaagcttcggttactttaggcagttcttcgttctctacttcaaagaaggagtaaacacccttcagatcaatacggccgattttattaccacgcagaccggtattgtcgcacaggtaacggagcatatcgccgcggttgaaatcatctactgaacccaggttgatgaataaacgggtgaatttgccatcgcttctgcgcggacctctgtcatctcccagtgtaccggcacgtctgtcgtcttttgcattcagatcaggcgcatcctggtaatattcaaggaactggttgaactcgagggaagcaaaacgtttgatcaggtcttccttgctcatggaggcaaactcttcgttaatgcgttccatgtaaggttcaatctgctcttcgtttactactacgttatgtactttatgcaccaggccaaacagctgtttttcacatactgcgaaaccatccggtacttcagactttacaaattttttctggatcacacgttcaatctggcggatctttccggtatcacggctgctgatgatagcaatagagatacctgatttaccagcacggccggtacggccacttctgtgtgtgtagttttccacgtcatccggtaaatcgtagttgattacgtgtgttacgttatccacgtcgataccacgggcagccacatctgtagctactaatacctgcagcgctctttcgcggaagcgtttcatcaccttatcacgctgctgttgggttaagtcgccatgcagggcatctgcattgtaaccgtccttgatcagcgattctgcaatttcctgtgattcaattttggtacgggtaaaaacgataccaaaaatttcagggttgaaatccacgatacgtttgagggccgcatatttttcacgcgggcgcactacgtagtattcgtgttctatattaacgttaccgctatttttgttacctacagtcagttcaaacggatcctccatgtatttcttggcgatacggcgaacttccgttggcattgtagccgaaaacaaccaggtagttttaccttcaggggtgttagacaggatgctgttaatgtcttcctggaatcccatgttcagcatttcatctgcttcatccaggatcgcataacgcacattgtcgaaattaaccgcaccacggtcaatgatatccagtaaacggccgggagtagccactacaatgtgtactcctcttttcagttcacgcagctgctgaacaatgctggaaccgccatataccgctacgatgctcacatcgccaaggtatttgctgaagtttttcagatcattggtgatctgtaaacagagttcacgcgtagggcataagatcagtccctgtggtttatttattttcagatccagttgctgcagcaatggcaggccaaatgcagcagttttaccggtgcccgtctgggcaagacctacgaaatcgcggtcacctcctaacaatactggtattgcctgttcctggatgggagttggggaaacgaagcccaggtccgtaattccctttaagataggctcttgtaagcccagtgattcaaatgtagtcatatttgcattaatcaagctccgtcgggagctgtgtatatagcttccagcagtgcgctgtcagctgttaaaaatattatttcagcttccagcggttagctatcggctgttggttaccttcagtgattagctgttggttaccagttctccttcgaggtcgtaatcaaacgccttggtgatacgtacttctacaaagtcgcccggtttcaggcgtttggtagtgtcaatgatcacttcgttgtctacttccaccgaatcaaactcggtacgggcaaggtatctgcctgcctcttttttatctactattactttaaagatcttccctattttctcctggtttttttccagggagatttcctgctgtacttccattatttcctgcgccctgctctccttttcttctgctggaatattatcttccagttcataggcgctggttccttcttcatgactgtaggtaaacacccctacacggtcaaaacgcattctttccaggaaacctttcagttcttccacgtccgcttccgtttcaccggggaaaccggcaatcagggtggtacgtaaacagatacccggtactttggccctgatgtcatgcaccagctgctcaatttcctccctggtaatctgacgcttcatggccttcaacatggcattggaagcatgttgcagcggcatgtcaatatacttgcagatatttgggaactcattcatcacatccaggatctccatcgggaatttggtgggataagcataatggagacgaatccattgcagtccttccactccggccaacgcacgcatcaggtctcccaaacggcgttgcttatacaggtccaaaccataataggtaagctcctgcgcaatgagcatgatttcctttacaccggatttcaccagtttctgtgcttcggttaccaactcctcaataggtttggaaacatggccaccccgcatcagcggaatagcacaaaaagaacaggtacggttacaaccttctgctattttcaggtaagcataatgagacggggtactcagtaatctttctccaatcagttctgctttataatctgcatcaaattttttcagcagcaatggcaattccatggttccgaaccaggcatccactccgccgatctctgattccaggtcacccctgtagcgttcactcaaacaacccgttacgtatactttatccagtttaccacgttgtttcagctctacctgctccaggatggtgttaatcgattcttctttggccttgtcaataaatccgcaggtgttcaccaccacaatgttatgatcgcgttttgcactttcatgcaccacatcgatttcattagccatgagctgaccgctcagtacttctgaatccaccatgttcttggaacaaccaagcgtaataatattaaccttgtctttctttaaagtttttgtcttcaagcgcgaatgtttttaaacaagcggtcaatcatttgttgagccgctaccgccacgaagacacacagacactgattgaatgtaacagcagacttactgtatgtgacttgagtcttagtgggggttaaggaaggtgcaaaggtagtaaaaagaattgacaattggaaattaatgctaagtaactgttgactagctacttagcataacgttgaaacccaggtcagctcagcgtctccatggccttgtcggcacgttcgcgggccttctgccgtttataatggtaccaccacttgggggccatcctgatcatcaggttattcattccccgcaggcccaccaggtgataaagcccgtttagtttattgacgaaagaaggatccagcgcccggagactcatggcgaaaccgccatccaggtactccatatgatgccagtagcccgccggcataaacatcgtgtccccgtggttcaggatagtagtatatccccgcgcatgtttcagcgccggaaactggtcctggtccagctgctcatgccagttgacgaagttcgccgcgctctctacggtaaaaggcatccggtaaataagcggcgactgattattctccagcaacaatacccgcttacggccaataaactgggtatggaaaatgtgtgaaaggtcgatgtcgtaatgcatatgcgccaccgaaccggcgccgcccacaaataacatcgggtattttttcagaaacccggaggcaaattcatccgggaaagtaaaatcttccaccagctggggagcatgctgaaaaatgttaaacaggaaaatccggagcgctaccggtccctgttgtatcatatcgaggtaggccccgaaagtaatataatcatctgctccgttgacaagcgtattctcgttggcgcgctcattattatataccccaaccgtcttgtctccgactatcgatttgaaataatcccatgtccacttgttgtaggccggccagtgctggctaagcgccgccgccggtataattacaggtttacgtggatggtaatagttcttcttgaattccgctggtgtaatatcttcaactcgatctatgtgctgtactatcatacttacgaattgttaaaaagggtacaaaaagggaacaagtattcaaatttaataaatgcagtgctatttataattacaaacgaagcgctttaatgttaatcaaataacgagccgggctcctgttgggagcccgattgtttcacctaaagtaaaatattaaataagatttgtgtcagttgttaattaacattcacaatgaacagaaaatcagccatttacactaaacagcgaatctacgaaagactctttattaaacacctgtaaatcttccattttctcaccgataccgatgtattttaccggtattttaaactggttggcaatggccagtaccacaccaccctttgcagtaccatccagtttggtaatagcaagggctgttacctctgtggttgctgtaaactgtttagcctgctccagtgcattctgcccggtagaaccatccaataccagcaacacttcatgcggcgcgtctgggatcacttttttcatcacccgtttaattttacccagttcatccatcaggtggagtttgttgtgcaaacggccggcggtatctataataattacatccacatctttagcggccccgctctgtaccgtatcaaaagccaccgcgcccgggtcagatcccatttgctgctttacaataggtacccctactctttcactccagatagtcagctgatccactgccgctgcacggaaagtatccgcagcacccagcatcaccgacttacccgctttcttgaaattataggccagcttaccaatggtggtggttttgcccactccatttacgcctaccaccatgatcacataaggcttcttaccggccggtatatcgaaatcacggaaaccactatcaggggcatctaccagcaacgctgcaatctcttcctgcaacattctgttcaactcactggttcccagatacttatctttagctacccgctgttcgatccggtcaatgatcttcacagtcgtgtctacgccaacgtccgcagaaataagggcgtcttccaggttatccaatacttcggtgtctacactggacttccctgcaatggcgcgtcctattttactcaggaagctctctttggttttttgtaaaccctgatccagattttccttcttctccctggaaaatagtttattgaaaaagctcatagtttagattaattgggtccggtacatcccggttttttgggtgctaaaatacgcgaaaattcgcggattttgtctttctcactgattacgcggattttgtctttctcaggattacactgattatactgatttaggggatttgatcactttggattttaaaagattttggaagatataagcgggtatatccgtatacccgcttatatcttccaaaatctctttaaatccaaaaaaatccaaaagtaaaaatcaaggtaatctgtataatcagcgtaatcctgagaaagacaaactccgcacccgcataacgcaaaaagctgtcccttaacaggacagcctttcagtattattagtaaagccgaattacttttgggtcatgtactcctggatcttatccttgtgcacgattgcttccttaaaagtataagcaccggttttaggagagcggatggctctgataaccttagtccatacctttgattcagctgctgctttagtatcttttactttcgcgttctttgaagctacttttgccatggtattctattgtttttatggtccaatggctaactggcagtatgctaatacagccattcaccatcaacaattacttatttaatttctttgtgtacagtcactttccttaaaataggattgtactttttcaactccagacgctcaggagtatttttcttattcttgttagagatgtaacgggaagttccgggtttgccagaagctttgtgctctgtgcactccagaattacctgtactctattacctttttttgccattgtgtattacaaattaagtgagtcttagaattagattgcctgaccagctgcacgcaattccttcacaactgcatacaaacctctcttgttgatggttcttaaaccgtcagcagaaactttcaatgatatccatttgtcctcttctgccaggaaaaaacgtttcttttgcaggttaggaagaaaccttctgttcgtcttaatgttggagaaggaaacatggtgacctgtaatcggcttctttcctgtcacctgacatactcttgccatgatctaaaaatttaggaatgcaaaagtccaatttatttatggattttgcaaatattattaaatgaatttattcacatatgcttaaaagacacgcgtgaaaagcggcttcttaaaatgtgaacacaatgcaaaatattgataaccattcagttatcaggcaaatttacatctgtcttttgccgaaaatattttttacaacagaacgatcaggctacgtaaaacggctcctaatcttaccgattccagcactctttgctgatcggttccgtgtttcaacaacgcttcttcgtgcgaagttacacacatttcacaaccattcagcgcagacaccaccaggctcagcaactcaaaaaactctttccccaaaaccgggttcgccataatgctcatccggatacccgcaggagtagtcgtgtaaaactccttgttcacaaaatgcctgaaacggtaaaatacgttattggcactcatgagggaagtacaactgattacttctgcaatctccttgtcggttgcgccttcctgcaccgccagcttctcaaaagacgcctgcagatccgtatgcttctcatttaccgccacggccagcccgatcatatacgcctctttcttcgacaatgtagccgctgccagggaattggatacattgatcttcagatccttcaggtaacgcgcatccacgtttacaagcgactgcagctttcctgaaaccgaatccgccgttaaacccactgcttccagcaattgaacagccgtatcctgatttgtagttgcaaacataatatctaatttttttatttaataattttattaccggaagaagttgtcccgccacgcttatcccggcaggacaaccctctttcttaataaaaccgtaaatgacttgattcattaagctgtcagcgtagcttcacccttcgtccagttgcaaggacacagctcatctgtttgcagcgcatccagtacacgcagcacttctttcacgctacggcctacagacaggtcgtacaaagaaacccagcgtacaataccctgaggatctacaatgtaggtagcacggtaagccactttttcattggcttccaggatacccagctcagtagcaagggatttggaagtatccgccagcatagggaactgcaggccacgcagatcatcatgatctcttctccatgcagcatgcacaaactcactgtcagtagatgctccgattaacaccgcatcacgatcagcaaaatcctgcgcatgtttgttaaattcagctatttcagtaggacatacaaaagtaaagtctttaggccaccagaacatcaccatccatttgccggagttcttcagttcttcagaagacaattcataaaattctttacctttttcaattgatactacagccgtttttttgaattcgggaaactctgaccctacggataagataacatttttcataattactaattctctttttgatttacagactaatgattttatgctttgacggcgcaaagatcacattacattcattattaatcaaatagattttaaaaatgtggtattgagtttctctatatatatgccttttcactgcggcagggcgggcaacaacaaacatggcaactataaggaaaaaaaatgttccggacttaacatttttatgctatttctgtaacattttggcacgttatttagttatataagtggactttttttaatcaatttagcatggaaatgaagaaaaaatactttttactggtggttatcacgattggacttgctttgatcccgtttattaaaaacagcatcatcaaacacgatgaattcgacgctacccgagatctgttcatttagtgtttagcgggtcccattgaccgttcctgaaaagccccaaagcggggtcggacttttatacgccggtaagtactgatgcgaccggcctgcactcctgccccctcaacttttcacaaccttactcagcggctgaactgccgccaaacatatcgtcactttatcattaaaaagagatgggcagaccatagcggatatccccgccgttgtcttcccatctcttccaaatgcataaacagccctatcaaattccccgctaacccaaaccaggcaatggtttccagatcaagtccacatcacctccaggtgacctccacctttactgcatgtcaaaggctactcctaagcatgtcccaggcgtgttagagccattctccagcgcagtcccccgcggatgttgtcttggctcaggattacgctgattttactgattacctggatttttattctttggatttttctttgatttttagattttcttaaaataataattaagggagataaaagcgaatatccgcttctatctcccttaatcctttataaaatccaaaagtaaaaatccaggtaatcagtaaaatcagcgtaatcctgagccaagacaaaatccgcgtcacgtcgtttcgctaatcatatccgcaaaattccggataccgatcatcttggcagacgtatacccctcggcatactccacccccaccatcttacccagcatttttgcgcggtaaataacgctgtcgaaaaagcccgaacccgaaatgtaggtttgcggttcatgatctttcggcgccaggaactgtgaactgaagcttttaatcgcatccagcttctgctccattacggcactgatatctattacaaaatcaggttcatgataacggtcctgcaggaaatgaaaaacctgcttcggacgccacgcttcctgcgcctgcccgtctgccatggtttctatctttcttaaccctgccaggaaacaactgtcggcaatcagtttgccggcccttccgtggtcaggatgacggtcgtccattgcattggccagcacgatgtccgggcggtacttacggatcgccgtaatgatcgccatttgctccatcgtatcgtttctgaaaaagccgtcagcaagtcccaggttctcccttatttccagtcccatgatctttgcagctgcctgtgcttcctgttcccgcagctccggggtaccgcgggtgcccagttccccccgggtgagatccaccacgcccaccttcattccctgacgcgcatgcaccatcagtgtgcctgcacaccccagctccacatcgtcggggtgcacggctatagccagtatatctagtttcatatgctgtaaattgaggtgcaaagatgggaaaatatttagttatctgaactggtgataacgatcccggctttccggtccatcacctggtacttatcctgtacctctttctcagaaataacccgtacagaacggaaggttttcgggtctaaggtcatcaaaccggtttcattggtaggcgtaaccggtttgccgtttacgatgaagtaaaagctgctgtcgttgccatatttccgcaacaaactgtcatatgcgggggattcattgctcaataacacattcacccttttacgggcaaagggtttcgtttctatatataccacgccgttctccgcctggctgccatatttcagcaccgcctttgcgcctttggcaatggtaatcacgccaatacggtcgggcgatacctgccccatggccgacggcgtcacgatcacgctgtccagcacgtacacgggatcgtcactggctacctgtgccatcgctccaacagaaataaataataagctgataagtaagatccttgctttcataataagccctttttcatgacgggcgaatattacgaagatagcccaattaattgtaggcgcggaattgctggtacatttccagctcctgcacaatcacctcgatgtcgcggtcttcctgcttgtcgtaatcacttttcaggttacctccaaaaaagaaagcaacggtttgccaaacacgggcattaaagccgcctttgagttccttgatgatttcaaagcagttctgacccgtttcacggtcgatcagtttcatcaatacttttccctggtaaacggagaggttttccagtttatcgccaaactgggccttgagttctttctctttagaggccaggaaggctttacgttcccttttattcatggtagccatgcggctgttcacatctttcagcacttttgccgccgatctggcaaaaggataggttacatataccgcgttgcgtaaacggctccagcgctcgcgttctttacgcagcgccttcggcattttagctactacatcaaatattgccagcgtgattaccggaacggtatcacgtcctactatcatggcatgcaacggtatcacatcagcaccatgcgcctcctgggccatcgcatccgtgtgacagagggatatgaccagtaccaggaataatgaaacgatgatctgtttaaaacggatgcgcatagttaacttaacgttgcttatgtacggaatgttaccacaagttataaaaagatttgaaaatccggtttaactaaaaagtgttactgtaccggcctcatatgtaacttatttactacgaaatcatctatggctttctctactgcggggatatcatgcccggtgagcgcacagcccatcacatggctgccggcgccgggtataggcaccgcctccttcagggaatcgggcgttcccagctgcttttccatctccaggatggcggctacccgcaccgttttatcctggtgcgtttcatctttataataatataaattgatcaccggctgatgcacctttttaaaggtctcctccaccatactggattccagcaggttttgcaactgcaccaccgcttccaggcggtaattgttgtaccagtactttgctatttcggggtctttatcatcgctccgcctgaaatcacctttgctcaccgttctggccagctgcaatccccaggggttattggccaggaaggccaggttgtcgttgatcgcaacattgggcgacatattgatcatcgcataaacatcacccgggtaggccgctgccagcttcagccccagtgtgccgcccgtggaggtggtcatcaggatcactttatcgcccagcgccttgcctatgctcagcgcttcttctgcatctttccacaaacccgccgcagtcatatgcagcaatgggtcgctggtatcgatcccatgcccgtcgagccgcgacaggtacaaattacatccgtaacgtgccgcaaagttgcgatgcaccgggttcccctcttcctggctggcggaaaagccgtgcaggtacaccacggaataaggcgttttatgatgtccggagtcctgccatactatacgggcttcattatccggtttgagccggtgcccggcttctttatgctgtatgtaggcttccagggccgggccggcagccggtactgcgggcagtttgtgttcgtaaaccggttcggccggtttggggccaagaagatacaccacagctgctgtggctataacgatcagggatatacgcaaccacttaggcatcataaggatatttattccagctaaatgtagataagaattctgaaatggcgctgcccggctggtgatttaaccaagaaaaaatccttcaacagcaacgccattgaaggattctttcaaaaaaatatccggaggttatcttcttcttactttctgataaatactcatggcggtaccaatcaccgtaataatgattcccagccataacacgttgatataagggaatatcagcgctttcatcacgatgtaatcgctgaagcccgacgcttcttttaccttcagctctattttattctccgccggcataatcttcgagaaccgtacattcagtcccagtggcgccagggtgtcttccacgctgtattggtagctgctgtcgcggataaaatagatcggctgcagtttaaaatgatcatctgtttgcgtatatacctccagctctgctcctacggccaggtcgccattctgcggaatgtaattgcggctttccggtttggtgtttaatcctttcagcacaataaatcctttggagaagaacaccgaatcgccctgtttcatttcatgggtaacataaggtgtggtatcttctttggcggcttcttcgcggttaggtgcggcagatacgtaggtgaaaatgtccttcgtgaggtaatgcctggaagccgggttggacgacagcgcattttcctttttattcacaaacgcatccgggtaaagggtgaaacgctccagcgccttgccggtttgtttatcctttttctcataatgcactacataatacgttttgggatctccctgcgctacggaatcgccggtataggtaacatgatagtcgcccatttccaccggcacatcctttggcagcataatattctcccgcggattctgtttgctttcctttgtaaaaataccatcgcccagcatcttcatgcggtccagtgaaatcacttccattttggcggaggaaatcagcacgcccagcaacaccatcccaaaaccgatatgcgcaacagaagcgcctgcatttttgattttgcctttcaggccggagaaaatataaaagaagttgcctacaatcgcataaatgctggcaaacaacatcaggtaaatagcagtaaggaaaccggcgccgtaagtatcgtaggtaatagtgcctttccaggccaccagcccggttaataagagcgctacgatagtaggtatcagcagtttcttcgtgatttcgccgcggggagtatccttgtaccgcataaactgcacaatcgccgttaatacacccagtacaatcgcaatccagatctggattttgttgtagtggaatatactgtcagacggcggcgcaatatcgttcatgttgaacgcagacttcagcccggtgaggctcagtaatttattccataccggaatagaagtagtgaaggtaatctggatggctgcaatcagcaggatcagggaacctacaaacagccagaactcacgcgagtagctgttctcttctttctttacggaagggatttcttttctgcgtacaatcagcagggcgatggccggcacagtgaacaccagcatggaaatcagcagctgtgcgctcatgcccatatcggtaaaggagtgtacggaagtatcgcccagtacgccgctctttgttaagaaagaggagtacaggatcagcacgtaggaaataaagaagaagaagaaggtagatttcagcgagtgcccggtggctttatacgccaggagtgtgtgcacgcccgccaccatggtcagccacggcaccagtgatgcattttctacagggtcccatgcccagtaaccaccaaagttgagcgattcataggcccaggcagcgcccatcataataccggttcccagcatcattatggcaaacaaaccccagggctgtaccggttttacccagccggtgtaatcttttgtccataacccggcaaatgcaaaagcaaacggaatgatcatagaagcaaaacccaggaacaataccggcgggtgaatcaccatccagtagttctgcaacgttacattcaaaccgtttccgtcgtggatatgctgcatatagtcagctgtctggaagataggcgccagttggttttcaggcgcttccctcaacagcatgaaaggattgctgcccactttatagcccaggatgaaaatacccagcaacatgctggccatgatcagctgtgcaagggagaagatcgtcattaccggcgcttcccagtttttggaagtgcggatcaggaaaatccccaggatgctgttccagatgctccacagcaggaagctgccttcctggtcggaccagaggctggataacaggtattggataggcaggtcgcgggaagtattgcgccatgcgtatttatattcgaaatagtgattatacaggataaagtagaggcagctgaatacgccgattacggcagccgactgtataacgaaagaccagcgcgccagtcgtttccacgaatccctgatcagcggttcttttcctttaactacattataataagccacggtggctaccatagatgctacaaatgccagtatggcaaagaagtggcctagttggcccggcagtaaatgttcccctacaaacttcataaaattcctctgagagatgtgaatattgtggcattgatcatccgacggcgacaatcatatacatatagctaattatatctgtttgttgctcactgcaacctggtcgtccttatacttggaaggacatttcatcagtattttgctgcagtgaaactcagtgccttccattttaccggtgagtacaatggattcggccttttcaaagtcggtaggttttgcgccgtagaaaactactttatgggattcccccgttttatcgtggacgtagaagctgaacaggttggcatctttagttggatcgtagttcatcgcttttaaggtatcgagtttaccaatcacatggaactctttcccttctttctcgcgggctgttgcaaaagtttcataggtgctgaaatcacccaccatagtcactatcactccaattgccaccgcaattaccaccagcagaataatatttgtttttttcatatgaaaattatcttccctattgattagacacaagctgcaaaaaccctttaccagcgcgacttcaacaactcctctccttttgccgtactttatttgtttccgattaatcggcaaaattaagtgaaaatgaccttcttccgacaaattttatataaaaggtaattctttttaggagaaggacggctgtaagtaaacagaatcctatctttgcgcggaatttagaaaagtacgactttatcatggcagatttatctcaatttgaccctaactcggttggcctgctgtccaacaacgtttttggtttacctttttccgaagaagaggcaagactggtattattacctgttccctgggaagtgaccgtttcctataacaatggtacggcccgcggcccggaacgtatcttcagggcttccttccaggtagacctgtacgacgcagatgtaaaagacggctggaaacagggtttctacatgcgggaaccagacaagcacctcctgctccgcagcgattacctgcgcaaggaagcagaactgtacctgaaattcctgaccgaagggggagatatttctgaaaatgaattcctgaaaaaaacactggtagatgtaagtaacggtaccagggccatgaatgagtgggtgtacatccaaaccaaatcgctcctggaaaaaggcaagctggtaggtttggtaggcggcgaccacagtacgccactcggcttcttcaaagccattggtgaacacaagggcgagtttggtatcctccagatcgatgcacactgcgatctccgcgatgcatatgaaggattcaaatactcccacgcctctatcatgtttaatgccctggcagaagtgccgcagctctctaaactggtacaggtaggtatccgcgactattgcgaagaagaagtggattacgtaaataatagtgaaggccgcgtagtaaccttcttcgataaacagatcaaggaaagacaatttgagggagaatcctggaaagctatctgcgacagcattgtagacaacttacctcaacaggtatacatcagttttgatatcgacggactggatccgaaattatgcccccataccggtaccccggtacccggcgggtttgaggcggaacaaatatattatctcttcaaacgggtgctggacagcggccggaaactgatcggttttgatttgaacgaagtaagcacttcacacgacgaatgggatgccaacgtaggcgcccgtgtgttgttcaaactttgtaacctgttgatcagttccaattcttaatctcacattcctgttcatgcatagtttgcgcatcctgcatccgaatacctccagcagaatccggttattaccggttatgcatgggcttacgggcatactgttcctgtttaatgcgatcggtatttaccgcagtccgcagccgaactggttcctggcgttttttttcctggtagtaggtgtattgtgcatcggctttccttttaccatgagaaggtttaagaaattcaccgaagccaataccgtcgcacggatgatagaagcgctcatctgctttaccggcagtttgtatttcctgtcgcacctcaacccggttaccgcattactgctgttcctggtaggcgccgggctcgcctacgtaggctggatggaacaccgtattttccagccatcgtatgtaaagatggataccaccggaattacccttcctaccaccttttcaaaaaggctggttggctggaacgaactgaataacgtaattttgcggaacgatctgctcacaatagactttaagaacaacaagatcctgcaactcgaaatactggatgaaccaggcaacgaacaaagggaagcactgaataacttcttccggagcagggtgcaataacagtatataaaaacagaaaatgctaaaacaaacaccttacatattatactcagacggtaacggtaatatttttgaagataccaccctgtatgtaaccggccgcagcggctgggatgcatggccggtagaagcagacgaatggattgaattaccggaaggaggtaatttgtatgagttgcccggccgccgtggtattggcatcaacgccgccaccggcgatatgcagctttgtgataaaggatgggccgtagccgcattcataccgccggcgcataccggtttttacctggctgcctacgaaaccatgccggatgcgcctaccctgccgctgttttgctacaccgcagtaggctggctggatggtaagttttatgtgcccgccacccgcattgaagcagatatccgccaggaatgcgcgggctttgacgataaaaaagtgaaacagggcgtaaaaaccctggtggaagcatacccgcataacaggctggtacagcatctcgcggaaaattgcgcgctcacctatgagtgtcctgctgcccgtaattattttatgggaagatgggagtgccctattccttcctctcctgcatgtaatgccaattgcgtgggctgcatttcattccagccggaagaagaaagcattgtttccacgcaggaccgcctccgctttaaaccaaccgcggaagaaattgtggagtacaccgtacctcacctggaatcggcccccttccctatcgtaagcttcggacagggctgtgaaggcgaaccactgctgatgtgggaaaccatccgcgaatccatcctggaaatacgcaaacacacgcctaaaggcagcatcaatatcaataccaacggcagtaaaccggatgcggtaagagccctgtgtgaagcaggcctgaatagtatccgcgtaagcctgaactccgcacaggaaaaatattacaccccgtattaccgccctaacaactacgtttttgaagatatcatcgaaagcctgaaagtagtgcgtgaattcggcggctggacctcgatcaactacttcgtatttccgggcatgaccgatagcgcagatgaatatgaagcgctgcgtaaactgatcagggaaacagggttgaatatgatccagtggcgtaatttcaatattgatcccgactggtacctcggtaaactgggcgtaacggaaacgggcgaatgcttaggggtaaaacagctgcaggaactgatccatgaggaattcccggatctgaagttcggttactttaatcctccgatggagcgtattacgggcgattatatgagcgacttcgctcactgagaatagaactctttatattaaaaaaggctgaccgcgatggtcagcctttttcgtttaacttactttagttcttccgcaaagcggtattgccttgcatacgccgaaggcgacattcccgttaccttccggaatacccggttaaaagtaatcgggttgttatacccggtagcataggccactgctgcaatactgtcgaagtcaccgttaataatattcttgcacgccacattgatcctgatctcattcagaaattcaaggtaggttttgcgggtatgttttttaaagtatttgcaaaaagcataagtagtaagatgcgccacgccggcaatttgtcccagcgaaatattctccgcataatgctccagcgtatattggtaaatatcattcatccgcagtccttccgactcgctgtaagattgcctggaaaaccccgtggataacgacttccaatccttcacctgtttagagaaatataccagcatgcccacaaacgccagcaacctttcggcgccgctgagccgggagatctttaatatatcggcagctgttttttctgcgtattcggccggcagttgcaaactgttggcgctgagttgcaggaactttcttaccgcctccatttctttcagggaaaataagccctgtaatgcatgttcatgatcgaaaaagatatggatggcgtggatattcttctcctgtaaattttcgaaataccgcgcatcccctttaaacatatggggctggttggcgccaatcacataaatatctccggccttgaaaggttgggtatagtttccggcaatcagggtgccttctccctttataataagtgttacctgcgcctctttgtgacgatgcaggtaattataaaagtaagggaggatatcttcctgtatgactacagcaccttcatcggcaacggggacagtaaattgaattactttcattaaccaatattactaatttacctgcaaaattagcaattatgtggcaataatggtaaagtgttggacaatatcatccattgatttgttttctgcccgtccctattttttgctgcaaccacaaaaaaccgccgcccgacaatatgcaccccagcgctgtaatcccccaccacggcctaaacccaagatgctgcaccacaaacgcccccgttgtgggcgatacaatattggccagcgaatacgaaatggtatacaacgcggcatactgtccgcggttatggtccaggctcctgccgatccagaaactgttcataaaggggaggcaaaacatttcaccgaaggtgatcaccaccataaatactactgccaatgcccataccggcggcaggaaacaaagtaacatataggacaagcaaaccatcatggcgccgcgggccacaaaggacaggttaggcattttcccgtcgaggcggtacaccattaccatttccaccagcgcaatcaggatcccgttaacagacatattcagaccaatagcccactcttccaggtgcatcacttctttaaaatataacggcacaatgctggaaaactggaacaggcagatggcatttacggtggcaaaaagcaggaaccacaggtaaatatgatccctccataccttctcttccgcttttacggctgccttggcagcctttggcggcgcaggtaccggcggcaggaaaatccgcatcaggatggccgccagcatacaggtgaacccgtctacccagaaaagcagctggtaactgaaactggcaaggataccgccgatagcaggacctactgaccaacccaggttcaccgccagccggttcagggcgtacgaccgggtccggttttccggcgaactgtaggcggcaatagcaatgctgttggccggccggaaggcatctcccacagaactcattacaaatacgcagatacatatttgctcaaaggtgcgcatctgacccaataaaatgaataataatccgttagagaaaagactccagaactgtacctggtagaaaccgatcttatcagacagccatccgcccagcagggcgccaacaatggcaccggtaccaaaacaggccataaccaggcctgcctgggcaatactgaaatgaagatgttgtgtaagatatacggtcataaagggaatgaccatcgttccgctcctgttgatcagcaatacaagcgagagccaccaggtagcaggagcaagaccagtataggcattttggtaaagacggatcgtttgtctggccaggttcataaaatcggtgaaaaataatttacgataattggattaacagcacagtttttgcaaagatccggaattcatcttttgatgagcgattattttttctggatcaaaacattaactttggtctgaacaggcactcaataaggttatcatggaggaaaaaaacggtaaaaaaaatatacaggctttaggaatcactatcggcgtgcatgcattgctgttagtagcgctggtatttaccggtttttctgcacctccgcccttaccggatcaggatcttggcatggaagtaaaccttggcacatccgatgatggcatgggcgacgaacaaccattgaaccctaatccgcccagtgctgcagcgccagaaccagcagcagctgaaagtccggctgctaccgctccggccaacactgaacctcagcaggatattgctacccaggatgaagaagaggccccggaaataaaaaaaccggaaaaacctgttgagaaacctaaagagattccaaagaaattagaaccaaaacctgttaagccaacaaagaaacctgcagaaacgccaccggcgcccacaccacccgcaccaaaaccaaaggcggtgttttcaggcggtaccggcaacagtgccaatagcggtaacagcgccaatggctccaataatgccacaggagaaggtaataccggcaaacccggcgatcgcggtcaactggggggtaaccctaacggcggcggatatacgggcggtggactcggcggcggacgctccgatttccacctcaatggaagaagccttatcggcaggccacaggttacttacgacggcactgaaacaggctatgtagccatcaatataaaagtagatcaaaagggaaatgtgacatctgccacttttagtatgaaaggatctactatcagtaacccccgcctgattgagattgccaaaaaggctgcctccagcggacaactgaaatacaatgccaacccggatgcaccagaagaacagttcggagtgatccgcttctttttcaaagcagaataagcagcgtaatatatacagattttaaaagaggctgttttatttaccggaccaggaactgatccggaacagcatagcttcatccagaaatctgtcgttcctacatcatctttacctatgattgcaacaactgacaagagcaatttttttgtgtcatttcgaggaacctattttttatcgccaacgatgattgtaaaacttaaccgtatcttttccggcaccgcaatattgctcgtgctgatgcaggccgctgtggctcaaactttcccgggttacaataacagtaactacgcgggtatttatggtgtattctccaacccggccagcgctgccggctatcgctataaatgggatgtaaatattataggtgcggatgtaaatgccggcaacacttatgtgagcgttccgaaatcattgctgtttaatattcctgatacgctgaaacgcaaccaggattatttcctcgatgaaggcgccaacaggaaacaaatgggctggcaaatggcggaaattgcactaccttctgtattatatgctattgatgaaaaacagtctgtttcctttgtatggcgtatgcgcagcagcagtagcggcggtaatttcacgacccccatcgccaatttctttggggtggatttcccaaatccaggttatatcaacaccaatttaagcattccgcgtgcaggcgtttcctcgcatgtatggcatgaactgggcttcagttatgcacgcaccatcaaagaaacttacagcggccggtggaaagccggcgttacactgaaactgctcagtggcgtggctgcgggttacgctgctgttaagggcgttgacttcaggctaaactcatcaaaaagtgccactattaccagtggtaccctctattatggctataataaagaaatggacgactggcagtcgcccgcacaaaaaaacctccagttattccataacaacggtatcggtgcagacatcggcgtgatctacgaataccgccccgacaacggcggctttggcgcctctgaaggctctgatgcagatgactataaatttcgtataggcgcttccattaccgacatcggcaggataaaatataccaaagcgcctattaacacggacctcagcctggtaaaagacaatgtagtaccaaaggatgtgcagtataagaaaaatgaaagtctgcagcaatacgcccgccggctcaacaattattttacgccactgggcaccgattctactttcaatatgatgctgcccacggcgctcaacctgatgggtgattataatatcgacagccgcttttttatcagcgcacatgcggttattgcattaaccgccggcaaccgcgatatctccaaaacatatgcactaacacagtttaatattacgccacggtatgaaacctacctttttggcgcctatatgccattcactattaaccgtaacggccaggccgatgtaggagcgggtatccgcataggtcccctcctgattggctccagcacaattttcaccaacctctttcaaaaacatgtcgatcgtgcaaatgcttttgtagctttgcgcttaaattcaagcatgttcgaacggggtgagggcggtgggctctttaagaagcgtaaccgccagttggattgcccggtggttaataattattaatatggcctcttacaaagaaacgctggactatctctatgcacagctgcccatgtttaccagagtgggcgccagtgcgtttaaaacagacctgcataataccattgcattactggatcagctgaaccaaccgcaacacagctttaaaaccatacacgtagccggtaccaacggcaaaggctcttccagccatatgctggcagccattttccaacaggccggctacaaaacaggactttatacttccccccacctcctggatttcagggagcgtatccgcatcaacgggcaaatggttccggaaaattttgtagttaatttcacagaacagatgcgcgggcatattgccgacatccaaccctctttttttgaactcaccgttgccatggcattccgctacttccagcaggaagcagtagacattgccatcattgaagtgggcctcggcggccggctggacagcaccaacgtcattacgcccgaactgtcgctgatcaccaatatcagctacgatcataaaaatattctcggcgatacactcccgcagattgccagtgaaaaagcaggcatcatcaaagccggtgtaccggtagtgatcagcgaaacacagtctgaagtacaggacgtgtttattaataccgccaacgcgctgaatgcccccattcacttcgcagaccaggaatggatggaagcttccggcgccattgaaagcaatcactttactataacgttactggatacacgacaacagcagatgcgccgtttacaactggatctgaccggtcagtaccaggaaaaaaatgtaatgggcgtattgtcggccgtaaaaatattacagcaaaaaggctggcatatcacctgggatcacatcagccacgccctttcccacgtaaagaaactgaccggcctgagaggccgctgggaagtaatacagcggcatccgctcactgtactggatgtaggccacaacgaagccggcatccgcgaagtgatgcagcagctcggacatgttaacttccagcagttacatattgtagtaggatttgtgaaagataaggaagtagaaaaagtgctgccattattcccgcctacggcgcattattatttctgcaaagcacagatcccccgtgcattggacgaagtagcactggctgaaatggcggcggtcagcgggttacagggccatgcttacccaactgttcaggcggcgctgcaggcggccaggcaacatgcccagccggatgatatgatcctcgtttgtggcagcttttttattgtagcagaagtgatgtaagttatttcatcgtcattttaccgagatacagcaacgcgtaaaagatacaggtggtgtgcaaactgtgtactattttgttatccagtaacagttgctgtagttcttccagcggcataatcaccacttcaatatcttcgttgtgatccaattcctgttcctgtacctttacccctcccgttgccaggaacatatgcgtgtagttgttgctggaagccgtattaggcgcaatggtgccaagcgacacccattccttaaatgcgtacccggtttcttccaacatctcgcgtttcatggcaaataaaggatccggatctgtggggtccatcgtgccgccaggaatttccagcaacgttttgcctactccctgccggaactgccggatcatgattacctgcccgtcttcacgaatcgccacaccgtttacccagttgctatactccagtacgtaataaggcgccacaattttacctgcgggcgtttcgcaggtatcgatacgcgccgtaagccaggcatctttaaaaaggtattccgatgacagtaatttccagtccatattcataataacaatgctttaccaatccattcgttctttcaggcgcaggatatgctccaggtgatgtttaccatgccaggcgtaattggcggcatgggtttttaaatgatgactggtgccattggcaggatgtacaaaagtacgttcccagtcggcatccgataagtgctccatcaaacttacccagcggttatgcagggcatgcagcagggtgatagatacgtttatgggtgtaaacttcacatcaggaagttccgcccatagttgttcctcgtaaggttttataaccggctgttcttctgtgagggccagcttcatgcgggtgtatccgttcatatggctgtcggccaggtggtgtaccacctgcgctactgtccacccatccgggcggtaaggcgtttgcagctggtattcgtccagttgctgcacggcgatttccaccagctggggcaaatagcggatgtcgttaataaatccccgcaacatttccggtgtgtagtccggcaatgcttcaaagcggccaataggatatttcagtgattccatccgttaggtgttggtttattcttcgcgtaagtctttccccgtgagatgaatgaatacatcttccaggttcgctttcttcacctccttctttctttcaaaaccggaagataccagtttatcaatcaatgcatcgggcgagtcgatagcgataataagaccgctgtcgacgatagcgcaacggtcgcagaggaattctgcttcatccatataatgggtggtgattaccacggtggtaccctggctcctcacctgctggatcagctcccacaagttgcggcgggcctgtggatccaggccggtagtgggttcatccaggaaaatgatctgtggtttattgatgagcgtagtggcaatggaaaaccgttgtttctggccaccggaaagttctttgaattttgctttggctttatcttccaggttaaacatccccaggagcttcatgggctccacgggctggttataaaggccgccaaacatttctatgagttctgtgagatttagtccggggtaatagccggaactctggagctgtacgccgatgatctttttaatatcgttggggtctttgtcgaggtcataacctcccaccatcactttgccggctgttttttcccggagggtttcaataatttccagggtagtggatttaccggcgccgttggggcccagcaggccaaagatctctccttcaaacacctcaaagctgattccttttaccgcggtaaactccccgtatttttttaccaggttgcttacctcaatgatctttttcttttccatggggccaaattacagaaagaatgcgaaaaaaaagagcctctgaacgaaggggacggccggtggctgtccccttcgtttcaattattgcttgataaacacctgcgtaaagaaggtaatcctccccttatcggcggtgccgataccaatgagcgtataatcgcccagcatatttttgcggtgccccgggctcttgatccatccatttaccacggcttcggcgtcgagagtgccataagctacgttttcagcggcgctggctacgcggcccatctttttggatacgttggctacgcgttcttcaaatccctcatgaccaaaacctgtgctgccgttggccatatcccggctgtggcggcgggcctgctggctgatggtggcatccagctgtaaaggcttcagccctttggactgacggaacttgttggtgtagtaaagaatctggtcatccatgctggcacctgcattactgctgtctgccgcatgagtggcacgtgagcacgcgctaacctggaaaacggccaacagggcgactaataatgcaatgatccgctggttcttcaaaatcgacatagaaataaaatggttaataattaaaaatgaataaagagtactaatatgactattaaaaccaggccaggtttagcaagccgggtgccagaaattaaaaacggtgtataatggacattttgtatccgctatacaccgttttttgtaatatttttttaagcctactcgttcatgatccgctgccaggtatccatcattgttttggaccctataaagatggccatccgctggtgcagctgtaccggtttcaactccaggagccgctgtttaccgttggccatggccacgccgcccgccttttccatgataaacgacataggattgcactcataacaaagccttaaccggcctgccgggtacttaccaaaagccgggtacatgaaaataccaccctggataagggtacggtgtatttcggccaccatacagcccacaaaccggtggcggtaaatacggtcattttcattcctcgccataaaatgatcgatcgatttacggattttctgctcgtataggtggtaataacccacattaacagagaaaatatcgctgtcgggcggacatttcaggttggggtgcgacaggcagaactccccgatagacgggtccagggtgaagccctgcacgctgcggcgggtagcatataccatcatggtagaggaaccataaataatatacccggcggcaatctgcttggtgcccggctgcaggaaatcctccagttcacattcagagccctccggcgtaagccggcggtacaccgagaaaatggtaccgatagatacattcacatctatattgctggaaccatccaggggatccagtaacaccacgtatttcgattttttggaatgctcatcatgaaaaggaataaagttttcattttcttctgaagccacgccacagcagtaaatactggtttccagtgaatcaatgaactgctcattggcaaattcatccagtttctttactgattcgccctgcacgttggtccggccggcttctcccaggatgtcggcaataccggctttatttacttccacatttacccttttagcagcgaggccgatatcacgcagtaaaccggataactgaccggtggctcccgggtaattccgtaactcctggatagtaaattcatccagtgtcattactttttgcttaagattcataacgttaggttgtatgggcgaatttagtcaattgaaactattttaacggaactgtcatttatctgcaaacagattttaaaacaattctaaacttgtcttactttgccgaataattttttaaaagaagataaactatcatatgaaggttttcaagtttggtggcgcaagtttagaaagtgttgaacgtatccggcaggtggctcagattgtacagtcatttccggacgaaaaactcctcattgttatttctgccatggctaaaacaaccaatgagctggagaaagtagcacaaaactttttcctgcgcaaacgggaaattgccgcgcagcttctctttaacatcgaggagcaacatgtgaatgtagccgaagccttgctgggaacaaaggatcatccattatttatccaactgcagcagtttttcaccgaagctgaatggacactgggcgaaaaacccctgcgcacctatgattactattacgatcagttggtgagcctgggtgaactgctgagtacctctattgtaagcgccttctttaacagcgtgggtatccacaatacctggctggatgtgagagatattttccgtacagacgacaacttccgcgacgctaatatcgactggatctatacccagcggcaggtaaccgaaaaagtggttcccctgttcaacaacaccaatattgtgattacacaaggctttattggcagcaccgaccagaacgaaagcgttaccctgggccgggaaggcagcgattactccgccgccgttttcgccaatatgctcgatgccgaaagccaaaccatctggaaagatgtggaaggattgaaaaatgccgatccaaaactgttccccaacaccgtgaatataccggagatcagctacagcgaagtgatagaaatggcctactatggcgcccaggtgatccacccgaaaaccattaaaccactgcagaacaaacagatccccctgctggtgaaatgtttcctggataaaaacctgcccggcaccatcatcagggaaaccgcagatgtaaaactgctgcctcctatcattgtgctgaaaaagaaccaggtgttgctgaatattacctctaaagactactcttttatcacagaagataagatcagcgacatctatgagatcttccacgggctgaaggtgaaaattaacctgatgcagaacggagccatcaatttctcctgctgtatagataataacccggagaagatagaactcctgatcaaaacgctccacgagcagtttaaaatcgtttacaacgaaggactggagctgcttaccgttcgttattaccaaaccggcctactcgaagaactcagcgacggtcacacaatattattagaacaacgttcaaccgccaccatacagcgtctctggaaaagataaatttatccagtaaaaatattatcacccttcgtgcaacttttttcgtacccgttcgtctttagtaaaaatgtggtatgaaaaaagttgctatcgttttaagcctgagtaccgtggtgatgctgatcatagcatgcggagggaaaatggtcaaccgtggctacctttccgccagcaacccggatgaattgcctatttacctgatcaccctgggatatttcagggaaacacctgcttgtcccactaccccatcgtcgtgtatgatgaataaaacaacagagatgcccctcggcaaaatacaggatgttttaagatcggcgcttcaatactaccaggaaaactgcagcaggaaataacagacccccttttttggtactagcttttgagaaaatttacaacggaaacgatagtatgagaacaatcatcgtagccctgggaatgctttttattggtgtgcacgctaccctggcacaacaatccaattccacaggaaaaattacactgacaattacagaccatgaaggcaagccgctcccctttaccagcgtaatggtgaggaatatcaaagattcttccctcgtaaaaggagaactgaccactaccaacggcagttgtgcctttgaaaaaatagcctttggccattatttcatccaggcctcccagatgggatacaacaccacctacagcaaaacatttcaactcaacgccgctcataaaaacgttaccctggataccatccgcctgaacactttaggcaaaaacctccaggccgtgaatgtaaccgcccagaaaccttttattgaaagttctgccgggaaaacagtcatgaacatcgagaacagcgtgagcgccgccggcaataccgcgctggacctgctccgccgcgcaccgggagtacaggtggataacaacgaaaacgtaaccctgaaggggcaaagcgttacggtaatgatcgatggcaaactgacctacctcagtggcgaacaattaaccaatctcctgaaaacaacacccggagaaagcattgcttccattgaaatattaaccagtccttctgctaaatacgatgcctccggtaacggcggtatcatcaacataaaaactaaaaaaggaaaaatgaccgggataaatggtaacgtgaatgctacccttacccagtcgagatacggccgctatggtatttccggtaatgttaactggagaacggaaaaattcaacctgttcggtaatttcgaccagggcgactatccccgccaggttacccgcgtatacagccggaacgtaaaggaaaacgatggcagctccacctatcttcagcagaatatatttcagcgtaaccgctttaaaaataactacctgaaaataggaatggattactttatcactgataaacaaaccatcggcgtactggccaacggctataaaaacgccttcagtaaccagatctacagcaatgccgaccttggccgggttaatatgccggcagattccaccgtgaactcccttaccaccaacaataacaagttcgataacattgcacttaacctcaactacaaactgatcctggatactgcaggcggaagggaaatcagttttgatggggactatgcacagttcaacaaccaccgctttatgcagctgaatgacagcctgtatgacgccaaaacacagttgaaccgcaaccccaacagcatccgcaccaccggaggtacacaggtaattatcaaaagcctgaaagcagatgtaagctggccgctcggcaaggaaggtaaactggaagccggcgctaaaaccagcttcgttaccaccaccaacgtattgcaattcgactccctgtttcatggcggctataaaccttcccccggattaagcgaccgctttaactaccaggaaaatatttatgccgcatacgccacttacaaaaaacaaatacataaaacgaatctgcagctggggctgagggtagagaacaccgaatctaccgggacttcttttacgaccggaacaaatgtgaaacgctcttatgtcgacttctttccaaacatcaacgtggagcaaaagctgaatgataaaaataagctgagcctggccatgtcacgcaggatagaaagaccgcagtacggtcagctgaatccatttatgttttacctggacaagtatacctacttccgggggaatccttacctgcggccgcaatacagcaacatcgcagaagttgcctatacgttcaaagacaaatacatcgccactttccgctatagccggattaaagatatgatggaagaattcattacacaggacgacagtaccaaagcctccatcagcacggaacgcaactatgataaaacagatatttacagcatcctgtttacgctgcctttccagtttacaaaatggtggaccagcgacaacaacgcagatttctcctataacaaataccgttttgaagatcccgtaacgaatgatccttattaccggtataacttcaattattatatcagcagcacaaatactattactcttccgaaagattttaaggtagaagtaatgggctactataactcgccttttatttttgggattttcaggggctatgcacagtataacctgaacctgggcgttcagaaaatgttcctgaataaaaatgccaccgtaaaactgagctataacaatatcctgcggaatgaaagctatcgcggggccgcagaatttgccaacctgaacatgagcatcttcaatacctggcagttccgcacggtaaacctttctttcagctataaatttggcagtgccaccattaaagcggcccgcgaaagaaaaaccggtaccagtgatgaacagaatcgtgcaggttaaaccaggatacgcatcatttgctgaatcagcgccatcatagcagtaggatatacacccagccctattaacagtatggttaaaatcaccagggtaatattaccggccatgggcagggccggtatcaccgttgtttgttgcccttttgcaggcaccgcaaacatagccgccaccagccggatatagtaatacaacccgatcacactgttaatcaccagcataaacaacaggaaccactggtgcccgtccacgcccgccagcaccacataaaacttaccgataaaaccggcggtaagcggaatgcccgccagcgataacagcatcgccgtaaatacggtggctacccagggataacgccagaacagccccctgtaatcagcaatcgtttccgcatcctgcgaactgctcgacattacaatcaccaccccaaaagcgccgatgcttgtaataaaataagctaccaggtaaaatgccagcgcctccagcccggtttgcacacccgataaaaaagcaaccaggatgtaacccatatgcgcaatagaagaataggcgaggatacgtttgatattctgctgtgtgagtgccagccagttgcccgcaaacatagacgctaccgcaataatagctactatccaccacaacatcgggtagtcgttcccatgaatgtcctggtaaaagcggatcagcaacaccagcatggctcccttggaaaccgtggcaataaacgccgccaccggcaacggcgcgccctcataaatatccggcgcccacatatgaaaaggaacaatgcccagtttaaaacccacgcctatcagcatcaaaccaaaacccgccatcacgctcaccggcaaataacccgcctcacgtaaggctgcccctattcccgggaaatccatatggcctgtaaaggcatacaccagcgccattccaaacagcaggaaagcagacgacaacgccgccagcatcaggtatttaatccccgcttcatcagaccgctcacgggcacgcaggtacgcaattaatccgtataaactgatgcttagtatttccagtccgaggaacagcgacataaaatgccggcttaccaccagcaccaaagcaccgatagtagccaggatcaggagaatgtagtattcttccttccgctcttccctttcttcaaaataattaaatgacaacaacaggataataaaccccgacacgaggatcaacccggaattaaagagtgaaaactcatcgatcaccagcagcggtggcacgggatgaggaatatacttaatggcaggaatcaccgccgccatcgccataccaaaagcaagaagggaaaagctgtacacgatgcggtgattacgccaggctgcaaccagcaacatggctatcactgccgcagcacatagggtgatcagcggccccagacttaaaaaatcagcgaacgacatagtcaatgttttgggaagtattcaataccggttgcggatggaagcccagccagcatatcactattaccaatgctattatgatcaccagctcacgcccgttcagatcggacatggcatattgccggtcgcacggaccgaagaaaactttctgcataatacgcagcgaatacgccgttgctaccaccaggccaatagtagccaggatagtgagcacatgactggcctgccagctacccagcaacaccaggaattccgctacgaaattgcctaatcccggtaacccgagagaggccatcacaaaaatcatggcagcgctgcccatcatgggaagccgcagccaaagcccacccatttgccggaggttgcgggtatgtatgcgctcatacaacgcgcccgcaataataaataacgcacctgtactaatgccatgtgtgatcatttgcatcactacgccctggtaagcaatttcattcagggcgaaggcgcccagcagtacaaagcccatatggcttacgctggtgtaggcaatcagccttttaaaatccgtttgcgcataggccagcatgcccccatacaggataccaattacgcccagcaacatggccaccggtgctatgtctgcggcggcagtgggaaacagcggcaacacaaaccggaggataccgtaagcgcccgttttcagtaacaagcccgccagcaccacgctgccggcagtaggcgcttccgtatgcgcatccggcaaccaggtgtgaaaaggtactgccggcagctttaccaggaaggcgatcaggaaacccagcatcagccatcgctccatagaaggcgtcataggcgtattcaacagctcaaaataattaaacgtatatacattagtgttagctttatgcacaaagtaaagaccgagtattgccagcagcatcagcaagcctcccgcctgtgtgaacaggaaaaacttgttggccgcatactcccggtgttcatgtccccagataccaatcaggaagtacatggggatcagcatcatctcccagaaaaaataaaacaggaaaagatccatcgtcaggaaaacgcctgtgatgccacaaagcacaaacaacaggttaaagtgaaagaaccccaccctcgtttggatttccttccaggaaattaataccgccagcgcccccaggaaaaatgtcagcgccagcatcagcatacttaaaccgtccatcgccaggtgcaggctgataccgaaatgcggcacccagtccatccggaactggtaccaccaacggctgctgctacccgtatgctccatccatacccctgcgataatgccgaggttcaccagcaggctgcatagggctatccaccggctggcagcgtggcttttcacgccaaccacccacgacaataacgccgcgccaaaaaggatcaatatcaataccagcaatatcataattgttcgtttaatcgttcgggttatatgtatatccgccagatcagcaccgacaatatcgccaccgcacccagcactacgccaagtatataccatctcagcaaaccgctctgcgtacgtgcgagcacgttatgacaccattccataaacgccgccagcccgatataaaacgtgtctatcagatcccttctgttgatacgcgacaagtacacaaaagggcgtaccagcagcacattgtacaattcatcaaagtcccatcccctgctccagtagccacgcagccacataatagcaggcatttccagaaaatcagacatgcctttgggatgcttcactacccaggcatacgccagcccgatgccgcccagcgccagcaaggccgataaggcctgtgaagtccattccatagaaagactttcatgcagtaccgtcaccgccggcaataccggttgcagccagttgctgaacaacgttacatgccccatcgtatgcggcaattctataaacccggcaaccgtagataataccgccaggatatacagcgggatcatcatactgctccccggccggtgatgcacctttgttttctcttctccataaaataccaggaaaaacatgcggaaagtatacatacccgtgagtaacgcacccagcagcgccgccagccagaagccaacatgaccaccggcagcggaccacgacaaccaaatgatctggtccttactgtaaaagcccgctgttataaaaggaatagccgcaagggaagcacagccaaccaggaatacccagtaaacgccgcgcaactgctttttcaatcctcccatcttaaacatatcctgctcgtgatgcaacgctacaatgatagcgcctgcggccatgaacagcaacgccttgaaaaaagcatgcgtaacaaaatgaaataccgccgccgaccacgcgccgcagcccagtgccaggaacatatacccgatctggctcaccgtggaataagccagcacccttttaatatccgtttgcaccagggcgctgaaacccgccagcaccaaagtgatagcgcctatcacagcagtagtggtttgcgccgccggcgccagttcaaataaagtatgcgtacgcgcaatgatataaacccctgccgtaaccatggtggcggcatgtatcaacgcactcaccggcgtagggcccgccatggcatccggcagccaggtttgcaacggcagttgggccgacttgcccaccgcgccgcccaacaacagcaaagcgataatggttaccactccatcgttcacagaccagatttgtgtactgttttccaatatgccgggaatactcagtgtaccggtatactgaaataacataaacaaagcaatggccatcgcggtatcgcctatgcgtgttacaataaaagctttcctcgctgcatacccgttggcaggatctttataccagaagccgatcagcaggtaactgcaaaggcccacaccttcccagccaaagtataacaacaataaattatctgccatcaccagcgtaagcatggcgcctacaaataaattcatacaggcaaaaaagcgggcgtagtccggatcgtcgtgcatataaccggatgcatatacatggatcaggaagcccacaatggtgatcaccagcacaaataccaccgacagcgcatccatccggaaatcgaaacctgttttaaatccaccggcttccagccagttgccggcatgctgaacaatcgcctgttcaccatttgcggcaaattgcatagcgatgataatagccactattgcagccagtccgatactgccgcatccgattacggtaacgcctatacggtcgaaacgcttccagcccagcatgagcaggaaggcgctgataaaaggaatgagcggtatgagtgcaggaaacatacaattgaatattttatccgttcatttttgctgcttcgtcgctgtccagtgttttgagctgatgatataactgtaagatcaatgccagtcctaccgatacttctgccgccgccatcgccaggatgaagatgaacatcacctgcccgtctgctgtaccccagtgagaagaagccacaacaaaggccagtcctgctgcgttcagcattatttccaccgacagcaacataaaaataatgtcgcggcgaaccagtatactgatcagccccagcacaaataaaacgccggcaagcagcatgcccgctgtggtaggatgtactatcatgattgattattttcaaggaaccggtgcaatgttttctctttctgacgccctaagtggtaagcccctacaatgcccgccatcagcaacatcccggtaagttccaccgccaggatataagggccgaataaagcaatgcccacctccttcggattcacgatctgaatacctgatacgggctggcggttctgcaacaccaggaaaacaagctctccaagcaggatgatacaaagcagcgatggaaagatccagatgcgcggcttcagccatagccgctcctgcgcggccgactcttttcccaggttcagcatcatcacaaaaaagatcagcaataccataatggcgcccgcatacacaatcacttccaatgccgccataaaaggcgcgccatagagatacaacaccactgccaccgccagtaaagacactacgagatataacaaggcatgcataatgttgtaccgggtgatcaccatcacggtagataacactgcaatcaatgcagcaatataaaatgcagttcctatcatggtatcaggcttttaatatctaccggtggttcttcgtgttgtgcatcgcctttgtcttttccgcgaatggccataccggctatattgtaatagttataacctggatatttgccttcactgttaatgagcaggtcctctttttcatataccaggttctgacggttatattctgccatttcaaaatcgggcaataactgtatcgcgtaggtaggacaagcctcttcgcagaagccacagaaaatacagcgggagaaattgatccggaaaaactccggatatcttctgcccgattcatcttccgttgcctgaagggagatgcagtctaccgggcaggccgcggcacacaggtagcaacctacacatcgttcgcctccatccggatcgcgggttaacgcaatgcggccccgccagcgggccggcaacggcgcccgctgttcaggatactgaaaggtttcccgcttgtggaacatgtgcaggaatatcagccacatacttcttaccagactaaacatgttttttgttttaagtatttaaccacagcttaatggcagctgttaccatcaggtttaaaatcgataacggaaacaataccttccatccatactccatcaactgatcataccgcggccgcggcatagatgcccggaacaggatgaacaacatgataaaggcaaacgtttttattacaaaccataataccggcggcagaaaagccggtccaagccagccgccaaaataaagcgttaccagcatgccggagatcagcgttacgcccaggtattcaccgatgaagaacataccgaacttcatcccggaatattccgagtgaaagcccgctaccagctcactctccgcctccgggatatcgaaaggtaaacggtgtgtttccgctacgcctgccaccagaaaaatgaggaagccgataaactgcgggataataaaccacaccttccgctgggcttccactatttcacccagattaaaagagccgctcagcaccaccacgcccatcagcgccaatcccataaacacctcatagctgatcatctgcgaagccccgcgcatagcgcccagcaacgcatacttgttattggaagcccagccgcccaacactacactgtatacgcccagtgaagacatggccaggaaaaacaacaggccgatattcaaatctgccaccacaattcctggtgcaaaaggtatcaccacaaagctcatgagcacactcagcatcactacaccgggcgcaaatacaaacactactttatcggcaaatggcggaatccagtcttccttaaaaaacaacttgatagtatcagccagcaccaccaacagcccgaagggccctgccctgttgggaccgtaacggtcctgccacagcgccagcatccggcgctccacccaaataagaccggccgccgtatttaacagtgcaaaaagcacccctcctattacccaccaaatgtttatcatagcattatacttttatcagttgcggcgcctctgaaatctgcatgccgggaaggcctacaggtattccggcaacgccttcctgtaatgtatcgttaatgatcaccggtaacgtatagtgatgaccgttatctgtgaaatgcagcaggtatccagcggttacctgcaaccgttttgcgtcttcactgtgcagcataatgtagggagccggaatacgttctgcaatacccggtgtatgcacgctcagttcttctgatccgaaaatatgatagagtggtaccagtaacagatgttctttgagcggcagaaagggctccggtacttccgtataaaaaggcgtttgcccgttcgcgtgaggttcaatcaatctcttgccggagttgccatcgtgcagcggtccgcctgtttccacctggaatttgtttactgattgcacagaattccatccgggcgaccagaaaaagggaatcatggaagaaggcggctctccccggtacccttccatggtaaaggacagcgcggtatctgtgtcctgtggcggacggggctcgcttacatctacatttgcctgcatagcggtacggccgctaaagcgatgtggttccctcggtaccttctgaccggcaattcgaaaatcagcatgcggcgcgagatgatctatactttcaaatttttcgtatgcgtgtgcaaggtgattcactacttcatcgaagtgttgcaaaccggagagtgtagcatgccccttaatgctggcgatctgcaacagccagcgccagctttcctgcactgcggagtcgggtgcaaacacctggaaaaagcgctgggcgcggccttcattattcaccagcgtaccgtccgattcagcaaaggtgccagccggtaaaatgatggtggctttctccgctgtgggattataaagatgatccagcaggatcacatctttcacctttccaaaaaactgttctgcccggtgttggttcagccggcggtacaggtcattttccaaaacgatcacggtatccacttcgctattcaaggcacggtctaccgccgaatccaggcggtggccacccagcatttcaagtcctacgctgttgcattccggcaccgtgtaggtaagcatggcatcgataccaagatcccgcagggaccaggccacattggcggcggctttgatgatggcttcactgccaccgccatagcctgcaatgataagcgggttcttagcggttttcagcaccgctgctatttctgcagcaatggctttcccttgctccgacattccttttacttcgggcattttactgctcagcaggtgactaacgccaaagcctatacgggcaatattgtccggcgccgtgtgataagcaccttttgcaagttcatcgagtttggtttcctggacatttaaaatatagagggggcctttgctgtcctgaacggcttcccgtacggcggcatcctgccatgcgggcatgtgaatatgattgatgacatcttccaccgggatacggcgtaccgcctgccgcaccgacaaggccagcatcggcgccgtattggttacatcttcaccgaggataagcactacatccgctgctgccgcttcctgcagggaggcgctgcgcaccggtccctgttgcagtattttgagagaaagggataccaggtcgtgatctgctgctgacacacccaggtagaagttgtcttccccaaccagttctttcagcacagcattggattccagggaagctctcggcgatcctatgccgatggtcttccctggtttcatccgttgatgcacatgctgcaacaccgggatgccattggccttatctgcagggccgtgatgcaccatcggtgttttgatccgttgtccgctgttcacaaattcgtagccatagcggccacggtcgcaaaggaaataaccatttaccgcgccattaaaccggttagtgatctgtcgcacggcgccataacgctcaccggcgatgatattacagcccagtccgcagccctggcatacagaagcagcagaggtcagatcccatttacgggtataatgctgcttgagggttttatccgtaaacacaccggtagggcatatttcggcaagattgccgctaaactcgctttccagtgtaccctcttcctgccggccaaaatacacatggttatgcgcggcgaaaacatccaggtccttaccaccggcaaagtctttataaaacctcacacaacggtagcactggatgcaacggttcatttcatgattcaggaatggtccgagatattggttgttgtaagttcgttttgtaaaatggtaatcacggtaagagtggcctgtcatcaccgtcatatcctgcaaatggcaggaaccgccttcatcacatacggcgcagtcgtgcgggtgattggtcatcagccagccgatcacatgctcgcggaagttgcgggcatcggtatcgtcaatggataaacgaagctggtcttttaccggctccatacacgacataatgatctttcccttcttatcatcttcatccttaaacaccttaacagcgcattgacggcaggcgcctaccgcacccagggcggggtgccagcaaaagtaaggaaggttcaaacccagcgacaggcaagcttcaagcaggttttttccctcctttacttcgtaaggtttattatcaatgtgtatgatcggcatatggacattttttttctttgatgtgttgttcaaaatcttcccggaaatatttcagcgcactttgcaacggttccatggcaccgggcgccagcgcgcagaaagtattaccggggcccaacagcttcgtatgcatttccagttgctccaggtctgcgtaagttccttgtccctgctccagtgcgtatagtatcttctccgtccagggcagtccttcgcggcagggcgtgcagaagccacacgattcctgtgcgaagaaatgctccaggttatgtacaaaccccaccgggcaggtgcggtcgtcgagtatcaccatagtgccggtacccaggcggcttcccgcggcagctactcctgcgaaatccattttcacatcgaggtgggcatcggttaagaaatcagtggaagcgccaccaggcaaggcaccgcgaaaacggaatcccgctttcatgccacccgcatgttcctccagtaattcccgcatagtaacgcccataggtagttcccaggcaccgggcttgtttactcttccacttacaccgtatattttcgtacccccgtcggcggtatagctcaatgatttgaaccagtcgcctcccttgctgatgatatgcggtatataagacaacgtttccacgttatttacaatggttggtttaccaaacaatccgcttacctgtggaaagggtggtttggcgcggggtacagcgcgtttcccttccagcgaattgagcaatgccgtttcttccccgcacatatacctgcctacgccggtatgcaactgcatttccaggctgtaatttttaccgagtatatttttaccgagatatcccgcggcataggcatctgcaattgcctggttcatgatcgtcgcggcttccttatatgcccagcgcataaacacaaaaccctgtgtggcctggatagcataagcggaaatgatcattccttcgagcaactggtgcgggttcccttccagcagccagcggtctttgaaggtgccgggttccatttcatcggcgttacagatcaggtagcgcggaccggttacttccgcgggaacaaagctccacttcataccagtgctgaaacctgcgccgccacggcctttgaggttggcgtctttcaccctgcctgttacttccgccggggtgagctcctgcaacactttgcgtaatgcggcatagccgcccactgcttcgtactccttcaggtgaagaggcgctccggaagcgggtatatgttgtgtgagcggtttttccatctttataaatattgatccagtatttgtgaaagggaagctgttgtcagattcctgtacaggtcgttgtctatcatcatggccggcgcatggtcgcaggtaccaagacaggcattgggcagcagcgtaaaacgttcatcgggtgtggtttgtccgtacctgatctgcagcaggtccatcagttgttgtttaatctccgtatagcccatcacgtagcagctgatactgtcgcacaacaagatgacgtgcctgcctaccggccggcggaagatgaggttgtagaaagtggctacgctgtctacttccgcggtgctcatttccaggatagcggcgatatccgccacgctttcatcagatacccagcggcgttgcccctgtacaatttttaatgcttctatacaggcggccttttttaccggcacgtgctgcatttcatgtgtgatctgttctatttcaatagcagaaagcatatgttgttgtattatctgtcaatatctgcgagtacataatccattcctccgagtatcgataacaggtcggccacggtatatccgcggctgatcaacggaatcatctgcatgtgcgggaaagaaggcgttcgtaccctggtgcggtaagaagcggtgttgccatcgctgatcaggtaatagctgttccatcctttggtagcttccgtgcaaacagccgcctctccggcgggtattaccggtccccagcttacgttgagaaagtgatggataagcgtttcaatatcctgcatggtgcgtgcttttacaggaggggtagccagcgggtggtgcgacttgtaatcgccggacggcatgtaggccacgcattgttcaataatgcggaggctctgtcgcatttcttccacccgtactaccgcgcggtcgtaacaatctccgttgtgtgcgaccgggacctcgaaagcaaaattctcataaccaccatatggccgcttcttgcgcatatcccactccaggccgcaggcgcggagtccggggccggttacgccccattcaatggcttcttccagtgtatagataccgatacctttagtacgggctttaaagagataatttttcatgaccatgctgtcgtactctttcagctgtttgggaaaatagctgataaagtttttcaccagcggctcccagccgttgggcaggtcctgggcaacaccgccaatacggaaccagttgggatgcatacggccaccgcaaatggcttcaatgatttcaaagatgcgttcacggtcggtgaacatatagaacacgggcgacagctgccccagatcctgtgcaaaggttccataccacaccaggtgactggcaatgcggaacagttcgcagagcataatgcggatcacctgcgcacgtagcggcacatcaatgccgcccagctgctccaccgataacaggtaagccaggttattattcacgccgccgagatagtcgatacgatctgtgtaaggaatgtaggtatgccaggattgccgttctcccatcttttccgcgccgcggtgatggaagccgatatcgggtacggcgtccacaatatcttcgccgttgagctggaggatgatacgcaacacgccgtgggtacccgggtgttgcggaccgatgttgaggaacataaagtcagcgtcttcgctatggctttttaagccccattcttcgggtttaaaccgcagggcctcctgctccctgtcctgcttctcgtcatagagcttaaaaggccccatttcagtagcgcgtgccgggtgctccttccggagcggatgcccctcccaggtggaaggcatgaggatgcgtttgagtaaggggtgaccattgaaccggatgccgaacatatcgtatacctcgcgttcgtaccagttggcggccgtccagatgggggtgatgctttccagcgttgggtattcgccgtgcagaccggcttttattcgcaggaattcgtttctgtcgaaggaaaaaagtgtgtaaacaacggtaaagtcatagggtttatgcccgttctgttgccgtttatacgcacgctcgtcaatggccgtgaggtcatagagcatgcgataaggcatttgtatttcagatttaagaaactgtagtacggccacaatatgctcctgtggcgtccagaaggtgggcgtcccatcccgtgtaacctgaggttcgaaggtgatatcaccaaaacgggagcttaattccgctgcaatgcgctctggcatggcgtattaagtttagatgggggtaagataaaattgtggtctttttccggtttaatctttcatatatccgttgatgttagtaagtattttatatttcatcgggtgttttaaaatttgtcatttgttgccgtttctcacggagggtgtctttcatggaaatcttttccggacggataacgccttgttcgccgatcacccaactgagtggccgtttctctttgcctacgctgtcgcgcagcataacgagtcccgacataaatgcgtccgggcgtggcggacaaccgggtacgtaaacatctacaggcaggaatttatctactccctgtactacgctgtagatgtcgtacataccgccggaattagcacaggagcccatggatattacccagcggggctccatcatctgctcatacaaacgttgaatgacgggcgccatttttataaatacggtgcctgcgatgatcatgacgtctgcttcgcggggagtacctctgattacttccgcaccaaaccgggccatatcatacttaggggtcatagcggtagccatttctacaaaacaacaggaaaggccgaaatggaagggccatagtgaatttttccgtccccatgccagcaggctttccacggaagtgagcattacactttgctgtatcacttcttccatagaagtattgccggatatcttacccgttacatcatttgcgttggtcagccaccatttcatataaaagttgatttaccatgaaatcataaaatcaacatgctgttgctacgtcagtgcctgtggtgttggagtcttaatgtccgtgtatccgttaacgtgagcggaggtttttttccgcatttttttatatgcgcgtaaaatctttttcccatcgggcccgaagtccaatgcgccgttacgccattcgtaaataagtacagccagtaatatgaagataaaaacggcaacgccgaggaagccggtccagccaacttcttcataggcaattgcccaggatatgattaataccgtttcaatgtcgaaaataacgaagagcatcgctaccaggtaaaactgggaagggaaccgtaatcgtgcagagccggtggagatgatgccggactcataagcctctccggtggcgcggtctttatgccgctgccccagtacataagaaagccccagtatgatgctgataagtatcacaacgatagcaccatatgctaaaaacggccagataggggtgatgtcagaaacagcgcttttcaaagtgttcgccctcccgagcgatttacttaaaagtccgtcatgcctgtctatcagttaaaaccagtagtatgctttccaatctactgaacatgtctattattggtaatgctagtctgtaaaccgccaaatcaagagggaagaccggatacggatccggtttcataacgtttcaagtgctgctatacggtaaagactatatgaaactgaagttacaaaaaatacaatgataaaacaaaagattaaaatgcgatactcaggtatgcgtacccgtaatatagcattcaagactggtaatgatatgctgctggtcgtcaataataaactttaccacgtcaccaatagatatcaaacccatcagcctgttctgctggtcaacaaccgggaggtgacggatccttttatctgtcatcaatcccatacaatcttcaatggaatcatcttcagtaaccgtaatagggcgttccgtcatgatttcccggatcagggtttcctttgatgcacgccccttcaggataacccggcgggcataatcacgttcggagaaaattcccataaaatgttcgtcttcatcaactactgtcaatgctcccacgttgtgatccacaaggagttgaagcgcttcaaaaacagtgttgtcgggatttatggagtatactgcatgaccctttacctgcaggatattacgtacctttcccatggcaagatatttagaatagtaaataaatgaaaaaccaccatttctaagttaccaattttcattgttaaaagcaaggcagtgaaaataaatcgtttgtgtaaattgtacacaaagctccacgcggaggttgtcttactcaggattaaacttatttcactgattacgctgatttgatcactttggattttaaaggattcggggagatataagcgaagaacgcggattttgtcttactcaggattaaacttatttcactgattacgctgatttgatcactttggattttaaaagattcggggagatataagcgaaaaccgcggaggttgtcttactcaggattaaacttatttcactgattacgctgatttgatcactttgggattttaaaggattcggggagatataagcgaaaacgcggattttgtctcactcaggattacgctgatttaactgattatattttttaaaagattcggggagatataagcgagtatatccgctttaatctccccaaatcctttaaaatcccaaagtgatcaaatcagcgtaatcagtgaaataagtttaatcctgagtaagacaacctccgcgtttgttaatgattgttaaaaaaaacgggatataaatacgcggccatttatatttgccccggtatgaaactttcggttaaaagaattggtcagctggcagtgccagccgccactgtagcattgctctttcagctgtattggctgagacaaacctggcttactgcccggcagtcgttccgtactactgcgacggagtgcctgcaaaaggcctatgattcagccatgatgagcaacctgggtcacataggccgtaccaacgactcccttcaacaaatgaatatatcgtcttccattaactttgaaaaactggaagatgatgaaaatgaaactgtggagcaggccgcgaaacgcgacagcatgatcaatacactcgccgcccggctgcatctcgataccggtaaatcccacagcatacctgtacccaatgtggaatatgcccagatgtccaatattctttcccgcatgttttcatcttttggtttacagctggtgcatatcgacagcctgcagcacgaataccggttgttgctgcatgaaaaaaatattgatctgccgttccgactgtacaccgactctaccctgaccgcagtaaagagtaatccgaggctgctgctcattcaccctgcattgaatacccaaaccaataccatcggcgtactgttttccggcgaaaccatctatctcctgcaacaaatattcccggctatcatcgtttctttctttataggactgctgatcataggctgcatatggacactctggcgcatcatcgtaaaacaaaagaaactggagcaaatgaaacaggactttatcagtcatgttacccacgaactgaaaacaccggtagccgtactacaggccaccaacgaagcgctgctcaacttcggcggcagcaacagcccggaaatgacaacacggtatcttcatctcaataaaacagaactcgacaaactccagggactcatcgatcagatcatgaccatcacccggctggaacaacaactgcatcagcggcaaacaaccgccatgccgttggaagagagcctcagcagcattattcagcgattcgcctaccaggacaatgtgcatgttcaaatagataaccaatcaggacacaacagtatagaaaccgataaacaggcgtttgaaatcatcttcagcaacctgctcgataacgccattaaatacaacaacaaaccacagaagctgattacattgacaataaaagataacagggaccgtatccttattacggtaaccgataacggcgaaggcatttccaacagccatctgccctttatctttgataaattttatcgtgttaccagtggcgatacacaggatacgaaaggccacggacttgggctcagtcacgttaaagcattggcacagcaactccaggccaccgttgaagtgaacagcactcccggcacaggcactacgttcacccttcaatttccgcgctatgcaaaaaattaaactactgctggtagaagatgaacttaccctggcaggcgtagtgaaggaaacgctggagctcaacggatttcacattatgcatgccgcaaacggccagcagggctgggacgcctatctttccttccggccccacgcctgcgtggtggatatcatgatgcccaaaaaagatggcatctccctcgtaaaagatatccgtaacgtagacgaacacacgccgatcatctttcttactgccaaaagcgaaacctccgacgtattacgcggactgcaaagcggggccgacgactatatcaagaaaccctttagcatggaggaactgattctccgcgttaaaacactcatcaaacgcgcgcatagcaacccttccctcaatgcccccaaaggtatttaccgcatcggccaatatgtttttgatcataaccgccaggaactgaaacatgaaactgccaccatccggctctccctacgggaagcagatatgctgcgcatgctggcagaacgtcctaacaccaccacccaccggaaaagcatgctgctggaattatggggcgatgataattttttcaacgcccgcaatatggatgtatacatcagcaaactccggagatacctgcaacacgacgccaccgtgcaacttatcaatgtaagaggacagggatataagctcgtcttttaacaatcattcacactatactcaggttcgttaacggttacgtgtacacgatgatcctactttcgtatcgttcaattacaaacgatgatacaaaaagcagcgatccttctttgtaccctgctggcagcagcggccagcagccatgcacaggctaccaaacaactgaaggaagtagttataaaaggtaaagcagacatccgcgcgaaaggagataccctggaatatgatgccgcgcgttacaaaacaaaagacaatgctgtagtggaagaactgttgcgcaaactgcccggtgtccgggtagaccgcgccggcaacatcatcgcccagggcgaaactgtactaaaagtattggtagacggaaaagaattctttggtaacgaccccgccattgccacccgcaacctcccggccgacatggttgccaaaatccaggtgctggataaaagaagtgaccaggccgcctttaccggtatcgacgatggcaacagcaccaaaaccatcaacatcgttaccaaaaaggaaatgaaaaaaggatactttggcaatgcatcagcgggtggaggaacccgtgatcgctatgaagccggggtgaacattaacagctttaccggtgataaacagctctcccttttattcaaagccaacaacgtaaataagtcgggcttcagcgcaggcgaactgcttcgcctcgccggcagcaaccccgaaatatttgaccagcttccctcctatgcaatggccgaaatccttaaaatgaagggcgtacaggcaacagcagataacccggaggaactggcgcagctctccaatcccacaggattaaacaatacccaatacggcggcgtgaactttaacaacgacttcagcaacaacaccgccctgcgcagcagctatttctataaccggttcgcatcacgcaataattatgataaccaccggttctatcaactgcccgacaccagttatcactactaccagcaagggcatcaaacagatatcaataacaatcaccgcgtaaacgccagcatcgatatacctgtaaatgcacagaacagtattaaaatctccccgcttttcaacagcatccgctcttccggtgtcaatcaactctcctaccgctcgctgaatgaagcgcaaacacaattgctgaacaacggcacccaataccatcaaagcaacgccagcagctggcagtcggccaccgatattcttttccggcacaaattccggcaagaacggcacaccttatcactcaccgtaactcccgcctggctggaaaacaataaccaggtacgaaatatctccctcaacaatatctataacattaaaataccccgcacagataccattaatcaacagctccggatacagggccgtggcttttcggtaaataatcaattcgtatataccctgccgttatcacgcacacacacgttgctgatcagtgaaaacttcttccacagcaatacccggcaacaacaaaccgcattcagctttgatccggtgcaacaacaatacacattgcccgatgaacgctaccacgacaacttctccacaaccaacacccgcagcacacccgctctggcggtgtccgcaaagtataagcgttttagttacaccgcggaagcagcactgcaaaccaactggcagcaaagtaattcgcgggtacagcgctaccaggtgaataacacctatcataacctgctgccccgtatcaacgcccggtaccagttttctccggcacgcaaaatcagcgtcgattatcagaccagcgttcagctacctgccatttcgcagctacagtccctccccgatatcagtgatccgatgtatgtgcgccagggaaaccctgccctgaaaccggctatcaggcgcagtatacgtgcatcttatcttttcacaaacgcggataacggcagttataccaatattatggcgaatggcagcatagtggcccgccagtttactgactatgccgttacagacagcagcggcaaacaactgatcaccactattaatgctaacggatacgccaacacgaatgtatcattccagcacttttttaaaacagacgacgaaggatcaggtatcacctatggcctgcagctggcttacaatgcctatctatcgctattcaacagcatacaacgcaacaaccggcaatacagcgtgacgcccgatatcagctttaattactatcctgcggcattcctgaatatttcagcgcacctcaacactgcctggaacaacaccactatgctgcaaaaaccctactggttgtttaactacgatctgtccgctgtcgctacgcttccctggaacatgcaggcagaaagcgaatggacaggttacaccacctccggcctcagtaacaactataacaccaccgccctgttatggaatgcttccctcagcaaaaacataggcaaaaagtatacactgaaagtagccgccaccgatttgctgcggcaaaacaaaaatgtgatgcggatggtgcggggcggatatacggaagatcagcggaacaacatgctggggcagtatttcatggcaagccttgtttaccagctccgctctttcaaaaaaaagtaattcatctcactaaatatatattatcatgaaaacaacttccatcttaacatttgtattactggccgctgcttatatgccagcggctgcgcaggacaaaagcagcggaaaaataagctatacgcttaccatgaacctgcacgctaacctgaagccggaacaaatgcaatacaaagacatgattcccgaaactgctacgcaggacgcgtcattgtggtttaacaaacagcgtttcaaaacattctataacgctaaccagaaaaaggaaggagacgacgtggaagtaaacgtaaacattcagtctgataacggggatgaattgtatgtggatctcgacagtaaaaaacaatgggcaaagaaaaatggcaaactgaaagaagcgccgttagacatacgtaaaggcaaaagcattgccaccggcgcaacaaaggaaatcctcggttatccctgccagcagcttatcctcgttaataaaaaagattccaccacaatatggtacaccactgccctgccgttacatgcaggcagtcctattggcatgttcaccgacaaaggcgtggtactggaaatgcagcacaggaaaatgagtttcatggctaccgcgattgaatttacgcccatcagggacgaagagttagccatcagccgttaaataaaaaaacgcagcaggagatgatcccgctgcgtttccttctcaaaaaaacattacaaactcactactccctttaccggtgcagctgtttcctggtgcaaatcaaacactacaatttcattggcgcctttctttagccatggagcaggacagtacaggtttttctgcggtcctatttcccagtagcggccaagattgtgaccgtttacccaaacaattcctttcttatatcccgacatatcgatgtaggtatcaccggttttatccaggttaaaagtagctttaaaaaactggccgggtttagcagcgttaccggaagaagcgctcagttcctgtacgaatttttccgtcataggcaagctgtacacttcccagttcatcagcgtcataccgttcaggactacacgatctgtgattcctttacggtcaatcagcgcttctgcaaagttgatgcggcccatgccttctaccaggatttccagtacgggatccttcacatcgcttaccggcaggtcaattgttttctccccaagcctgcggtcaattttcccgatgtacttgccattgagaaacacggttgcatagtcgtgcaggtcttttacactcagcttgccgcttttatgccctatcagcgtggttttatacaccataaagccatagtcctgcccataagcttcaaatggctttggctgcggggatttaaccggctgtggtaaatgatcccataccgaagtgaatggggtaagattaaattcaggaattgtaatggccggaacaggctttggtatggcaggtaattttttgcccttcgggagataagaaccgatcagctgacgcaatgcctggtatttaggcgtcgcatttccctgctcattgataggcgcatcatagtcgtagctggttacatcgggttcatagccctttccgccggaatttgcgccggcagtatagccgaagttggtaccgccatgaatcacatacaggttgaatgagcgtttggtatccatcaggaatttcacttccttcgaaatgccgtctatgcccggccgttgccattgttcgccccagtgggttaaccaacccgggtaagattcgctgctgaaggcgggtacattggggttttgttttttggcggcggcgaaatcagcttccgatccgccggagtccagcccgatggcagcgccttccacgcctcctgcttccagcatataggcggtagcgccatcggccgtgtagaatggaacattgatgccattctttacccacatatctttcagcgtatttaaatattctttatcgttaccataactgccgtattcattttcaatctgcaccattactaccggtccgccgttagttaccagcaacggctttatttctgccgccaaacgatctacataggtggataccgcggctatatagcgcggatccatacagcgcacctttatatccggtgtttgcaggaggtaaggaggcaaaccaccaaattcccattctgcacacacatagggaccggggcgcagtaatacccacatgccttcttcctgggctattttaataaattccgcaatgttgtgattaccggtactgaaatcaaactggcctttcaccggttcgtgatagttccagaacacatatgccgcaatggtattacaacccattgccttcgccatctgaatgcggtgacgccagtattcgtgtggtatacgggtcgggtgcatctctccgctgatcatctggaagggtttgccatccagcataaaatcagttttacttaatgcaaaagaatgtttgttttgcgcctgcactgcctgccccatccaacaggatagcgccagcatgccgcttaggattactttcttcattgttcaaataagttgcagataagcgtacaaaatacaccaaaatatttgattggaaatattttttataagacgcctggctttactcctgaacactgatatccgctactatggcccggtggtctgatacatacactttcaacacctcgtcataaccgccgatattattataccgggttactgagaagcggtttaccggggtggtcatgatgtaatcaatggtgcgatccggcttatctgaaggaaaagtaagcgggcattgctggaggcagcccaggttcatgaaactccgcataatgcctatggtctgcgatgcgggaatagcattaaaatccccgcccaatatcaatggcttccccagttccgttactgccttttttaactccgctgcctgtaataaacggctgtcttcctgcgccaggtggtcgagatgagtggatgcaaaataaaattcccggccgtcttttttcacgcggatcatagccattgtccggaactcgccacctatatccggcgccaccggcaaggcatagcgtttccgttcaagaatgggtaaccgcgaaagcacggcatcgccatactgccctccggttacatccattgcttttgtaaagtaccagtccattcctgtgagctttgccagttctgctgcctggtgaacgttcacaccggtacgacgggtatacacatctacctcctgcagtgccaccaggtccggcttttcctggttgatcactttagccagggcctccaggttggccggcggaccggtagaagcccgggcgccgtaaatgttataagtcatcactcttaccattgttttcggacgcgccggttcttccggtgaagtatttgctgtttcccgcttgccacaggacaacaggcagctggttaagcctatcaaccaaaatatgttcctcatcatcagaaggcgttgatctctgcaatatgcgtcaggtagatgtctccctggctggtgttcaccgtcagtttcacaaacctggcctgctgcgcatacgccaggtaaacggtgcttactttatcattagccagtgtgaatgattcagtatagttccaggtggcgccgtcgcggctcaactccacgataatatttttggggttgccggtagcctttacctccccggtatttttatctgtccggccggtaatactgataccgtgtatcttttgttccacctgtgtatcaatggtaatataatgcggagggccgggcttcgacgctttccaccgggtgctccaaaacgtggcagtatcaccgtccagcgagtggatagcatggccgttggtggccccttcgccggtggtttcctccgatgagaagccggtaatattccagttgctgcgatccagcataggaaacggattggcagcataacgcccgctgatcaggaagtaagcagtgcgtagcttctcatttactttcatgctggtttcaatagtcaccggcaacaggtagctgcctacgccatccagtttatccatatgcaccaccaggtttaacggcgccgtgctgaatctccctgccgggattgtggcggaagactgttccagctcatagcttccctcgggtaataccgggtaactggtaaagttgttagtgttgaaatgatctgtcagcgaagcatctactttgaattttacatttatatcagatgccggtgaatgcggcccgccataacaggcgccataaacaatactgtcgccctttccggatatttcaaatgaatacactgcgggagcaataactgcctgtggcatgtacacaacagcggtgctgtcggatatattttccagttcggcactgttgttccggcaaccgctccaggcagtggccgcagcaagcgataatatcaataattttatcttcatttttctaatattgatcatcaggaaataatttaccagcctggattttgtaccagctttctgtcacggtctatttccgattgaggaatagggaacaggtaataattcttcaggaaaaccctccgctcaaatatggttctttgataaaaaacctggtcggtaagtttggtacctgcgtctacgttcatgccgtagaagtttccgccatcggtttgttcagcgatcttccagcggcgggtatcgaagtaacgaaggctttccaatgccagttccactctcctttcatgcctgatctttgcgcgcatggcggcttgccccagcccacctgcaacatcaggtacgccggccctgttacggatttcgttcaggtatttaaggatatccgggttaccaggctcgtactcgttcaatgcttcgatatagttcagtaatatttccgcataacgaatcagtataaaaggcctggccacatactgggtgatcctgggattactgtcgggatgcacgtttttccgggcgatgtagccggtacgcggaaagtcccacgatcctttcttaccagtattgccggtgaagaaagtttcaatcactttattgccttcgcttttattgatccagagactgccattgtaactaacatttacataaaaccggggttccctgtttacatacatgttataggtaccggcagttgtatatttagtagcagtagaagaaaaaccggtttctttataacccgatccggattcatagatcccttttccattttccatttcaaattcatctaccagttgctgcgtaacagccaccgcggcgtatccgctggctaaacggggtgttacggaacgttcccagtctttcagcccgttagaagtcctggtgaaaatcacttccgaattccagggatccaggaatacatcgcgggtagagaggtaaggatcaaagtttccgctggtatcattcttacggtacagggagaaactgaaaccggtcattacatctttggcggcatcggcagcacgtttccatttttcacgatcatattgcgcgcttaccagctgtttgccatccaggttgcggaagccggcgtagtcggggttaccgttgaactgcggacttgccgccagtaacagcaccctgcttttaaaagccttgcatgcggcctgtgtggcgcggccataatcattttcgccctgtgcggtaaaatgtttgggaagtttctgcgcggcgaggtccagctctgatacaatgtagttaacacattcgtcgtacgaattccgtggcttctgcatctcttcatcggtaggcgccaggtcgcccgcaaccgggatatcccccaggataatagcggggccatattgacggataataccgtaataaaagaacgcccgcaggaaacgcgcctcggctttatattggtcaataagatcctggccgttaggcagcgccagtatctctttattcccatcaatatgctgcataaaataagtagccgaacggataccctggtagaatttagtccagttgttcatgtaatcggatgccgcactccagttacccaggttcatgggataggtgttataaccggaaccgggccggtcgtacgtaatatctgcatcgtctgaacatccttcccaggcgcaggtattgcggtaggcttcattggggatggtaacgtagatgttagcgaggtattcttcagaatatcttcttctgttaaatacctgctcaatggtgatacggtcgctgggaacctggtcaaggaagttactgttacaggaagccgtttgtaaagaaacgccgaccagtaaaatgtgaaccatcttttttattttcatccggagagaattataatgtttaggaatgatcgttgttatcagaagttgacggcaacgccggcagaatatgatttagtacttgaataagaggcgcctcttccattgcctacttctacatcccagagcttaaacggtgagaaagtgaggatgtttaccccttgcaggaagatgttggcggatttaagtttcgcgcgtttcatccaggcagcgggcaggttgtaacttagctgtaaagtctttaaccggatatagtcgctgttctttatccaccaggtgctggcggcgtagttatcattcagtgaacctgccatcaggcggggataaaaaacatcctggcgtggattttcttcggtccaccggtcgttgatattgctgaataaatttccgcggctcagtccctgctggaaaggcatggtgccttcaccgttcagcagtacatccacatgagcggcgccctggaaaagggccgacagcccaaacgctttgtagccgagtgtaaaaccgaagccatataccatttcaggaacatcgccatatccgatgggcgcctgatcataggaatcgatcacgccgtcgccgttgatgtctttgtatttaatatcgccggcccgcacatcgcctgtttgcctgggtgagttctgtacttccttatcgctttcaaaaagtccgagtgcgatgtacccgaaccgctgtcctacgcgcagccctttgcggtccagccagggatacttccagctgggatcatcattctccactactttattcctgttataggtaaaattgcccagcagctgcagcgtgaagtcgccgaagcggcggttataagtgacggatgcatctattcctttgttatcaataatacccacattaccaaacggtgcgttgatcatccctatataacccggtaacgatttccggcgcaggaaaatgccgctgcggtattcccggaaaagatccacctgcaacgtgagattatcatgcagtagcccgatatcaaagcccaggttggttttgcgggaggtttcccattgtacatccacggcatattcaccgatttccttaccggtaaatttctggttgatgttctttccaaaataataatcgctggtattagctacggttgccaggtaggcaaatcttctgccgtcgatgttgctattgcctacgataccatgcgaaaagcggatcttaaaaagtgatactgtatttttaataccggagaagaaattctcttcagatactacccagcccaggcctgcggaaggaaaaaggccataacgctgatcggggtaaaagttttccgatccgttataaccaaaatttacttctgcaaaataccggttgcggaaaccgtaggtgaaacgccctgccaatccctggaaccggtaaggcaatgatgtttccaggtcggccgcataggtattggctttgtcgctgcggttgtagagcaacatgccggatacatcgtgcttaccaaaactcctgttatagttgagtccaaattcagaatagaaggtgcgttcgccctggttactttttgtatactggagaaactctgtaccaatggccacctggtcaaacatcaggttaccatcggcatcgcggcccgtggccagccaggtgtccggtattttcgtatagcggttgctggtatagttataggcatcaaatgaaaacatacccgttacagataatcctttggtgaggaagggcagctcctgcgtgaggcgcagattggagtatacctggcttctccactggttggcataaccaccctgggtaaggcttgcccagggattcgacaaaccgccggaacgcacgtctgccactttaccatccgggtaacgggttggaatctgcaccggcgtcataaaatatgcatccgtaaaaatatcggatacgccggtagtgggcaggtttacattactcaggtaaccttgtatgcctagcttaacagtagtagtggcggaaggcttcagggtgatattggaagtaacgttataccgtttcagaaaaatagaggaattgtatttggtgagttcatctgttttatacattcccagctcatcgtagtaaccaagtccgatatagtataccgctttttctgaaccgccgctgatattggcgttcgcatttcgtactttcccattgttgcggaaaagttctttaaaccagtccacattaggatacaggtaaggatcactgccatcggcggttttccggatagcctcgtcagaatacaccggcgcgctgccacgggtggtcagcgcttcgtttgataatttcatataggtagggccgtctgcaaacgaaggcaatttggtaaactgggtgatgccttctgtataacgcaggttataggcgggcttaccgggcttacctcctttggtggtgatcaatataacgccgttggcgccgcgcacgccgtatactgcggtagcggaagcatctttgagtacagaaaaactttcaatgtcttcagggtctacattggaaatactcctgggcacaccgtccaccaatgtgagcggtgcgctgaagccctgcgtaaaagtggaaatgccgcggatgtaaatattggcatcgttgtaacctaattccccgctgcgttgtacggataccattcctgctacgcggcctccgagcgactgtgtaaggttggataccggctgtttcagttccttgggggtgatagtagcctgcgcacctaccaggctgatttttttctgctcaccaaaacccactaccactacttcttccagcgcggaagacgcttcctccaacactacgtctattttatttttccgctgtaccggaatttcctgtttacggaatcccatcaaactaaaaaccagcactgcgttatcatctaccgataaaataaattttccgttgccgtcggtaccggtgcccaggcgggtgcctttgatggcaacggttacgcctaccatcggctgacccgtagaatccaccactacgccggtgacttcccttttgcctccggcagcaatattaacaacaggaggtacttcttttgtagctactgaaatattctgaccggaagttctgaactgcaaaccggtacggccttccaggtcctgtaacagtttggcaaccgccatatttttatagttcacggttaacttctttccaaaagcttccagtgacttatcgtacaggaaacggaaagtggtttgtttttcaatggcgcgaaagagggtggtcaccgtggcatctttcagctggatggtgactgtttttgtttgggggtcctgttcctgtgcgtgcagcggcgccatataaacggctgccgccaggaatgagcacagagcgaccctcgcggcctttttcaggccgcgtgaagcggataataaaattaggatcatacgttaggttttgttagcgtagtatgtattaaaacaggattaagcggtttattttttatctatacggattatatttccctggcgatgatattgcagatgataaataaaacagatggattccagcacagagtccagcgaagtgtttgcctgttgcccggacaatacatgccgccccatttccggtgtgcccagcacaatactaacactgtaccatctttccagcacggtagtaacttccttcaatgtaagattgtccatcgtgataataccctcctgccaggagttcattttatgcggctcttccctgaacctcgtaaatccgttgctggcgctgtcgtaacttactttgctgccttgttccaatatggcttgttgtccttcagcagccattacttttactttccccgtggcaacgcccaccaccagcttttcgccggggtaatgcttcacattaaaagaggttcccaatacctgcgtttgtacctgcccggtgcgtactataaaaggagccagccggtcgggatgtatctcaaaaaaagcttcgccgttcagcattacctccctggatgtgccggcatatgcttcgctgtaacggatcaccgaccgggcgtttaatattaccgtagaactatcgggaagcattatacgttttatttctccgtcgcctgcagcaatggtggtatatgacggctgatgacggggccatagtaatatcaggcccagcaacaccagcagcatggcggcatagggcaaccagcggcggaattgaccgccccggatatttctttgcagcgccgtgttcactactttatttttcaatccggcagacagtggttgcggctcgttttgaaaccattcttcaggcggcatcagatcgccggggttgttttcttcgagcaactgtaaaagcaaccggagctcctcccggctggcagtattatgttgtactttttctatcagctcctgtaacaggccggcatcaggtttcatcatatacagttcacttctacctatatatacactaaaaaaaaggaggctacttagtggaagaaaaaaattatttcaggaagaataatatcagcagcaaaatataggaatctttcagctcagcttttattactttcagactgctgtggatgtgcgcttctacagtacgtatggagatacccagtttatcggcaatttcgcggtgcgataatccttcttccctgctcatacggaacacagcccgctgcttgtcgcccagcgagtccagcacgccctggtattgcttgtacagctcattataatccagccggtgtaaaatactgtcggccggctgcaacaaagcatgctccggatctgtggtcattagccggcggctgactttattgcggataaaattcaggatatgatttcttgcgatcgtgaatagtaatacctgtatatcagcagtctcatccagctttgcgcggaaatgccagagtttgaggaaaatgtccagcagtaattcttctgcatcttcctcaatacccacctttttcctgcaatagcctaaaacgcgcgggcccagcagatccagtaaagaacgcagtgcttcttcgtcgccttcacggaaacggcgcaacaggaaaggtgaaataagaatagttgtattgtccatgcaggagacaaaattaataagccattgttaacgtaaggttatgatatgattaacagcgtgcagtctataattttcattgttcgtctggtggaattttacgtccatcaatattaataaaaataatcttgtggagaaagaaattccggtgatctcttttattaaaatataccgctcagtggccggttgctaattactactccggggattgttcggggtcaacggtaatctttgcagtatgcctgctaaaaacaaaagggaaaccagtaagctggtttcccttttgcgttgtttagatatttcctttcttcagttccttaacggcatgatcacatgcccgcgcagtaagcgccatataagtaatggaaggattcacacaggaggaagacgtcatacaggcgccatctgttacatatacatttttagcggcgtgtacctggttaaaaccattcagtacagatgttttgggatctttacccatgcgggcggttcccatttcatgaatgcaatgtcccggaggaggcgcaccgtcgtagccatgcacatttttcaatcctgctgcttccagcatttctattgcactggcctgcatatccttgcgcatggccatctcattgcctttaaattcgcagtcgatatcaagtgtaggcaatccgtatttgtctttcttatttttattcagcactactttattttcaaaataaggcaggtgctcaccccaggaacctatgcccatgctccatttgccaggttcaccctgggcttctttcaactgaacgccgataccctccatgctggtgccacggccccttcctgcgccgccctggtagccaaagccacgcacatagtctttttgcatggtgttggcgttggtgttacggaaacggggaatataaatgccgttgggtctgcggccactgctgtaatactggtcttcaaaaccttcataatcgccgccggcgcctacgccataatgatgatccatgaggttatgccccagttgtccgctgtcgttgccaaatccatccgggaaccggtctgacaccgaattgagcatgatccagctggtacctaatgtggaaccgttcaggaaaatgatatcagcatagtattctaccgttttcagggtatgggaatccatcactcttacaccggtagctttacttttatctttatcatataatacttccagtacaatggaatccgggcgcagggtcatattacctgttttggcggcagcaggcagggtaacgccgttgctgctgaagtaaccggtaaacggacatccgcgggcgcacaggttacggtactggcacggaccacggtcctttaatccttttgtgagatgcgccacgcggcctatggtcaggatacggtcgttatacttttctttgacgcgtgccgcaacatgcttctccaggcagttcatttccattggcggcaggaaaacgccgtcgggcagctgtggcaggccttccgcctggccgcttacgccgatatattcttccacatatttgtaccagggggcaatatctttgtagcggattggccagtcaacaccatgaccatctttcgcgttggcttcaaagtccaggtcgctccagcggtacacctgccggccccacatgagggatcggccgcctacctggtatccacgcagccagttgaagggctttatttcgttatagggattctctatatcatttacccaaaactgctgcgtgccttcatcaaaagcatagcaacggctctggatgggatgcttctcccgcatttcattggaggtattgagatgatgagcaaattcccagggcgctttcattgcggtagtgtagtccttgatgtgctctacattgcggcctctttccaataccagcgttttcagtcctttttcactgagttctttggcagcccatccgccgctgataccggagcccactacgatggcatcatacgtattttccttctctgcctttatattcaggttcatatcgttgtgtttaaagccgcaagcggccaggaatgagcttctgaaaagctatccctgaccgctacgcacctattgtatttttaaatattgcctttcttcagttctttcacggcataatctactgcgcgggcagttaacgccatataggtgagagaaggatttacacaggaggcggaggtcatagccgcaccatctgttacaaaaacgttcttcaccgcatgcatctggttaaagccgttgagcacagatgttttaggatcgcggcccatacgtgcggtacccatttcgtgaatggccatacccggataagatccgttgtcgtatgttttcacgtttttaatacctgctgcttccagcatttctgcggcatcattcatcatgtctacgcgcattttcttttcgttctccttgaactctgcatcgaatttcagtacaggctggccccatgcatctttcacggaggtatccagggttacctggttggcttcataaggcaaacattcaccgaaaccacctaagccaatgctccactgaccgggttcggtgatcatttccttgaagtctttacccacgcccatttcggcaataccgcggctccatcctgagcggctggcgccaccctggtaaccaaatccgcggatataatcacgtttatcgtcgccgatgttgcggtaacggggaacataaatcccgttggcacggcggccgaaatagtatttatcttcatatccttctgcagtaccggaagcgcctgtacggaaatggtgatccatcaggtatttgcccagtacgccactgtcgttacccagcccgttcgggaagcgggaagacatggagttcatcatcacaaaggtagaaccgagggtagaaccattgatgaagatgaccttcgcatagtattccaccatttctttggtgtgcttatctatcacttttacacctgttgccttgccttgcttttcatcatagatgatggaatttacaatggaatcaggacgaagtgtgaggttaccggtagctcttgctgccggcagcgtggaggattgtgtgctgaagtaagcgccaaacgggcatccgcggctgcagaggttacgatactggcatttctcacgaccaggaagcggttgggtgatgttggctacgcgacccatcgtaatgttacggcctttgaattttccttctacgctggccttcagatctttttccacgcagttcatttccatggcgggcataaactggccatcaggcagttgtgggagaccttcgcgggtaccgctgataccggcaaatttctctacgtaatcgtaccagggggcaatgtctttataacggataggccagtccaccgcaatgccatctttcaggttggcttcaaaatcaatatcgctcaggcggtacgactgacggccccacataatggatttgccacccacgatatccgggcggtaccagtcgaaacgttttacttcattatatggactttcggaatcgttgatccagtatttttcgttgtgttcactgtaggggtagtcgcggctcagtttaggatgtgtttcgcgctgatctaccgtgatacggccgcggtgtttaaattcccacggatctttggtggccgtttcatagtctttcacatgttccagtggtttaccacgatccagcatgagtactttcaggcctttttctgtcagttctttggctgcccatccaccactcacacctgagccaattacgatggcatcatacgtattttcagcctgtgcttttatattcaggttcatttaattcagatttaaaaagtaaagagaagattacactgcccaggctttttctcctttggtgtaaggagtacaaccttcgtacttgcccggaacgggaacatagcgcaacgctttggtggcacccggttcggaggtgaaataacccagcagggttaattctttcaggtactggaaataatgggtaggatccccttcttttttatctttacgcttgttgtagtctacgcgctctttttcaatccctgtgaggagctcggtgcgctgttccggtgtaatgtccatgaagccttttttgaattgcttctcacttgcctcattgatttttgacaacccatcgaggaatgcctgctgatcttctttcttgtaacaatcgttcatcattacaatgataaagtcttctactttggcatcttttgctccaggagtgctggttctgggtatgatagtttccgctatctccgccagcaaagctttggtttccggcttatgaagatcgtagttcttaggaccagaacctgtgcagctttctaaagctgataacgtggaagcggaaatggcagtacccaacaaaatcgccacattccttattgcgtctcttctgtgcataaatagtaagttgatttgaccttcgaacaagttggaaaaaattcttctaaaaaccaaataaacaggggtgaaatatgcatgagcggctaaaaataggaagaagtaaaaaagaagatgggtagatgtaagtctgtaatgcgacttccatctacccatcggcctgtacagtgtggcaactgttacaggatatattttcctttgtcgtctaccagtacaaccggcaggcggtggtgtttttcgaaataatcataagccgaccggagttctgcccagaattgtttggaagagctgtcggtcatggtaaaagtgcccaggtagttcatggaaccggggttgccaaacttcacggggaatacatgcaccggtatgaaatcctgtcctgcgttctttgcatttaccgctaaaatgtatacctcatcaatgaattcatcggttaagggaatacaacctacggtgatgcagttgccgtggatatagatttcaccaccggggttcttcggatcgctcaggatgcggtcggagaaattcgggtagttgatacccagcgacaggtgatagttgctgttcgggttaaaatcgttgatataatagaatccttccggcacctggcggtccccttccttacgcttgggtcccattttaccggaaagtgtacacacccggtaagatttgaacaaacggaaagtgtcctgggggttatttttcacccagatctccatttcgctgtccagtttgaaggaacggacaaacatatatcttgcagggtaggcaaggcccttcttttcgaattcttttttcagcaactcctctttttcacggtatgcctcccctactttgggaaacattttctggttgtcgaggaaagattgctgggcaaaaattttacctgcacccaacaaaatcaggacgattacaacaagtcgcttcataatattattcaacaaaattttaatatttataccaggtttatataagcaagataaaacaataacagggcaaaaataaaatatatcaccatactcactttcctgttggctatctttaaaatatagtgtttgtgcccctgatagatcaatatcgccgtaaaggcctggaaaatcccacctaacaaaaacaatacaccgaacagcgtttgcatcctcataaaaaacggaactcttattttaatattgtaaagttacacgtttattgctttactgtagctttatccattccagttttatggtagtctcgtccatgccggagctgaaagtggcgcgcacggggtacttcccgttataggcgtaggtataggtgttggtgatcaccctggaagtgttgggactgctaatgttttcggtgagcacgttgtgggccgagaggcttccgccaccgccatccagcaggatacccagctctggttgcagctgctgcgggttccgcatgcggtcgtaggtgtagctaacagaagaggtatacacaaacttgctgtatcccggctgtttgccataggtatccatccgttccacgtctccttcctggttccacgtatactccaggtatccgctgttttcccacgctgctttggcgccattatggccaaactggtagcgccgggctattttgccactggcatcatacgccagggaatcataggaatacacggcgttgtcgcggtaataactgatcctggacaccttgtcgctgctgtactcaaacgacaggtaaggatcgccggtaacggctttttcatcggcagccgacaggcacttcaccaggcggccattttcatataccggcagctggacatcgctgtaggtagcattttccgatttccgcagctgtataatccggcgaatggatttgtcggggttatattccaccgttgtttgtcctgcgggcgataccactttgtgcaggtaagtttgctgatcgccgccattacggaagctgatatggttgccttcgctacggaaagcagtaaggatggtgaacgatgtcaccaaagcggcatagatagccccgcgggctatggaagttgtgtgcataggttacaaatattaaatataaatatactgtataaaaataactaaagtgtggctaatgtgggaaaagacgcaatatatacgcgcattttgacaagttggtttaaaataacaagttatttacatatcgttaacattcgcatgcgtaggttgtcttactcaggattacgctgattttactgattacctggattttacttttgggattttttaaaggattcggggagatgttagcggaggttgtctttctcaggattacgctgattttactgattacctggattttacttttgggattttttaaaggattccgggagatataagcgtagcttgtctttctgcctgattgcgattttacttttttctttgggagatgggtatttaaaaaagctgacgtgaagatggaatagtccacgccttacatctgctttgtacatgctttgcacatgctttgcacttgctttatatgtgcttttgatttgctgttaatgtggaggtgacgtggacttgatcggtaacgtattgtgcatcaatgcgccagagcgggttttaagatattctttagacaggttcctcagaaaaagaacctggatatcaacgctttaggcatattataaagataaacataatcaggcaaaaaacaacgtttgcattttttttagctttaaaagatcagggaagataaaagcgcatcttccgcttttatcttccctgatctttaaatctaaaaaactcaaaaaaataaaatcaacttacgcttatatctccccaaatcttttaaaatcaaaaagtgatcaaatcagcgtaatcagtgtaataagtttaatcctgaggaagacaacctccgctaacatctccccaaatcttttaaaatcaaaaagtgatcaaatcagcgtaatcagtgtaataagtttaatcctgaggaagacaacctacgcgtttaatcctgagtaagacaacctacgcggcgcattataaattgccgcgcagtgcctgttctctttctatagattcaaacaaagccttgaagttgcctttaccgaaagattgcgcacccttgcgctggatgatctcaaagaagacggttggccggtcctggataggcttggtgaagatctgcaacaggtagccttcatcatcgcggtctaccaggatgcccagcttttgtaacggcgcaatgtcctcatcaatcttaccgaccctgtccagcagggtttcatagtaaaccggtggcaccgtcaggaattccacgcccctgttttgcagctcagtcaccgtgttcacgatgtcgttggtggcaatggccacgtgctgaacaccgggtccgccatagaaatcgaggtattcttcaatttgtgatttcttctttccttcggcgggttcgttgatggggaatttcacacggccgttaccgttactcattaccttgctcatcaaggcagaatattcggtggaaatatcgctgtcgtcgaaagagatcaggttcctgaaacccatcacgcgctcgtaaaatccaacccaggtattcatctcattccagcccacattacccacgcaatgatctacatataacaggccggtatctgttggattgtaattcgttttccattccttgtaacccggcataaacaatcctttatagtttttacgttctataaaaagatgcacggtgtcgccgtaggtatggataccactccgcactactgtgccaaattcatctttctctgtaaccggctccaggtaaggcgtggcgccccgtttaacggtttcttcgtaagccgaccgggcgtcgtctacccacagggccagtactttcacaccatcgccatgtttggcaacgtgacgggcaatttcggtatcgggcaacagggaggtggtgagtacaaagcgcagtttgttttgcactagcacataggaaaccctgtcttttacaccggtttcaggaccggcataagctaccgactgaaagccgaatgcagttttgtaataatgtgccgcctgcttggcgttgcctacataaaactctacgtagtcggtaccattgagtggtaaaaagtcctgctgaccggttaagttgtccgcattcactaatgctgtttccataacattcaattgttttggttttataagttggttggtttttgtgaatcatttattctgcccagctcatgacgtagctgccatcttcaatacccaatgctgcttcggtgatctgcaaagggtgaaaggtatctaccatcactgccagctcttttgtttcttttgcgccgatacttttttccacggctccggggtgaggcccatgcgggatgcccgcaggatgtaaagtgatcatcccccgcaccacatgcttacggctcataaaatcgccgtctacataatataatacctcatcactgtcgatgttactatgattatacggcgcagggattgactgcgggtgataatcaaataaccgcggacaaaaggaacatactacaaagttgttcccttcaaaggtctgatgcactggtggcggctggtgtacccgcccggtgattggttcaaagtcgtggatggaaaaggcaaacgggtattcacatccatcccagccaattacgtcgaagggatgatgtttataatgaatgggatagatcacccctttcttttttatacgaatgaggaaatcgccttcctcatcaatggtttccaggtgctgcggctgccggatatcccgctcgcagtaaggggaatgctccagtaattgtccgtatttgctcaggtatctttttggataacggataggactaaacgattccactataaacaggcggttatcttccgtattaaaagtgatctggtaaatagtaccgcggggaaccaccaggtaatcgccatagccaaattccagttggccgtattgtgttttcaatacaccgcttccttcatgcacgaagatcatttcatccgcatccgcattcttgtaaaaatatccttccatgcttttgcggggcgatgccagtacaatatgaagatcactgtttaccaatactgctttgcggctttccaagaagtcgtcttccggcttaatattaaaccccatgaagctccggtgcttcagcatcttttcttccgccacctttggcgcaacggaatagggttcatctacttttacaatctccgtaggggggtgacagtgatacaacaggctggagtgggaagagaatccttctgtagaaaacaactgctccgaatacagctggccgtccggtttgcggaactgggtatggcgcttatgcggtatttgtcctagtttataataatgtggcatgacaagtggtttgaaaaaattgttctggtgtacaattaaaggattgaatgggtgtatgattcattgtactggtgtacgatccatatttatatgatacagtgcaacctgctgatggcagcaaaaaattaagatacacatgcgcaggaatagcaactgaatactattacaaagttacggtatataaatacgaacgatggccggtagcggccgttgggaaaggttatgccaaagtcgaatccatggcaagcgtggccatgagaaagtagtagttaagctgactattgcttgtatatttcagtgaaatggacaagtggcaattgtttaggcaactaaggtaaggaaaaactgtgattccaaaatgatttttgtcacgggcaattatcagtcacacaattgtcacaaaacaaccattttgcccaatgtcaggaattatgaaatcgcaactatcttatttatattttgaatataattctaaaaaataaccataataagtatcaaaaatcaacaaacgaccctaaatttaaaacatttctaaaaatcaccactgcacttttatttaccagtgtaattgtagacttttgttacacaatcgtcatattccaatagtgataccgttctacacataccagttctcttcggtttctgcctccaggcggatagcggacactatggcgacaacgaccaccattattacaaccccactgcggggttagttttcacatattatccaacgaccacaagggtggtacataaccgggaggccccggacttatctacgtataaattttccatatgcaagtattaaaatttggcggcacttcagtgggaagcgccaaagcaatagaacaggtttgcaacatcctcaaacaatataaaccggccggtaaatatgccatcgtcgtatctgcactcggcggggtaacggataagcttatacgctgcggacaactcgcggagcaaggcaatgaagactataaaagtatattacaggaaattgaagccaggcatctcaataccatccgtgaattattccctatcaccgcacaaagcgggcaaatcagccagctgaagaaaaaactcaacaccctcgaaaacctctgcgacggcatcttccaggttgcagaactcagtccgcgtaccctggataaaatcatgagctacggcgaactgatgtcctgtgttatcgtcgctgaaaagctaaaacagcagggattctccgctacctgcaaagacagccgcgaactcattgtaacagataatcacttcggccacgccaccgttaactttgttgccaccaatcaccatattacgcagttctttgcacagtcgcccgccgattatgtagtactgccaggctttgtagccgctacccccgatggcgaaaccaccaccctcggacgcggcggctccgactacaccgccgccatcgtggcggccgccgttaacgccaccgtacttgatatctggacagatgtgagcggcatgatgaccgccgacccgcgcatggtgtcacaggctattcccatctcacacatttcttatgtggaagcaatggagctgtcgcattttggcgccaaagtcatttatccccctactatccagccggtgatgagtaaacgcatacccatctggatcaaaaatacttttgcccccgaagatcatggcaccctcatacaggacagcgccgaccgcagcttcccggtaacaggcatctccggcattcccaacatcgccctgcttaccctcgaaggaagcggcatggtgggcatccccggcttctccaaacggttgtttgaatccctcttacgggaacgtatcaacgtaattcttattacccaaagctcatctgaacactctatcaccgttggcattcatgaaacagacatgctgaaagccaaaactgcggtggacagtgagtttgcacaggagataagcgaaaaacgcattgaacccctcctggtggaaaaagacctctgcattgtggccgtagtgggagataaaatgaaaaaccatcacggcaccagcggtaagctctttggcaccctgggcaggaacggggtgaacgtaagggccatcgcacagggatctaccgagaaaaatatctccgcggtgatcaacaaagccgatatcaaaaaagcgctgaacgttatgcacgaaaccttttttgaaacacccctcaaacaggtgaacctctttatcgccggcgcaggaaatgtgggcagcaaactgctggaacaactggaacaacagcaatattacctccagcacgagctgggtttgcagatccgggtaaccggtctggccaacagccgccacaccctcatcagcgaaaccggcatcaccttacgtgagtggcgcgaacaactggagcaggccaaacatatcagcaccgccgatttcgtgcagcagataaaaaacctgaacctccgcaacagcgtattcgtggataatactgccagcagcgacattgcagctgtataccacgagttcctgcaacacggtatctccgtagttacctgcaataaaattgcctgctcatcagactatgcttattataaacaactgaaagacctcgcccgtaaatacaacgcctccttcctgtttgaaaccaacgtgggagcaggactaccggtcatcaatacactaaatgacctgatccgcagcggcgacaaagtacacagcatcgaagccgtgctgtccggcagcctcaacttcgtattcaaccatttcttaaatggcaccagtttccgtgaagtagtaaaagccgcgcaggacgaaggctacaccgaaccagatccgcgcatcgatctcagtggtaaggacgttatgagaaagatcctcatcctggcccgtgaaagcggcgccgccattgaaatggatgaaatcaccaactactcattcctgcccgccgaatgcctcgacgccccttccgtacccgccttctacgaagagctggatgtacacgccgctcacttccagggactgcgcgaagccgcagcggctgaaggtaaacgcctgaagttcgtggcccgctatgaagatgggaaagcctccgtgggcctgcaaagcgtagcccccgatcatccgttctttaaactggaggggaaggacaatattgtgctgtacactaccagcaggtataaagaccagccactgatcgtaaagggcgcaggtgcaggagcagatgttaccgcctccggcatctttgctgacatcatccggagcgccagattgtaaactttccatgaaatgagttgcaatcctgacaatcaattattaaattaaactaacttaaaggtgatatggacagtataaaagtatttgcgccgggaacagtggccaatgtagcttgtgggtttgacgtgatcggcctggcgctggacgcgccgggagatgaaatgatccttcgcaggagcagtgaaccaggcatccgcattactgccatccatggcgcagacctgcccctggaaacatcacgtaatgtggccggcgtagccgttcaggcattattacagaaatacgaccagccggatatcggcattgaaatagagatctttaaaaagatccaccccggcagcggcatcggctccagcgccgccagcagcgccggcgcggtagtaggcgttaatcatttactcggggaacccttcaccaaaaaacaactggtaaggtttgccatggaaggagaacggctggcctgcggatcagcgcatgcggataacgtagccccggccatcctcggcggcttcaccctggtaagaagttaccgtccattggatattaccaccctccatacaccggagcatctgtgggtgaccgttatacatcctcagatagaagtgaaaacgtctgacgcccgcgaaatactgaaacaaaaagtgctcatgacagatgccatccggcaatggggcaacgtaggcgcattggtggcggggctttaccaaaacgattatgaactgatcagccggtcgctggaagatgtgatcgtggaaccgatccgttccatcctcatcccggccttccacgagctgaaactgaaatgtaaggaagccggcgccctcggcggcggtatctccggctccggcccctctgtattcatgctcagcaaaggagaagaaaatgcccgcaaagtagcggctacgatggatagcgtttacgcaccacttggcgtggattataaaatctacgtttcccagattaacaccgccggtgtaaaagtgattgactaactaattaacaacgttttattcatgcagtatttcagcttacagaacaagcagcaccaggtaaatttcgaaacagcagtagtacagggattggcgccagacaggggactctattttccggaacagataccagcactggataaagacttcatcaataacctgcataattatacggaccacgagatcggactacaagttatccgcccgtttgttggcaatgaaatacccgaagaggctttaaaaaagatagtaaccgatacactacattttcctttcccggtgcagaaagtgaccggtcatacctacgccctggaactgttccacggccctacccttgcatttaaagatgtgggcgcccgctttatggccggctgcctcggctacttccgccgcaacagtaccacccctgtaaccgtgctggtagccacttccggcgataccggcggcgccgtggccagtggtttctataatgtaccgggcgtggaagtagtgatcctctacccttccaaaaaggtgagtgtattgcaggaaaaacagctcaccacccttggcaataatattcatgcgctggaaatagaaggtactttcgacgactgccagcagctggtaaaaactgctttcctggaccaggaactgcaggcacgccggccgcttaccagcgccaactccatcaacgtagcccgctggctgccccagatgttctattatttcctggcatacaaacaaatgaaggcagcacatcccaggctcgtgttctccgtacccagcggcaatttcggcaatatctgcgcaggcatgatggccgctgccatgggattgccggtatcacattttgtagccgccacgaatatcaatgacactgtgccccgctttatggacagtggtaaatatgaaccaggcaaagcatcgcctaccatgtctaacgctatggatgtggcagatcccagcaactttgtacgtatcctggaactattcggcaacagcctcccttcccttgctgaaaaactcaccgcctacagctttaatgataaagataccgcccgcaccatggaacaggtatggaaagaaaaccattatatgctggaccctcatggggcagtaggctttatgggactgcaacgttacctggaacattccccggagctgacaggcgttttcctggaaacagcccacccggtgaaatttgaagacaccgctcctaaatctatccgggaggagatatatacccccgcgaaggtgatgtctttatatggtaaagaaaaacaagctaccctgctggctgccgattatcctgctttcaaaaactggttaatgcaataatgattctgtagttttggcgccagtatgaagtatttacctatcctcctgttattaatgggtgcgcaggcatgtaataatgccggcacccggcagctaaatacagccagccgcccggactccgtgctgtacagcgatatcatccggccggtaacggattctatttcacagtttcctgaccatcccgatttgtattatcgccgtgcactgctgttgtttaataccaaccctgcactggcgcaggccgattttgaaaaagccgcctccctgatgccggaaaataccgactactgggcaggggcaggcgaagccgccctgatcgtgaatgattataaaaaggcagccgcaaattttcagcaggcgctggctaccgctcccggctatacgtacctggaataccgcctggccactgcactgatagaaaataaacaatatgcccaggcagacagtatcgctaacgtgctcgcacaaacgacagatgcccgcgataaagcattctacctgaaagcccgcatggcagaagataaactggacaccacctcggctatccgtcaccttacctccgccattcatgccgccgggaaacagcctgaatttgaggccgtcatggaactgggcgacctgctccgcagccgcaaagccactgccgctcttaactattaccagcaggcatggcaactggatactaccaacgcatatcctttatttgaagccgctcaattccaggaagaactgggcgaccttcccgccgcgctcggcgcgtaccggaaatgcattgtaacagatcccggctttgaaccagcctacctggcactggggaaaatttacagcaataaaaaggactggaaaacggcgtacacctattacaacctggccgccaaatcagcgccaacagacgcatgggcctattactacagggctatggcacaggaacaactgggcaacaaagcactggctatagaagactataccaaagctacttcctttaaaaaagatttcagcgaagcaaaggaagccctgagaagattgaacccgtaattacttaaatttacatcattcaaaaatagagcacttggaaaaacatcctgttttagtggcgccatctttactggcagcaaatttcctggagctgggaaaagaagtggatatggtgaaccgcagcgaagccgactggttccatctcgatgtaatggacggtcggtttgtacctaatatcagctatggcttgcccgtgattgcacagatcaaaaagaaagcgcagaaaccctgtgatgttcacctgatgatcgaagaaccggagaaatacgcagccgacttcaaaaaagccggcgccgacatactcaccgtacacttcgaagcctgtatccacctgcaccggaatatccagcagatcaaaggactgggcatgaaagctggcgtggcactgaatccgcacacaccggtagggttgctcgaaaatgtgatccgggatattgatgtagtgctgatcatgagcgtgaatccaggcttcggcggacaaacattcattgaacaaacttaccagaaaataagacaactgagacaactgatcaccgacaatcacgcacatgcgctcattgaagtagatggcggtataggcacagataacgccggacaactcatccaggcgggcgcaaatgtattagtggcaggcagtgccatcttctcctctgccgatcctgaaaaaaccattcacacgctcaagacaagtgtgaaataatttcctttgatagtggcttggtgagatatcctgttacaaaattgtaagcattcacacgctccctgtccttttcatcaatggaggaagtcagtacaaagatcctgatttgcttcggcaactccgcctggaaaacggcatattcttccaggaactcccagccatccatcacaggcatattgagatccagcagtataagatccggcaaggcctgtgcttctcctgcattttcccggagaaggtccaatacatcctgtgcgtcggaaaatacacggatattactgctgatagcctgacgttcgatcatgattttggcaatctgctggtgaatcgggtcatcatctacaataaaaatcgtattgattaaactcataaagggggtttattctgatctaaaagtaataataaatttggttccctctccgggatgactttctgctcttatattaccacccatcgcttctacctgcgttttcgtgataaataagccaattcctttcgcatctttatttttatgaaaggttttgcggaagccaaaaagcttgttgccaaaccgctccatatctatacccacgccgttgtcttccacgctcagaatgatgttatcattttctttccagctccgcagatgcagtgcaggcgtacgttctgaagaacggtagcggatagcgttggtaataaaattcagcaggatactgtcgaggtacacccggggatattcaatcaccggctcctcctcaaaatcgtaggtgatctggatattgctggtttctatatctaccagcaatatatcttttaccttctgtaatctttcggcaaacgacagtttttctttttccacattcacatctttccggatctgcactacctccaccaggtcgttcagtgtttcatcaatcttctttatcacctcgtgtaccatacccaggtaaagatccttttcctgctgggcggcagcttcattgtgcatttgcatcagcgccttcaggttggcaataggcgcccggaggttatgggaagtgatgtgggcaaaatcttccagctgcttgttctggttcagcaggttcttgttcaggttagataactgctcgttggccttccgcagctctttctgcaatttccggctgtcggtgatatcgcgcataaacacggagatcccgccgtcctgcatcggggtaagcaggaaatcgtaccatttgtctgcccccgggaagtagatgccgaacgactgtgatgcctgctgctggatgcattcctgcagccgtgcataaaacacggtgccgcttaagcgcggaaattccttgaagatattgctgcccatggccaccgggtgaccaatcattttctcggccttccggttcagaaagttgaggttccctgatttctccatagcggcatatcccatatcgatggtatcaaagaaaagacgcatcagctctgtgttccgggtgagtgcgtccctgatttccagttgttcggtgatatcctgcactaccccgtacatgcgtaccagccggctgtttacataaccgggttgtccaatagaccggaccctttttacctgttgtttggaagaaatgatggtgagctgggcatcgaacggcctgcctgtttccatacattgctccatcagcgcttcgaggctttcacgggcctctggtgtgtaatagcccaatgctttttcaagatcgacgggggtatctacggggcagtcgtggatgtgatacgactggtccgtccaccgcacctggccgctgtctacatccagttcccatccgcctatcttaccgatggtacctgtttgctgcaggaattcctggttcttcttaatctccagctcctgcagttttttgtcggtgatatcatttaccagcgctaccacaatcatttccttgtccaccggttcaatcaccgggaacacggtcaggtcgaggtatacttcccggcctacggtcgtccatcgcttgtcctgggagaagtcgatccgcttttccacgcggagtgatttattctgttccagcgcctgtacaaacagtttgtccagttcaaacatggtggccagttcatcgttcatcacgttgaaaggctggcggctcatgggatgcggcgaattaaagaagaagcgttgtgtttgattgatccggcggataaagccaaaattatcaaactggatataaccgatgggcaggttttcgatgatgttgtcgaggagtcgttcgcttttctggaggctgagttccgataattttttctcggtgatatcatccagtatcaggaagatattatccatattcctttgctggtctgtgagggggaatatggtcgcttcgaaatatacgggataaagcctggtgatgttttcgtggtgtttctcgcggtagctgaggaggatttcccgtttgatcgttttccctgttttgcgggcttcctcgaacataacggcgagaccattaagccggtagaaagggtctttcagccatttataatccggttgggtaaagaaggcgtggtgtttgccccagatctgccgctggcgggtgttcatgtccatactatcaccatcgggcgagaactgttgcagtccgagtggaagattttccagcacctggccatagtacacttcattacgggcgcgttttatttcggtgagtttccgttctgtgatatcgatgccgatgagcatacaatgcgtaagggcgccggcttcactgaaaaacggggtaatgccggcttccagccacagtggtttattttcgggattgataagaaagcagagctgttcctgtaccggttcccctttcatcagggtaatccagagatcctgccagtgttccgggttatcaggccggaagagggcggtaaaagggcggccggtaagggggccttctgatggctgcaatgccgctatcacctgcgtattaaccgcagtcaccgtacctgccgcatctatggtgacagagagtgcaaaggcattaatagcggtttcaagatgctgtaagtggctgtaatgctgttgcagcataactacattcatatgatagcagaatctaaaatcgttgtgtcaggaaacgcctaaagtaggcattatataataaaaaacactattggacaggtaaaagtaataaattgttagatatcggtcaattccctataaacgcagaattaacaagggaaagagtggattggttcaatcatttatccacctgttgtggattttgagttttccgaaattgttaaacgatcaatatctttggggtatcttattacattattatttttaaaatattatcagatgaaagttttgattatcatgggttccgagagtgacaagcctgtaatggaagaatcacagaagcatttacagtattttggaattgaaaatgagatgatagtggcttctgctcaccgcaatcctgataaagtaagagaattgtgtataaccgctcaggaaaagggttttggcgtaattattgccgcagcgggcatggcagcagccttaccgggagttgtatcagcttacacttcgctgcctgttcttggagttcctttagatggtggtttaccgggcggaatcgatgccttgtattcaattgtacagatgcctgcgggattaccggtaggtacattggcggttggaaaagcgggtgcgcgtaatgcggctatactggctgcacgtatcctggctttgggaaataaagatatcgccgctaaagtagaaggcttcaaacagaacgggtacagaatttagtgatagcttaacaattgcgttctccaggttatactagatttaaatatattcggattgaaaaataccgatcatttcctggacaattaaaccttagaatcattgactgaatccattatcaatttagacagtattaatcccattgagtttttcggcattaacaacggaaagcttgatctgctgaaaaagaaattcccattgcttaagatcctgtccaggggcacccagttaaaattgagtggggcaccggaagaagtggctacagcggaggaaaaaatcggtcagatcgttaaatacctggagcggaacggtaacctgacagagaactattttgaacagattcttggagatgaggaaggcactaaaatcgacaatttcagcgagcgcaatcccaacgaagtactggtatttgggcccaacggcagaaccgtaagggcccgtaccgccaaccagaaaaagatggtagcgctggcggaaaagaacgacatcattttcgcgataggtcctgccggtaccggtaaaacctatactgccgttgctttggcggttcgtgctctcaaaaacaaagcggttaaaaagatcattctaacccgccctgcggtagaagcaggggaaagcctcggtttcctgccgggagatctgaaagaaaagattgatccatatctgcggccattgtacgatgcgttggatgatatgatccctgcggaaaagctgagttactacatgaccaaccgcgttattgaaattgcaccgttggcgtatatgcgtggacgtaccctggataactcctttattatcctggatgaagcgcaaaatgccaccgacctgcagatcaaaatgtttctaacccgtatcggtgcatctgcacaggccatcatcaccggtgaccttacacagatagatttacccaaaaatcagcaatccggtctggaaagggctacccgcatccttcgtaacatcgatggtatcggtcatgtggaacttgatgaggaagatgtggtaagacaccggcttgttaaagccatcatcaaggcttacgaagccaataaggaaaaataagacagttgatatcctgttatctgatagctggttatttgtttggatggcacaaccgccaccagacaagcaatcagctatcaaaataacaattatctaaatatttaactctttattaacggcgattgccgtaagttcacctgtttttatccaagggagacattcagtccggaagcctgtgaatgtgctgagctatagccgatgactttgcagtattgaagtttacccctatttttgttgtgatatattataatttatcgaccgcatgaccaatttttttcgaatcatgacactggcattgattacaaccttgctgttaggcagttgtaagaaaagggcttcccctgaagaggtggcgctggcgtttatgcatgcgattcaggattcgaactacgaccaggcaagggattatgccacaaaagaatcccaacaggtattacagatctatgccatctttgacggccgccgcagtggcgctgaaagagaaaaaattaaaaacgcccgcatcgaggtagttaatatcgaagaaaacggcgataaagcggctgttacaatactgaattcctccgctcatcagaaagaagttttgcagatggtgaaagaaaacggccaatggaaaatttccctgacgttcgacagcatcattcccaattacacaccgcaaaccggtggtaatgcagccttcgactctaccgcgttacccgcagacagcgcacctgttaacggtttaacggcgccgggaaactaaataattatccgctcttttatattttacataaaaggaaaggataatttttagctattaacggctagttcccttaattttgccacgcattaatgatcagatgtgtggcttattcctgtttttacttaccggaaacctgaccatatctccatgaaaagtgaggtgaatactttattcacttttcaacattaatccaatattgaacaataaaccttaaagtaaagtagattattatgatgacaaatccctggcacagtgtgagtcccggctctgaagtgcctaatgttgtaaatgcaattatagagattccaaagggatgccgagctaaatatgaactggataaagaaagcggtttgctgaaactggaccgggttttatattcttctgtatactatcctgccaactacggttttattccacagtcttactgcgatgaccatgatccgctggatatcctggttatctcccagatcgaatgtgttcccatgtgtatcatcgatgccaaaataatcggtgtcatgcaaatgatagacggcggcgaagcagatgacaaaatcatcgcggtagcagccaacgatatgagcgtaaactatatcaacgatattaccgaactgccgcctcacttcatcgacgaaatgcgccatttcttcgaagaatataaaaagctggaaaagaaaaccgttgtggtggaagaattccagaataaagagaaagcaaaacagatcattctccaaagctttgaagattataagaagatcttcagacagagctagcggattttgtcttggctcaggattacgctgattttactgattagctggatttattcttttggattttataaaggattaagggagatagaagcggatattcgcttttgtctcccttaattattataaaaaaaatctaaaaatcagaaaaaatccaaaagtaaaagtccagctaatcagtaaaatcagcgtaatcctgagccaagacaaaatccgcgctcttaaaagtatctctttatgatccgcaggtgatgcgtacgcaaccccgtatctgcgtttataattccttcgttatctatcggatcaatccgtacctttccggaagaatggataatttcatgatcgttcagcaaaataccaacatgcgtaatcctcccctcgttattgtcaaaaaaggcgagatcccccaggcgcgcttcctgtaaaaaaccaacaatgtgtccctgggtagcctgctgataagcatccctcaaaagtggaataccggacagcttgaacacctgctgcgtaaaaccggagcagtccacaccaaaaacactggaacctccccagaggtaagcggtgttcaaaaactgctctgcggcgctttttaaggcagtaatatcaacggggctgtgatgggtaagcggaagcggtttatcctcaaattttacagcaatagttccccactgcgtggaaatatcgctatcgctctttacaaggcagccaaaaggtaccagcatgggccggttattcatggtaacccggtttacccaggccgggaaatagtatttcgccggagccaggtacagcgattcatctatcgtttccaggtgggccgctgtggcccagccggtataaccgtcgtactggtttataactttcacccagccgtcgggagccgtttcggtgatctccaccgctgctccccataatagctgggaaatcatttcgcttttatgtgaggtagcactccttaatggcgcaactggcacaatgacaatggcgtatggcatattaattgtataaatcccttttactattcaataatcttatgcgctaaatgaactttttccgcttttgtacgtaaatataaagtaataagtttatgcaacaacagttaaccaatttatcggacaaggagttaatatcccgcgccaggaaacagcttgaccgggaggcggaaagcgtattgatagacaggtacagtcatttactggtggctgttaccattcctcatttgagtagccaaccgaatctcgaccccaacattgttttcccggcccttctgcaaagattaaatgccagtcttaaaacacaaaccatctataaagccaacgaatggatcctgcatatacaaaaaggatacctcgggaagcctgaaaagaacacccccttctatccatcccgcgacggaagagacctgctgcatatcgaaaatacggtagacaaagccgctacccatatcatcgaccgacaggatctcattgtgcggctggaacaggcgcttcaacggctgagtgcagatgacaatgcactgatcacgcaattctatcttgaaaataaatcctttgccgaccttacagctgctaccggacttccaagagagaagttaagatcgcaactcaaagccgccaaagcgaaacttgccaagttatttatgaatcagggatatgctaagtaacaaaccgaataatgagaaagtactgaagatcttttctgccatccggtgcctcagcagggaccagctgccccgttatatggaaggcaggctgaccgatgtggaacggcacctggtagaacaacacctcaccgattgcgatctctgctatgatgcattaaccgcactggagcaggaagagaataccgaaagataccaggacctcaccaataagctgcaacgctatgtacaaaacagcatacagcctgtttcgcacgtacaaaaagtagcgcaatacacccgtaaggaaaagaataaggaacacatgctggcttatttctggatcattgccttcatcggccttggtgtgggcagtgtgtatgtgttacgcggacatatgcgtaatcagccaccggtgcgtatcatggcgtcgtcactgccgcagaaagactctgtgcgtgaagaggtggctaccggcgttcccctggtaacagctgcagaaaataatcccggaacaaccacgccggcccctgctgctacgcctgccattcaaacatcagcaaaaccagcggcagccctggttgactccgccgcgctgaaaaaagcagccgctttaaaagcgctgcaaaagaaaaccgcggcagacagcatcaaaaaacatacactattgcaaaaacaggcagactcccttaaaaaggaaaccgccgataaagtaaccgccaaagcagaagaaaagaaaccggaacaaagaccggaacaaaaacctgcggcgcccaaagaaaaacagaaagaacaggcgccaccaccggaccctccaaaaaaagaaacaccctccacagctgttaacagcgatgaatacctgtacaaagcagccatggtataccagcaacagggaaaccttaatgaagccatcaacaggtacaaaagaatagagtccgtgagctcaggcaaatacgtggaaatggcccgctaccaactcgctatctgctaccgcagcaaaggacaggctggcaaggcccgccgcatgtttaaagaagtgatcaggatggatggttccatgaaagccgctgcccaacaggcattggatggtatgtaaaaaataaaatatcaaaataattatggatttttgcaaatgctgcatcttagatgcagcattccatttattagcctgtgaataatccagatatacaacaactaacagaccaggagctactgcaacggttcaaagctgataataacagtgattggataggtgtgctgtttgaccgatatgccctgcttttattgggtatgtgcatgaaatacctgaagaacgaagaagatgcacgcgacgccgtgcagcaaatctttctcaagatgttatccgacatcaacaggcatgaaatccagtatttccgggcctggatttaccaggtaaccaaaaactactgcctgatgcaactgcggcagaaacatatgaaatacaaggaagaaatctccgacaaacatatgggcggtattgccgctgatcccgaagataagcaggtgtaccaggaaaaggatatcttgctggaaaatatggggcaggctatgagccagctaaaccatgaacaaaaaatctgtgttgaattgttttacctgcaaaagaaaacctaccaggaaattgctgatcaaaccgggtatagcctccttcaggttaaaagctatatccagaatggaaagaggaacctgaaacttttattggaaaaacaacaacgcgcaaacaaaagttaatttgcatcaatagtgatatgaacgagcatttcaacgatatctttgtaactacaagctgtcctacgcaacagcagctgcttgactatgttcagggtaagctgtctgcggaagaacaacatgaagtagaaatgcacctgtctgactgtgagctttgcagcgatgcattggaagggctggcggctataaaagataaggagaagattcccggatggattatccagatgagatggagtcttcttaaaaaaatacacaaacgctacaggaccaggagaaaatcagaaaattatatatccctggccgttattattctatgcatcctttttttactgcttgcattgttctgggcataccatttctctgtaaaacattagcggggggaagtattttttcctccgccacatttagctgctaatacaactttttatcccccttttctttccatctccggaaaacattcagcgcctcctgatcaggtaaagcaatcagcggaatttttttatccgcatgatccttctctatttcccggtaaataaatgaatcatcaaaatcaatggcagcagcatcttcctttgtattggcgtagtaaacacgttgtggcctcgcccagtaaatagcgcccaggcacatcgggcagggttcacaggaagtatatatttcacagtcgtgcaactggaaagtgcccagcttcttacatgcttcgcggatcgctaccacttctgcatgggcagtagggtctgtgtttgccagcacctggttccagccctctcctacaatctcatctccccgcaccactatcgcaccaaaaggaccgccgtcgccattgtccattcctttacgcgacaaggcaatggcatgctgcataaatcttctttctctttctcccggcatacagttactttttgatttactcaaatttaacgaaagctggccacacataaaaaagccccgcgaagaatcgcggggcttatcgttaactatgtatcgtcgtatttagaattacttgttcctgattactactacgccatcaaacacgtcaatcaacactggtttggatttatcaatatctcctgccagtatcttcttacttaacaggttaatgatttccttctggatgaggcgtttcagcggtcttgctccaaactgcgggtcgtaaccctgtacagaaagatactcaagcgcatagtctgaaaagtccaatatcatgccattctttgctaccatatccttcagttgctgtaactgaatgttaattattcccttaatttcacttctcagtaacggctggaacataatcacctcatctaccctgttcaggaactccggacggatggtttgtttcagcaatgtcatcacttcatctttcgttttatctactatttcttcgcggttggtatcatcaatattttcaaaattttcctggataatatggctacccatgttactggtcatgatgataatggtattcttgaaattcaccacgcggcccttgttatccgttaaccggccatcgtccaatacctgtaacaaaatgttaaaggtatccgggtgtgctttctcaatttcatcgagcagtatcacggagtatggtttacggcgtaccgcttctgtcagctggccaccttcatcatatcccacatatcccggaggcgctcctaccaggcggcttacggagtgtttttcctggtattcactcatgtctatccgggtcatcatgttttcatcgtcaaacaggtactccgccaatgctttggccagttctgttttaccaacaccggtagtaccaaggaagatgaatgaaccaataggtctgcgcggatcctgcaatcctgcgcggctgcggcggatagcatcagacaccgcgatgatagcttcgtcctgtcctactacacgctgatgcagttcttcttccaggtgcagtaatttatccttttcactctgcatcatttttgataccgggatacccgttgcctttgccacgttttccgcgatatcttccgcgtctacttcttctttaagaagacgtttatgattagcagatattttatttagttcttctgtaagatctgttaccagtttttcctgttcctttattttaccatagcggatttctgccacccggccgaaatcgccgttacgctctgcctgttctgcttccagccgcaggttttcaatcgctgatttggcactctggatctggtcaaccacttccttctctgcctgccattttgctttgaatgtattcctttcttctccaagccgtgctatttcttcacccagctcacgcaatttatcttcgtcgttttctctcttaatcgcttctctttcaatttccagctgacggatccttctttccagttcatccagttcttccggcatggaattcatttccagcctcagtttagccgcgctttcatcgatcaggtcaatagccttgtccggtaaaaagcggtctgttatatagcgctgcgataattctaccgcagcaataattgcttcgtctttgatgagtacgtggtggtgactttcgtatttctctttcagtccacgcaaaatggagatggcatcttccacggaaggttcatctaccaacaccttctggaagcggcgttccagggctttatctttctcaaaatatttctggtattcgttcagggtggtagcaccaatggcccggagttcccctcttgccagggccggtttcaggatgttggccgcatccattgcgccttccatagcgcctgcgcctatcagtgtgtggatttcatctataaagaggatgatttccccgttactttcggctacttcctttaccacgcctttcaatctttcttcaaactcaccacggtatttagcgcctgccatcaaagcgcccatgtcgagggcatagatgatctttgatttcaggttttcgggcacgtcaccattaatgatccggtggcccaatccttctacgatagcggttttaccgacacctggttcacctaccaggatggggttgtttttagacctgcgggagaggatatgcagggttctgcggatctcctcatcacggccgatcaccgggtcgagctttccttcccgggccatttcattcaggttcttggcgtatttctgaagcgtgttatactgggttccaccgctttgggaattaacggtatctcctttacggagttcccggatagcggctttgagacctttttcagtaagaccggcatctttcagtaatttggccgtatcatcgttaccgccgaggatgcccaggagcaggtgctccacgcttacaaattcatctttaaattcttttatggccgctcctgcacggaggatcacgttattggcgtcgcgactgagcgactggccgccttcacctcctaccatgcgggggtatttattgatctgctcatttagcttattgtttacaaatgaggtgtttacatcattctttttcaataagtattcaatcgggctatcttcatcatttaacaaagctttgagcaggtgcccggtttcaatcgactgattctgattattaaaggccagttgctgggcctgttgcagtatttcctgcgattttatagtgaaattattcaagttcatatctgttgttttttctccttttttgatgttatcaaacgtcttctggtaacaacaaaccatgatccaatgttgcaactccggaaattatgacatataagggaaaggattactgcatttttagcagaaaattagcctagtaactgctaatttttcattataaccgcccgtttattccgggtatatttatggtttacctctgatgttatgaaaaatatatttgcctgtatcgtatgtgcagtaccgttattcctgttctcccctgtgctgctggcgcaaaagaagccggccataccactgctggtatctgcccatccctctgcaaaggatggcaaaccgcctatgagtttaaagaccgccatggggttggcgcatacttaccagcagcagcaacccggaagaagtattgaaatacaattccagcccggtacctatttcctggatagcaccctgctgataaccgcgggctgttataatggtaacattacgttccggccggccggaaaaccaggcacggtaactttcagtggaggaaagccattgcagttgcaatggacaccctggaagaatggcatatacaaagcctccgtggacattccttttgagttcagccacctttatattaacaataaacaacagatccgggcacgttatcccaactacgacagcagcgcaaaacattataacggtaccgctgcagatgcgttgagtcctgccaggataaagacctggcaacatcccgaaggcggctatgtacacgccctccaccgctcagaatggggtggttatcattaccgcatcaccggcgtgaacacagatggtacgctccaactggaaggcggctaccagaacaatcgccagatgggtatgcatgaacagcaccgctttgtagaaaatatttttgaagaactggacgcgggaaaagagtggttctatgataaagccactaaaacgctttactataaaccggcagcggacattaacctgaaaacggctgacgtagtggtttccaggttctctgaaatcgtcgttctgaaaggagatgcagcgcatccggttaaagatatcacgtttaagaatatacgttttgcgcataccaatgccacgtttatggatacacgggaaccgctgctgcggagcgactgggccatatacaggggtggagcggtgttgttggacggcacggaaaactgcgttatcaccggctgtgaatttgactataacgggggtaatgctgtatttgtcagcaactacaaccgccatgctgatatcagtcattgtaacatccatgatgccggtggcagcggtatctgttttacgggcaaccccgatgccgtaagagcgcccttatttgaataccagcaatcccccgtatttgccggcatggatacagcagcaggtccgcaaagcctcaactatcccgattcctgcctggcatacgataatcttatttaccgtaccggccgcatagaaaaacaaagcgccggcgtgcagatctctatggcaatggacatcactgtttcacataataccatatacgatgtgccgcgtgcaggcattaacgttagtgaaggtacctggggcgggcacctcatcgaatacaatgatgtattcaatactgtgctggaaaccggcgaccacggggcgttcaactcctggggccgcgaccgctggtggtatcccgaccggcaggtgatggacagcatggctgcattgcatccatggctggtgaaacaggatgctgtgaaaacaaatatactccgcaacaaccgcttccgttgtgatcacggctgggatattgacctggacgatggctcttccaattatcacatttataataatgtttgcttaaacggcgggcttaaactaagggaaggatttttccgtactgtagaaaataatgtgattctcaacaactcttttcatccgcatgtgtggtttgaaaacagccacgatattttccgctataatattgtaggcagcagttataaaccgattggcatcaggtattggggagatatcatcgactttaacgtattcccggatgcagcggccatcaatactcctacggataaacattcacagacaggtgaccccttgtttgtgtcccctgcaacgggcgactaccgggtaaaaccaggatcaccggcgttgaaagccgggttcaaaaatttcccaatgaaccagtttggcgtggtatcggctaacttaaaagtgctggctaaaaaagcaccgctgccggtactaaaagcagccactgatgcttcatccaccatcagcaattggctgggcgcgcaggtgaagaacatagaaacactgggcgaacgctcggctgctggcttacctgataataaaggcgtgttcctggtggccgtacccggaagttttaaatatgccgtaaaaacaggcgatgtgattttacagcttggagaacgaagtgtgaataacgtggatgacctgctaaaagcaagcactttctatacagataaaaaagtaccgctggtagtattcagaaatcaacagcgggttactgtcaattgatatagggggttgttcctttgagcgctcaaaggaacaacctttcctttattcctatcctttggccagctcctggctttacctcttctgcagctttgtttaattatacctcgccggaattaccgggaaatatacatcttgttataaatcaacatcttgcggacaatcatttagatgttagaacttatatccggatgtttattattgaggtaatcaaacaacacggcggcctccgttgttataaaagtccttgaaacacaaactgtacattcctgcttacggccggatgattcagcctaaaaaactggtcaccacattcttcatcactaaaccctacaattatgtctttcgatttactggaaagcgctaaaagtattttcaacagcaatgtcgttagtcaggcctcctcacaactcggagaaagtgaaggcggcattcagaaagccatcagcggtatcataccggttgttttaaccggccttctcaataaggcggggtcctccggaagcgccggcggtttgctcgacctcgtgaaaggagcagcgggtgatgccaacccttccgccattacgggtgcgctgcagggtggtgccgggggcctgctcagcaaaggcgccgatttgttacgcagcctgttcggcgataaagtgaattccattatcggtatgttatcttcctatgccggtatcaaggaatcgtctgccagtaccctgctgcaatccgctacccctgctacgcttggtacagtaggacaatacgccgcccaaaacaatctatctcccaattcctttctttccctgctggactcacaaaaagataaaatacttggcgctatacccggaggactgaacattgccggcgtacttggtttggcgaatatcggcgacctcggtaaaaagctcggcagcctgctgcatatggacaccgctactaccaccggcggcgctgtaaatatcaaaccggatgcaaaacccggcagcagccgctggatatggtcactgctgctcattctcattgccatcatcctgttgtggtacctgatgcgcggttgcggcgccaataaacacgacggcgttcctgttacggacagcgttaccaccagccagattgcagattcggctaccatggcggttacagaaggcggtccggtgattacccgtgaaagcattaaggttacccttcccgatggcgttgtattggatgcctataaagggggtatagaagatcagctggtggtgttcctgaaggacaacagccgtccggccggcaaagatgtatggtttgacttcgataacctcaacttcaaaaccggcaaggctgaactaacggaagaaagtatgaaacaggtaggcaatattgccgctattatgaaagcgttccctaaagccaaaataaagattggtggttatactgaccgcacgggcgacagcaccagtaacctgcggctgtctaaagaacgtgcggaatctgtagttgcggcattaaagaaaagtaacaccaatccggcacagttactcggcgcagaaggctatggttcacagtttgcaaaggcagcagctgatgcttctgaagaagaaaagaaaagagaccggcacatttctgtaagtgttcgcgaaaaataaaatcctataagcaaaaagggaaggctgaatggccttccctttttttattcttttaccagcaccagccggcttctgtctgattttagcatagtggcatagaacttcaccagctcggggtagtctgccgccgggaaaatccccgcctttctttccacttttcgtatatagttcagcgtattccctttgatagaaaccgcagcattataactgccgaatttagcggttacagataccggcgccgggagcgattccggtttatatcccgcgggtaaagtgatcgtcacgctatccacatcccggtaagcaaaatcaaactggatatccgatttgcgggtggtgtcaggttccagcttcaccccatcgcgtgtgaggatattgggaaccaggaacattcgtttacccgttaccgttgcatagttatttcctttgatgcctaatttctcttcaatggaaggaataggtgtttccagctctgtacagtgataattattgatatcataactggaaagatccaatcctttacgcagttcctccagttgtttttccgggctcagtgaatgcaacatgtcacgtaaatcatcctgctgaagaccactgtaaacggttgttgctttaatatcgatgttacctgtagcatcaataacggcatccacatggcggatctgttcattgcaatccattccgtaagcaggggtacgtattaatttgctgtcggttgcatctaccaggagtaccggccggttgtcggtaaaggagcctaggtatccggcgggggcggtgttactggtacattccagccaggtagtatctttctcaccgggtacacagagtatctcgtggttaaactgggaagacgggaaatcttcgcgcagggtatgctcatcgtctcctgcttttaccagtacacaatttgatttaatccccgcttctttcagtaacgccatcatataattagacaaggccttacaatcgccatagccattagcagccacagatgccgcatcaaaggtttgccatccgcctatgcctaactggatactgatataacgattatttttctgaagaaatttatacagtaccctgatcttttcctggcggctgctgataccatcaaccagttcatgtactttggctttgatattgtccggcaacacatcccggcctgcattaagctggtatgcaaagtttccgaaatctttccaggtggtcattttacccttatagctccccaactcaaaatccgttggagccagaaaaacgcacggagtacgctggtacaattcaaccgggtaaatttcatatttcctggcaggcaactggttgacttcccatgtgattgttttgttgcctttctccgtggcgacgactggtttaccctcatagagataactgcggtaacgcaattcatagttctccgggtaaataaccgtcagcctgcttttttcaacagccgtgtaaatactcggctgcgcctgcaaaccaggtatcccgtatattgtattgagacgcagctcaatggtatattccaccgtataggggtatacgttatagtagaactggtgaagcttcgcacgggtatcagacatcaggctgccatcccctaccgcacttatatcgcggatatcgctttgtttcaaacgtttcaactgcttgccttcagcatcatataaggcgccactaatagagcggatctctgacagcttattataatacatccccattttcatatgttcagcccctgcctcatccagcacagtaaccacgtaatgagaaatataacgggcatctgtaagatcgtttattttcaacgtagcctcatctaacctttttaccaggtgcgcattggcccttaatgaatcaggaatagcgctcaccggataaaacggttctcctgcccgcactatctgcgacacggtaaacaggaaaaacaggatggcaatcgataattgcttgcgcatattttactttttcttttttaacacaatttgttctgcttctttctttactaccaggtcataaaaatcgcgcagggtcgggtattcttccggcccaaagttggctttgtttaattttacccggcagcgcagctgtatgtggttttctgtttgctggataaggtattgaaacagcccttcatctccattataattcgctgcagcagatttcggcatttcatctactacatatccttcgggcacttccatattaaaggaatatacttcatcagacacgctgttcatttctacggggaacttacgctccatcgctttaaaaggattgcttttataggcttccgacagcagcgggttgatgtatagtacttcgccgtcgcctacctgcattttaaaatcgtactttaccatcacaggtgactccagttctttcagatcctctaccgccttattctccagttctatttcaccggtataggattttgctatccgtttaaaaaattcttcggggtcttcatcttttacagccgtccgtattttgtaagactcaaagtaggtgggccgttgcataaaagtgcccgacaccatgccgttttctatcttccccaaaattacactggtaaaccgctgttccttcagggaatccgctcccaggatcacaggggtggcaaagtcatccaatgaacgggcggcgccattgtagcactctgccggaagttttccgaagcccagcaacggttttgaggcatccagcttcaggtattcttctcccaggttcacgccggcaattacgtagttaaagtgggtatataaaggatagaactggtatacatatccattgctgcgggtactcagcagcagcggggtagcaaaaaggtttgctttcttcagcatcgccaccagcaacatgttgatgtcggatacgttgccgttctttgaattaaaaacggttttgagcgacttgcccatccacagggcgctgtgatccgtgcaggtaaaattatcgcggacccaggtataaattttctgtactttctccttatcggttttagcgtcttttaccagctcttctactttatcggaaagaaaaccgttgtttgtggtcagtactttgcccaattcttcttccttcatcaggtctttcatcagctcttcccaggtactctgcaccggcttacgcggctctcccggccagttataggcagataactggaattccaccctgttaacatagttatcggtagtagtgatatagctctcgttataaatcggcggcacatctttcagcgcccatttataggtggtgatagaaggcgttaccgttaccaggttggaaggcccggtagacccctgtgactcgttacggaaagtaaaggtagaacgggaataggttttcgtttttaccacatagggctcatatccctgtggaatgagcatatagtcgaagtattccgggatggctacgctgtattcgctccacaggcagggatattttccctggaaatcccaggcgcgtaaatgccggtaaaagggagaggcgatagaaaaggtgtattcaataatagacccttcctttacagcgggcagggtgaatttctttaccagcagggatttatcctgcttgtcgttgaatacgtttttgctttccatcctggtttctaccacttccccgttttcgaggttgtaggcagccgctttcaggttcagtaatttctcttccgatgtttctgatttatatatcggtacgtgaacggtggcctcatcatagccgtttttatcaacgatcttaatgcgccggtgtactttgtacaccaggcgaaggtcgtttccatccgactcaaaaatggaggagcctatctcagacaggataatggcgtgggcgccggtatctttctctgatctattaatagcaaattcttctttggacacttttccaaatttcattttacttccgtcctgggcaaaggtggacagggcgaacaaacagctggcaatgggagccagcataacaaaggtatagcgcatcagttaacaggcatatgggatatatatgcgggtcgaagatataaataatatgctaattttgcccggatgacccacactttattcataaaagagctggcaaaagagttaggatttgaccattgcggcattgcgaaggcagtgcagctggatgacgatgcccgccggctggaaacctggctgaataaaggcatgcatggtaacatgcagtatatggagcatcatttcgacaaaaggatagatccccgtaagctggtcgacggcgcgcagtcggtgatcaccctgttgtttaactacttcccttccgaacagcagcgtgccgacgccccgcgcatctccaaatatgcttacggccaggattatcatgaggtgatccgggcgcggctcaaaacgatgttgctgcggatgcaggagcggataggtcccgtgcagggccggggatttgtggactccgcccccgtgctggaacgcgcctgggccacccgcagcggattaggctggatcggcaaaaacgggaaccttatccataaacaggccggttccttcttttttatagcgaccctgattaccgacatcgaactggaatacgacggtccggtggccgattactgcggctcgtgtacccgctgcctggatgcctgtcctacggaagcgctggtagcgccgggtgtagtggatggcagtaaatgtatttcttactttaccatagagctgaaagaacaattgatccccgataaaatgaagggacaatttgataactggatgtttggctgcgatacctgccaggacgtttgtccctggaaccgcttctccaaagccaaccaggaagcggcgtttacacccgtgccggcgatcctgaacttttctacccgcgattgggaggagctgacagaagaagcttttaaagacatcttccgtcattctcctctcaaacgcagtaagtttgccggtatcaggagaaatatcaacttcctgaacacctagcgactggccgctttaatcagccattgggtcaggtctgttgctgcttcatagttttggaaagatgccggcagcttctttccgtccacatattcgttataaaaccaggggtcgccaacggcgaaaaccttgccttttcccacttcagctactgccataacaacgtattcaccatccttgtaaaccgctcgtgcaggggctttcaaggtcaaagtggataattccttgatgtacacctgccggccagcctggaatatttcatgtccggccgggatccggaaagtaccctgctcccagtttttgccttttacacggttgcggctgtcgccattaaaatggatcccaaatttttcactcagcttgttaaagtgcgaaaattccgcgttggcagaatcgttctccagcaataccagcaccccgccagcctttacccagttataaatactgctggcgtccttttcattcatatagttcggcgtgggcgattccttgtccgtgtccggatcaatgatcatataaatatccgtgtgtttcaggttggcggccgtgggcgcctgcagcaggctatcccttttcaccccgagggagtcgaaaatatgcccccagagcgacacgccgccgttgtccgtctcgccccagatgtaatgccaccttacgggattgccggcattgtcctttttgaattcattattgtaataataatccagcgtaacggtgagttccctggcaggcggctgctgcgcgaaggcggccaaccccgttcctcccagcagcatcatacataaaataatacgtttcatggttttcatattggcaaaaaagtactcaataatcttcaaagattatagcccccaaagcgtgaaattatccagccagggggaaaaatatcgccctgtggtgttttttacttttttttaaataatgtttgctaatttcttgacaatcgttttaccttaacctacttttgtagtaaagtgaacgcaaaaccccataacaaaccgcaaaatatcatttatcatataccggctatgccggattttagctgattaactttttatggacctgagtgccataacgtggaattttagcaataaaggtcgaattctttcgacctttctttttttatatccgttttatgttatattgccgggcaattctattaattgtcagaccaacaatttttcaaccaggtaaggtgtgtacatgcggaagcgggtcttaatattcatcttgttattcctccatactttggtaatgcggggacaaacactcccctatcaattcaaccggattgatatcaaccaggggctgtccaacaaccaggttaactgtgttttcagggatagtatgggtttcatgtggattggtactgtatcaggactgaaccggttcgacgggtatcacttcaccgtataccagcatgatctgcgcgacaccacttctgtttccgacaataacatcaataaaatcatggccggcccggggcagcagctctggatccggacccgctcggggatgaatatctatgatcctgtaacgacccgttttaaccggcgccccgaaaacattctgcgtcagtggggcttttccggaaacgtggttaccgatattgtgaaagacccgtccggcggatattggttcctgcatccgtcagcaggcattttcctggtaaataacgggaacagggcgcaacagtttacacacaccagtgatggtggcagcattggcaccaacagcgtatcggcactgctacccggccaagccgggcattactggctgctgcacagcaatggcctgctggaaaagatggacgcccgcagtcaccgcatcgtttaccgcaacaacacgctcgtgaggccagacattgccggcgccacctggtcgatggtggcggatgccgacggcgacctgtggttattcagtaccaatgaagacaacggcgtttactttttcgatatccgctcccaacagttccggcatattgatcagaatacccccggccttgcgctgaacaacaacattgtaagaggggtggttgccgacaataacgggttaatatggataggtaccgatcatggcggcattaatatcattaataagaaagcacaaagcatccgttatattgagaatatcaacgaagatgaacgcagcctgagccagaacagtatcaacgccctttataaagataataccggcattatatggatcgggaccttcaaaaaaggattgaactattaccatgaaaacatggtaaaattcccgctgtatcaataccaggcgtatagccgtaatagtttgccctataacgatgtaaacaggtttgtggaagacgcggccggcaatttatggataggcaccaatggcgggggcctgatttactatgaccgcagccgcaacacgtttacccaataccggcacgacgccggtaacaacaacagcatcgccggcaatgtaattgtaagcctttgcatagatcacaacaaacaactatgggtaggcacctacttcgggggcctggaccggttcgacggcagccgttttattcattataaacatgacccggcagacagcaacagcgtaagcgataacagcatctgggaaatactggaagacagtcgccaccagctgtggatcggcaccctcggtgcgggacttaaccggctggaccctgccaccggccggttccagcgttttccgcaggtaaaatccacgtacattgccgccctgctggaagaccggcaggggaatctctggataggtacttccgatggtatcgatgtgctacacctggccaccggcgttttcaaacattacaacaacgttcccggtgtaaacggcagcctgagtcataataacgtagtatgcattttccaggacagccagcaacgcgtatggataggcacccgcgaaggactgaacctgttcagtccaaaaaacaataacttccgcacccttcgcaaagaagacggtctgccggacaattctgtcctgaacatccttgaagccaacgatcacagcttgtggatgagtactcccaatggtttgtctaatatgaagatcgggccggacgcctttacctttaaaaattatgacgaatccgacgggctgcagggaaaagacttcaacgaaaacgccgcgttgaaaaccagtcgcggggaactgatctttggcggcggcaacgggtttaacctgttttatccaaacgccattgccctgaacaacaatattccgccggtagtgctcaccgatctgcagatatttaacaaaagtgtgctgccgggcgaaaagatcaacgggcgggtgttgctgaaagcggctatcccggaaacacaaagcatcaccctgaaacccggtgaaaacgtgttttccattgaattcgcgtccctgaattatttccacccggagaaaaacaggtatgcatatatgctggaaggatttaataaagactggctctataccgacggtatggaaaggaaagccacctttaccaacctggatcccggggattataccttccgggtaaaggcctccaataatgatggtgtatggaatgaaaaaggaattacgctgaaaataaaagtacttccccccttctggaaaacctggcccgccttcctgggttatgtattgctgatactgggcgccctgttgctggcccgccgcatcatactggaacgggaaagactgaaattcaggatggagcagcaaacacaggaagccgcgcgcatgcatgagctggatgccctgaagatccgtttcttcaccaacgtaagccacgagttcagaacgccgctcagtttaatcatcaccccgctggaaaagattatccggcaaacatctgaaagcagcctaaaagtgcagctggaactgatgcagcggaatgcacggcgtttactcaacctggtaaaccagttactcgacttccgtaaaatggaagtccaggaaataaaactccataccgccgaaggcgatattatcggttttgtaaaggacctcacctcgtcattttcggacttgtctgataaaaagcatatccagcttaactttcagagcaatgtacaggagctgaagatgttgtacgatgcagataaaatagagaagatcatctttaacctgctttccaatgcttttaagtttacgcctgaaaatggcagtatatccgtttacgttagctaccaggaaacaacctcgcaactggaaattgctgtcaaagataatggtattggtattcccccggagaagcaggagtatatctttgaaaggttctttcaacatgaagtaccggcatctatggtaaaccagggaagcgggatcggcttatccattacaaaagagtttgtgaaattgcatggtggcagcattacggtagacagcgcccctgaaatgggcagctgcttcactgtatacctgccggttaaaacggctgctgttgctgttcccggcgccgtacaggaaacaattcgtactaccaccgccgttacaccggccgccaccgtgaacagtaactctaaaaaaccggtggttttactggtagaggataatgaggatttccgtttttacctgaaagataatcttacccagtacttccagatcatagaagccgaaaacgggcttgcagcctggaaactgctgcagcaaacactcccgcacctgattgtaagcgacatttccatgccggaaatggatggattggaactatgtaaaaaggtgcgcgcacaacagcgcacggcacacttacccattgtattgcttacggccagggccgaagaagcccagcaactggaagcgctggaaaccggggcatctgattacatcaccaagccttttaacttcgaggtgctgctttcgcggatcaaaaacattatctcccagcaatcatctctcagaaaaacattccagcagtatatagaagccaacccgggggaaatagctatttcatctgccgatgaacaatttatccagcaggctttacaaattgtagagaagaatatctccaatcccgacttctcggtggaagaactgagcagggcgcttttcatgagccgggtatctgtttataaaaagatcctggcccttaccggccggtcgcccattgaatttatccgggggatccgcttaaagcgggccgcccagctgctcgaaaaaagccagcttaccgtagccgaagtagcttatgaagtaggattcaacaacccaaaatactttacaaagtatttcaagatggaatacaatgtactcccctccgtttatgggaagaagaaataataccactactacaatcctacatcattcgcctaaacaacaaatttgccctattaaataacgaaatgcgccccatgcctacgggatgcaatggataattttgtggactgactattaaacctgactatgttcaagcaaaactttaaacgaagcaaccgcctgtatctgctgattgaaatcctgctgtactgcgtgatcaccggtttgctcattggcctcttcttcttataacagccttaaaaccagcctgttccttctccatacgttaacatttaatgccctaaccggaatcaattaattacctcgctgctacaaacggttaacataatcgccctacatctaaaacatacccatcccctctgattccggagctccctttacatttgttttacacgttttgaagtaacacgttttgaaaaatagatcgcggataccacatccgtaattgtaacaaccacgttcaaccgacgaaaaaaatccattcaaatatgcacataaagagggcgataccgatcgtacttatgacgttcctcacttcctggtgttatgccgggcaggtggaaaaactgtctgatggcctgttgattcatttaaaaaatcctgccccgaatggcgcccggcaggtgaagctgcaagtggtttccgataaggtgatccacgtaaccgctacccccgacgaccatttcaccggctctcccagtctcatggcggtagatgcacagggtaatagtattaaatgggattcggaagaacgaaatgaaaccgtgactttaaaaacagccagcatcaccgccacagtggcgctgaatacaggagaagtagtattccgcgataaagccggcaacattatattacaggaacaacccggtggcggtaaaagctttacgccgattaccattggcaacaaatcattataccggatccagcaggtgtttgaatcgcccgccaatgaagcgttctatggactggggcaacaccagaccggtttaatgaactacaaaaaccaggacgtggatctcacacagtataactccgtagcagccgtaccttttgtagtatccaaccgtaactacggcattttatgggataattattccattacccgttttggcgacaaccgtccttataaacaaatgtccgaattacacttaacgtcggctgatgggaaacccggattcagtgcaacctatggcgaccggtataataatacggtgtatgtaaaagcggtggaagataaaattgactatgagttcctggatcgcctgtcgtcgcttcctgcagcttttccaatggtaaaaggaaaagtaacctgggaaggcaccgtgaatgcagatgaaaccggcgagtataaattcttcatgaccacctccggttacaccaaagtatggatcaatggtcagctgaaactggaccggtggcgggaaagctggaaccccggcgcttccgttttccggcatctgcttcagaagggacaacccactaccgtaaaagtagaatggatcccggaaacaacccagtcctttatctctcttaaattcctccctcccactcccattgaaggagcggataaaatgcaactgacttcagaagcaggtgaaaaaattgactactacttcatgtatggccagcatatggatgaagtgatcagcggctaccggcaggtaaccggcaaagccaccatgatcccgcgctgggcgctgggcttctggcaaagccgggaacggtataaaacacaggacgagattgaaaataccgtagcagagttccgcaaaaggaaaatcccgctggacaatatcgtactggactggagctactggaaacaggatgaatggggcagccagcagtttgatcctgcccgttttcccgatcctgtgggcatgatcagccgcctgcacaaacaataccataccaatttcatgatctccgtatggccgaagttttatgaagggatcgacaactataaacttttcgacagcaaaggctggttatacaaacagaatattaaaaataagcaacgcgactggataggtaacggttatgtatctacgttttatgatgcctttaaccccgaagcacgtaaactgttctggagcctgttgcagaagaatctgctcaccaagggggtggatgcatggtggcttgatgccacagagccggatatcctgtccaatgcctctattgaagaacgcaaaaagctgatggatcctaccgcgctgggatcagccacccaatacttcaacacctatgcgctggtaaatgcgcaggggatttacgaagggcaacgtgcggccaagccgggtcaacgtgtatttatccttacccgctccgcctatgcagggttgcaacgctatgctgctgccacctggagtggggatatcgccgccacctttgaagagttcaaaagacaaatccccggcggactaaacttcagcctttccggtttgccttactggactacagatatcggcggtttctttgtggaagataaatacgatcagcctaacccacagggtcctgcactggaagaatggagagaactcaataccaggtggttccaatatggcgctttctgccccctgttccgttcacatggtcaatatccttaccgcgaaatgttcaacatcgcgcccgacagcagtatagcgtaccagtcgatgttatactacgaccagctgcgttaccgcctgctgccttacatctactccgtagccggcaatacttaccaccacgactatacgatgatgcgtggcctggtgatggactacggccaggatacagcagtgctgaatatccgcgaccagtatatgttcggtccttcgctgctggtaaaccctgtaacggagtaccatgcccgcagccgggaactgtacctgcctgcaggcaacggctggtatgatttctacacaggaaaatatgaaacaggtggtcagcatattaccgcagcagcgcctttgcagcggatgcctttgtatgtgaaagaaggcgctatcctgccggtaggtccggcactgcaatacaccaatgagcgtaaggcagatacgatacacctgtatgtgtataccgggaaagacggggaatttactttgtatgaagatgaaaataataactatcaatatgagaaaggcgttttcagcaacatttcctttaaatggaatgaagccgcgcaaacactgacgataggacaacgggaaggccgttttccgggtatgctgcagcaaaggcacttcctggtaacgtttgtaggtaaacaaaccgccgcaggaccggatatcagcaataagacaggtaaaatgataacatataatggaatagcaaaaacggtccgggccatctgacctggaccacttcttctaaaaacatttaaacattattcaacctcctttgcctaaataaaacacgttaaacatgaaaatctggtacacaatcagcaattattttccgcggcaaaccgttctaaagacgcttgctgtatgcagtttggctacagcagcgcctccggcactgcatgcagctgccaataacgggaaggcatatacgcaacctgtaaaacaagcaatcacgggcaaggtaaccgacaccaaagatggtgtccccctgcccggcgttaatatcattgtaaaaggaactaaccggggcaccgtaacaaatgtaaacggcactttcaccctgcaggcagatgcgggagaaatactcgtagtgtcgctggtaggctataacaaactggaagtacccgttcaaacgggcagcccaatgacgatacgcctggaatcggcggctacaggactggatgaactggtggtagtaggttatggcgtgcaaaagaaaaaagtggtgaccggcgctacggtgcatttaaataatgatgacctgataaaaaaccacgccatcagcgtggagcaatctttacagggacaggcgcccggtgtgcaggtaacttccaactccggtcaacccggtgacgcgctgaaattcaccatccgtggtatcggcaccaatggcgattcccgcccgcttttcatcattgacggttttccggcggatgatatcagcttcctcaatccaaatgacattgccagcgtagatgtgctgaaagatgccgcttccactgccatttatggaacccgcgcagcgaatggtatcgtaatgatcaccaccaaaaaaggccgcgccggtaaaatgaatgtcagcttcgacgcctcctacggattgcagaatcctgcccgcaagctggacttactcaatgcgcagcagtacgccaacattatgaatgaggcatccatcaactccggctctgtgcctatctatacaccagactccattgcgaaactgggtacaggccccgactggcagaaagcagctaccaataaaaatgcacccatacaaaattatagcctgagtctttccggcggtaatgaaaagtccgttttctcttcgtccttttccttccagggacagcaaggcgtgatggggcttcccggcaggtctaattttgaaagaacttctttcaggattaattcagaacacaagctgtacaaagacctgatcaaaacaggagaaaacctcacgtttgcgcatacacgccagcggggtatcggtacaggtaacatctacaataactctatccgtggtttattaaacgccactcccatttacccggtgtacaatgcggatggcagctatggcaaatcgccttatgcagatgaacccaacccgatcggttccattgattatacacaaaataatcaaaccattaccgacaggatcatcggtaacatctatgcggaagctatcctggttaaaggattgaccctccgtacagatttcggcgcggatatttcgtataactacaacaatgcttttattcccgtatataacctgggaaccaataacagcaacgaacattcctttgccagtcagggtatgtaccgcaacctcacctggaactgggataacaccctcacctaccaactcactgccggcaaacataacctgaacgtaatggtgggtactaccgccaaaaaatacgaaggctataatgtaagcggcagtaaaacagacctgatcatcgccgactttgatcacgctattattgataacggcaggaatgattccacccgtaaagtatttggcacaagaagcatgaatgcactgcaatcctactttggcagggtgttttacagctacgacgataagtacctgcttaccgccacgcttcgccgggatggttccacgaagtttggctccaacaaccgctatggctacttccccgccttctctgcaggatggatcgttaccaacgaatcgttcctcaaaaacagcagctggattaacttcctgaagatccgcggcggatggggacaaaatggtagtgacaggattgatgacttcaggtacctggccaccatcaactccacttaccgcgattattatttcaacggacaaaaagcgataggcgcgtctcctgataaaatacccaatcctgatttgcattgggaagcatccgaacaaattgacctcggatttgacgcaacactgttcaaagacgtaaccgttacattcgactggtatcagaaaaatacccgcgactggctggtaaccgctcctatccccgatttggtgggtaccggcgcacctaccatcaacggcggtaatattcagaacaagggtattgaacttggtattaattataaccacacatttggagaagtaaacattggtatcggcggcaacattgctttcaataaaaataccgtgatagatattccaaaccaggaaggtgtattacatccttcttacaacggcgtattgtcgtccaacatggatgaatacttccgcgcacagaacggaatgcctattggttatttctatggtctgaaaacagccggtatcttccagaaccaggcggaaattgatggttacaccagcaaaagcggccagaaaatacagccaggcgcacaacccggcgatgcccgcttcgtagatctgaacggcgacggcgtcatcaatggtgatgataaaacaaaggtgggtgatcctaaccctacacaaacgtatggtatctccctgtcggcaggctggagaggatttgacctgagtgtattgctcagcggtgtaggtggcaatgacattgtggatggtaccagggcttacgaccgtttttataacaactataccacggctgttttcgaccgctggcatggtgaaggaacgtccaacagcacgccccgtgtaacactgggtaatgaggccaaccagaactacacccgtttctctgatctgtatgtacacaatggcgctttcatgcgtgtaaagagcatcaactttggatacgatcttaagaaaactttactgaaacgtttaccggttcagcagctccggttgtatgtatccggattgaatgtatttacgtttacccattaccgtgggttagatcctgaagtaggttatggaatcgacagctggtcgtctggtactgacctcggttattttccgcagccaagaactgttttattcggtcttaatgttaaattttaaactccggcaatcatgaagaaaataatagcagctatcatcataacggggttaatgagttcctgttccaaaagtttcctggaaacattgcccatcaataccattacagaggaagatttttataaaacaccgggagatgcttaccagggactggtttccgcgtacagcgtattaaactgggatggttacggcaatattgcgctgacatcagaaattgcgtcggacgattgctttggcggcggtggcgcttccgacaacggatggaaccagtgggacaagagcattaaaatgaatgatctcaacagcgctgcctggaagaaatactacactggtatttaccgcgccaataaactgatccagaaaattgaaacggtagactttaaaggagatgatgctacaaaaaaccgttacataggtgaagctcattttctgcgggcttacttttacttcgacctggtgcggatgtttggtcatgtgccattgatcacaacgccactggaacctggtaattacagcatcccgcaggccaatccggacagcgtatacatgctgattgccaatgatctgaaagtggccgcagcgaatattccggctacgccttttgccagcatcccttcgggcgaatatggcagggttaccaaatgggctgctgaagccttgctgggcagggtattcctgtattataccggctactacagcaaacctgatattgccggtgtattttcccaggcagatgcgattgccgctattgaggatgtgatcaacaacagcgggtacagtcttgttccaaaataccggaacctattccgtgcttccgctgaaagcaccactgactatgccgggcagaataacgcagaaggcgtatttaccattcaatatacttacctcggtatgggcgaccagaaccagcagaacggaaaccgtatgcaggtgatgatcggcatccgctcacaggtgctgggaccttactacaaaggatggggtggcgctactgtgaatgaagcgctctttcattcctatgctccgggcgacagcaggcaaacagcttccattatttctattgccggagaaggatttgcagatagttataagctggatgaccaggcgcaatacaccggcttcttcataaaaaaatatacgccgctgaaagataaaaatgcagatgacctgggtggtagtttccagtgggacaatttcgataactatatggtgatccgttttgcagatgtgttgctgatgggggcagagttaaatctcacggcgaatgcaggcaaggcgcagggttatatcgaccgggtacgcgaccgtgcatttggtgatcaaacgcatcgcattacactgagcagtaaagcacagatcatgcaggaacgcaagctggaactggctttggaagggcaccgctactgggacctgctgaggcagggaatgcctgcagctaaacaggcaatagacaatgcttcttcccaggcggctttcaacgtaagcttccgtccggaaacaaatggtttgttctctattcctgaaacacagatcaatttatcaaacggtacgctcaaacaaaacaccggctggtgatattgtccactttaaaaactacaaaaatgaaacgtctgcatatatattttctcggattaattactgcattgttttatgcgtgcagtccttacgaagacaggatcaccccggcagatcctgctggtattaaactggatttttctgtcacacaaaacccggattacgataaccaggtaacgctggaaagcaaaacgaaagatgtgattccattctgggactatggttttggtactaccaaagaagcgaaggcggtagtgatcctgccttttgcgggcgacttctttgttaaatattcggcttatggcacaggtggtcctaaaacagattctgtaaaagttaccgtgagtgcaaacgatccgaagttcttcgccagcaagctgtataatttactcaccaatggcgccgatggtaaaacatgggtatgggccatcgatgttccgggtggttattgttttggtaatggtcctggtgataccgaaaggccggcatggtggactgtaggaaaagcagggctgcaaacccagggcgtactggatgatgagatgacgtttgatctcaataagaacgcaaatttttccatcacgcataaaggtgttactactaaagggtcgtttaccctggatactttagcgcagaagatcaagatcaatggcgctgatatcagttggggaaacaacgtggcctacaatattattaagctgaacgctaatgaaatgacgctggtacagcaaggtgatggctggcgtaatatctggatgttcaagcgcaagggttttgtattttaaaaatccacattatggcccccggcgggaatttccccgccgggcttttttaacaattattttatggagatgataaaagcgtatcacatatatcacaaataattaaaatactcagtattaatcaatgctgttttggttgttacctgttgccggtgcttttcagccccggctatttttttgggtatatactacttttctgcggatcacttaattcgtatttggtgattctttttactatctttcaagacacaacgcctctatgtcatggaaataaaagttctgaccgcgccggggctgggtagctccggaaaattacactggcaaacattatgggaacaatctatacccggaacaaagcggattgagcaaacagattggaatgcgccggtttgtgccaattgggtagcgcagatagagaaagccgtagcagaggccggaccgcaggtagtcatcgctgcgcacagcctggcttgtattgcactggcgcactgggcggggcaaacaaacaggaagatcaggggcgcattgctggtggcgccggcagatgcagaacgaccgggattccctcctgaggcaaccggcttctctcctattccattggtgaagttgccgtttgaaactattattgtggccagcaccaatgatccattctgttccctggaaagagctgcattttttgcccgtcactggggaagccgctttgtaaacgcaggcgccaaaggccatattaacagcgaatccgggctgggagaatggcccgaaggacagaaccagctgaaggaactggtacagaactggccaaccctttaatgttgttaccgccggtattacgctattcactgccgcaacgcttaacctgtaatttcacttttcattccacttttccaccttttttttgaaatctgaataggatatgttgttgccggaagtcttaactaaatcgatttttttaaatagataattaacataaagataaacacggcagcgccgccggctaacaggattataccacctttgcccgctgaatctttaaaactaccttttactatacaatgaaaaaagcactgttcattttatccggtgtaatgatggttaccggggcatccgcacaaataaagcagtatacaatggcgcaggcgcactctcataatgattatgagcgggccactcctttttacgcagcggcttccctgcagtttggttctattgaagcagatatacacctgaaggacggtattttatacgtggcacatgatgccagcgccatagaaccgttccgcacctttaaggaaatgtacctgcagcctgtgctccggcagttttctctttacaacggtaaaccctatgccggcaacgcccccatgcagctgctgatagatctgaaaacagcaggcacgcgtaccttacaggcattacaggaactgctccttccctatcgcaaatattttgatcgcaacgcaaaccctgctgccgtaaaactggtgatatccggcaacctgccgccgatgacagaatgggacaaatatgatcctatcttcttttttgacggccggccagatagcgtatatccggctgcgttacagccacgcattgccatgctgagcgtggattttcacgcttacagtacctggaacggcaaaggaacactgataccggccgaaatgcagaaagtaaccgccgtcatcaataaagcacatcagcagggatatgccttccgcttctggggcgccccctccaccaggtccacctattacaaactgatggacctcggcgccgactggatcggaacagaccacccggaggaattgtatgatgtaatgcacaacactgctcgtaccaccgcttccaatatgccggtacatgaagtgtatatcccttcctttgcatctgatgccacacaggtgcggtctaaaaacgtgatcctgctgattggcgatggcaccggcctggcggaaatgttttccggctatactgccaataaaggcgcactgaacatattccagatgaggcaactcggcttatccaaaacccaatcgaccgacaactaccacaccgactccgctgctggtggctccgccatgggcgccggcgctaaaacacataaccgcgctatcgggctcgacaatacctacgtatctatacccctgatccctgaaatactagcgcctaaaggcattcagagtggtgttatcgtcaccgaagaaattaccggcgccacgcctgcttctttctatggtcataccgcggaccgggatagcacctatacgctggaaaaacaactgctcagcagcaaactgcaactggccgttggcggcggaagggaagaactggaaaaaaacttcggccggcagctggcatcctccggtatacgcatcgacgacaacctggataactgggacgccactacgaaaaaccgtacgctcgtgattctgagcagtaaagtagttacctctatgcgcaacgggcggggcaactacctgaaaactgcactgaaaaaggccttacagcaactgaatgcttccggcaaaggatttttcctgatggtagaaggttcccggatagatcaaggcgggcacctcaacgacctggactacctggtccgtgaaatgctcgacttcgatgaagcagtaggagaagccctccgctttgctgaccaggacaagcaaaccaccgtaattgttaccgctgaccatgaaaccggcggcctcgccctgatggatggcgatatcgccaaaggctccttacgcggtcattttgccaccaacgaccacaccggtatcccggtaatggtattcgcctacggacccaactccaacctgttccgcggcgtttacgaaaacaacgagatctttcacaagatgctcagatgcttcggtaaataatgcagcggaggagcgcctttggcgcttttaaattgtcttggagcaggattacgctgattaaccgtgattgcgctgattttgattctgttttgattttatttttttgattttataaaggattagagaagatataagcgaatatatccgcttatatcttctctaatcttttataaaaatcaaatataaaatcagatataaaatcaaaacagaatcaaaatcagcgcaatcacggttaatcagcgtaatcctgctccaagacaatttaaaagcgccgaaggcgcaccgcgaaaaaaccgctccaactccgcgtttcttttttgtacatttaaaggcattttaaaattcccgacatgttagcaagaatcctattgctgcttacaggtgtgttgtgcctgcatgcagcgtttgcccaggaaacccggtacatctatctttcaggcaccgataaagatcatactgttaactgggactttcattgttccggcggacaacgcagtggcaaatggacaacaattcccgttccatccaactgggaacagcaggggtttggcagctataactatggccatgataaagaaaaagccagtgaagaagggctttaccgctaccgtttctccgcaccggacaactggcgcgaacggcaggtgaatattgtatttgatggcgtgatgaccgatgccgaagtaaaaatcaacgggcgcctggccggtgaaattcaccagggcggcttctaccggttccggtatgatatcagtaaactgctgcgtaacggcagcaatcttctggaagtaaaggtgagcaaaatgtcggcgaatgcaggcgtaaaccgggcagaacggaatggcgatttctgggtgctgggtggtatttaccggcctgttttcctggaagtgaagccactgatccatattgatcacgtggccattaatgctaccgccaaaggctatttttccgtgcaggctttcactaccccattgccggaaggatactctctcagcgcgcaggtgaccaccctggctggccaggccgttcagcaggcagtgaccatacctgccgcagccacccaccctgccgcctatacgttgcagcaacaactcgaccatcccgctacctggagcgcagagtttccccaacgctacctggcagtagtagcaattaaaaaagataaccggaccatacaccgtatcacccagccctttggtttcagaaccattgaaataagaccacgggatggcatatacgtaaatgataccaaagtaatactgaaaggcgtaaaccgccacagcgcctggccggaaacaggacgcacgctcagtaaagagatcagcatactggacgtgaacctcatgaaagacatgaacatgaacgccgtgcggatgtcgcactacccgccggatgaacacttcctggatgtatgcgattcgctgggtttatttgtactggatgaacttaccggctggcaggccgcctacgacaccgtagtaggacacaaacttgtaagagaactggtggagcgggatgttaaccatccttctattattgcatgggacaatggcaatgaaggcgggtttaaccgcgcgctggatggcgactatcacctgtacgatccacagctccgtcccgtactgcatccgtgggaaagatacaatggcgtggacaccaaacattatcccaacttcaattacctcgttaactccagcctgtacgaccaggacatttacctgcctaccgaatttatgcatggcctttacgatggcggcatgggtgcgggcctgaacgatttctgggatcgtatactacaacatccccgtggcgccggcggtttcctgtgggcattcagcgacgaaggactggtacgcaccgataaaaacggcatcatcgacacagatggtaaccacgcccccgacggcatagtaggcccccaccgcgaaaaagaaggcagcttctataccatccggcagttgtggtcgccggtacatatatccctgcccgttattacatccgccttcgatggccgtataccggtggagaaccgttatgactatacgcctttgtccaggtgccggttcaggtggcagctgctgcggtttccatctcccggaaaaaatgaccaaacagacaccattgccgcgggtacaattgcagcaccggatctggcgccccataccaaaggcttcctgcagctgtcacttccaaacggctggcaggatgcagacgcattatatgtcagcgtagacgatggttacggccgcagtatcctcacccgcagctggccactacaaccgccttcccgcattgtacggcagtttcccggggtgagcggccgcctgaatattgtaaccgatcatgatacgctggccgtagataacggtaccggcacttattatttcagccggacaactggtcagctgctgcggattgttaccgccaaaggcaggatttcattaagcggaggacctgtactggcaggcgtttcacaggaactgaaggagttcaggccgggtaccgattccagtggttattttatcatcgcccgttatgaaggcaatggctacctccaggtaaagtggactttcaaacccggcatcccggtacaactggattacagctacagtatcaaaggcgctacgcctttcagcggtattacgttccggtacccggaggaaaaagtaacgggactgtcgtggacaggtgaagggccataccgggtatggaaaaacaggctgcagggacagctcttcggcaactggtataaagcctataacaacacggtgacgggggaaagctgggagtatcccgaattcaaaggctaccatgccaatgtgtaccaggccacctttcatacgaaggagcagccatttaccttttataccggtaacgagggtacgtttttacaggtatttcatccgcaggcgccaaagggagccgctaacaacaatactacgccggcgttccccgacggggatatcggtttcctgagcgccattgcgcccataggcaccaaattccaggatgccgcacagatgggacctgaaagccaggataatatgatgctgaactatacgccggtgaaaggcactatctggatcggcttaccgtaagttgccgggatctgttacaaaattgaggaaagcattgaacttggcgttgtacttacgtttatccagcttgaaatagaaggcgccccgcttggagctgagccggtctttatctttttgtttgatcagcaggccggtagacaagaccttacggctgaagttacgtttatcgaaagtaacgtcatacaccgcttcatacagcagctgtaactggggaatggtaaacttcagtggcagcagttcaaaaaggatggggtgtatggcggccttatagcggagtttctcctgggccatcttcaccattccggtatggtcgaagatgagatcgggcagcttatcaagcgaaatccattctgcatggtactcgtcattgatctgcagtttgtattgattgatatcaatgagggcaaagtaggtgatagaaaccgtgcgttctaccgggtcacgggccgggtcaccgaaggcaaacagctgttccatgtataccccttccaggccggtgagcttcttcaaaatccttgcagcggcggcttcaaagctttcgtcggcctgcacaaatccgcccatcaggctccatttattcttttgcggttcaaatccgcgtttgatcagcagcagcttcagcgcctccccgtcaaaaccgaaaatgatgcaatcgactgccaccagcatccttgattgccctgaataacgtgtcataccagcaattatttatataacccggcaatttatggttccctgctgacattaggaaattatattacaattttccttgtttatctaaacagctgttgcaacacaggatcggtataatccgccacaaaagccctgatattattgtaagcggcaaactcttcacgtgtatgcatggtcgttaacacaatggcctccataccggcgttcaaagcagcctccacacctttgggcgcatcctcaaacacaatacaaccggccggtgcgacgtccagtaactgcgcacatttcaggaatacttccgggttgggcttgctggtagccacgtcatctgcactgacaattgccttcaggtaatgccggagatgcaggttatcgagcacatagttaatgttaaaagtattggcagcagaacctattgccatcgggataccggcagcggcagccttttccaggaaagccgggaggccagcaatcagctcaaggtgaggcctgaatgcttcctggtacaatacttctttttcatgggcaatttcctccatctgttgtgctgtaaaatggtctttcccgaaaacacgcaccaacagttcctcattcttcccgtacatgtggcttcttacaatctcccggggaagattggcgcccagcttattcaacatgttgtaccagccttccaggtgatactccatgtcattgatcatggtaccgttaaggtcaaacagaaatgctttttgctgctgtgtcataatgcctttttttgtaaggcgcaaagatacgggcgaattttgtctttctcaggattacgctgattttactgattagtttgatttttacttttttgatttttttatgatttaataaattaagggagataaaagcgaatatccggttctatctcccctgatcctttataaaatcaaaaaagtaaaaatcaaactaatcagtaaaatcagcgtaatcctgagaaagacaaaatccgcggaattacctatatttgatacaccaacagacaaatccggcatctcaaaataacctgtcttttcagcagctatagttatcattttcaaatattattgtagtatggacattattctaagaaacaacatccatgttaccggtaacctggaaagccctcagacgctggttttcgctcacggatttggcattgatcaaacttctttttcaaaagtaattccctcatttgaacatgattataaaattgtgctgtttgataatgtaggtggcggaaaggccgatataaaagcgtacagtcccaaacgttatgaggctatcaatggctacgctactgatgttgccgatattatccaggcattggatttgcggcaggtgacttttgtgggacattcggtaagtggtatgacaggtatgctcaccagcatccactatcccggcatgattgataagctggtactgctgggttccagtccacgctatcttaatgatccgaaagacggctataccggcgggtttgatcatgcaacgctgacgagtttatttgaggcaatggaagcaaactatcacgcctgggctgccggcttttcaaaagtagcgatgcgaaatgaagacagaccggaattagcggccgcctttgccaaaacgctgaatgacatccgtccggatattgcgatccaggtagccaaagccattttttacctggactaccgcggggagctacccaaagtaacactgcctgtgctggtagtgcaaaccgccaacgatattgccgtaccggccgtagtgagtgagtacctggaagccaatattcccaacagccgccggaccaaagtggaaacagaagggcatttcccccaaatatcggcgccaatggaagtagtagctgccatacaatcgtttctttagttcatcttttcaatttcatattgtgagcacctgggagcacaaagctttaaactttattaatcaaaccggcagatgggataaggataaacatatctcctcctttctcgcattcagcatctccctggtaaaaaacctgacggaagcagacattgcgctgcaactggaatttgaagatgaagaaacagccaaggtgaaatgtgcctctccccttcacctgaacgatatggtactgaaccctgaacccatcaaaaaactactgtatacacagggctttaaaaccatttactggcgagagataccgcctccaaaagagaatgtatttaaagaaatactactggccctgtcatctgccattatcatcccggtaaataccagtcccaataacagcctgcttattcttggatggagtgaaccaccttcctttgaacccggtttcctggagtgtatagaaacaatccggttacggttgaaagaaatactggtgcaatcccagcaacagatctatttccagcgtatagccgtgcggtttgccgctatccttcatactattccgcatgcgctggtgttcatcaacaacgacggattttccgggtgggtaaaccaggaaggcgctgccctgctgggcctgtcgggcccgggagagcaactgcccgcggtactttcagatgccatgatgcaactgcggaacaaaacattgaacctggaagctattgacagggaagcgatgcacctgttttcttcccccgaaaattccatcagcaactggcgctggcaaatggaaaataaggtactgctggtatcctgtttaccggttaccacgcaacagatcagcggaagattatggatttttgaaaacggtgatcaataacgctggcgccagagaaaataaaaagtgctgccttcacccggctgggaatctacccatactttacccccctgctcttctaccagcaatttgaaaatattaagaccgataccggtgccttcttcttttccttcgttgtccagccgctcaaatagtttgaagatacggtcggtgtcacgtttagctacccccggaccattgtcttttacataaaactcatagaactctcctttgtcagctcctccaatggtaatgatgccgtccttcttgtcgttatacttgatagcgttggaaaccaggttctgaaatacctgctgcaacttgagtttattggtttccagtaccggcagggtgcccactgtttcaatatgaatattggcaggtggaaataacaactttgataattgcgtcaccagttcgtggacgtttacctcttcaatggtttgttccatatcgctttgccgggtataatccagcatagacgtaatcatttctgtgaggtgattggtagcgcccagcactattttcatatactcactcaggtcgggcgcatcctgaatgcgttcatcttcgttgatcagcgccagcaggccaatagcgcccgacagcggggatttcagatcatgcgccaccacatacataaaccgctccagctgtttattgatcttttcctttgcggccatggcttctttcagctcatattggtagcggtataatttttcaaatacactcacttttgcgcgggtaacatttacgtcgaggggcttcgacaggtaatctaccgctccttcttcaaagccccgcattacgtattgctcctctttattgatggcagttacaaaaatgatagagatgtcttttgttttaggatttgtttgtaagagacgggctacttcataaccatccatatccggcatttgtacgtcgagcataataagacctatgtcatcgtgccggagtactgttttcaacgcttcattacccgaatcagcctttaagatctccctgttatcgccttccagcatatgttccagggatacgaggttttctgctttatcatctaccagcagtatggtgaatgtttttggtttacgctgcttcatttatcgacgtttattttcgtgctaatatttcttaagtaacggatgatatcattaacggacatggtctgaataccggagcaaagatccagggcagcctggggcatcgtgttaaactcggcggtctgaggatcctgtacaatcgccgtgccaccggacgcggcgatatggcaaagtcctgctgcaccgtctttattggcgccactaagcagtattcccacggcggcattgccaaaggcaagggccgcactctcgaagctcagatctatagcaggccggctgaaatttaccagttcggaatagtccagcgaaatagttccatcggcttctatcagaaaatgataattttgcggggccaggtaaatatgccctggcaataatagttctttatcatccggttctgtgattttttgtttcccggatagtaaggtacccaattcactttgtacatttttcaaacggtggataacgatcaccactggcataggaaatgttgctggcagctctttgatcaatttggtaagcactgtcatactgccggcagaaccgccaataacaaggatcctgtatgaatggggcgttgtcagctttcttacattttacgcctgaaaattttattagcctggtttattgtttcaaattttgtcctttcttcattatataatagtgattctttaatccctaatgccaggtaacctaacgaagttaagctttcataaaataattttactacccggttctgcagtgttctgttaaaataaataaaaacgttccggcaacagataagttgaaattcattgaacacctggtctgtcacgaggttgtgttgaaaaaaaataatgttgcgccgcaaggccgggtggatgatcgcattatcataacgtgccgtatagtagttggaaaaatcgttgataccgccggaccgcatataattagcggtatactctttcatgtctttcagggcaatgatcccgctttctgctttgtccaggttggcttcattgatatctgtggcgtatatcctgcagcggtcgagcaagccggcttcttccagcaatatcgccatggaatacacttcttcgcctgtagcgcagccggcatgccatactttaatgatcggataagatgccagtcgtggcagcacctgctccctcaataccttataaaacgaggggtcccggaacatttcggttacattcaccgtgatatactgcaccatttccctgaagaagttttcttcattcaccaggcggtgtttcagttcaaagacgctgtcgattcccgccatgccggtaaagcggctgaagcggcgcttcaatgaagcgctggcatagtctgaaaagtcatacccgtagcgctgttgaatgatcttcaccagttctgtaaaatctccatgactgatttcctctaccatataatttttatgacaaccatacccgtaacagggaaagcagctttatattatctacgggtttggcgatatagtcggatgcacctgcctccaggcatttctgccggtcgccagccattgccttggcagtgagggcaattaccggcaattgctgaaaccgggcgtcagcgcggatatgtctcatagcctcataaccatccatttccggcatcatgatatccatcagtaccaggttgagtgttggatgctgttgcaatacttccagtgcttcccggccatcggcggcggtgagcaccgaaataccctgttcttccatcagtgcgctgatggaaaaaacattgcgcatgtcatcatccgccagcagcacggttttgccggaaagattgccttccgtccaggtagtggccgtatcttctatgtttgttttcttctgcagtttgtaaaggaaaagctcgagttcatccatcagccggtcggtggcatgcgtggagttgcgcacaatagcagaagcatactttttcagctgttgctcttcgctgccggtaatatcctggtcgaggtacacaaggagcggcgtatcacctgattcggggatctgcgtcagcgcttccagttgttgtaaaccggcctggagatccttaccaatttccactattacggcgtcatactttgttccggcgagcaacgcctgcgcctccggaacacctgcggcgatatcatacctgctgccaagatttctttcggcactcatggtttccagcgtggcgcctgcgctcagcggtcctaccgacaccagcagtacttttttcagccgtgcctgcagttgtgcgctgatgctggtgaatacggcttcaaggtcgctcagttcaagcggcttcctcgtatagccatgtatgttatcttccttaatagcctgtatatctgcgccggttacaacgtgtacaaggattttactcaattcctcactgcttttgaggattttgagaatgctgctgccgtcaattaccggcaggttcatatccaggataatggctaccggcaaaaatttgcgggcataggccagtccgtcctgcccgttatgcgccacgatggttttaaatcccttgttacgggcaaagtcgcgcaggatatccgcaaaatgaacgtcgtcttcaataatcaggatcagtttatcctgtttggtgaggttatcgcggtcgtcgttcacagcaacgggagattgtatctgcggggcaatgtcctttaccggtgttactggcactgcgcccggtatggtagcgtttaccggtaatacaatggtgaaagtgctgccggtagggctgctgtgatcgaggcggagcgctccatgcagcagctgcgtcagttcccggctgatgctcaggccaaggccggtgccaccgtacttacggctggtactgccatctccctggtgaaaggcgttgaatatcagctcctgcttgtctgccggtatacccggaccggtatctgtaacgctgatacagagtgtgccgggagtgcttacatacagggaaagactgaccacgcctcctgctggtgtaaatttaaatgcgtttgacagcaggttgcggattacctgtaacagccggagtttatcggtatggatagctgcaggaacatccggcgctaaatttttggcgaaggaaatctgcttctcgtgcgacaccacatcgaacaggtcggaaaggtcgtccacaatgctctgcaccggcacattttcaaattccatctctactttaccggcttctattttagacaggtccagtacatcgttgatcaggtgcagcaggtcggaaccggatttatagatgataccggcgtactccacttgttttcctgtgaggtttttatctttgttttcctgcaacattttcgccaggatgagcacactgttcagtggggttctcagttcgtgggacatgttggcgaggaactctgatttataacggttgctagcttccagttcagtagccttgagggaaagcgctcccctggccatttccaggtccttatttctttctgttatttctgcgtttacctgccgcagttcttcttcctgcacctttaattcttcttcagatgcctgtaatacttccgactgcctgctcagttcctcattcgactgccgcagttcttcctgctggctgatcaggatttccctttgttcctgtacctgttgaagcagatgcaggatcttttcacgggcattggctgcattaacggcgacggctatatcttttgacaatacttccagcaaccgcaattgtaaaggcgttactttccggaaagaggcgagttcaataacgcccagcaattcattttctatccaaagcggcatcattaccagggagcctggctgaaggtgtccgctggaagagttcagttgccaatagttagccggcacgtcgctgataacgaagatctcctttccggagacggctgttcccaggaaaccgtcgttcagtggcaccgcctgtggaatagcagcgggcatgctaacagcagcgtataaacgaagatcctggtatttatcgtcgtagcaatagaaggcgcctgccgtaaaatccgcgaatgcagtaagggtatgcaggcatttccgtaccagctcatcgcggttattcacgccctggaggctgtcgttcatattattgacgccagtcagcatccagttcttttcattggcagcggcgttgatttccaccacttcatccagtttgcggttcagcgcctgttgcacgcgcagacggcgtttaaactctgcgtaggtgactctcatgaggatagaacctaccagcaggatgaatgcattgttgatcaacagggttctgacagctttggtaaaagaactgctttttacgttctcgcgaacagccagcaaacggcgttcctctccatttaccttgcctacctgtgcccgcaccctgtccatcaacagcgtttctttttctgtaatgtccccattctgttcgaagcgttgctgtactaaggtatgatccagtacattccagtagctgagcagggcattgatattatcttccagggagtctatattttttagctggttcgggttgtccgctaccatggtacgcagatcgtttacggcgggaggcactttgggaagcgccagctcatagggttgcaggaattttttattaaaagtgccccggaaacccctgcgggaagcttccatatcaaataataaacgctgtaccctttcggaaccattgagtacgcgataagtgtgctgtacccatcccgcctcttcagtttgctcggtaaacgtttgccacgttaaaaatccgccgagtaaaacaagcaatacaataacggcaaatccgaggtacagtctgttaactaatgaaatcttcatataatattaattccttaatatagcataaaaatacctaaatgcactcacattcaatacctttggggggagcaataaatctgtttaaacagtaatgtaaccatttgtttttatcaatggaaaactattcatttatttttaaagtatatatccatataacatcagccatttcaaataccacgaagcgcatctttagaaaacacaataaaagtatcaccctgccgaacaattaaatatcagttttgtttagcggattaaattcagccacgatgagtaaaattttgttagtagaagatgatgagataatgcccaaaatagtggcaaggattctcccttctgcagagtatgagctggaccacgtatcaaacggaaaagaagcatttgaaaaactggaagccaccaattacggttatgacctgatcattacggatattatgatgccgtatgccaacgggtttgaaattctgagccgggtaaagagccagcccaggcccatcccggtgattattgtttccaatgccggcaacgaggacatgatcatggagggctttaaactgggagcagatgatttcctgaagaagccgatcatacctgcagaattactgatcagggtcaaaagattgttaatgaagaataaatagctgcatgttcgatatacccattcctgctttcctggatcccgccctcagcacattcagggaagcgccattggccatcaggctggcaatgatatttattatagtggctgtcctggttaccctgctggcttatctttctatattaagaagccggttcctggggcatcagcggagaaaaagactggattacctgctcccgaagatcgataacctgatcattgatgagatcatggctaaccccgaagtagccgcaggcacaccggccagccagatacagctgaacctggatggattccaggaactgcctttacataagaaatgggccaggcaggctaccacggaccgcattatacatttccgccgcaatgtaagaggcaatgccggccacctgctgcgcaacctgtacatccagctggaattgagcaaggataccatgaagcagatgaagtcgcccaaatgggcccggaaagtacgggcactgacagagttcatcgacatggatatccccgtggcagatgtaaccattttaccattaacgaatagccgtaaccgtgagttacgtgccgccgcgcggcatgcgtatatcaagctcagtaaaaatgagccctttaaattctttgatgtggtaaccgatcccctgctgatgtgggaccaggtggaattattccggatcattaccactacggaagatatctccattcccaacttcgccaggtgggtcacctactcttccaataaaagcgtggtttccttttgcctgaaactgatcgttcattataaccagctgcccgctgtacctgcagtaacccagctgctggacacgaaagatcattacctgcgcgcagacgccattaattgtcttggtaaactaaaggtccccgacgtggaagacaggctggtatccatgtacagcagccagccactgcaatgccagatcgaaatactgaaggccataggccgcatcagcagcggacgtcagatcgacttcctgaagcaggaattcctgcattctaccaacttcgatctgcgcaaagctgccgccaaatccctggtacgaaacaaccagctagccggcaacgtaatacaggaactgctggaaaccgctaatcgcgaaaacctgctgatactgaagcattgtatgaaccctttaattaaatactgatggagggcattttatcatggctgggcagggcctacgaaaatacacttttcgtatatgggttggttttactactggtatacgccttactggccctgctgtcgatgctggctatccgccattacacccggaaaagcacccaacatcagctcgacatactggccagctcgccgatggcgcctggtcttactatccttgcacctgcctttaatgaaggcctcaccattatttccaacgtgcggtcgctccttacgctcaactatccacgctatgaaatcattatcatcaacgatggcagcaccgataataccatggaacagctggtctcggaattcaggatggtggcggtggactttgcctataaccccaggatactgacgcaacctgtgcggaagatctataaatccactgaccccgcttattctgccctgatggtgattgataaagtgaatggtaaaagtaaagctgatgccgtgaatgcagggatcaacatcgccacgtttaagtattttgtttgcaccgatgttgactgtatccttcataaagataccttgctggaactggcactgccggtaatgcaggaagaaaaaagaaaggtgattgccgttggcgccactttgcgcatcgccaattcatccgactttgacgaaggagtgctgatccgtatgcggcctccccggcagctgctcccccgcttccaggaggtggaatatatccgttccttcgtattggggaaaatgggctggagttatattaattgtgtgcccaacgtttccggcggactgggtttatttgataaagaagtagccacccgctgcggaggctatgaccacagctctttcggggaagatatggaattgcttaccaggatgtgccgctatgcacacgacaatcagattgactatgcagtgaagtatattccaaaaaccctctgctggacggaaggaccggcttctgtaaagatattcagccggcagcgcacccgctgggcgcgcggactggctcaactaatgtatgcccatttcagtatgttcctgaatccccgctatggaaaaatgggactgatcgtatttccttttaacttcttctttgaattactggcgcctttggtagagttcagtggtgtgattatttatatatacctcgccgtaaccggccaggtaaactggccttatgcatcgttgctgctgcttttcgtatatacatacgccgttatgatcaccactatcgctatcctatgggatcagctttcttttggttattataagaagtggtgggaggtagcctatttgtgcctgacaccttttatggagtttttactataccatccgctcattgtatttttttccctgcggggatattattatttcctgacgggcaaaaaaagtacgtggggaaatatgcagcggcaaggctttggaaaaaagaagaaataaagaaaacagtgtgctatgctcagaacaatttttgaaggaggcgtatttatatatggttgcgtactgttgtgcatgtacgccttgctggcgtatttgtcttaccgtggtattatccgtttccgtaaaaaaagtagcttcaccgactataatcacctgctcgattccccgctcacaccgggcatatccgtgattgcgcctgcctacaatgaaagcgttaccattatcatgaatgtacgttcgctcctgacgctgaactatacacgttatgaagtgatcattgtaaacgatggcagtacagacgatacgctggaaaagctgattatggaatttgaactggtgccggtagatttcgcctacaacgaaaggatagtaacacaacccgtgcggcaactgtttaaatccaccaacaccgcctacgataaattgctggtggttgataaagtaaatggtaaaagtaaagccgatgctgccaatgcagggatcaatgcggccgccttcgactacttcctgaacacagatgtggactgtatcattgaaaaagatacgctgctccgtatgatcaaaccattcatggatgaagagcataagaaaaccaaagagatcggggaaccttgtccgcagtgcggatatgtgcatgtgatggaagacagccggcaggtgatagccaccggcgctacgttacgcatagctaactcaacggaaattgatgaaggcgtgatcatacgggtacgcccccccgaaaaagtgctgccccgtttccaggaaatggaatatatacggtcttacgtgctggggaaaatgggatggagcgtgatgaacagtgtacccaatgtttccggcgggctgggcttatttgataaagaagtggctatcaaagccggtggctatgatcacagctcttttgcggaggatatggatattgtaacccgcatgtgcgcatttatgatcgataacaaactgaaatacgccatacgttatattcccaccacgcaatgctggaccgaaggccctccgaatatgaaagttttcagccggcagaggacccgctggggtcgcggattggcggagatcatcaccctgcaccggaaactcattttcaatccgcgttacaagaaactcggactgattgtgttgccttataacctgttcttcgagtttctggcgcccatcatagagtttaccggtatcctttattatatctacctgattattacgcaccaggtaaactggccctatgcacttatattattactctttgtatacctgttctccgtgatgatcagtacgctggccatctgttgggaccagcttacctacggctattacaaaacctggcgggaagtgatttcactgtcgctgatggccttttttgaaccgctgatctaccatccgctgattgtattttttgcactgcgaggatactggttcttcctgacggggaaaaaatcatcgtggggaaatatgcaaagacagggatttggaaagaaaaaataaacttataaatgacaagcaaatggctgtattaaaacatctgttaaccggaatactggtgtgttgggcgatgcaaacgcaggcgcagattttaaaacagaaggataatgcagaagcactgtataaccaggccgtccaggaaacaaaactgcagcactatgataaagccatcagcttatcgcacgaagcgctgaaggcgcaacctgattttattgatcagcagctgttactggcgcgcctgtatatgctcaccaaacaatatgacctgtccaggaaatataccaaagcagtacttgccaaaaatccgcgttaccgcgatgcctattattatgcgatcaatgtagaacttaccacggggaaatatgcagaagcggaatgttatgcagatgaggccctggcgtattttcccggcagccgggaatttatgctgaagaagctgggcatactggatttgcagcacaaagtatatcgtggcaatgaactggccgaaaccatcatgagcaaatatcctgaagacaccaccgtgcgcaatgcctatattgaacactacctgcaaagcggtaagtactaccagcaattaggcaacagcggcatggcacgtcagagttacgaccgggtactattggctgatcctcataaccgcgatgcccgcgaagccaacctgggcgtggcattaaagggcggaaattaccagtcggcgctggagcaggtgaatgatgaacttgccgctcatcccggcaattacgacctcctcatgcggaagctcagcatcctggaagacatgcacgcctacgtagaagcgctgagtaccttacaggaaatacaacggcggtacccgggagatgccaaagcacgcactatggaaacttccctgcgcatggaagccgctacttactatgctaacatggacccctatacgctttatggcagtgtgctggaaaaaaatcccggcaaccgcgaagcgctcgataaactcattggttacagtatggcccgtggcgcttaccaggaagccctggcatggattaacaggggactgaaagccaatcccaacgacagccacctgctggcattgaagatggatgtattggaaggtgaccgtaagtatggcagcgccgcggcactggcaatgatactgtatcagcgctcacccaatccgatgctcaaagaaagactggtacagctgcaaaccgtcaccgggcgcgaataccttgcacagcagcagtacgacctggcacttgcctcctttgagtcggccctgaaggtaagtcctggcgactctgcggtgctgcacttgctcgccaatacctacatctcccaaaaaaatacctccgctgcattaaaagtactggaccaggcactcacttattacccggccaatgaatcttttctcctgaaaaaatccggtgtgctggcagatgccggcaggtatgaagaagctgccgccattgccggtgaactggcaacccgctatccttccgatgagcgcttcagcaacaactttgttgacatgcgtttaacagcaggacgtaatttaatgaaggcagaagaatatgacctggctaagcaacagtttgaacaggtactggccatagtgccttccaaccaggaggcgctcgattatatgatcaacatgcaaagcgccaccggtaaacccgacagcgccctgtactttgcagataaagcgctgaccttgtatcccggcaaccgtgatttcctgctgaaaaaagcatccgtgcttcaggacatgcatgcgtataacgaatctgctgccattaccgccgacctggtgaaccgctatccctacacactcaaatacaaaaatgcataccttaccagcctgatgtcggccggtactgattaccagcgtaatcagcaacccgacagcgcgctggccgtgtttaaccaggtactggccttgcgcccgaaagattcaatggcgctgttgtacagtatcaatatcctcaacgggcagcaacgctacgacagcgccctcgcctacatcgcgcagggaataaaatattacccggacaatgaaacctttttaatgaaacgggccatcaccctggagaataaaaaagatctcacggccgccgcactggtagctgattcgatcgtaaagctgcagcccactgccgtgaataccgactaccgtgattacctggcaagtaaaacattgaagaaccagttcggattgtattacctcaactccagctatgattacatgtccgacaaatataacattgccactattgaataccggcgctacatcaaacggggctcttacgcggtgcagttgaactacgccggcagaaaaaccggcaatggcttacagggactggcagaaatgtattacacccacacgcctaaactgtattcttatggtatgctggcttactccaacaaaacggtgttcccacaattacgggcagcctactcgatattcaagacctttaaaaaagatatagaagtggaactgggaggccgttacctgaacctggacagcaccaatagcatttccggcgtggtttctgtggcaaagcctttcggcgatttctgggtaaacctgcggggatatgccatcagcgaatcttctgatttttacacgtcctttaatctcaccacccgttattttatgaaccggcggcaggactatctgcaggtagtagcaggattaggtacctctccggacgacaggagccggctgattaactttcccaatcttaccggtttgctgacacatagcattggcgcaggctaccagaaagtgatccggtaccggaccacactcggacttttcggcacctggattaaccagaagatcagtgataccgggtaccagaaccagtacgatatttatgtaacgcttcagcgtaaattttaacggaattacaatgtgcagaattatgaacagccttttgttaatgatcactacgttgttatacagtgcctgtcggcctccggcagaagagattacactggtacagcagggacgcagcgaatacgtgattgtgctgccggaacaggctaccaaagcagaaagcaaagcggcaggtattctccgggattatatccaacgtatttccggagctgcgctacccgtgatatcagaacctcaatacaaggaccagccggcggtgtttattggcaataccacccatagtgcaggcccggctgaaattcatggagaaggttttttcaccggcagcaaaagcaggcagctctttatccgtggtggcagtggccagggagtggtgtatggggtatattatgtgttacaaacgtatatgggttgccgtaaggatgctgcgggtccggcagtaatacctgcggtgaaggatatacgactaaacggcgctatctccgatttgcaggagcctgcatttatttaccgggaaagctactaccctccttccatggatgccgaataccttgcctggcatgggttgcaccggtttgaagacctttggggcgtatggggacattcctttttcaagattcttccaccggatacttacttcagggatcacccggaatactattcaatggtaaatggtaaaaggcagccgttgcagctttgtttaagtaatgaaaacgtatatactttaacggtagactggtttaaaaaagcgatggcaaacaacccggatgccatgtactggtctgttgccccgcaggatggcggcggcggctgtacctgcgatctatgccgcaaggcagatgcagaagagggcggtccacagggttcattgatccgttttgtaaaccgggtagccaaacaattcccggaccaacgctttactacgctggcttatggctacaccgccaaagctccgttaaaaacaaaaccggccgccaatgtatatattatgctgagcactattgatgcattccggcaggaaccactcacccaggcatcttccgcagccgggttccgcaaaaacctggaagactgggaagccactaccggcaacctcttcatctgggattataccacgcagtttaccaattacctgaatccgttccccgattacagcaacctgtcatccaacctccaatattttgcggcccatcatgtaaaaggcgtattttcccagggcagcggcgaaacctatggtgacatggcagaatacaacagctacgtacaggcagccttgttatggcaaccggctgctgatatgaaaaaggtcaacagtgactttttaaagggctattacggtgctgccgcgcctgcgatggggcaatacctcgacgcgctcacgaatgctgttaaaagcacccgtgcggtgctggatatctacggtaaccccatctactcatcgcgcgattatttatcgccggtgcaaacagaccagtattccggttttctcgataaggccgaagcggcagtaggtaacaacccgctttatctccagcgtgtatataatacccggttattcctggaatatgcggtgttgcagcaatcgcgtttttatggcaccgaaaaatacggctatctccagcctgatggcacggtaaacccgcgatggccgcaacgtgtacagaaatttgtagcgcaatgtaaaacagccggtgtgcaggaactggcagaaggcgggttggcccctgatgcctatgcgcaggagtggcaggagttgttttcccgtaaatgggtgaagagtcttgcgttaggtgcggcggttacccttgcaaatccgtacacgccggagtatacgcctaaaaaggagcgtacgcttaccgatggattaaccggtggcaacgacttcagttacaactggctctttacttatggtaaggatatggtagcgaccattgatatgggcagcagtaaaactatccgccaggtccaaatgaattttttacaggatgcacggcattatattttcaatcctgcacaagtgttggtggaaacatctgcagatggtactcactttacctctgccggcgtaaaggatattcctgttccggaggaagattacgcagtgcgcattcatcactatagtttctctgtcccgggcgtttcggccaggtatatccggatcactgccaaatgtccggctacacttcccgattggcgcctggtggagggaaagaagccctcgctttgctgcgacgagattacggtggaataacccttacgtacaggcggacttgatacggtgtatcttaattatcagttaaatgcctgccggaattcaagaggtgacaaactggttttcttcttaaacagcgtactaaacgattgtgcgtgttcaaagcctaatgcataagcaatttcgcttaccgacaaatttgtagtcgagagtttttccttcgccttttcaatcaatcgctgatgtatatgttgttgtgtattttgccctgtatgcatgcgcagtagatcgctcaggtagtttggagacaggttcatgagttcggccatgcgttgtaccgttaatagttccggttgcgttgtcgtactgctgtcaaaatactcatcaacaaggcgttcaaatttggcaagcagttgatgatggtggtttttccgggtgataaactgccgctcgtaaaatcgattggaataattgagcaacaactcaatttgcgataggataattccctgcgtatatttatcaatatgcaggcattccttgtcgatcttgttcaatattgtaataagatcatcttcttcttcagcagaaagatgcagcgcctcatttacagcgtaagagaagaagttataaccgttgatgttgcttgccagaggatgggccagcaaaaagtcaggatgaaaaacaagcaggtaaccggatccgcattctacgtttttcagatccaggtattgaacctgattaggtgcggtaaagctcagaacacccttattgtaatcataatgttgctggccatatcgtatttttcccttgacttcccttttgagggcaacacaataaaatctattcacaaaacctttccatacatcatcttccaggaaagtactttcggcgaggttaatcacacttaccaatggatgacgtggctcgggcaaagagagcaaccggtgaaattctgagactgatctgatggcattcatcatactaatttaaacattttaaggtgtagaatagcggttgcattcttaaaaatgcaaccgtacaatacgctagtcaataagccccatactaaactcatcgtatggattaccggtatcagtacccaacggcacaatgctttcgagtttcaacagatcagcttcgtttaattcaattccggtggccgctatgttttgctctaaatattttcttcgtttggtacccggaataggtaagatgcccttatttataatccaggccagtgccaactgtgatgtggttatttttttctctccggccattgcctcaatggctttaaccaactcaatattcttgtaaaaatgagcttcctgaaaacggggaattgcccggcgaaaatcattttccggtaagtcatctatggtccggatctgcccggataaaaaaccacgtcctaatggggaataagcaacaaaacctatcccaagttcattcaaagtattcagtatgccacgttcttctgttgtacgctcaaataaagaatattcactttgtaccgccgtaatcgggtgaaccaagtgagctcttcttatagtttctgaagatacttctgatagtccgagataacccacttttccttccttcaccagctcactcatcgcctcaatggtttcttcgatgggcgtgtttttatcgagtcggtgcatatagtacaaatcaatgtactccgtgttaagatttttaagagaacgttccaccgcttttttcacatattcttttttgccattaatagcccaggtcactttgttgttatcatctatttcccaaccgaattttgtcgcgataatatacttattcctattaccagctattgctttagcaatcaactgctcatttttgaaaggaccgtacaaatcggcagtatctaaaaagttgccacctaattcgagcgatcggtgaatggtagcaatagcttcctgctcatctgcctctccatatatatttccttcttcaaaacccgtcatacccatacagcccaaacctataattggtacagccaaaccttcgcttcccaaatttattttcttcattaccatactattaattttaataggtcaaagttcgctaagaacactttaatagctgtatgcaaagccctgaaagttgtatgcaaatcaaggacctgacacctgatctccccccctttccggggcccagaaatctctctccctaaaaataaatttggaaaataaacactgttcagtatatttgcactgtaaacaattcaacgtgggcataatagaaagaaaagaacgtgaaaaggcggaaatgcgcaggcgtattgtagacgtagctattcaaatgtttgtggaagacggatatgaaaaagtatcgatccgcaatattgctgataaaatagaatacagtcctgcaaccatttatctttattacaaggataaagatcagctgttatatgatgtgcaaacagaagcatttgcaaccctggcaacagagttcctgcaaaaagtaaatagtaacgaaccattcaaaaggctggagcaactggcacgtgcatatgtggagttttcgagaaatcatccggagttatatgacctgatgtttatcataaaagcgccgatgaatgccgtgatgaaagaagaaaagtggatgaacggagatcctgcctatgatgctttatataacctcatgcaggaatgtatcgacaaaaaattggtgaagtttaaagatgctacaataggcaccctttctgtatggggctttgcgcatggccttgtgagcctgcacctgcggggaagatgttccaaagtgtccagggtttcagatgaagatatgccgggagtggtagatgaagcgattaaggaatacctgcgaatgattaaagcataagcactgctttgtgaagatgaagtgaaaccaaaatttacttaaaagccttgacggcttttttttaagaacatcattaaacactgttcattatatcaacaacgattaacagaaagccagccggctttatttttttcggcatcaataaacaccgttcattatgtacacatcaatcacaaaaggagcattgttaataggcctgatcacagcgggcttcagctcctttgcacaaagttctgtgctggatcaatacatacaatccgctttcagcaacaataaaggattaaaagatcaaaacttccagctgaccaaatcaatgctcgccttacaggaagcaaaaagcctttttgggccgaatgtatcggtactgggcagctacaccaaatcagcaggcggccgtaccatcgattttcccatcggggatattatgaacccggtgtacaatagcctgaatcagctgaccaacagccatgatttcaaaaacatcgacaacgtatcggtgcagctaaaccccgataacttttatgatgccaaagtaagggcgagtttgccgctgatcaatgcagagatttattacaaccagaaaatccggagagaacagattacacaacaacaggccgccctgaacgtatacaaacgggaactggtacgcgatattaaaacggcctactatcaatactaccaggccgcacaggcggtagctatttacaacaatgccttgtcgcttatcaatgaaaacatccggatcaatgagagcatggtgcgtaatggcatacgtaacaacaccgccctctatcgcgcacaaacggaaaaacaaaaaacagatgccgatatcaacaaagccattaacgcccggcagaattccaaagcttattttaatttcctgctgaaccgcggactggatgaaaatattacgctcgacagcacccttcttcagatgccggcacagctgcctggcaaagatatcaacggccgtgaagaactggcccaatataaaagcgctgctaacgtataccgcttaaacgaacaacttcaacgctcctacctggtacccaagctcagcaccttcatcgatctcggctcacaaggcaccggcgcgcgtttcgataaagatacccgctactatatgtttggcgtaaacctggaatggaacctgtttgcctctcacaaatacaaatacaaaatcaaacaggccgccaacgaagttgctaccatcaccaatgccgccgatcaaacaaccgaccagctacggttacaactatacgaagcagtaaacaattaccagacggccattctaaattttaaaacagcgcaaagccagctgtcttttgccgaaaggtactaccgcgaccagatgaaagtgtataaagaagggcaactgctgtatatagaactgctcgatgcccaaaaccagcttacccaggcccagctgcaaacggccgtagcacaggcttccgtgcaaacggcctacgcgtcggtagaacgcgcacaggcatcttacgatattaacaacaattacaacaaccaataaactcacactcatgaaaaatacattgctcctgctgcccttttccctgttgctgttttcctgcggcagcaaaccggcagcaaccaccactgtttccgataccatcccggtaaaaatcatgccgctggaaaaacagggaaccgccgttacgatcaatgcttccggtcagtttaccaccgacgatgaagtatatctttccttcaaaaccaacggtatcatcagcagcatcctcgtaaaggaaggtgataaagtacataagggacaactactggcgacgctcaatcttacagaaataaatgcacaggtgcaaaaagaccagctggcatttgagaaagcccagcgcgattatcagcgcattgtgcggttacataacgacagcgtggctacacaggaacagctggaaaacagcaaaaccacgatggaccaggcacggcagcaactgagcaccacccagtttaaccgcagcttctccgctatccacgccacccaggatggttatgtactgcataaactggtcagcagcggccaaatggtaaatgcaggtacgccggtattagaaaccaacggcgccagcagctcccactggttacttcgtgtaggcgtgagcgacagggaatgggcgcaggtgaaaaacggtgataaagccagtatcgaaatatccggtatccccggcgacagcctcactggcatggttacacgtaaatctgaaggcattgatgcacaaagcggcaccttcctcattgatgtacaactcaccggcagcaagcccgccgctatcgcggccggcatgtttggccgctgtcatattcaggccggtgcagcttccggcagcaccgcatggagcattccatacgcctccctcctggatggaaacggcagcagcggttttgtatttgtaaccaacgacaataaaaccgcacagaagatacccgttaccattgcagggatggaaaaagaaaatgtactcatcagcaccggcatggaacaggcaaaggcactcatcatttccggcagcgcctacctgaaggatcaatcacctatccgtatcatccaataactattacgatcatgaaaatagccagatatgccgtcaaaaattaccagttcacgctggtaatattcataatgatcattgtgctgggcatcaccaccatcctcaatatgccccgctcggaagatccggaactgagatccccgcaatttaatatcgttgtagtgtatccgggtacaagtcctaaagatatggaagacctggtggtagatccaatggaaaaagaaatctacggactggatgatatgaaacgtgttcgtacctccatcagcgacggtgtggccgttatgcacgtggaatataaatacagctccaacgtagaccagaaataccaggagctggtgagagaggtaaacaacaaacggcaggaactgccggcagatatttacagcattgaagtgcagaaacaggaaccctctgatgtaaatatcctgcaaatagcgttaatctctgaaaatacctccagggacaaactccgctactacgctgataagctgcaggacgaactggaaaaagtaccttccctgaaaaacgtaaagctgcatggcttgccggaacaacaggtaagggtagaactgcaattagataaaatggcgcagctccacctgccggtgaataccgtaatggcagctatgcaaagtgaaatggccaatatacccggcggcagtatcgatgcaggtgataaaagcttcaatatcaaaaccagcggtaattatcagcacctcgatgaaatcagcaacacgattgtatctgccggtaatgggaaaaatgttttcctgaaagatatcgcacgtgtatactatggttttgaagatgagaagtactttgtacggctgaacgggcaccggtgcgtggtagtatctgctgctcagaaatccggtgaaaatattaccaaaacacagatcgcctacaaaccggtgatcgaaaagttcaagaaaaccttacctgccaatatcgatatggtgcaatacttcgaccaggccgacgccgtaaacagccgtttaagtggcctgggaaaagattttatcattgctatcctgctggtagcctttaccctgctcccgctgggtcagcggcctgcactcattgtgatgatctctattccactgtctttgtcgatcggtattgtattgctgcagctgtttggctatagcctgaaccagctgagtatcgtaggactggtagtagcattgggattgctggtagatgatagcattgtggtagtggagaatatagaaagatggatgctggaagggcatagccgtatggacgccacactgaaggccacctcacagatagggctggcggtaataggctgtaccgcggcattggtgatttcgtttatgccgctggtatttatgccggaaggcagcggtgactttatccgcagtctgccgctggcggtgatcttcagtgtactggcatctatggccgtgtcactgactattattccattcctttccagccgtttgctgaaggagcataccggtaatcctgaaggcaacctgtttatgcgtttgctcaaaaagctgatccatggcagttatgcaaagctgctcgacaaagcactgcatcgcccggtgatcacgattgtggtatcactggtaatttttggcgcctctatcgggttgtttaaggtgattggtttcagcctgttcccggcctcagaaaagccacagtttctgatcaatatttttgcaccgccacagtcgaacctgcactataccaacagtattgtacagcagatagaaaaagagctgaagcaggaaaagatggtaagctcttatgccagtaatatcggcaagggaaatccccgcatctattacaacgaattacaggaaaatgaaaaaagtgactatgcacagctctttgtgcaactggccccccataccagtccggctgacaaaaacaagctgattgaatcgctccgtaaaaagtggacgccctatcccggcgccaaagtagaagtaaaaaactttgaacagggtccgccgatggtggcgccagtagaagtacggctattcggagataatctggacaccttacgatctttagccggtaatgtggaaaagatgctggagaaaacccagggcaccatctatatcaacaacccggtaagtaacctgaaatcggatatccgggtgcggatagaccgtgaaaaggcgcagcagttgggtattcccaccgccaatattgacagggtagtacgtttagccgtggccggtattaacctgggccaatataatgaccagaatgataatgactacgacatcctgcttaccaagcagaaaacggcccaacccacactggatgtattcagggatctgtacgtgaacaacagccagggaaccgcgattccgctttcacaggtggcacagctgcagctggaaacatctcccttaactattaaacaccaggagaagaaccgggtagtagcagtaagcgcctttataaagaagggcttcctgaccgaccgggtgatagaagatgtggtaaaacaaatggatgcgctgaaactgcctgcgggatatacttacgagatgggaggagaagtagaaagccggaaaaattcctttggcggatttatgagtgtgatcattgtgacgatcttcctttttgtggcggtgctgatcctgcagttcaaaacgtttaagagtatgctcattgttttatcagtaatacctttgggtattgtgggtgctgccatggggttatggctcaccggcaactcgctgtcgtttgtagcgatcatcgggctgatagcactggcgggtattgaagtgaagaacaccattttgctggtagacttcaccaaccagttgcggatgcagggcaagcccctggaagccgctatcagggaagccggcgaggtacggttccttcctattgtgctcacttccctcacggctattggtggattaattcccgtggcgatatccaccaatccactgattgcgccgctggccattgtattgatcggtggtttgatcagctctactttgttgtcgcgtatcgttacaccggtggtgtataaactgattccgccgaggattgaagctattaacaacaacggacatagttcacaaaaacggcaggacctggaagaggaggaagtgatattagcgccgcatgctataattcacaattcgtaattagcaattagttccttacttttatggctaatttgcagtcaccaatcctctgaaaattagttcttatgaaaaaaatcttcctggcatttgcaaccatgctcctgatgatctgtatcagttcacagtcgtcacaggcacaattgaaacgattcagtatcggtccttttgttgaagcaggcttcccggtaggcgacttcggtgatacccacaataccggttatggtgttggtttgggcgctgatgtaaagctgatagcaggtttaactgctgtgggttccgtaagctactttcattttggcggtaagagctttaacacaggcactgtaaccggcgactatccggactacaacgtagtacctatccgtttgggattgcggtacaacctgatctctattctttatgtgaagttagaaggcggtactgttcagtataccggtaaaaactacagcggcgtaggcggactggtagctcccggtgttggtatccgcgtactgggtttggatgtggaagccaagtatgaagcatggtttaaagatggcaccagaagtttctttggcctgaaagccggatataatttttaaagataaaaaaagctggtagttacaactgccagcttttttttatctctttagaatatcgttgctgtccatgttctttcaaacagtccatccggcgccagccggttgatcccctctttctcttccagttccccggtcgcatttacgctgtcggcaatgccgcaccagggttcaatacaaacaaagtccgcatctttagccgcccatatgcccatgtacggaaaaccttcaaaggccagtgttaagccgtgcggtgtacggttgcttttaatgctgatggccgtggaggccaggtttttaaataccagggcatcattataaaacagggatttcttaagcggcagttcatgcgtatgctgaagatatggaacaggtgcggtttctacctgtccgccagccgacaatggccagatccctgcttcttcttctttattaaaatacaggtaataatcttcatacgttgtatccggcaccagtggcaatttaaaggccgggtgggcgcctaccgagaagaacagggttttatcatcgcggttgagcacctggtaggttacctgtaactgatcgtcctgcaggaggtactggatggtaaagtcgaaacggaaaggatatactttacgggtagtttcattatccgaaagacggagactgacgtattccgctccctgttctgacaccgtaaacaattgttccctggcaaaaccatggcggccgagcgtgtagagctctccgcggtattgataggtattctctttcaggccgccgacgatggggaataacacggggctttttttaccccagaaggcggggtcgccactccataaatattcgaggccggtatctttcctcacaatgctctgtagttctgctccctgggggttcaccagtacggtgagtttttcgttggaaatctgtatcatagtctgaagctgttataatggatccatgcgaagataggctgtaaatggaacaaagctttgtacctttgccaggtattttttaaccttacaaagcgaaggcattatggaatcattaaaaggaaaaaaagccctgatcaccggtgggggcaaaggtataggccgggcgctggcagtggcgctggcacaggaaggcgtggatatagccctgttggggcgtagtgccggttcactggaggccgtggcaaaagaaatcagtagtataggcgtaaaagcagcttacgcaactgcagatgtgagcgatctgctggcggtaaatgaggcagtggcccagctgacaaaagagctgggggaacctgatatcctgatcaacaatgccggcattgctgcttttggcaatttcatggaactggaacctgctcaatgggagcagatcatccgggtaaacctgctgggcgtgtattatgtaacccgggcggtattaccgggtatgatagaaagaaaaaccggcgacattatcaatatatcttctactgcgggacaacggggcgcaccacttaccagcgcttacagcgcctccaagttcggcctgctgggcttaacagaatcgctgatgctggaagtaaggaaacataatatccgggtaagcgccttaacgccgagcactattgcgacggatatggcaaaagacctgaacttaacggatgggaacccggacaaagtattgcagccggaagacctggcggaatttgtagtggcgcagctgacgctgaacagaagggtgctggtgaaatcagcggggttatggtctaccaatccataaacgcggggatccttgtttcagcaggcgctgttctgctgaaacaagataatccgcttatttattacaaatacgataggcgtatccgatagaggcagtagcggcgccggtattatttttaccattagcactgccttcctggatattgaggaagccatagtttccacccccttccacaaatacctggtgacggccaaaaatataggccagtcctacgtttccacttactcctagattgaaagtatgtaactggtctttgatgtctgttgttctgtcgaaagactgaggctgctgcgtaatcggctgtttcccttcttcatcgaggtaaaggatgctgctgccgctggtaacctgtttagcgctcaggaggaagccgaaaaacgggccggcatccacgtagaggcgtaacggtgaggtaggtcccaggttccagccaaatttagccaggatggggaccatcaggtagttcagttttgcctggctttcgaaattggcatacaggtaggttggcgcaggcataccgggaggcaatgcggctgccatttcaggcgggaacgggaatgcctgaagcccttcttttttaccaccctgcgaagagtaggaaatcatggcttcaatagaaaacagtttgctgacgtggtattcaccgaggataccgaaatccggcccctggcgggagctgtaaccggtgttgagtgggttgctctcactaccgccggcagtaagattcggaatactgatgcctccgcggacaccgagatcgacctgcgcctttgcctgtaaaccgaaaaatagcaagagggcaggcaggagccatttgtaagagcgatagtgtttcatagtaaatagattgtatatcgaatttaacacttatctcacattactcagccaacctgctacaaacaataatacctcacggctggtgggttcgttatgcatttcatggtacatgccctcccactcgcggtaggtaagcaaggccgatggcgccctttcagcaaataagcgggagccttccacagcggtaaattcgtcggcattaccgtggataagcagggaaggcacgcatagttcagccgcatgcaacaggcaccaggcgccgttttggatcatatcattggccagtcgcaggctcagtttatcatgccgcaggggatctgccctgaatttttctacttccgccttatcatgtgaaattttgttgatgtccagcccctgtttgatccggatattgggggcgatggcactggccactttcagtactcctttcaggaaaccgccggggcgcatgccaataatcaaagccggcgcggagatcaccgccgccagtatatcgggctgccgccggagtaaaaagccagtgagcacgccgccgcccatactatggccgtacatcaccaccggtttgtgataggtatccgccacataacgcacgaagctctgcaaataatcgaacataaaatcaaagcctttggaagcgcctttggcgccatcacttttaccgtggccataatggtcgatgccgatcactgtatatccttccttcatgaaaaaagaggctacctggtcgtagcggccaatatgctccccgatgccatgtacaatgatcataacccgcccggagttttcggggctccagatgataccgtgaaacctggtacgctgataaaaccagtgaaattcattcatagccggagatgctggtgcagaaacgaagataaagaatatctttacgccctatttcaaccagataaaattaactgaataacacacatgagcaaacaagccaccacttcgccggtatacagcattcctttaagttaccgtaagatggaaaacctgcatattgttttctggctattgaaagatatcagctggtgcatgatatggaagcccctgggcgtagcgatgatctttcccaccctgatcatttctatcgtgatcgcctggcgtacccgccagttcatgtcggagctgtgtcataatgtggcgatctctgtgtggattgcggccaactcctactggatgatcagtgaattttttcatttcgatacacaggtaattacgggcgatattacctttaaacacctggcgctgattccttttgtaaccgggattcttatactggcctatttctacctgtattatcaacccaggcataaagaagaagcagaagtaatcactgaataaggcgtgtatgcaacaaggtttgtatttccggttccaataatgatttcttttccaccgtaatatttaccaggtaataactattcccgctgcagagtgcatcccatctccattcaagctggctgttgctgtggcgggtacggctttcgtaccaccaggcagtgtataacgtagtgttctctttttgtaattcagcagtatatactttcgtgtccgctatcgttacttccgctattttataaaacccaaagccacttcctttccagcaaatcatcggctggtgatctgtaaaataaaagcccggaattccttttacatacaataatgcgttggccctggtttgtttgataacatgatcgtccaatacagcgtagctgtagccgggcaaatgttttacctgctggtccatttcgccggaagcggcctgtttttcctgcataaaaaagtgcccaccgataatgcctatggccagcacgccgtgtaacaaccagccatataacggtggcggttgcacgccggtatgcacgggctttgcctttccatagcgttgcagcatccatttaacacccggcagtaagggaaggattacatagatcagcagtgtggcaatccccatagcatcatgcgccattgcttccggcggtaaggcaaactgcaccagcagtataatgcggaacaggttagcagttatatttaacccggtaatagccagtaacaccaccaggattgcggtaaacgacaatactttctgataacggcgttgataaagggctatcagcatcacgccgcagagcagcgaggtgagcatcatctgtaaacccatacaggcggggtctacactgaacacattacttcccagcaggatcatattacctgcggtggtaacggccgggtttatgcccgccagtatattaccagccacacccgtgagccatagcctgatcgggaaagtgaatacattgaccataaaatcaattgccggcgcaatgagcgcagccgtgatgaaagtgagcgtttgtaatctccccaagaaatattctgttacaaaaaataaggcggtgataagcgtggcataccggatagttaatacagggatctgccacgacagtaacaaaaagaataatgctatccaaccgcaacgggtacttccggggcgtgaccggtcgggctgaaacaccactcccatcgctattacacacaacataaagaaagtactcttccaggaaaaataatgttgcaactgcaatacaccagttatcgtataaaccaccggcagtatcaataccggcagttttgttcttcccgttaataaccgtatatgcggtaacgttagcatacgcttcttttccgattaaataatttttcgaaccgcacataggcgagtatacctatcgctattatgaagagtgcccattcatgcggttcgggtacggccccatgccctttaagagaggcgttcttcaggctgtttacatcatcgctgatctcaaatttatcatagtcggcctgcgtttcgagtacaatcaaactcgacaatggtgttaccacgtaagcagcttttgcagtattgatcagcgctgtttctgaagacagatcctctcctgtaacttttggtcccagatccttcagaatggaattataggcaaagaggcgcgccagatggtcgggtccctgtgtttgcatactgcccgtgctgcgggcaatgcggatacgcgcatcttccatgatcagctgctggctatcctcctcttgccgcaggaagctgttgttgcgtaattgtgacagcaactgattcgtggatccattttcgtataccagtgaccgtgattctttcaacgtagccaggtaagggctcaggatgttacctatatgatataatcttattttcccgtgagataaaaaactgcgcagattactcctgaaaacggaactttccaggtcgctgagctgaggcgaaatattgtctgaactgctgatcaccagtgctgttggaggatttattattttataaaacggaaagagggagaaacgctggtcgtgcaattcgttaaaaagatccttcctgttttcttcgttcactgctatcattccgttccggggatgaaacatccatactttcttacctttcagttgggtaaggatctctcggtaattatcataattccagctatgatttacatccaggtaatagttctccggtgcaaaaaattcataagatggcttgtaaggtaacaacgtatatcgctcaccgttaaagctgaaggcagcattgtttattgcctcatcaggcattgttaactcccagtccgcattatacttcccgattttgccaaccgtcttctctttatccctataaaacccggccggataattcagtcctccgggccatttatccatattcagttttacttcataacgcgccccctcatatgccggcccttcaaaccataccggttgatacaccagtttaccctgttgtactttcagcggagaggtaatcccgatcttaaatttccgttcttcattttgcggcaccggaaatacacgcactactacgcggttgccttcctgccagtgtaccaccgacggatcacgacgttgcctgccaacgatttccgaataggcttctgcagcttttgcctgggtagtgaggatggctttttcttcatggttattgatccacaacgagagggaggtaaccactgcgccttccggcaaatgcaatgtatagatcgcctcctggctgttactccatcgctgtttcggaatatttttaaccgtgtaggtattttccgtgtatgccaggtgatactgtggccagatgtcggcggttgtgcccacactggtagttaccaggtctttcccgctccagtagcggtctactgcataatgtcttttatcaaacattacattcagcatcttcagccggtcttcttcagggatagcaatagtgccaaacagggcgcccgcggtcataaacaggggatcatgcgtcagcttttcaccgaactccctggtaggcgtactccaaagattgaaacccgaccggatacccgggctggtataaacaatacctgttttcagcagctgtgctgttataaaatcaatccgtgcttcctgcgcggcccggatccagggcggcaactcatcccttactgcaacatggctgttgttgtaggcgtgttccattttacttttgtctgctatatatattacggaatacagcaccaacgttgcgaatgccagtgcacctgaccataagtaaatgagccggtaacggtacaccggccatatgagatttctcaccatccggaagttaaaccagagcacaaaaatgggcgaaaacgtaacgatagaaagcccgatggcaatcagggcaatcatgctgacaagatacaccggtaccaggtaaacagcgaggtagaaaggcaacagcattgtaaatccaagcaccgcgcattgcaggtatttcatccattccggccatctttcaaaaaatgcaaatgccagtatattgacacaaataaaaatcagcatgaccactagccaggtggctgaagactcaaacagacggatactgtcatttactgtataggcatcagtgagcaacagcaccacgaatacagacatcactttccttctcccctcccatggtttaagaaagccgccgatccagcagctgaagaaataaagtaacgttagcaggtgtgtaatgatgaatgaagcttctgtgccttccggtaaaaagcaggaatagcacttcgcgaaaagggcaaaacataacagtgtcaggccgaacacataaggcgccggcaaggttctggaggtagtgacttccattatagatgatttgaatacgcctcaaatgtatgaaacaaaaagtactttgcgttacaaagtataaataaaagattcactagatcagaagacgcagggagaattaatccgttataccgtatgctttacggatatccagttgcagggtgttggcagcaggaagtgcatgtatgccggccttattcatcgttaatccagcgtaagacaggtattgctgatagttaacaggagcgggcgtttccacatatatgaagaagtcggccagggattggccggcaatggtttcacatgtctcccggaactcttccggtgtaaatccacgttgcagttgcaaataatattgacggtataaagtccgcatcacatcatccagcgattgctgattgtgggtagcatggcggatccgcagatccagcaggaaggcaagcaccggtcctttttcatagcaggaaatagttttggccggatcaccgccaaaaggaccatcatcccaggtttcatagctggcagcggtaacagattgtactctattgcccggacgttgctcacacgactgtatatgcccgtgcaacgcctgcagcaggttggcgcctgacattaatccagccctttgcagcaccaggtactcatagtagacagtgaacccttccgacacccacaacagtttggtacgattagcagcatcataattaaaaggtcccagttccaccgggcggatccgcttcacattataatgatgaaaatattcatgtgccaggaaactataggtacgctgacgcgctgctttatcatttaattcgtcgccggtaaaagatacggctgttgaattcaaatgctctatcccaccctggcctggtccgattcccagaaacgtgtagtggttgtagggaatatccccgatgattccggctgccgtgttgactatcttttccaggtcgtccatgaaccgggcgcggttgaagttacctggctgaaaggccgtaaaataatgaggaatcccttttactttaaaggcgggaaaagattccagctcccccatcagcagggggctgtcgtacagcacatcatagctggcggctgtataagtatgcttactgagtgtatccattcccgtagccacctgccagttgccatatggctgcacggtgagcacaacgggacttcctgttttcccttccgggtgcataaaaacacccgccggtgtaatatagccgtgatctctatcgaggtagctggtcgctacaaaattgcggtgggcgcttatcttataagtgatctttatctcagcgccgggtgtatgaacgatctcccagctgttggcgtttgttttatgccaccgcaatgtatcattagcggtgttatatacatgaaaatcttttacctgtccggcatagtccatcagttgatagtaaccgggtgtccacaccgggagcttcaccgtggtgtgggtggtgctgtctgttttatagttcatttccacttcatatacaccggcagccggatcaggcatgcgcacattgaacgctatgcgcggtgatttcaggcggataatattcaccgacaatgcgggtacgctccagttgaactgtgccgctgcatttcgaatagtagaagtatgcggtgtataggcttccggcgatgcaaatgaattctctgcatccggtttatctgccgttaatgtaatcacttgtgcaacgggactcacagaagctccctccagccggatatctgcatctacgacactttcaccggcattcacgatcttgaggatgatatcgccgttcttttcatcccggcctgcaatggaaaataatttttgcggctcgcggtaggtcatgagcagtgaattatctacaaaacatttcacttcatcattgcttacctcgaggcggatatcataccagcggccggattctaacggggctttcaggcgcaccggattactgataccggccacgtcgtatccgttggtaagactttcgaacatggcattggaattcagccaggagcctatatgtgcgcgtaagcaggtattggtatcctttactgcgaaaggaataataaaggcattgaccccgccggttttacgggctttgagcgacaacgtataggcgttaaagtggcgacctttcaagatagccagttgttgcgcaccggcagctgtttgcgccagcaggccggattgtttttcccagttgccccttaccgggagccagccggttagctgcggatcaaggcgactgttatacaccgtatctccctgttgtacgacggtgatatctttatattctgcttctgtatcccaggtagcgagaccaatacttcctgaaaatttcggtgttacattcttttccggcagcagggtggttgttaccgggtagttgaaagtggctttatgatcattgagcatgttgagcgtgtaataggagatccttgcgaagctggcgcctgcgttgaagtgaatgaggttcaccggccagtccacatcatgttcattgaccagtaaaggtgcatagctactcatctttaccaggtcggcatttttctccatgctcattacatacacggcatcgctgagggccgcctgcatgttaccgttgcccacaccggcgttggtggcatactcccctacatacatctgccagctgccacgtttgtatttatcgaagtgatcaaagttgcgcaggctccagccggcatctttataggcatgttcgtccacgatatctgtatgctgcatactatcgagggtatggcggtttacatcaccgatgcccatgctggcaataatttctatttgcgggtatttcttgtggatggcgtcataaaaaaggttataccgctttgcataatcagggccatgttgctcattccccacctctacgtacctgagcggaaacggcgccgggtggccattggcggcacgttgttttccccagcgggaagtaaccggaccaaccgcatattcaattgcatccaatgcactttgaatatagggcgctacgctatcatctggcacaaaggtgccgctgcggtattcacaggaaatgcccacattaaaaacatacaatgcggcggcgttgatatcttcacagaattgcaggtattcatgatatccgaagccattactgctccaataaccccatgggctatacgaagccgtgcgctgctccaccgggccaatcgtagttttccaattgggggcactttccacggtgatcccttccacgtaacaaccgcccggccaccgtacaaaggcaggcttcattttttggatgagcgtggcgatatccgcccgcatgccgttggggcggtcacggaaggtatgcaccgggaacagggataccatatccagcagcagggtgccgttttgatgaaaagtgagtaccagccggccggcaggatcacttcccttcgccgtaagagtagcgttatattttttccaggaagcggaactgctgatctgcaacacggtatctgccaggacttgtcctgatgcggattgcagcgaagcagttacttttcccgtatagcctttaacggtatttgcgaagaaggacaaccggtaggcggctcccttttccacgttcatgccccagaatccttcattcaccagggctgcacctctcccggttatcttcacctgcatcgcatgcggcgttgcggcatttagcggatgatccgttaccagcgacagctgtgcattgctttccgcatgccaggccggccaccggctttgcagcggccattccattttccagtccgatacctggccatgcagcataaaatgcggcttttgcgggaaaggcaccagccagccattttccagctttgtgccggcgggaatgcggtgatcttcaaagccgcggttttgcaccatttcagcatatagtcctccttccccggcatgactgatctcttcaaagaaaacgccgtgcagggtagccgggatagcggcgcccttttccgtggcatttacagtgattgcagccctgttctgggcaatggcggagctacttcctgcaagcaggcagataacggccagaaagccttgtttcatgcgattcatatattactcaacgatccattcgtgtattccggtggcattatctgccggtaattgtatttccagttttaacgcggtagtagttaccggctcaaaagtgatcacattatacttatccttttccaccgtgtagggcgttttggcatttaccggtttccattcggctccctgcttgtaatacagcttccaggcagcaggtaccctgcatccaccaaaaggaccgtcgtcgtaccaatacactttggaactgcttacggtatgagtgctgtcgaacgtatactgcacccattccgtagtgcctttggcgggccaccaatgcaggtaaagagcgctgttatccttggaatcttttggctcgtactgatcgttcagggccatatacatgcgctgattttttacagacgctgttaccttacttttggaagcaatggtgggtgcaggttttggacgggcagccgaagcttcaaacggaatccatacggtcatttcagcaggaccgcggttagcccaggaaaaatagggtatagccgttaccgtttgactgctgttaatcagcgaatccgaatgcagttgccggctggcggaattgccaggcatttggagggtcattaccccactgagcagatccgggcgatacacgggagaaaccaatgtctgtttatccactacaatattctgtacggtagcatctttattatccggtccttccaggcaatacataatagggccgcgttccagtgcaaagcgggagtggtcgtcctttactgcatcggcagccaggatctttcttacttccatcgggaactctagtgtcaccttatctcctttcttccaggagcggctgatcaccgcataacctttttctgtcttgtagtcgatagggctgccattgagcaggatggggatttttacggctgaactgtcgtcttcaaaatacaggttgcctggtaccggcctgttttccgcccagcccggaatacgcacccggagcgagaatgtggtaggtttggcagtattgatagtgatgtcatcttttccattccagggataatccgtttgctgtacgatatttactttaccggctttcaattgaatagtagcggagtcgcccacaaaaagatttacgtacaggtcattgtctttctgcgcatacacataccccggcatagaaggcaggaagcgggtcatattggaaatgcagcaggcgcatccaaaccaggcgcttcgctgatgctgtcccatagaggccagcgggttgggataaaagaaacggtcgccgctgatggataccccggagagcaaaccgttgtacagtgtacgttccagcacatcaatatattttgcatcgccgtgcaggaggaacatacggctgttccagtatacgttggcaatggcggcacaggtttccgcgtaagccgacatgttcggcaattcatatgcagcaccaaaggcctctcctgcgccggtggcgccaataccgccggtgatatacagtttccggtccaccacatcatcccagatatcatcaatggcttccaggtatttgcgatcacctgttaaggcggctacatcggccataccggtgtacatataggtagcacgtacggcatgtcctactgcttcgtgctgatctgttactttcttgttcgattgactgtattcctggctgtatttgctacctggtccgcgaacgtccaggaaaaattttgccaggtcgagatacgacttattgccggttacccggtacaggcgggtgagccctgtttccacgatctggtggcctgggaatttttcctccttcccccagccgaagtcacgtaccagcaggtcggcattgcggatcgcaatattaagcagcgtttttttaccggtagcctggtaatgtgctaccgccgcctcaaacaggtgacctgaattatataattcatggctcaggtcctcttccttctcccatctcctgctgccaatccattcatgtggttttgccgctttcaccgtgcggaaggtatagagatatccatctttctcctgggcggcgccgataatactgatcagtgtatccaggtacttttccagaccgggattaggctgcatctgcaacccgtaggaagcgccttctattactttatacagatcggtatcatcaaaggtgtattcggtgagcttatccccagggattttacctgccgcgcgtaaaaagttatcgatgcgacctgtctttttacattgctccagcgtatacggaatcgttacactggcgttggttcttattttcggcgcccagaaattgtcattcacccttacctgcgtaaaggccaccggtttaatcggataatctttctgcaactgcgcctgcacgatagtgttggccatcagcataccggcgccggccagcgccgcctttccccaaaatgatctcataccttttgtctttatagtcttcgaatataatgttttataactgtctaaataacaattatttgtcataccgcagatgctgatccagcacgggattttactgatttttctcctggcaataagaaaatagatagttattcataacatgaatggattcacggtcggcaaaatatatccaccaaatataattgtcataatgacatttaaaagtattgataaaaaaagaggaatactgcgtagatattaacgagtattcccaacattttgtcaatccctgaaatcctgtctgtcacgaagtttcctgcaatcgattactacctccgccaggataactatgctatcaatttaccgattattagtcgctgcagcgaagcagcactaccccatgcgggggtatatctgcggtgtaggcaacgggaatagctcccaggttccgctgggtccatacattccttacctgtggccgtgcaggcataccgatatctttccacggcacggtgacgcggcggtattgccggtctttattaaaaatacctatcgccttactcccatcagccagcggtttcacccatacttcatagtgcgcagtggctatacgtcgccccgcagccatacccagcgtgtcctggtcgatagccagcacttcatcattggtaagcaggttaagcgtaaaagtatctatcctgctgatatcgcacccgataagcaacggtgcggccagcaagctccataaactaacatgcgtatattgctcgtccggtgtaagccgggtgggatgcaggttttcaccccagcccacctgccctacgatcatcatgtccggatcgttccagttaccaggacgggcatacttttcaagtggatactgtccgaagccgatgccagccatgctttcccaggtatcatcaatatcttctgtcgtgcgccaggtttgtgcatccacctgggaaccccatttccacacttccctcagtccgtactggcacaggttatacacaatatcacgcggatacttccggatggcccgccgcatcacacggaacgggtgaatgaacgtttccaggctggtatcggcgggcatcacctggtcgtaactgcaccagtcgtatttaaggtagtcaattccccagccggcataggtggcggcgtccttctcctcattccggtaagagcccaggaatccgccacaggtaagcggaccaggagaagaatacattccaaatttcaatcccctgttatgcagccaatcgcccagccctttcatatcgggaaactttccgttaggaaggatgctgctgtcggcagcacgccggggttgctgccagccgtcatcaacattgatataattccagccgtgatcggccaggcccttgtccagcagcgcctgggcagagctttttactttttcctcactcacgctgagtccccagcaattccagctgttccatcccattggaggcgttaatgcaataacaccgcctgccttgagcagcagcgattgtgtagcaactcccaatgcattactcacagtaacaactatacgataattgccagcctcttttaccacgccggtaatcacgccatggacgctgtcgatcattaacccttccggcagccccgatgcacggaaatgaagcggtgctgttccggtggccgccactttgaaaatgacgggcgcacccggactaacaccgtacaccggggcactgttaatccgcggttcaggcgcaggcgccggggtctggagataaggcacgtccagttctccttttagctgatgcccggtagccgtttctgtgaagcaataacgtaaacggatacccgctctgtgaggcgcctccatgataaacgcgctttttgagccgggtgtaagtgtcatggcctccacatggctcgcaatcttttttccggccgctatatcaaatatatcgctgcggagtgtaccctttaccgtagtattgaacacattcgtcaatttcactggcagcgatgttttcttatcacggaacacaatctggtcttccggcagcgttagccggataccatcaattttccggagcagatccacgtaaggtatgcccataaagatccctcctgtaccaccgccatcaaacactcttacagctatcacgttttccgcgtcccagcggatagcgctgtctgaagccggaatatgatactcccggatgtatggccacttgctgacataaccacccacgtcgtgcgggaagctaccggtttgccctacccgcacgccattcagccaggtttcatctacatcatttacatgcgcaagataaatcctcaatgaatctttccaggcagcctgctgcttcaggctgcggggaatcatcaccttcatacggtaccagccatatccgtgatagtccgggaatccctgcgactgccacacttcaccggtttttatccgcttccagtgccggtcgttgtagcctggtgcagcccactgcagggagtcgcctgttgcaaacgccgctcctttcaacatcagggcatcaggatgctgggctatagctggcaaagcaaaacagatcattaatactataaaccatccatgtttcttacacccggtcattgtgtctttctttagttacttataacttcgtcacgttaggcattcttatcgtcacttcatagctgccttcaaatagtatctggaaaccaaaccgtggattggctgcccaggctttggcagcggcgccatccatcttaataaaccacgccgggatgcggtaatagatcaggtaatttacataacccgggatcagcttggacggataaggagcgatggcatagtctgtgatcagtgcagtatctgttacaatcaccgggttaaacctcgcataggaagcaaaagagggacgatcaccacgggtaatcacttctccgttcttcggattaaacagtttgccgttcttatccatgatcttcaacatcactttggtaccggtagcggatacacgttttaattccatcgttcctttcatctcacccgggaaagtattggtaacagagtcgaaaccggggatcaccggtacttccgtcatacggatatactccggatcttcaatatgcagccgggccagattctggtataccctgctcccgtttacattcgttgccttcacatcaaactcatacaccccattgggaataaaggcggaaggcgatttaaacaggaatccgccgtttaccgggttaaactcaaaaggcaactcctgcaaactgtcctgttttgcgcgtaaaagagcaatggtggtatcggtatccgggtcaaaagacattttatctttaaatacccataccgggtacctggtgttaaatgccgccggcaatttgccaccgcccaccggccgtatatccagcatttcaaattttaccggtggtgtagatccatcaaataaaataccgggatagcgggcggtaatccctttcggaataaatatctccggacttttgtaacggataccatcgctcagaaaaccttcttccactttgctacatgccgtattcatcaatacaaatgcgatgatggcgaataagatatatttcatagtcatcttattttagttttccctgtaaatataaaatcccatgttggcgttggcctctaacacatgcaccatacccgtagcagtacgcacttcagaagtttgcacatacgcgtaaaaatcaggttccgtgttctcggtaccatccggtacgtcttcatctgccagtccgaatacccgccgtatctgtatcctgttggtggttgaccggataccgcttacatcgatataatacttctccagcagcaggaaataattaccttcactattgatgttggtaaagctcttctttgtatagctcatggcttttttatcaagtacgcctttgaatatatgccgccgcaggaagaacttaatactgtctgtcgtcaaactatccaatgtgaatttgatgttctcattattatacttcctttggatagcgcgtgtttgctgcgccaggaaactggtcacacccaaattagtgggcgaaaagaaggtgatgtcgccgttgatctcgtctttcatacctgcgcggtcaatcagcattaccacggtatccagcactttactttccttcaggaaatcgtaggtcgacatcttcctgatcctctccacgtcagtattaccttcattaacgaggtagttatcttttttacatgctgccaggatcagcagtgatccgagtaacagatgaatgatcttcatgatgaataatttggataaaaattaaattttacctgcccagtatttattctgtaccagcaacctgttgttattgaacaacgcgggatccagcggcagcaggaagccttcctggttgtacctggagggcgtaagccagggaaccatcgaccgcttcattctcacatcatcaaaatacagctggccttccataaacaactcgcgtgagcgctccgttatgatttcatccagcaggctgttgtaactcagcggcgactcgctcacatacatcgcagagtccatctgcggcaggttgcgcgagcggcggaaactccgcagctgcgaataggcttctcccagttgtcctttatacacggcaatttccatgcggttcagtagcacatctgcataacggatcagggaaacattgttatccaggtaaggttccgcctgttgattaggattgttatagataatgttactgtattttgtaaagatgggttgggcgccgtctgcatcatatagaaacaagcttctgcgtatatccgtattaggtagtgtatcctccggattaggtcccgtttgaataatgcggggatacaggttaccaacgaagctgttgcccagcagcaggtcgctccagtctgcttttgccaggacgggaatccttaaaaacttcatgggcatcaggttgttggaaccttcgttataagcataccgtgtatataattcaaagatactttcgcgggtgttaccggtaaatgcctttgcatactggatgctgtctatcttcccgttgggagccggtaagccgtataacccactgccaataatagtttccaccagtgcggaagctttggctacatcggccatatcgggagtggcctcaaacaccggctttttgatcacgcaggcgcgccacaggtatacctgggattgcagcgccatcaccgcagctttattaggcactgtgcccctgttggactccacttcatatgccatatccaggcagttggcggccgaatccaggtcattcagtatttgctgcaccaccaggttcttgtctgtacgtgccagtggtttgttggcaataggatcaggatccggtgttaacaccagtggtacatcgccaaaggtgcggagcagttgaaaataaacataggagcggataaaaagggtttgtccggcgatgtttttccggcctttttccggatcatcgaggaaggtatcgtccggtatcagtggcagtttttccagtatcaggtttgtttgaagaatagtgctgtaaaacctcgaccagttccggaaaacatccaggtagttcatttcaaatttacccacctgtatgttccagtcggagttggaaaaatagggtccgctcctgatgatgataaactgatcacccagcgtcatgtcgcccaggttatgaaagtaatcctgctcaagcatattggcgcgcagcgaagcgtatgcacctgccaatgccttcttcatatcattttccgacttccagaatttctcctcgtaagtagtatccttgggctcctggttcagcattttcttacaccccgataaaaatgctgccactataatgatgataataaaagtccgtttcataaaaagtgtttagctgtttttaaaatcctacatcaatgcccagtgtatatttatgcgggctcggatagccgacaccgttatactcgccgtaagggttcacattttctgcatccggtaatcttttggaagcctggaacatatacacattgtccatcaggccgtaaaaccgcaggcggttcaaatgcagcggcttcagggctttttctttgagggtatagccaaatgatacatttttgatcctgaaataatcacctttctccaggaagaaagtttgatcggcacgatagtaatagcggtaagtaccgatatccattcttgcatactgggccttatcaccgggcttacgccagatattcatggaagaaagatctgacaccgcatatttggagaactcgttaccggaaccatcccagccgtagcggccataggtatccgactcatacaggttcagcacatctctcttaaacgtgaaagtgcaaaggaacccgaaggtgaaattcttccagtaaaaattttgcgtaataccaccagtgagaaaaggattgggattgccatacggaattttatctcctgtgatacctccgttaaaggcatcgataataccatcgccatccaggtccgcaaaaataaattctccggctctgaaaggattattggcagcaggatcattcacggctcccacctggaatttcttaccggtatatttgtctgtgggcacatcatcatcggtagcgtatacgcccagtgttttcagcaggtagaaagtattcactgcttttccgcgggtgagaatatgcgtggtattaaacaaattgccaaaggtaagatcacggttattgttaggcatacttaccaccaggttttgattcatacttacattccacatgatttcccaacgcaatgcactcttctccggcatcacattcctgaactggaaattgatatcaataccggaattgcgtaattgtgcaccgttggttttggcggtggcaataccggtagtactttgcaggttcatatcaatgagtcccgctttgctattcttcacatatacatcggcactgaaataatatttgccattcatcagttctgcctctatcccaccgttccagctggcggttttttcccagctgatatctttctgcgctacaccaccagaaccgaattgcggggtaatagttaccgcgccgttgtatgtattggggctcaatccgctgccattatacccggcggcgcctacgttataaagactatactgcaaataataatcgccaggcaggttacccagcacaccataactaccgcgcagtttcagcatggacaaccagctggaatagcgccgcataaaaggttcattactaatcatccagcctgctgagatagcgggaaaatacccccatttattatccggtccgaagctggaagcagcatccccacgcagggatgcggaaaagagataggtacttttataatcatagttcacccttgaaaacagggagagaataccaaaggccgcgtaggacgaactgccgtacagataaggtccctgcgggaaaccattcactacctggatttggtcactggcgccgcgatcgccgcgcgcataggtattttgataagtgctgtactgtacttcctgccctacaatggcgttaatggtgtgttcttttccttttccaaatacagcgttccagttcaggtcattggaggtggtataactttgctgcaacccgctgctagaggaagcagagttgccaaggtctgaattcaattcacccggcaccgacacatcgcggcggctcattaccatcgacactgagttacgcgagcggaacgacaactggctggataaccgtaactgcacagagatatcgccatttacctggttatccgtgttgatatccatattactggaatagcgtcctaatacgcgctgcaagctgttttcatccggtgcaaacagggaggagggcatgctttgtcctactgctccaaaaagatctgcactgccggaaccgcgtcctctttccatgcgggccagccggatattgggtactacttccagcgcaccgtttttggtacgtatagaagaggagtagttaagcgtatagcgtttaaatcccgaggctttcacaatgccatcttccatgtacataccagccgacaggcgataagtattgtactccgttcccccgtatacgttaaagtccacgttccgcacaaatccgttgcggtaaaacaagcgttgccagtcggtcgacttattcagatccgggttcaggctgtctgtcatgatgagatttttatgcgtcagcctgtcgtagttattttcaaacgcatcatcatacaggcggatcttttcgcggcgttctgccgcgcccaccaatatctggcggagtttagggatctgcgttaaaccgccataggccgacacgctgaagcgcggcgcaccggtacgggcacgttttgttttgataatgattacgccgttggcgccacgggagccatacacagccgcggcagccgcatctttcagcacatcaaccgattctatttcgttggggttcaaaccggcgatattgttggtaccggtaccaatgtccggtcccaccatatcatcgttgaactgcggtacgtcatcaattacatacagtggcttgtttaatattttatactgattgctttggtaagaagtaccgatagcggtattacccctcacggagatggtgggtgccgcgccgggttccccggtgaagttctgcacatttacgccggccatgcgtccctgcagcagttgttcaaaactaccggcaggaatgttttcaatgtcttttcctttgatgctggaaacggcagcagtagctttacgccggttcaccgtctggtagccgatcaccactacatctcccagtgcgccgctctgagcggtgagcactacgctgagatgtgtgcggccttttaatttctgttcctgtttaagatagccgataaaactgaactctaaagtagcatcaggtggcgctgccagggaaaattcccccttgtcgtccgtaactaccccctgggagttccccttaattttgaccgaggcgccgggcagtggcccacttctttcatctgtaattttgccgctgacttttacgttctgggcaacagatggtaagaccgccaataaggcgataaaggccatgacaattttttgcatgggattaggtttaagcagtgttgaaaaattctggttgatatacgatgttacaggtccgcacacagtgcgtagactagatataagattttattccggttgatttattttaattgtattgttgacaattgttattacaaatctatctaaaaggaccggatattacttcccggaaattaactgataggttgctgattttaactggtaaggagggaaaaggggaacatctctcaacggagacgttccccgcaggattataatttgtaaaaacgccagctggaggtaaaatcctttggcacaggcttattcaacaggatggcccggagcatttcaacaggcatcatattctcccggagcaccgcgtcatgatattgtttgaacgacatcttaccactgtctaccagttctttcttcagcgcttcaaactgcaatccgccaatcatataggcgatctggtacagcgggctgtaaccgccaacaaaagaacggcgtacttctccttctgcgtttgcccgctcgtggcctacgcggtctaccaggaaatcaatacattgctgcggcgtccacttaccggtgtgatagttaatagagaagataatgcgcgcgcaacggtgcttacgccagaacaacataccaacgcggtcttccggcgactttgcaaatccctggtcccatagcaaccgttcccagtacagggcccatccttcgatccagaaaggcgtttcaaaatggcggtatgttttatagcggttctgcataaactcctggagggcgtgtcctgccaacagttcatggtgaacggtggcgcgggaaaagtgcgggttgttaccacgcatactcatcattttgtcttcctggctcatgctgctaacgggataggatacactaaactcttctccaccggtgaagaacgggttcaccagctgccgctccggcgtcatcatgatcatgcgccaggtttcttccgcgagcggtggcagggtgatcaggtcgtgttgctttataaaatccacggattcattgtaaagcttcaccatctcagcaggttgatctgccgggggcacgtaactgttctttactttctccatggctgctttccagtctgttcccaatcccatttctcgggtggctttttccatttccgcatcgcaccaggcaaactctttattggcaatggccagcagttcctctggtgtataaggaatcatttcctcctgtaatcctttgatcagcgcggctcttccgatagggtgaccggcaataccactgccatcatcaggcatacgggcggtacttttttctttattggagaaagtagtgctgtatgttttcaggaggctgtctacctgtttatagggagcgggtacccaccaggaaaacagcggatcataaccgttataaaaattaaaagcatttcccagtgcttcccgtaagcctctcagggtagagatgccgcggcggatctgcggcagcgtgagcgagctgtcgccttccagctgctgcctttttttgatgatctccctggctgtttcgctcagctgggcggccagtgccgctgcatcgggtttctccccccggcggcgatgctgctctacctggtaaattttatcggcaaagggaaaccatttttttacctgtgcgctttcctgttgtgcaagtaacagttcctccattgtttgtgaaagccggcgtttaaacagggtgtaatctacctgggcgcctacattaagccccgcatagttcagttgctccagccgttgctggtagctttttaccagggtggtcatgcgggtgaacccttccggcgagctgtctacaaagtaaaaccggcgcaggttaccggcatccgcatcatattgcaccatgatgttattcacttcgctggtctggagatacaggtcattatctgcagattgagcggaggctgttgcctgctgcagcagcacgcaggcgaggagcatgtataatttcttcaaaagaggcatattttactcgtttatatttctgtcaggcggattaatattcaacaggctttttacaaagaaatcgcggcgtttaattcgtccgtaggggcctccgtcgctgtgccccataccgggtaccggcaggaattcgaaggtctttccttttttaatcaatgcgttgatcacgcggtaagtagattccggcggcacgtttgtgtcggcctctcccactatcaacagcaggctcccctgcaatttcccggcattggttacgttggattgttcttcatattctttgcctacagggtatcccatccattgttcattccaccattgcttatccacccggttatcatgacagccacaggaagccactgctgccttataaaattcgggatgaaagagcagcccgcccagtgcgttttgtccgccggcggaagttccgtatagccctacccgtgaggtatccacaaagggatacttttgggccagtgccttgatccatagaatgcggtccgggaaacctgcatcaaccaggttcttccagcatacatcgtggaatgcctttgatcggttggcggtgcccatgccatcgatctgcactacaataaatccaagatcagccaggctttgcatatcgatataataactcataaaactcttgggtacaaacgcatcctgcggacctgcatagatattttccactaccgggtacattttcgtggagtcgtaatctgttggccggcacattaccccccagatatctgttttgccatcgcggcccttcgccgtaaaaggtacggggaaaggcacgccggtagcttcccagccgctcacgtctgttttttccaacacggtgatcagtttcccgtcggacgtgcggcgcagttcatttaccggtggcacgtttacctgtgagtatttatctataaaatattttttatcgggagaaaagattgcctggtggttacccgtggccggagtgaggtccagcagatgctgaccggcgaagtctgttcggtagtaatggaggaagtaaggatcttccccggcattcctgccccctgccctgaaccagatctctcttttctttgcatctacgctgtctatatcccggactacccaatcaccttttgttacctggtttttaatttcgccggtgagggtattcaccaggtaaatatgccgccagccgtctttttcggacgtccagaggagttcattggtttccggcaggtaatgggtataaaggcgcgattcgtagatgaaggagggtgttttttcatccagtatggtgcgggtattgccgttggtggcgtctacttctatcacgcggaagcgctgatggccgcggtctactttttcataaaggaagtagcgcgggtctttatgccgccagtgcagttccggtgcttcaaaaaaatcgatctgttctgtttttactttagcagtggtttttccggccagggtaaacaggtacatatcgaaggtggtaaacggatcgcccggttgcttatagggttgcgagcgcagttgtccgcgggtggtaccgggtacgtcggtgagtatgtagtacacggaggaatcttccacggggtgaatgcggtaaccgaccaggtatttgctgtcgggcgaccaggccagggcgccatagtagtcgccggaggcttttccgtctgttgtaaacggtgtaagggcgccggtggctaccgagcgtacatacacgttaccatctatcgtggtggcgacccattgtttatccggggatacgctatctgttgcaaaactctcccagcgactgggttcatgtcgcctcaccggacgggtagcggggtagtctttagccagttgcgcaatttttgcggtgtcggtgatcacctcttttttaccggtggcagccgtcacaagataacctgttttactgctgtctttccctgtaaccacataccagaacgacttcccgtcgggcagccagttggcctccacgttgtgccggaagatggttttccgggtaatactgtccagcagctgtacttttttatatcgctgcaatatctctgcatgtgaaggcaggtaaggtgttggcttgttttgctgtgcgagcaacagcccggttggcaggctccataaaatcaccaggtaaagaaatcgttggtatttcataagttgtgttgatccgctataattaaatgtatactggacagttaatatttactccctgtccgattattttttaaaagtacatcaggcattgattagattttaaacgttttttaataacttgttctcatatcttcacctaaatttggttgcaatctcttcaaaggtgttaaaaaaagaataatgtaagtgcatgaaagtattacagtttacgatacctgtggcgcatgataaaaccattatcacacaaaaggactggctgccggctttttacccgcatctccatcgtcatgaggaaatccagcttacgtggatccagcatgggcatggtactttgatagtagaaaataatatgcatgccttctggtcgaatgaaatatactggataggcagtaaccagccgcatgtattaaagagcgaagaattgccttttggcagcaagaataaaaagaatgtgcaggccctaacccttttcttcaacccggaaggcaagctgggacccttgtttggcttgccggagtttaaaaagataaagtcttttatagatcagtcgcaaaacgggtttaaggtaccggaggcccatgtagtggaaatatccagccggttgctgaaaatccaccagtcgcagggcattgcacagttcctggcatttgtggagctgatcaatttcttccttactattaaggacctggagccactgatcaccgggtcaaggttatctgctgtaaatgaacaggaaggaatccggatcgggtacatctacaattatatcatgcagcattatgatgcggaaataaagctggaagatattgcccgggaggcgcatatgacgccgcaggctttttgccggtatttcaaaaaacatacgcgattaacgtttgtatcattcctgaatgaagtacgcatcaatgaggcctgcaaaaagctggcaggcgggtcgtatgatagtattgccaccgttgcctacaactgtggtttcaacagcatagcgaattttaaccgggtatttaagagtattacccgcaaatcgccccgcagttacctgcgggaatatgagcagctggaaaacccgccaccgggcactgcaacaaaatctgcatagtattgatcaaaaagcgaatagaattgccagcaaagtaactgtagttttaggggagataaacctgtaatatcaaccaaactacgattcgctactatgtcagacgctcctacctttaagccgtccatcaagttgctggatgctactatgattgtagccggcagcatgatcggctccggaatttttattgtcagtgcagatattacccgtcataccgggagcgccggatggctgttgctggtatggctgatcaccggttttatgacccttacggctgcattgagctacggagaactgagtggtatgtttcctcgggcaggcggccagtacatctacctgaaagaagcctataatcctatgacagccttcctgtatggctggagtttttttaccgtgatacaaacggctaccattgccgcagtgggcgtagccttcgccaaatttaccgcctacctcttgccggctttcagtgaagaaaacgtgttattgtcggcaggaacgctgcatatcactgctgcgcagctgctttccatcggggtaattgtgttactgacctatatgaatacacggggtattgaaggaggtaaaattattcagacaacttttacacttaccaaactggtaagcctcgctgcgctgatcatattcggactgctggcgattaaacccgaaatatggcaggccaactggcagcatgcgtggaacctgcatcccctgacaacaggtggcagtatatcgtcatacagtaccattgccgcttttggcgctattgcttccgccatggtaggatcggtgttcagcagtgactcctggcataatgtagcttttgttggcggggaaataaaaaatccccggaggaatatcgggttaagtctttttttaggaaccgcgatcgtcaccatcatttatgtgctaaccaatattacctatctcgccgtattgcctttgtcagaaattgcaaatgcaccaaaagatcgtgtagccgtttccgtatcacaggcggtgctgggaaatacaggcacagtacttattgcagtaatgatcatgatatccacttttggttgtaacaacgggcttatacttgcaggtgcgcgggtgtaccataccatggccaaagatggtttgttttttaaaaaagcaggagatttaaaccgttctgccgtgccttcctttgcattgtggatacaatgcctcgtggcatgcttatggtgtctcagcggccgttatggcgacttattggatatgatctcttttgtggtggtggccttttatatgcttaccatagcaggcatctttatcctgcggaagaagcgcccggatgccgaccggccttacaaagcgtttggatacccggtgttgccggtgctgtatattttaatgggtattgctttctgcggattgctgtttgtttataagccacgatttacctggccgggactatttataacgctgtccggtatacccgtgtattattttgccaacaggaacaacatccgcgataacgcatctatcaaaaaagaaaatataaccaccgctgattcttcttactaaattatctgtcaaccagggggactatcaaaaaatagtccccctctttttttgtgccttcccctataagcgtatcccctacgccttttcgaagtattaatatataattaatccagtattataaccaggcaaaaaactatacatgtacatttacaaaattcgttacctttctgacagaaactgatgcgatgttatgtagacatgtaattccttttctgagtaagcattacgacgtgccatattgatcatgtgaaagaccaactttttttcatctcttttggggatccagtgaattatataaaaaactgcctccagcgggcaaatgtgcaataacgatttagcaacttttattttataacaaccaaaaaactaagcgacaacacgagagacaggccgtatatctgttccattcacgtttctattcaagttcacgtcttattcattaattatgaggtactcattcactggaaaattatgctttctgatggtctttctatgcgctgccaccagcgcagtatttgctcaaaagacccttaccggaaaagttaccggcgcggcagacggtgcaggtctgcctggtgtaaacgtaatcataaccggcaccgccagcggcgccagtactgatgcaaaagggaactacaccctttctttaccgccgggtgctaaatcggttttgttctcgtttatcggctacgaaccacaaacggttaccatcggtgaacaaaccgttatcaacgtatcactggccgcagccaccaaaggattaggtgaagtagtggtagtgggttacggtgtgcaaagccgccgcgacgttaccggtaccatcgcttccgttaaaggagccgacatcaaaaaccttcctgtatcagacgccgcgcaagccatccagggccgcgtaacaggcgtggatattgtacggtcggatgcagcccccggcagcacgcctgccatccgtatccgcggtacaggcaccatcaataatgccgacccattgattattatagatggcgtaccggcaggtggactcgcagatgtaaaccctaacgacatcgcctccatggaaatacttaaagatgcgtcttcctccgcaatatatggtacccgtgccgccaacggcgtggtgatcattaccaccaaaagaggaaactatggagaaaaactgaaagcatcggtcaacttctatcgcggcgttaccaataccatccgctatatcccgctgctcaccgcacccgacctggtaaaactgaaacaggaacgctataccaacgatggcgtggcaatagagcccatctggcaggatccttactacgccactcaacgcaccgactggcaaaaagcattgttcggctccggtgatattaccaatgcagatgtaagcctgcgcggcggcaacaacacctccaattatatgctcagtgccggttattataatgaaaatggtatcatcaccaattcctatttcaaaagatactcggtgcgcattaactcagaacacaagctgggtaagcgtttgaaagtaggtgaaaatctgcagctcacctataaacaaaacagcggcccggatacctactcttcccagacaggccttattttcagcgccctgcgctttaaccccgccatccccgttcacaaccccgatggcagctggggcacctccaaagccagcaatgaactcggtgatatcaacaaccccgtatacaccgcggaaaccaccgacacctggaccaaaaactatcgcatgctggccagcgtatacgctgaactggaaatcatggatggcctcaccctgcgcgccaactatggctttgacggcagcctgatgaaccagttcaacttcgcgcctaaagtactggatcaaaccagggcacgcgatcatgcagaacttttcaatcgcagcgaaagctataacaaccagctgagcgaaattttccttacctacaataaagtgctggcaaacgtacatcacctcaccgttaccggtggctactcccagcaaacctataacggctcctggaaccaggcggaaagatggggctttaacgatgaatcgaaagaccagctggtactgagtaacgggaacgatattcacgatgcaaaaggcaattattttaatgccaacgctatcgcatccgggtttatcaggggcttctatggcttcaaggataaatacctggtcaccgttaccttccgtgcagatggctcgtcgaagttctcaccggatcaacgctggggctacttccccgctttctccgcaggctggcgtatttcagatgaaaccttctttaaagacaacgtaaaggccgtgagcaacctgaaaatcacaggcggctggggacagctcggtaatcaaaacgtaacggagtttcaatacctcgcacagatcgataaagaccgccgctataacttcggcgaaacagcctacaccggcgtatggaactcaaggctcgccaaccccgatatcacctgggaaaaggccgaaatgaccaacatcagcctggaagccggcttcttccacgataaactcaataccaccatcacctggttcaacaaaaacaccaaagacatgctggtacccgctcctgaaatggacctccacggcacttccgccatccccgaccgtaacctcggtcagctgagcaacaaaggctgggaagtggaagtaggctaccagggcggcaacgacaagttccattacaatgtaagcgccaacgcttcttttattaaaaatgaagtaaccaaactatacgacccttcttcctatatcggttccactccctatggccggcagggacaggaaatttcccgcacctatgtaggtcagccactggcctcttattatggctggaaaacaggtggaatctaccagaccgctgatgagatcaacaacgatcccaacatcaacaaagatcccaacaaagccaatatcaaaccgggtgatgtgcgtttcctcgataccaacggtgacaatatcgtaaatgataaagaccgtgtaaacctgggcagccccaatcctaaaatggtatacggcatccaggccagcgccggttacaaagggtttgacctgagcctttcctttgcgggtgtgagtggcgtaaaactttacaacgccgataaaatgcagggcatggatcccaactatccatataacctgtatgcagatgcgctgaaccgctggcatggcgccggcaccagcaattccgtaccaaggatgaccctgggcaatgccaatcagaataaccgcacctccgaccgctttgtggaaaacggcgattacttctccctgaaaaacgcatcgctgggatataccattccttccaaagtatggggccgcagcggcatttcagatatccatgtatacgtggccgcgcaaaacctgtttatcctcaccaactactccggtttaactccgcagctgggttataactacggtaccggcgatggtaacaggcagagaggagtagacgtagccgcctatccgcaggccaggacctttacttttggcgctaccctcaacttttaattcacggcaaccttaaattaactactatgcaacggatcaaatatatattagtactcacggcattactctttgccggctgtaaaagcgtactcgatgtatctcccaaaggagtgtacagcaccggcaactactggcgcaaccaaagcgatgcccttgacggggtaaccggtatctataatgttttactggaagaagattataccggctttaatgagtttgtattcgataactgctcagacgaccaggtacgcggcggcgaccatgattatgacgccgtgatagaagacttcacctacgatgcttccacctacagcgtacgggtaggatggagatggaaatatgaaacgattaaccgctccaacaacgtgctgatctatgttcctaaaattacagacattgatccggacatcaagaaccgttgtctcggtgaagcacacttcttccgcgcattcgcctactggcgcctgctgctgatctatggcgaagcccctatcatcacagaagatgatgtgctcaaatctttctataacaaaccaaaagtaacggccgatgaactgcgggcccagatagaaagcgatctcctggccgccgccgaccagcttcctgaaacctacgacgacgccaataaaggccgcgtaagcaaaggtaccgcctggggactgttatgtaaactgtatatgaactggtcgaaactggacaaagccatcgaatacggcagcaaagtagttagtaatactaactataaactggcaacaaactatgccgataacttcagtgtagccaccggcaacaattcagaaatgctgctcgccgttcaaacagtagacggaaacggctactccgatttcatcacctatcatgctccacgcaactggaacggatggagcttcttctaccctaccaaaggactggtagatgaatttgaagcaggcgatccccgcaagaatatctgcatcatgcaacccggtgataaagtaaatatcggtaccggtattgccacttatgaagcatcagcttcctggagcggttatcattataaaaaattctgtagctggaaaccttccggcggactcgactactccctcaaaacaccgttgatgcgcgccgcggatatttacctgctggtggcagaagcaaagatccgtttaaacggcccgggcgccggcgactcggagctcaatgccgttcgcaagcgcgcttccgccagtttaccggccgttaccaatgccggcatggcagcactgatgcatgaacgcagggtggaactatgcggggaaaatgaacgccaccaggacctcctgcgctgggataaagccaacctcatagacattgtggcgttgtacaagaaaccaaagctggcgtatgatggtaccgtgattacacgagggggagccccacgtattttcacgaagcctaaaaactacttcttcccgatgccgcaacaggaaatcgacagaagcaaaggcacactggtgcagaatccgaattattagtgcgaagggccgccttcggcggcttttaaattgtcttggagcaggattacgctgattttgctgattataaggatttgatcttttggatttttataagattaaggaagacagaagcgaatatttaaaagacttcggggagatataagcggatatactcgcttaaatctccccgaaatcatttataaatccaaaagttcaaatccctataatcagcaaaatcagtgtaatcctgctccaagacaatttaaaaaccgccgaaggcggtcctccccttacttcaccgaaaacttatacaccgttgtttgtgaaaacgtttcacccggtttcaggattacgttcgggaaagaaggttgattaggagaatcggggaagtgttgtgtttccaggcaaagcgccgcgttctgcacatacttctgcccgttacgtgtattcgtgagcgtgccatccaggaagttgccggtatagaactgaataccgggttgggtggtagctacttccatataacggccgctggttgggtcgtacagggtggcaatggtttccagcaccccttcctgtttgtccagtacccagttatgatcatatccgccttttactttgccgatatcagcaccgatctttttggcagtggtaaaatccattggggtaccttttaccgggtccagtttgccggtaggaatcagcttatcatttaccggggtataacggcttgccttcagcgacaactcgtgtccgaggatggtgctgtcttttcccgcagaaagattaaagtaagcgtggttggtaaggtttaccggggtcgctttatcggtggttgccttgtaggtgatctgcagggcgttgtccggtgtaagcgtgtataccaccgtagcctggaggttaccgggatatccttcttctccgtctttgctgttatataccagttgcaggctgctgtcgccggcaggcgtggctgcccatactaccttatcaaatcctttcagtccgccgtgaagcgtgttgccgttattattagcggcgagtttgtattccttgccatccagtgtaaacttagcattggcaatacggttggcataacggcctaccagtgcgccgaaatagggctggcctttttgctggtagcctgaaagtgagtcgtaagacaataccacattgcctttctgtccttgtttgtcggcagtaatgatatctgtgatagtaccgccgtaattcaggatctttacttccattccgtttgcattctgcagggtatactgcaaaacttcctggccatctgcctggccaaagctttgtgggccagctgttacagccgttgctgtggaatccttactttcttccgtcttcgcagcattgttgttgcaggaagccagcatggtgccaccggagatcacgagggcggttagcgccttaaagttcatgtccataacgtattttgatgttaagtgaaaaagagtcactaaatatcgggataatccggctaaagtcaaatatttttatttaaaatttattgtcacaagaacaattaaaacgcgattgattaaaatacgtgtactttctgtcaataattggaaagtaagtatacaccgggcgaactagctttagcctgttaaattctgatgaaatgaaaagactgctccttacgggattgttgctggccggcagcgttccgctgtactatagcgcctgtgcccaatcttatgtaccagggtggaaagaaagcaagatgaaagtgttgcctacagccactataaaagcatacccgttcccgataacggacgtcaccctcctggacggcccctttaaaacggctatgcaggcggatgcgcgataccttttaaaaatagatcccgatcgcctgctgtcggctttccgcaccaatgcgggattgcccgcaaaagggaagcaatatggcggctgggaaaccggcgggctggcaggccacaccatgggtcattacttgtcggcctgcgccatgcaatacgccgccaccaaagataccgcctatcttaaccgggtggcctacctggtaagcgagctggcactgtgccagcaaaaccgccgcaatggctatatcggggccttccccaacgataataagctctggtctgaagtcgctgccggcgatatccgctccaggggcttcgatcttaacggtggctggtcgccctggtacaccgtacacaaaattatggcagggttactggatgcatggctctactgtaataacgcggaagcattgaaggtaaacaaaggtatcgccgactggaccggtgacgtcatcaaaaacctgtcggaagaacagatgcagaaaatgctgatctgcgaatacggcgggatggcggaaacactggtgaatacctacgccctgagcggcgataaaaaatacctggacctctcctatcgcttttatgataaacgtatccttgattcactggctatcgggaaagatatattaccaggcaagcactccaatacccagatccctaaagccattgccagcatccgcaggtatgagctgaacaaagatcccaaagatgccgccattgccaggtatttctgggaagtggtaaccagggatcactcctatgccaatggcggtaacagcaactatgagtacttcggaccagcaagacagctcaatgaatcgctcacagacaataccaccgaaacatgtaacacctataacatgctcaagctcaccaggcacttgtttgcattggagccacaggcgcgtttcatggactactacgaaaaagcattatacaatcatatcctggcatcgcagcatcacgaaaccggtatgatgtgctacttcattcccctccgcatgggcggccacaaagaatacagcgatgagtttgaaacctttacctgctgcgtaggctccggaatggagaatcatgtgaaatacggtgaaagcatttattaccgcggcgccgatggcagcctgtttgtgaacttgtttattccttccgtacttgaatggaaagacaaaggtattacagtaaagcaggaaaataacctcccggcaaataatcgtataaccctcaccgttagcactaagaaaacaacgtcatttacccttcgcatccgtaaaccggcatgggcgcgaccaggtattacactgaaagtaaatggtacggagcaatccctgcaaacagatgaaagcggatacttcgtggttacccggagctggaaaaacagcgaccaggtaacgcttaccctgccagccgatgtgtatacagaggcgcttcccgacaatcctaacaggcaggcattgttttatggcccggtgttattatccggtatactcggggagaaagaacccgatccggtaagcggcgttccggtactggtagcgcctaacgggcaacccagcacctggatcaatcgtagcaacgaccccggcacactggtgttccgcactgccggcaccgcaaagccaatggacgttacacttacgcccttttaccaaacccgtaatgagtattacaccgtatactgggatgtgtttacgccgcaaagctggcaggaacagcaggggaaatatgcagcggctaaaaaagcgcagcaggagctggatgcgcgtactaccgacattcttcgcccgggtgaaatgcaaccggaacgtgatcatgaattcaccggcgagaaaaccagcaccgaagaagaacatggacgcaaatggcgcattgcctggcccggaggatatttctcctttaatatgaaagtagatcccaactcccgtcattcgctgcaatgtacttattggggcatggataaccggggccgtacatttgatatcatcgtagacggcactactattgccactgaagatatcaacaaattcaaggagagcaggttctatcctatctcttatcccatccctgaacatcttacaaaaggaaagcaaagcgtgaatatccgtttcgtaccaaaagccaataacagcgcaggcccactgtatggctgcagaatggtgaaagaataaaagaacaggcgttagcggagtggatccgctaacgctgttttactaccggccacccgttttcccattgcaatagctccactctcaatgttggttttcccccgtcgccggcatcataaccatgaaaaacgagataatcatttccattaaatgccactacggcattatgcccaacgccatgccagcgggcatctcccgctaatagcagcgagccgccgccatcggtcattcgccggttttctttatcagtataaggtcccagtaattgtgcagatctgcccaccatcattttgtaggtactcttttcgccgcggcaacaataatcgaacgacacaaatagataatagtaatgcgctttcttataaataaaaggcgcttctatagccgcattgccaggtaaagcatctgctatcccttcatcgcggtgacgcgcggccaacgtgtaccacacctgtggcacagccgggcgtgtagccgtactatccagtttaaacattttgatgccaccccagaaagagccgaaactcagccatgccgtacccaggctgtccgtaataaaattgggatcaatggcattccagttatccctgccgggaacagattgtatcaccatgcctttatcaatccattgaaaaccgggcgattgcggatccagtgttttgttaaccgccacaccaatggcggaagtatttttcccaaacgcggaaactgcataatacaaataataccatccgttgtagtaactgatatccggcgcccatgtatgccctttaaagcctggcacagcagcctttgtccaggctggtggcgcagtaaatactggtggttgccggttccagtttttcatatcgggagatgaatacaccgtaatcccgtttcccgtacaaaacaaataccaggtactatcctggcggatcattaccggatcatgaacaaactgcgcctggctatgccatgcgtaaaaaagtagtatccaaattaatccccgtttcatgatcattctttttataacaaaaaaaaggcggcagaaaaaactttcctgccgccgtatatacttgccagatggctatttatttatcttcgcgcggatcacgtaaaaggaccagggtgcaatatccgtacggatcgtttttcctttgatgtttatatctttttcttccggggagatgccggtgggacggtccagcgaattaagaccctgaagatcattgctacgaagcgtagttaacttcccgttggcagcaatgctttttacaccctgcactgccactgctaccggcttaacggtagcggacgtgttcaccagtttgatgaccaattcacccgtggcgtcatctactaccgtggatgcatatacgctatcctgtccgctgattacctggttacctttcagcatgggtaccactgcagtgcctttgttattggcatacagtttttgcacatagtagttaggggtaccataggaacgcaggttatcaaaccagataaggtcgggcgtccactgccatccatccacatgtgccagcagcggcgcataggaagccattaccactacgtcggtgttgcgttccagtccggtcatgaaggcggcttctgccaatgccgactgccagttgtttttattatcaccgttgcctactcctttgctgtgtgcagcatattcaccggcaaagatcttaggccctttacggtcgtaggaatcatagcgtgctgcgttgctgaggaaccattcgggagagctgtaatagtgctcgtcgaggatatctgcattcagtttacgcagcgtgtcgttgaggaaagtaaatctatcgccgtcagggcccgggccaagactgtttatcagcttgatatccgggtatttacttttgatggcttttgaaaaaatagcgtaacgttctacgtattgcggtccccactgctcattgcctacgcccatcattttcaggttaaacggcgccgggtgccccatttttgcgcgcagcgcgccccatttggaagttacgtcgccattggcaaattcaatcaggtccagtgcgtcctggatgtaagggtccagttcattcacggctaccacttctccgctgttaaactgacaggccatgccgcagttgaggatcggtaaaggcgacgcgcctatgtcttccgacaactgaaaatattcaaagaagccaagtccgaacgactggaagtaatccggtgtggcgcgatgtggaaattcgttgttccagcggttgatgatcagttcacggtcattcacatcgcctactgttttcttccactggtagcggtttaccagctcgcgtccttccacgatgcagccgccggggaaccggagaaagccgggatgcaggtcggccagcaattgtacgagatcggtacgaagcccgttgctccgctccttccaggtatgttgcgggaacagggagatcatgtcaacatctatcaccccattgccgctgaaagttactttcagtttgcctttggacgcggtggcagcagcggtgaaactggctttatactgctgccagctgctgccggcaggtgatacagtggtgctgcctatttctttacccgcatcatcgagtaaggtaacggtgagctttaccgcagcgccttcctgttgccgggcatacaaagagaaattgtattgttccccactcttaatacccatgccgcggaaaccttcgttcactatttcaaaactacgtgtagccggcattgttatcctggcaaagcgtggattggatgggtggtcttcctgccggttaacgaccactatctgcccactagctaccgcgttccttgggacgctccagcccataagcggcgtgctgaactcaaaggaccggttctttaccagctccgcataaataccgccatcagcgctgaggttaatgtcctcaaagaagataccccacatattgggcgataccggcgtttttatttcgccggcctttacggtaaaattcaacggttgctgggctgccaacggcgtggtataaacgcccatgagcagtgataatgccgtaataatacgttgtggtttcatataattattccagttttttcttgccccggattgttcaaacccggtgagcactaataatttatccactttaccttttcgtttataccccgtcgttatgttgcagcatgtgcggatcgggaacaaagttcaggaaggcgtggaaattggcgttatactttttccggtcgatcctgtaataaaaggcgcccttcttggagcttagcttgtctttgtccgcgagctttaccagcagtttggtagaaaggatcttgcggctgaaattacctttatcgaaagagatgttataaacagattcgtacaggtgttgtagttgcgggatggtgaatttagccggcagcagttcaagcagcagcgggtgcaatgcagccttataacgtagcttctcctttgccaggtctaccatcgctttatgatcgaagatgaggtccggatggtggttaataggaaaccataccgcgtgaaaatcctcattcagctgctgtttgtatttctgaatatcgatcagtgcggtgtaagccaccgatacagtgcgttctaccgtatcacgggaaggggaactgaaggtatggagctgctccatataaatgccatccagtccgctgagattttttaacaccctgctggcggcatcttcagcgctttcgtgctcctgtataaaaccgcctaccaggctccattgccccttacagggctcaaaacccctttgtatcagcagcagtttcatttcctggccatcgaagccaaaaatgatacaatcaacggcgaataataaccgggtctgctgcgaatatcttttcataacaataaattaggcggtaaaagtacaacgcggattttgtctttctcaggattacgctgattttactgattttctttttttgattttttctgatttacttttattctggtaagatttatctaaaaaaatcatataaatcaaaaagaataaaatcaaactaatcagtaaaatcagcgtaatcctgagaaagacaacattcgcttaccagaagcggatgtacagcgcggataataacaacaatgttattacgatcagcacagtggttgccggggtaattttgaacatagccttatcaagtacaaaggctttcggatttacttttggtcctgcaaagctgataacgatcatcacgatcatggtaaacataaaagccagtcccatacagatgaggaaaggaatttcgtaaccgcctttaccattcggataggctgtatagaaaattgtttcatgtccaagtacggcaggtgcaaactggttaaagaacacacacagcgtaaacccggtgataatccctgctacggcagcggcgccggtagtgcgtttccagaacatacccaacaggaacatggcaaatacgcccggactgataaagccggtatatttctggataaaggtaaatccgccctcaccgccaatacccagcaaatcgttccaggtaaagaggatgcccagcaacatggcagctactacggtgatgcgaccagtccataccagttttgcttcagaggcatccttcttaatatatttacggtatatatccagggtaaaaatagtagagatactgttggccttacccgccagggaagctacaatagcagcagttaatgccgctatggataagcctttcaacccggaaggcaaaaagccgaggatcgctgcgtaagcgccatctttactagccaggccagggaggtgtccgtttttctgcagcacatatgccgcaatacccggcaacatgacgatgatgggcatcatgatcttcagtaagcccgcgaagaggataccgttacgggcagtttgcagattggctcccagtgcgcgttgcgtgatatactggttgcaaccccagtagttgaggttcacgatccactgaccggcggcatacatcaggatccccggaagcaccaggtacttgttgatatagtcctgcgaagagttggcatccggttttgccaggatcatatgaaagtggtccggcgcatccttcatgagggcattgaaaccagccagggcgttgtgtcccaggccaaacttttcactcaccagcgtgagggccatataagtggtggccagtccgccgataatcaataccgccacctggatcacatctgtataaccgattaccttcataccgccgagcgtgataatgatggcaaatatggagagcgcaatcatcactacatgcaggtattcgcctcccagcaggccattgatggccagtgcgccgaggtatagaatagaggtgaggttaacgaacacatagagaaataaccagaagatagccatgatcaacgctaccgtttcattataccgcgttttcaggaactgcggcatggtataaattttattcttcaggtagatgggaataaaccagacggcaatgatgataagggctattgcggctacccattcataggccgctacagcgatacctacaaaataaccatcaccgctcatgccgataaactgctctgcagaaatatttgatgcaatcagggatgccccgattgcccaccaggtaagggttccttccgcgaggaagaagtcttttgtattcgtttcggttttcttttttcgtttgtatatccagtaaccgtatacggaaacaataatgaaataagtaatgaagacgagtatatcgccggtggaaaggatgttttgcataacgggcagtttattagcttttgctttaagaagttggcaaattataaagcagccggcggtggcgcttaagcgccttccgccggcaggtggaattatttataggatacatcgttccagcgcagttcatttttgaactcgcgcaggtcggtgttcttccctatcaatgccagttcaatacccgccatttctgcaaagtcctgcatatgtacggaagtaaggttttggctgtaacaggtatgatgtgcgccaccagccagtatccaggcggtgcagcctttcttcatatcaggataaggtttccataacacgcgggctaccggcagcttcggcagatcctgtggcggttctaccgcttctacctcatttacgagcaggcggaaacggttgcccatgtctaccagtgaagcgttgatcgctggtcccgccgcggaattgaataccagtcttaccgggtctgccttccctcctatgcccagcggatgcttctcacaggatggttttccgctggcgatggattcacagatctccagcatatgggaaccgagcaccattgggttagacggatcaaaatgataggtataatcctccatgaaagagttaccaccttttaaaccgctgcccattactttcatggcccgcaccaatgcagctgttttccagtcgccttccccggcaaacccgtaaccggctttcatcaggcgttgcaccgcaatgcccggcagttgtatcatgccatgcaggtcttcaaaggtatcggagaatcctttgaagttcccgtcttccaggaatgctttcagtccgagttctatgcgagcggcgtctttcagcgcagggtcctgcagcagtgctgcagatatcgtatatgcatccccgtattcctttaccagggaggccactgctccatcggaaatgccattgatcacacttacgagatcaccaatgccatgcgtgttgcaggagaagcccagtttggattctgcttctactttatcgccatcggttaccgccacgaagcgcatgttgtcgccgaagcgaacaaagcgtgctccctgccagtcgtgccaaccggcggctacccttgcccaggcgcccagttcctccagtacttccggatcctgccagtggccggtgatcaccttgcggctcatccgcatgcggctcatcataaatccgaactcccggtcgccatgagcgctctggttcaggttcatgaagtccatatctatttcactccaggggatatcacggttgaattgagtatgcaggtggcagataggtttggataatgctttcaggccacggatccacattttagccggggagaaagtatgcatccaggtgattaccccgatacagttgggagcagcattggcttccatacatacggcgtaaatttcgtccggtgtttttacagtgggtttgtaaaccaccgtaacgggtatgcgtgtatccttgtgcagggaggcggcaatttcctggctgtgtgcggctacctgtttcaatgtttcttctccgtacaggtgctgactgccggttacaaaccagatttcgaaattcttcagattaatcatgttgcttggtttattgcccgtaataggaattggggccgtgtttacgttcaaaatgtttccggatcagcgcatctttcagtcgtggtgcattcccgttaatcgactccgtgagatacgccatttgtgccactgattccagtacggcgctgttgtaaactgctttggcgggagttttgccccaggtgaagggcgcatggtttcctaccaggatcatttcaatatcttcgtagctaagtcctcgttccgtcagtgcattcatgatctggaagccggtctggtattcatagtcaccggcaatcatttcatcagacatgggcggggcgcagggaatatccacggtgttgtggtcggcgtgcgtagtgccataaatgggaatatcgcgctgactctgcgcccatgcagtagcataagtggagtgggtatgcacgataccgccaatgtgttcccagtgcttatataataccgcgtgggtgagggtatcggaagaagggcgcaattgcccgtctactgttttaccatcgaagtccactatcaccattttttcgggagatagttccgggtagggaacaccactgggtttgatggcaaacacgcccagctgccggtctgctgcacttacattcccgaaggtgaagaggaccagtcccaatgcgggcagttgcatattggcttcgtatgctgcctgccggatatgttgatactgttgcatacaaaattagtcaatggtgatggcggcagtaaatgcgcctaatgctttatacttctggtacctgttttcgtatatgccagcgcgttggctatccgggtgataggtaacttcaaatccctgtcccattgcttccatcgcatcttccaccctgttaaacaatcctgctgctgtggcggcaaacatggcggcgccgagggcgcaggtttgttcggagcggtgaatacggatcggcatattcatcacatcggccatcatctgcatgatgaacgccgactttttggctacgccgccaatgcctatcaatccttttacaggaacgccttccctttcaaatctttctacaatggctttggcgccaaagcaggtcgattccgctacggtgcggaaaatacgcggtgcgtctgtagcgaggttcaggccggtaagggtacctttgagcgactgatccgcgtctggtgtacggcggccgttaagccagtcgatacccaattcactgtgttcttccggcgggatctgtgctgcctgttttgccagttcaacgatcatcctggcggaagtttcctgcgccagtttagcggcagtttctgcatcaatcagggaagacgacggcaggaggtgctgtaacggccatgccagtacgttactgaaccaggcgtacgcatcaccaaaggccgattgccctgcttccatgcccatcataccggggattacagaacccggtacctgcccgcagataccttttaccagtgtatgtttcatttcgtccataggcgccaccagcatatcgcaggtggaggtgcccattaccttgctgaggtggtagggctctatttgtccgcctaccgcacccatgtgcgcatcaaacgcaccgatgcctattactacgctggtaggaagccccagccgctctgcccattcggggcaaagatgacctgcggcttcgccggaggtgtatgtttttgtaaagagccgttgtgtgaatccctgcagtaacgggtcaatggcggagaagaatgcatccggcggaaggccgccgaattctgctgcaaacagcgctttatgtcctgcgctgcaaacgccgcgtttcagctggctgacatgtttcccaccggaaagcaggaatggtatccagtcgcaatgttccacccaggagtaagtggcgtttctaacggcttcgtctgcacgaagaatgtgcagcagttttgcccagaaccattccgatgaataaatgccgcccacaaagcggaggtaattttcttcaaatgtagcggcagtggcgttgatcgccgctgcttccttcagggcggtatgatccttccataacacaaacatggcgtttgggttatcctggaaggccggtgtaagcgcgagcggcgtaccggtttcatcaacggctaccggcgtggaaccggtggtatctaccgatatagctttaatattagcggcagctccggggccggcctgttgcaggcattgccggatggtagtttccagcccctccacataatccaacgggtgctggcggaaccggctctgggctgcattgcagtacaggccgtctttccagcgcgggtaataaaatactgccgaggcgatttcattcccgttatgcacatctacgatgatagaacgtaccgaatcggtaccgtagtctacccctattacccaggatgaattcatattgaacgttatattgacacttataaaaaaaggtaaaaaattacgaatgacggcgggtagaaatgataccggctggattccagttcagccaatatcccaccgcgccgttatccgttactttaactccaacactactactgagaaaggaggcagctttacgctgacagtattatttttcagcgaggcgcctttaaagtctaccggtttaatattatccggctttgtaaaactgttatagtcctgcaattttgcggaggccagcagtcggccgctgatagatttataagcctggctgcgggtatccagcgttacttcctgcgttttatgggcatcaatatttacgagggaaatatgcgtgatgccatttttatctttggaagcagaagcagacactgcaggcagtttctcgttattgaacgtatagtcgttggagtgaatatccaccggaattaaagtagcatcctggtggatgttatacatctccattacatagtaagtgggtgtaagtaccatcttatctcctttggtaaggataacggattgcagtacattgatggcctgtgccaggttggccatgcgcacgcggtcggagtggttattaaagatgttcagggtggcgccggcaatcatggcatcgcgcatggtgttctgctggaagaggaagccaggattcgttcccccttctacgttataccatccgccccattcgtctaccagcagcgctatctttttcttcggatcatatttatccatgatcgcggtatgtttgctgatcagcgtatccatcagcagggctgatttcatggtagcgaaatactgtttctctgtgaaatcaaccgcatctcctttattgttccaatccacggaagagtaatgatgaagggcaacaccatcgagtaaacccgcggggatgtttttcatgagcacttctgtccagttgtaatcgccatcactggcgccggatgcaatacggaagagaggcgcgtttttccagtcgctttgcatgaaggtggcaaacttgcggtaaaggtcggcgtagtattccggccgcatattaccgccgcaaccccaggcttcattacctactccccagtaacgtaccttccagggctctttacggccgttttgctgacgaaggtcagacatgggacttttacctgcgaagttggtatactgtacccaatcagacagctcctgtgcggtaccgctgcccacgttgccggacaggtaaggttctgcacctagttcctcgcacatgttgaggaagtcgtgcgtaccaaaactgttatcttccgttacgtttccccaccaggtatttacgatagtgggccgtttatctttcggacctatcccgtctttccaatggtaggtatctgcgaagcagccacccggccagcgtagattgggaattttcattttacgcaatgcggcaatcacatctttacgtaccccgttggtattggggatgtgggaactgtctcccacataaaacccgccgtagatacaatttcccaggtgctctgcgaaatgaccatagatattgcggttgatagtttgagttggcgcatccggacgaaaggtaactgtattttgtgcctgcgttgcttgcgtggaaagcaaaaggcccaggataccagtacggatataacgatattgttttttcataacgaggttttaaaaatcaggaccggcagcactgttttgctgcgacaattcaaaagaacaaaataattgtcacatttacaattaaaacagtaaaaaaaacatttaaaggcagcaggaggccattctatggcttatttccagtaaatatttttttcaggaaagatagaaatcatcaggatagtgcggatttaccacgggcatggcagcgaaatgggtggtttttgccggctgttatattcgggctattaatttaccgcagcagcttttcaattcacagcggaatttcgatatttgcgtaaaatactgtacaaaccattcttatgccattcaccaacctggaacagttgtccctttgtttgttattatttgcgggctgtgtgcctgctccatctcccgaaaaaaaggtaacggcagatactgttgccctgccaacagaacaacatatgataatgccggcggattccctgccggtggacattgaagaagacagtacggttgcacccgccggtgcggtgacacgtacacctgcagccaccaacaaggtacccaggagaatttagccggaagaattacctttgcttaattttttaactatgaggcattttatactggcgagtacctccacgttgtttggggaaaattacctggcttatctgcaaccggcgataaaagcgttgtatgcaggtgtagaagaaattgtgtttattccgtttgcccgtccgggtggcatttcccacgacgattacaccagcagggcggcggcggcctttgaagaacccggtatccgcgtgcgcgggctccacacctttgaggatcccgctgcagccatcaaaaatgcgaagggtttctttaccgggggcggcaacaccttcctgctggtgaagcaattacatgaacagggaatgatgcaggtactccgcgatgcagtgaacaacggcgctccttacctgggatgcagcgccggcagcaacatcgggggcgtaaccatgcaaaataccaacgacatgcccattgtgtacccacccagttttgaaacaatgggactgatccctttcaaccttaacccgcactacctggacccactgcccggctcccagcatatgggcgaaacccgggaaacacgcatcaaagaatatcatacccaaaataccacgccggtactggggctgagggaaggcagctggatctacgcccatggcgatactttaacccttaaaggcacgctgagcgccaggatctttgaagctggcaaagatccttatgaactgcccgcaggcagctctctcgtccatctgaaataaaaatcaggatgaccctttaaaagaacaaccattcttttatctttgcctcatgcgtgcaaaagacgaaaataaagagtggatcatccgggaaagagccatagaaatgattgttcatgaaggctttgatggcctgagcatgcataaacttgccagggcagccaggatttcggtatctaccatctatatctatttccgcaaccgcgaggacctgctgaaccagttatatacggcagtagtggccacttttgtacagcatagcatgaggggatttgacccggatatgaactttgaatcgggtttatggctgcaatggaaaaacaggtatgaatttgtactacgcaacccgctgcattaccatttctcagaacagttccgtaactccccgctaatcaaaagacaggatgacgcaccggaaattgttttcaaaaacgccatgcggcggtttgtagctaatgcgacagagagaggcgaaatagtggaccttccgccggaagtgttctgggccattgcctacggcccattctatacccttgttaaattccatctcgataactccacgatgtccggcgttccctttttcctgagtgatgaactgctgcagctaacctttcagcggaccatgagggcactgcgggtgtaaggaaattataagctcaagccaccatcgcaacgtatcaccgttcccgttatattaccattacgcatcaggaaaagaatcgtatccgctacctctccgggttctcctaccctgccaacgggcagctgtgacgcatactgctgaaaggtatccgctttggtatctgccggcaggaagtcccaccaggcggtatttaccacgcctggtgaaacagcgtttatgcgtaagggttgtatttctttcgctatagaaggaatcatcagctccagggcgccattgatagccgccagtccggatacgcccggcgccttgctgactgccgaaatagcggtgatcaatgtaatgctgccgcctttattcacataaggcaacgccgcctgcagggtattcagctgcggccagaatttgccttcgaagccatcccgcaggtcttgcagcgacagctctgcaaacgcacctgcacctttggccccactcagcgcaattaccaggtgatcaaaatttccttgtgtccggaaaaattcatccagctcatcccggttgttgctgtccagcgccacggcctggataccggggttctcttctgccgccgctgcaagcttggctgctgaacggcccgtaactgttacattcgctttttctttgaccagcattgcagcagtagctaaacctatacctgaagagccaccggcaataattacttttttactttcaaatgtacctgacatattgttgctgttttatacccacaaagttgagatataaaacactggtccttgttaccggaatcatgcatcgtattaaccggatcatgcatttttacggaatgccagcggcgtttgcccggtctgctcccggaagaagcggttaaatcccgcgggatcactgaaattaagctggtaagagatttcggccaccgatgtatcagtataccgtaataccgcctttgcttcctgtaccagcatatctgcaatagcatctgaggccgtgcggcccgttacatcttttacggtacggttaagatgattaggcgttacgcctagcaaagcggcataatctgctacccttttttttgaaagaaaatgctggctgaccagtttcttaaaccggggcaccaggtaagtagttcgtgtatccgtagccgttaaatggagctgctgtgctacataacttctttttacttccagcagtaataaataaagatacatacggatggccttcccgcatcccggccggtgatgctgcagctcttcattgatcttagcacaaaaatccgctacggctgtgatctccgtttccgctaattgtataaagggcacgcctgcataatcgaagaacggaaactcctccgaaaccttatctgccgggataatttcctgcagaaaatctgcattaaacaaaatataatagccgaaagtatctgcgctgatattgcttttactaaacacctgtcccggaaaagtaaagctcaaagtaccggggcggtgtttaaattgttccagtcccagctgtacatccacgctgcccctgagcgtaatactgatccggtagaaatctgattttaaaggtccaaccgccggccgcaatccttcactggaatagatttccaggccggcaatctttttctccggcgccaggttactatagccaaagctggaagtatctgcctcctcccggtgaaggtgacggaaatcgtttaatacgtattgcggtatttccggtttgttgagcttggttttcattgccatttgcctatattcgttctttaaaagtagataaatattaccaatggagttaaccaccctttatcgccctgtaggaccagatgaacttgttttgattgagcaatccggctggaaacggttcccacccaggagaccggatcaacctattttttacccggtcatgaatgaagcgtatgccatccagatatcagtggaatggaatgttccggcatatggatccggcttcgttaccaaattttctttgagcagcgatttcctgaaaagatataacgttgaaaatgtaggcggggaaatacataacgagttatgggtaccggcggaagagttggaggagtttaatgataatattgtgggaacgattgaggtgacgcagcggtattataaggacacacaatgaaagtcaacgtttacctcgccccatttgtgaaaccgcaaatattttttgaaaaagaaaacttcatcccctcaactctccaacttttttgtcatcgctttaataaatccggccttatcctttttcacttctttcaactgcgctttcctgtcttccggtatagcataatacttttccgcccatagatttatttcaatcattacgggcagcaaatcaattcctttacgggttaacctgtacaaccctttgactttactatccgggtgcgccaatttttcaatgatcttattctcctccagcgccaccagcctggcggctaaaatattagtcgcaatcccttctgccgattttaaaaagtcgccgtaagagcactcttttgcaatcaataaatccctgacaatcaacagcgaccacttatccccccatacatccagggaacaactcaccgggcaatccgaccttttttttgctttagccataaaaatattttaaaaaacacttgcattttgcaagtaaatactatctttacacttgcaaaatgcaagtaaaggtacaaaacaacctaaaatgaaacaaacaattttagcgacagggtttaatcccgcaagcttcacgaaaatggtatacactaaaaaattaagctcatgatcatagcaggaaaaacggtattgataaccggcggcgcgtctggcatcggcctggaagcagccaggcaattcctggccaatggcgcaaaggtcattattaccggcagaaaccaggagaaactggacattgcccaaaaaacacatccggcgctgattaccatcaacagcgacgtggccaatgctggtgacgcagctgcgctattcagccggataaaagatcttggcggtatagatatactgtacaataatgcaggtgttggcgtgccgccattaaatctggggcttaccaatgatcagcactgggaaggagcagcctacgaaatgaatgtgaactacgtgggagtaatccggttgaacaatctgttcatggatatgttgaagtcaagaaaggaagcagccattatcaacaccacctccatacttagttatgtaccatcattgatcgaagctacttactccgcttctaaaacggctttggctttttacacccgatcgctcagggaacatctgcgcattttaaacagccgggtgaaggtatttgaactgctgccaccactggtagcaacagaaatgactgcggcccggaacgataagaaaatgaccacagaagaactggtaaaaggactgatagccggactcaaaaagaaccaatatactatccgcgtgggtgatacaaaattgatctatatactcaaccggcttttcccgaaaatagcttttggcttaattaattctaaaaagacgtatcagtctctaacagcatagcacaaacttcgcacatgaaagcatttattataaatcgctacggcaggaaagaaaatttgcagctgcgtgaaatcgcggagcccatcataaaggaacatgaagtattggtgcaggtacatgctgccagtgtaaacttattggattcaaaaatcaagaatggtgagttcaaactcattctcccctacaaaatgccccttactttgggacacgatgtagcaggtgtgatcacaaaaaccggcgctaaagtgagccgcttcaaggtaggcgatgaagtgtacgcccgaccggcagatcatcatattggtactttcgcggagatgattgccatcaatgaagccgatgtatcgctcaaaccccaaaaactaaccatggaagaagcggcatctgtccccctggtggcgctaacagcctggcaggcgcttgttgagaaagccggcttgaaaaaaggacaaaaagttttcatccaggcgggctccggtggcgtaggcaccattgccattcaattggccaaacacctcggcgctactgtagccactacaaccggcacctcaaatgttgaatgggtaaaagcgcttggcgcagatgtggtgattgattataaaaaggaagattttgaaaccatcctgcaggattatgacgtagtactgaacagccaggatgcaaaaacactcgaaaaatctctcagggtgctaaagccgggcggaaagctcatctccatatccggcccccccgaccctgcttttgcaaaagaattccgattgggctggccgctgaaaatagtcatggggctgctcagctttggcgtacgcggcaaagccaaacgccggcacgtcaattattcttttctttttatgcgggcggaaggtaaccagttaggcaagatcgctgcacttattgacgcaggtgttattagccctgttatcgacaaggtatttccatttgagaaaacagcagaagccctggcctatgttgaaagcgggcgcgcaaaaggcaaggttgtcatcaaggttaaataaaattacacttataatgttagcggcaatcgggttgctatcctcatgaatttatccagttcgtcccgaccattgtttttgtaacccgctactgttatatttgagcgaatgttagccaatgcaaaaaggtaacaacatctctgatgtacattggaataccagcttctaacccatgtaaatgattcaattatgataaccgcccaaatgttacgcgatcttgaacaggatccggcagtgaaaaaaaattacgcagcagcaggcagctggggacagcataaaatagtattccttcccgtggtggtgctgatttttagtgcatttgcgctttattttttctacgacctttctaaaaccgataacagttattccacctatacaatggtttgtggtgcgctggtattactttccatcgtagccattgccctcatacaaaaaagtgcaaagcaacaggtgataaataatattgcttccgtaccggtatgcgtagcaaagaaaatatatggcaacgattccaacggcatttactattgcatttatactacgggcaacaaacgccatgaccttgcatttattgatgcaattgcccataaaatatttaatatcgatcaggaaccggaggcggcatcatataagcgggaaatagaccgcctgttcagcgtgcaatttgcaaataccaattccgcagcggtaccgctgccaaccggctttacggaaggggaacaggtatatcagaaacagtttgccacggctcctattgcggcggtaacaacggcgaatgacggcaaatttgccgtgctggcttttaacggaacaagtgtgccggtattgaaagaagcgctttaattgaaaaaaattgcctggaaacaaagagaagctgtctcataattaattgagacagcttctttgttttagccaaaagatggcctaataatcattatgatgatcaggtgttttttaagagaataaatagttaatgtcagcttgctttagcaagct

SEQ ID NO: 13 - DNA, 245230 bp, Chitinophaga pinensis
  source 1..245230: mol_type = genomic DNA
tcgagaatatatagaatattataataacgatagaatcaaattaaaactaaatggcttgagtccaatacaatatcgaactcaagccgcctaatcaaaaaagtctaaactttggggagcagtacatattcgcttttatctccctttattattacatctaaaaatcagaaaaaaatccaaagtaaaaatcagcgtaatcagcgagaaacacaaaatccgcttctatctcccctgatcctttataaaatcccaaaaatccaaaaaagtaaaaatccagctaatcagtataatcagcgtaatcctgagccaagacaatttccgcttcgccgaaggcaaaagcggcccgcaaaaaaaatcgctgcatttattttgatttccggaatatacccttatctttatagtgtactagttaagtagtacactaaaccacaagatatgattaacatccaatccctgacattcagctaccggaaaaacaaacccctgtttgaaaacttacagctacggctggaagcaggacatatttatggtttgcttggaaaaaacggtgcgggcaaatccacgctcctcaaacaaatggccggcttactattccccgacagcggcacctgtgaggtgatgggctatccatctgccaaaagacaacccgccttcctccgggagatattcctggtgccggaagaattctatctcccaaaagtaagtgtgaaaagatatgtaaatacctacgcccctttttatcccaacttcgacgaggccgcgttttacaactatctcaaggaatttgaaattccaaaagaccagcagctgacggaaatgtcgtacggacaaaagaaaaaagtactgatcagttttgccctggccgccaacaccaaagccctgatcatggacgaacccaccaatggcctggatatcccctccaaaagccagttccgtaaagtgattgccgccgcagtgagcgacgaaaaatgcattgtgatttccacccaccaggtacgcgacctggataatctcatcgatagcatcgtgatcattgatgaccacaaaattattttccgggaagatgtacaaacagtgacagacaaattgagcttcaaaaccgtgagcaggatcgaggaaacaaccggtgtcctcttcgccgacagcaacctgcgcggacataccatcattacccgcaacgcaggccaggaacaaagtaaaatagatatggaactgctgttcaacgcgatcctcaccaatcataaacctatccaggaaatattcaactgatccacacatgcaaccaaacaacgtatttaatgttcgtcgtatgcagttatacctgcaaaaacactttaccgatcattaccgcttctacggaatgggcatgcttgccgtattcgggctgatgacaggtatcgcgcttttaacgatactggtggcccgcgaacctttccgccaaacgagcgacattgtaggcttttattacgccggcatgttcttttgcggattgctgttcaccagcagggcttttaatgaactgggcagcaaggaaaagggcgtagacttcctgatgttacctgcttcgcagtttgaaaagttcatcacattgttcctggttaccggcataggctacctgttgttttatcatatcagctgttacctcagctttaaaattattgaaagcgtacaactggcggcatttggcaggggaatagttaacaactatgcgttcctggatgatcccaaagaaaaagtatatatctattacggctatattattctgcacgcggcatttttactcggcgccacctacttccataagtacagctttatcaaaacagtgttatcgatttttgtattaggatttgcattgtggcttattaactgtgttatcgttaccctgattttcggattcgggcacgacttctggaaaagatcggtaccattcctgctggtctcgagcctggaaggcgggcccacctcatggcacactacacaatacctgatcccagaatggctgcaaaacacttacctgtttataataaaatttgtgatagcccctgtactctggaccattgcttatttccggttgaaggatcaagaaatttaaaaacttagcgaaatggaattcaaagatacacaggcaatatacatacagatcgcggattatatctgcgaacagatattgcttaccaaatggcagccggaagaacgtattccttctgtaagggaactggcggtttcgctggaagtaaatcccaatacagtgatgcgcacctgcgagctcctgcagcaacaggaaattattcagaataaaagagggatcggctattttatcagcggagatgcagtgaagaaaataaagcaattcaaaaaagatgcttttatccggaacgaattgccaagtttcttccgcagtatgtacctgctcgatctcgatctcgatgaactgaaacctcactttgagaaattcaaaaaatcaaatttcaactaacatgaaaatcagccataaattactaataggtttttcaggggtactagtgttactcatgctgttttctgccattatactaaaagccaattacaataaaggcatcaccaatacagagaactaccagccacaaaaggatccggattatgcaaaagtgaccgtacctgctttcaaagcgctggtactgaagaacactactgcaaatggcgaagctactatctatgtgcgtgaatcgccggaatacagtctcgaattctataagaacgctacttatgatatgtcgggcgacacactttacgtagcgatcaataaggcgcgtgacatcaccttgtatgctcctgctatcggctatatcgacaacaaaagtgattacagcctgacgatttcggacgttaaatcgccaaagctggaaatcaatgcaggtaaaagtctgcggacttttgtgatcaatacaaaaatcaattcttttgcctttacgggaggagaaaacaatacgcttgaagtaaatgaagataatattctggactcggtgaaagtaacgatggctaaacatggctcactgtatttttatgcaccgtatcagtcgggagaattcagcgtggatagtttagacaacctgaatataaccggcaggtccttacaaagtttaaaacggattaactaaagatttagcaataaattctatcaatgcacaaaccggtttttcagccggttttaaattacataacaagtttttgtgttaaaaatgaacgtcccgatttctatcgggacgttgctgttatatctttttaaagttgttatctttctttaaaactgcgtagctaggtaggccatcgttccgatacctatctcgatcgcatgttcatctacatcaaaagtgggcgtatgtacaccggaagtaataccacgggctgtattgccggtacccagccggaagaagcacgccggtaccacttgtgaataaaaggcgaaatcttccgcacccatcctgatttcggtatcccccactgcttcggcgcccaggtaatccgtggcaaagccacgggctttcgtggttacttcttcattattatataaagtaggatagcctaccaatatttcaatatcaattccggcgcccatcgcttcggcaataccggtggcctgtttgcgtatcagctcatgcgctttgaaacgccaggtttcatccatagccctgaaagtacccatcagctttacttcgctgggaatcacattggtagtaaatccgccattgaaagcacagattgataatacagagggggagaaaggattgttgttacgggagataatctgctgtaagcttactaccagttgagaggctaccaggatggtatctaccgtaagatgtggctgcgcggcatggccgccttttcctttgatggttatataaatttcatctgcactagccatatacttaccggcatgaaatccaagtttaccggcttccatggaaggatgcacatgcaatccgaggatggcgtcggggcggggattttcaagagcgccttcttcaatcatgatgctggcgccgccgggatgtttctcttcacccggctgaaacagcactttaatggtgccttcaaactcctcttttaattcattcaatattttggtagcgcccagtaccaccgaagtatgtacatcatgcccgcaggcatgcattacgcccacgttggtagatttatagggcacatcgttggcttcagtgatgggcaatgcatctatatcagcacgcagcgcgatggttttggaggcggggttctttccttctatcagcgcgatgatgccggtaccggcaataccagccttaaaaggaacaccgaacgcggttaactgctgttgtatataagcagtggtttcaaattcctggaaagacaattcggggtgggaatgcagatgcctcctgatggcagtaaattcaggggcatatgcttttgccagctctttaatacggttcttcattcgatagttctttatccagtgacacgttaataatggcgggtactacaaatacaccacctgcaaacaggtcggataatttgtcccgtaattcagatgcttcctcacgggttttaaaatcgcctacgcgcactttaaaatacggggcctggtaatcgagataggtgcggtagtcgccaaaaagctgcattacttttgctttggcttcattggcatcgccgcgtttgttggtagaaattacctgtacccggaaaccggactggttgcggatggccagggtgttaatgtagatctgttttttaatcagcgcgtccaaacgactatctttcaccactctcacatttccgttgccggcggttgcattgtcctgcgccatggccacaccattccccaacagacagcacaccaggatgaataacttttgcatgaatacggtataattaactatgaataatcgttactgggcttccttgccttcttttactatgttcacactggcactggccccgatccgggtagcgccggcatctatcagctctttcgcaaaagcaaaggtacgaatacctccggaagcttttatttgtatgttagccggcaaattagcccgcatcagctttactgcctctacggtagcgcctctttctgcatatcctgtagacgttttcataaaatccacgccatatttcgcatacagctggcagcactgcacaatttcttcttccaataatatgccactttcaatgatgatcttaatgactttattcttttcccgcaccaggtacatgatattggcgatctctttttccaggtattcccaatctttatttttgatagcagagatattgatcaccacatccagttcatcggcgccgtctacaatagccagtactgtttcggctactttggcttcaatagcggaataaccgaaagggaagccgatcaccgtggctattttggtattggtagcgcccaggaattgtttggcgagcttcacatataacgggggcacacaggccgctgcaaaatcgtactccacacactgcatgcacaactgtttaacgtcttccagcgtggtggtgggcttcaatacggtatggtctatatagcggttaatctccatcattcatttacttgattacaaggcgaaattaatgcaaaacggattacgttgccgtaatccgttctgatatcatttccaggcaggtgcgcttaggcgttcttaccgtggcattgtttgtattttttaccgctaccacatgggcaaagatcattgcgacctatttgtggaccctggtggcggataggctctgcttttacttcttcagccgtttgaatttcaggggcgctgttctggtgactgccgttttccgccagttcctcatgagaagcacgcatgcggctcatatcggttttttcttcccggccttcccggatttccggagcagcttcctgttcctggttgcttacggggataccgcatttggtcaggaaggaaacgatatcgcggctggtttcaccatccatcgccttgaacaggttgaatgcttcaaatttgtagatcagcaaaggatccttctgttcgtatacggcactctgtacggattgtttcaggtcatccattgcacgcaggtgctctttccacgactcatcaatcaaagccagggtgatgctgcgttccagggcgctcatggtttcatgtccctttgtttccactaccttttgcaggttggccagtacgttgataccttttttaccatctgtaaatggtatagagatattttcgatctggtggccctgttcctggtagatacgttctattaccggtaaagtattactgataagatcatttaccttacgtgtatagttatcttttccttcgaaatacagcttgttggccaggttaggaatatctgtcttggccagttcttcactggtaatttttgtatcgatggagaagttcatgatcgcatccatcttgaatgcttcataatctccgctggctttgtgggtagacaccatgttttccgctacatcgtagaaagcgttatcgatgtctattgccagtcgttcgccaaacagggcgtgattacgttttgcgtagatcaccgtacgctgtttattcattacatcatcatactccagcaaacgcttacggataccgaagttattttcttctactttcttctgcgctctttcaatggaacgggtgatcatgctgtgctggatcacttctccttctttatagcccatacggtccatcaggccggcaatacgttctgaaccgaacatacgcatcaggtcatcttccagggaaacgaagaactgtgaagttcccggatcaccctgacgaccggcacgaccacgcagctggcggtcaacacgacggctttcatgtctttctgtaccaatgatggctaacccgccggcttctttcacgccaggtccgagcttgatatccgtaccacgacccgccatgttggtggcgatggttactgctccgggcaaacctgcttccgcaacgatttgtgcttcacgggcgtgttgcttcgcattcagtacattatgcggcactttttcgaaggtgagcattttgctcagcaattcagacacttccacagaggtagtacctaccagtacaggacgtccttttgtctgcagctgcttgatttcttcgataactgctttgtatttgtctctctttgttttgtatacaagatcttccgcatctacacgggaaataggaacgttggtaggaatggttaccacatccagtttgtagatctcccagagctcaccggcttcagtggatgctgtaccggtcataccggccagcttatgatacatacggaagaagttctgcagggtgatggtggcaaatgtttgggtggcagcttccacttttacattttcctttgcttcaattgcctggtgcaatccgtctgagtaacggcgtccatcaaggatacggccggtttgctcatccacgatctttaccttaccgtccattaccacatactccacatctttatcaaataaagtataggctttcagcagctgctgcacggagtggatacggtctgatttagcggcaaagtcctgcagcagtacatctttacgctgcagtttttcttctggtgtcagcggcagcttttcaatttcggccagttcagttcccacatccgggaggataaagaagttagcatcttctccgccctgggtgatcaggtgaatacctttatcagtgagatctacactgttttgtttttcttcgatagcgaagaacaggccttcatctacttttggcatttcgcgttgctgatctgccaggtagtagttttcagctttttgtaataataccctgttaccaggttcgctgagatatttgatcagtgcactgctctttggcaagcctctccaggcgcgcatgagggccagtccaccggttttaggatcatctttaccttctgcaatcagtttctttgcttcctgcagatattgattggttgctttcttttgcatttccaccaggtattcgatacgtggttttaatgcgtggaattcctgctcttcaccgcgggggatagggccggaaatgatcagcggagtacgggcatcatctaccagtacactatccacctcatccaccatggcataatggtgtttgcgttgtaccatttcatcggggttgtgtaccatgttatcacggaggtagtcaaaaccgaattcattgttggtgccatacgtaatgtccgccaggtaagcgttacggcggtctggtgtattgggttgatgcttatcgatacagtctacggtaatatcgaggaattcgaaaagaggtccgttccactcggagtcacgacgtgccaggtaatcattcaccgttacgatatgtacgccttgtcctgccagcgcattgagataagcagggagtgtagatacgagggttttaccttcacctgttgccatttcggcaattttaccctggtgcagtacggtaccaccaatcagctgtacatcataatgtaccatgttccaggtaaccatgctgccggctgcgctccagctgtttttccagatggctttatcgccttcaatggtcacataatcctttctcacagcgagctgacgatccaggtttgtagcggtagcagtcagcgtggtgttattggtaaagcggcgggcagtttcttttactactgcaaaagcggcgggtaataattctttcagtactacttccagttgcttgtcacggtcttttttaagaatatctatttcctggtatatcgtgtcctttacagttacatcttcctcttcatctgcgctggcttgtttttccgctatttctttatcgatagtggcaagatgctcagcgatacgtgcgcggaattcctgcgttttatggcggaggtcatcgataggcagggactgtagtttttcgtactcctcattaatctgctgcaccaccggagagatggatttaatatccctttctgatttattccctccaaatagctttgataaaaaacctaacatgttaaatgtttaattacgaattacgatttctatttattgtaacctgatcccatccaggcagcgtgtatcagttgatagatttctgcttcatcagcctgtggcacaaaggctgcgggcttcgtcagttggatagacggcatccagattactcaaatattgtgcttgttaaagacgaactgtcaaggtgtcagttttacagcccgccccggcaaggcctgtaaaagtaggaataaattcggtgattcaagggggattttgaagggattttgcattttgccattatcaattaacatatctttcatatcagcggaaaaagttagtggtatagccactccggccggataccctgtattctttttactaaccagtcctgccatttttaagggcagtaaatctcataccaagccaatttccggaagtaatacaacaaaccacggccggcaatgccctggaaaatggcttcgtacaatataggactgtcgcaggaaagcagccaatcagccagctgccggttatttgtttatagcgcagcgcccaaattggcagtattgctgccgggagggctcaggcttatatctgccaaaataccagtacacggcgtggtgcatggatatccgtggctgtaagctaagatccggcaggatattttgcaacgcattaagccctggctttctaaccggatgttcccgttatatctttcgccaacgcctgtacgaaattgcggctgatgccactgttagccttattatcgtgttacccggggcattccggcactttccccgcaaaccgcttatcataaaatatgaccagccaaacgggggatctgcgaccagctccccgctgggattgctggtcagcgtcagaaaagaaaattttcaaaaaaaatgcccatcgcccatataaaaagatggaaatatgaaaatactttttataaatttaaaggtttaatagccgttttaacttatttacacaaatatccacgtttatggcaaatgcaattcagccgcaaaaattgttcgtagcaagctgtatggcgctactggtaacatcattatcctttggcatccgtgccggaatattaagccgcttaggcgttgagttccacctggataccaaacaattgagcatcattgcgggaactgctttctggggattcccgctggcagtgattataggaggattcattgtagatgccataggcatgaaacggttactgctggcagcttttatcctgcacctgctgggtattgtgctaacggtatttgcgaacggcttctggtcgctgttcatctccaccctgtttatcgggatggccaacggtaccgtggaagcggcgtgtaatccgctcgtggccactattttccccgacaacaaaaccaccaaactgaatcactttcacctgtggttccccggcggtatcgtagtgggtaccctgctggtatttttacttaccaaaattggcctcagctggcagctgcaggtagccactatggtgatccccaccctgatctatggttatctttttatgaagcttgagtttcctgttacagaaagagtggcatccggcgtatcttctgcgcagatgtacaaatctgtattaagccccctgtttattgtgatgtttatcctgatgtttggcactgccatcacagagcttttcaccggacagtggattgaagtattactgaaaaatgtaaccgaaaattccatcctcatactggcattaactgcaggtgtacaggtacttggaagaggcatcgccggccctgtggtgcataaaatttctcctaccggcgttttacttatttctgcgattttatccgctttgggcttatatttactttctcatgtatctggcaacatggtatttgtggcggcctttatctttggtatgggcgttacttatttctggccaaccatgctgggctttatatcagaaaatatccccgaatcaggtgcactgggcatgaacctgatgggcggcgccggtatgtttgccgtatctgtatacatgtattttatgggcgggttctatgatagtatcatcgtaaaacaactgcctgccggtgcatccctggatgcttaccgctccgctgcccccggttctgctgaagctaccgctttcagtcaggccaccgcagtagccggtccggaaatcattaacgccaccctagtaatacccgttatcctgatagtggctttcgcaggacttttcttttacatgcgcagccgcaaaaaagtagaaaaagcacacgttcaaatagtataaattataaaacgataattgtaaatatgacacggaaacttagaatgggaatgataggaggcggtaaggatgccttcattggtgcaattcaccgtattgcagccaatatggacggactgattgagctgactgccggcgccctcagcattaataacgacgtagcagtggaatcaggtaaaatgttgttcctcgatccggaacgcacctatctcgattttaaaaccatgctggaaaatgaagcgaaaatgccggcagagaagcggctggacttcgtaaccatcgttacgccaaacttcgcccattttgaacctgccatgatggcgctggacctgggtttcaacgtagttatcgaaaaaccgatcacgttttccctcgatgaagccaaacaattaaaagcaaaagtagaagccaccggtttaacgcttttacttacacatacctacaccggctaccctatggtaaaacaagccaggcagatggtgaaagacggtgcgctgggcaaaatccgcaaagtatgggtggaatatccgcagggatggctcagcaaactcagtgaaagagaaggcaacgcacaggcagcctggagaacagatccgaaaaaatcaggtaaaagcggctgtatgggcgacatcggtacccacgcagcaaacctggcagaatatatcaccggcgctaaaattgaaaaattgtgcgctgatctcaacattatggttccaggccgcgcgctggacgacgacggcgcagtattgctccgcttcgacaacggcgctgccggcgtattaatggcatcgcaggtggcagccggtgaagagaacgccctgaagatccgtgtatacggcgaaaagggtggcctcgaatgggcacagcacgagcctaataccctcctggtaaaatggctggataaaccaaccgaaatttaccgcgcaggcggcggatacaatttccagtcgtcttacatgacccacaacacccgcacgccgggcggccatccggaaggatacctggaagcattcggtaacctgtaccgcaacttcgcccaaacgctatctgcaaagatcgatggtgttcagccatccccggaatcactggatttcccgggtacagaagaaggcgtacgcggtatggcattcatcgataacgtagtacgctcttcacaaagcgatgctaaatggactaacttcgagatatagcatatgaaaacgataaaaggacctggtatttttctggcgcagttcatgggagaagaagcgcctttcaataatctgaaatctatctgtgaatgggccgcctccattggtttcaaaggagtacagatccccacctgggaaacgcgcctgatagacctgcaaaaggctgctgaaagcaaaacctatgcagatgaaatcaagggcattgttaatgcagccgggcttgaaatcaccgaactgagcacacacctgcaggggcagttggtagcagtaaatcctgcttttacggagatgttcgacggctttgcgcctgcacaatatcacaataatatccaggcacgcacggagtgggcggtaaatcagctgaagtatgctgcgaaagccagtcgtaacctgggcctcaatgcccacgccacattcagcggcgccctgttgtgggctccggcgatgtacccgtggccacaacgtccggcaggattggtggaaacaggttttgctgaactggcaaaacgctggctcccgatcctcaatgaatttgatgccaacggtgtagacgtttgctatgaaattcacccgggagaggacctgcacgatggtatcacctttgagcgcttcctggaagccaccggtaaccatacacgcgccaacctgctgtacgatccaagtcacttgttgctgcaatgcctcgattatctggaatatatcgatatttaccacgaaaggatcaaagcctttcacgtaaaagatgcagagttcaacgccaccggccgctccggcgtttacggcggataccaggcatggatcgatcgtccgggccgtttccgctctctgggcgatggccaggtagactttaaatccatcttcagtaaaatggcgcaatacgattttgccggctgggccgttatggagtgggaatgttgtattaaacatccggaagatggcgctaaagaaggcgcccccttcatcaaggatcatataatccgtgtcactgaaaaggcatttgatgactttgcaggaggcggtacagatgatgccttcaataaaagaatattaggcttgtaagccaaccaatccaccgatcgttagtaaacaataaccaaataaaaaaatcaacaaatgagaaagagatatctggcgccgctcgtattaagtgtattattctttgcagcttgcggaggtggtgagaaaaaagcagaaaacgcagacagcgttagcactcatgaaagcccagcagcagataattcaatggtttcgccaaatgccaacaaaccagtaagcaaaggcgaaacactgatggctgaaagcgattgtaaaacatgtcataaagaagaaatgaaagtggtaggacctgccctgaaagacattgcaggcaagtatcctaacacaccggagaatgtggaaaaactggccgataaagtaatcaaaggcggttcaggtaactggggcgaagtagccatgttgccacacccacagatttcaaaagaagatgccaaagaaatggtaagctatatcttatctattggcaaataattgatttatcataaactcaatcatcctgaatgaaaaaattaatcatgggtgcactgatggtagctgccgttctcggtaccaccgcagtaaaagcccagaaattaaataccctgtcagcgaaggagaagaagcaaggatgggtactcctgttcgatggtacttctaccaaaggctggcatacttacctgaaatccacagccagtcccgcatggggcgtaactgatggtgcgattggcctgaaccaggaagccaaaaagaatggcgcacccggcggagatctcgttactgacgcagaatacgaaaactatgagctgagttacgaatggaaaatttctcccggcggcaacagcggtcttatcttcagcgttcatgaagatccttctttaagccaaacttacctctccggtcctgaaatgcaggtaattgatgatgccggccatcccgatggtaaaaaccccaaacacaatgcgggtgaattatacgatctcatcaaagcttctaccaggccagccaaaccggttggtgaatggaattccgccaaattaacgaagaaagatggtcacctgaccctctggctcaatggcgtgaaaactgctgaaactaccatgggcacacctgaatgggatgcactggtggcaaaaagcaaattccacgactggaaagagttcggcaaacacgcgaaaggtcatatcgccctgcaggatcacggcgatgatgtatggtaccgtaatatcaaaataagagttctttaatttccgatagcgcaaaggcattaagcaaaaagctactgaagcggagatgggcgctcgcttatctcaatacttcagtagctttttgctttttgcttctctgaattttttcatttccattcccacgtaaaataagatgaaagcattaaccgcgtttattacactcttgctcctcgccggcaccatttccgtgcaggcaaagcataaacacaagaccaaaagggtgctcgtgttctcaaaaacaaaaggcttccggcacgattgcattcccgcttccaaaatagctattatgcaactcggaaaggaaaatggctttgaagtagacactactgaagatgccagtgcctttactgccgacaacctgaaaaagtatgcagccgtcattttcagctgcaccaccggcgacgtgctcgacgacgctcaacaggtggcttttcagaactatatccacaaaggcggtgcatggatgggtatccacgcagctacagatacggagtacggctggccgtggtataacaaactggcaggcgcctggttcctgagtcatccgagccagcaaacagctaccctcaaagtagtggaccataatcatccggctacaaaagatttaccggacgaatggatccgcaaagacgaatggtacaatttcaaagatcttaaccccgacgtacatgtgctcatcaaaattgatgaatccagctataccggtggcaaaaatggtgataaccatcctatgtgctggtatcacgactttgaaggaggccgcgccttttataccgaaatgggccatgtgaaagaagcttaccaggaccccgtatatctgaaacatttgctgggtggcattgaatacgccatcggcaactggaaacccaaaaaataatccgtaataatgaaacatactctcagaatttttttgctgctggcactcgttgttgttggtctcgcagcctgtaaaaaatcacgccccggtaaacccagggtactggtatttaccaaaaccagcggcttccgtcacagctccatccctgttggtattaaagccattcagaaactggggttggaaaacggatttgatgtagacactacagaaaacgccgctaaatttaatgaagataccctggcgcaatatgccgccgttatcttcctgagcactaccggtgatgtgctcaataactaccaggaagccgatttcgaaagatatatccaggcaggtggcggttatgtaggcgtacacgccgcagccgacaccgaatacgaatggggctggtataaccacctcgccggtgcatggttccagagccatcctccgggcgttcataaagctatagttgatgtaattgaaaaatcttttcccgctacagaaggactcccggaaaaatgggaacataccgacgagtggtataattataaaaatgtagataccaccactacggtgctgctgaaactggacgaaaagtcgtaccagggcggtactatgggcggcaatcaccctatcagctggtatcacgattatgatggtggccgcgctttttataccggtcttggtcatacggaagaatcttataccgacagcctgttcctgaaacacctcgccggcggtatcaaatacgccattggtaaaaaccaggtacttgactacagcgccgctaaaacgctgcgtgtaccggaagaagaccgctttaccaaaaatgtgctggtatccggtgagttcttcgaaccaacggaaatggctatactccctaacctggatatcctggtggcgcaacgccgcggggaactgatgctctacaatgcagcagaaaagaaactttcacaggtaggtttcctcaaagtatatcaccacaccgatgtaccaaaggtaaatgcagaagaaggattcctcggccttgccgcagatcccgactttaaaaacaatcactacatctatgcgatgtattcaccggtagatacttccgtaaaccgtttgtcccgtttcaaatttgaaaacaacaaactggatatgtcttctgaaaaagtaatcctgcaattttactcccagcgtgatatctgctgccataccggcggttctattgcattcgggccaggcggactgctgtacttatccacaggcgacaacaccacgccgtttgacgaacccggacagcaatatgtgagcaaaggctacggtcctacagatgaccgtcccggtcacctgcagtatgatgaccgccgcggttctgcgaacaccaacgatctccgcggaaaaatcatccgtatcaaagtagaagcagatggctcctatactattccggacggtaacctgttcccgaaaggtacaaaaggcacacgtcctgaaatttatgcaatgggtacccgtaacccttaccggatgtcggtagaccagaaaacaggatatgtatactggggagaagtagggccggatgccaataacgacgactccctgcgagggccgagaggatacgatgaagtaaaccaggcgaaaaagcccggcttcttcggttacccgatgtttattgccaacaataaaccttaccgtcaatataattatgaaacaggtgaaagcggtccttattttgatccgctgaaaccgatcaatgattcccgcaacaataccggtctgagagagttgccaccggctactcccgccttcatctggtatccttatgcgaaatcagatgagttcccgattgtaggtagtggtggccgtaacgcagaggcaggccccatttatcacagcgaattttatccgaaagaaacccgtttcccggattactataacgataaactgtttatctacgactggatccgcggatggataatggccgtaaccatggataagaacggcgacttctccaaaatggaaaagtttatgcctaacaccaagctgaacgcacccatcgatatggaaatgggtccggacggccgcctgtatatcctcgaatatggtaacggatggttcagcaaaaatgcagatgcaggtctttcccgcattgatttcaatggcggcaaccgcgcacctgtagctaatatacacgctacgcgcaccaccggcggcttaccatttaaagtgaaattaaccgcagaaggatccaaagatcctgatggcgataaactcacctacctctggaatttcggcaatggcacaaagaaagaaaccactgaaccgagtgtagaatacacctacagcgctgcaggtgaatatcctgtatttgtggaagtggcagatgataaaggcgccaaaacaaagagcaaatccattgacctctacgccggtaatgaaacacctgatgtaaagatcaatattaccggtaaccagatgttctacttccccggtaaacccatccagtatgcggttaatatctcggataaggaagatggcaattctgcagatggtaaactggacgccaataacatttttgtaaaggcggactatgtagaaggtcgtgacaaagcagcgcaaccacagggacaccagatcattaccggtgctattgccggtaaaaatatcatggaagtatccgattgtaaaacctgtcacaagccggacgaaaaatctatcgggccttcttttaagcaaataacagaaaagtataaggacgatcctgccgcacctgaaatgctcgctaaaaagatcatcaacggcggtggcggcgtatggggcgaaacagccatgtctgcacatccaggcatctctgtgggtgaagcaaaacaactggtggaatatatttattccatcggtggcaatgcacctaaggtaccatccctgcccgtaaccggcagcgtcaaccctacattgggcggcgaaccaaaagacaacggtgtgttgtacctgttggccagctataccgataagggtggtcctggcattaagcctatcaccggcactgcttctgcagaactgatcagccccaaactggcggcggcagatttcagcaaagcagatggcatggcggtattcgctgtaaatggtacgaagttccttattccttctaacacagcaggatgggccacttacaacaacctggatctgacgggtgtaagcggtatcgaactcgcttacctggtacaggaaacaccacaatccggctttatagttgaagcattcctggatgatgccaacggcacccgtctgggtgaagtgaccattggtccgggtgcacaaccaaaagttccgaacaaggtgaacttcaactttaccccggtaacagacggcaagaaacacaacctgtatttccgctacaaagcaattgatgcggcgcaaacagtacagttgggtatcgtgtcatttaccctgcatccataacactagttttttataaaaagaaaggggagctctgtataagagttcccctttctttttataagacaaattcacttatgcaccgcataattcctgataacaaactgttcttcaaatcccatgtccaggtatatgcctttccccatttgtgaggcctgcagcgtggcatagcgtgcattcagcgccagggattcattcagtacaaacgccataatttcattggcaaatccttttcttctcgcttccggaatcacgcccactccatgtataccggcaataccatcttcaagatggaggatagcagtgcctaccggctgtccgtccagcaaggcaagataataacggagattgctatacgtagcttccaggattttctgatcaatgctgtatccgaatgcctgtggataaattcccgcccacaacgcagcatctgcaagggtattaactgcccggaacaacagcctgttctcattccggaacggccgttccagtttcaacgacatccctgcctgctcagaaccctttatccctccctgcgcgataataatttcttccccggtagcattccaataagggataaccattttgccggaaggaatactatccagtgccgttcgcattacttcttccgtaatatctccattaaaccacagtttattgggccattccaggccaggcacactgcaccagctgaaatccggcgtttctacacaggcgttgaaaggggtgctggctatacgccatacaccaatcaggttgttgatatttgctttaacaatagcaatcatttttgttatttattaccgccaagataggaatatggtggcataaaaaaggctgcttccgtaatcggaaacagccagttgtctgattgggcactcttgttatttctttggtttggcgctcatataaaaagtgatggtgccgccgttcatgatatccgcatgggtgatatacaaacggttcaacggcgtgccgttgagcaataccttttgtacatacacatttttatcaccctgattttttacatctactacaaaggttttgccgttttccagctgcagcgttgccttatcaatagccgggctgcccagtgaatactggtcggaaccaggacaaaccgggtagaagcccagtgtggtaaaaatgtaccaggcgctcatttgtccgcagtcatcattaccgccaagaccatcaggccccgggtggtacatctttttcaggatcatgcgtacacgctcctgtgttttccacggatagccggtccagttatacaggtaggccacatgatgcgaaggctcgttgccatgaacgtagttaccgataataccgtcgcgggtgatatcttctgtttcagcaaaaaatttatcgggcaattccatggtaaacagggaatcgaggtgaatggtaaattgtttcttaccacccatcatggcaatcatttcatcggggtagtgaggcacatataaactatagttccaggcgttcccctcaataaagccctggtcgtgcgtttgcagcgcatcaaagttagctttaaaggtaccgtcgttcagttttggacgcatgaaaccggtgttggaatcgtatacattcttataattcagcgaacgtttaataaattcttcatagagatctgtccgccctaatttcttagctacctgtgcaatacaccaatcgtcatatgcatactcaagggttttggaaacggaagaaccgtttttatcttccggtacataacccctgtcgatataatattccaatccgtcgtaagtgcggtgacgcgccgtcgttacgcatgcatccagtgctttgttcacatcaaacggagcgttgcctttcatgatggcatcagcaataacggacacgctgtgatagccgatcatgcaccagttttcattggcataatgtgaccagataggcagcatgtgttgtgcactttgttcatagtgattcagcatcgactggatcatatcggcattccgtttaggctggatcacattaaacagcgggtgcaatgcccggtaggtatcccagagtgaaaaggtagtatagttcgtatacccgtttgcggtatgaatgttcatatccagtccgcggtattgtccatccacatccatgtaagtggtagggttgatgaaggcatggtacatggcggtatagaagttttctttctcttcccggctttttgattcaatatgaattttattcagctctttggtccaaagtgcctgtccatcgcgttttacctggtcgaaatcccaacccggaatttccgcccgcaggtttttcagtgcgccctcggtactgaccggagataaagcaaatttaattttgaccttttcaccgggtgttgttttaaagtcgaaataggcgcggatctgttttcctgccatttccgggaagttcttcgactggtcaaactttctccagaagcctttgtacacatctttggcataattctgatgcccgtactgaacaaagggtttcgagaaggtcatggcaaaatattctattctcgtacgtgcccaaccgttagtttggcggaacccggtgatcagggtatcattttctacccggataaaggtccacacgtttttattgtcgtagttgtaaataccggacatcatatccaggatgatatgcgcctggccggcaccgggaaaagtatactggtgaaatcccacgcggttgctggcggtaagttctgcgaggatgttatcatcttccagtttcactttatagtaagcaggctccgctatttccgtgctatgggaaaatttagatctgtagccactttcaggatgatctgccgtgccggggtttaattgcagtgcgcccacggtaggcatgatgagaaaatcacccaggtcggaatggccggtaccgctgaagtgggtatgactgaagccaacaatcgttttatcttcatactgataacccgcgcaatacttatatacatcggggttatacttcccattcatttcgtaaggaatggtatcggtttcaggactaagctgcaccataccaaaaggcaccgtagcgcccggataggtgtggcccatccgctgtgtgccggtaatcggcttcacatattgtattacattctcctgtgccattgcgcacagggatggaaagaagagtaaaggtaaaagtagtttcctcatagcggttgattttagcggaggttgtcttattcaggattacgctgattttgttgatttcactgaatttttttttaataatttgaaagaaaatcttttaaaatcaaaaaaaatcaaaagagaaaaatcaacaaaatcagcgtaatcctgagtaagacaaccttcgcgtaagaaatttggtacatcccgaagagtcgggatgaaatatttcagtgaacaatgaaaatcgtttacaggcggtatatattacttattcgctgttgctgaataggaataaggataagccgccggatcggttcctcttgatttctcaggagtagcgcccatgttaaattccagggtaccgcctttctgcaggtcctggtggctgatccagttcttcgtataaggctgcccgttaagggaggccttttgcacatacaggttcgtgtcgctgttgcccggagcattgatcaccattttcttaccatcttcgaaagtcatggtcagtttggagaagagtggcgtacccagtacatattgttgggtacccggacaaacaggatagaagcccatggccgagaacacgtaccaggcgctggtttgaccgttgtcttcatcaccacagtatccatccggggtggctttgtacaaacggctcattacctggcggatccagtattgtgttttccagggctggcctgcataattatataaatagatcatgtgctgaatgggttggttgccgtgtgcatactgtcccatgttcatgatctgcatttcgcgtatttcgtggataacggtgccatagtagctttcatcaaataccggcggcatattgaaaacggaatccagcattttggcaaacatttcacggccgcccattagtttggccaggccttgcacatcgtggaatacagaccaggtatagtgccagctgtttccttctgtaaaggcatctccccatttgaatggattgaacggcgtctggaatttgccatccttgttttttccacgcatcagttttgtttccggatcaaagagattacggtagttctgggaacgtttttcaaaacggtcgatttcgttcttcggacggttgagtgcttttgccagctgatagatggtgaaatcgtcgtaagcatattccagtgtacgtgcagcgttttcatttacttccacatcgtaaggcacgtagccgagtgtgttgtaatatttaacgcccaggcggcctacagagctgagcggaccttcgttttccgtgtttttcagaatcgctttgtacaggttattgatgtcgtatccgcggataccttttaaataagcgtcagcgatcagggatgcagagttggaacccaccatgcaatcgcggtgaccgggacttgcccactcaggtaaccagccgctttcattgtaagcgttggatagtccttccatgatatgcgagctgagcgtaggatacatcagggtaaagaaaggatgtactgcgcggaaagtgtcccagaacccgttatcggtgaacatgtagcctggtaatacctggccattgaacgggctatagtgtacgatttcgttctttgcattgatttcatagaacttgcgcgggaagagcatggtacggtacagggaggagtagaaggtgcttacctgttcgctggtaccgccttctatggccaatctgccgagttcctggttccagctgtcttttgcttttttacaggtagcgtcaaagttatcctggccgatttcgcgttgcaggtttaattctgcctgttcaaaactgataaaggaagacgcggttttaattcccaccttctctcctttctttgttttaaaaccaaccacggcgccggtatgatctgcctgcagttccagctggcctttcaccagtaccgagtcatgccagatatcggctaccgtaaatggtttatcaaatttgataacgaagtagtttttgaaattggaaggtacgccaccgctgtttttggtggtatatccaatgatcttcttttcgtccggcaatattttaatataggaacctttgtcgaatgcgtctaccacgataaaagcgctgtcggtagcggggtaggtaaaacgcagctgggcggctctttccgtgggcgtaatttccgtggtaacatccgggtcggccaggtatacgctgtaatagtatggtttcgctacttctgatttatgagaaaaccagctcgcacgtttgttttgatcaaacttcacggtgccggtaacgggcataatggcaaactggccatagtcgttgatccagggtgaaggttggtgtgtttgcttgaatcccctgattttatcagcggtatattgatatgcccagccattccccatggtattggtttgtggcatccagaagttcataccccagggcagggcaatggcaggataggtgttcccgtttgataagctcactttggaatcggtgcccatcagggtatttacccagtccgccggctcagcaactttatttaccgtttggctgtgtgcaccatgcaggcataataaagcggctgctaacagtccaacttttttcatgattagatattatatacaacaaaaatgatccttaggccaatatcacactccgttgtgtgaagataccgtgaaatttttacaaaatcgatttagcacaggtacagaaaaaaaagattcatcgaatccttttctcttaaacgacaatagccggttctaaaagtataaatatttttccagcatttgcaagtatttaatggtttttttacgagcggtaccggcaattatgccgatccccgcaggatgaactttccgggcaattctatcgccgttttcttcattggcccgctgtttttgtccagctgatgcataagcaggtctatggccgttttggcaatgccttctatcggctgttctatcaccgatataccgggaggatataaacggaagatatcgtgatcgtcgaaacagagcacggcaatatcatcgggcatcttcaatcccatcctggcgattacttccagtcccaggatacccaggtagttggtggagaaaaagatggcgtccagctccgggttagcttctataaaggcctgcagctcattcagcgagtcttcccgctgccggtggtactgcaactgcaggatatgttttttctttacggggatcttatgttctttcagtgccgtggtatagccccgcaggcgctcctccagttgtatcagtttcacgtccaccatcacaaagcctattttggtgaggcctttacctatcaggtgtttcatcccctgctgcacaccgtcaaagttattgatcagcacatagggcgttttgatagatggaaaatagctgtccatcagcactaccggcttatgctggtgcaccagttgctggatttctttttccatacctggtgcaggcgtaatcaggtaaccgtctaccatttgccggccaagcatacggattaactccccgcctttctgcgcattgttttcggtgctgcaatacaccacattgtatcctttgcgctctgcttccgtttcaattgttttagcaagacttgcaaaaaaacttccggaaatactttccacaatcagacccagggtcttggattgcccggtgcggaggttcaccgccatacggtgaggctcatacccggatttttccgccacctgcatgatcctggtggctacctcgtcgcggatacgcatttgcttcccctttccgtttaaaacgaaagataccgtggaaggcgctactccggccatttttgcaacatccttaagggttaatcgcttcatgtatagtgattggttttggcatatatgaaaatggaattacctggacattcccacacatccatctattacatattacagggtatgttaccctctgacagatacacattgaaacggaaattacaaaaatacctgtaattactaccagggaagaaaaaaatggttatcttcagtagccccgtacggcataatatatcttccgtgggaacgttataataatctaccggctcctggccaacattattacaactgtagtaaaaaatacactgagcatatgaagcaactttctcaacttactgacccggtttacatcaagcctatacatgaaactgcacttgaccgtcttttcaaaagctggatcagggatgaacgcgaccttccctttgtgtacctgacactgaaaattactttcaccctctggccgctggctatcctcatgtatattcccggaataaataactgggtttggtggggcgctgctattgcttaccagttcctgaataactttactttcaaagggccttttggcctgatgctgcattgcaccagccaccgtgctttctttgaaaaaaaataccagttctggaataattatctgccctgggccatcggtccgttgttcggccaaacgccggaaggctattattctcatcatattggcatgcatcatccggaaaataatatgcccgacgatgatagctgcaccatgatctaccagcgcgactccctccgtggatttctttcttacctgggaagctttatcactttcggtgtttatgacaccgcccgctatcatttacagagaaaaagaagtaaactgatggtaaaactggtaaggggagaagtattatttctcggcgcctgcgttggtttatcgtttatcaacttccctgctactttcgtggtattcatattaccctttatgatttcccgcgtaatcatgatggtgggcaactgggcgcaacatgcttttatctgccccgaggaaccggataattcctataaaaacagcatcacctgtatcaatacaaagtataaccataaatgctggaacgatggctatcatatcagtcatcacgtaaaaccaaacatgcattggacagagcatcccgtatacttcactaaaaccctggacgaatacatcagcaacgaagctatcgtatttgatggcatccatttcctgcatgtatgggctttccttatgggcaaacgttacgacctgctggcaaaacactttgtgaatatcggcgaccgcttccagacagatgctgaaatcatttgctttctgaagcagcgtacccgtaaaattaccgcactgcctgtaccggcagctgtggctgcagcctgataatattactgtctatttacgggagggttttcttttttaaggttacaattcccttgcattctcacatttttaagataaaaatgccgggaaaagagtaagggaactgtcagatcctgcgccctcatgcgcacgaacccgcgtctgcacagcgcttcatcgtaaattccaaaaagttatattatattatcttaatgaatatgcttaatcataacaataagtaactaaatttgcgctctaactttttttattaaagtaaaaaatatgcgtactgttacactgaaaagggttgtggttaccggattgggagcattgacacctatcgggaatgatgtaaatactttttggaacaatatgaaggcaggcgttagtggcgccggccccatcactaaatttgacaccacagagtttaaaacaaaattcgcctgtgaagtcaaggggtttgaggtggaaaaatatatggaaaagaaagaagcccgcaaaatggattgcttcacccagtacgctatggcggctgcacaggaagcagtacaggatgccggcctcgataatgccaacatcgacaaaactaaaattggggtgatctgggcatcaggcaatggcgggatgcttacgttcgaagaacagatcgttgaatttacacaggccaactttgtacctaaattcaatcctttctttatccctaaattgatatgtgacattgcagcaggccagatagctatgaaatacggtttcatggggatcaacttctgtacagtttctgcatgcgcttcctctaccagcgccctggtagatgcttttaactacatccgcctgggtaaagccaacgcaattgtggcaggtggctctgaagctcctgtaacccgcgccggtattgccggattcaatgcccttaaagctttatccacccgcaacgaagatgcagcccacgcttcccgcccgttcgatatagaacgcgacggatttgtaatgggtgaaggcgcaggcgctattatcctggaagaatatgaacacgctatcgccagaggtgctaccatttatggagaaatgattggcggcgccatgacctgcgatgcctaccacctcacagccacccatccggaaggcatgggcgcacgcttaggtatggaacaggccctggaagatgccgacatcgcgactaccgatgtggattatatcaactcacacactacctccacaccagtaggagatctcagcgaattaaaagccattgttaccgcttttggtgaccatgtgcaaaaacttaatatcagcgctaccaaatccatgacaggtcacctgctcggagcggccggcgctattgaagccatcgcttgtatcaaagccacacaggaagatatcattccacccaccatcaacacttccgtgttgggtgaaggcatccctaccaacctgaacctcaccctcggtaaggcacagcaacgtacggtgaacgtagccatgagcaatactttcggttttggcggacacaacgcgattgtaatattcaaaaaatataaggcgtaggcggcgccttcggcgcctgtaaattgtcttgagcaggattttgggattaactgtgatggcactgattttcccacttcttgttgtaaatatttcggggagataaaagcggatagatccgcttttatctccccgaatctgttaacgaccttgttaataatcaggaaatccgtgtaattacaattagtaattatccgcttacatctcccttaattaaattaataacaaaaagtgggaaaatcagtgccatcacagttaatcccaaaatcctgctccaagacaatttacaggcgccgaaggcgccctcccctcacttcgctaaaattcttagcattacagaaccgaaaattcgcaattatgccgtagcttagtagtttaatattatggcaaagaaaaaagagaatgtacccgatacttccgttgcgcaagccccggcagatgaacaaatagccatttttggcgcccgggagcataacctgaaaaacctggacctgcagttgcccaaaaataaactggtagtgatcaccggcatcagtggcagtggaaaatcatcactggcatttgataccatctatgcagaaggacaacgccgttacatggaaagcttttccgcttatgcccgccagtttatcggcgatatggaaaggcccgatgtggataaaatcaccggactttctcccgttatttctatagaacagaaaacgaccaataaaaatccacggtctaccgttggtactatcacggagatttacgatttcctccgcctgctctatgcacgcgccggaaccgcctactcctacaataccaacaaacccatgacccgcttctcagaagaggaaatattggcgcatgttttcaaacattataaaaataaaaagctggccatcctcgccccgcttgtacgtggacgaaaaggccactaccgggaactgtttgaacaggtacgtaaacaaggctacctcaaagtgcggatcgacggggaaatagaagatctgaaagaaagaatgcaggtggaccgctacaagatccacgacattgaactcgtgatagaccgtatccaggttcaggaagatgcgcgcacccgtatcagccagagcgtacaaaaggcgctcaccatgggaaaaggattgctgtttatcatggaccacgataccaataaagtgagccagtacagcaaacaactgatgtgtgaggaaaccggcctttcctacgaagaacccagccccaacaccttctcctttaactccccctatggcgcctgcccccgctgtaaaggtcttggcaccatctaccagatagatatggacgaagtaatcccggattacaacatatccatcaccgacggtggactaaaaccattaggtgaagcacgcgatacctttacctttaaacaggtacaacaactcgccaaaaagtataaattttccttaacagcccctatttccagcatcccgcaaaaagccctcaacgtattgttgtttggtgatgaaaacggcaaactggaagtagacctggaatttggagaaagcaatggcagcaccgaatacgtcactgaatacgaaggagtagtaaacatggttcgccgttattttaacgacacctcctccgatcatgtacgcagctgggcagaaggtttcatgaagctaagcacctgccctgaatgtaacggcgcccgtctcaaaaaggaaagcctgtttttcaagattgatgaaaaaaatatctccgaactcggtaacatggacctggataagctcctggcctggtttggaaatatcgaaacccgtcttgagaaaaaacaaaatgcaattgccaaggatatcctgaaagagatccgtgaaaggctcgggttcctgctgaacgtaggattaaattaccttacgctgaaccgccccacccggagcctcagcggcggcgaatcgcaacgtatccgcctcgccacacagataggatcccaactcatgggcatcacctatatcctggatgaacccagtatcggtttacatcagcgcgataacatgcagctgatagatgcccttcgcaacctgaaagacatgggcaataccgttattgtagtggaacacgacaaagacattatgctccatgcggatcacctggtagatatcggacccggcgccggtgttcacggtggccagatcattgcacagggtacgcctaaacaaatacttaaactcaatacacccaccgcgggatacctgaatggtaacgccaccccggaagtacccgaacaacgccgcaaaggcaatggtaatttcctcgagctgaaaggcgctaccggcaataacctgaagaatgtaaacctgaaactgcccctgggcactttcatttgtgttaccggcgtttccggcagcggtaaatctaccctgatcaatgaaacgctgtatcccattctttctaaacatgcttacgattccaagatggtgcccatgccttacaaaagcatcaagggactggagtttatagataaagtgattgaaattgatcagtcacccataggccgtaccccgcgcagcaacccggctacctattgcggttttttcaccgacatcaggaccctctttgcttccgtgccggaggctaagatccggggatataatgccggccgtttctcatttaatgtaaaaaccggtcgctgtgatgtttgtgaaggcggcggcatgcgcgtgatcgaaatgaacttcctgccggatgtatatgtgcattgcgaaaaatgtaacggtcgccggtataaccgtgaaacgctggaaatccgctataaaggcaaatccatttccgatgtgctggacatgacagtagacgaagctgtggaatttttccagccggtaccatggatctaccgcaaaataaagacgctgcaggatgtgggactcggatacattacgctcggacaatctgccgtaaccctttccggaggcgaggcgcagcgggtaaaactggctaccgaactatccaagaaagataccggcaagactatttatatactcgatgaaccaacaacgggactgcatttccaggacatacagctgctgttaaaagtactgtacaaattggtcgacaggggcaacaccgtactggtcattgaacataacctggatgttattaaaatggcggactacattgtagacctggggccggaaggcggcggcggcggcggcaccatcttatgtaccggcactcccgaacaggtaagtacctgcaaagaaagtcataccgccagattcctcaaaaaggagctgggaatttaatatcttgccaactgtaaacaagcaatgaaaagcatctaccagatattactcacctgtttcatttttgcgggcatcattgcctgtgaaaatgaaacgaaagtatgcgatcagactttacggaatgattaccatacgcatcttatgcgcaaactcaatgacagattatcagacactgttatgccgaaagtaaccgcatatgcatttggcagagataccatttacaggagccaggcattgggcgacctgttcttccagctatcaccgatagcagacagcagcctcttttacgtgaaagtggattccagctttgtgcctgatactttaaagatcaggtatacgcggcaacagcattttatttctcccggatgtggttttggtacctattttaatatagatactgttatcaccaccatgcataccatcgattctgtcgtaattaataataagtccgtaactagcagtaatgacacgcatcttactttgtatttcttttttgactagtatcctgctcagcgttgctgccacggcacaaaacaagccggccgccgctaaaacggatacgctgcccaaagctgttaaagctgataccactcataaagtgctggctgattcagcaaaagcggtggtgttggcgcataaagacagctcctggtttattccgggtgcagtgcggataggagtggatcttagccgtatcgtttctgctatctattatccttacagaaaagaagtaactgccgtggcagatgctcgtatcaacagtaatctttacgctgcctttgaagccggatatgccaataccccgtacagcgataccaattatacctataaagggaatggtatgtttgttaccctgggcgttgattataattttctgaaaagacaatatgtttccgaaaagaatatgttctatgtgggcttccgttatggattctctcattttaattattcggttcccacctactccattaaaaatacctattggggcgataatctcacgggcagcgtccccaaaaccgcagtaaatgcccattgggtggagctcctggtaggattgaaagtagaagtgctcaagaactttttcatgggctggaacatccgggaacgcatcctggttaacaacgtaaaaaccgataacatgacgccactcgtcattcccggttttggtaatggttctaaaagatcagtttttgatgtgcaatacaccatttcatacgctatccccttctaccggataaaagaacacgcgcccgataaagaagtgaagaagaagaaaatacctaagcgataacgcggtgcggaggttgtctttctcaggattacgctgattatactgattacctggatttttacttttggattttttttagatttttagattttcctaaaataataattaagggagataagagcgaatatccgcttctatctcccttaatcctttataaaatcaaaaagtaaaaatccaggtaatcagtataatcagcgtaatcctgagaaagacaacatccgcggcgatcatccccttagcatttcaatgtgaggaatcccatcttccatataagtatcgctggtttgctcaaatcccagcgaagtataaaaccgttgcaaatattgctgtgcccctatccggataggaatcacgccataatgcttctgcaatgctgcaatagagcgctccatcagttcccttcccgcacctttgccgcgggccagcggggatgtaattaccctgccgatagatgcctccttaaatttgattcccggtggaaaaatacgggtatatgccagcaaccggccctcttcatctgttcccattaaatgcagtcctttctggtcggaatagtccaggtcctggtaggcgcagttttgctccaccacaaatacttcactacgcaaatgcaggatagcatagagttcggcagtagttaactcctcaaatgattttgtattccagatcataccctcaaactttgccataaatttagtggaagctttcaataatcggattaattttatatccgatagaagaatattgagcccaatcgttcaaactatggcagaacagcaaacaccgttcctttcgctggaacacattacggtgaggtatcttgataaaacattattcaataccctcacctggcagatcaacaaaggagagcagtgggccattacaggacccagcggttccggtaaaacagccctgctgaataccattcttggtaaatttaatatcatcaatggcagtatccattaccacttttacgacgagtggtgccggcaacataccgtcacagatccctggtttaattaccgtaacctggtagccctggtagggcatcaccacactttccggaatctctccaatactaccacggacttttattatcagcaacgcttcaacagcatggacgccgataattcccctactgtaatggaatacctggaactcactgaagtgccggcattactccagcctctccgcattgcgccgctgctggaaaaacggctcatcaaattatccaatggcgaaacccgccgggtaatgattgcacgtgccctcatccaacagccgcaactgctcatgctggataatccctacatcgggctggatgtgcaggccaggaaagatttcagcaacatgatcaatgaaatcattgccggtggcgccactgtattgctggccaccgccccccatgaaattcctgagcatattacacatgtccttaccctggaaaatggcggtataacaggtaagtatacacgcagtgaatttatacagctgccgctgcccgcagcaacagcaatagcgctgccggaaatggaagcccataaaatagccgcgctggtgcataacagtcagcagcaacagttcgacactattgtccggatggaagacatccatattaaatacggtgaaaacaccatcctgaatggcatcaactggacggtaaaaccaaacgaaaaatgggcgctgcttggtcccaacggcgccggcaaatctacgctgctgagtcttgtgaatggggataatccgcaggcatatgccaataagctctggttgttcgaccggaagcggggcagcggcgaaagcatctgggatatcaagaaaaaaatcggcttcgtttcccctgaattacaccagtattttacctcccgtgataactgcctccaggtagtatgttccggcttctccgatgtaatcggcagcaccaggccagctaccgctgaacagcaacaggtggcccgcgactggatgagcgttctcaatatagcggaacatgaaaaggcaccgttcaaacaggtgcctgaaagcgcccagcgcttaaccctgctggcacgcgccctggttaaaaatccacccctgctgatctttgatgaaccctgccagggactggatacccaacaaaagctacatttcaaaaaagtaatagaacagttgtgtgaacacatgccggtgacactcatcttcgttacccactacgaagatgaactgccttcgtgtgtagataagttcatccggttgaacaagggtgaaatggtgtagtgcggatgttgtctttctcaggattacgctgattttactgattagctggatttttacttttggattttataaaggattaagggagatggaagcggatatatcgctcttatctcccttagttatattaatcagtaagaaaatcaaaaaaaatccaaaagtaaaaatccagctaatcagtaaaatcagtgtaatcctgagaaagacaaaatccgcgtttaaagaaaattcccgacattcgcacctaatagttaatcacctaatctgctttcccgatgcacccaacaaaaaggcttaccgctgtagcagcattgtttttattcctggccgccctgtttgtgatcaatggttgccgtacggcgaagaaagaaatgaaccccgaatttgcccggtacattgaggcatataccgcggggatcatttccaaacaaagcgccatccgtgttcacctcacctcacaaaccaatgtaacccatactcagaacgaacccctggaaaaggaagtatttgagttttccccttccatcaaaggaaaggcttactggattgatgccaccactatcgaattcagaccggatgaaaacctgcaacccggtaaaacgtatgaagccaactttaaacttggcaaaatactggaagtgcccaaggaactcaaatcgtttgattttgaattcaagatcatcaagccatcattctctattgagaatttcgggctgaaagccagcactaataatacgctcgaccgcatgacctgcaccggcgctatttatacagcggatgtggaagacccgcaggcgattgaaaaaatactcaccgcacaatacgccggtaaaggcttacctattacctggcaacacaatgccgcagaacgtacttcccgcttcaccattgccaacattgcacgggctaacattgcccgtaacatggaactgagctggaacggcggatcgttgaaagtggataataccgggaaaaataccatcgaagttccggctatcggcgactttaaagtattgaatgtaaaagcgctctcagatccggagcaacatctcctggtacagttttcggaccccgtaagtatggcccagaccttggaaggattgatcggcatcagcggtcaaagcgacctgcgttacaccattgatggcagcgaagtaagcgtatatgcaccggtgcggctggaaggaagctataacgtcatcgtaaatgaaggcgttataaacatcacggataaacgcttaggtaaaaccttcagcgccaacgttaactttgaaaatactttacccagcgtgagcattcccggcaaaggcgtaattctcccggaaagtaataagctggtgatgccgtttgaagcggtgaacctcaatgccgtggacgtttccattataaaaatctacgagaataatgtgccgcaatatcttcagcggaatgacctcgacggcagccaggagctccgtcgtgtaggcaagcccgtagtagagaaaactatccgtctcgatggagataaatctgtaaacctgcataagaagaaccgcttcttcctggacctggataaaatgctgcgcaccgaacccggcgccatttaccgcattactatcggcttccggaaatcatacgctatgactgcctgctccgcagatactaccaaggatggtgacaatgcgtcttccgatgaggaaggagaagaagaatattatggcggagaaaaaattgatgatgatgactcattctggcaacggtatgacagctactatccatatggctataactgggaccgccgcaatgatgcctgctccaactcctactacagcaaagataaatgggcatcccgcaacgtgattgcttccaacatcggtctcatcgccaaaagaggaaacgataacagcatgctggtggctgtaaccgatatacgcgacaccaaaccgctcatcggagtggagctggaattacttgactatcaaaaccaggtcatcttcaaaactaaaagtgatggggaaggacttgcctcctttgatctgaaacgcaaaccctacctgctcatcgccaaaaaagaaaatgagagaggttaccttaaactcgacgatggcggctcgcttccattaagccggtttgatgtgaaaggagaagaagtacaaaacggtatcaaaggcttcctctatggcgaacgtggcgtatggcgtcccggtgattccgtttatcttacttttattttggaagataaaggagagaaattaccggcagaccatcctgtttcgctggaattatataatcctaaaggacaactctacaagcggatcaatcaacatgaaggactaaatggcttctacagctttgctaccgctactgcaccggatgatccaaccggcaactgggtggcaaaagtaaaagtaggcggcgccaccttccagaaaaatgtacgcattgaaacggtgaagcctaaccgcctcaaaataaaaatggatttcggcagtatcacttccttgtcgaaaggcagcgctacaggcaacttatctgccatgtggctgtttggcgccactgcacagcatctgaaagccaaagtagatgtgtcgctggtacagcaaagcactagcttccctaaattcggggactacgctttcgatgacccggtaacccatttcgaggcagagaacaaaaccatctttgaaggcccgctgagtgaaagcggcagcgctcccgtgaacgcagatattcaactgggtaaggtagcgccaggccagctgaaagctaactttgaagtaaaagtatttgaaccgggaggagatttcagtatcgaccacttctccatgccttataatcctttcacttcctacgccggcatacgcattcctgcaggcgaccggactaccggcatgctgcttaccgaccgcccacattcgatcgacctggtagatgtagacggcaatggcaatctcactaccggcagccgtgaagtgcaggtagaattatacaagatcaaatggagatggtggtgggatgaaggtgaacaggacgactattccaacttcacacaagacagctataaccagttactcagtaaagaaaccgttaccctgcagaatggtaaaggtaaatgggaactgcgcgtaaactcgccggactggggccggtacctgatcagggtaaaagacctgcaaagcggtcataccgcaggtaaggcggtgtatatcgactggcccggctgggcggaaaggatgcagaaggataatcctgctgaggcctccatgctggtgtttacctccgataaacaaacctacaaaaccggcgatgatattaacctcaccattccaagcagtgaaggcggccgcggactggtaagcattgaatccggcagcaaagtgctgaaaacatactggatcactaccaaacagggacagactacttttaaattcaaggcagaaaaatcgatgacgcccaatatatacgtgaacgttagtttgctgcaaccacatgcacaaaccctcaacgatttgccaatccgtatgtatgggactattccgatttccattgaggatccgggcactatcctgaaaccggtaatcaccatggccgacaagctgaaacccgaaacagaagccagcatcaccgtaagtgaaggtaatgggaagccaatgacctataccatcgctattgtagatgaaggcctgctcgatcttacccgtttcaaaacaccagaccctcataatgcattttatgcaagggaagcactcggcgtaaaaacctgggatctgttcgactacgtaataggcgcctggggagcggatatggaccgtatcctgagtataggcggtgatgaaggattggataaaaatgccggtggcgctaaagccaaccgctttaagcccgtggtaaaatacatgggtcccttctacctgaaaacaggacaaaaacaaacacataaatttaagctgccgccatacataggatcagtaaaagcaatggtggtagccgggcaggacggcgcctatggctttgctgaaaaagcggtagcagtaaagaaacctttgatgctgctcaccaccgcaccacgtgtacttggtccgtcagaaaccatccaggtaccggtaaccgtgtttggcctggagcctaatatccgcaacgtgaacgttagtttatctaccagctcattactggaagttgtaggtgaacaaactaaaacggtgaccttctctcaacctggggaacaaattgtatacttcgacgtaaaagtgcgtccgcaaacgggcgtagctaaaataaaagtaacagccaccagtggtgcagaaaaggcagaagaaaacattgagctgaatgttcgtaatcccaacccggtgatcaccaacattattgaaaatacgctggagggaaataagagctggcaatctgctttcagcccggtgggcatgacaggcaccaactccggtgtgctggaagtatctaccattccgtcgctcaacctgggcaaacgcctgcgattcctgatagagtatccacatggctgtattgaacaaaccacttcgggcgtattcccgcaactggtgctgaaccagttgatggatctgaaagaaagtcagcgggcagaagtagaccgtaacgtgaaagcgggtatcaacaggctgaaaagtttccagacttccgacggtggtttcagctactggccgggtgaaggaaactctgatgagtggggtaccaactatggcggtcatttccttatagaagcacaggcacaaggttatacgttgccagcgggattattggatcagtggaagaagtaccagcgtaataaggccggtacctgggcgcccagcacccttaatttctatggtggagatcttacacagtcgtaccgcctgtacctgctggcactggccaaatcaccggaactgggtgcaatgaaccggttaaaagaattcaaatatctgtccgttccggccaaatggcggcttgctgcggcttataagctttccggtcagccggaagtagccaattcccttatccagggacttaccaccgaggtgaaagcgtatacacagttgggcggcacctttggttctgatctgcgcgacaaagctatgatcctggaaacgctcaccatcatgggacaacgtaaccgcgctaatgaactcgtgaaacaaattgctgcgcaactatcgcaaaacgatcagtggtacagcacacaaacaactgcttattcactgattgccgttgccaaatattgcggcaacaacaagggcggcagcaagatgagttttgcgtatactattaacggtaccaaaggcagtgtaaacgggcaatcttttgttacgcaaatacctgttgcggtcaacggcagtgcgggcaatatcagcatccagaataacgggcaaaatgtgttgtacgtgcgccttatcctccagggccagccggatgctggtcaggaacccgtggctaccaataacccggatatattgggcatgcaggtaagcttcagtacccgcgatggcaaaccgctagacccggctacattgcgccagggaagcgattttatggccaccgttaccgtcaataaccctggtaaaagagggtactacgaacaaatggccctgtcgcaggtcttcccttccggctgggaaataataaacacccgtttgatggaaaacgacagcgcgttccattcttcaccagctacgtatatggatatacgtgacgaccgggtatacacttatttcaatatagaagaaagcaagaaacgtacttataatgttttgctgaacgctgcctatctcggcaggtattatctgccggcaacctcttgcgaggcgatgtatgataataccatacatgctttcgcaccaggcaagtgggtagaggtagtgaagtagaaaaagagatgctcataaaaaatgcgttccgggatttccgggacgcattttttatgagcaaattactactgttgtaaccgggcaaaatagatgacggtacgagccaactgtgatacataactcatctcattatcgtaccaactcaccactcttacaatctgttgctcccctgcaggtaaaacttttgtttgagtggcatcaaagagggagccgtagcggctgccgatgatgtcgctgtgtactcttcaaatccgttgatggcaatttttttgtgcgacataaaatattttttagtaattatctttttaagaaatcatgtatcagggcagctatttcctcatggtattcttccagtgcgaagtggctgccttccagtaagtgaacttctgcattgggtacgtcttttttataagcttctgcgccgggccaggtaaagatgcggtcgtgtttgccccatactaccagcaggcgtggctggtgggtacgcaggtattgctgccattcagggtacctggggaagttggtgccataattctgaaacaaggctacctgtactgcttccacgccgggcctcgacatataggcatgtgccagttcataactgtcggggctcacactttcggggttggccgcgcccaggagatgttcttccttgattttttccaggcttaatttatgcacaatagctgccagtaatgctttctcatctccggcctgctgcaatgcgccaatttcctgtacatccgggcccaatccttcgttatatacattagcgttttgaatgatcagcgcttccaccagttctggtcttttactaatgatgcggaaggcaacgggaccgccatagtcctgcaggtaccagctgaattttgttaatcccagcttgtcgataaactgttctattaccagggccaggttatcgaaggtataatcgaatgctgattgcgggggaatactgctttgaccaaatcccgggtaatccggggctattacatgatacctgccggccaggtcatggatcagatcacggtacatgtgcgaggtggatggaaagccgtggagcagcaatatcacgggcgcgtctgccggaccggcttcgcggtagaaaatattgagatgattgacagtaactgttttgtggagaacgggggtagtagtgagtgtttgcatctgaatgttgtttttgtactatttggtacattattagttaaaaaaatatcgtttgtggtgggtgtttgtttatgattattgcgtgaagtgtgtcatatagaagtaatttgctgccgtaaagatatatactttaccaattagtacaaaatatatttaaaaaacaattgagtagagaaaaacgggcaaacaatgtaatctgactttttaaactgatcgcgccggcttccgcagataatttcacgaataatcatggctcagatatcaaccagcagccagggattgcatagccatcaactccagggaggggctgcggtacgcatatcccctaattcatcagacacagatagtttaacttgatacccggaatctcttcatcaccgcaattacgccccatgtacccgctaagaacgcagctatggcaatgaatagtacagattgctcccgtaaggggttcaaataataaagtaacaggaggttaaatgataggaggatacccaaaatgaattttcctatccaattgacaggtttaaaaactgcagctgctttttccttttgttgctgtacaatggcctgcattaaacgatgggagaagaattccgacggcttttctatgccgtcttctttcaggatagccgggagcttatcttctgacacattattatttttcatagtaaatttcttgtttcatggtttaacaataaccctaattcggcttccagctgtttccttcctcttaataaacgcatctttatggcagactttccggcgccaaggatctcacagatttcagcaatattcttttcctcgatatagtggaggatcagcaccagccggtcttccttcgatagcctgttaagcgctaaggtgacgtatctttttctttccgcgtcctttaccagattccatccatgattttctgtagcctcatcctgttcggtttcgggttgttggtctatactgacagtaggcgttttcctgtttttaagttttgtcaacgccgtattataaacaatacggtatagccaggtagaaaatctggacgcctgtttgaacttacccagcgctgcaaatgccttcataaaagcatcctgtactacctcttccgcgtcctcattattggtaacaacagattttgcaattgtaaaagaaaagtccttataggtatttaccaaatcggcaatactatttatatcgccatttatggctttattccatatttcattttcctgtttattttctctgtgggttgccatctcatgatttagactacctggggggcaaagtggtcacattgtgaccactttggctttttagcagtcttattattaggaactcaaaaatatctaaaaatatagtcatgcaaataacgtccgcatctttaatcatttcgcttgcacttgtcgttttcgggataagttattactatttcacaacaaggtataaagagcgaatgaccattattgaaaaaggactccctcctgactattttaaaggaggtaccaactacctgttatttatattgcttcttggcattgtgagtattggcatatccctgggagttgtactcggaacttttttgagatcattaaatattgatggaatacgagattttatactgccggctaccatattcctgtttttgggaattagtttgataatctcctattttgtactaaagagcatagataagaaaaagtaatacttcctgcttcatttattgcagccagaactggcgggttaaacccgctaggggaagcctttgctcttttttaaggattaaacataaacaccatgagaaaattattgataatagcgctgtattccatgttgatatatctgccacttatatcctttggtcagcacctggaaaaagagctggatgccatgttagcccggacgtttccatccgcaggcccgggagctgccgtgctggtggctaaagcaaataaaattgtttacaaaaaagcatttgggaaagctaatctggagctgaatgtacaattgaagtctgatcatgtattccggataggttctattaccaaacaatttaccgcctgcgcaattttaaagctggcagaggaaagaaaattatcgttgcaggatgagatcactaaatttatcagtgattatcctgtgccggatgttaccattgaacagctgcttacgcacacttcgggaataaataccggtgcaggcgcatggacagctgaaacaagaaagcgcgattttactctgcaggcgctgattgattcctttaaataccagccgtcagactttttgcccggcgaaagtttccgctataataataacggatatgtgctgttgggctatattattgaacgcatttcgggtatgccctatgaagcatatatcagtgaaaatttctttaaacctttaggaatgaaaaattccggctacgacaatactgcgtctataattccccgccgcatcagtggctatcagaaagacaacgacgcatataaaaatgccgatttcctaagtatgacacaaccctattcagcaggttccattctttctaccgttgaagatctgtacatctggaataaagccctgatggatgggaaagtgatcagtagaaaaagcctggaaaaagcacatacctcccatcaactgaacaatggaaattccactggttacggatacggttggtggctgggaaatatccagggaagcctggatattaaacacgatggcctgatcaatggattctcaacattcgctgtttatcttccgcaggagaaagtatttgtggctgtttttaccaactgtgaaaacaataaccctgaagtcatcggatcaaaaattgcgggcatcgctatcggtaaaccttatcacaccaacgaaatcgggttgcccatagcgcaacttaaatcatatgcagccatctatgaatcagcaacagagggacaaagaaccgtatcttatgaagatggacgactcctgtactttgtaaaaggaggaccgaaagaacagctgatcccctttgggaatgacaaattttattttgagaacaacctggtcatcatagaatttttgaagaagaaagacggaagtgtcggcgggctcgtttctgaaacggcagggaaagcggttacattcatccggacaggtattaaactgaacaacctgtacgcgataaatattccccctgaagcgctgaaaagatatattgggaaatatcagtttccggataactttattcttgccattacccgggatggtaaccggttatatggcacaggccccggtcgcaggcaaatcaggcaggaaatagttccctatgacacctgcgggttttttgcaagaaatttagatgcgcagctggtgttcatcctggataaaaatggaaccgttaccggattaacaaaaattcaaaatggtgtagctgtcgcagagaaagtggaatgagccgccggtctcaatacaactgattacgtaaaattcttttgatcatttgtatagtggaacggctgatctggcctttgtatttttggagaatagtactttcactaacgccatcactcagctcgtttactacccgcagccatttgccaaggaattctgaattgggagtacggtaccgcattaatcgcctcaccgtttcaataatggatttattcactgtgccttcatgaagctcaaatacctcgtcattattaagtcccagcttaatgtcatcagcaatcctggaataatcctgcaggtatttttcattggcttccattacctgtaacaggggattatcgctgaaagcaatgtcagtatacttccggtgctgcttctgtaaggcctgcaaagcatagttccgggcaatattatcgcagatgatgaggtcgctcttgctgagctcaaaccattcgccttttacacgtttatgctgaaaaacaatatgcagactctcttccaggtctgtcatattcaacgctgcatattgcctgataacacggaacattacgggcaggtgtgtatgataagccgccagacgcttatgcaggtcctgcgttttaccgatcttatacaggtttttacccgtgttcagaatgtacacacacttaccaatttgtacttgctccatgaggtgatttcgcgcttgctggtgataattatgttatcaatttacgactatgattcttatatacaaaatggaataatcatcttaaattataatatgaagtgtatgcggcgcatagaggagcatcacctgtgcgcagtgtggttgttaaacaatgatcttatactacgatacagatatttgaaatcggcgctattcctgccagttactcaggtacctcgcggtaaaattcagcccattggtatacataaacttcccaatcacttcctccaggtaattcatatccagtgatccgtctgcaggattgtagcgaagtgagcgcgcattgataccatctcccgtattcagatatttatcggcaacgggtaaatatttttttaacccggcagccaggtcggataatttcaggatattatctatccggttgataggattaatcagtccatcgaaatcagagccaatacagatatgatcccacggtgaagtaccaggctcccatcccatgccggcattcccgatccttacggcataaataatgtgaagacacaacagcatcaggtgccgctccgccctcgaaggaatgctcaggaaatcaaataatttctctgcgcctggaagttgaccatccctgaaaagcttttcccattcttcccgggcaatgtattcgggatcaaaatattcaggccggttactgtcaaccattttttctgcacccaggatgcgctggtcaagactgataccgatcattccccgcgagctcatgatctctataatttcttcatcgaataaattgatagtccagggattgccataaagaccgctattaatgctgtcgtttgtttttccgattttccggttttccgattccactatactcaccaatacgccatcctgctgaccagtggtggatctgaattgttttttagcgagatagttattcaatgaagtgaatgtgaaaccagtgtgagaggtgatgatcggcagcctgttgacggctggcgattcattgatcagcgattcgcggtaacggtaataatgaaaccgcgtgtatacgctcatatgtttcagatcgatgagcaccggtctcttttcatgcagcagcgcctggcgtattaccttttttcccagctgtgtaagcccgagaccggctttaggcatgaagtcctcgctgctgaaagctatttgcgcctgcttgttaagtccctgcgcaaacccgcccagcggctgctccgggatataactgaggtgacagagattaatactgataaaatccagttcgctgttatcctggatatctttcaggtttagctccggcgtcctggataacgcagcgccccggataggtacgtcggataaattatgaccgccttctatagaaaagatgaggtagcgttgtgtgctatcatctttcagcacatctgctatttgttgcgccgttttaccttcccaatctttcctccccgtatattttatatgatagggcgcctgttccaggatggccttactatccaggtacatttttacctgttgctgaaactcggcgtagtagctggttttaccatccctggttttatttacgatgtctttgtttaaaggtaatatatgggagaagtcgatgccgagcacatgcaaaattctacgggcaaaagcatgttccaggctgataatagaagccactcccagatagagctggctgtctttcacctggtcgggtgacgactggctattaaacggtccgccgaaaagatcgttcagcaaactggccaggccggtggttttcacctgctcatttataggggtaccattgctgagataatgtttaaacagcagatgaaaatgaaagtcgaatatcttgtttgtcatggggtcacttatttagcggcattttcaataatagactgaacggtgttaaaccgttgaagcagatccggataggtggcaggagtggtgctttcataggcgcttctgctttttccaaaggtggcgctttccagcatccgcgcgctgtcggacattggagtggaaatagcggtgagcgattcctggttgcctcttctcgtaccaaaaatggcattgtgaagtttgttccagtaagtttttactatttcgccatagccctgcagcgagttcaggaaagcgctttcgttccagccgttgtattggttgtttaatttgccggcaggtttagggggagtgtttagaagtttttctgcgttgagaataccacttccaaaacctttcgtgggtagttgatcgcttttgcgggcagagtctttcagcgcctggcggaaagcttctactcttttccagccggcatattccggcgccctgagctggtcctggtattttgccaaccagtaggctgctgcggcggcaacatgcggtgtggcgtagctggtgccatcgccatatgcaaaaccttccaggtggtcgcctgccgcctgccagatgggtaccagcacatcttctcccggcgcagtaatatctactgtatctcctctcgaagatccggtccattccctgtccagcggattggatgctgccaccgcaatagtgccggggaacacagcgggcgctactaccgcctgcacgctgttaccggctgcacagcaccagataacgccactttcatatgccttttttgccagccgtgcagtggtgagcgtagggggaatgcccatgctcatggtaatgatatcaaaaccctgggcaatggctgcatccaatgctgctgccagttgctgctgcctgttgatgatgactactgtttcggctatacgaaagggaaccagtttgtaattatcgggagccagtaagccgcagttgccgttacctgccgcaggtgaaaagtcgtggccaattaacaggctgccggtacgggtgccatgaccgggttgctttcccagcgaaatggtgcgcaagtccagcgcgtcattggtattatcgaggaagttataatcgttgtcggtgtcaaatgcaccggctactttggaatggtcggtataaccggtgtcaaactgtacgacacggatgcctttttcatgaggcgatgcaggtgtttgttgtgtcagcagtatcttatcgaacccggtggcgtaccagttccaacgccggtactcttctgctttccggccggcaacaaatttgctcacagccgttaccgtataatttttcaggaaagcatcttcgttgggcgtgccataaccgtcgtcaaacagaaagccggattcggcaggaccgccacccttcctgataatattaacggtatcggcattcaggtataaaggcagatctgcttctgcataaaagatgcctggtacctgtgccagttttccggcttcttcatgtgcgttgccactgaagttggtggtaaacgtaaacaactcttctttgccggcaacggcggtggcgggtgtaagcaacgacagcttaatgcccggcggatattttacagataataccgcttctatctgcgacaccgtttccggtttattcaatgcagagattataaatgcggtgggagtactaatattggcagatgaaggaacatccatagtattttctttgggagatgaaggaatatcgggaacattggatggagcgctgttattgctcatagtggcagctgttactacattgtttacaccgctacggacgctggcctggtcgggtaaggcctgcttcagctgcggtgcaatattgtcggtatcttttaataaagcgcggcggcccttttccatatccggacttaacgtggcttcccgcacggcgctgacaattacactcactttaattccttcattgccgatccagtcaatctcgtcgtccggtgtttcaggggtggccagttgcccactccgggtaagtacgcggttttgatcatccgtgcgggaaagcccgctgtgatggagggcaatgatctcgcaggtacccattccgaacaccggggagccgctgctaccggggagtgtatccgattcatataccaggcgggtacctgtttcagagaagaagcggatatctttcagtaccacttttttaggcaggccgttggggtgctgcacaattacacaggattcgcctttaatgattttgccgaggttgccgtcaagacggataggcggaaactgcgacagtaattcaccgaaagtgccggtcaggcttacacctatcagggtgaaatcgagaccgctgttcagcgtagttttacttacttccaggctcgatgtcataaaaaacttgcgggcatccagtttgaaggaagcgcttcttttcagcgcttttgtagtagcgtccacttcatagttgaattctgcaatcatgtcttctgcatcatcagccgattcaatcacatggtggttggttagcaggatgtcttctgttacgaggaaaccggtgccaatgggcgtcccgcctttcaggatacggcacacggccctcgacatttcagataacctgtccagtacatatttgtcctggaagtcggccgtgcctgtaatccgctccagcgcagttgccaccaggggcgtgttttcgcgggccacacgatattgcacccgtgtgggattatcttccagttgtactaaaggctgattggcttcccgtaaggcacacagctttctttcggcagcttcaaactgtggctgacggtcaccaaaacgatttgctacttcctggataactttccaatgaggtatcatttattgagggtgtttatttggggtagtacacttaggttttcgctaatgaatttaatcaaaaaagaagggaataaaaggtcatttgaaatatcttttttattataaaatgaaaagagcggcatttgtaatgaagtaatacttccgggcaacaggttggcggcccggaagcaggagatttatccgtaaataatgaaccctttttcaatggaatttatcttccggaatttaatacggaacacgccaatcccgttactgctgccgttggggttgctattgccttcaatggtttcaataaagccaccatttacagcggttacaataccggtatgaccgaagccgccaccatggcttttaatgaagatgctgcccggaactatcagggaggggttgttgatagcctttgcggtggtgattttcagcgcttttgttttgttccagtggtccaggcagccggcagttttaacaacgggattagcaatacccaggtctgctgcggcttttttgaagcaccagtacacaaaggccgcgcaccagtagttgccgggaggggtattggtactggccagataggcttctacctgtggtccccggttgctgccaggaggtacttccatcacgccaatctggctttcggcaacttcaatcgctttggcaagtagcgtattgggcgcatttgtttcttccggtacaccatcgtcaaacaatacttcccaggtaatggcgcccacttcaccatccacaataagcggattaccaaaccggtcgcggtgcagcgcctggaattgttttacggcagacacagttttagggccaaaggtgcctgtgccctgtagagtaccgataccgagttcaatcagtctttgttgaatggcttttacaatctggctgtttgtttcgccagccttaattactttgttggggtaattcataacaattgatttttaaaatttggggtaagaatattatttcacaatggttttatactgttatgggatagctgtctgatgaatcttttttggagttatctaaagataacaacttcccggcattttaaaaaccgggaaaaaggaggccgcttcatccccgatgaagcggcctcctttcatttattgaccatatatctttagaaattggtattaatgatcagcgtgttccggtcggccgctgcaaaatccatcgggataataccatatctgccatgcgtgttactggtaaagtaagtgttgatctgtggattaatggcatttgaaacggtagtaatgctgggaataccaaagatcagggatttatacccactggtgaaattgatatatagtaccgactggctgccgttctttgcctctgtgagcaggttggtaatgcctgtccatttcgcgttattatcgggtactacatactggtcctgcacccgcagggaggagttggtgttattgatagaaaacgtggtattatcggcccagttggtggcttcaataccttttggggtactggtggcgccaaatctcctcagcagcacaattttgccccttacctggccgaggttgggaaccgcatcgcttagataccatttggaaggttgcagctgcgtatagctgtcgaaagtttgctcaaaggagcgggtgttgttggtaggatcatactcttcttttacgcacattacaatcgtttctgaaggatttgctgccaggaaatcataacaggcggtaagtacgtccgtaaaattgaggttctggtaaatagaaccgtggtgaatggcgaaagcatcgccgatgtgccggcaacggatatcaaggaagcgtgtaccggcatccagttgttcgcggatgctgaggttttgacatttggcggtgccgctaaccggttccacacgggcgccgctgtcgtgtgtgccgggaatagacagggccgtgagactggtattgtctgcaatggcgctcatccagccggtaagagttacgcttaaagcgccggttacagcgttttttgtcattgcttcaccgccggctgcagcatcaggaattgccaggtcttttttacagccaaaaagagaaaggatggccagggccaccaaaagggttttcaggttcataatggaagtatttatattaaaaatacaggagaatactgtttggttcattgcagtggaaattaattgttggttaacaatccgtgatgtggaattaacatttccggcaggtggtcgaaaggtgtgattttttatcagcacaggaatgcatacctttacgttatatcaaccagattagcttcgggggaagcacttacatttattttgaataccgtgcaattaaatagtgaaccagatttactattcagggtgtcgcagggcgatgaggctgcctttgcacatttatttcatacctaccaaaacaggctgggagcatttgttatgcagctgacggggtccaaaccgctggccgaagagattgtacaggaaatatttatccggatttgggaaaaacgggagaagttaaggcaggtagaacattttcatccttacctgtatgcagtagccaggaactatagcatatccttcctgaaaaagcttggccgggaactggccaggaaacaggcatgggaaaccagtatagcggctacccacgaccaggaagatgatactgttatccggaattaccgccgcatcatagaccaggccatttcagaactgccggcccagcgtcagaaagtatatcttttaagccgggatgaaggtctccgccaggctgaaattgccgagcgcatggccatctcactggaaacagttaagaagcacatggtactggccctgcgttccatccggagttatgcaatgacccatccggaaatcaatttgctgatgcttattctggccacacctttcagggggtaaattttttttcttacaccattacctcttttttatacttgttgctgtcttatagggtagaatcaatctatgctgatggataataccaggttgcgctacctgcttagccgatatgcgggtaaaacaatcacccaggcggaacaatccgagttaagtgattttttaaatgcggcagataatcaaacgcagctggaattgctgatcgaagaagcctggatacagtccggtgaggaagatgaaatgttttttccctcgccccagctgaaccaggaaccggcgcggcagccgcttaaatgggtttactggcagcgttgggccgctgctgtattattattgatcgtcgccaccagcatcttgctgctggtcaccaaaacacggaaagcagataagttaccagctgtggtaacagaaaatataaaaaaagatgtgaaaccgggcggaacaaaagccatgctcacactggcaaacgggaatgtgatagcgctggatagctcactgaagggcacactggcgaaacaagggaatgtgaatttacatgtgagcccgggaatgctgaaatacgaccaaaacaagcagacagctgctaatagtatagcctataacatattaaaaacccccaaagggggacagtatcagctggaactgccggatggctcaaaagtgtggctgaatgccgcctcttccctgaaatttccaactgcctttgttggaaaggaacgccgggtggaactaaacggggaagcctactttgaagtagccaggaatgccagccagccattttttgtatccgttaataacgccagtatcgcggtattgggcaccagcttcaatgtaatggcttacgccgatgaagcagccatgagaactaccctgctggaaggcgccgtaaaggtaagccaggcaaatgcttccagtgtattaaagccgggagaacaatcactgctggaaccaaacggcaaaatgaaagtaatagaaaatgctgacgtaagcctggcggtagcatggaaaaacggacttacttcttttaaaagtgcagacatcaaaacaatcatgcggcaggtggaaagatggtacgatgtggaagtagtatatagcggcgcaatacccgtccgcagcttcacaggagatattccgagagacgcgaacttgtcagaattattgcgattactggaaatcagcaggatccattttaaaatggaacaacgcaggctgatcgttatgccgtaagtatcttattcattatatcaaccaaattgctattaccatgaacaaaggtccctgaatgacgtgtggtaagaaccggcataaaaaaccaggagcgatctcacccgcccctggaaaagagcctgggtctggtacctgacatcaatacttatcagaaatcaagatttatctcaacccaaacaccacaaatgtatgcaatctaattgtcatgcaaagcccgtctttgtacctgggctattatcaaccatcaaagatcgcgtcctgacattcagaaaatcaggtgcccatctgaggataaaaaaacaactgattaagcaaatgaagattacggctatcctcttaacggtagtttgtttgcagatcagcgccaaatctctgtcgcaacagataaccttgtcgcaaaagaacgcaccgatccaaaaggtatttgaagaaataaaaaagcaatccggctataagttctggtatgaagatgctatgctcacgaaaagtaagccggtagatatctccatccggaatggttcgctggaagacgtactggcactgcttttcagaaaccaacccttcagttatgaagtgatcggcaaaatcatcgctgtaaaagagaaagatatcaggctggaaaatgccactcccttcatcgccataccggaagtagtactccgtaaaataagcggtacggtaaaagacagcaccggaacacccatccccggcgtcaccattctcatcaaaggcactaaaaacggtgccaccacagatgtacagggccggttcagtcttgatgtgccggaaggcaatgtagtactggtattcacctctgtaggatatgaatcaaaatcagttaccctcggcacctccacattcctgaacgtaacactttccattgcctccagcgggttgaatgaaatggtggttaccgctctcggtatcaaacgcccgaagggaacactcggatacgcgatcagcaccattaaaggcgatgaacttaccaaggccggttcaaccatgaacccattccttgccctgtatggtaaagcagccggtgtaggcgtaaacgttggcgcatccggtccgcagggcggcgttaggattaacatccgcggcgcagccagtatgaaccccgatcagaacgtaagacccctgtttgtggtagacggcgtaatcctgagcgaccgtaaaacacagataggcggtgacgtggggcagggattcgactatggcgccggtatcaatgatattaacccggacgatatcgaatcaatcgatatcctgaaaggcgctaaagcgactgtattgtatggtagcgatgccgccaacggtgtaatgatcattactaccaaaaacggccgtaatgtgaaaggatttggtatgaccggtaacatacaacacaccatagaacaaccggtatcttacctgaagctgcaaaccaaatatgggctgggtgacaacctttatgatacgacctatgaaaccatcaatggcgtaaaaaccaggatgctgcccaataagcgcttcagcttcggtcctgctttcgatggtgccaatgtgatgttctacgatagttccatggtgaagaattcgccgcatgcgaataactttatgtcactcttccagaacggtcactctacttctgccaacgtagcaattgcaggcagtaatgaaaagggtagtatcagggcttcttataccaactataattaccaggatattgccggtgataattcctggcagaaaaggaactcctttagcttcaatggtaatatcaaagcatccgaactggcttcctttgaagtgatctccaacatttacagcatctctacccaaaaccgccgttcccagaacgatggaccggtagcatggggatacccggttgattatgattataacctggtatatccttattatacagatgccaccggctataaaagggatctttccaatgcacgtgtatccgatgcctttaacttacttggcaactatatctggaataacaaaaagaaccgctacaaggatgaaaacatccacatgattacctctgccaaagtaacattaaactttacgaagaatattttcctcgtaggacaggcggggttggattatgataataccaattataatacagaggtaagtataaccaggttgcttcccacggtagacaaaggaagttttggcgtagcaaaggaaaacgctaccacccaaacttaccaggcgttactgaactataataaatcattcctgaacaacgatctccgtttgttcgcatttggaggcggtgtgtaccgcctgcgtaatgtggattacctggccaccagcaccgttggtggacttaccttccccgattggtattctttctccaatcagctgggaacacccagtgccgacaatgcacacctgctcagaaactatacaagaggttctgacgtattatatagcttgctggcctcagcagcactgtcctggaagaatgaatttacattggaattgcagggtcgccaggactggaactctactcttcctccggaaaacaacaagtatttttatccgggcgctgcacttacctggaattatacagaacgttaccggcttgccggcgtaaacagtggacagctgagattgtcctgggcggatgtaggtaacggcactacccgttatttcgccaataacctgtatggatacactcgtctgccaagtacaggcgccaactccgtttctcctcccgacaaattgttaccgggcgccctgaaaccagagcgtaaaagggaatttgaaattgggatcaacaacaccttcctgccacaggatagggtgatcctcgatttctctttctataccaaccaccgctacaaccagatcatcagcttacctatttcttcagcctccagttccactggtctgatcgtgaatgcgggtgatgtaaaggcctggggttttgaactggcattaacaggcgtaccactggtaggtaaaaactaccgctggagcctcaccctgaatgccgccagccaggcatcaaaagtaatagacctgtatccgggcgttaccaattatcctttcagtaacctgattaatggcgctgctgcatctattcatgcagatgaaggtcgcccgtatggtgaaattgtaatgaacgattataaacgtgatgaagctggcaataaagtagtcaacaaccagggtatctatatactcgatgatcagaaatcaaccgtagccggcaatgtaatgccaaaagtatacggcgggtttatttccgacttccagtataagaacttcaacttccgtatcgggctggattacaaatacggcggtactattttcagctacaccaacaaccgtttaacaggtgttgggcagttagaaaataccatgaaataccgcgatgaagaaaacggcggtttggcctattatattaattctaacgaacagaacgtgccgtggcagcattcacagccagcgcctgctcagtctgcggatggtaaggtgtatcacgatggtctggtcctgcctggtgtgaaaattgatgataatgggaagtatgtaaccaatgatatcatcaccagtgcttcttcttattatggaagctatgcaaacgacctggctacctctttcccaccggatcgcgtattcaaaaacaattacatcaaagtgagggaagtagcgctttcctatacattacccgcggaaatttccaaaaggataagaatgcaaaggctcactgtcaccgcagctgcccgtaacctgttctatctctacaaatctattcccaatattgatccggaaggagcgctgggtgcagatgttttcgtggaaaataccatctacccttcccaaaggacttactccctggggttaaatgttgctttctaatgtataaactgaaaaaaatgaaaaaagcttacttatatattttcctgctttctgcttccgtcctgggagcttgtaaaaaagacctggaagaccggttctacgacaaagacaagctctccaccggtagtactatagatgtggtgcccggcttatttaccggcgtgcttacaaataataaaatatttgcacaggactacggcgagtggtattacctgctcaacggaggtaccagtatcaccggctatgagcaagtggtgcaacggtttgtatcttatcgctacgactggttctccacatacaatgatttaaccaccggtaacggatttgatgattctcccatcaacgggcaatctttctttcaacacagttatacccggttgaagaattatgaagtgatcagggattctgtgaatgcacgtaccgggcaattgaaacaggatggagatgtatacctgaaactggttagctttataaaatgttaccaaagcgccaagctggtagatttctttaattcggttccttattcagatgctttccagggagcaaaaaaagaacctaaatacctcttccctaaatatgatgatccaaaagagatctaccagtctatcatacaggaactgggagctattgtggatgaactgcccgctgcctattcacagatgtcggctgatgccaaaaccgtatttacggagcaggatatagccttccacggtgatatcaataagtgggtatccctgatcaattttacccgcctgaaattgctggtaagaatcgccggagtggaagaagcatatgccaaaccgctgatccaggcagcactggctaagcctttgccacaaacggatctttactggttctactggtttgatattgatcccaccggtggcggaacatggattcgtggggtgtatgaaaataccttcgcctcctttatcccgaacatcatcatgaaaaggatgaactacggcacacctgcttaccaggaagggattgatgatccgcgcctgcccgtgctggctatgcctaccaaatacctggattaccgtggtgtatctgctaatattgaagaacaatctgcattgtataacagcggagaaaggtattatccgtatgcagataatatcgcttctactttttctaccaatgccaaatctacttacaaccatgctaccttccaccagaatgcgaagatgccggtttatatgagttcattgggagagctggatctgctgctggcggaaatagcgctgaaaggattagcgaataccggcaaatccgctgaagaacacattaaagacgaagtaacacactcgatagatttctggtacaccattaatcaactgagcagctacgctaaaactcagatgacacctcagcaaacagccatggtataccctacgaaaccatctgcagcagtagtgagcgcatggggcgatgtggttaaagccaaatttacactggccgctacactggacgacaaaatggaaatcctgatgcagcaaaagtatattcacctgaacctctaccagccttacgaactgtgggcagaactgagaaggacccgtcacccgaagttggaacccttcacctggcatacttccgtatggaaaccaatgcctgaaagagtacgttatccaactattgagctgaccaataacccggataacttcaagaaagtagcaggagaaaataatttaaccagcccgattttctgggtgcctgctgcagcaagagcaaaaaatccttactgggataattataattatcaatagcagagagcaatgatgtcgatggggagctgaccatattggttagctcccttttttaatgccataccgctatgcaggcggctgccagcgttgacgccagtaacgcatagtaagccggctttgtaaatactttgtttgtgaaacgtatattgatgaacgttaccactgcgaacaggccggttttgggtatcactttgtaataattgacatgcggatatttcagcgccaccagtatgataccggttaccagcagcacaatgcccagtatcagtcctttatggtcgcgcacttttgtatggtaatcggtccgctgcgccaccaatatagcgagatatcctaaaaagcatccgaagtgcagaagcaacacaatattaaagagcatgggatgttttttgggcggtggaagaaagataataacctcccagcaccagcgccattacaatagctaccacgtgcggaatcagtttgccggtttcatatacgggattttgcaacaccaggctgaaatccaccaccgggataatggctcctgccagcaatagcactcccaatgcacggcgctcgccggtccatagtacgccaagtatagcaatgccggtaaacagatcgcggatgcctttgatataatgaaaagagaaattaccgtttacaggtacgtggatgccaaaagcagcttccgccaccagcggggagaggaggaagcgaagcccgataaataccagcaatatccccatagatacggtggcgtaaaaggcgattttttcagatgtgtttttcatttgtcgcattattttatgatgatgcaacaaaggtaaaaacagctttccgcgggttcgttcacccaggttaataaatctacatcgccagccttttcctgatccggcttaaagacggaggctttacgcctacaaaggaagaaatataatactgcgggatgcgctgctgcaggtcgggatagttgttgacgaattgcagataacgttgctccggctgatcgctataaatagaagtgattttttttatggcattcaaatacaggtactcacaaatcaaccggccaaatttttccccttcttttattttgctgtaaagcaattgaagattttcataggaaatcgccagtattgtggttggctcaatacactggatgctgcgctgcgaagcagaatgatcgagaaaactttcgtaattacaggtaaattcattttcctttccaaagtcaaatgtcagctcctccccggaatctttgatgctgtagtaccggatcaatcccttctcaataaaacccgcttcccggcaaacctgtccttcccgcagaaaataatcattcttctggtattcccggctcacaaacaacgaggaaatgaatagcttctcggcttcatccatacggatgaaatgttccatagccctgatcagattagtgtgtatgctcatcggtaagccggtttatttgtacctgtatgccttgtttttcggtgtctgtttttgccaactgccaggctctatgaaagctcgctttcgctttatcattgtcaatattcttatacagttctcccagcagcacataatagaaatgattattctccagcttcaacttttctgcttctgccagcgcttcctgctgcccgtttgctttatacagggcaaaagtacggtttagtgctacactgggggagtaattgatcatcagcagcgcgttgtatagctgcaggatctcttcccatttttccggcgtatcctctttcatgcaatgccagtaagcgatcctggcttccaggtgataggaactgatctcattgccttcagcagaaagctgcaggaaataaatgccctggttgatcaatgcctggtcccacagcgcttcgttttgcgcttcatacagcaccacctcgccttcgccggcctgcctggcattgaagcgggaagcgtggaaacacatgagggcaatgagcgcatttgttttgggccggttggttttgtcgtaagccgtcagcattaatcccaggcggagcgcttccaggcaaagatcctgttgcaggatctggttctgtgtctgggagtaatatccttcactgaaaagcaggtagataatatgcaagacattatccagccgctgcggaatttcattttccgggggcaactccatcctgatcttttcttcgcgcagtttttctttcgcccggaacaatcttttattaatggtttctttattggacaaaaaagcttctgcaatttcatctatcccgaaaccgcaaaggatgcgcagcgccagccctatctgcgcttcgctggcaatagacggattacagatggcgaaaagcatttgcagctggctgtctttgatattctcctgcgagaaactcagcgcttcggcatcatccaccagttcctgtctggccactatttcaggcagtacttttttgtcgaatattttatttcttctgaaatgatgtatggctttttgtttggctacggtataaagccaggcagcaggattgggagggagtcctttcacgccccatgtttccgacgcgagtaaaaatgtttcactcacaatatcttctgctatctcaatatgctgcaacccaaaaagtttgctgatcacagctaccatctttgagaattcctgcttaaataaatgcttcagtgattcgtgttccttttccatactaaaacagtaaaaaccactctaacgaaagagtggttttctttatttcccctgatactggttacgaaactatttcccttacttccacacagccctgggcatccagcaccgggcagccatgagccaatgtagtagcttcttccagcgtatcggcctgcactaccaagaagccgccaagccgttccctgatttccacaaacggaccatcggtaataacgcctcctggttttaatactttcccttccgtagaaaggcgacggccgttactcaccagtttgccctgtgcagcaataccgcccgcccaatcctgccacttcttcatcagcgactggaagtcatccggcgataattcgcggtacgcatattccgactggcgaaataacaataagaattctttcatctttttataatttaaatcacggatgaaatatatgaattaatttgctttggcggcaaacatccccggcgtataacttcctgctgaggtacggaaagctacattaagacggttatagctgttaatggtagtaactgctatggtcaggtctacaatctcttcctctgaaaactgctgacgaactacgtcatatacttcatcgggcacatcgccgttggtaagcctggtaactgcttctgcccaggcaaaggcagcccgctcacggtcggtatacacagtagcttctttccagcccgccagcatataaatgcgctgctccgtttccccttctgcacgtgcatctttggagtgcatatccaggcaaaatgcgcagccattcatctgggatacccggaaataaattaaatgctgcagggatttttcaatggatgattttgcaagatatgcacctacgccatataatgcttttactgcgttagctccttttgtcagcagattgattctctgtttcatggttttaaatttttattggtgatgaatttgttcgtttatacaccaataaggatcgggaaaaaggaaattggacatcttccggaaatttttttaaaatattttttaggcagatgggtaaaggatattcaagcatgtgtccggtaaagaagaaccattggtccccatttttcttatgcctttgcagaaaaacacgcaaactaccacgctaccattccggtgagtcatttgttaatcacctcgtttttacaattgtaaaacactccggcgggccggaattttttcttttgacggatgattcaacacaattatccccgcatcgggaaaatgctggccctccttgtttttgtgctgccatttaccgctatatccgtaaaggcccaggaaataagacctttgtacaaagattccattcccaacagtatcgggaaaactgcaccggcagatgcccccaccatcaccatctataagccggaaaagcccaacggggcggcagtgatcatcttccccggcggtgcatacgccttcctggccttcgcagaggaaggcaccaaaatcgcagaagcattcattacaaaaggagtcaccgccttcgtggtaaaataccggctgccctcagatgccaccatgcgcgataaaagcataggaccgcttcaggacgcacagcaggccattaaactggtacgcatgaatgccgcggaatgggggctggacccgcataaaattgggattgcaggctattccgccggcggacacgtggcctccacgctgggcacccacagcgccaggagctatgtgcccaataaggaaaacaccgatctgcgcccggatttcatgatcctcgtataccccgtaataagcatgaacaaggacctggcacaccagggatcaagcatcaacctgataggaaatgatccttccaaagaaaaaattgccttcttttccaacgaagagtgggtgaacaataatacaccaccggcctatatcacgcataccagcgatgatgccgtggtgaatgtaaataacagcatcgccttttaccaggccatgctgagaggaggcattcccgctgaactgcatctctatcccaccggcaaccacggcttcacccaacggttacccgtaaacgaatggctggaccccatggtgtggtggatgaaaagagggggctggattcccaacaccccctgatctgatataaatcatggcatagccgtatgaacaggtcgcgcagcgggcctggaatgcagcagctttatcagcggccgctctaccttgtagtagaagaaaacccctaccgccaccgccagcaccatatgtacgataacggaaagatcggcattcaggaagtagccggtggcggcatatatctgcgcgatgaaataataaaaagtatagtgggtcaggtaaatagaataagaagcatcgcctatcagtaaaccccatttgttattccacagctttgtccatacaccctgcttctccaggaaaatacaacccgccaggatacacgcactgggcaaaccccacaataacacccttttcaaactgccggtgccaccggtcacactgcccagttcagaaatatttccaaagccatacacaatgttataaatataaccgcccacgcccagcaggagcaacagcccggctacgccggcagccacttttacatgccggtacaaccagaaaatgatcaccccaaagagaaactccagcatgatagggttagtgtaaaatatcagccggaaatcagctggcttcagcaactggcccaccgccacaagcgcaggaataacaagtaacagcaataaggttttgtattttgtacggaacaggatcaggaagaagaaaaggaaatagaaccaccactcaaaactcagcgaccagcccaccaccaggataggcgccagccacttctgcgagttcaatacaggcagcataaagatcgtatccctccacccgtaaaggatagccgtgatggggtacatctggtcaaaaaaacaaaagaataccatgtaacacacactggctacataataaatagggttgatccgcaggaaccgcttcttcaggaagtccaccccgtcacgcgcaccaaaatagttactggctacataactaatgataaaccccgatatcccaaaaaagagatctacgccaatagcaccaaagttttcgaggaaataaaatttttgctgatgggaaacggtgaatgcttcctgtaagtcgatggcgtgtacatgtaccacgaggataactgctactgcccttaataactgtatgctgttaatcttcataaaaagggatactgattgagggtaaaggatggcaacaccggtcacttttgtgtaaagcaagttaaaccgggctgctgtaattacacttcagtcagtatcctcctgtcagttacgcgatctgttccatgcttcccggctgattgtaaaccagttaagcatcgtttcgccgtcgtgaaaagtgccgtccaggctcaggcccaccttctctaaaacgcgcttcgacgcatcgttgtttacatcggcaatggcataaatattttccagcccgagccggttaaagccatattccaggcaggcccgcgcacattccgtagcatatccctttccccagtatttttttataaaacgatagccgaggtcgtagtagttaacatggccgttggtaggttcttttatcagttttaatcccgcccatcccacaaactggttggtgtctttttctatcaccgcccatctgccaataccgttctcccggtattgctgccggataaactgaatggcctcccgcgattctgctatggtgcttacgggtttgttacccaggtataaatgtaccgcttcatctgaatccagttcaaacatgccggcggcatcagcaggtatcagttcccttaaaatcaaccggggggtagatgcgaaaatctccatacacgtgtcatttgccgcccaatttaaaggaactatctataagaacaaaaattgggagtacttacctggtcatcaacaggaaattacttcctgcttctgcttcagtcgattttttctggtactggtaaggagagaagcctgcaaactctttgaaggccctgatgtaatgggattggtcagcataatcatgctcaaaggcaatatcagacaacttgctgtagttgttgctttttaattgcttcagggaattttgaaaacggcatatccgggaaaataatttcggagagatgccaacgccctgtttaaaccggcgctcgaaacttctttccgttaactgcaactgctgctgtaagtcctttaacggaatactgccgccggatgcaatgatctgcgataaggcgaagtgcgtcacctcatcggcaggcgtgctgttttcatttatctgcttaaataaaaaggcagcaataacggctatcttctctgttaatgaaggcgtgttgccaagcctttctgccaggtaaaaatccctgctagccgacagtatatcaaggtctaaacaggaattggttaactcatcggcattcaaaccaaaaacagatttcaacgcatgcggataacagcacaccccaatggaacagatagtgccggttacatgcagctccgtatatttcgtggtttggccgtacaacaacaaatcaggcaactctttgttttcctggtaaaaggtaccgctgtccgactgctggaaaattaaaccgggacaaccatctgccattggcccgaaaattttaggcacgtgggcaacatcattactctccagcgtccagaaataacggacgtggtttttaagatatgccggcggtggtaattcctggtacttcattttaatagcagatgaattatattcaaggtaataatttttaatgatttcataataatctactagatttgtagactaattacattcccccatgaacattgcaacacaccgtttcatcgccagcctggcattattattagctaccagcattggatttgcacaaaataaaatagttgttttccagtcggatttcggtttgaaagatggcgccgtttctgccatgaaaggagtagcctccggcgtatcgcccgacctgaaactatatgacctcacccacgaaatacccgcatacaatatatgggaagccgcctaccggctggaacaaacagttccctactggcccacaggtaccgtgttcgtatcggtaatagaccccggcgtaggcaccagccgtaaatcggtagtgctcaaaacaaacaatggtcactttattgtaacaccagacaacggcaccctcaccctcattgcggcctccgaaggcatcgcggaaatacgtgaaatcaatgaggccgtgaaccgccgcaaggattcgcagaaatcctacactttccacggcagggatgtatatgcctataccggcgcgcgactggcagcaggcgctatcacctttgaagaggtaggaccggtattgcccaaagaggtagtaaaaataccttaccaggcggccgtgctggaaggcggaaaactgaaaggcaacatctccatcctggatgtgcaatatggtaatgtgtggaccaacatcaccgccgatctcctcaaccagctgcatcctcaatacggcgatgtactgcaggtaacatttctccataacgggaaaaaagtacatcaaacagcggcgccgtacagtcaaacttttggcgccgtaccggaaggaaaaccattgagctacctgaacagcttactgcaactgtcttttgccctcaaccagggcaactttgccgctgcctatcacatcggaagcggtagtgagtggagcgtggaagtaactttatctcctaaaaaataaatcgctactgatgataagatctttataccctgcctttatgcttgtattgatcagcagcgccgccactgcgcaaaacgcagcagatactataccggccccggctatacgtactttgaatgaagtggtaacagtaggtacccgcagcagtggccgcacacgactaaacaccgtggcgcccgtagatgtttttcatctctccaaaatacaaatactcacaccgcaaaatgatctgaaccagatcctgcaatatatttccccgtcttttaactccaaccggcaatcctcttcagatggaagcgagcatattgatcccgccagcatccgcgggctcggccccgatcagctgctggtattgattaacggcaaacgccgccatacaacctcgctggtcaataaccagggcaccgttggtaatggttctgtaggaacagatctcaatgccatccctgctgctgccatcgaacgcatagaagtgctgcgcgacggcgcctctgcgcaatacggctccgatgccattgcaggcgtgattaatatcatcctgaagcaaaacacgcagcagctgtttgctgcattaaccggcggcgttacctcccgcggcgatggtggccttggtcagctgagcctcaactacggcgctggtctcggcaaacagggcggttatatcaatatcaccggggaagcttaccagagaggtaaaactacccgcgcacaaaataataacctgatcatcttcgatcagtcgtctctcgacaattatttcgcgtacgactttaccaatgatcccgccgcttcccggaaatacgacgacgatatgctgaagcagaaaggactaaaaagagatgattttaatttccagatcggcgatgcacaaataaagaatggcggcgtattctataatttatcgcttccttttaacaacagcaaaagtgaattctattcttttggcggctacagttaccgccagggcgaaggcttcggcttcagacgcttaccaagcgatcctaccgtaaacgtatatacgatttatccggatgggtttcagcctactactgattcacgtatccacgaccgttccatcgccgtaggactaaaacataaatttggtgaatggcaggccgacctgagcaatacactaggcgataaccgtttcgactatgaggtagatcataccgtaaatgcctcgttgcagaatgcatctcccaccagcttcaaagccggcggacatgaatttttacagaacactaccaacctggatttcagccgtcgatttgcaggcgtggctgccggctttaacctggcctttggcgcagagttcagggtagatgattaccgcatccgcaccggggaagaagcctcctggaaaaattacgcattagtggaaaacccggatggtaccgtgtctaacccctccgggctggcaggcggatcgcagtcgtttaccgggttttcaccggataatgccatccataaaaacaggaataacaccggtgtttatatagatggtgaactggatgttacctccaggtggctgatcagcgcggcagcgcgactggaacactacagcgatttcggaacagcgctgagtggtaaatttgcgacgaggtataagatttctgatgtgctcaacgtgcgtggcgccgtgagcaatggtttccgggcgccctccctgcatcagcagtatttcagttatgtgagcacggatatcttaccggataacacgctcggtcaatccggtttctttaccaaccagagcgccgtggcaaaagcattgggtatcccaaagctgaaacaggaaacatctgtaaactacagcctgggctttaccgcacaggccgcccataatttcagcatctctgtagatggttatcttaccaacatcaaaaacaggatcgtgttaaccggcagcttcggcttcgatgccaacggcgatccggtggatgccatccagcagattatcaatccgctgggcgccagttctgcacgctttttcagcaatggtattgatacccgtaccgcgggcatcgatgtggtagccgactataatctccgttccggttcccatagtttcaatgcttcgttgggattcaactacaataaaaataagatcaccggcaacctgcatattcccgacggtttaaaaggacaggaacagatcttcttttctcccaacgacagtattcttatcacggatggtacaccacgcgtaaaggctaatttatcgcttacctatggttataaaaaattcagtgtgttactgcgcaatgtatatttcggagaagtatcccgcaacagtttcccctttggagaagtgcaggtgcacaaaggaaaagtagtaacggacctgtctttcagctataacctgaaacccgttaccataacagtgggcgccaataacatcctcgatgttttcccggacgaacaggtatatggcaacagttatttcggcgtgtttaaatatgcgtcggtgcagatgggcacactcggatcattttattttgcaagggtgggaattaatataaaccgccggaattagcgtatttgcctgttttaggaagtatatataataagctgatgccgtaaatgtcgggctgtcgctttgttaagctcttcatataggagcccctgatttcaatagcgccgttcttctttttgccaagcccgatccgcatccccaggttacctatcggccccacagcatgctgggtagtagaatctgtaaagctgccgccgttacggtctttgtactttacatttacaggaccgtaatggtaggccagtccgcctcccacaaagaaacctacggagtttttattatccagagacgaaaatccggcgaagttcaggttaatgattagcgggatatccaccatacccctgggctttgtcctgggaccatcatcctcattgcgggtgtagtaatacacaatattaccttccgcatcataatacgattccatgttgctgtcagattcccccgacccgccaactgataatggaatgcccaccgaaacagtcatcttatctgtttccatcacattataacggatggcataggaaaggccgaagctggcgatgctgccgtacctggacgtatgatcaataaatgtggaaaaccctatgccgtgtacaaagcgttgagagaaaaccggtaacccggccatacaggcaattgctaacagaacaatttttttcatacggcagcagtgggattagaggtaccgtataaaggtaaagtaaaaagctattgaaacggaaacccgccccaatagctttttacaaacttctcttgtgttattgtaatacgtccagtatcggatgatcgatgccctgcaaggtgtttgcagcgggcttgatcagttccagcacagtaattttattgctgccttttttcagccattcagcaggtacatacaaggtttgttgcgggcctacctgccagtatctgcccaggtggtgtccattgatccatacggctcctttaccccactgcgtcatatccaggtaggtgtcgccggtagaggaaagcgtaaagctgccttctttcaacaccggtgcgtccgtaccggcagcggaaggctttacagccggctgaacatcaaagggcagtttaaattgcagccactgatgaatagcctggccattaaataatacctggccggcaataccttttttatttttaagaagataggggccaaaattgatacgcccaagattttctaccaggatatccagggtaacagtaccggctggaagcattacctccacactgtcctgcgccaaacggcggtccagtatagccactcttttgccgttcacgaacacaataccgtaatcacgtagatcttttattttcagcaggccactatgcccaccgggaacggtagtgcgatacagcacaaatccataagcctggttaaggtcttcaaacgttaacggatctacgcttttaatggccgctggcaatttgctgaaaactgctgcgctgcgttcaaaggtgatctgtggggtggtgatcaccggtttctttgcgggaacttccggtaaagttacacctgccggcagatgcctggctatcacttcgcgaaacttcatgaattttggcgtggcatttcctgcttcatccagtggtgcatcatagtcgtaactgctgatctgcggctcataagggctcttatcattatagtttgcgccattcatatagccacgggtagtgccaccgtgaaacatgtacatgttaatggaaatgccggctgcgagtacacgatccaggcggtcgaggaagttttcataaggaatggtatggtgcttttgtccccaggaatcaaaccaggcagggtaccattctgcaatataaaacggccctttgccattgtggttttctctcaccagctgctttactttttgcggatcatcgatgccgtttacagccggcagcaaaccaggcaaatgccctttggctacatcggctgcgggatcgcaggtgtaaagcagcccgtcgaaacctgcgtcaataaacatcttccggttaatgtcgaggtagcttttatcattggaataagaaccatattcattttctatctgcaccatcaggatgttgccgccgtgatttatctgcaagcccgatagttgttttccaactgccttgatgtaattattataagcggcgaggtattgcggttctttactacgtacttcgagaccctttatgttctgcagccagtatggatatccgccaaattcccattcggcgcaggcatacggactagggcgtaacaccacccacaacccttcttcctgtgctatttttacaaaggcggctacatcgttgttgccggaaaaatcataatgtcctttttctggctcgtgcatgttccagaacacataggtgcctacggtattcagtcccattgcctttgccattttcaggcggtcacgccagctttcacgcggcacgcgcaggtaatggatctctcctgaaatcatctggaaaggtttgccgtccagcaggaaggcggagtcgccgagctggaaagtgtgttgtgcaaacaactgtatgctgcacaataccattaaaattacaacgcttagttttttcattatctactgtttattgcttaggttacctgtcaatgtaactactgactgtggcggaatgtgaataatgttaccggaaatatagcctggctttaggttttcctttgcgctggtggtatagctgcgcatactgcctgcttttagctccctgcagtgtatgttggcgttggcggcagtgctgccgttgttaataactactatccggagggtattatctttgtttttataagcagacagatagagatttttcgacgctgcgctatcgctcataacggcctgcaccctggtagcgccgggtcttataaaccggctgtagttacctaatacccacatcattttggtatcacgcagttgcccgtctgttttatttttatcgatataaatcaatccgtctttataattatacggcgaaatggccagccaccattgccaggcagcggcatttgcaatagtaagatcggagtggattacacgcgccatataaagcgctgcatccatgcccaggtctacaccggcgccatttatttctcccgcgttatctcccagtatgcaatattccgattgccagaattccagcccgttcagggcggtatgcagccgttttcgtatagtggtggccgtgtcttccggggaagtagtgaaataactatgtgcggcgatgcctttgtatacattaaggaggttgcccacgtaagtccggctctgcggatcaaagaaggcatttatctgtgagcctttgtccggtttgtcttccggggcatagaggtaattgatttttcctgcttctgtaatcagtatgttaaccggcagttttgcttcgctgaaagttttactgatggctttggtaaagccggcaatctgttcattattataagggcagccttcctgtccgccatcgctccagtcccactgcggttcatttaccgggctgatatagttaatactaacgcccgtggctacacgtattccctgcactacctctttcaggaaaacagcggcagcagcgtacttatccggggagagattgcattgtcccttgtcagcaaaggctttgccgttgctggtaaacgctgccggcgggctattcaggaaacccaggaaatccgtaacgccgcgttgttttgccgcctgtaaaaaccacaactggccggattgtttcttccagttgtaggtatgatccgcctgcagaaaggattccgcgcggcgccattcgtctttgatgccactgttatcgccttgttccgcactgccggcgccgatgttaaaacgccacatcgacaggccaatgcctttgggctggccgttggcggtggtatcggtgctaaacagccagtcggctatctggttacgtttgctatccggccagttgccggtaaactgacccgcccacgcatccgaagccgcgaagttgcggatcgtttgcgccgttttatgtaggtcgatgtttacctggataacgttactgttgctttgttgcgataatgcagtatgtagcgcaaagcacagcggcagtgagcaaatgatttttttcatgttcctaaaacgctttgcttcacacaaagccgccggaaaatagcaaaatgcccgttaaatatttttcaattatgataaccggcaggctaacatagcagctttgtgtgaagcggatgagtgtttaataacccttgttctgctccaacaggccattggaagacagaatttctgttctcggaatcggcagccagtaatttttttcagcgaacaaccggccggcaagcgctacttttctagtatacgtatatacgccactgttattaacgctgatgttgatgccgtaagcaggaacattttctgttacaatagctgttctccagcgccgtacatcataaaagcgatgttcctcaaatgccagttctacctgtctttcatgatgaatagcctcgcgcatctggtctttactcaggccaaccggaagcaccggttgctgtacactggcacgctgccggatctggttaaccgcggcgtatacgctggcatcaggccctgctgcttcattttgtgcctctgcatagttcagcaatacttctgcataacgtaaatagatccagggctgtaatccggctacgtcccagggattatcgatcgggtttttatcgtccatgaattttttaagatagtagccagttttagtggagttccagttggaagggccatcctttccatcttttccaccgggagaaaatggttgtaccgtagatcccctgtatggtgcgccattataaaggatagtggcgtaaaaacgggcatccctgttcgcatacggctgttgggcgttatagccggatgttggatcggtgatcagtttaccatttttcatttcataagcatctaccatgttctgcagcggcgtattacctgcccatccgccgtaaccgtttggtccgttggatatttccaggcacacgtggcgggcgcctacggcgtattgccgtgcaaaaatgatttcattattatctgctttcaggaacaactggctgtagtctgctgccagggaaaacttcgacaggttcatcactgctttggcagcatcggcggcggcttgccaggtgccaacgttgtacaacggacttgctgcatataataataagcgtgctttcagcgccatggcaacggcctgggtagccctgccggtctgccagctgccgtcgttgtcaaccggcaggtctgctgctgcggcagtgagttcgctcacggcataattcatggattcctgcagggtggcccttttaaataaagccggatctgtaaggtcgctggtgagctggtactctttatcacccatcagcaccacgccgccatagttgcggatcaggtcatggtaccggaacgcccggataaagcgcaactctgcggtcagctttttacggagagaggcgctcatttccacgctgtcaatgttattcagtgcgtaattacattcccggatactgcgatagcttcttccccagatagtacctgcaatgccggtattttccggtgcaatctgcccttgttggatcacccaggtattatcgtcattgttataaatggattcgtcggtgatagagctccaaaggccgtattcaaagcctctgccaaaacccggattagtaccttctccttctttatcctgtaatttgatgctcgtgtaccggttgatcacgtaattctgaaacaaagcggaatcgcccagtacggcgtcggccaggatacggtcggtaggcgtaatattcagaaagtcctgtttgcaggaggaaaataatcctgcggcaactaaagttaaactgtatataaagtgtgttgttttcatgactgctttttttctggtttagaatctaacatttacacccacattgatgatccgctgctgtgggtaaaactgtcccctttcattatttccttcaggatcgtagtcttttaccttggtaatggtgaaaaggttaaatgcgttggcatacactctcagactgccaatatttatgcgggacagaatgtccgatttgaacgtataaccgagcgatacatttttcaaccgcaggaaagcagcgttgttgagccagaaattattttggaaacggccgccatttacagaattagaagcgcgttcatctactcttggatacgagccgccggtattggtgggactccagcggttatctgcccagctgctgtaatagttaccaatggtaccggattcaggtaatacatattgacttacatgcgactgtccggctaataacaccgacaaatcaaatcctttgtaatcaccgccaagtataataccataggtgatttcaggaatgttgccatactttgttcttacctggtcatctgcattaatttgtccgtcattattcacatcgcggtagatcaggtctcccagttgcgcacccgacaggtgtacgttcttattcaggtcatccgcagtccggaatataccgatcacgtcatacagcaggtaattgttcataggaccaccggttttccgttgataagacagtgtgccgggggcttcatctataaatttgatttcgttctttgcataggtgatgttaccggaaatgttatagtgaaaaccgccgctggtagtgttgtcgtaacccagggtcgcttctataccattgctgtttaccttaccgatattttcagcaggtaccagcgggaaagcaggatcgaatggattcacaatgccggaagtctgcggcagcgacgcattccgttgggtaaggatcttggaacgcttctgctggaagtaaatgaactccaggttgaaatgttgcaggaaagccatattaaaacccaggtccattttccgcgcaatctcccaggtgatatacgggttgcccagtttggtaagatcaatgccagaaaggatctggccaccggttacgtattggtttacgatggagtagttatcgaaatactggaataaacccacattgtcatttcccagggtaccataagagccgcgcagcttcagatcattaataaaacttacgtttttaaaccactcttcttttgaaacgcgccagccggcagatacggaagggaaaaagccatactgctcgcctttcgggaaaatagaagaaccgtcgtaacgggcctgtacttccagcaggtatttttccatatagtcataggcaattctgccgaaataactttttctcgtaaaactgtaactggtgccggaattgtttttatccgtggcagcagatcctccctgcgacatctcaggcgtttgcggcgttgggaagttcaagcggatcgcacctaaggtatcctggtcagttttgctttgctcatagccaacaagggccgtgatattatgctggccaaaacgacgggcaaagttcagcttaatattgctggtgatcagcgtcatgttccgctgctgctgggcaagtgaagccagtccgttggaaccgcctaccactgttttatcgtacgattgtgtagtctggttataagtgtattccttataaggagtggcgaagcttttattggaactccaggatttatcagccgataagtatccgtccagcgacaacccttctacacccggtatggcatacgatcctttcaggataccattaaatacctgtgtaggattgcgcgcagtaccaccggcgtcagttacctgcatcaccgggttattgttttcaataccggtggtaggcaatccgttcggatacctgtccaacacggtaggataagcacggtaaataccccggaaaatgtcatctgcactggtagtagggtaaaggcggtcttcctccctgcccgataaatacaggcttacctttaatctcttcgttacatctgcatcaatatttgaccggaaattatactggttatatttggtcaccccgcttttatacaatccatcctggctgatcatgccaagtgaaacataataacgcacattttcactgccaccatttacggaaagactatgttggttttgggtggccactttctttaaagtagcttcctgccagtcggtattcgggaaattcaccgggtctgacccgtcacggaatttctggagttgctcgtcagtataaaactggttcataccaccagcaggattattataatattggatttcattcctgatctgcgcataagtggcagcatcggccattttgggcaagcggctgggagatgaaaatccctggttaaagctgtaattgatcaccggtttgccggttttaccccgtttagtagtgatcagcattacgccgttggcggccctgctaccatataccgcggcagatgcatccttcaatatcgatatgctttcaatatcattggggtccagccgttccaaaccacctatttgtccgggtacgccatctactaccatcagcacatcattgttgccggtagtggctagtccgcggatagtaatgcgggaaccatcctttcccggctcgccggagcggttgttggcaataaccccggaaaagcggccggtgagagcattggacacgttcggctgtggactctgcaaaatatcagctccttttaccacggaaatagatccggtcagcgtagctttcttttgagtgccatatcccactaccactacttcatttacacttttgctcagggatgtcaatgctatttttaagggagacaggttctttacaggcaccgtcatcgcttcataggcgatgtggttaaatatcagggtatcacccggtgcggcgttaagggaaaatttgccctccgcatctgtcagcgtaccagtagctttattttttacacgtactgtaacaccgggaacaggctcactggcatcggttacttttcccgtaatgggggtttgttgtgcctgcacgttcattcccatcaataataaggtgattgccagcataagttgaaagaaaggttggcgccgtaataggacaaacacctgatggtccgttccggattgaagttgtttcataacgcaataatttaaattggaagagtggaatacccattttggttgcatggaagatgtgcgcatcttttcatgatacccgcaatgtactatgccgggcagacatcatagagggggtaaatcatttaaaaaagggggtaaaatcgtaaaatattacaggggtatttcccccgggcgtcttgcccggaagatatcgaaagcgccaaccacggctatttatagggatttacccctctgtttcggtgacattgaagtcccggttaaaggaatggcggtatttttttacataatcggaagggttcatcccaaacagttttacaaactgttcacggaaatatttgacatcaccaatgcccacctgcatggctgcctgcgtaatggtgtagttttccttgagcagcaaaacggctgccttccggaggcggatggaccggataaaggaattgatggtttgaccggaaatggattttacctttttatacaaactggagtggctcatcccgatttccagggtgaactttttaatggagaactcctcgttttcgaggttgtcttcaatgatctctatgcaccgtttcaggaagtcctggtattcggcaggtaccttaatattgctgtttttgagggtgatgcggtcgaagaagtactgctgcagcaggtttcggttcttgatgatgttattcaccttggccatcagcaggtccttgtcaaatggcttggtaatataatcatctgccccgccttccaggccgcggagccgtgtatccgatgcggaagacccggtaagcaggatcacagggatatgacttacagtgtccgtttgtttgattttactgcatagctccaccccgtccataccctgcatctggatgtcgctgatcaccaggtcgggcataaatttctgaaccgcggcaaacccgctggtaccattgtcagcttcatatacaataaatttgtctttgaatagctgccggagatattgccgtatttcatcatgatcatcaatcagcaggatcgatttcttttcggtaatcgtggtagtcgtcccttctgcctcgggaacttccggttgaggcaaggccgcaacagtggtgagttcttcgaggaaagcagatttctgaggtgcattttcccttagcagcacaccggcaaaatgtccgcttccctttttcagggtgatatggaaagcggtgcctttgttgacctcactttggtaggcaatactgccatgatgactgtcgatgaaacgctttaccaggtaaaggccaataccaaagcctgtttgcagcgactccttccggtcctgcgcccgctggaatttttcgaagatccggttaccggcgcttccttcaataccacagccactgtcttttatgacaatcgtaacccgtgcgtcatcactggttacttcaaaaatgatactgccgttttcgggggtgaatttaaacgcattggaaagaagattaaatacagcgatttccagtttctcactatcgccatatatttccagttgcgtatcccggcattcaaaacggtagtcgatctgtttcatcctggcctgctgggaaaagcactggtatacttcgttgcacaagtgcacaatatccagccgggagatgttcagctgatcgccctcccggtcggctttgcggaacaacaggagctggtccaccaggctaagcagacgccgggcattgcggtataccacgctgagatcaggatattctttattttgcaggagttccttcagcggggtaatgatcagcgtgagcggcgtccggaactcatgggaaatattggtgaagaaggataatttcttctcattcaactctttttctttttcattttcaagatgcgccagcttgatctcatatttcagcctttcttcccgcgccttataccgggtgtaggcataaatagcggccataatgctgctaatgtacaggagataagcccaccaggtccggtaccagggcggcaataccaccactgataccgtgtgaatggcattgctccacacgccgtcggcattgctggctttgatctcaaaaacatagctgccttcctgcagatgcgtatagttggcggttctggtttgccccacatagttccagttattatcccacccctgcaggcggtacgcatagctgattttatccggtaaggtatattccagtgctacaaagtcaaatgcaatggtggccttatcataaggcacggtaatttcccggatctcttcctggcttcgtttggatacatattgatccagctccgtcacggaagtattattaattctcacggcggttaataaaaccgggggaattgtggtttgagaataaatactatccgggtaaaaaatattgaatcctttgatgccaccaaacaggaattccccggattgtaatttcagggcggcattaaaactgaactggttgctctgcagtccatcggaagcagagaagttgcggaaactctttttcttcgggtcaaaccgcgataaaccattaaatgtgctaagccaaagattgccggttttatcttccagcatccgcagtatagagttactgggaagtccttctgaggtggtaaatcgtgtataatttccgtttttgcggtcaaagttcaataatccgccaccatcggtgcccacccaaaacgttccgttctggtcctggtggatggagcgcaccgtgtagccaatgttgaaacgccggtgctgtttccggtcacggtctatccggataagggtggaataattgcctccccacagctggccatccctgtcttctgccaggcattgcaggtttaccagactgctgtcgaaaagttcaaaacggttttgctgccggttaaacaggtacagggtgccgttgttggtggtgctggcccaaagttgttgctgccggtcttcatacacggtccacacattgttttcggcagtgcgggtgtaaggattaaaacatacaaagtgttcaaaagtgccggtggcagcgttatacctgtttacgccgccaaaccaggtggaaatccacaggttctgccgggcgtcctggataatggaggtaataaagttgctgctgatatccgtattactgttgccggtatgtttataggtggtccaggtattgttttccctgttccagtatttaagccctccgccatcagtacctatccagatatttttgtggttgtcttcacaaaaagagaagataaaattgtccactacgcgggccaccgggtccctgttgggcatattaaattcaaacgggttgcgtttgggttctacaatgttgatgccgccacgcagggtgccaatccatttgcggccctgacggtcttcataaatggaatacacggcattgctgctcagttgttgttcgtcagcggtggtaaaggatttggcggtactgttggcggtattcaccaggtaaataccattaccatccgaggcgctccacatggtcccgtccttatcgatgtacaggctaacgatcttgctgtttacgggtagtacattttctgaatatttgccggtggcaggaacgtagcggaataccccggcatctgtacccagccagatgttgccggctccatctgccgtaaggcaattgcccctgctgatatccctgttgatgatggtcaactgctgtctcgcaatatcatatttgcacaaacctacatgttgtacaaatacccaggctgcagttccgctgaattcaatggcggttacttcataatcggtaacatcgccgtggtacattgttaagggaatctgtttaccggcagattgccggctgttaaacagcaataacccgcttttttcggtgccgattaaaatattgccggtttcatctgattttatggtatgcgtattttcgctgatgatccgggaagtgttgctgtgaaggggcaggtagcgcggcagtgtgaatttttcgctcaccgggttgaaaacacaaacgcctcttcgcccgcctacccataactggtgatggatgtcatcggccagggtgtatacaccattatccacgagggaactgctgtcattaattttattccggtagatcctgaatttatagccgtcaaacctgtttagtccgtcgtaagtaccaaaccacataaagcctttgtggtcctggtatacactggtaacggcattgttggaaagaccgtcctctatacccaggtatctgatggggtaaccaatagcgaagctatctcccgttaccattcctaacagtaataaaataaaacaaaatttcctcacatggtgcataggctcattttaacagccataaagctattatttctgccagagattaccaccatcaatcttcttactgatttaactcttctactgtttgctttacccggtaaattcttcctttccatattttccactggaaataggcctgtacaccaacaatgataacgagcgggatcaatgtcaggtacttttgctgcgtccagcgaatgctggcaagaaagaatgcaaagatgcccgcaaaggcaaggatttttgtgaagatggtaatcagcgcgtacttcctgatattgtacaatttttttcgcatgctctccagcaggttgtattccaccgcaggactgcgggccaatacataccctgtaacactttgtgccagcatacataataccgataccaccaacagcaggttcaggtaatatggttttttgtcgccgtcaaaaaaatcatagtatacgatcaggaaaatactgtatccgatggcttccagtatcacctgttttctaatatcttttaatacgggagaagtgtgtttgccaatgatagcggaaatgtcccggtcaggggtgggagcgttgtcccatgctgattttaaaggatccatgtgtttataattttagaatatttttgatcttgcttttaatcctgttaagttttacgcccacataattttcatctatgccaataatatctgcaatttcctggtagctcatatcaccgagatacagtgcaatgatggctttttctgcatcactcagttgtttgagtgcggcaaaaagctgttcctgttgtactgatgccgccgcattgttagcgctgtcgggcagttccggcaaactatcggtataggtaatatcgggtttcttccggcggaagtcggccagcgcggtattgagtgccacccggtaaatccaggtgctgatgcgggcattgccttcaaaagaaggatatgatttccaaagctggtagatcatctcctggaacaggtcttccctgtcttcccggctatcgcggtacaggcggcacaacttatgcaggatgccctggtgctgctgtatggtatcgagaaatgcgggtttgtccatgcagggtatttatcagggttagttgcaggatgcggaaaaaacttacactttcacaaagaaattattgatccgttaccagatcaccttgttcaccgtagcccagttgcgggtagtacagggaagcccgagctttttttccagtcgcgtaatgacatcgaggggtttggtttccaggtctttccgtataagggtatacacttcgcggccgttcatatgcagggtttccgcggccgactgcagcgaggcgatcacggatgcggcatgtgcgccggcgtcggcagaaaggaaggtgatgtacacctgcgtggttttatccgggataacgccggggaacggggtgagtttcaccacgttttccagttcgggcaccgaccggataatagtgggcacttcaaaaccataagtagtgagcagcagcttttctatttttgcagacagcgccgccgcattattgctgccggattcaaacatcacattgccactctggatataggtgcttacatttttgaagcctgcggtatccagctgccggcgcagatcttccattttaacggttcgtttcccaacgtttactgctcttaaaaatgcaacgtatctggccatgtggttttcaactttactttgtatgtttgttttatcatgcactatctacaaatcatccacaaattatacaacttaccggaagatgccaatcacggttatacagccgcagaaatagccgcgctggaagcccgcttacagcttcaattaccggcagcattgcggcaatactatcttgctataggtaaaaacaaaatggtgaacgatagttttaaccgtttaacttccctgggagaaattggtttttcggaagatgatcacctgattttttatgaagagaatcaggcggtggtactgtggggcattgccaaagcagatctcgcgttgccggatccgccggtatttggtacctacgacagtgcccggcaggagtggtttaccgacgccgatacaacggaacatttcctgttatcgatggcctggtggaatggcgcgctgggtggacttccatacacggccttcactgacctggaagaagacctcacgccggaacacatcgccgccgttactacaaactggcaggagcaaaccggtatttctaaccagctgctacgtttctttaccaatgattatgaagatatccttgtgcttaccaccgagcagaacgggcaggcgaatggtgcgtatattggtaccagccggaaagaaaagtataaagctattatggatacgctccacatggaatggagttaccgcatagaccgtgatgaataagtaacccaccaataccatcccacggtaaacaggatgccgtagaaaacgccgcccagcgcggtggccaggtaatccatgcctttacagtcgatatgatgaaagtactcattcaccagtaacattaatccgcttattacggccacggtaatccagaagcgtgctttcagctgcagtgatactttcgggagattattcacccgcggaagtttcagaaagaaatataacatcaccaacagccctgctacagaactgaggtattgcatcaggtaccacattttcatgggatgatgccataccgttacatctttttgtaaaaaagatatgtatgacacaaatccgccttcttcatgcgtaaacgcatcgaggaagaaatgcgtgagtatgcccagtataacagaatagatcactacgccgtaatgttcgcggaagtaggtatcccagttaaacggcctgaacagatgcagtcggtcgctggcccacgccggcaggtaaggaagcactaccggttttacgataagatgataaacatacgcgagcagtagggctaacggtatatcatatacgaaaattccccaccactgatgtccgccactgaagtacggattcagtaaaatgaagtaaagaaagtcgggtaccatactgccgatgattaaaccggttgctgacaggtatttgcgggaggtatttacaaaggggacaactatcgctgcatgtgatatcgtaaatggcattttcgggaattgtctaataaatttaattgaattttaataaatctggtaaggaaatgttaatgttataatcgtccaccatttccggtaaaatgtccaacgtcattgctgtgatttacacttatttttattgagtctttgaaaacataaaaaacaatgtgctatgacaaactggaaaattgatgaatcacacagcgaaataggattcaaagttaagcatctcatgattacgaacgtgagtggatattttacacggtttaccgggaaaattcaaacagagagcgatgattttcgtgatgctacgatctctttcgaagcggcagcagatagtattgacacgcaaaaccatcaacgggatgagcacctgcgcaacggcgaattttttgacgcctccaatcaccccaagatcagcttcgtttctaagaaagtgaagaaaattgatgacgagaaatacaaactgctcggcgatctcactattaaaggcgaaacacatcctattgaactggatgtggtgcatgcgggcgtaaccgtagatccttacggtcagaccaaagccggttttgcactcaagggccgcctgcacagggccgactatggtctgcgctggaatgccaccaccgaagccggggggattgtgctcagcgacgaagtgaaactcaacatggaaatacaactggtgaaagaatagctttccctgcaacgtataatggcgtggagaagaagggatttcccttcttctccacgccattttgttaaaaaaggaaagctaacagctattggctatctttgtgctttccaatgatgtcacatgaaatttgaacaatataatatctcctcagaaataaaggaaagtttagaagaaatgggctttaaaaagcctacagatatacagtttaaggccattccttccatcctcaacggggatgatgtaatggcgatcgcacaaaccggtaccggtaaaacagcggcttttgccatccctatcctgcaccgcctgcaacagcaggaccgccgctcccggaaaaataagtacgaagtgaagtgcctggtaatggtgcccacacgggaactcgccatccagatagcagaagttttccaatctatcgcccaatatacagaactcagcatcctggcccttgtaggcggggttgagcaagctccccagatcagggtgctggaaaagggcgtggatgtactcattgccactcccggccggatgtttgaccagattaaccagggacatattgacctgagccaggtgcaaaccctggtactcgatgaagccgatcatatgcttgatttgggctttatccgtgatatccgcgatgtaatcaaacacattccccgcgaacaccagaccctgtttttctccgctacgctgaataaagacattaaggacctggcatattctgtcgtaaataatcccatccgcatacaaatatctcccaaagatcccgttgccaaaaatgtgagccacgcagtagcctttgtggaaatggatgataaacgtttcttcctggaaagactgatcaaggaatttcctgaaagcaaaatccttgtatttgttcgtaccaaagtacgggcagaacgcgtaatggccgctatggcacgtatcgggatcaaatccctcaccatgcacggtggcaaagagcagggcgaccggctcgatgtaatggcagagttcaaaaatggcgatataaaagtactcgttaccacagatgtaaacgcccgcggcatcgatatccccaatgtcgactatgtggtaaactacgacctgcctgatgtcccggaaaattatgtacaccgtgtaggccgtaccggccgtggtgtgcagaaaggtcaggccgtttccttctgcagcacagaagagaaaccgatcctggatgaaattcagaaattcctcggtaaggaaatcactgaaatgaagatcaataaggacgattaccgcgaaaccatcagcttctctgaagatattcccaatgacaactggcaactcctgctggatgagcacaacaaggaaatggaggaagtgcagaaaaaagtgaagaagagagcggcggcgaatgtgaagaaaaaagcgaagaagaaataaaacgatcttaaaaagctcagaaaaaagctattccggaaggaatagctttttttctgagcttaagttggcatattttgtcaatttttctgtaatttcaaggatgaagatcatagaaaaatcatccgggatatctatagatgttttgattcaattgattgaaaaagaagattttaaaacgatatcacgggaacggtttttatttgattggaagaaggtggttaagggtggcgaagtttataaactggttttgccagatcataacattctgggattggtatgtttgatatgttatgccgtggaagaacgggtagaaataaaattattggaagtttccagacaatatgtaggaaaaaatggcccgtatgaaggaattgcgggttgtatgatagcctttgccggccgcacagcactcgctaagtatggaccttatgcttgtgtttcgctggttccaaaaactgcattgaaaaaacactatatgaaaaaatatggtatgctcgatgccggctggcaactttatctcgatatggacgcattaaataacattgttgcaaaatatactttatgagacagaagaaatcaagaaacgaaaaatctccagatgagttggcatcttcttttgtcttcccggttaagctctctgaaaagcaaagaaaggaagcggcagtacagctggcaatggccagggaaaaaagacgggcggctgcaacagataaggataagcttatcagcggcttattaagtctgcgttttcagctcgaagattatataaatggcaatacttttaatcctgatttgtcattcggatatttccttggtgaatatgttggcttgttagagaagaaacggaaggtatttgcagaagaaatcagtattgatgaaaccttgttgagccagttaatcaatttgaaaagggatccgcctgattatgtgacagtaagattggaattgcactctaaccgggccattcccgccgattactggtatcggctagtggaaaagaaaaaagaacattttattaaaacagataaatctatcaggaagaaggaaaagcagtttgtacagaataaactgaatgtccatatttagtatcatcaactaaaaaacggtcccggcttacaccgggaccgctactcaaaaacactatctaaatctgtaactattgctttactgcctctacgtttacagtgatgtcaacagtaggtgctactgcccatacaccggaaggtaatttgtctgcatactttactccaaaatcaaggcgattgatggtagtcttagcagtgaaccctgctcttctcaaaccccacggatctttaatcacaccgttgtatgtaacgtcgaaggttacacgttttgttgtattgcggatggtgagatctgccagcaaaacatatttatcgcctgtcactttctttaaggaaacgcttttcagggtaatagaaggatattccgcaacgttgaagaaatcatctgttttcaggtggccatcacgttgatctacgccagtggaaatgctggtggcatctaccgtgaaatctacttttgcattctgaaagttggtgctgtcggccgtttcaatggtgccattgaatttggtgaaatgaccttgtacgtagctcaggcctaagtgttttacgccaaagatgatgctggtatgtgcaggatctgcattccattttacctgggcaaaggtggcgatgctggctaataccaggagggtagtaaaaaagaaacttttcttcatgattgtttttttattgagtgtgatagttatttatttagaaagctgacggtcaacggaccagcgtccggcgcccttgatgatcaatgcaatgttgattccaattacgagtaaatgatactcaaagccttcacctgcctgcgtgccgccccagttcataaaaaagccattagcagaatgtatgttcgtagctaccagcatgataatagttagcatggctgcccatatcctggtggtgaatccaaaaaggattaacagtgaaccgatgctttcggtaaatattaccaggaaagcaaggatagaaggagtaccctgtgaagtgaagtaacccatagtggccttgaatccataaccgccaaacatgccaagtagtttttgtgcgccgtgtggcaacattaccagtgctacggtaatacggataataaaggaagtgaggtgatcgtctgtgcgaagtaatcttttaaacataagggtataattattagcgtttgaacttttattgtatatacaagtattagggcaaaaaaaatcaactacgtagtttatccagcaaattgttgagggtattcacctcttctttggtcagtttcatggtcacttcctggtggttattttctatcaccggatccagttcctttaataaagccagtcctttgtcagtgatctcaatttccactttccggcggttgctgtcgcactgctgccgcgttaataatcccttctggcgtaacttttctaccagccgggtggcattactcatcttatccatcatccgctcctggatatccagcaggttcaacggattaggactgcttccacgaagtatacgtaatacattgtattgctggctggacaaatcatactgctttagcatatgagaagcgcccacctccagccagttaccagtaaagatgatattgagaatagctttttggtattcgtccttaaatcgggtttgcttcagttcctcttccagtttcataattacatttacaactgttgtttatacaacaaaggtaagtgtatttttcatattgccaaattttatgcggattttgtcttggctcaggattacgctgattttactgattacctggatttttactttgggatttttttggattttcagattaataatataataagtaagggagatagcagcgaatatcaccgctgctatctcccttaatcctttataaatccaaatgtaaaaatccaggtaatcagtaaaatcagcgtaatcctgagccaagacaaaatccgctggactagctattcagcccgccatcgatcgtcagcgcggaaccgttgataaaaccgctttcaggacctgccaggaagctcaccaggccggctacatcagtggccgtaccgtaatgacccagtgcaatgtgctggcgttgataatcggcatgagggccatcggccggattcatatcggtatctactggtccaggttgtaccaggttggtggtaatacccctggaacccaggtcgcgcgccaatcctttgttgaaagcggtaagtgcagatttgctcatgctgtacagggtaccctgcggaccaaccacacggtcggccatgcaactgccaatagtaatgatcctgccgccgctgcccatatgccgcgtggctgcctgtgtggctacaaatacggcacgggtgtttactgccatggtatgctcatagtcttccagcgtataatcggaaaacggtttcattacggcggtaccggcgttattaacgagtatgtctatacggccataactattaaccgtatgctccacagcggccagcactgcattcacatcagcgctgtctgctgccacagcagtagcttgctgtccttttgcggttaattcttccaccagcgctgctgccggcgctgcgccctttacataggtgaacaccacggtggcgccctctccggctaaacgctttacaatggcggcgcccataccacgactacctcctgttaccagggctatcttattctccagacgtttcataaataaatgattttatgctggcaaaactagcccggctaaccggtgtaaagaagaggagtactaattgttaactactaaccttcatgttagaattgggctggaggtacttctcacggagtatattcaggtggtgtgtctgatgcccggcaatggcaaagcccagggcaagtaccgacatttccgttttccagcacatccctgtccgtaacagcgccgcttcagagaaattattgaactgcataatgctggccgcacgtacggctttcagttccgcaaggatttctgatacgctccgctcatctatttctgcattcgctgcgtagtcgtcctgttccatcgtgggcggtatctgggcatctttccgggcaaataacagggcgcggaaagaaaacacccgctcggtatccgtaatatgctgaagtacattctttatagtccatttgccgggaccataggcatagttccccaatggctccagctgcgcggcatcaagttcattcagtgcgtgtaacgactgctccagggcagttttgatatctacgtctggtaccaggttagtataggtggagtaatatcccgagtcagggtggatggcattttttttcatctggtgagttttaaaggaaactgaatatacgaacattttcccctggcagcagaccgtttccccttattatatcatcttaataatatatttaatatatttgtaagtaatatatcctgactacctacaatctctttctatgaaatatctgttacggggcctgctgctgcaggcgctcatcggatttgccaccaccctgcacgcgcaggagaagagccctgatagcccctttcaatgggacgccaggtggatttccggcaataatgccaccccggccgcctatggggtgtatcttttcaggaagcagttccagctgctcaattattccggtccctttatcatccacctttctgcggataaccgttaccgtttgtatgtaaatggacgctttgccggaatgggacctgcacgctccgacgctgccaactggtactatgaaacaatagatatcagcccttacctgaaatatggagtcaacgtaattgccgcagaagtgatcaacttcggcccctgtaagccgcgcggccagttcaccaatagcaccggcctggtcatacagggacatacaccacgcgaagccgctattatcaacaccggttctgcttcgtggaaagtaatggaagatgagtcggtacatccggctgccgtaaaaaccaccggtaacgctttctacggcgccttcccgggcgatagcataattgcgcaataccatccctggggctgggaacagcctgcatataacgacagtgactgggaatccgcagcagcagggcatggcgtagcactgcaaggcaatagcgcggataactggccgctgcttgcaccatctcccataggccgcttgtaccaggaacggcagtcgttcgccggcattacttcacaacagggaattactgcagaagcagccctgctgaaaggcaccgcgccattaacgattccggctaaacgaaaagtaaggctgctgctggacgcaggacaacaaaccatcggcttccctgaaatgctgatcagcggcggactggatgctgctatcaaaattacttatcagccggcgtataccagcagcaccgtgatacaggatgttattcatcccgatggcggcgcccgccgtaagttcatctcttccgggtatcgcagcttccggtatgtgcaactggatattgaaaccggcaaatcgcctgttacattacacgactattataacgtatatacacagtacctgctgaatgataaatcaaccttcaccgccggcgcggcagcggattcgctctgggccgctggtaaaagggctgcactcacaggcgcgcaggataacctgtacaatgatccgttcaatgagcagcttcagtatatacaggatgcccgcatacaggggcttgccatcagttttttttcgggagatgatcaactgctcagaaatgcgctggtacaaacagaccagtcgcgcattccagagggccttgtccgttcccgttatccgtcggacgaccggctggtatcggtaacagatgcgctggtatggataggcgctatccacgattatttgtgctataaagcagataaagaactgacgaaacaatgtttcccgggagtacgcagtatcctcgattgggtggatcgctaccaggaccccgttaccggtttacccggcactatgccttacaacgatagcgtggcgttgtcgcccgccacaggtcagtacctgtatgccctgcggcaggcagctgttattgcgggctattgcgacaagccggcagactctctcgcctatacccgcacggcagataaagcaagggaagtatggtatcagcaatgttatgatgcggggaaagggttgtacgcggaaaccgccgcaaagaaaactttttcgcgctataccaatgccctggctgtactggcacaggcggtgccaccccggcaggtaaaaaacgtgatgcagcggttattagcagaaaagccggcgccaggcgaatcgctgcgtgaaaagtattacatcttcaaagcaatgcaggaaaccggcatcacagaaaccttcccggcagaactgcagccgctcaccgtgctgctggaacagaacaatgcagccgcttaccaggcaacggcctcagtggccaatcttttcctgctgggcattacggccggtatccaatcctcctcctatggcttcagaaccgtattaatagcgccggatcccggcgcctcgccgcaggtaaaagccactatggtacatcctgatggcttaatagaagtagaccttgcatttaaaaataatcgtgtaaccggcaccgttagggtcccgttcggtatcactggcaaattccgctggcgcggaaaggagatcacgctgcacggtgggccgcaggaaatcgctttgtaacgcggattttgtcttggctcaggattacgctgattttactgattagctggatttttacttttggatttttttggattttcagattaataataagggagataaaagcggatattttcgcttctatctcccttaattattattaaaaaatctaagaaatcaaaaaaatccaaaagtaaaaatccagctaatcagtaaaatcagcgtaatcctgagccaagacaacatccgcgttacgcgcgttttcttcgcgagtaaaaataatttatccccaatgcgccgatacaaatgaacaatccaaagaattcgcgtgtttcttcaatccagggcttggttgctttcatggtttcggcaaggttctctgcgttgtgtttggtgaaccagtcctccaccccgttctgatcaaaaaacttataaatggcataagccaggtataccagtataccagcaatgtaccacttcgggtaaaagcggttacgggcggcaaaccagcaaaacaaggcagaataaagataaatgggcatccatatataaggatcgggatcattgtactgtaaacctgcaaacaaaacgaacatcaggcaaaacacaatattcaatattttcatgacacaaaaattaggacttaaacatacacaaaagaatttcaaaactatattccttgtattattttatcccggcagtgtggaatagtggaatgacagtctgcaattttgtcacttttaaagaaaatgttaaaagactacttgtttgggctaaaataatgttatatattcggttcattacatcgttccacgtgagaaccaaaatctgagattagaaatgtttgttactagagcaaaagattctcacattattattaattaagttatcgtatcggattaaacaattaaacaaagtcaaatgacctgaatcagcttgattatcagtgtttgttttatagtataattcatcattcactagtagttatcgtttaactgttgaacagacacttgtttcttttttgacaccgtgtagcgcatcatgcacagtgatgaaaaactaatgctttgtatttattgaaaattgacctgccgcaaaaaataaatgcagcgggtaaggaatctgtatgcaaagttgtgactgttcaataaggtgacatatatagaatagataggaatccttatttactaacaattttttttcttaaacgtttcccttaaatcacgttatgaaaaagcaattttaccaggcactcgccgttctatgcggcctcttgttgctattggccggcaacactgtatcagcacaaacaaaaatctcgggtaaagtaacagacaaagcctccggcaatgcgctgccaggcgttacggtgtttgtgaaaggtaccaaccggggtactgccacagatccctccggtgcattttcccttatggccaaatcaggcgaaacacttgtattctcctttgtgggatatgatccgcaggaaacagtagtgggaaccggaccagtaaacgtttctctcaccgagaaagtaggatcactggaagaagtagtagtaaccggttatgccagccagaaaaagaaagaccttaccggtgcagtgtccattgtaaaagtggaaaatctcaccaaacaacccacttcccagatagctaaccagctacagggacaggtttccggcgttaccatcctcggctccggtcagcccggccaggaaccacaagtgaagatccgtggcgtaaataccttcggaaataatacaccactgtatgtagtagatggagtacccatctctaacatcacagacataaaccccaacgatgtgcaaaccatgcaggtactgaaagatgcaggcgctgcctctatctacggtgcccgtgcagccaacggcgttatcattatcaccaccaaaagaggaaccggaaaagtaaaggtttcttatgatgggtattatggaacacagcgtcccaaaggcggcaatgtatggaatatcctcagcccgcaggaacaggcaaacctgaaatggatggccatcgccaacacaacgcccaatccggtatacaaagatgaacaatatggttccggtgccacaccacgcctgccggattatatcgcaccgcagggcgcaatggaaggagatcccggcacagatccatctacttatttcgtaaatccaaactacaaggtagccagtgatgtagatgcttttcaccgtatcgtaaaagccaacaagtcaggtaccgactggttccacgaaatatttaacccggcgcctatcaccagccacaatatatcagtagcaggtggcggcgatatcggcagctactttttctctttctattactttaaccagcagggtacattaaccaatacctataacaaacgttatgcagttcgtgctaacagcacttataacgttacggatcatatccgtgtagggcagaatatggaatattccctgatcaataacccgcagatcggcgcacttacagaaggtagcggtatcggtatggctttccgcgaaatgcctatcatcccggtacacgacatcaagggcaactatgcaggcagcttcggtaaaggtttgggtaatgcccgtaaccccgtagccatccaggaccgcttcggtactaccaaaacactggccaaccgcctgttgggtaacgtgtttgcagaagcagacatcctgaaacatttcaccctccgcaccagctttggcggtgaaatctattcattcaataaccacagctttacgctgcctgaatacgaaaacgccgagaacaataaggtgaactcgtacacagaaaacgcaggaaatggttacgactggacctggaccaacaccctcacttaccatcagaactttaaccaggtacatgacctgaaagtactgctgggtacagaggcattcgataaccagggacgcaccgttggtggaagcaacctcgattattttacttttgatcccgacttcaccaaccttagcacaggtagcggtacgccaaccaattatagcggccgtttctctgatggactattctcactgttcgcaagggtagactattcttataaagaccgttacctcctgggcgccctgattcgccgtgacggatcttcccggttcggttcatccaacaggtatggtaacttccccgctgtaagcgccgcctggcgtatgtcgcaggaaggattcatgaaaggtgtcagctggatctcagatctgaaaatccgcggaggatatggtatcatgggtaaccagatcaacgtagatcctcagaactccttcaccgcttacggatttgaaaaaggaaactccttctatgacctgaaaggcaccggtaactccatcatgcagggcttctaccgcacacgtatcggtaaccccaatgcaaaatgggaaagtaacgtaaacgctaacatcggtatcgacgcgaccctgttcaaaggcgcactggaagttaccgcagactactaccgtaaagatgtaaaagacctgctgtataaccccgaattacccggtgtttatggtatagctaacgctccttatgtgaacgtggcacaaatgaaaaataaaggattcgacttttctgctaccgccaacctgaatcttactaaagacctcaagctggaagtgaacggtaacatcactacctataataatgaaatcgttaaaatatcagacgctgctccttacttcgaccaggaacaacgccggtttaacggtacattcattatccgtaatgctgtgggccagtccatcagcgaattttttggttataaagtagatggattctggaacagccaggcacagatagatgctgcaaacgaagctaccaggaaacagtataacgacaattcactggtataccagacagatacaaaaccaggccgtttcaaatatgcagatgtgaatggcgacggcaggatcacagaagcagaccgtacttacctcggtaaccctaatccgaagttcagctacggcctcaatatcaacctcacttataaagcatgggatttcagcatgttcgtgtatggagtacaaggcaacaagatctggaaccaggtgaaatggtggaccgacttctatccttccttcgaaggtgcgaaaagcaaaaccgccctgtatgattcctggttgccaacccgtcagaacgcaacagcacctatccaggaaacatctccatccttcagtacctccaatgtgccgaactcctattttgttgagaatggttcttacctgcgtgcgaaaaatatcatgctgggatacaccatacccagtaacatactccagagagtgggtattacaaaattcagggtatatggccaggctgcaaacctgtttaccattacaaaatactcaggtatagatcctgaaattaccggtggtaccagcaattttggtgtggatgaaggagcatatcctaatcagcgtcagtacctgcttggtgtgaatgtaacattctgataattttttcctgaaaagtaaaattgagaaaaatgaaaacattacgatatttaagtgtaattcttgcgttggcagcagtaggaatcagtgcttgtaaaaagagcttcctcgaacggggaccactcggctcccttagtgatgaaattgtagcgaataaatccggtatcggttatttactcgtaggcgcctatgcctcactcgacggacagcaaaccgcccaggcagcactcggcggcggcggcccctgggaagcgtctcctaccaactggatctatggcagcgtagccggtggcgatgcacacaaaggcagcttcagtggtgaccagccaggtatcgatcccatcgcaaaatttacggtagatcccagcaacggtttctttaataccaagtggagagctgtttatgaaggggtgatccgttccaatgcagtactggtagcacttccaaaggcaacagatatgagtgccgccgaaaaaacacaagtggaagcagaagcccgtttccttcgtggtcactattattttgaactgaaaaaattgttcaataaagtaccatatatcacagataccacgttggaagtccgtatcaagaatgacaaggatatctggccttttattgaagccgattttaaatttgcaacagataatctgccgccaacacaaagcgacgtggcaagagcaaataaatgggccgcacagatctacctggccaaaacttatctctatcagaaaaagtatacagaagcaatgccgctgttcgaccaggcaatcgcctccggcgttacttccaatggccttaaatacgcactcaccaacgcattcgaagataacttcgatgccgccaaaaagaataactcagagtccgtatttgctattcaaatgaccgcaaatgatggtaccaacaccatcgcaaacgcaaaccagggagaaatgctgaacttcccgtacaacagccccttcggctgctgcggattctatcagcctacccaggaccttgtaaactcatatcgtacagaccccgctaccgggttgcctaacctggataactggaacgcaaacccggtaaagaatgatcaggatacgttatccagcgctccattcacaccggaaacaggtacactggatccacgccttgactggactgttggccgccgaggactgccttatcacgattggggtaaccaccctggtgccaactggatcagagatcaagcttatgccggtccatatgcaccaaagaaaatggtgtactggcagtttaaccaggacaaatacaaagatgcacactcctgggcgcccggatctgctatcaacgtactgctgatccgctttgccgacgttatcctcatggccgctgaatgccatgcccaaaccggcgacctcggcggcgctaccgcgctggtaaaccagatccgcgacaggatgatcaatcaccctgaaaactggctgcataaatacaaagacccaacaaaaccaatgttaggtttcgatcctgcggtaatggcagctaattataaaataggcaggtacacggctgcttttacaagtaaggaccaggcattaaaagccatctattttgaacgcaaactggaactggctacagaaggccaccgcttcttcgatctcgttcgctggggcattgccgatgtggcgctgaatgccttcatccaatacgaatcagccatcaccaacgacctgaaaggcggacatttcaccaaagggaaaaatgaatatttccccatcccgcaacgccagatcgatctgacaatggtgggcggagtaagagtactcgatcagaacccgaattattaatagctatatctgtcgccctttttaaacaaaacgaatgcagcgatctttttcgctgcattcgtttttatataacattttagtactttacaatgcccgttaaaatattcactgatgaccaaccaaccaatgaggaaccggtattgtctcgccgttttatttttaatcaccaattgccttgtcatcatcagcagctgtgatacccctaccccggaagaaaaaggaaaagccctggcagataaatattgctccggctgccatttgccggtgtcttccgaccttttggataaggaaacctggacaaagcatgtattgcccgctatggcccccaaattgggcattaaagtgtggggagagcattcttattacccgccaatgcccggcgaaaagccagggcttatttcaatccaggattgggaactgctggtggcatactatgaacataccgccccggataaactgccggcagaaaaaataccgcagccgttgcaacgcgactggtccttctttaccctgaaacacccggcactgaaagataccgtccccgtagctaccaccatggtggcctttaatccggacaatggccacctcatgaccagcgatggtctcaccaacacactcacacagtgggacgaaaatttacaagtcgttaacatccggaatttaccttcccctgctgttgatatactttttgtaaaagatactgcaggacaacaacaggccatactcacagaaataggcaacatgcgcgcattggacgcgcctgccggcattattaccagcatccggcccaacgacgcggaaagcaggcagcacgacctcatggctttcctcaaacgaccggtacaaaccctgcaggcagattttgataaagatggtctgccagacctgctggtatgcgcattcggacataaccagggaggcctgtactggctgaaacagttaccagaccacaagtaccagcaatttcccatatgggaagtgcccggcgctatccatgcagaaaccggcgattttaaccacgacggctatacggactttatggtattgttcgccgctggtgatgaagggatctggttatttgaaaacgacaggaaaggtggctttgtatctaccaacctgctgaaattccctcctgttaatggttctaccgggtttcaactggcagattttaacggagatggaaggctggatattttatatacctgcggtgacaatgcagatttttctatggtgcttaaaccttatcacggattattcgtctacctgaatgacggaaataacaagtatacagaagcatggcattacccggtgaatggctgtacaaaggcagtggcagcggattttaacggtgatggtaaactggatattgcttccatcgccttttttgctgattttaaacaccgcccggaagagaaatttattttctttgaaggtggaaataaaccacttacgtttattccccattcaccgccactggagaaggaaggaaggtggatctgcatggatgtgaaagattatgatcacgatggcgatcaggatattgtactaggaaactatgcgcagggttttattatacttgatgattataagcctgactggaaagagtatcagccgtttatagtattgcagaacaatgctgtgcattaaacggaacgtaaaaatcacttgtttatttggaatgaaaggagaaatatgtatcttacggccgtatttattgctgcatggatttttgctttattgccggatctgaatttataggaagagcactcatatattacagatctttaaagtgccatcgttcttgatcaacgttttcccaacatataccttattgcgctgtgcctgtcgtcagaggcaccgtggctaaagatatcctgatgtataatcaggttttagaatggcggaaggagaggcagtaatgcctctcttttattttggggcatatcccatcgttcaaccattgatgtgaacggtttaatcttctttttttgccatctatcataaaaaagtggccggattcttaaaatcccattattactggttaattttattgggaaatcagcattattattttaaacaggatatgtcagtggctgaatatgtatacgatcaggataaagtgagcacgctgcttggaacgatcatcaggaacaacggaaacgaaaaagcgaatacctggctgcaacaacgtttgcagctacaacagcaaaccggtgccatcccgcagtttaatcaaactttcacagctattccgcgcttcacaggtaaagaattgatccatctttccgcaacggaaaatgaacagttgcaagcgctgcggccgtcattattcgtacatggatggacgttagaccgcctcgtacgggtatggtggctgctccggttgccggtaacaaacaaagccatatacctggaggtgctggaaaacctcttcaatggcgcggaaatgaatgagctggcagctttatacagcggactcccgctgttgccctggccggaagaatggatcgcccgcacgtcggaagggatcaggtccaatattggtattgtacaggaagccattatgctgcacaatccttacccggccgaatatctcccggaacccgcctggaaccagctggtcatgaaagccatctttaccgataaaccattacaccggatcaccgggctggatgaaagagccaatgctgcactggccggcattctcgtggactttgcccatgaaagatgggccgccggcagaacgctcgatcccatgcagtggcggctgctggtgaattttgtaaacgaaggtaactttgccgacattacccgcatctggcactccgtcaacagcgctgaaaaagaagccgctgcactcgtttgtgcccaatgccattacgaacccgctaaagcattgctggccacagacccggcactgcaggcagaaatacacgccggtactatctcctgggataccctggcacaaaaaataattaaataattaaattaaaactgatcagatatgtgcggaattcatgacttaacagaaaaagatcttcaaccactcacctatagccccgcttatcttaataaaataaaaggcatgcgcttctttgatccgcatgtgcacatgaccgcccgtactaccgacgactaccaggcaatggccgatgcaggcgtagtagccatcattgaacccgctttctggttaggacaaccacgcaccggcgtagataccttccgcgattatttcagcagcctcctgggatgggagcgtttccgcgcttcccagttcggcatcaaacactattgcaccattggcctcaactccaaagaagccaataacgaaaagctcgcagaagcagtaatggaaatattaccgcagtttatttataaagaaggcgtagtaggcgtgggcgaaatcggtttcgatgaccaaacccccctggaagaaaaatattaccgcgcccagctggaactggccaaagaagcagggctccccgtacaaattcacaccccccaccgcgataagaaaaaaggaacccagcgcagtatggatattgcactggaacatggtttggagcctcacatgatcattgtagaccataataacgaggaaacagtcaaagaagtgctcgatcgtggcttctgggctgcgtttaccatctatccattcactaaaatggggaatgaacgcatggtagccgtggttaaacagtatggaagtgaacgtattatggtgaattccgctgccgactggggaatcagcgatcccctggcagttcccaaaaccgccgctttaatgcacgaaagtggtattgacttgaatgacattcatttggtaacttacaccaatgctgtaaaagcctttgcgcagagcggccagattaatgaagcagattttgatgtagcagcaaatattgatcaaagtgagaaatttaacggaagctctatactacgtggaggacagcagcctcgaattgataaaaacacaaccatcatccggtaacggcctgacagcttcgtccctgctggcaatgaaccatgaaaacctaattacgcggtgagttatattgttagcaaattatttggatacctacgcctgatgcgaccagccaacatcgtaactgcaatagcagatatattggcaggcgtcgctgtgtcggcctattttataaatgttacgttcagtactgttacactggatcttacgctgccggtggtatgcctgtgcctcgctaccatggggctctatggtggtggcgtggtattcaatgatgtatttgatgccacactggatagtacagagcggccggaaaggcccatcccaagcggggtaatctcaaaaacacaggccattatcctcggcagctacctgctcctggtaggtatcctggccgctttttccgtaggccgccttaccggctatgccggctggctcgccatcggcgtagctgccagcgcactcgtttatgataaatgggggaaacatcattccttcctcggccccctcaacatgggactttgccgcggacttaacctcctgctgggcatcagtattgtaccggaaatgctggaaatatactggtggatgggattcatccccattctctatatcgccgctgttaccaacatcagcaggggagaagtacatggtggaagcgtgaaaagcctgcgctttaccgctgtatgttatgcactggtatatattacaatgggtatcctggcatatatgcaccaccgcttctggctggcactgccttttatcgcgctgtttattattatgatcaatgtgccgcttttcaaagccatgaaaaacccttcggggccaaatataggaaaggcagtgaaaggaggaatcatcgcactgattgccatgaatgccgcctgggtggccgcttttgctactataccattcgcaattgccgtaatattattgttaccgatatccctggtactgggcaaaatatttgccgtcacctgatcacattaccggtgtccggccacaagccgggtaccggcaccattattccggtgatagctattccgctattccccgcttcatcgcttcttttaccagcccggcggtattcttcaccgcaagcttctgcgtaagatttaaccggtgtgtttccaccgtacgcaaactgataaacaacaggtctgcaatctcctggttggaatattcgtccgcaatcagtttcagtatttccttttccctgcgcgtaagcggaatctcgtaattaatgcgcttttgaccggtaatggcttcattcactatctgattcctgattaggtcgtcgagaaactgcccgccggcatgcacctcctcaatagcgcggataagcgtttccggatcagtgccttttaacaggtagccggcggcgccattacgcagcatttgcttcacataatgcgattccataaaactgctgatcgcaatcacttttacagacggatgctttttcttcacctgcttgcaaagcgctatgccatctatttcaggcatctggatatccagtaataacacgtcgggttgtataccgggtaaagcctccatcagcgcgcccggccggttgctttcataaacaacggaaatgtgcgggtaaggcgtaagcatcgccttgatgccactgatcaccagcaggtgatcatccgtgatagccagtttgatactcatcttctttttaaattaaaacgatgactgcacttccatcagctgcataatggcaatattaaattctatatatgccgttgtgccgcaacccggtatagccgtcagcgttaggtgtccgtttaatgatttgatccgcgtatgaagattctttaatcccataccggtcgtgcttttcgcgatatcttcaaagccaacgccattgtcctctacggtaatggtaagcaactggtcatgttgcgtaagttgaaccagggcttcggtagcatgggcatgcttaatcacattgttgatcagctcctgcacaatccggtataccgataattcaaagttgcccctgaaccgctgcatgtcgccggaagtatagaacgtgatctgcagcttccgggagtgactcacattatggcagaataattccagcgcacccgcaagccccatcctggaaaggatttcaggcatcaggttatgggcagttttccggacttcaccaatggcgtcgtccagcatgctgagcgcatggttaaagcctttgtcctgctgcagaaaagtacgttcatatttgagcgcccagaaatgcattttcacggcggataacagcccgccaacgccgtcgtgcaggtctttcgacaagcgcgtgcgctctttttcctcgccttgcatcatcgcctccagcacctgtacggttttttctacttccagcgtttgaagctgctgtttttgtaaacggtgccggtgcagtagtttctgccatatcaggaaagaaccaaccaggatcagtattacgccggcaaagatgaaaccaagccacctgttcttccgctgtaacagcaggtctttccggatcagctctaattttttctccgccaggtccctgtcttttttctcagactggtactgcatttccagctgctgtacattcagcctggtggcattccctaccagtgaatcattcagctgctcataagccttccgcagttgaaaggcccgctggtaatgctgctgcgcggcttcattgtcggatgccgccaggtaagcccgccttagttcatcgcccgcataatattgcctggccagggtaattgttttctgtagatagataccggcagcggggtgcttcccgctccggtaaagggcattggcatatcccatgtataactgcatccggttttcaagcccgggatcatcagtggaaataagcagcgctttttcaaaggttcgcaaggattgctcatgttgcgaaagatccgtatatacccgcccggttgcagtaagcgcattcagtaccagcagctggtcgccagcttttttaccaagctccagcgcccggttgaaatacctgccggcagccgtatagttcccctcccggcttttactttctccaaggttgagcagggccgccgccatgcgcgaattgctgcccagccggcgcccatgatcataagcctgcaccgcataattaaaccccttcttataatctcccagggaaataaaaacatccgataaatagttcatgatcatgcccgtgctggcactgtctttcgccgcatcggccagtttcagcgcttccaggtaagccgccgcagctgccgggaaattcgccatctgctggtattccatcccgcaatagctgatggccctcacctggctaagcgtatcttttagggaagcataaatgatcaccgcctgcttcagcatgtacagcgactgcaaatactgcccccgcatatcctggatatacatatagtaacacgcaaaatcggctacccctttatggtaccccaattgcctgctgatccgcaaggcacgcatgaagacggcagccgacttatcaagctggtaaggaaaaagccggcagccatagtcaatcagcgcctgtacctggtttgcacctgccggctgccggttaatcgtttgcaacacactgtcatccgcaggaaacggggatgcctgcagcaccccgccgctgcccatcgaaatacaacaaacaaaaagtaatattctcagcatttctgattcacttttacagcccggaaggctgttattgttaataattcaaggttaccggttatcacgcacaatgaatgccccggcggataacagccggaaagctattacccgccatcgcgcagtgcgttgacaaatgctcagcatgcaacaaaagatgtgaaatacaaccgatgttacagggttaacaacatgggcgtcccatgtttttttggtcaaacaatttaattctcagactgtgaaaccgtcgttcatttctacagcggcctaaagttcagtatttctgttttaatacgcaacagcgtatgggatgaacggaagcaggagcggatcaggagatcgggagaactacgtagattgcctgctggtaaggcattggcgggtgccctgcgcacataagtagaactacgcaatttataaaataatggtttataccgtagctaaaaccgggtaaaacagatttctttgcataccgataaattgattctacagactaaccccaaaaaaacaggctccgttcccggggcctttttctttgtaaaaaatcacgtttttctatgtacttttaaaggctatagttttttttagtcagatgatgcggatttagccatggaatatattcaacaaaacttcaatgtcaacttctcttacggtgttttctttagcagtaatttattcgatcctgccaacacctgtttagctaccttcctggaatcaaaagcggagagtgcatacgttaagaaattactcgttatactggatggtggcgttgcaacgcatcacccggaactaacccaacagatcaatcagtactttcaacaggtgcgcggctttcagctggcccctgaaatcatcaccatcgccgggggcgaaggcgtgaaaaatgatctgcccctgcttttcagcctggtcgatgccatcgataaatatagcatcgaccgccactcctatgtgataggcatcggcggcggttccctgctggatctcgtggggtttgccgccgcaatttcacaccgcggtgtgaaacatatcaggattccaacgaccgtactgtcgcaaaacgattccggcgttggcgtgaaaaacggcgtaaactataaggggaagaaaaatttcctcggttcctttgcgccgcccgcagccgtgttcaacgacccggtatttttaaccaccctggacccgcgcgactggcgctccggcatggtggaagccgtgaaagtagcccttattaaggatgccgctttctttaaccgcatagaagaaaatgcagtgacgctaaccggcggtgatatggccgctatgcacgaacttatttaccgctgcgcagaactgcatatccaacatatcggcggcgccggcgatccgtttgaaagcggctcctcccgcccgctggacttcggtcactggagcgcacataaactggagcaactcaccaactttgaattacgtcatggtgaagcagtatctatcggtattgcggtcgacagcgtatactcgttcctgttaggatggctctccgaaaaagatatgcaccgcattctcacggtattaaaaaatatgaaactgccggtatggcatcctttgctggaaatgcaggatggtaagccttccccggtggtagcaggactggaagaattccgtgaacatctcggtggccgcttaacaatttccctgctgcgcgcagtaggaaaaggagaagaagtgcatgaaatggaccttaacttattatataaagcagtagctatctgcaaaaataatcagtaatgaaaacagctgcaggacatcttacctactgcacaaatattcatcccggcgaaaactgggacgaccactttgcgcaactcaaaaaatttatacctgccattaaacaacaggtatcaccagataaaccttttggaataggattgcgactggctaataccgccagcctggaactgagcaaggaagcgcccttgaaggcatttcagcaatggctccgggaagaggattgctatgtgtttacgatgaacggttttccttatggcggctttcacaacgtagtggtaaaagaccaggtacatgcgcccgactggaccagcgctgaccgcgtagcctataccatccgcctgttcaggatcctggcagcattgctgcccgaaggtatggaaggaggtatttccaccaatccgctcggatataaacactggtgcaaccgctgcgaagaagacaagaattcttacacagaaagcgctacgctgaatatgttgctggtgctggaacagctggtgcgcacacgtcgcagcggcggccctttgatgcacctcgatattgagccggaacccgatggcatgatggaaaataccagcgagtatattaactggtacttcgaaaatttactgcctgccggcatcccgtttatcaaagagaaatttaatatagaagatgaccaggcagcagccgatatcatcaaaacgcatattcagctgtgttacgatgtttgccattttgcacttgtatacgaagcaccccagcgggtcatcgaacgcatgcagcatcatggtttgaagatcggcaaactgcagatcagcgcggcgctgaaagccgatatgcccgcagataccaccgcacgcaacgaagtaacagacgccttccgtaaattcgatgaaccggtatatctgcaccaggtgatcgcgaaaagaaaggacggcacttttattcattatcccgacttaccggaagcgctggcagatgaaaataatgcagccgttacagaatggcgctcccattttcatgtacctgtgttcctcgataaattcggtgtattgcaatccacgcaggaagatataaaacaagtactggccatacaaagggaacatccttttacacagcacatggaggcggaaacatatacctgggacgtgttaccacccgcccttaaacagaagatgtctttatccgtttcccgtgagctgaactggataagggaacagttataagtatctttgcatagtgccgcgcggcgccaccggataaacaccggtagccccggcggcaacacgcaatcttggaattgtccccccggtattatagctttatgccggaattgtaacggcgattgaatatatgagaaagacagtagtaattgatgtagtagggctctcctcttctttgctggagtacctgccttttttaaaggcctatacacaacagcggcacctggccaccgtaatgcctatgttacctgcggtgactacggctgtacagagcacgtaccttaccggcgaatggcccagtgagcatggaatagtaggcaatggctggtacgacagaaccgatgcggaagttaagttctggaaacaatccaaccggctggtagacgctcccaaaatatgggaccgtgcccgcaaactggatccatcttttacctgttcacaaatgtgctggtggtacaacatgtacgcgaacgtggactactcactgacaccccgtcccaactatctttccgatggccgtaaagtgcccgattgctatacttctccatctacactccgggattatctcaccgaacaactcggcaagttccccctgtttaattactggggtcccaccgccagcataaaatcaagccaatggatcgctgatgcgtctatcctcacggataaactatacgatcctacccttacttttatttaccttccccatctcgattactgcctgcagaaattcggacaggacccggtaaaaaatgcaaaggaactggcagaaattgatgcggtatgcaaacagctgattacttattatcagcagaagaattgtgatccgattgtactgtcggaatacggcattaccaatgtgaataaccccgtgcatcttaacaggattctgagggcagaagggctgctggccctgcgtgtggaaaatggcctcgaactgctggatgcaggcgcctccaaagcattcgcagtagcagatcaccagatcgcgcatatctatatcaatgatccttcctgttataaaaaagtacgctccatcctggaaaaggtgccgggtgtacaactggtgctggaccgggaaggcaaacggcaacatcatctccatcacagccgcagcggcgaactcattgccgtagccgatgccaacagctggttcacgtactactattggatggatgacaacaaagcccccgatttcgcccgaattgtagatatattccgtaaaccgggttatgatcctgtagagatgttcatggaccccgcagacccgctcattaagctgaaagcggcaggaaaattgctcaaaaagaaactgggtttccgctacctgatgaacgtcatcccgctcgatgcaacccttatcaaaggctctcacggcaggatcgaagaaaaccctgcctatcacccggtggtcatcagttcccaacccgctcccaagtcgcagctacaggcaacagacgtgtacggggttatctggaaccagctgacaggcaaataacggctccgcaatgaccagtaatcagccggcaggtaaataatcctccggttgtattaacttattcataaccatctggttacgactacagggctgttctaagcagcttcaaaaaaccgcctataacccaatgataaacaatcagttaccgatcaagtccacctcacctccgcatcaagagcacatttactccatgtcctaagtatcaccaaagcatctccaaagcatatccaaagcatcgcctatctaactttgcttcatatcagaggtatcatacgcctattcatgctctatctttaaaaatctcccaaaaaccgtctaaaaaatccaaaaatctccaaaaaatccaaaaaactaaatcagtataatcagcgtaatcagtgctcaagacaaaacttgcgttcgcgcgttcatcaaaaaaactcccccatcactgatttatttttctacattcatgcaaccgattgaaacgaataaataatatcaccgttatggaaagaagagattttctcaaaaccggtagcatggccggattgggagcaggattaaccatcctcaatttccccgtatttggaaaaaatgcccccagcaacaaattggtactgggcgtaatgggtgttaattccaggggcaactggctggcacagtgtgcagcgaaactgcccggagctgaaataggctatgtctgcgatgtggaagacggcgccatcgccaaagggctcaaggccattgcgggcgctcaggaccgcaaaccggaagtaattaaggacatccggaaactactggaacggaaagattttgatgcactcatcgtggcaacgcccgaccactggcacgctcctgcggccatcatggccacggcggcaggtaagcatgtgtacgtggaaaaaccctgtgcacacaatccgggcgaaggcgaaatactgctggcagcggcaaaaaagcacaaccgcctcgtgcagatgggaaaccagcgccgctcctggcctaatctccagcaggcagtaaaagaagtgaaagagcaaaacgtattgggaaaagtgtattatggccgcgggtggtatgtaaataaccgcgaacccattggtattgggaaaaagatcccggttccaggtacgctcaactgggacctgtggcagggacccgctccccgccgcgattacctggataacattgtacactacaactggcactggcgctggcattggggtacctccgaaacctgcaacaacgctacccacgaattggattgcctccgctggtttatggatgtggaattccctaccaaagtcacttctgccggtgggcggtatgcttatgccaaggatgactgggaaacaccggatacccaaaccctgaacttcgagtttgaaggcaataaagccatcgcctgggaaggccgcagctgtagcccgtttaacctggaaggcagcggccgcggatttaccctgtttggcgaaaacggaagcctgtataattccggcggcgacagctacaaactgatcgacaccaaaggtaaagtgatcaaagaagtaaaacaggccgccaatcctaaccagagtgtaaccaataccgttagtcccgccggtgagttttatgacgctgtgcatatcaacaacttcctggaaagtatccgcggcaacgctaccctcaactccgaaatcaatatcggttaccgcagtacgctgctttgcctgctaggcaatatagcgcaacgcaccggccgcatccttcataccgatccttccaatggccatatcctgaacgataaggaagccatgaaaatgtgggaaagggagtatgaaaaaggctggacaccgaaagcataaatcagtaaaacgggttccgggtaatagtgctgcaagcacaaaatttgtaaaaaaatgcttgtactattacccggaattcctatctttacgaagttataaaccctttctcctattgggtttataggctaacaataaatataatatcttgttatcccccataacttttagttatcgttgtaattaataatgatcccctacttttgacctacctgtaatttttataaccaaccacaccaaccacaaaagttgcgcgttccccggagggatgatttgaatggagtttttacaacaatctcagtacctgtcagtattgctgataggcttagtagtaggctatttgtccggtttattagggaaagggggcagtgccatcagcacaccagccctgcagatctttgcaggcgtaaacccgttttttgcactggcatcgccgctgccggcatctatcaccagtactttatctgccacggcagtatacagtaaggagaaactgtttaataaacgggtgatcctgctgggggctgctttcggtgtcccggccactgtcattgggtcttggctcagcagttacctgcccggcaaaacgctgatgatcatgacagccctctttatcatggccacaggtatgtcgctcatgtattcctttctgcgcagtaaatcaactggtgaattaaccgtagtaagtgaagatgtgccggcgggtaaattagtggtagccgctttgtttatcgggtttttatcagggctgctggcaaatgccggtgggatattgttcagctctttctttataaagaaattaaaaatgcccattaaacaggcgctggcctgtgcggtagtgttatcggctgttttatccatacccggcgctttaacgcactggtggctgggtcatatagactggaatatagcgctgctgctgtcgcttactgcattccctgcttcctggctgggagccaaaacggcggtgaaaatgaaaacgcccgtcctcgaaaaattatttgcacttacccttatcgtatttggggtatacgatatcttctttactatctggaagtaatcaggcatgcgccttcatcttatggatggcttcctgctcataagggggcaggctgctcacgataatttcgtaggcattctgcaggaatgtttccagctcggtagccggcagcatatcttcctgtttcagctgcacccagtgataccgcgccaggtgaggggccggtacaataccaggtctcgaaatcaattcatgaaactgcgattgactgcacttaaacgatacccggtgaggcggctccagggatatcatgcagaataatttttcgcctacgtaaaagcgcaattcgttgtcccacttttgttcagtgatgacagccggaagtgaccggcacagatcaagggtatgatcaaacatagcagcaggttttaaaagaatattatttagggccgttttttaaggacgacatgtgtcaatagtttacatgcacagactaacatattaaaatatgaagtatgtgtggttaacgtaaatctaagctgtaaatagtgaatgaaactgccctataaaaataggaaataaaaaccaatcctgaatgttaaaatgaactttccttccggcaggaaattcctttgccccgtaccagcgggtatttcaagggaacatcgttttttttcttaatcgaaatttaatcccttccaggcaaaaaagtttcggcttgtactatcacccccaggggtgtaatacaagccgaaagtcaatatggataagcctttattaaggttgggcagctgcccagcgcgccattttttgttccagcaccgacagtggcacacaaccatctttcagcaactcatcatgaaaagatgataagctgaaccggctgccgagcgactttgtatactggttccgcagtccgcggatcttcagttccccgatcttataggaaagcgcctggccgggaatggccatgtaccgctcaatttcagcggtagcttcctgtgtggataccggctcattatccatcatatacttgatggcctgctcacgggtccagcctttggtatgcaaaccaacatccacgactaaacgaatagcccggtgtatttcatctgttaaacggccaaagtacatatatggatcggtgtataatcccagttcttttcctaaactttcacaatacagggcataaccttcgccataggcgccaatccacgagaaacggcggaacttaggcagggagtcgttttcctgttgcagggaaatctggaaatgatgacctggaatggcctcgtgtaaaaaaaggcattccataccggtatatgaaaagtccgctgcatcaaggataggcacgtaaaatacgcccggtcttgtaccatcggcgctgccctgcatatactctgcggaagcggaagcagcccggtaagcttcggtttggcggatttcaaattttgttttgggaagatgaccgtacatcttttttacacccggcatgatcttgtcctcgatggctttgaaagaatccaggacagcagcaggtgttttaaagatgcgcagcttcttatcagtacgcaccgatgcaaaaaaggccggcagatcgcctttgaagccagtgctgttcttcactgcttccatttcaccgcggatccgtgctacttctttttctcccaaagcaaaaatttcttcgggggtaaggtcggtggtcgtccagctttttatcaggaaagcataatacgccttaccatcaggaatagcgccaatgccgctgctggtgcgggccttagggaggtattcctgctgcatgaagtcgcgcagctttgcaaaagaaggcaggatgtgtgtttcaatggccgcgctgtactctttcaccagggttgctttggtggctgcatccagcgaatccgggatcgttttcagcggcgaatagaatacgttgttggcagtatctttttttgccaggtctgttacctgcggaatcactttcaccaccaggctttgcggcaatacatagccggtggccattcccctgcgcatattggcgatggcggtgtcggtccatatggcaaagcgctccatacgatgcatgaagttatggtagtcctttagcgttttaaaaggttgggcggaagaaccggaacccagttgcgccagtgtgatgggtaggcaggtgaactgctgcactggcatcaggtgatcgtgaaaggtaagcccctcgcggttgatgctgaactcccgttgcaacatgtcataggtaatacggtcgttgccggagagtaccgctgtatcaatgcctttgattgcctgctggtagctggcatagaaagaatcggcttttacgcggtagccttcactgatatctatcggcaactggtcgttgtattggttttccccgttctgggtagcctgcaacgggttcagggccatgctttcattgtagtaccgcgtggccagttgacgcagggagtcctgcgtggcctgcggattactatgactgcccggttgctgacaagccgcggccagcaaagcccccgacaggaggaggtagccttttcgttgtaacattttcatattgatgggttgtgaacaggtagtaatttaccgttttatccaagaaaaaaagcattccgaagaatcggaatgcttatttagaacagtgaacaatgaaaaaaaaggtaaaaaatattatttaagaatttttatacgaatacttttgaaagaaacctcattaccatggtcctgtaaaaggatgtgcccttcaggccacagaccaaaattcttccagcttttatacttgctgatcgccaccagatccttgaaggcctgggagccacgctcgtattccaacactttaaatccatttaaccagtgttctacgtgattatttggatacacaataatacgacctttgttccattctccaatagggttgatggcacgtttttcctgttttcttgtcatgaggtcgtaaagacttgctaaagtacggtttccatcgcgtcctaatttggcatccgggtgcttttcgtcgtccagtacctggtactccagcccgatagccgacttgcctcctgtttcgtaggactcgctcacgaagtattttaccccgctattggcgcccggcgtgagtttgaaggtaaattccagttcaaaagcaccgtattgtttctccgtaataatgtcgccgccgctgccttcttcatctcccgtagaattaccaatggtgagcacaccattctgcatggtccagccggcagtggggaaattctttttatacacgcccctccagcctttgctggtttttccgtcccacaacagctggtagccgtttttcttttcctggccggaaatagtgttatccacattattaacaacgtagatgttgtcgtagggagaatactgggaagcagccgggttttctatcagccttacatttttccagtagatatttttgttgtcgtctgccgcatttttgccgatgctatgcacctgtaaagcgatgaaaccctttggtaatgcggtatctaccaggtgggcagtaggcacgccattcacccaggtacgcatttcattgccgcggcactcgatgcggtatttgttccagccgtcttttttaaaggcattctgaccggcagggttcagttccatcgggtactgccagcctctgcggccttcttcataaataccaccgctccatttacggtcggatgggtcaatctccatctggtagccaaatacacggccattctggtagtcaggcctgctttgactgcggaactggatcccggaattgaattccttgcccagcttgaattccagctccaggataaagtcgccgtactctttctcagtagcaaggaaagagttaggcgtattcatcaccgtggtgcccacgatctcgccattctgcacattatattttgcttcaccccccagttgtttccagcctttcagatctttaccattgaaaagctgctgccactgggctttctgagcgaaaaggccaccatacatacacagcagggtgccaaataaaaggatcgtctttttcataacttaaacggaataaggtgaccaaaataaacaatgaaaatgatttttacaaccgattgcaaaactttaatcttattttttattttttaaccacatgataatctgaccaatatggggttttacagaattagaaataaaaatattcatgcaaacgattgcagcaatgtaaaaatatcttattttggttccgaaagtatccacgtagcaacagccaaaatcgaaaaagtaatactctttatctacaatcattataaactacgttatgaaaaaagttttttcacgtcttatctgtatgatagcatgtttgctattctaccaactcacccaggcacaaggcaccccaattaccatagaaggtaatgttctcgacgcccagaagcaaccactggtaggcgtaaccgtttctatcaaagggaaaaatgcaggcacccagtcagatgcccagggacatttccggctcaaagttacagatgccgccaacgcagtactcgtatttacctacatcggatttaacacctatgaagaacctgtaaaaggtcgtgcaatcgtttccgtagttttaacagaagaccgcaaaaaactggaagaaattgtggtggtgggatatggccagcagaagaaaaaagatgtaacaggttccatttcctccgtaggtaccaaagctatccaggacgtaccggtaaccaacccgcagcaagccctacagggccgcgctcccggtgtggaagtactcaacaacagcagcaaacccggtgatgaacccactgtgcgtatccgcggcagccgctccctcagagccggcaatgaccccctctatgtagtagacgggatcccttacgccggtacactcagcgatatcggtacgggagtaatacaatcgatggatattttgaaagatgcctctgcaacggctatctatggctccaggggcgctaatggcgtagtactcattactacccagaaaggcaaggaaggaaaacccgtggtttcctataccggctcctacggttatgtacaacagctcggcgaatccgatatgatggacgctaaccgcttcatagaaatgcgccgggaagctaaccgcaccatcggtaaatacgatgatgccaaccccgatgcctccgacaagaaaatatttaataccgttgaatacgcgaatatccagaaaggcacaaacgtagactggcaggacctgatgatctctcccggatatcaaaccaatcacggcctcagcgtagccggcggtacggaaagaacaaaatacaccgtgggattgggctacttcaaagaccagggcgtactgaaactgcaggactacgagcgttataatttcaatgtgggcatcgaccagatgatcggcgaccgcgttcgcgtgggagctaccctgttgggcgcttacagtgaacgtaacggcgaaacctacaacgggatagacaatgccctgaaaatgctgcccatcgccgctccgtacgacgacaatggaaagctgatcacctatcccaccggcgatagccagcagcctaacccgttactggattatgtacccggcaaccgcgttgaattaatgaaacgtttccgcatcttcaccagcctgttcgcagaagtggaaatcatagatggtctgaaataccgcctcaacgtaggtccggatgtgcagaactataactatggtcttttccagggtaaaaacaataccaacctgctgatcggcggtggcgacgctacagctaccaaaggaaacgctgctaccatggcgtataccattgaaaacatcgttacctacaacaaagaaatcaaaaaacataatatcggcttcaccggtttgtacagcgtgcaacgtcagaatgtagatatttctactaccaacgtgagaggtatcccggtagaaacacaacaatattacaacctgggtcagtcgctcaacgtaaccggcgtaaccagcagccttagttcctggaccatcctttcctatatgggccgtttgaactacgggtatgatgatcgctatctcctgaccctcacccttcgcgcggatggatcttccaggtttgcacccggcaaaaaatggggttatttcccctccattgcagcagcctggaacatggtaagtgaaaagtggctgaaagaacagaaagtcctggataacctgaaactgcgcgccagctttggccgtatcggtaacaccggtattaatccatatgctacacagggtaacctgagcaggattccttattccttcggaaataaaggcgtactgggctttgtaccgctcgatctgcgtaatcctaatctcacctgggaatctaccacctctaccgatattggtattgatttcggattcctcaacggccgtatcaccggtgtggtggagtggtacaaccaacgcactaccgacctgctcatgccacaatcgctcccgttcagcaatgggtttaatgaagtgctgatgaacctcggtacttcccagaaccgcggttttgaattcggaataggcgccaccattatcgacaaccctaatgggttcagctggaaaatggacgccaacatgttcctgaacaggtccaagatcctgtcgctcggcgatggcagaacagccgatattggaaacgcctggtttgtgggtcagcctacctatgtatactatgattttaagaaggtcggcgtatggcaggaaaaggatgcccagctggctaaactttacaacctgaagccaggagaaatcaggctggaagatgtaaataaagataccctcattgatgctaagaacgaccgccagatcctgggctccccgcagcctaaatggtctgcaggtaccacccagcgcttctcctataaaggatttgaattatccatcgtggcctttgcccgtatgggaagcatgatcaaaagtgatttctaccagaactataacaccctgtttggccgttataataacctgaatatcgactataacacaccggccaatcctaccaacgatttcccgcggcctaatgccaaccaggaaagacccagcaactaccagtcgctgagctactttgatggttccttctttaagatcaggagcataacactcagctacgccttctcggacgcagtggtgaaacatatgcgcatgcaggatctccgggtaaacgtaggagtgaaaaatcccatgatcctggcgccttaccgccaaacctggaaaggagttgatcctgaagacgtaaatgtgatcggcatcgatgcaccagccacctggatgctgcagttcggaataaatgccaaattttaaatcaacggatcctgattaaacatctttaaaagaaaacgttatgaaatatatagttcctctcatcatactgctggccgttggtaccgcctcctgcaataaaatgctggatgaagagattgtcaccaacgtaacagatgatttctataatactaaagccggctttcaaacagccgtgaatggctcttacgtgtctatgcgcaacttctacagcacggaacgcggtatgacgcttacggaaaccggtaccgatattatcaccaacggttccgacggtaacttcaaatttacaagtcagtatacttcacagttggattcccgctacgatcatatcagggaagtgtggaacagtttctatcaaaccatcaacacctgtaacgtggtggtagaccgggccgacaaggtccccgacctcgaggaagcaacaaagaaaaaaggcgtggcagaagcgctgttctgccgggcgcattatcattttgtactcatgcagatgtttggcgccgtacccttacgcctgcacgaaaatgcggaaattataagagaagctcaccgcgactccgtatctgccatctacgatgccgtgatcaacgacctgcttgcagcagaagctgaattgccggctacacaggcagaatggggccgtgccaccaagcccgccgcagagcacctgctggcaagggtttacctgacccgcgcctcctctccgcaggcaaaagcaggagactatgccaatgccgccaaatacgccgacatggtcattaaaaactatggtttcaaattactcaccgacgttggacaggtatgggcacagggaaaagaaaacaacgatgaaactatctgggcagcgcagtataccaccgacccgctgtatggttacgctgataacaacgcctgccgctttttcctgatgcagtacgatgtgctgaaaggaatgaagcgcgatttggccaatggcacgccctggaagcgtttcagacctacaaagttcctgatcgacacactgtataaagacagggtacacgatgtacgttatgaaaaattctacaccaccctgtggagaaccaatgcaccggttgacaacctgaaaatgggcgataccgcggtgttcctgcctggttatgacgtacccgacgcagtgattgccaccaaaccttatatgctggtgccgccaagattgtacactgaaaagctgtatccttctttgaataaatttgccgatgcgctccgtccggataaccaggcttccggcgtaagaccctttatcgccatgcgtcttgccgaagcttacctgatagaagcagaagcgctgatgatggatggcaaaaaacaggaagccgccgacctcgtaaatgtggttcgctggagatctgcacgtattggcgctacacctgccgaaacacaggctaaccgtgatgcgatgaccgtaaccgccgcagacatgaccatcgattttatcctggatgaaagaggccgggaactggtaggtgaacaattgcgctggtttgacctcacccgcacccataaactggtggaaagggtgaagctgcataacgacgaagcacgtagtaacatcaagcttacacatatgctgcggcctattccgcaggaccagatcgatagaacagtgaatgagttcccgcagaacccgggatattaatacttctttctttttaaaaaaaaatcaaaaaggggctggccaggtaaaattggtcagccccttttttgaccttttttgctacttttagcagaaatcaaccaatagctgaggagggtagcatatttcaggatgtccaataattcagacaacgagcgggaactgctccggcaggtagctgccggagacgagcaggcgtaccgggtattatttgaccggtactcggacaggatgtatatgaatgcgctgcattttacgaaatcagcagaactggcgcaggacctcacacaggaaatctttatccggatatggatgaaccggttaaaactggccggtgtagatcgctttgatgcctggctgtttacagtggccaggaatgtaatccgcaatgagctaaagaaaaaggtgctgccggtagagaacggggagatgctgcatgcttatttcagggacaataatttaacgccgcaggaacggatagaatataaggagctggaaacatctgttcatcaggccattaaaaacctgccgccacaaatgcaaacggtattcctgctaagccggcaggaagggttaacgcatgaagagattgcccgccgcatgaatatttccgttgtttcttccaaaacctatatggtccgctgcctcctggcgattcgcaggcatcttggcaaaaatgccggtaaactgggaatcgtgatctttttcctctacagataaaaaatatttttttccaaacgtcttacccctgcttatctggttgtctttacctggaatgaccttcgggttgcaggtactattaccattttaacaacgcatcattatgtcgccatccgaatttcagcaccttgtacaaaaattcctggacgatagcattaccacagaggaattgcagcgcttccggcaatgggtgctggaagaaagagacgtagatatgcaggaagccgcaatagaagcggtgttgcaaaaaagtagctaccctggtgaaatgccggcagataaacaggtagtatttagttacatattggaagaagcgaaccgtcgcactgctccgctcccgcgtgcaggagtggtgggcatgcgcacctggtgggcggcggcagcggttttattattgctgggtacgggcctttatttccttacccgtccgaaagcacatatggaaatagcgcaacgctccaacaacatcatccatccaggcagggaaggcgccatacttactcttgcggatggttcgcaggtggtactggacagcctgaaaaacggcgtgatcacgcagcagggaagcaccgacgtacagctccggaacggacagttgttgtacaacagccggaatggatcttcatccgcttcacttgcctacaacacggtggctacgccaaggggccgccagttccaggtaatactgccggatggtaccaccgtttggctcaatgccgcatcttctatccggtatccggttgcttttcccgcaggagaaaggaatgtgatgattacgggagaagcctacttggaagtggccgctgatgcccgcaaaccttttaccgtggaaacagacaacggcacggccatccaggtactgggcaccagctttaacgtgaacgcctatacggatgaatcggcattacgggctaccctgctgcagggaaagatactcgtaaaatccgctaccgccagcaaggtattgttacccggtgaacaggcggtggtagccggatccattacggtagatgcgcatgccaataccagtcaggcaattgcctggaaaaacggcatcttcaatttccagcgagccccgctggaagtggtaatgcggcaaatcgcccgttggtatgatgtagaagtagtatatgaaaaaaatatcccggccattactttcggtggtgaaatgggacgggaccttgaactgaaagacgtgctggaattcctgcaggaatcaggggttcattttaaattatcgggaagaaaactgacggtcatgccttaatttttttatcaaccaggtcatatgccacaaaaaaaccggaagcggttcgaagcacttccggttaaagattggcttaactgagaaaacaagtcccacaagactgcttatttatcaactaaaccattgcaaagctatgcaattaaatgctctttgtaaccggtccgggaaaggtatgcgacgtccgcatgcccctggagcaccagctatgtgcagcgcccggttgtcaactaaaatcgaaggatccctttaccgaacggggatcccaatactgaaagtcatgaaactgaccatgcttcttcttacagctgcattcctgcatgtaaccgcgggcagctatgcgcaacagatcaccttttccggaaaaaatgtaccgcttgagaaagcgttttccgtcatcagggagcaaaccgggtacctggtggtgtataatgctgacctgttgaaagatgccagaaaggtgacggtagatgcgcataacatgcaactggaaacgttcctggaccttgcgttcagggagcaaccgctgaaatatgtgatccggaacaataccatccttgtaaccgggaggccccggccgcagcaggcgtcgaaccccgcacaaaccagcctggcggctgcccggccagtcctgttaaaaggaacggtggtcaatgaaaagggggaacccctgcctggtgtgaccgtgctgttgaaaggtactacccgtggtaccgttaccgatgatgacggcgctttcctgatcactgccgatatagaagacggcgcaacactgatggtaaagatgatcggctataccccgcaggaagttgccgtgaatggccgcagcgatatccgcatcgcccttcaggcagatgtgcggaacctggaaaacgtaaccatttccacgggatataaaaagattcctaaatatcagctgaccggcgccgcttctgtgataacgcaaaaagaatacgatcagcgtgtagccgttaccggtaacttcctggaaagcctggaaggcaaggtccctggtttagtgtataacagtcagtccggcgagttatctatccgcggcgtttctacctttgatgcggtaaagaagccgttgatagtggtggatggctttccaacagaaatagaccttaacactatcaatcctattgatatcgtttctatttccgtactgcgggatgccgccgccgcggccatttatggcgtgcgcgcttccaacggtgtaattgtggtagaaaccaggcgggggaaatccggtaaggcaaaatttagtttgcgcgcgaccactgcgttgcagcagtcgcccgattttggctacctgaagtttgccggggcaaaggaatttgtgaccttacaggaagcacagtttaaacgtgccaatccgaatgaaatcggctataccgcttatgaccggcctatggctcctgccattgccatcctcttcgacgagcagcaaaaacgcattagcccggaggtagcaaggcagaaactggattcgctggggagctatgataatacacgggaatacgaagacctctacttccgtacacggcaggccaccaatcttaacctggatgtaagcggcggaaatgaaaaaagcacttacctgctgggggtgaattacattgcggagcaaccggtgaatgtgggatcgaagaacaaccagctgatcctgaattttgccaatacctaccagctttccaaccggctgaagatggattttcgcggcgtgtattcgcatgcggaatcgaagaaaggtactaccgctcccatgaatgatttttatccgtatgaaaaactggctgatgccaacggtaccccgctgccggtagctcagggagtgaacagggactatctcaactttggtgtaaaccgcgcaaggaacaaccggctgatcgccctgggattgtatgaccagctttattatccttaccgggaactcactgccaatacaactaaggtcaacacaaatgcgtttcgggtgcaagcccgcctggaaggaaagatcacagactggatgtctgccgaagtaggcggtaattatgaacggcagcaagggatccaggacaacttcctggatgaacaatcttacaccgtacgcaggctgctgaaccttaaagccaccaaagaccccagtggaaaacctatgttcatcgacattccgcagggtaatattctccggaggacagatcagaaagccatcaactacacactgcgtgcacaactgaattttgataaacgttctgccaacagccggcatgaaatgtcgggtatcctgggcgtagaacagcgaaaaaccactaacgacagctatcttaacagttacttcgggtatgacggacaatcgctgatcagcagacccgttaacctgcaacgtgcgagcctttatatcaattctgccttcccggatgtaacccagttcggcggcgctcttgccatgagggattatgtcaatgaaaccagtgccgaccggcgctttctttcctactatgcacaaggcacctatatctacaacagtaaatatattgttaccggtagttaccgtatcgaccagtccaacctgtttggtgtggaccccaaatataaatatcgtccgttatggtcagccggcgccgcctggcggttgcacatggaagattttctgaaagacaacacctggatcagtgagctgaagctgaatgctactacgggtttcaatggtaatgtgccggtgagtaacaacggccccttcctgatcctggcttcgcagctgaacaatgtgtttgtggttccccaaccatccttttatgtgataacacccgagaaccagtcattgcgctgggaaaccacccgcacttataacctgcgcctggactacggattctttaacaaccgcctgtttggttctgtggattattattataaaagaacgggagatgtgttcggacaatacgatgctgatcccaccagcggttttaaccagtacaatgccaataccgctactatccggaatagcggcgtggatctgctgatttccaccgtgaatgtacaaaaccgccggttcgggtggcgtacaagtcttaccgcttcattaaacaataataaagtactggcggtaaaagccagtgaatatgaaagtacagaggatataaccagtagccgtattaaccggcagggttacccgatggatgcgttattcagctataattacggcggactaacgaacatgggcaaaccatttgtgtatgaccggaaaggaggccagcatatcctgtatttttatggtaatgcaaaggtagatgtagcatttgaggacctgatctacaacggtactaccactcccaaatatgtactgggcctgaataaccagttctccgtaggcgcttttgacctgtcatttctcttcatgtattatggtggtcatgtgatgcgggtagaacagcccaatcctgtaaacctgagtacttacagcacatcattactggaaggatctgccaattactggaaaaaagccggagatgaactgcataccaatattcccgggtttacaccaggtgctgcacaggatccattctatttttcttcgtatgcccgttacggttaccagtatgcatcgcagttcgtacgccgggcggattatatccggttgcgtgacctgatcattacctataacccgaagtttaattttataaaacggatgggacttagtcaaacgcagatccggttacagggccagaacctgttctactatacgtttagcgggaacgacattgatccggaagcgatagaccggaccagtggggtgcgccaattgccgcaacggccactttacagcatttccctttttactaacttctaatcattcatctatgagatcaatcaatattgtctttatccttttacttgccatcgctgctttttccggctgtgataagttcctggaagtgaagccaaaagggatcgtaattccggagaagctgagcgactaccaactgatgctgaattccaggtcaatgacgcttacttttccgcctgcattgttgtattgtacagacgattattacgaggaatttgatgacctgagcacagtaccgccagccaatgcttattactggcgccctggcattgaccagaatgaaaaagagaatcccgcagcgtggggcgatctgtataacactatttacaatgccaatgtaatcatcaataatgtaatggctaccacagatggtacaccggcagcccgtgcttccacactggcggaagcgctggtgatccgtgcagattgttacttcatgttgctgacgctgtttgcaaaagcctataatccggccaccgctgccaatgatccgggtttaccattggtaagaagcacgaatgtgaccgataaaacgccgccgcggtcttctgtacaaacaacactggatacgatccttaccaatgtaacggatgccatcgcatcgctgccgctcaccaatctcaacaagtaccggcccacaaagtacgctgcgtatagtttgctgtcgaggatctatctctacatgcaggattatgaaaaaacgaaaaagtataccgacctggcattaacggcgccgcacagcatggttaattataatgattacgaagatccttactcattcccggaaacggacctgagcccggaagtactatggcaacgcggttcgttggattatacgatcccttctatgatgggcatgcaacacgcgctgagtgatttatacgaacccggtgatctccggaaactgttgcttacttatgcgtttgacgactttcctgatgactattacttttccggcacaaacggctatgccaattttggcacaacgttccaggaaatgtacctgacaaaagcagaaatgctggcgcgtgataatcaaatcgaggccgccatgaacatcgtgaatgagctgcggaaataccggtttaaaacagacgcttatacgccgctgactgctaccggaaaggaagacgcgttaacgaaagtgttgcaggaacgcagaagggaactggctttccgcgggcaacgctggatggatatgaaacgcctcgaccgcgaagggcggatgccattggtagagcgcagcgtgcacagcaccggcgctttgaaagccacgctggaaccaggcagcaagaagtatgttttccagatccccgcccgtgtacaacaatttaatccagacatgcaattaaatgaccgttaatcatcttatatgaaaaatattattcccgcactgatatcctgcacactgctgtttacaaccgctgctgcgcagaaaacgactactacgctttcaggaaaattgagtggcaacgatattaccacaccgctgcacctgaaaaatatggccggcgccgacctgctgattcctgtaaatggagacggcacctttcattcaaaagtagccctgcctgcaaagggattttattccctcaccggcgtggggcaggtatacctggagcctggctaccagcttcagatggcactggcgccggatagtacctaccgcttcagcggcaagggcagctttgaaaacaatgccactgcagacgcacggaaagcattatccaaatatgtagccaccgaccccgaacatatgcttgggcaggaagctttgtatacccctgttccggaatttatcgggaagatggatgctttcgtgaaagatggacaacatttgtttgaccaatcctccagcgtatttttccgggagatggccggtaaggatctggcctactacggtaaatatgtgttagcccattacagcctgtattacggaacagacctgaagaaacaggaggcattttataaactgatggaaaccggtaacaggaaagatacagcataccagcggctcatgcaggaagcaggccgcgccatgcatgtgaaaaggcttgacagcacagaacgtgcgcagctggataaactgacaatgagcgactgggataagaatgatgctgcattgtttcaacaatccgcctggtacagacaggtgctggatcagtatctttctactatccagtactacaagtacaggcatctatttgaagcatctgtagaagataataatatacggaccctgatgggattgtatatttcaaagggtgaaataagtgattcttttatgctccggtattacacttatacaggcacccggaatgcattaaaaatgctgaaggataaaccggtgcgggatagtttgtataacagttacgtggctagtgcaaagcaccctgcttacctgaaagagatccgggaaatttaccgcaatgccaatacttacagcgacaatacgcctgctcccgatttttcttatgaagatgttaatggcaaaaaagtttccctgaaagatttacgcggtgagtatgtttatatagatgtgtgggcaacgtggtgtggtccgtgtaaaatggaaatcccgcatttgtcgaaaatagaagcgctgtatgaacacaaaaagatccggtttgtaagcctgtcggtagacaaaagtgcagacaaacaaaaatggatagattttgtgcagaaaggaaacctgaaaggcatacagctgctggcggataaagattttcaatctgatttcatccagaaattcaatatcaatgccattccgcgttttatactgatcgggcccgatgggaagattgtgagtgctgatgcgctgcggccgtccaatcctgcgctacaggcattgttggataaattgctggcggaaggataaatgccggcagataaaataaaccggtatctgctactgtattttatgagtagcagttaccggttatgatgaaatgaaaattaaagcgttattttaaatatcagccgggaggtggtgcgggaaactgtaaactgatggtcctcaattacaggatcagttacactgatataaaacggtttacatttactgtctgattttatttccttattaatataagacagggtagcacttcctacagagggaatgtttattttatatttgaatgcgcccttttttgtatcagcaatatgaaaaatcagtgatccatacataggcgctcctgatcgtttttctatcactccccgttctgaaggaagatctgccggctccggggtaattgttatagtggcagtatcaatattttttgacaaaagaatattctctcctgtttgtccatctataaacattatccccacctgggtaggcatgccttcgctcagtacgtcttcacagggatcggcgtgttttgctttctgacaccctggtccgaaacttacggcacccagaaataacagtggcagataaaatttctttgtaagaaaataggttaattgtttcatttctatctggaatttgctttgatatagggtaatgatgagcttaacatgaaaactttaatggcttgaattataaattcatagccgaatttaaacaaaaattattacgggagtaaaaaaatgcagcaggagatcacaccatgatcgtttgctgcatttttgctaaaagctaaatgcgtatcttcatcagccttttttaacgcaataaaactttcaattctatggcacagaaaaagatattattactgacaggagattacgcagaagattatgaaacaatggttccgttccagatgctgcagatgattggtcatgatgtacatgcggtttgtccggataaagcggcaggagataaaatcaaaacggccatccatgattttgaaggagaccagacttacagtgaaaagccgggtcatgggtttgtgttgaatgccacttttaacgatgtggccggtgctgattacgatgcgctggtaatagccggcggccgtgccccggaatacctgcggctgaataaaaatgtgctggagctggtgaggcattttttcctggaagataaaccggtggcggctgtttgtcatggtatccagatcctgacggctgccgacgtggtacgtggaaagaaactgacggcttacccggcagtagcgccggaagtaaccgcttccggaggtacttatgtatctgtaaatgtttacgaggcggtggtagatggcaagctggtaacggcgcccgcatggccggctcatccgcagtggattgcagcgtttcttcaggtactgggaaccagcatcaccctgtaaccgataggtatgtataaatagttgattatcagaagaggaaagaaagtttaaattatctttccacggattttcaaattaaacggccattgcttacctttgcagccaaattcaggaggctatccctgcattggtcattgataattcgtaattcgtaattgatttttatatatgtccggacagcttaaagaagttcgtaaccgaatcaaatctattcaatctggtcagcagatcaccaaagccatgaaaatggtaagtgctgctaaattaagacgtgcacaggatgccatcatgctgatgcgtccgtatgccgtaaagctccaggaaatgttgcagaatattgtttccaacagcgaaggcaatatcgatacaccactggcagctcagcgtcaggttgaaaaagtactggttgtggtcatcacttcagacaggggtttgtgcggcgcctttaactccaacctgatcaaaacagctaaacgtgtgatccgcgaaaagtatgctgaacagtttgaacagggccaggtagaaatcttaccaattggtaaaaaaggatatgatcactttgtacagaacggttacaaagtaaatgataagttctggcagctttttggcagtcttacttttgatcatgtgaaagaagcggcagcagtagcgctgcagggttttaccgatggtacttacgatgccgttgaaatcgtttacagcgaattcaaaaatgctgctacgcagatctttgtagcagagcagttcctgccaatcgcgaaagtagaaaataaggaaaagagtggtctgaaagcggacttcatctttgaacctgaaaaagataccctgattgctgaactgatgcctaagatcctgaacacccagttcttcaaagccatcctggattcccacgcttccgagcatggcgcccgtatgaccgcgatggataaggctacagaaaacgccagcgaattgctccgttccctgaagatctcttacaaccgtgcccgtcaggctgctattaccaccgagctcacagaaatcgtgagtggtgcggctgcattggcgaactaaggatagaggggttattaacactaagtcaacaactgaattaatattttcagattagggtcaaagactgtattttcggtctttgaccttttttgtaaatccacatctcctgttaacgtatggaaatatcacagatcatcccgcacgtggaagcattaattttcgccgccgaccggccgttacctttgctggaaatagtggatctgctcaacaatgcactggcttttctggaagaccgtaccaacctggatcaggtggaagccgctatggaggcgatcagggagaaatacaactctgaattttatgctttcgaagtacgtagcagcgggggaggctaccagttcctcaccaaaaaagagtattaccagacagtggcgcagcttaacggggataaattcctgaaacgcctttccactgccgccctggaaaccctggccatcatcgcctaccggcagccgatttccaaaggcgaaattgaatatatccgcggggtaagcaccgattattctatccagaaactcctggaaaaggaactgatcgtgattaccggccgcagcgaagaccaacccggtaaaccgctgctgtacgccgtttcccgctcctttatggattacttcggcatcagctccgtagctgatttgcctaaactgaaagaattatttgatgaggaaatggtgcaacctactcttatcaccgacgataccgctaccctcggccggggagaacataacacccataccgccgaagcggaaacagtccattccctgatggtgtcggaagacggagaactcctggaccccgatcaccagctggatcacctggcgccccccgccccggacgccgaagaagagccgcccgcctcagaagatgaggaagtagaacctgacgatgaaattgttcgttttgatgatattattgaagaagtaaatgaagaactcagcggcggagaagaaggtgaaagcgacaccagcaccaccgaagaggatggggaggaagaagacgaagacccttatgccgtaaaggataccgctactcatagccccgacgaagagaatgaagatcctgatggtatcgtggaagatgtcatctccggagaagaagaaaaagaagatgatgtggaagaggagaaagaagaagatactgaagaagatgatgatgaggacgatggcgataaagatccggatgatatgatggaagatgccattttaggcgagaagctgctggtggtcagcggacccggtgtggaagatgaggaggaagaagaggaagaagaggaagacgatgaagacgacgacgatgatgaagacgacgataatgacgaaaaaaacgacaattccggaaaaaaataaagaaacagcggctcatcgaagccgctgttttatttaaaaactcaaagtaatcagtataatcagcgtaatcctgagaaagacaacctacgctacaatcccgcaatcacccccgcaaaaagtccgctcagcaatttatccgccttacccgctacggcaataatttcttctatggaaacggcgtgcaggttatccgggtcgcattcatccgttaccacggaaaccgcagcacaaggcaattgcagctgattggccacaattacttccggcacggtgctcattcccaccaggtctgcgcctatcatgcggaggaagcggtattccgcccgtgtttcaagattgggacccataacggatacgtatatacccttttttaacgtggtgcccagtgaggcggcagccgcctgtaatttgttgcccagttccgggtggtacgggcagctcatatccgggaagcgtggaccgtatgccggtgagttgagcccccgcagcgggttttctggttgcatattgatatgatcatccagcaatacgaggtcgcctttcttaaaatccggattcatgccaccggcggcattgctgagcagcagctgctggatgcccagcgctttcatcaccctgatggggaacgtgatctgttgcatcgtatagccttcatagtaatgaaagcggccctgcatggcgatcaccggtgtatcgccgatatgcccgaggatcaggtggcctttatgtgattctacggtagattcagggaaatgagggatttgctggtagggaatggaatgggctattttaatatgatttaccagttccccgaggcctgtgcccaatactacgcctacacgcggctgttcaaaggaaaaggattgcagataggtggtagccgcagctatttgttgcagtaacaggtccatacgtttgttgaatttgctgcaaattaattccctttgcgcgcaatcacgtaaaacagtggtggaaaatatcttttaatccatagcaggagcttttcttcccgggcgatgagcactattttttttcgtttatgcatggccctgaggatctgctgcgcgcagcggtcaaccggtatgccattcgcctggccggggtccattttcccgtaaggctcgccgttggcagtgatggcggaataggtaatgggcgtgtgtatgcggcccgggcaaacaatggtggtatataaccgggggatgggttgttcggtttgcagtgtttcgaagtatccctgcagggcgtgtttggcggcgttatagccggagcgccagggatagcccataaggccggccatgctgctgatcaccacgatctggccgctgccctgttctttgaaatgtggcagcagggctttggtgagcatcaccgcgccaaagaaattcacttccatcagttggcggatagccgctatggaggtatctatcagtttggaccgttgcgtaacgccggcattattcacaaggatatctatcttcccaaaaaactgaagggcgcgttgggcgccttcatttacctggacttcatcggttacgtccatcagcaatatttcgcaatggggtgtgtacagcaggcattggttgcgtactgcttccagggcgggctgattccttgctgcgagtatcagccgggctttttcctttgccagcaaaagcgccagctcgtggcctatacccgagctggcgcctgtaattaatattactttatccgtaaagtacattcaacggtgtatttactttaaaggcaccagtttgatgtttttccatcttaccttgataccgccgccggaatgaatttggagggctatctggccattggccgcgccaatcttgtcatctttcagggtgatcatttcatgaccattgagccaggtggttacattatcgccctgcacctttactttcatggtattccattcgcccattttcaggaacttttctttctctttatcgggctgaatgagccatccacggccataagattcgtagataccgccggtatgcatatctggcggcgctacttctgcctgccagccggtgattttggtgccatctaatgaagagtggaagaacacgccgctgttgccattggcttcctgtttgaattgtacggtcagctcaaagtccttgtactgcccatcggtggccaggtagccgtattctttatccgggccgctttcgcagatcagttctccgttttccacgtaccacttctctgtaccatatactttccagccatcgaggtttttaccattgaataaagactgtgctttttgtgcgaatgcactgccggagcccaataacagggcggttcccagtaaacaattgaaaaaggtttttttcataacactgctaagatttagtgattttcaggtgaatgaagatcagtcattgatctataaaaaaagtcccccggtaaaaccggaggactccaatataagttcaaattcctgaattattaaatcagaaaactatcttgctatattcactgctcttttttcacggattaccgttactttaatctggccgggatattgcatttctgtttgtattttattggcaatttcaaaggataagcgatctgcgtctccatcggaaactttatcactttctacgatgatacgcagttccctgccagcctggatagcataggctttttccacaccatcgtgggcaagcgccaggttttccaggtctttaatacgttgcaggtagctctgcatgatttcgcggcgtgcgccggggcgtgcaccactgatagcatcacaggcctgaacgatgggagaaataacatattgcatttccatttcatcgtggtgggcgccgatagcatttaccacggcggcatgttcgccgtatttttcagcgagcttggcgccgagcagggcgtggctcagttcagtttcttcatccggtactttaccgatatcgtgcagtaagccggcgcgtttggccagtttagggttcagtcccagttcagctgccattaccgcacaaaggttagcggtttctttggagtgcatcagcaggttctggccgtaggaagagcggaaacgcatcttacctaccaggcgtaccagttctttatggaggccgtggatacccagttcaataacggttctttcaccgatatccattacctgttcttccagttgtttcttggttttttctactacttcctcgatacgtgcagggtggatacgtccgtcctgaacaaggcgttgcagggataaacgggcaatttcacggcgtaacgggtcgaaggaagataatacgatggcttcaggggtatcgtctacaatcaggtccacaccggtcgccgcttcaatggcgcggatgttacgaccttcacggccaatgatctggcctttgatttcatcgctttccagggtaaataccgtgatggtattttcaatggtttgctctgcggcagtacgttgaatggattggataatgattttctttgcttccttgttcgcttttaatttagcgtcttcaatgatttcctggatatgagagagggcctgtgagcgggcttcttctttcaaactctctaccaactggtgtttcgcttcgtctgcggttaagccagccactttttcgaggcggcggatgtgctcttcctggtgtttttccagttcggtacgtttgatggttaccagttccatctggcggttcagggtttccttgatcgcctcattttcatttaattgcttctggatttgctcgtttttcaggtttaatgcctgttccttctgtttgatgcggttttccgattctcccagtttctggttgcgctgcaatacgtctttttcgtattcgctttttagttgcaggtatttttctttggcttccagcagtctgtcttttttaagattttctgcactgatctgcgcatctgcaatgatttttttagcctgtagttcagcttcgtctatcttatgctgcgtatttttggcaaaaatcaccttacctagcacaatcccaatgatcaatgccactactgcagctattgtcgtgataagtgtaacatccatatgaattatttatacttgatttatgtagtatcctcatacccatatcgctgctaaaacacgacaggggcgagaactgacccgcgaaaatacaaaaaaatagcagttaaagcgtgtttgatacgtgataattagccaattagctaattcattgttaagcaatgggtaacgtgatcaacccaatgcctggttgataatttcctccagcttttccagcttctcctgcaaaaaaggcgcagtactagcctgggctttaccgccgctggttacaggatgcgtggcgtacatgataagggccatagcgatatagtcctgcaggtctttccctgcataggcagttttaaaatcgacgatcttctcattcacttctttcataatacgacgtacttccgcttcttcttccggttttatcttgatccggtaagagcggtctgctacgataatattaacaggaatgagttgctccatgatgtatgatttttaattcagctgttcagcaaagcgatacaacggtcaatttctttaatgtaatcattgattttgccccggatctcttttttgaacgcttcgtcttctgctgctatggtggtacctccctgggcggtagatgcaattttcatcagttgcagtctttcctccagtccctgtaccgcctgttgctgctgttgcagctcccgttgctgtatgctcacttcttctttcagcaatgcattctcagcctgcacctgctggagcttttttaccagcaggtgcaatttttcttctacacgttgaatgtattgctcgagcaccatttcatttacttattttcttatctccgcctgtaactgcgtttcaaacgttttgataagtttgtccattacactgtcaatttctttatctgtcagtgttttctgagcgtccaggaaggtaaagctcacggcgtaagacttcttatcagtacccagtttttcgctctcaaatacatcgaacagatttacctgttgtaacaggcccgatttcacgctgcgtgcggctgtttccacggcggcaaacttaacctgtttgtcgagcaccagtgccagatcccttctaacggcctggaatttcggaatttccttgtaaaagttatcacttttttgcaagagtcccagtattttatcccagttgaaggtagcaaaccatacaggctgacggatatcaaactgcttcagtttagctgtgggaacgcctcccagtgtcaccaccacctggttttttaccttgatatcccaggatggctgcaggcccgcttcggtgctttccacccaggtgaactgcttataacccagttgctgcaggatattgatcacaaaacccttcaggaagtaaaagtctaccgggctggatttgtgcatccaggtttccgctgtttttttaccggtgagatataataccaggtgattattttcgccatagcctttttccagcacctggtaggttttaccaaattcgaagaacaggaggtcttcgtttttgcggttcaggttatgagcaatgctttccaggccggtttccagcatggacgggcgcatgatgtccagttccacggtaagactgttcatcatcttcaccgcatgctccagtacttccggcgtatagtatttactgttagtgatggagttcgtgaatatttcgttgaacccgttgccggcgagatagtctgcaatcttctccttaaccctttcagcgtccggttgggcggagagcgcaggcgaaatcgctattttagccggtatttctatattatcgaggccatcgatgcgcattacctcttccaccaggtcggccggcaggctgatatccggtttgctaaagggcacggctacccggaggccttcggtggtttccgacaggatatcgaagcccaggctgcgcaggatgtttttgatcttatcgccgggatagttgccgccgctgagtttacggatatagctatacgtagtttccacctgcgtttttacttttacagccggatatacatcgatgatctcagaagctgcttttccgccgctgagctcacagatcaggtctgcggcgcgttgcagggcgaacacaacgttagagatatccactcctttttcaaaacgggtggccgcatcggtgcgtaacccatgacggaacgacgtggtacggatgccaccggcgctgaaaaaggcgctttccaggaaaatgttgtgggtggtatcggttacgccggagtgcaatccgccgaatacgcctgctatgcacatgccttcgccggcgccgttgcagatcatcaggtcggtggcatccagttttctttccttctcatccaatgtaacaaagggcgttccctgcgggaggttcttcaccacgatggcattgccttttaccgctgccgcatcaaatgcgtgcagtggctgaccggtttcatgcaggatgaaattggtgatatccacaatgttattgataggacgaacgccaatggcggtgagcctggctttcagccattcgggggatggcgccacctgtacgccggtgattgaaataccgctgtaccgggggcaggcatctgtattttcgatggtaacgctgatggctaaaggagcatctgctttgggcagggcctttatttcaggcagctgtacctggtatttatgcgtatgttctaaattattaaggaatgcgcaaacatctttggccacaccaatatggctcatggcgtccatgcggttgggggtaagacctatttcgaagatgcaatcctgtgcgggtttaaagactttactggcaggagtgcctggctgcagggaggcgtccagcaccaggatgccgtcgtgactgctacccagcccgatttcgtcttccgcgcaaatcattccctggctttcttctccacggatctttgcttttttcatggtcagcggttcgccgctcagcgggtaaatggtggtgccgatgggcgccactactactttttgtccgggcgccacgttgggagcgccgcaaacgatgtgcaggggctcgccgttgccaatgttaacggtggtgagtttcagcttgtctgcgttggggtgtttttctgccgtcagtacttctccgattactaatccagccagacttccctttactgcttcaaatttctccaggctttctacctccaggcctattctggttaaaatggtagacagttcctccggtgtaggcttcaccggtaaataatcacatagccagttgtatgaaatcgtcatttatctgctcggtttatataagtggcgtaaagttaacaactagaattgattttcgggctttgcggcttatctgctttgattctttgaaattaaaaatagcccaaaaccgctacagtgctgtatttttgcaggatgtggaaaatctttttacacaatgtgtgtgaataatcggacctttgccagggaatttcctgtgttttggtggataaccatggcgctgtcagtggataactgacattttgcttgtggataacctgtgtatgaggcttaataaatttaataactaaggagagggtattaatcggaaaaatgcctttaccttagtttgtacggcttgaaaaagtttacaatttcttaacgtagctatgacccctatagaatgcgggaaaatgcagatatcgattgtaaaaacaacaggaaaggcccattgacagtaaccttttattaactttttttaatacactaaccataaatggatctcaatcttaagaaggaccgcaatgtgcgcagaaaaccgtccattgatgtgtcatccttggtgtatggcaagataccaccacaggctaaagaattggaagaagctgttttgggagccgtaatgctggaaaaaggtgcatttgacaccgttatcgagatattgaaaggggagtgtttctatgtagaagctcaccagattatttttagtgccatgacccgcctggcgggtaagtcgatgccggtggatatcctcaccgtaacagaagagctgaaatcgatgggctcactggaacaaatcggcggaccatttaccgtgatgaagctcaccaacatggtggtgtcttctgcaaatatcgaagcgcatgcccgcatcatcctccagaaatttatccagcgggagctgatccgcatttcgggggaaatcctcacagagtcttatgaagacactgcggatgtgtttgacctgctcgacagcgccgaatcaaagctatttgaagtaacaaataatcacctccgtaaaaactacgattccatcgaccgcgtactggtgaacaccatgaaacgcatcgaggacctgcggaataaaggagatgatattaccggggtaccgtcagggttcccttcactggacaaagtaacctatggctggcagtccacggatctgatcatcatcgctgcccgtccatctgtgggtaaaaccgcctttgcgctgaacctcgcgcgtaacgcggccctccacccccgcttcccgaaaggagcagcagtattttctttggaaatgtcgtccggccagattgtacaacgtatcctctcggccgagtcagaaataaagctggaaaaaatttcccgcggtaagctggaagaatatgaaatgaagaagctgatgacccatggtatcgaacgcctggcaaaagctcccatcttcattgatgataccccggccctcaacatctttgaactgcgcgccaaatgccgcaggctggtacataaccacggcgtaggcgttatcatcatcgactacctccagctcatgagcggcagcagcgatggtaaaggttccaaccgtgagcaggaaatcagtaaaatttcccgcgacctgaaaggactggcaaaagagctacaggtaccggtaatcgccctctcgcagttgagccgtgatgtggaaaaacgtaaagacggtaacaagatgccgcagctgagtgatctccgtgaatccggagccatcgagcaggatgcggacatggtaatgttcctgtaccgtcctgaatattatgaaatcaacaccaatgaaatgggcgaatccaataaaggtgaaacccacgttcgtatagccaagcaccgtaatggtcagctggataccatcaaattgagagccgtactggaatatcagcgctttgaagatgatggcagcctggagaaccccggtggcggcaatccctacgcaggcatgaaccgtccgcaacaaggtggcggcggcaacgatgaagcgaagctgtacatacagaaggggtccaaaatgaacgacatgaacttcgatgaaggatttgaagatgcaccattttagcgcataaaaagatattgctaaaagccggcatcgaaatgatcgccggctttttttatacgcggaggttgtcttactcaggattacgctgattatactgattacctggattttattttttgggattttttaaggatttgggtagatacaagcgatatattccgcttacatctacccaaatccttaaaaaatcccaaaaaataaaatccaggtaatcagtataatcagcgtaatcctggtaaagacaaaatccgcataacagaacaatcaatgaaacaactgtatttaaagtacaaaggtcattacaaagacaatttcagtttagcttaccccgtagttatttcccagctggggcacacgttagtagcattatcagatagtattatcattggtcataccgggaaggtgccgctggcagcagtatccctgggcaatggtttgttttccgtatttatggtggccggtattggtatgtcgtacggactaaccccgttgattgcacaggaaaacgggcgtggcaacaaaggcgccatcgggcatttactgagtcatagtcttattatcaatatggtggtgggtgtgttgctgtctgccgttatttattttggcagcgcccatttatctttcctgcaccaggaaggggatgtggcagatcaggcccggccctttctgcgtttcctgggattttcctttattccgctgatgctgttcctttccttcaagcagtttgccgaagggcttgggtttacccgccaggctatgaatatcagtatcatcgggaatgtgctgaatatcctgatagggattacgttggtgtacggcctgttcggattgcccaggatgggtgtgatcggcgtggggatagccacttttaccgaccgccttattatgggaattacgatggcgttttatgtgctgcgtgcgccccgcttcaaaccatacctgcaatcgttcgggtttaagaacctgaaggcagccgccattaaaaagatcctgggcatcggtacgccggtggcgctgcaatacctgtttgaagtaagcgccttcagtggcgcggctgtgatggtaggctggatgggagcggcagaactggcggcgcaccagatagcgttgagtcttgctgccatgacctacatgatggccagcggtatctctgcggcagcgggtatcaaaagcgggaataattttgggaagaaagatttcggggcgctgcgtttatccgccatcgccagttatcatatggtgctgctgctgatgggagccgctgccctgttgtttacgctgggtaatcagctgttgccgtcattttatatccaggacccgcaggtaatccagatagcttcccacctgctgatcattgcggctttcttccagttgtttgatggtatgcaggtggtgggacttggtattttgcgcggcctcggcgacgtgcgtattcctaccgtgataacattgctggcttactgggtgctggggattcctttgggttacctgttgggtatcaaattggattatggcgtggaaggcgtgtggtgggcgttgctgctgggcttactagtggcttctgtgctgttgtttgtgcgtttccaggttaaaaccaggaaactacggatatcatctgccggataaaacccatatcatctccgtatactatcttcgcacatcaggataatcaaaaatatatgtcagttttttacgcgccggaaatacagcaggatgccgcagtgtataccatgaatgaggatacttccaaatattgtatccaggtgcttcggcatgaaaagggcgatgaggtgttgctggcagatggacgcgggcacaaaattaccgcggtgatcaccgatgataaccgcaagaaatgtgtagtaaagattgtttcttctgaaacgatgccggcgcctgcgcgggcattgcggatcgctatctcctttacaaaaaatgcctcccggatagaatggttcctggaaaaagccacagagataggcattcaaacgattatcccgctggtaagccagcgtacggagaaagaaaagatgaaggcggagagattgcagaatatcctggtgtcggctatgctgcaatcgcagcagttttacttaccggaattgcaggaaccacaggcttttgaaaagctggtgaaaaataataaagatccgcagcggctgattgcgcattgtttgccggagcagaaaaccccgttgcagcaagtgatgcagcctgcaaaggataccattatactgataggccctgaaggtgattttacaccggaagaaataaagctggcgctggacgaaggctatatacccgtatcgctgggagatacccgcctgcgtacggaaacggccggtatggtggcggtaacactaatgaatgccagttgggcgtaagcccgcacagatctttttcacgatcgttgggccctcataaatgaacccggtatacacctgcaccagcgatgcgccggcatccagtttttcctgcgcatcttccgcggtgaaaataccgcccacagcgataatgggaatcctgccctggctatgcgtgtggatatagcggattacttctgtggctttcttttttacaggtaaaccgctgagtccaccggcgccgatatcatttacttccgctgccggtgtttttaatcctgcccggctgatagtagtattggtggctacaatgccggcgagttttgtttcttttattatttcaataatgtcatccagttgctcggtagtgaggtcgggtgctatcttaagtaagataggtttcggttttactttctgtgcattcaatacctgcaggtgatgcagcagttgtttcaacggctctttctcctgcaaggcacggaggtttggtgtgttgggagagcttacatttaccacgaaatagtctaccacatcatacagcgcatgaaaacacttttcataatcgctgacagcttcttcattcggggtcactttatttttcccgatgttcccacctactataatattggatcttttgcgttgcagtctttttgcggcagccacagctccttcgttattaaagcccatgcggttaatgagggctttatcttccggcaggcggaataaccgcgggagttcattacccggctgtgggagcggcgttacggtacctatctccacaaaaccaaaacccaggcaggccaattcatcaatgtactttgcatctttatcgaaacctgccgctaagcccacgggattagaaaaggtaagtccgaatatttcgcgttccaggcccggggtttttactccgcaaaaggcgttcaggatattcttgccaagtggcagcgaataaattgttttcataccacgcataacgctgtggtgaatactttccggcggatagcggaaaaggaaatttttaatcagattgtacattgcgggaacaaagataagcattacgcgattgggagcaagacagggggcgaattttgtgtagtttggggtaagacaaaattcgcgtaagtgaaaatccttcctatatttgcccttcatcatgctggagctccaaacatttgaagcattatttaaggaaaaccatgctcattgcctggcctttgccactcactataccggggatacccatgtagcggaggaaatagtacaacaggtattcctgcggttgtgggaaaaaagggacactatcactattacaggcccggtaaaagcatatttgttttctgccatccgtaataccgccatcagccagtggcgaaaggatgttgtgcgctcggaaaaggagaatgggtatgggaaaataacagaaacaacggttggcgcgggggaagaagtgaaggagctggagcggttgtaccgggtggccttggaaaagttgccggagcgctgccgcgaagtgtttatcctcagccgccagcagcatatgaaatatgcagaaatagcggaagcgatgaatatttccgtaaaaacggtggaaaatcagatgggcaaggccctgaagatcctccaccaggagttgaaggagtacctgccgttactgacaggattcctgttctaaaaatatttccgggcgcataggggcatctgtatttcgcgtgcgtcttcttaatatattaccgcccgaagggcgacgactgtaaaaacttacaacaactgatgacaccatcttttcctaacgaggcactgcccgatgaggcgctgtataccttgctctgcaagtatctgctgaatgaagcggatgaggaagagcgtgcgtgggtagaagcatggagggaaacggaccccggtaatatggccctgctggtatcgctggggaaagtactggatactgctgcggccaacgaaaaaacagtggcggcagataccggtagcgcctgggcgcaaatccaggaaaaaatggatgataagccggcattgattgccatcaggtccaaaccccgctttacctggctgaaaattgccgctgtactgctggttgcattgggcgccgggttgtggtttctcacccgtaatcagccggaccaggtatattccggcccggtaagcgcggtgctcagcgacggaagtaagattgaattatcagcaggtgcaaaaatggaagtggccaggggctttaatgaccgcaaccggaaagtaaccttcagcggtaaggccagttttgatataaatggcagtgcggaaaacccttttgtgatcatacttgggcataacgaagtaaaagtgctgggtacccggtttatgatcaattatcaacccggcgaagccacgctgaaagtacatgtgagcaacggtaaggtaatggtgattaatcatgataaaaaagacagcgtagtgctcaccgatggtatgttattacaaaaggataacgacaagcccgctttccggatcgcttcccatgtaactgatatgggtaaacggtcgttgtcgttcaacaataccccgcttgaagaagtactgcatacgatcacagaggtgtatgatgttaaaatagaagtaatggacaccgacctgctgaaactgccggtacgggccagctttacagatgaatcaacagaagaggtgatgaaatcgctggcacttatgctgaacgcatcatacgaaaaagtaaacgaccgtcaatacaaattaaaataggttttagccgtcaactaaagctgtagtcacactttcaattcagatatactatgtcgttagccttaaaactgctgacgggaatattaatatgtagtttccccttacaggttttcgggtgggactggcaaacaagagtaacaatagtagcaaaggatctgcccctggaggcagtatgtggattactggaaaaagaatatggtattcatttttcatatagcagggaacttgtcaacttgtcccggaaggttacgttaaccgcccatcagcaacgtcttaaaaaattactggacgaattattttctcccgatgatatccgtttcacccgtgtaggcgatcagatcgtgctatcgcccgcgcaacgcagcagccgcaccatcagtggttatatcaaagatgcggtcagtggtgaaaacctgattggagccactgtttattcacctgcgctcaaacagggcactactgccaatcagtatggtttttatagtttaactacggtgaaagacaccaacagcctgctgatttcttacattggctacaagccttatctgcaaaaggtaaaagctaagggcgaccagctgatcaacatccacctgcaacccctgggcagcttaaaagaggtggtgatcagcgcaaaggagggcagtaagctccaggagcaaacgcagatgagcagggtgcatcttagtacgtctgatttgcaggcaatgccgcggttactcggtgaagtggatgtaatgcgcgccctgcaatcgcttccgggcgtaagcggtggtaccgacggcgccggcggcttatatgtaagaggcggtggccctgatcagaatctcgtgctgatagacggcacgccggtatttaatttctcccatttcttcggcgtatactctatgctgaatgccaacgtggtaaaaacaaccgacctgtataaaggcgctttcccggcacgcttcggcggcaggatatcttctgtggtggatatttcgatgaaagaaggggatatgaagaattttcatggagatgcgtccatcgggttcattgcggctaaatttaatatcgagggacccatcgtaaaagacaaaacatccttcatgttttccgcccgccgttcttacccggatctgctgctcaatgcagctttcaaatcagataatacactgggccccgatggagattttaaggcattcttttttgatgtgaatgcaaaagtgaatcatattttttcatccaaagaccggctattttttagtttttataagggagaagataacctgttgctgaaacagacggtgcctgatacgtcccgcctcagcagtccgtcgaagtacattgctgaaagcatccggttccggcttggatggggtaataccattggcgccatacgctggaaccatatctataatcccaagctgttttccaatgtaaccctgaactattcgcaatacgaattttttacagaaattgagcataggtatatgttggccgcttccggtgaaaaggcggatgtatacgggaaatacaactcgaggatggagaataacggtggcaggatagattttgactaccgcccggatccccgccattctattcgatttggcgccatcactaccatacataaatttaaacccggcaactccagtttcgaagacagggacagccaggtgataccattggatacggcggatgcatcgttgaaagtaacgggctatgaattgtcgttgtatgcggaagatgactggcagatccggcctgatttttttgccagcataggcttgcacgcatctgcgtttttggtggaaggccgtttttattactccctgcaacccaggctgggattgcgttacgtgctgccccgcaactgggcggtaaaagcggcgtttacgcatatgaaccagtatatccacctgttgtccggcgatggaactaccttgcctacagacatatgggtgccatccacgcaacatgtagcgcctatgttttcgcggcaattggctgccggcgtagctaaaacttccgctaacctgaagtatgaattttcactggagggttatttcaaatccatgcacaacatgattgaaactcgggaaaccaacggtatcattactactgccgctacccggtgggatgaaaatgtaaccgtgggtaaaggctggagctatggtacggaattaatgttgcagaagaaaaaaggaagcactacgggatggctggcatatacattggcctggtctacccgccggtttcccggcgtgaataacgggcatatctatccctataaatatgatcgccggcatgatattgaactggtgctggtacagcaactgggaaaacaatgggagctttctgcctcctggcattttaacagtggaacgccgtttactttgccggtatccacgtatgccggaacggagggctcctctccctgggagccgggtaccggtaatagcagtattgatcgtttcgacaaccggaacaattaccggggcgcggctgttcaccggctcgatgtgggtgttacctggagtaagcaaaaaaagtactggatccggagctggaacctgagtgtgtttaacgcctataaccagaagaatccttacttctattatatcagtgaagatgcggcagcgcaaaagcggtacctgtccagggtaagcatcctgcctatattacccagtattacttattcggttaagttttaaagagatgagtatgaaatattttttcgtaggtacgatcgggttatccatgctattgagcgcatgtgaaaagcgggaagaaattaagttgccttatgaaggcgataaaatagtggtgaacacgctgatacaaccggatagtgtggtttatatccgggtaacgcgcagcgtgccctccaacgtgtataacgatggcgtgtataaggatattcccggcgccaccgtaacgcttaccacaaatgaatcatccgtgatgccgttgcaggtacaaacgataaaaggactttcctactatgtgtctggccagaaagcggtgctcggacaacgatacaaagtggccgtggcagcggcggggttacaggcggtaacggctacggatacactcccgcaggccccggtggcatacaatgccaccgcgcagcgcagcagcagccgggtgcagttcacattgaaagaccagccagcctccgcggattattaccggatccgcatttatatgaccgatgcctccaccggaaagggcgccttcctgcttttcaggctggaccctgcctttaataataacctggttgactatttttcccaggataattataacagcctgatcatgaatgatgagcgctttaatggtaaacccgtgaacttcgttttacaaacagcagatcccatcatgaatgcaggtgaaatgactgtagaggtaagtgcgctgacccatactacctaccagtacttcaatactctcgccgcccaaaaagatgcagggatatccctggggtctcatgtaagggtatttaccaatgtaaccaatggctatggcattgttggcggcatcaataccaggaagatgacctttaaaatacagtgatccccgcggtgatataacatagctaaataagataatatcacagtgaagacgctgccatttaaagaaacgggcatgctttaagccgttttacggcgctatattaatacttcgctatatttttgttatcccgttttttatcttaaaaacctgctctatttttaggatatatatatttatatgcctgaacaattccccattgatcttattcaccggttacgtgctggtgactttaagctttttgagttgattttcaatacatactgggaagagctgtatgcctacgcagcaaaggttacgggtagtgaagaagatgcacgggatatcatacaggatttgtttgccagtatatgggagcgccggcagcagctggagctgcatactcatatccgttactacctgtttagcgcggtaaggaagcaaatcctgcgtaagttccgcgacgacggattaaaagaaaagcacctcgaaaaatttattacccatagtgagctgcggtccgaacttacccttaactccctgatccataaagatattctgaaccagctccagcaagacctccagcatttaccggaaaaagaaaggcaggtatttgaatggtaccacttcgatgagctgagcatccgcgaaatagccatgatgcatggcacggccgagcaaacggtacgtaaccagctcggaaacgcctacaagaaagcccgcccattgctgaaccgcctgttaatgttcctctgattttccctctccatgttaccttaacgttaagccgggattccggatagttaaaaagggtggtttgtgcaacttagtcataaacaccacaccttgatccgatcaaaaataaatgcactcatcggtaaatacctggaaggcaaagccactccagaggaggagcaattgcttacccactggctggatgcactggcagaagacgccggtccgggaacggaacaggatgcccgtagccgggaacggctgcgccgcagcattttaaaggtcataaagcaacgtaccggcgagccggctgccatatatcctgtctggaagaaactggccgcagcggcggcggtattgctgatggtgggcataggcagctggtggatgatgagttaccggtcgtcccaaaagatcgcctggctggaactgcgtacggccatcggtgaaaagaaagtgctgttattgcccgacagcagccggatctggctgggcgccaatagcgtactgaaatacccggaccattttacggatagcaggcaggtacaactggtatcaggggaagccttttttgatatagcccaggctccgggacaacctttcagcgtaatcaccgacagcctgcaggtgcaggtgctgggcacttcgtttcacatcagggcctatccccggcagctgctggaaataggggtgaataccgggaaagtgagcgttaacaaaggcggccaggtaatggatatcttaacagccaatcaactactgcaggttaacagaaataattatacttcttcccggttgtctgtatcctcaccagatataaatggctggaagcaggataaaatagtgttcgataatatgcccgttatggatgcattgatgttactggagaattattacccggtgaagttccacgttaagagcgcgcccggcaggcaaatcagcggatcgctcaacatgcacttaacaattacgcagatcataaatgtactggaagatcttacggatcatcagctgaaaataatacctgccggcgcaggaaattacaacatatatcaataaatatttattccctgaactgaaactaaaacaccggttatgaatgtacgtagtacccacttgcgtacaaggagctctgtgaaacagatatttcttgtagcgcttatgctgtcgctatgcggcagcgtcatgtcccagcaaaaaacaaccgtcgtgcaggaactgcatattaccgcaggcccgcttgccgacgcactgaaaatgctgcaaaaacaaagcggcgctgacattgtatacgatgcagctttattgaagaacctgacggtgaaaacacaggacttccgttcacagcccatagaagaagtattacgcgttttactgaaaggaagcgggttccacttctccgctacagaaggcgtatacatcattaaaaaagaaaagaacaaaacaacggtcaccggtaaagtcaccgacgaagaaaccggcgtgggtttacccggcgtcagcgtactggtaaaaggaaatacacaaggcagcatcacggatgctaacggtgctttttccttgcaggctgataacgccggcgataccctgttatttacttccctgggatataaatccacccgcctggtgttaaacgggcagcaacggttggcgattaaactgaagaccgatgccagcctgttaagcagcgtggtagtagtaggttacggatcaaccaccaaaggcgatcttaccggcgccgtatcccatgtaggcgctgaaaactttaataccggtgtattcagttccccggaacagctgttacagggaaaagtacccggcctgaatattacccgcagcggtgatccaaacgctacacccgcagtgatcctccgcggcccgtccactttccgcgatggtgaagcacaacagcctttctatgttattgatggtgtacccggcgctaatatccagctggtatctccgtcagatatcgtatcaatggatgtattgaaagatgcggcatctactgctatttatggtgcacgcgcagccaacggggtgattatgatcaccacccgccgcgcaaaacccggtcaaagctggatcagctacaatgcctacgtagccagcgagcgcatctccaattccatcgatatgatgtccagcgccgacctcacgaaatacctggaagacaacggtaaaagtattacaccggcttatgatgataacgctgataacgactggcagaaactcgtaacccgcaatggcctgtcgcacagccataacatttcctttggcggcggcaatgagaaaaccgtattcgacggaagcgtgaactacctgcagaataatggtatcatgcaaaaatcatcactggaacggctaaacgtaagagcaaacctggaacaacgcgcgttcaacgacctgttgaaactgaacctgtcgatcagtaacagcgtaagcacacaaaaccagatcccggaactggtgtttatgaacatgctgaactatatgcctaccgtgaatatctttaacccggatggtacttataaagaagatttctcccgtacacgcaactacctgaatcccttatcactccttaataacaacagcgaccgcaccaaaaacaagatcatgttggggaatgcccgtgcggagctcaatcttttgccgggtttgcgttatacgctgaatgtatctatgcaggatgagcagatcaaccgggacatttataacaaccgcgcttccggcctggcacagggcgttaacggaagagctacccgcagcgcctatacgaatacacggaaagtactggaaacctatttcaattacgacgtgctttttggtaaacacgacctgcgtttgctggccggctactcctggcaggaagaccgccgcggcgacggattccagacctccaaccagggttttgtatcagacgccacccaaggcgataacctgggcctgggaagtcccgatggcgccttccagcctaattttggtgccacccgcattcaaaccctgcgcttcatctccttttatgcaagagccaattaccagtttgacggaaagtacctgctgatggcctctgtaagaagggacggttcttctgccttcggcgcaaacaaccgctggggttatttcccggccgtatccgccgcctggaaaatcaataaggaaagcttcctctccggcgtatcctggatagaagatcttaaactgcgtgcaggctatggtgttaccggtaactcgctgggcttcgatccgttgatcgccacgctccggtatgatatcaccggtaaattttataacaacggcaggctgatcaacgctatcggacccgtacagaacgataaccccaacctcagatgggaacgcaccggcatggctaatataggcgtggatttcaccacgctgagaggacgcctcggcttcgcagtggattactatgataaacgtaccactgatttgatctactcctacaatgtacccgccacacagtattttgtatctaccatgctggcgaacgtaggctctatgagcaataagggtgttgaattccaggtgaatgcggtacctgtgaaaacggctcatttcaactggactacctccgccaatattgcacacaataagaaccgggtactctccctctccaatgatattttttctgtgaaatatattgaaaccgcagaacttggcggcaggggacaatcaggcaataaatcacagcgcgtggaaggcggatatgcactgggttcgttctacctctggcaatacgtggataaaaacgctgccggtctttcacaattccgcgacgccaaaggcaacctggttaccggccctacttccaccgaccgggtttataccggagacgcacagccggcctttacctatggctggagcaacagctttacctggcgtaattttgatgccaatatttttctgcgcggcgtatccggaaacaagatactgaacgctaccctggctaacctgaatgcaccttatgaagcgggtattatcaatatcccgcagtattccaaacaagagtcgcccagcgatgtaaatgcaccttacatctcttcccgctacctggaaaatggcgcttatctccggctcgataatgctactattggctacacggttcctatgcagaataagtatatcaggaaactgcgtttatacgtttccggtaataacctgtttatcattaccgattattcaggtattgatccggaaatcaatatgggcggacttacaccgggaattgacaacagcaatttttatccaaagacacgttctttcctctttggcttaaacgcaacattctaaaaactgacggttaaaaatagcgacatgaaaaatatttttatcacaggactagcaatcagttttactttactttcagcatgtacgaagctggatgtaaatgtggaatctgaatatgtaaaggaaaattttccaaccacacccgatggctttattgccgcatccggccccatttatacacaactgagcggaggctacgccgttgactactggcggatgcaggaactctctaccgatgaagccattatcccagcccgcggtggtaactacgtggatggaggcgtgtacgcgcagttgcacaggcattcctggacgaaggatcacaccaccgtgaaaaatgtgtggagctgggctttcggcggcgtgaacacctgcaaccgtattctcgcgctttttgaaaaagcacccgacagcgattccaagccgcaggcaatggcggaggccagggcgatgcgcgcgctgtattacttttacctgatggacctgtacggcaaagtacccatcatcaccacatttggtaatccaacgccgccagaacaatcatcacgcgaagaggtatttaatttcatagaaaaggaactgaaagaagtgttaccattgctgagaagggaacgtgggcaaattacctattcgaagcctactgtatggtttgcctttacactgctggaaaaaatgtacctgaattcaatggtatacaccgggaagcccaggtataacgacgtggtagtaatggctgatagtatcctgaccaacggcaaatatgagctggatgccaactacgccagcatttttatgcctgataacggtcctgctattatggaaaccatttttgcgattccttatgatggatatgtgatcaaaggcaaccagttttcccgtttcggattacatccaaacctggtggcaaagtactcattacctttccgtccaagtattgcaatgagcaccatcggttccttctacgaaaaattcaacttaacaggggatgtccgcaataatacctggctggaaggaccgcaggttaattccgacggctcgcctatcctgattaccaccaccaacaaaggattagatgataagtatgccggctcggaacctaagaaggaaatcaaatggcagcttacgttctctaaaacaatgaccttacgtgtagatactaccatggatatcgggaatgatgaactggcaaaagcggccggtgtgcgttccattaagtattaccctgataaaaatactgaaccttcagaacgtaactccaataatgatgtgcccgttttcaggctggcagatgtgatgcttatgaaggcggaagccatcctgaggggtgctgctcccacagcagtgaaaggcgaattacaggatgcagatgtattggtgaacaaaatccgcacccgggcgcatgccccatcggtaagcggtatcaacctcagcggtttgctggaagaacgcgcgcgggaattagcctgggaagcatggcgcaggaatgatatgatccgttttggcgtatttgaaggcacctggggttttaaatcagatgtaaatacccagcaccgcatttaccccatacctgtagatgaaatcacgctgaatccaaagctggtgcagaatcccggctactagcgcggattttgtcttggctcaggattacgctgattttactgattagctggatttttacttttttgattttataaaggattaagggagatagaagcggatatcgcttttatctcccttaattattatctaaaaatccaaaaaaatccaaaagtaaaaatccagctaatcagtaaaatcagcgtaatcctgagccaagacaaaatccgcatcgccgaaggcgatcttttcccttttgcgtaagtcgttttcctgatccgatcattactccccgatttcctgctgtatttttgtgagatataaataataccccggagtcattaactatacatagtccatacatccgttgtttgccaccaccatttttcaaaggtaaagagtgatgaattaagtcctgacagcggccgtaacccggtcgctggaggcacaaacccataggcccatgtgtaattaccagacattataccacggcgctgcaggatatgtgatccgctgcccgcattgcaaaggcattcagttagcctttggtacaacggttgttaaccttgatatcaccgaatttgagtgcttcaaaaagatggtcaaccggctatcggatgaacactatcacacatcagaaaatgaaaagatgatttgtttgcccctgccggcggatcatgtgatgatgttggtaacccctgctgaaataactgcgctggcaaatataacagcggaagtacaggcattgattgatgcctatgatatcctggaaacatcctccggatgccagtctgccggctaatgataaatgccgccccttcttttttgaaatgtatataatcccggatcagcgcgtgctgtcatattccgccttcagacggaatatgacagcacgcgctgttgtttaacaaccgggatggccacttgttcagccatgatcaaaattgattttatgtgaacaaatgtgaaacgacttgtgttacctattacaattgaatgatgaccatattcttcttctcataatccatatataaatgagttggttacagcatgcattccaggaatatcctgaactggccgtatttcttactttgtccgcaggattttttataggtagcatacgggtagggaaattttcgttaggatccgtaaccggtgttttgttaaccggagtaattgtagggcagatggacatacaggtatctgccaatgtgaagtcggtctttttcctcatgttcctgtttgcagtaggctatagtgtgggaccacaattttttcgtggtttgaaaaaagatgggctgccgcaggtattgtttgctgtacttatgtgtgttgtttgcctggtggcgccgtggttgctggcgcttgcctgcggctataacgtagggcaggccgccggtctgatctccggttcacaaaccatttccgctactatgggagtggcctctgataccattaaccagttaaatgtgtctgccgaacaaaaagctgcatggatcaacgccatgccggtatgttatgcagtaacctatatcttcggaacagcaggttcggcgtggttactatccagtattgctcccatgatgatgggcggaattgaaaaggtaagagctgcatgcaaagagctggaaaaaacaatgggcgccggtgatcccacacaggatcccggcatgcgctctgcttttatcccggttacattccgcgcctatttaattgatgcatcatccattgccgcaggcaaatcaatacagcaactggaaggggaattgctgcaacgcaatcaccgtctgtttgtagaacgcattcgccggaaagacaagaagctggtggaagccacgccggattatgtaattaatcccggtgatgaaattgtactcagcggccgcagggaatttatcctcggagaagaacagggtatcggtaaagaaatagtagatatggaattgttgaacttccccgtggaaaatgtacaggtatttgtgatgaataaaaacgtagttgggaaaacagtgaaagccttacgtgccatggattacatgcacggtatcccagtgcagagcatcaggcgcgcaggaatcgccatgccagtatatccggaggccgtactggaaaaaggggatcatgtggaactggtaggctacaaaaaagatatggataaagcggccaaagaaatcggttacgcggatattccgactgataaaactgatatgatttttgtgggccttggtattgtgttaggggggcttgttggcgccatgagcattcatgtaggaggggtgccgctcagcctgagtacaagtggcggcgcgctcatagcaggactggtttttggctggttacgttcacagcatcctgcctttggcagaatcccggagccggcattgtgggtgatgaacaatgtgggtttaaatactttcattgcagtggtgggcatcaccgcaggtcccagctttgtagcgggtttcaaagaagtagggtggggactttttttagtaggtattgcagctacagctatcccgttgttatccggggtgttgatggctaagtatatttttaaatttcatccggcattagtgcttggttgtactgcaggcgccagaaccactaccgctgcactttccgctatccaggaagaagtacaaagcaacctgccggctctgggctataccattacatacgcggtgggcaatacgctgctcattatctggggcgtggtgattgtgctgctgatgacctgatgttgtgaataactattcatcataaatgagatacaccgtgacagacacccctaccagttatttacgtttggtcgtttacgttatatccattcttttgtgggcggcgcagacacatgcacaaacagatactgctgaaaacggaaagggacttacccgtaacatgattgagggcgggaaaacgcagggctttctttttacggatgtaaagggcatccggctgcagtttagcggatacgtgcaggcggattttatccacgacttcagcgaaatcggcaacatacatgccatgcagccatctactatcacggtgcccacgttgagtgatggcaacacggcttttaccatccggcagtcccgttttgctttttccgcctttggtgttccggacgccaaagggcgcaccctcaaagccgtgctggaatttgatctctggggtaatttatccggtgcgccaagattgcgccatgcttatattcaacacggcaaatggatcttcggtcagtattggagcaactttatggatggtgataactggcctaacatcatggattactgggggccaaattcctatgtatggacacgccaggtacagctgcgctttacacaggccatatctgaatcaatgactttctccgtttccgcagaacaacccggtggcgatatttccattccttccacctggagcagcaaaactatctacccggatgtaacagccgcttttcagaaaaactttggaaaaaagaatgccagccatgtacggctctccggcctgctgcacccgatcgattacaagaacagtgacgcagatacgaaaacaagtataggcggcgcctttaatatctccggaaatattaatctcgctaaaaacgatgatgtgaaattccagttcgcttatggcagcggctatgcaaaatacagcgaagatatcagcgggcagggatacgacggatacgcaacggcagatgataaaagtatcagtaacatcagcatgctggctacctggctgtacttcgatcatttctggacaaaaagtctcggatctactctcgggtatggttacctgcaactgaacacgccggatctcgatatgcctgtaggcacactgaaagcaacgcactatggttcttttaataccacttactatttcacttctttctttaaaatagccggtgaagtactgtatgggaaaagggtgaatacggatgatcattccggcgatgatatccgcgctcagttcagcgcattcttcaaattctgatcatctgcataaaaatagaacgctaaagttgcgcttctcctgctgcccgccctgccggacggcggcgtaagtccctgctggctatgctgtggctgtttacctgttatttttccccgttaattcgtaaattcataaaacaagttatcaccttaacatgttttagagctatggacgtaaaggattattataagattttggggatagagaaaacggcaacagctgaacagattaagaaagcctaccgtaaactggcggtaaagtatcatccggacaagaatcccgatgataaagccgctgaagataaattcaaagagatcaatgaagcctatgaggtgctgagtgacgctgaaaagcgtaagaagtacgaccagtttggcgaaaactacaagtattacgagcagcacggaggccggccggaagactacgattggtcgcagtacggtggtggcggcggacagcgtcgcacctactcttatggcagcggggatatggatgatatgttcggcggcggtgaaggtaacttctccgatttctttgaacagctttttggcagccggttttcaggcgctggcggtggccgccggcagcagcagggccctggcaggggccgcgatgtgcaggcaaccatggaagtatccctggaggatgcttataccggtgctacccgccaggtagaagtgggtggcagcaggcttaatatcaagctgaagccgggactgtacgaaggccaggtgatccggttaaagggaaaagggaaccccggccgcaaaggcggggagaacggcgacctgctcattaccgtgcaactggcgccaaacccgcaatacgagctgaaagggaaagatatttatacagatctggcagtgcctttgtatactgccgtattgggaggaaagctgaccgtaaacacaccgggcgcttccctgaatatgaatattccggccggaacagacagcggcaaggtttttcgtttaaaaggcaaggggatgcccgcttacgacaacagcggaacagccggggatctatacatcaaagcaatggtacatataccggcaaacctctccgacaaggaaaaagaattgtttcagcaactttcacaattaaatgagaatggccatgcttaaactttttgattatctggaagaagtgatttccacagaacggatttcacaactcaataacccacgcctgctgtataccgccagcgaaattatgcaggaaatgggatatggccagtcgggcatggaacaggagccgctcgaccgggccatgcatgcgtgtgccgccctgaacatcccggtggactataatttcaagaaagtatactgcttccgtgatggggaacttactaccgactggcagttatcggaactggctacttacctgttcatgatcaactgtaatccgctgaatccttttgtggcgaaagcccagctgatatttatgatgaaagaccgggtatgagagatatcaaccggacaggcatcctcatagtagtgatcatgggcaccactatggcagggatagactccagtattgttaatatatcccttcccgttatgagcaggcagtttaactgtacgctcgacgagattgaatgggtgattaccgtatacatgctcagtttttccgtattgatgccactcaccaactggctgaaaaacaggattggctttttcaatctctatattggcgccatctccctttttacgctgggatctttaatgtgcgccttgtccaccagcctggacagcctgcttaccgcccgggtgatacaggcgctgggaggcggcgctatggcgcctacctctatggctattatttcctacgtgttcccggcgagggtgcgcggtacagtgctgggatggtggggactcggtaacctggtgggccctgccatggggcccacgctgggaggtatactcactgaaaagttcgggtggccttccatattttatatcaatcttcccatcggtatccttacggtgatcctcgccttccgttacctggatgtactgcggaagcagccgaaactgaaactgccatttgatcttaccggttttgtaatgctcaccatattcctggtttgcctgcaatatggtgtggcacgggcagaagtagtagggatcacttctcccgaaatactggctacactgggtgtggccctgattgcgtttgctgtttttatctggatagacaaacataaaaaagagccgatcattaacctggatctttttgccaattattcttttgtgagttgtatcctcgtaactatttcgaggtcggctgcgctgttcggcggcttattcctgatgccgttcctgctacaggaacagatgggtttttcagaaggtatgtcggggttgctgatactccccaattccgtatttatggcggcgatgatgccttttgcagggcgctggtccgataaacacggctcccgggagatatccatgctggggattgtgttactggcggtatctatgtacctgtttgccctgttggacaaaggcagtactatttccggcgtgatcatcaccatgacggtgagagggctgggcatggggcttttactcgccccactgaatgccgcaacattaagcgcagtacggccaagcgaagtaacaatggcctcatctatcagcaccctgatgcaacaggtgggcggcgccataggcatcgcagtgctggccattgtaacccaggctgcctacaataaacatgtactggccggacaggaaggccattatgcccatcacctggcactgaagcagggttttcatatttccctttttatcctgttgataaccctcatacccgcctggttccttccccgccggaatgtggtattaaaagatgcagatgtccacattgacacctgacttttttagtgcatgattattggtgaggataggttaacttttccggcatttatgataacaaatggtaagaagcacatattgatgatcgacgacgacgaagatgattttttccttgtaaactctttactacaggatatttcgcccgatcaatacgttttgcagtgggtttcttcctacaaagaagggttgttggcaattgaagcacgcgcacacgatctttacctggtagattatcgccttggcgctcatacaggtattgatgtgttgcatcatttccgcaacctgggatataaagcccccgttattttatttacggggaagggcgattaccatatagataaggaagccatgctggccggtgcgtctgattacctggtaaaaagcgagatcaacgcagccttgctggagagggccattcgttacaccctcgataaattcagccacctcctggccattgagaaaagtgaaaaacgctatttcagcatcttcgaaaaatccaatgatctcatcctgctggcagactgtgagcataaaattgtggcggctaacccggctgcacttaatgtattaaagtatgaggaagcggaactgtatagcagccatctccagggcctgtttgcggaagaaggagtgatcaacgctttcctcgaccagttgtgcagcgatgaaggtgtggtgcaaaaggaatatgtattccgcagcaaattgggtcaacagctcgatgtaatgatcaacgcttcgctgctggatgaaaaaaagcagctatacctgtgcattatccaggatatcaccgcccgtaaacggaaggaaagggaaaagcagcaacaggaaaaattcgcgattaccgggcgcattgcccgcctgatagcgcatgaagtccgtaacccgctgacaaatatcctgctggcggtttcccagcttaaaacggagccggtggccgaaacagaagatgcgaccttatacctggatattatggagcgcaactgccatcgtatcaaccatctggtcactgaattactgcagtccacccggatgtcggagctgaatatgctgccactgggactgaatatgctggtggaaaaagcgctgcatcttgcggacgacaggttgcagttaagcaacgttaacgtggtaaaggaaatgtgccagcctgattgtatgatcctggcagatgaagacaagatcctcatcgcttttctgaacattattatcaatggcattgaagccatgaaagccggggaaggaaaacttaccatcaatacatggaaagacgcggagaaagtatttattcgtataaccgataacggtagtggtatttccccgcagaacctggcgaaactttttgagcccttttttaccaacaaaacaaagggaacgggattgggattaacggctacccagaatattatacttcagcataagggtacgattgcagtagatagtatattgggagaagggactactttcctgattagttttcctattgacggagaaagccagagtgaatagactaccggccggtaaatgccttacagcacttaccggccgatgatattatttatcctcttcttctgctttgatgcctgtttgtgtaaacacgatcttccgttgtttgtacaggttgccaatggtcattttgaatgttttcttgctcatcccaaaaaactcctgtatctcttccggtgtcgatttatcatgatacggcagatagccattgttttcctgcagtaaccgcataattttctctgactcgtcttctactttattaaatccgggtttacccaggatcacatctattttatcgtccttgatctggcggatgaagcccggtaatttgtcaccgatttcaatggtccggaatatttcgttgtgatgcaggataccggtatgcaggttgttgatgatcaccacgtaaccgatgtcggtacggcggtaaatcaccaggtttacctggtctttttcctgtacggtgaggttttcattgctgaggtaacggtcaatcttctctgtggcagcaaggcggccggtcagctcatcgatatatatttttaccaggtattcctgtccaggcgccatgcgggtaagctgttgggaagaggccacaaacaagtctttcatcagcccccagtccaggaaagcgccctgtttggtaacgctcaccgctttcagcatcacaatatcccctgcaatcccgtaggggcgctgggtagtggcaatcaggcggttttcggaatcatggtaaagaaatacttccagttcatcgcctacacgggtaccgtcgggtacaaaccttgtgggtaacaggatctcctgttctacgccttcgaggtacacaccaaaatcagcttcttttttcacccttaacaggttgtattcacccacctttatcataaaaaacgattaattgtcaggctgcaagttacttatagattgccggattgcgagaatcatattctgcttacttttgtaagcatcagataccgggcagtattggtaattccccggtatccggtcttaaaccaaccaaactatcttatgacgattttattattcaccctgatcctcctcggcggggcctttttggctgggctgctgggatcgctgaccggcttaggcgggggcgttgtgatcatcccgttactaacactggtatttcataccgatatccggtatgccattggtaccgctttggtagcctccattgccacttcttccggctcagcggctgcttatgtaaaggagggcattaccaatatccggctgggcatgttcctggaaatagccacaaccacgggcgccgttgtgggcgcactgatagccgtatatatgcccaccaatatcgtagccattattttcggactggtcctcattttctcgtccgtaatgtcttttcgcaagaaaatggagtttccggcagggcatagcgacagcaaagcagcggagcagctgcggctcaacggaagctatccctccgacggtgagatggtcaattacaaagtgcatcatgtaccagggggctattttatgatgaccttcgccggcatcatgtccggattgctgggcatcggctccggcgcgctgaaagtgatggcaatggacaatattatgcgtattccttttaaggtgtctaccaccaccagtaactttatgatcggtgttaccgctgctgccagtgcagtggtatatctgcaacggggatatatttctccgggcctgtgtatgccggtagtactgggagtgctggcaggcgcctttgcgggctcccgtttgctcacacgcgccaatgtaaaagggttgcgtatagtctttagcgtagtaatcggattgctcgctttacagatgatctataatgggataaccggaaaattataaacgatgaaacaggcactcgcaaagtatttccgggataaggatatccaacagctcatcggcaaacaactgcgtataggcgtaattgtttccagcatcatcgtatttatcggtggtgtcatttacctcgtccgtcatggccatgaacacccctcctatggcgactttaccggtgtaagagaaggtttaaccaccctgcccggcatctggcagggtgtaatggaaaataaaggcatgaacatcatccagctgggcatcgtattattaattgccacgcctatcatccgtatagccttttccgttatagcctttttaatagagaaggactacctgtacgtaggcatcacactcctggtactgggtatcatcctattcagcatgctgggcgggttagcggggtgagcggattttgtctttctcaggattacgctgattatactgattttttggattttgttttttgggattttataaaggattgggggagatatcagcgaatatttttaaagattagggaagataaaagcaaaatatccgctgctgtcttccctgatctttaaaaatcaaaaacaaaatcaaaaaaaacaaaatcccaaaaatcagtataatcagcgtaatcctgagaaagacaaccttcgctacagggttaccgcaattaccgcgtcaatagggtccgatggtgttgcaggaacggagatgacgaggtcctctgcgttgccggtggtggagagctgctggccgtttgccagcaggcgggcgctgtttacttttccttttataccaggaacatgcagtttgccatcggttggccagttgaaaacgtgcaggtatagcgtggtggtggctccttttattttttgggtgcagcggccccattccaggggtggcagcgggctgccttgtgtgccgtatatggaggcgccatttactttcatccattggccaattcctttcagcgcggtaagactgccctcggggaattgtcccagcgcatcagggcctacgttgaggaggtagttgccgtttttggaggcgatgtctgccaggtttcgtataagcgtttccgtgcttttccattttgggtcgtagtctttatatccccaggtgccgttcatggtcatgcaggtttcccaatccctgccatccagctccgactggttggggatcttttgctccggtgttttataatcgcccgggaagttgggtcttcttaagcgatcgtttgtaatgatattgggttgcagcttcagcacctcctgtagttgttgtgcgtattcatcagtcatattggtaggggtgtcccaccacagcacggctacttcgccgtagttggtgaggagttcctttacctggggcacggctactttagtgatgtagtccgacatggtagcggaggtttgcaatgggtcccagtggccggtgtgcgcctgggtataagcatctattttggcggaatcagggttgggccagccttcggtggccactttgcgggccgcggcgccaccggggttgttccagtcctgcgcctgggaataatagaagccgagtttgataccgtatttcttgcaggcggcagccagcggcttcagtacatctttaccataaggagtggcatccacaatattccatttgctggcggcagatttgaacatagcaaagccgtcgtggtgcttggcggtgatgacgatatacttcatgcctgcatcccgggctgtttttacccaggcgtcggcgtcgtatttaacgggattgaattgtttggcgtattgctggtattccagtaccggtattttgccgcggttcatgatccattcgccgccgcggcctacctggtggcctttatagttgccggccagtacggcgtagtcgccccaatggataaacatgccaaagcgggcttcgcgccaccattgcatgcgctggtcacgggtaagtgtgtgctgtgcatgaagagaagctgcgggtaacagcaccatcaggaatagcgtgagttttttcataaacgtcatgtggaaagtattgtcggttatgcaaacgattgcaaaaagggtttaaaaataagcgcttatcgcgctgatctttattcaattcacataaatgtctataaaaaaactggtccggaatgggctgattttaccggaaactggtatttttttagttggatattttattccgggagaaggaataaaatatccaactattggaggaatattattgcgccatttccatttcgtcgagttccagcacctgggtagtccaggtacgcagctcatcgcagagggcagggttattcaggagcgactgtccgtaggacgggatcattttcttcagtttgatctgccatgcttcggtttcaacgtcttcgttaaagcaacgtttcagcaggttcagcatgatggatactgcagtagatgcaccgggagaagcgcccagcagcgctgcaatggagccatcagcagcacttaccacttcggtaccaaattccaggataccgccatgttcaggatcttttttaatcacctgtacacgttgtccggcaatttcaagttcccagtcttccattttagcttcggggaagtattcccttaacgcctccagccggtcttccggcttctgtcttacctgtgcaatcaggtatttggtcagcggaatattatccaaaccagcagacaccatgggtacaatgttgttggctttgatggataaagggaggtccatgaaagaaccatttttcaggaacttggtggagaacccggcataagggccaaacagcaaggctctttgtccatctatcatgcgggtatcgagatgcggaaccgacataggaggcgcgcctacagaggctttgccatatacttttgcacggtgctgttcaattatttcaggattattgcaacgcagccattgtccgcttaccgggaaaccgccgaaaccttttccttccggaatgtccgacttctccagcaacggcagggaaccgccgccggcgccaatgaatacgaatttagtgttgatggattgtctttcacgtgtaccacggttttttaccttgatggtccagctgccgtcgtcttcctttttaaagtcacgcacatcatggttaaagtgcatgcttacaccatccatttttgcgagatgattaaacagggcacgggttaatgcgccaaagttcacgtctgtacccatttccatgtgggtagccgctactttctgggaggcatcgcggcctttcattaccaggggcatccagtttttcagcttttccggatcttcagaatactccatcgttttaaacagatggcactgttgcagggcattgtagcgctttctgaggtaatccacattctcttctccccaaacaaaactcatgtggggaacagcctgtataaaattgtgcggattggaaatgatgttattttctaccaggtaggaccagaactggcgggatacttcaaattgctctgcaatgttcaccgcttttttaatgtctactgatccatcctgtttctgtggcgtgtagttcaactcgcaaaatgcagagtgtcctgtgcccgcattgttccatgcatcggaactttctgcagctgccacatccagtcgttcaaaaattgcaatggttaactcaggttccagctctttcaggagcattccaagtgttgcgctcatgatcccggcgccgattaaaaccacatccggacctgttccagctgtactcttgcttctaaacataaccccatttttattcgaggtgcaaagttacaatcaaaacacttatgcagggagaataaattgattgtttactacactttaacaatactattacaattctttctgaacggattgaaagttttgaatttctcgttgcgtatatataaatttatattttggttaagcatttggcaatgaaataattgactgcccggaaagtttatttttattttatgatgaacagacgcctgtttttaaaaggagtatccgcagcagtagtgatttctgcctgcggtaaaatagtaaaggccgtaacgccccggcacttcgacagtaaaaccgttttccgctttgcggtcgggtccgactggcattacggcgagcctaaaaccaattacgaccagtatttcctggatctgcaaaccgcttttaaccaataccagcaccagtatccctgcgagttttttacgctcaacggagatattatccacaacgatcccgccctgttgctgcctgcagccgccaaattgaagcaattgcatcccaagttgctggttacccatggtaaccacgacatggtgccggctgctgcctgggaacaggcctggggaatgccgctcaaccacgatatggtaatgggtaaccatgttattctcctcggtaataccgccgatgagaaaggaaaatacatctgccccgatgttgattggttcacgcaaaagctcgaacaatataaaaccgctcaaaatatattcatcttcttacatattaccccggtaaaatggacagataacgggctggattgccaggattttcaacagctcatccggaagtatccgaatatcagggccatcttcaacgggcatgaccatgatcaggacagcgtaaaaatgctcgataactgccccatcccattcctgttcgatggtcacgtaggcggcagctggggagttggctatcacggtttccgggtagtggagttaaaggaagacggcagcctgctctcttttattatgaacccgctgaaaagacagaacgaaagggtttttccgaaagtttagctattttgccggtccaatcgggatgctaaaagaaaatctatgctggaggaacttgaaaaagactacggatttacctatcctacgctctataaacaattatataaggatggtatgctgaactggggtgagtttggggaagactggctggataaagtataccctgctattaaaactgcaccgcctttactgctatacgccaacgatctcgaaataatggccctgcctacggtggatgaagaaatggacgaagggctgctctttgcagatcctgtacaccagttcgttccctttgccatgagcggcgccggcgattggttcgccttttacttcaacctgcaaaacggcgacgatgtgcccattgtacaggtgtttcatgattccaatgaagcctgcatcctggctaaaaacctgcaggactttatttttttacaaatgctggaagcagtaacagacctggatcccaggaatccttcgctgattgcacatggtaacatgaaagaaaactgccgcaacttcctgcgcacacatgcaccttacctcacaccacgccaggcaggtattatagaggcagtatatgattttggaagattgaccaatgtggccctgcacgaaattgtagagaaagaaatgagctttgaatggctggacagcagcttcccttaccagacaagaggataacaaaccggctaaaaatgttggggataaaatcacatttttagccggccccgcttattttaatctttataaaaatctatcagcgagccgaaatactgctcattccagccggcaataatatcttcataagcttcgtccggaatattcacatgcttcaactccacatctgttccttttggagatggatgcagtttgatggtgacaatggatggattttcctcttcttcctcttcatcgtccataaaataccattgctgcacaatctttttgtcctgctcaaattccaggtttttacccacaatacttccttcccataaagcgaattcagaacccggctctgtcgacatttcagctacttcgcctgtccacagctgaatggtggcgggattggtgagtgccgcatatacttcttcaggcggggccgcgagtataaaatgttttttgtaatctttcatggtttcaaagctactgaattgatgaattattatttacttttctataaaaattgagcatatgcaactaaccaaactgatcccgaatatcttttattcggatatgaatgtgggtttgcagctatttgtggatacgctgggcttttctgtggcataccgtgatgacagcggggaacagccgttttgcatcatcaagcgggacaacctggtgattcacctgattgaaagtcatgaatgggcgatcaaggacaggccggaaatacgactcgaaaccgatgacatagaagcagcatatgcactggtgaaaggaagtcaccctgagttactacaccccaatttaccggagatcaaactccaaccctggggagcactggaatttgccctgagagatacagaagacgtgtgcgtgattctccagcaaccttcctgattgttcatttccgggcatttaccgtccatttccggacaaaagaagacgaatacttcccttgtaaccctttgtggataaggccatgcaactatggcggtcttcttgtgtctttaagggcgtccatcaaatccgccttgccatgatcaggaattatttgaaaatagctttcaggaacctgttgaagaacaggggcacctcctttatcaacatcttcggcttatctgccggcatggcggtaaccatgctcataggactatggatctggaatgaattgtcgtacgataagtaccacgctaattacgatcgtattgcccaggtatggcaacggatgtcgaagggcgacgaggcgggcgcttttaattcaacccccattcccctggcagccgctttgcggacctcctatcccgacgattttaagcaggtggtaattatggcagatggcacacataccattgctgcaggagaaaaaaaatttacccggaccggcattttttcagaacccggcggccctgaaatgctttccctgaaaatgctgaaaggcacctatagtggcctgaaagaacaagcatccgtactcctgtctgcccggttagcaacagctttgtttggcgacaaagatccaatggaccagctggtgaagatggataacaaccgtaacctcgtgctgaaagtaacgggtgtatatgaagacctgcccgaaaatacttctttcagtagcactgactatattgcgccatggtcgctgtttataaataactggacctggataggcgacgcgagagacaagtgggacttcaacatgacgaaactgtttgtgcagttggcagataacgcggatatggacaaagtatcagcaaaaataagccaggtagcaacaccgcatttaaccctcgagcctggcctgaaagaggaattattcctgcacccgatgcgtaagtggcatctgtattcttcttttgaaaatggcgtgaataccggcgggcaaatacgttatgtgaagttatttggcctgataggcttgtttgtgttaatgctggcctgtatcaactttatgaacctgagcaccgcgcggtctgaaaagcgggcaaaagaagtaggcatccgtaaggccattggttctatgcgccggcagctgatctggcagttcttaagtgaatcggtgctggtggcattcttctcttttgtgttatccatattgattgtgttaatagtgctgccctggtttaaccaggttgccaacaaacatattggggtattatggggcagtccggtgttctggctcattggcctgggatttagtttgctcaccggcttactggcaggcagctaccccgcgctgtatctatcctcgtttcagccactaaaagtattgaaaggcactttccgcgccggccgctttgctgctgtgccccgtaaagcgctgatcgtagtacagttcaccgtatccattattttaattatcggcaccattgttatttaccggcagattcagtttgcgaaaaaccgtcctgtaggatatacccgtaacggcctgctttccatacaaatgaccaccccggagatctataggaactataagatcatcaagaatgaattggaaggttcgggtatggtcaccgctgtatcggagtcgcaggggccactcaccgacatatgggccggcgccggcggttacaagtggagaggacagcgatctgaccaggaagacggttttgctgtaattggcggcagaatgggttatggcaaaacagttgactggcagtttattgcaggccgggacttctccgagcaatttgcttccgattctatgggaataattttgaatgaagcagctgccaagtacatgggatttgataatgctgtaggtgaaattatacgtaaggatagcctcgagtatcatgtactcggcgtggtgcataatatgatcatggcttctccttatgaagaagtaagaccggctatttattaccttttgagtgaacccggcaattttgtaaacatccggatcaacccggacgtgaccactggtaaagcgatggcagtgatacagcaagtaatgcagaaatataacccggctgcaccatttgaatataaatttgccgacgaagaatacgcaaagaaattcagtgaagaagaacgcatcgggcaactatccaccttcttcgctatacttgctatcatgatcagttgtttgggtttgtttggccttgcttcttacctcgcagagcaacgtactaaagagataggtatccgtaaaataatgggcgcctctgtattccagttgtggaaaatgttgtcgaaagattttgtgatactggtcagtatttcctgttgccttgcgattccggtagcctggtattgcctggacagatggttgctgcagtacgaataccacaccaccatagtatggcagatatttgtgttcaccatgttgggagccttactgatagcgctgctcaccgtaagctaccaggccgcaaaagcagcactgtcgaacccggtgaagagcctgcgggcagaataatttttcttttccctgtgcggtaaaaaaggtatttttattgaatatcctcaacccgcttttgaataatgaaaaacgtccggctgtttgcggcatacctgttattcttattgtgcgtagctgcctgtagccatgcacaggcgcctgccgcatggatacgcatcaaccagctcggctatcttcccggtggcgttaaagtagccgtttggggcggcaaaggaagcatgcagccacgcacctttcaactggtgtcggcggttaccggtaaagttgtttttacagccggtacaggtacacctttcggcgcctacggcccgtttgatcaaacctatcggctggacttctccgcgtattcatctcccgggaaatattacctgaaaacagatagtatcatttctcctgaatttcgtataggcgataacgtgtacgcgcgtacgccagactttttgctgcgttatatgcggcagcagcgaagcgggttcaatcccacgctcaaagattcctgtcacacgcacgacggctacaccatgtacggtcctatgccagacagtacgcatatcgacgtaaccggtggttggcatgatgccaccgattacctccagtatgtaactacttctgccaatgcagcctttcacctgctggcagcttaccgcgattttccgggtgtttttggagatagctactcagccaatggcctgccgggcagcaatcatatcagcgatgtgctggacgaagcaaaatggggcctcgactggctgttgaaaatgcatccgtcggataacgtgatgtttaatcagttagccgacgaccgcgatcatcatggtcttcgcctgcccggtgaagataacttttatggcaaaggctttgaacgacccgtatatttttgcacaggagaaccgcaaggtttaggtaaatacaaaaacaaaagcaccggcgtagcttctacggcaggaaagttttccagcactttcgcgctgggatatgatctgctgaaaacaactgcgcctgcctatgcgcagctgctgaaaacccgggctttgtctgcctggaaaatgggaagaaaacaacccggcgtatgtcaaacggcgtcggtactatcgccctacatttatgcagaagataactggaccgatgacatggagctggccgctgcacaactgtaccagatcacaaaagaaacggaataccaacaggcggccaccggctatgccgcgcaggaagaagtaacgccatggctgggcgccgataccgctcatcattaccagtggtatccgttcatcaacctggggcattatgcgttggcccagcaaagcaaccgtgcagaaaaggagcgtctcaccagttattatgaaaccggtatccagcgggtgtggaacaaagcaaagcataatgctttttatcgcggtataccatttatctggtgcagtaataacctgactaccgcctttgccatccagtgttactggtaccggcaactcagtcataaaaatacttttgctgccctggagcaggcaaacatcgactggctttttggctgtaacccctggggcaccagcatggtatacgggttgcctgcaaacggcgatacacctgctgatccgcacgccgccttctccgctgttggccactacccggtagatggcggactggtagacggacctgtgtataccaacatctacaaaaatctcatcggcatccggttgtcgaaccccgatgaatatgctatgtttcaaagtgacctcgccgtgtatcacgatgatgttggcgattacagcaccaatgagcccaccatggatggcacggcttccctggtgtacctgctggcagcaaaagcacaggaagaggccgggaagcggcaatacgatcatggtggattaatccgcggagatagcagcaaaaaacaattgacacttgttttcacaggagatgaatatgcggacggcgcgcaggtaatccgcaacacattgcagcaacagcatgtaaaagcggcattctttttcaccggcagattttatcagcaacccgctaaccaggcgctcatccggcagctgaaagcagacgggcattacttaggagcgcacggcgatcagcacctgttgtattgcgactggcaaaacagggatagtttgctggttacaaaaacacagttcctcgacgacctacaggccaattataaaaaaatggcagcagcaggaattttaaaagaagctgccccctggtttttgcctgcgtatgaatggtacaatgacagcatcgctgtatggactgccacagcgggtttgcagctgattaactttacaccaggcacccgttccaatgcagactatacctatccggcgctgggaaagcaataccgtacctcagcagaaatttatcaatccattctgcaatatgaagcaaaccgtcccggcggtttgaatggcttcctgttgctgctgcatataggcacggatccccgcagaacagataaattttacaaacagctgggggcattgatcacggcgctgaagcagcggggatatcatttcaatccgctggcacaggtgctgcaataacattaatggtccttttggtgacctgccaatttttagcgaacttaaagtattgataaacacataaatgcgagaattgaatcaaaacaaagacaaccaaaattagaaacggtagttagtatgctacccatgactgtaatcgaccaaacttaaacccgctaaattttttctatgagcttgtttctattgaagatggctaaaggccggtcctttttgctattcctgttcatgaacgtgctggccgttgctacctatgcccaggtaaaaatttcaggccaggtaacggataaccagcaatctcctattcccggcatcacggtagtagtgaagaattcaaaactgggcgccaaaacagatgtggacggacgttataccatcagcggcaacctgccgcccggcaattacacactgggttattcaggtattggcttcgcacccggtgagcgggtgctggtaataagcgccggcaacaccacctatacgcaaaacattcaactgtcggcagaagtgtccaaactggatgagatcgtggtaaccggtacctccgaaggaaccacgcgccggcagctgggtaactatatcagcacggtgaaagctgatgaactgagtaaaagcggctcgggtaacgtgctggcagccctgcagggtaaaactgccggtgcacagatttcccagaactccggggatccggcaggcggcatctctgtaaaactccgtggtatcagtaccatatcaggttctacagaacctttgtatatcatcgacggggtaatcattgataactctactacgcgtgtaaccaatgctgatccgagctacggcgttggaggaacaaccgatccggcaggtggcgcaggcaataacttcgtaggtaacgtagggcaaagccgtatctctgatattaacccggcagatattgaacgcatagaagtactgaatggcgctgctgcggcagccatctatggttcccgcgccaacgccggtgttgtacagatcttcactaaaagaggcagcgccggagcaccggtggttaatttttccaccagtttttccgtgaatcaactgcgtaaaaaactggacgtgaatcaggccccggtaaagtttggcggatctccggacgattccacacaaaacatcctgactcctgctatcgtgagtaaaacaccggtaaacaggtacgactaccaggattatattttccgcaccggcgtaggaacggataataatatatccgtggccggtggcaaagacaaaacaaaatactacgcatccggcagttacttttataaccagggaattatcaataaaacagatttcagccggttcagtttccgcttaaacctcgatcaggagctggccagctggataagcttcaatgccagtttgaactatgtttacagcaaagcaaatgaaaaacctgatggcaataccttctattctcctatgaatggcgtaaccatcatcggtaactactatgatatacaaaagcgtaacgccttaggtcagctgatgaaagtaggagaacgcggccgcgtaaaccccgtgtctatcatggaggattttaaacagcagcaacatgtaggcagggtgattgccggcgccggcgtcaagctgcggccaatcaagaaccttacggtagattaccggctcggtatcgacaactataaccaggaaggcaccaccttcatgcccgcattcgcttactttgtaagtcctggtttttacggcggcggtcctaccctggaccctgcgcagaatggttatgccagcgccggtaataataattcctttctgatcaaccacgacctcaatgctacctataactgggatatcaatgataaactcagttcggtaacacaggtgggctactctgtgcaataccagcgcatgcactacaccctggaacagggaagagggctgcctccttttgtgcaaacagcagataaggccactactattattcccggtgcagatcaacggacggagttatctgtttccggagaatatatccagcagaattttaaataccgcaaccagctgtttcttaccggcgccctgcgtgtggatggatcatccgtatttggggtagatgaaaggaaccagttatatgctaaactcagtggtagctatgtgatatccggcacagatttctgggaaaaatcatccgtggccggatggtggaacctgttgaaattaagagcggcctacggcgaatccggtaacttaaccggtatccccgcatatggccgttacaatacctatgctgccacagcctttataggcgccgctgctttccagtcgccctccacctatacaaacccggatgtgaaaccggagaagcaaaaggaactggaagtaggtacggacctggcgttctggaataatcgtataggcttatccgttaactattataagaaacgtgttgaaaacctgttaatcagccgcgcagtggcccccaccaaaggctactctttttaccaggataatatcggtacactggaaaacaccggtgtggaagtagtgttgaatgtaatgccggtgaagacgactaatttcaactggaacctgactgctatctataaccgtaaccgcaataaagcggtggatatcggacaatcgctgatcctctataacactgtaggcggcgctcctgtgggcattgccaatggagagccgatcggctttttctatggtaccttcttcgccagggacgaaagtggtaatctcctgaaaacacctgccggcataccggttacggaagcaggcaaacaaaattcaccactaacgtatacggttgcacgtgatccggctaccgggttgccgccaacaacaggcgttacggcattgaataaaaaaataggtgatcctaaccccgattggaccggcacacttaccaatgatttccagtataaaaaactgggtcttcatatacagatagacgctgtgcagggtggcgatgtattcaatgccgactggcgaaccaggcaaggtgttgataacggaaaggtagctgaacaggaggatctcgggttgcttccacgcggttttgtagcgggcaattacaatatacaggaatggagaattgatgacggctcctttgtgaagctgagggaagttgccttcagctatagctttggcaagctgaaaggactcagtgatttaacgataagtgttggcggcaggaatttgatttcctgggacaactacaaaggatacgatccggaattaaatgcggcaggacaaagtaccgtattgcgcggaattgattttggcgccgtgccggtgccccggagttataacctggctatccgcgcaaaattttaatcacaaaaaaagagctattatgaaacgatatatgcaatatagtatcctcgccatcgctttgttctgcattttcaccgcctgtaagaaagattaccaggatccatcgggaccttcatcagaacaggcttacagctcgcccgctacgttggcgaatgcagcagtgggcctgcaggcatggtatgcaaaagatcgcacagggttgttatacaccacggttacttccggcagtttgctattgggagaaacctttgtaaccaacccgggtaacgcagatgaagggcagatcgccgcaggagggaataaaatcctgaccaccaacgtggtagttactggtatgtggaatgtatctaataagatcaggtatgaagccgatagcattttacgccgtaccggcgttgttgttgccgataaaagctttgccagtggccttattggttataccactatttttaaggccctcgccctgggcgtgcaggcgaatttctgggagcaggtaccggaaaataccggtacccctgtgtcatccggtggggtgaaatttgttccggccaagcagggttatgtaatggcagtagccgccctggacaacgcgatcagcactataacggctacgcctataggaactagctttttggccaatatcccccagaatgtggatatcattaataccctgtatgcactgaaagcaaggtacgccctctacgcaggtgactacccggcggcaataagtgcagctgataaagtaaacctgggtgtacagtctacgctttcttttaatccacagatcaacaaccccatcttttcgctggtaacggctaccaacaacatctataacgttgttgactctacgatgggattgccggtgcctatacagccggatctggctgaccagcgggtgccgttttatattgcccggccagccaagccgaagtttaatatcaacggctttttcagaagtagtttaacagcagtgcccatctatctgccgggagaaatgctgcttattaaagcagaagcttatgcccgtcagcatgacattgtgaacggcttgctttacctgaacaaagttgttaccaagaaggcatctgaagatgcgttcggtgttggtgcggcattgccgccggtagtggcggtcactgaagcggaattgctgacgttgatctataagcaccggagaatagaattgtttatgggggcccaggaactggaggacagccgccggtttggaagaccagtgttggaacggaagcggagttattttccatatccgtttgtagaacggaatgacaatccgaatacgccggacgatcctgcattttgatgaaatgttttacaggttgccgcgggtggcggcaacctgtaaaacgttttgaaatgggggacaaagttgttatcttgatgtttaagtatggaaatatatacaacccttcagataggcgcctatcatgttaaccactgtgaagactatctcttcttcgatcatatcgatagcaataagatcatttgtgccgttatggacggctgtacaatgggaaaggatagctatctgatttcttcactggtaggtaagctgttgagaaaaatctgtaaatcgctaagctataaatcgttttattccaaagaataccccgaaatgtcattggatgactatctgaaaatcatcttaaaagaattattctcagaattaaaagttatcaaaaatcaaatacaactggagagagaagagttgttaaccacattgattattttgttggcagataccaaagcagataaaggtttggttttagtagtaggagatggtatagtgaacattaacggcgccgttattacctttgatcaggataacaagcctgattacctgggctatcatctgtcggaagattttgatcattggtatgaatgtcagctgcagaaaatatttttacatgaactcatcgatatcagcattgctaccgatggtttagaaacatttaccagggtggcagcgccggaaaattccgaggtaataaatccggtagattttctgttaaatgatcaaaccgggagaggcaatgaagaaatgctgaatatgaaattaaaagcgattgagcacaagtttggattgaatcatacagatgatctggcagtgataaggatgataaaataatcttataccgcattacgtccatatttttccccgtggatataaagagaaagatgtcccattatattttactgaactaaacccaccaaccgcctgctgattgccaatcccatacagagatggcgttttccggcaaatgaagcaaacacaggagcaaagcaacatcgttgtggtgtagtttttgatttggcctttcgtagcgaaatcctaaaaattactatcatgaacaagaacaggctttcagccagcttacaagcaggacttaataatcaaatgacccaggaagcgtttgcagcacagatatatttgtcttatggatcctgggctgcaagtgaaggatataatgggattgccaatttcctcttccgccatgccaacgaggagcgtaaccatatgatgaaattcctggaatatatcctggaaagaggtggtaaagtggagatagccgctattccgcaaccgcctgcaaatcctgtcagcgtacaaaactgttttgagcaggtatttcagcaggaggttaataacacaacgggaatctataaattggtgaagatgagttttgacgaaggcgactgggcttcatggaatttcctgcagtggtttgtgaaggaacaaacggaagaagagaccctggcgctgaacctgttggataagatcaaagtggcaggtggagaaaaggcaaccggtgaagcattgtatgcactggatagggatctggaaaaagaaccggatgaggcggaactggcagaaacaaaaacagtagagaatccatagcagagctattcataatgataaaaaggaggggttgcattggcaatccctcctttttaattattgcacgctaactaaagtagcccctgttggcttgcagcgctgataagcccggctacattttttacctggaatttctgaagcagatttttacgatgattttcaacggtgaatttgcttaggaaaagcatttctgcaatgcgcctggtggtgataccggaagcaataagtttcaggatttcaagttccctggtagtaatcgccggaacgtcttttgtggcctgccctccgggccgggcaataatttctttgatggcattgctgaatacgatctgatgttgcagggcttcatggatgcagcgcaccaattcctctacagatgcatttttgagcaggtaaccacttgcgccgttttcaagcattttcataatggcgctgcgttgatcatgattactcagcgccaggacaatggtatcgggagctgttcttttaatttccttacagatatccattccgtttccatccgggagtataatatcaaggagcaccacatgaacggggttggtattgaaaaactgtaggaaatccctggcatgggtaaacgtacctgcaatttcgaatgccgcttccccggcaagaacattcacgagcccctgaagtaccaccggatgatcatcaagaatggccagcttatattttggttgcaacatacacttcaatatttatggaagtacctggttgatttcctctggaaacgatgtctattgtaccattcagatacgctacacgggttttaatactaatgaagcccattcctttattttcatgcagcatatcttcattgaaaccggtgccgtcatcttcaacagtaataaaaaacttattatcccgttgattgcattgtaacaggatactttttgctgcggcgtgttttactgcattggtgagtaattcctgtgcaatgcgataaatgatcagctgttctccctgcgggatatttgtctgaatcccgaaactcaggaagcggatggttgttttttcagaggaaaatgaatcgcaaagatctttcaatgcggcttcaagacccagtcgtaacagcatttcgggcatcatattatgagcaatgcgtcttaactctgtcactgatgtatccatctgtgcgatgatgccttccagttcagggcggttactggtattgacggcgccggcaattttggaaagattgatttttgtggaagccaatagtcctcccaggctgtcgtgaagatcccgtgccacccgtttgcgttcttcttcctgacccagcagcatggcatgcgaaacctttatttgttcctgctggatggcagttctctttttatttttataaaagaagtaagccagtagtaagatcataaataaaagaatacttaccaatcctaacgaccagcttagcaggatagttcgttttaatgcgaagtttgccttgtcgttggacgcgttcagttccgtaattttccgttgatgttctgcattcctgaattttatttccagggcatttatttttgtctccaggttgctttgcgcaacgctgtcgctcaggtaactataacgtttcaaccactggaaggcctccggaatatttttcagatcttcattggttactacgaggccatagaacaataaaagccggttggctgaattgttcataaatggttgtttactgtacagatcgagggctacgctgcgggcctgctgcagatctttcttattgtataatgcatagaatttctgtaacaataaccgttgttcaggataaggctggtgcagttgcctggccaatgcaatacctttctctgcaactgcaagggactgctcaaatttttccgcgatggtaagccgcatactttctccggcataataatccagccactcatttgcttcggggtagggagccagtaacacccgcatgctatcaaggtacaaagcggctttcgcggaatcacccgataacgaataattctcggataaggtatgataggcagtagccaggtattttatatttccttgctgattccgtaacgtttcaatcgagagttgcagataggctttagctttggcgtattctttcaggtttttaaatccataagccagatccaggtaattctttcccaggtacagttggtcgccggctttttgggccagcgggatggcccggtttacaagcaggtttacataagtttccggatcatctttttcgaagtggaatacccgcgcgtaatcatgccagcacatggaacggaaaagcaatgcatctttgcccggaaatttcttcaggatgttttccgcctgcatgaacatcttggcagcagaatccggcgccgcggcggtaagtctcctggcttcgtaaaacagtgtcacgccctgcagaaatggataacccttgctaaatcttttacctgactgcatatattttttcgagagcgtagtgtccgtctcttcccattcatccgacaaacgaaagcttacacgggctttgatgctatcgtttaccgcttgttcaaggatatgggcaagactatccttgtcaaattttccgggagcctgctgcgcataactccggactgccgacaacagaagaataagtacgagtgtaaatgatttcataacaatttgcaagttgttacatattatcgtcataataaagatacgggaagagaatgactgaaaacagctatacgcaaaatgaccatttcacggtataggacgcccttgttttcataagtaattttgttctgcgtactgacataaaaaccgggttaaattcaaagaatatcatttcaaaccatagcatatgtacagaaaattatccattgcaagtatcctgttcgtagcaatgctcaccacgtcctgttccaaagataaggatgataacaattccccaacgacacacaaagtagtatttaaagccgaaacttcaggaggtggcacagtcgacagggccgcctatggggtcgatgcggacgcccacagtgctactaaccttagtggtacctcctggagcagtcctgagcttacggcaccggcaggcgcgtacaatgccaatatcgttatgaatggaataggcaccagcaatgcctccacattgaaggtagggatttatgtagatggccaattgaaaaaggaagcatcatccaatccaggtacggtattaacggttaccctcaattacaaattttaatactttttcatgcggctcctgaaaaatacatccatcatcattgtgctgacgctcattttctctgcagccggttcttatgcgcagtcgaaactggacaaacggacgaaagaggcgctgggacagcgttatcaggatgataagtattacgctgattttcaaagaggtatttataaccgggaaaactggaagaattcatgggtaggggccaggctgtcagatatttataaaaaatggggtgctcccgcaaaagccttccctgatgcagatgggggccaggtagtggtatatgaaaagatgtctaactatgggggaggcagctatacccccggatatacgataacgggttacaatgttttcggacaggctgtaaactcagaaacagtgcagtctaaagatacgcgctgggccagtcagtatgtggaaactaccactgtatttgtagataaaaacggggtcgttacaaaagtggactataaaataaacagctcgcggtcaggtaactatttttgatatgaattacgtattcaagacaatactcgcggccagtttgctggccataaacttttcggggttctcacaaggtaaatactttgaagtagctattgagaagggcgtgttcaatggaatggactatggaagaataaggccacttaataaccagtacgacgtaaaacttccttatgggggcaaaaaccggcagcagcttttggagggcatactggaatacctgaaaaacagacctgccctgaaaattgatacagtgcttaataatggatctgttgttgtatatcgtgattttgccacgatcggcaacaagcaaaattgttttgctgatcttaccgggcttattttcctgtttgcgatacctgaagaaggatatatttccatccgtcccggaagcaattcaaagatatacgcttctgtttttgatgcaaagctgcgtatcagtccgggcgacgatgtagtatctgaggaagatgtgcctttcaatgagtataaatttatacagcccaccgacggccgtacgcaaagtgccgtggctccgcatggcggccttttgggtaaggcaacttcacgtaaaatcaattataaactggcttatcccgacagtatttttgatccggatggcaaagttgtaaaccccggcaataagaagcgcctggaatcattcttcgatggctatgtaacggatcttgatcagtttctgaaaacaaaatttaaaatgaagtaaagtaatttaaaagaaaagccaacttgtgtaggcttttcttttaagttataatttctcggctacatattttaccaattgaagcgctgcatcccaaccttcatttgcttctttaagcaggtaatccgtaatttcataattgatttcctctcttgctgaaagaatggttccatctccattttttgtaaattcatacgttatcacggaaagcaacctgcttttatctttgaggtcaaataaattatgcttcagtaatttttccggttccaattcaaggattactccgttcgtataaaggctgctgtctttccctttccatccaaaagaactgccagctttccattcagaaacatattcaacgcccatttgcctcgttaccttaggatctgtgaaaacgcgccatactttttttggggatgcgtttatttcgatcgtctttgtaataaccggtctgttcatatgttatgtttacggctttaaattaaccattcggtgggtgccttcccaaatttctttttaaaagaatgagaaaaatgagagaggctttcaaatcccaggtcaagataaatcccggatggttttttattctttttttctatgagatgcagggcttcctttagccgcatttccaataaccaccggcggggcgccatgccgaatattttttgaaagtcacgtttgaaccccgcaagactccttcccgtgaggtgtgcaaatttctcaatgggaacgttgtaatgaaaattggtgagcataaatttttccagatccatcttataaggttccgaaaagtcgaacaggaactctctgagtccgggcatgatatccaggaggagatacacggcttctttcactttaagcatgcctacttcattcgttattttcttttccgggtgacgaacatagggcatcagggattgaaagaaagcatgcaaaaaatcgttccccgggatcagaagattggaagcttctgtatatttttgcgctacctctatttgttcctccagcgcgattttcctgagcaagtcttccgtcaggcgaatcacaatggtttgataatcctggccatccaaaggcatcttggtaatttctcccagttgattttttcgtatcagcaacatttccccggcctccatggagatcttttgagtggcagtttccaatgtgaaccggcctaaaacctgcaataccagcgtgttatgttccaggaatgcaatcttctcctttctcatggcggagtggtaagagaaaaagatgactcccgggattatttcagttggattcatcatgatgtaaagatataaaacaggcggggtgtatgtgtcatttcactatcgctggaggtaggtacctccaagtattgctccttgcgaaaaatgggtattaagcgtgtttaattcatcggcggtgaacctgatatccatggcctgtatgttttccggtagccgtgatctcctgctcatgcttactaatggcatgatatgatcaccctgcgcatttacccaggcaatcgccagttgggttggtgtgtatcctttatcctttgccatctgcttcaatagatcgattttctccaaattctttatcaggttctctccctggaaacgcgagaagtgaagatggtagtcattggccggaagaggcgctttcatttcgccggtgagtagtccttcagcagtattggcaaacgccaccactcctatacctaactcttttgcggcaggaagcaggtcgttttctatctggcggtctgccaatgagtaacctatttccaatgctgttaccgggtgaacactattcgccttgcggagttgatctgcagtgatttcagaaacgcccagataacgcacttttccttctttgatcaggtcggctacagttccaatcacatcttctaccggaacactgttatcgagtctgcaaggttgataaagatctatggtatctacacctaaacgtaccagggagtagttaatgaaattcttgatggctatggggcgcaggtcaagtccaagcatttgattgccgtagaagatagcgccaaatttcacacttatgaaggcgtcgtcgcgtctgcctttgatggctttgcctaccaggagctcgttgtggccgctgccgtaaaagtctcctgtattcagaaaattaatgccgttgtccaatgcactctgaatggtagcaatactctcgctttcatcatttgccttgctgccccaaacggacgacatccgcatacagcctaatccgagtttagacacgagtggtccatttttgcctaagggcatctttgttattgttgtcatgattgctgttttattgattaacagcacaaagatcggctttgcaggctaccaccacttgcttttatggctcaatttacttgtctgtatggctcaccttttcggggagatgttcaggtcgcaaataaccctctggattgtcgtatactccccctgcccgaatcctcatttcttatcatctttgttttaacgaagtaatcaaacaacataaataaaagtggagcagcaaccacaaaaaacgggcgggaccgaaaagccagatgagtaggaacaaaatatatcttatgtcaaacaatacagtttcactgcacagagttcttaaaacatctccggaaaaagtattccgcgcatttactgacgccctggcaatcgcctcctggctgcctccttacggatttttgtgtaccgtacatgaaatgaaggcggagacaggtggttcttttaagatgtcattccagaatttcaccaccggcaatggccattcattcggcggaacctatctggaaatcaaacccaatgaatttttgaagtacactgataaatttgacgatcccaacctgcccggcgaaatgatcactaccgtatggcttaacaaaacaatggtgggtacagaaataaaaattacgcaggaaggaatacctgccgctatacccgtagaaatgtgctacttgggctggcaggaatctctggaaaaattagcgaaactggtagaacctaatataccggatgcctgattatattccggacggaaaacaaaagccgcgtaaatttcatgatttatgcggcttttttttgttgctaagcattatttcatcaggctgatatttgtcatcccgccatctgaaagaagctcggtaccgacgataaaagaggaatcatccgatgctaaaaatactgccgcctttcctatatcggatggaaggccttgccgccctgcaggagtcagatctctccagatttgtttaacctgctctacctgttcctgcggcactattttaccaaataccggcgtgtcaatagaacccggcgaaagtgcatttaccctgatatttcttgataataaatccagcgacaagcccttggctaatgatataactgcagcttttgcggctccatatatcgtcatgcctggtgcggcccggtgtgcagcactggaggcaataagaataacagaggctccgtcattcaggtaggggagtgatttctgaacagtgaagtaaacactcttcagatttaagttcatgtactggtcatagttgtcttccgtaacatcggcaacggctgccatagggctgccatctacaaccccgcctgcgttgaccaccagcgtatcaatttttccaaacctgttaaacgtttcctcgaatacatgttccaggtcatccaggtttgttacatcccctttgatacctatgaaaccctcgcccagcgttttaaccgcagcttcaatggttgcctggttccttcctgtgattgcacccacagcaccttcctgttggaaggcttccgcaatgccgaaccctattccgctattaccccctgtaactactgttactttgttctttaattttcccatcttctttgattcttttattggttacaccacaaaactaaggagtgattgtttatatttgatattaagtaacaaaaagtaacagtaacttttgagtaaccaggtaacatatgggtgacaacgaatttcaacaagaattcaggaaagaaatcatggcggtccatgatgcaatggatgtgctgaatggaaaatggaaaatatctattattacggctctttgctattacaataaaagacggttttctgatattttgaatgatgtaaatggcatctccaacaagatgttgagcaaggaattgaaagagttagagatcaataaactggtaaaacgaaccgttttggatacacagcctgtaaccgttcagtatgaacttacaaaatacggtaaaacgctgcagacagtgattaataatctttccgattgggggatggagcataggaagacgataattggcagataggtaggattgcggggctgttaagttgaatgaacaaagaagccttcaaatcttgcgacttgaaggcttctttgttcatttttcgtgacccccctggggctcgaacccaggacctactgattaagagtcagtagctctaaccaactgagctagggagtctttccaccgtctttgttaaaaaacgtgagcgcaaatttaacggatcttctgaatatttgtgtactttatttaattaaatttgataagaaggacgaaatgtggataaatatccattatgttgataatctaaccgttagctcattataaattttttttcatgcaagaagcgtacatagtagccggataccgcactgcggtgggaaaatccaaaagaggcggatttcgcttttacagacctgatgacctggctgtagacgtaatcacgggattgctgaaatccttgccacagctggatcctaagcgggtcgacgatctcattgtgggaaacgcggtaccggaggcagaacagggtttacagattggccgtatgatttcagttagagccctgggcattgatgtgccgggaatgacggtgaaccgctactgtgcctccggcctggaaacaattgcgattgccaccgcgaaaatacaaaccggtatggccgattgtatcattgcaggtggtaccgaaagtatgagcctggtgccggtagccggctggaaaacagtccccaattacaccgtggccagcactaatcccgattattatattggaatgggactcaccgctgaagcagtggctaatgaatttaaggtaagccgccaggaccaggatgagttctcttataaatcacatcagaaagcgctgaacgctattcagaacggctatttcaagccgggcatactccctgtttcagtagaagaagtatatgtagatgaaaaaggaaagaaacaaaaacgttcctacatcgtggataccgatgaagggccgcgtgccgatacttccctggaagcgctggcaaagttgaaacctgttttcgccgcgggaggttccgttacagcaggtaattcctcacaaacttccgacggtgctgccttcgtggtggtaatgagcgagcggatggtgaatgagttgggactgaagcctatcgggcgtttggtgggttgtgtttctgcaggagtgcatccgcgtatcatgggagtaggacctgtggccgccataccaaaggtgttgcaacgtgtggggaaatcgttgcaggatatcgacctggttgaattgaacgaggcatttgcttcacagtctattgcggttatccgcgaactgggcatcaacccggatattgtgaatatcaatggcggcgctattgcgttagggcatccactgggatgtaccggcgcaaaattaaccgtgcagttgttgggcgatttaaaacggctgaataaaaaatatggcattgttaccgcctgcgttggcgggggacaaggcattgcaggtatcatagaaaatatcaactgataaataccggtcaactcacctttatactaaaaaaggagccattggctcctttctttttttattctcctgttatttccagttcacttaaataccagtataccggttgtggaatcttactggcgtctacaaatacaatacgacgcgaatcggccggctgtcgcaggtcaatgccaaattcggacatcattctctcataaaaaaaagaacgctttccctttgctcttccattctcataggtcacaaagcaggcgcgcgatacacctaacaaattgctcatttcctgctgcgttagttttagcgatttacggattattctgattacccgcttattatataattgcatggattaggattaaaaatgttacaaaaatgtgccactgtaacaattattaactatatttgtatcgtaatgtgtaaatcactgatcttaaaagtgttgaattgatatgagcggcgaatttttgatagatagattttcattttgaacataaaacatccattaccggcgtaccggtaaaaaagatgtggagatgcaatcatttaatagcgggtactaacagctgttaaaatagtcagatgaagaggaaggaagaagaggtgaagggaaaactgattgatgtaacaaccggccaatcgccggatttctaaaaaaatccatcgtaaatttttttgtttgtaagacaaaaaccaaaggagctgtctttctttccaggaacgggcagctctcttttggctattaaggtattaaacatacattttcaaatgtagtagattttggtgcatcgggcaaataaaatattttgtaacaaattgatatcaaagtaattagatagatattaaaatgataatttagatatcaatatgatataaaaaatatcattgtgaaacttcttattaatataatctcactttctttttaattagattaaactttttgttaatttggcgctataatcggcccctaagccatcaaccatatcgccttatggatcgcagacaattcctaaccttatcacctgaccgccagcaacagcggactgccactactgtcgcccgtaccgccaccggcattactccgtataccggcgcctgggatactttacaacgcattcacctgctgaaacgcaccctgttcggggttacacccgcaaacgtcaatgccttcagcagcctcagtatgcagcaggcagtagatacattgctcaccgcgcagccagatcctgctcctcccgttaacaactacggtatcgatgacaccggcgttacgcccggtgccacatgggtaaaagctcccctcggtgatgaaatgctggaaagaaagagaattgactcctataaagcatggtggacaggccagatgattaaccaacaggcaagcatacacgaaaagatggtgctcttctggcacaatcatttcgttacagaaactggcatggttggcgatagccggtttatctaccaatataaccttaccctgcgtaaacatgccctcggtaattttaaagatcttacaaaggcaataaccctggatccggccatgctggtgtatctcaacggatacctcaactccaagggcgccgcggatgaaaattatgcacgcgaactgcacgaactttttaccgtaggaaaaggccccgattcccattatacagaagatgatgtaagggccaccgcccgtgtactcaccggcttccgggtagatagaaccaacatcgtcagcttattcgataccacacaacacgatcttaccaacaaagaattttcaggattctatctcaataaagttatctctggtaaaacaggccaggatggcgctaaagaactggatgaactcctcacgatcatcttcctgcaaccggaagtcgcaaaatttatctgccgtaaactataccgcttctttgtgtattatgatattgatgccgccacggaacagaatgtaattacaccactggcagatattttccgcagcagcggctatgatattaaagtcacgctcaacgcactgttcaccagcgaacatttctttgatccgctgaacatggcctgcctgattaaaagtcccgccgacttctgcatcggtatctgccgcgaatatggcatcaccttcccttcggattataccaatcaatataaagcatgggctgtggtccacgacagggccgcttcgatgctgcaaaacttcggagatcccccattggtagccggatgggacgcatactaccaggccccttcgtttcatgaactgtggatcaatacagatacactgcccaaacgtaaccgcttcagcgatggcctcgtcagcagcaacggttataacggcgtccgtatagacacactcgcttttgccagccgccttcctcacccggaagaccccgtggcactggtcaacgattccctggatatactttatcgtgtaggcgtttccgataaccttaaaggatttctgaaaaataaaatcctcctgagcgaccaaagccctgatagcaactactactggacgcaggcctggaacgcatggaaagcctcgccttcggatgccaccctgaaagataatgtggaaagccgcctccaggccctgtataaatacattatggacctgtctgaatatcaattatcctgatagcagaaaaacctttttatgaaaagaagagacttcctgaaatatacagcgccagctgctatcctgccaactttaatcaatggcttttctatcaaagctttcggttcatccccgatgctggacgcactgagcaccgcctcggcagataatgatcacgtactggttatgatccagatgaccggcggtaatgatggcctcaacatggtcatcccactggatgtatacggtaaataccaggccgcacgttccaatatcgctatccaggaaggaaaagtactccgcctcgataattatattaaatcaggcctgcatcccgccatgacaggcatacagaaattgtataacgacggaaaagtaagtatcgttcaaagtgtcggatacccttctcccaatttctcacacttccgcgctaccgatatctggctcacagggtctaattccaacgaagtgctcaccaccggctgggcaggacgctacctggatacacaatttgaaggtttcccggatggatatcccaacgataaggcgcccgatccgctggctgtacagataggttctatcgtatcgcccgccttccagggccccaacgccagcatgggcatcgctatcaccagcgctacggatttctataacctgatcgatggtgtaacagatcctgttcccaataccaaatggggaaaagaactggaatatattcgcctcatcgccaaacaaaccaatagctacgaaaaggccatcaccgcagccgcgaaaaaagtgacctcacagggcgcttacccggccaataacagcctcgcggaacaactgaaaatcgttgcccgcctggtagccggcggactgaaaacaaagctctacatggtaagcaccggcggctttgacacgcatgccaaccaaacagaaggtggtgataccaccaaaggaggtcacgctaacctgctcggtggcgtttccgatgccatcaaagcctttatggacgacctgaaaggattgcacgcttcccgcagggtagtgggcatgaccttctccgaattcggccgccgcatcaaatcgaactacagtatgggtacggatcacggcgctgccgctcccattatcattttcggagattacgtgaaccagggtgtgctcggaaattcacccgcactgccggacgcttcttctgtaattgataacatccccatgcagtacgatttccgctctatttatgcatctatcctggaacaatggttctgcgtggatcaaaccgtgctgaaaactattctccgggaagactaccagcgcctgccccttatcagcggcgtggcctgtggtaccatcaccggtctgcccgacctgaatacagatgataagaagctgattaccaactctcccaatccattttcaaattataccactattacctatatcaccggcagcggcaatacattggtccagatctttgataccaccggccgcctcatcagcgtaccggtcaataaagtacatacgcccggcacctatacgttcaccttcgatgcgcatagcctgcccaatggtatttactacgcccgcttccagaacggcccggtacaacaggtaagacctatgctgaaagtaaactgaccttataatttcattaatattcgtgcaacgctgttgcaaatagatggattttgctacctttgcctccgtgtacaagagctatctgcataaaatattagcgattattctcctgggtgtattttctctaaataccatcccaagggaatttatacacgaatttgcaggtcaccacgatacaacagatcccctccatcaacacgatggcctcacgatatctgaacatcaccggcactgtgattttctgcagataggggtagaaccttatgagtcatttgttactttatatatagcaccggtccaaaaagtaatctgggtattttctccgcttacgttaccggaaaccacgcacgtcccttattttaatcttactcccagagcgccgcccgcacagctggcataacttctttttttgcaacgtgaaccatcggtacatgttgtttattcttaattactgattctatatttttcagatatgcattatttgcgtgtatttatactcggcctttggagtgtaatgttactggcgttacctgctgcctatgccggcactaaccccgaagaaggggaatactcaaattcattaaccggtaaagtggtggataaattaacccatacaccgttacccggcgctactgtttacctgccggatctccgcgttggcgctgccgctgatgcacagggaaactatatcatcaaaaatcttccaaaaggaaagtatgtagtagatgtacactacatcggttacgccgcattcagtgctcctgtagctatttccggcgctactacccgggattttgaactcggggaaacactgatagaaaaaaatgaaatcgtaatcaccggcgccaacctggcaacatctgcgaggaaaacaccaacgcccatcagcgtaatccgccgcgactatctcgacgataatatttctaccaacattatagacgctattgccaaagtgcccggtgttacacaactttctaccggcccggccatctccaaaccctttatccgtggccttggctacaaccgcgtagtggtggtaggcgacggcgtacgccaggaaggccagcaatggggcgatgaacatggaattgaaatcgacgattacaatgtaagcaggattgaagtgctgaaaggccctgcctccctcatctacggctcagatgcactggccggtgtggtgaacattgtgccgcctgcaccgctgcccctgggaaaaattaaaggcaacgtggaagccaactatcagaccaacaacggactgatggcctatcatgccgacattgccggtaataacaacggctttagctggggcgctttcgtaacacagaaacaagcgcacgactacaagaataaatacgacgattacgtatttaattcccgctttaataacaccaacttcggcgctaatatcgggatcaataaacaatggggctactctcacctgagcttcacgtcctttaaccagcacctcgggctggtggaaggtgaccgcaacagcaacggcgatttcctgaaactcatcaacaacaacggcacagaagaagaagtacccgccaccagcagcgataataaatcgtacagcatgacggtacccaagcaacagatcaaccatcagaaaatagtatgggacaacaacctgtatctgcataatggtggccgcattggtcttacgctgggttatcagctgaaccaacgccgcgaattcggtaacgtgctggaaccttccacaccggaattgtacctgcacctgcaaactttcaactacgcgctgaaatattacctgcctgaaatgagcggctggcaaacaactgtaggggtgaatggcatgcaacaaacaaatcagaacaagggagaagaattcctgatccctgcatacgatctgttcgactttggcgctttcgcggtaacaagcaaaacttttaataaactcacactgagcggcggactgcgttttgataaccgttccatgaacgccaaatcactgttcctggatgcagatggcaaaccatccaatacaggagattcaaaatttgatgcattcaaacgcaacttcaataacgtatccggtagcgtgggcctcagctatgaagccagtgaacaggtagtgctgaagctcaatgcagcaagaggtttccgtgcgcctaatgtggcagaattgtctgctaacggcgtgcatgaaggaaccatcaaatacgaatatggtaaccaggacctgaaaccggaagtaagcacacaggtagatgcaggagtggatttcaatactcagcacgtttccctgtcggccagcctgttttacaatcatatcaataacttcatattctcccgcaaactgtttaatgcagccggtacagactctattccggcaacggataatgacgaaggatatgcggcatttaaataccagcaaacagatgccaacctgtatggcggagagctgatggtggatattcacccgcatccgatcgactggctccattttgagaatactttctcgtacgtaagggctactactgctaacagcagcgactctacgaaatacctgcctaatattccggcggcacactggctgtctgaattaaaaggaagatttaaaaaagtgggaaaaagtccgttgcataatgcttatatcggtgtgcagatggacctgaactttgcgcagaacgatgtgttttcagcttacgaaacagaaacgcctacttccggttatactttgtttaacgcagggttaggcagtgattttgtaaataagaagaataaaactttgttctccctgcatttcgctgtcaataacttaacagatgtggcttaccagaatcacctgagcaggttgaagtatgcacccatcaatgaagtaacgggcagatcaggcgtatataacgttggccggaatttcagtgtgaagcttgcaattccgattgatttcaaatagtgttaaggtttcttttaaagagctcctgcgtcagcaggggctttttttatggtgtcaggcgccggtcctgccggagcgtttcccattttagtataggtagccctgttattttttattttgaagaagatcttccggttggccgcgggttcggtattaaatccaaccgcagtatccgttcccgttatcatcagttgaggcaccggtatggttgcagcagcagaatcaattgcccgcatgtagttgatcagccgtttgccttcccgcgtaatatggatggtttgcatgcccgttcccgaattggcgatggaagccgtaatgcctgctgcctcaaacacagcgctgtcgctgtttatatttccacttataaggctaaaagggacgggtattgtttgggttccggtaacattggccggagttgcttcctgcggggttttggtagccggctgtttgcagccaagtagtaaaacagggagcagtaataaggttctttgcacgataagtaactgtttgaaagataaagctattaaatttttacggaactcatcatgaccccgcttaatatataaggcttacttatacattatttttaataataacgttatgatattttctaatttatattaatttgctgcgggggatgtaaacccggtcctgacgggcttgataagtaaaatcgttttttcagtataaatacacggtggttttaccattgatgtaaatatttaattgaaatattgatagattttgtagtttagaggatcgttaattatgtaagtgtcagattgaatgtcctgccaggaggaacagtcccctcagttttcaaaaattggtttttgttattaagacttttctgaccaccattggttcagattttggttgaaaaagaaaggggctgtttttacagccccatatttttttcagttattttttttaatgttgatgtgtcggcttttccagtttctctgtatcgtcatcataatacacaaagaaataaagataaatagccctggatagccgcatcagccatggttgtataagtaccagcaggaccccattcacggcaagccagataaaaatgctgttatctctccaggttaatccaaaaaataaccagaaccagatcaggttaaacacactgaatgccaccgataaagcataactaacatagcccgttccaaaccagaagccagtttccaactcatatttttgtccgcatacagggcagtgatcatacatattaaagatcttcgaaaacctcacgtgaaacggattctgatctctgaacatatctcctttcctgcatctcgggcatttcatagtcagcatgctgacaaaatagttagggcgcctgggctgttgtgtactcatgctgcaaaattaatcaattactttcagcaactgaaagtggcagcttacaccgcttccgttttgcgctcgccgatctgttgtctccacatcgcatagtaaagtcctttttcagctaccaggtctgcatgtttacccatttccacgatctgtcctttttccagcacgtaaatacggtcggcatgcataatagtgcttaaacggtgtgcaatcatcacggtaatatgctgtttgctggccgttacttcacgtacggttttagtaatttcttcttctgtaatagagtccagcgcggaggttgcctcgtcaaatacaagtaaacgcggtctgcgcaacaacgccctggctatggataaacgttgtttttccccaccggaaattttaataccgccctcgccgattaccgtttcaaggcccttgtcggccctggccagtaaagaataacacgaagctttatccagtgcttccattacgtccgcatcagtggcgcccggatttacaaacagcaggttttcacggatggtacctgaaaacagctgggtatcctgtgtcacaaaacctacctggtgacgcaggtcttccatatctacttcattggcatcaataccattgtagtagatatgcccttcatttggtttgtataatcctaccagcagctttaccagcgtggttttaccggagccagatggtcctacaaacgcaatggtttcccccacatttacggagaagttcaccttatcaagtgctttggtggctgcagtcaggtgcttgaatcctacctgcttgaattgcagttcatcaatatgcgttaccctgatgggattagcgggcatttcctctaccggcgtattcaggatgctctggaaattcagcagcgatacctgcgcttcgcggtaattcaggataatgttaccaagttcctgtaatggtccgaaaatgaagaaggaatacagttgtaaggtcatcagctgcccgatgctcactacatcgcggtaaatgtagaacagcagcaggaacaggatagcagaacgcatcaggttcacaaaagtaccctgtacaaaactgatactgcggatgctccgcacttttttcagttccagcaacaggatcttcatggtagtggagtttaaacgcctgatttcctggttggagaggcccaaactctttaccagttcaatgttccggagcgattctgtcgttgatcctgccagcgcggtggtttcttttacgatcgtcttctgtatcaccttaattttcctgctcagtaaactcatcaggatagtcagtaaaatacagccggtcagatatacgaatggaaggctccagtgtacggtggtggcgtataccatcacaaacaatacacctatcagcgatacaaaaagcacgttcacaaaggcggtgatgaatttttcacagtctacccgcactttctggagaatagccagcgtttcaccgctgcgctggtcttcaaactgctggtatggcagccggagtgagtgtttcaagccatccgtatatacctgggcgccgaatttctgaacaattacgttcacaaaatagtcctggaaagccttagcaatcctggataccattgcaacgcctatcgcagcgccaaccagcagcagtacccctgtgaggtactcgttctccggccggaatatagtgccacccttaaaagtttttggatgagaagcgaacctgtcaatgatccatccgaagatcatagggtccatcagtgagaaaagctggttaatactggccagagccattgctaatacgaccaaccatttatatctcttcaaataatgcagtaatagtttcatatgtccgttttcctgaggtgcaaagttactgtatgttgtcacatattccggggaaaagtactggctattttagtcaaaaaacgttaacttaatagtaagttctttgtaaagacacaggtgagtatctattatctaaataaatctccacatatgaagacgtatgatgaaaaacacatcaaaaacatcgtactgttaggtgcacccaaaagcggcaaaactaccctctccgaaaccatgttatttgaagccggcatcatcagtaaacgaggctcaattgaagagaaaaataccgtgtccgactaccacgatattgagcacgaacggggaaactccgtatatgccaccctgttgcacaccgaatggaaagattataagataaatattatagacacacccggactggaagattttatcggggaagtaattgcagccatccgcgtatccgacactgctgttctcctgctcaatgcccagtatggagtggaagtaggtacagaactggtatgggattatgtggacaaataccggaaacccaccatattggccgttaaccagctggatgctgaactggccaattttaataaaaccgtggaagacgcctcccgggtattcggtcagcctgttactattatgcagtaccccgtaaatgccggccccggattcaatgcgatcatcgatctcctgaaaatgaccatgtaccgctttcccgaaaaaggcggcaaacccgaaaaactccccatccccgacagcgaaaaggaaagagccgaccagctgcacaacgaactcgtggaaaaagcagcagaaaacgacgataccctcatggaactgtattttgaaaaaggaagcctggatgaagatgaactccggcaaggcatcaaaataggcatgctcaatcaccacgtattccccctcttctgtttatccgccaaaaataatatgggcagcggccgcctcatgggatttatcgataatgtagcccccagtgcagcggaaatgcctgccgaagttattaccggaggtaaacctgttccctgtaatcctgctggtccggcaggattatttgtttttaaaaccttacaggagccgcatatcggcaggctcacttattttaaggtaatgtcgggagaagtaaaaggcggtatggagcttatcaacgaacagggcaatactaccgagcgtatcagccagctgtttatcgcagacggaaagaaccgcaataacatagaacgcctgcaggccggggatatcggttgcacgcttaaaatgaaaagtaccctcaccaatcatacactggctgaaaagaatttccccgggcaaattgttcccatcgattttcccgcccctaaagtgagggtggccattgaagcaaaaaataaaggcgacgatgaaaaactcagcgaagtgcttgcggaaatacacatggaagatccaaccctcctagtggagttcaaccgcgaactaaaacaggtgatcctccacgggcagggagaactgcacttgctggtgaccaaatggcgccttgaaaatatttataaaatgcaggtggcttttcacgccgccaaaataccttaccgcgaaaccatccaaaagcctgcccaggcttcctatcgccataaaaaacaatccggtggtgccggccagtttggagaggtatacatgaaaatagaaccctggtacgagggtatgccgccctacaaggaacacaccgtgcgcgattcggaagaaatagcgctgaactggggcggcaaactggtattcaacaattgtatcgtaggcggcgctatcgacaaccgtttcctgccatctatcctcaaaggagtgatggaaaaaatgcaggaaggcccgctaaccggatcatatgtacgcgatatacgtgtaagcgtatacgatggtaaaatgcatccggtagacagtaacgacatctcctttaaaatagccggtatgatggcttttcgcgaagcattccaccaggccgccccgcagttgctggaaccggtgtacgacctggaagccgtagcccccgatgttatgatgggcgacataatgagcgaactgcaaacacatcgcagcatcataacgggaatggatacactgaatggttaccaggtgatcaaagcacgcaccccacaggcagaaatagataaactgtttgctgcactgcgcaatgttacccagggcaaagccaagctgaaatcccagtttgcggaatatgcacccgttcctgcagagatgcagcgtaagctgagcgaaagttacaaggaagacctgggcgtttaacgggataatgtgtgcgccaccatcgttaccgctggcagcggccattgcccgatgctcagttcccccagttttccctgtcgaggctcctgaactgtatggcctccgccatatgtgcaggttctacactgtgactgccttccagatcggctatcgttctgcttactttcagtatccggtcgtatgcacgtgcggagagctttagtttttgcatcgcctgccccagctgctcccggcatttatcactgataacgcataccgtggccagcaaccggctatgcatttgtgcattacaatacacgccgtcatgaccagcaaaccgctttgcctggatcgccctcgcagcaatcacacggttacgtatatacgtacttttctccgtcgcactggaggacgacaggtccgcaaattttaccggcgttacttctacgtgcaggtctatacgatccagcagcggaccggataccttattcaggtattcctgtacctgcccgggcgcacaggaacattctttttccggatggttgaaatacccgcacggacagggattcatagacgccagcaacataaagctggctggaaagtcgatggctgttctggcacgggaaatagtcactcttctttcttctaccggctgccgcatcacctccagcaccttgcgtttaaactccggcagttcgtccaggaataatacgccgtgatgcgccaatgaaatttctcccggctggggaatgctgccaccacccaccaatgccgcatcactgatggtatgatgcggagagcggaacgggcggtgcgtgatcagcgaagtgtgctcggggagcttccctgccacagaatggattttagtggtttccagcgcctcctgcaatgtgagcggtggaaggatggtgggcaaacgttttgccagcatagtttttcctgctcccggcggaccaatcaatatggcattatgcccacccgcggcggctatttcaagggcacgtttaatatgttgttgcccttttacttcgctgaaatcaataccccaatggtcctgcgtggcgtaaaattcgtcacggacagccgttacaggtatgaggcaatccgggtcatttaaaaaattaatggcctccgaaatatgagcaatgccatacacttttaaaccactaaccatggcggcttccagcgcattctgtttgggcagtataaagccgctgaaaccatctttcagtgcctgcatggctattggcagcgcacctttgatcggttgaatggtaccatccagcgacaactcgcccatcatcaggtaatgctcaagatgaacgggagaggcctgtccggaggcagcaataatacccgcggcaatgggcaggtcatacgcagcgccggccttgcggatagcggcgggcgccatatttaccactgtgcgcgttctgggcatacgcaggcccatgcactgaatagtggattcaatacgccgttcgctttcctttaccgcattatctggtagtcctactataaataatttgttgcctttggaagatacatttacctctatggtaatggtgatggcatttacgccgaggatggcgctgccgtaggttttaacaatcatatcgatatctgggttaacagatacgaatataagcatttaactgctggaaacatcgttacatcgcccgcagttaaatgctttccttttttattttatctgcgtaagcagatccagcaccttctctcttttcaggatcaggtaacctattttttctttggcaattccatctttgagcaggtaggtgaaatgcaggtcgtcatcaataacggtagattcaaaatatttaaactggatacgtttttctgtgctcagttcatccgccacttcataaaggtgagtagaaaggataaacaggcagttggtacttttcaaaaatccccggatcactgccagcgagcagtttctggcatcttccacattggtgcctttaaacatttcgtcgatcagcaccagccagtttttaccattgctgatttgcaggatagtgtttttaatacgctgtacttcgctatagaaataactttctcccttaaaaatattatcctgtacctggatgttactgaagatgccgtgaaagaagctcagctccatattttcagcgggcacgcccatgcctatatgtgccaggaatacggctacgcccacggctttgataaaggtggttttgccggccatattagcgccggtaaggaacatgaaatgagctgcttcatccagttttacatcataagccaccggctcaggaaggatgatatgatagagttgtgtggctttaataacaggtgtggtgccgccggagaaaaccgggaactgcaggttatagtgcttcatggctttggccatcgcatagtacgcatccagctgctggtaaagggttaccagctcctggattacttttctgtgtcgcttccggatataattatcataacggaggatctccacaaagttcagttttccctcttcatctgcctttaaaatttcatagaattcttttttggcaagtagctgttgcgccctgtccagcaacactttcagcactgttggggtctcgtttgaattgaaaacgttgataaacgaacgaaatcctttcagtaatatcaccagttgtgtaaacgaaaatttgatatagccataatcaggcgcatacagcgttttgttgagtgctgcatgaagatataaggcaagtccttctgtgctggaaataggttcgatctgggcatccatgtaattctccaccactacaatggtaccgttggaaataatggaaggccagttgctttcctgttccagtatatattgcaatgcacgctgccggttcttaatagtgttgatatcggataaaggattgctgtatagctgccgcaggtattcacggccgcctgcagtggtagtaaaatcgaggcggtggaacagggaaaattcttcgtcgcggttaaagatagacaggtcgtagtaggatgttttgtccagttgcatgcagcatctttttggtgaatatacggtggaagatgcaaggatagaaaaattccataagaattgaaaggccgtaccggcatttccgtaaatgcagcggctgccgctgcatttacggaggcaaaaactaccggctgaaagccagtcgctgacccaatatgttctcattaaaaacgccatccgcataagcgaggtgtccgcttacaaaggtatgcgtaacggccgcagggaaggtatggccttcaaacgggctccaggcgcatttataatatatgttttctttatttacgttcgtctggtgctgcaggtctacgattacgcagtcggcataatacccttctctcaaaaatcctctttcctttatctggaaacagatagcaggagcatggctcatcttttccactactttttccagggtgatgtttcccttctttgcatattccagcattagcaggaggctgtgttgcaccagtggaacaccggacggcgcctgcaggtaaggcagttgtttttcttcccaggtatgcggtgcatggtcggtggcaatgatatccagccggtcgtccaggagtccctgccagagtgcggctttgttttccggcgctttaatggccgggttgcatttgatcaggttgccgtattgtgcgtagtcatcggcagtgaagtggagatggtgtacacacacttccgccgtaatccttttttctgccagcggcagcatattgctgaacagctgaagctccctcgctgtggagatgtgcaggatatgcaggcgggcattgtgtttctgcgcaaactgtatggctaccagggatgattcaaaacaggcttccacatcgcgtatcagcggatgatccgcagcggtgaggcgatctcctttttcccgttgaaaagcctccatattggcgcggataatcttttcatcttcgcaatgggtggcaatcagcagttcgctgttggaaaacaccgtttccagggtgagataattatctaccagcatattcccggtagaagatcccatgaatattttcacgccgcaaacgctttcttttttggcgtttgttttcagtatttcttccacattatcattggcagcccccataaagaaggagtaattggccagtgaatgatgttgtgcaatggtgtatttgtcttcgagtagttcctgggtgagcgcggccggtttggtattgggcatttccataaaactggtggtaccgccggctaccgcagcgcgtgcttcggaataaatggtggctttgtgggttaagccgggctcccggaagtgtacctggtcgtctataacacctggcagcaggtgcttgccttccccgttaatttccgtgtaattaccgctgatagtgatattaggcgctattttttcaatgcggtggtctttgatccatacatcctgtaccgtggtgcgcccttcgtttaccacggctatattcctgatgaggtaattttgcatggcgcaaaggtaaaaaaatcagcgtaatgatggttaatcggtgtggttgggaggcaatctctccggttacccttccaggtgaatcgaaaacacaatcatcctcgactgtaatttttccaccacattggaatatcgcaggttagggtctttcacatgcacattgccaaaaccattgctgatcttaaactccggggcaaagatgaagctctcgaaatagaactcaaagccagcgccggcttcgtaaccgtagtcgctctttttgatctttaccaggtcctctgctctgcgcagacgtgcgttggaggccaagtcatagtcatatttaaggcccgcaatggtataaacgcgcatattgccgatgcggtccgatttaaatttaatctgtagcgggaagctcagtaatatcgactcaatcttcttgtcagtatcctgtggcttgggataagtttcgcggtagtaaaggtttttggatgcaaaaatgagctgcgggttaaagcgaaggtcaaaatgctcactgagcctggcattggccagcagtcccaggttgaatcccatggttttcagcggttccgctaccataatagaatcatcggccaggaaggcaggagaatgctccagtttgaaatacgactggtttgccgccagcgtaataccaaagtaatagggttttgcatcgtgttccaacatattcatctgggtttgcgcccttgcaggaagcaccccgaatacaatgaatatcagcgcgtagcgcagtaaatggaacatatgccgaatgttagcgttttgcatgtaacggcctggaaacgggtattggttaaaatagttcgcattgcttcaccctgcggaaacgctttcacagattccggcagataactataagccgcctggcttttagctatccatttcccgatcagcggtgtgatataacgaaaatacgaattatataattgtttaataggaaaaactgtgggattcgaaaactctagtatcaccaacttgcctccgggcttcaacacacgatacatctcagacagccccttttccaggtgctcaaaattacgcacaccgaatgccaccgttatggcatcaaacgtttggtcgggaaaacttattgtctcactatcgcccgtttgcagggtaattttatcgcctaaccccgctttcaggatcttttcacggccatgactcaacatcccttcagaaatatcaatgcccacaattttgtcgggatgaagacgcttttccgccataatagcaaagtcgcccgtgccggtagccacgtccaacatgagtttgggctgaagcgatttcaaataccccagggcttttttacgccatataatgtcgatccccagcgacataaagtgattaagaaagtcgtagcggtaagcaatatcatcaaacatggtcgctatctgctccttcttgcttaattttgacccttcaaagggaacgatcttctgaacatttgcattttctgacatagtgcgcaaagttaaagaaatgtagtcatgtgacagtatgcaaaaacagggatacgggatttttaatggaacaaagcaatatcattatggttattaagtcagcagaatatcttatcagtagtcccgattgggaaaaatgccccaatcccatatggcctgaatacgcattcatcggccggtcgaacgtaggtaagtcttctttgatcaatattctggctaataatgaaaaattagccaaaacgtcgggaacccccggtaaaacacagctgattaatcattttgccatcaataacgcctggtacctcgtggatctgcccggctacggattcgctaaaagaagcctgtcgcaacgccgccaatgggaacagatgatcgaaaattacctgcgcaaacggcccaacctcgtcagcgtatttgtactcatcgacagccgccatcagccacagaaaatcgacatcgattttattaccaaactgggagaatggaatatccctttcagcctggtattcaccaaagcagataaaagtacccaggcagaagtcagcaaaaacgtaaaatcttttctcaataaaatgagggaaacctggcagttcctgccccccaacttcgttacatctaccgtaaagaaatccggccgggatgccatcctcaactatatcgatgaactcaacgcacaattccgggccatcgcctgatccgctgcatcatcttttctgcacactattattacctcagtaatctggggtaattttttatttttatttgtttatcttaatcagtgatggcatttttttacccaaatacttgttggaatgctggatgcaacagatgaaatactgtgtaaaaagataatagcgcaggatgaggaagcgttcagggtactgtatgaaaaataccgggatcatatttatggctacaccctgaaactctgcggcctgccggaagtagcatccgacgccgttcaggaagtatttatgaagatatgggtaaaaagagataccctgaatcccggattatctctcaaagcctacctgtacaccaccacccgaaactatgtattcgactacctgagaaaggcggtgcatgatcagaaattccgcgaatattttctgcagatgtatacagaagataccggcgctatggacgacatgctctacacccggcagctggaaaccattaaaatgaatgccatcgcccagttacctgcacaacggcagctgattttcagaatgagcaaagtacagggctgttccaaccaggaaatagccgatcagctgggcatctctgtcaacaccgtgagagaccagctcgtaaaggcttcccgctttgtaaggcactacctttatcaacatgccgatatctctgttattattgccgccttttgccatatccttcgctgagaaaaaaatatttttaagtccggtcgtcttttaaatccgcccgatcgtactattgttatgtcaaccaggaacaatggaagaaaataaggaacggatcactgctctctttattaaattaacggaaaggaaatgtacacaggaagagcgtttggagctcctcgcctggttacaggaccacccatcgccggagtatttacctgcggtggaagagttgttgctgcagcaaaactggcccgcaatgccggcggatagggccggtcaggtttttgctgccatcctgcaacatacaccgtccaaaccggtgatcccgttatggaaaagaaccggcttcagagtggcggcagccctggtaccactcattggcctggctaccctgttgttatttttttacagagataaaaatgataaacgccattttgtaaacaacacccgccaggtgcaaaccttccggctggaagatggtacggtgatcagtctcaatcaacgcagcagcctcaccgtaaacacatctccccgtaaaaatcagcccagggaagcatggctgaaaggagaagctttttttacagtgattcaccaggcagcaatgccctttgttgtgcacacggaaaacggcgtggatgtaaacgtactgggcactgcctttaatgtaaatacggcaaatggaaacgcagtggtagtgctgaacgaaggacgcgtgaaagtcaacgccggcgccggcgtcctgttgctcagtcccggcgaaatggccagctataatgcggtcactaaaatgctcaccaggcaaaaggtagataccttgttccagacatcctggaaatacaacctgctcgcattcaaaagtgaaccactgaaaatagtgatgcaaaaacttggggaacaatatgattatgaaatagtatttgaccaggaaagaaccggggaactgctgtttacaggctatctcccgtccgataacctgcagcaggccattattacgatagaagaatcctttaatttacaatttactttacaacacaagactattcgggtgaacaacaaaaaaatcctttagagacaaccaaaattcagttatgaaaaaatttaaatcaatcagtttccaactggtaatggttaccgctttgctatgctgtttgcaatggtcaaaagcacagatactaaaagcagcaacccgcgaaaacaaggtaaccactgtgccgcttatttcggtgatcaatgaactggaagcaaagttcgatgtccgcttcagttacaacaccaacctgctgaaagggaaaaatatcctcctgcagaatacggacatttttcaggcagataacattgagaacaacctcaataaatgtatcgcaccattaggattggtatgccgcaaaatcaatggaaagctttacgtggtaaaagcagaagatgctgctaatacccggtctgtgatggctgccgccggcaacattgcaccacagcaaaacatcaggggatctgtaaaggactccaccggtaatgccttaccaggcgtgattatccaggtgaaaggctcctccaaggctacgatgacggacaaagacgggaacttcgccctcgataacgtaaaagatggcgatgttcttttattcagcttcatcggctacacaccaaaagaatacaccattaaaggggaacaaaccattaacatcgttctcatcgatcaggccatcagcatcgaccaggtggtagtaaccgccctcggtatcaaacgccaggaaaaagccctgggatacgcggtacaaagagtaaaaggcgaggccgtacaaacggtaaaaggagtggacctggccacttccctcaccggccaggtatccggtctggttattaaaaactccaccgagttttttgctaaacccgctattgagttaagaggggaaggtaccttgctggtggtagatggggtgccgtatggcaacatgtcgttacgcgatatccctaccgatgatattgaaagcctggatatcctgaaaggtcctactgcatccgcattgtacggctccagggctgccggcggcgtgatcctcatcaccactaaaaaaggaaccggcgaagccctgtctgtaaacgtgaacagcaacaccatgatccagagcggttttctggccattccaaaaacacaaacttcgtacggccgtggacaaaacggaaaaattgacaacgattatgtatggggcccccggctggatgcaggcaacactgcaagggactggaacccggtcaccaaacagtttgaggataaccggccactgaattcggtaggaaaaaataacctgaagaattttatggaactgggcgtaatcaccaataataatatcaacgtatcacaaagtgggaaatacggtagtttccgcgcttccctgaaccatatttataacaaaggacagtttcctaatgcgaaactgaatatgtacaacttcaccctgggcggtgagctcaaggcgacagagaaattcagcctcgaagggcacatgggcgtaagcaaaagaatggcgccacaggtatggggcaccggctatggtaaccagggatacatttaccagctaaccatgtggaccggtcccgaatacgatatccgccagtaccgcgactactggaaaacacccaatcaaacacaaaactggatgtacaccaactggtatgataatccctacctgattgcctacgaaaaattaaatgcgatccagcaaaataccactaacgcaagtctcaccgctaactataaattttcccctgaccttagcctgttggtgcgtatcggctatgatgtgtatcataataaagaaacctttaccaatccaacggctaatatctactccacccgcggcggatggaatgccaggggattgtacagcatcaacaacacctggggctggagtaccaacgacgacgccatgctcagctacaataaaaaagcaggcgattggaacttcgaagcaatggtgggcggaacaatttattattgggtagacgaaggactgaaagcttccaccaaaaacgggttaacaagccctactttcttttcgcttaatggctccgtagaaccgcctacattcacacctgcctatagcagcagacaggtaaacagtttgtatggaagggctgctgtaagctggagaaataccgtgtttattgatgctaccggccgtaacgactggaactccgcacaaccggaagaaaacagggcgtatttttatccttccatcggttccagtgtagtattgtccgaattattcaaaatgcctgcatttacagatatgtggaaaatacgcggctcctgggctacctttaaaacacccgcaggcgtatatgatatcaaccgtctctatactaccactaccggcgcgtggaacggcgcaaactccgcgagctaccccagtaacctgctgggcgttaacctgctgccaagttcacagcgtacctgggaaattggtactgccgcctacctgttcaaaaaacgtttgaatatcgacgtcgcttacttcaataaatactattacaaccagcaaacttctgtatctattcccggctcctccggattcctgaataccctggtaaatactgccgaaacctatgtaagaaaaggactggaaattacgctcggcggaacggtattaaagaaaaagaatttccaatggggatccaccatcaactggtctaaccagcaccgctactatgtaaacctcgatccggtgtactctgcgcaaaatccctgggtgaagaaaaaagaaagactcgatacctatacagattactattggctgagagaccccgatggcaatgtaatccacaacaacggctatcccgtggaaagcgattaccaaaaaaaatatggttacagtgatcccagtttcagttttggttttatcaataccttctcctataaaaattttacagcatcacttaatatcgatggccgcgttggcggggtgatgtataactatatctacgataagatgtgggattccggtaccaatcccgaatctgataaccaataccgctacgatgaagtagtgaacggcctcaccaattatgtaggacaaggcgtaaaagtactctccggaagtgtttcctacgacaactttggcaacatcaccagcgatacccgcaagtatgcggtgaatgatacagaagtatcttaccaaaactacgcgcaaaatttcaggggaggcgattacggcatacaaaagaaaacatttgtaaaggtgcgtgaaatatctgtcggataccggtttcctgtcaccatgctggcaaagagcggtataaaaaatgcatctgtttctttaactgcacagaacctgttcctgtttacaaacttcaaattttcagatcccgatgtggatgatgaaaacctgaattcaccatctcaacggatggtgggagttaatttcaaagtagggttctgatatctttcaccatcaaagaaaatctcatgaaacacaaatcactgaaatatatattatccgtatctcttactgccgcaatggtaacaggctgctcaaaatttgataaaatcaataccaacccaaataaaactacacaggtgagttccgccatgctggccaccaatatgatcctgagtattaccaggtcggatatcagtaccgccaaaagttttatgcaaccttatctgctgggtaaatatcttacctggggagaaggacaggaaaatttccagtataataaattcggaagagccagttttaacaggatcgcattattgcgtaatgtgccgcccatgataggctatgcacctgatgaagaactccggaaatcatacaatgcactgggacattttataagagcctggcaattttttcaaagcactatacaggtaggcgatattccctactcacaggcggtgaaaggagaatcagaaaacgttatccaacctggctacgatacgcagaaggcagtatttctcggcatactcaatgaattggatagcgccaatcttctttttgcagcagggaaagattttagcggtgatccggtgtataacggcaaagtggataactggcgccggctgaccaacagttttgaactgcacgtgctgatgaacctgtacaggaaaacaggcgatgcggatctgaaagtagtggagcggtttaaagagatagttgccaacaggcctttaatgcgttcttatgctgataattttgctcttacctatacggcagcagcaggccagaattacccttggtccgatgtgccggcgggctccggcaactcttttgtaaagtcaaattacaccatgttgtcagccacgctgatagatccgctgaaaacattgcacgatcgtcgtttgttttactatgcaaagccctcaccggtaaaaattgcagccggtaaaacagcggatgattatgacgcttatgtaggtgcggagccttctgatgcattccctgcactgcaatctatacgcctgtcaaaagattattccgacctgaacagccgttatgtaaacatggtgaatgcagaaccggtaagcgttttcagctactcggaattacagtttgtattggcagaagcagccctgcggggatggatcaccggcacgccggcgcaaagttattatgctgcaggtattaccaattccatgaaattcaccgccgcctatacaccggacatagaagattatcaccacaacatgaaaatggatgatagttatattcagtcgtatgtagcatcggtggtactcactggcagcatgcagcaacagttatcgcagattattacacaaaagtatctcgcggggttcctgcagggctccaattataatgcgtggtatgagcaacggagaacaggttatcccgtattcaaattgaatactaccaccaacctgaatacgcctgctacgcagtttccggtaagatggctttatcctgataatgaactgagttataacaatgcgaacctcaacgaggccatacagcggcagtttagcggcagtgataatgtgaatagcgtgatgtggttattgaaggattaaagtataaagcggggatgaaagcgatattcgttttcatccccctgcttaataataattgctgtattaataggctaccttgccgtaagtcatggtgcaggcatcagaaatgttaccggtcagaattattgcatcgctcgtaaaagtgacaaagaattcattgcttttccctattgtcagcacattttgattgttaacctgtttaaggtgaaacgtatcggcggtttctcttacaccatcaacaaataattcgtattgtttacccttgaatattatttcctgcttattggtaacaggcgcaccctgtccgctgaaacatccttctacctttgccagccgccatctcccttctatagaagtaagcagtggagcatctttctttttacaggcagaaaaagcagttattaaaaacaggacaaggagggaataataagttctcataacggggtgattggttcaatgatttatagatggatgatcagttaaatactttattattgataatcgtttgattgatctttctctcaaattccgcgaagtaggcgggagcgggaccaccgggtatatctaaataaatggcggtagtgtctgttggatttttttgtacatatataaatgcccggaagatgccatctgctgccccacgtgatgagtaagtattaggatcggcttttatagctgcccggggaaagttggtgagataaggtttcaggctgtcttgcacgttatttggtaatttccttgtacttttttcactatttttttgagtaataatatagctgccatctgcagtgatctgtagcgttttgaattcggcgttgggaatgctcgagcctgcgtcatacacaaacaacgacgtagtatcgggagcttccactttatcttttttacaggaaagaacgcagaggcacgccagcaacagtatggctgccaatgattttggtagtgtcatataggaggctgttttactgaatgtatagcgtagaaaccaggaaaaagttacaacagaaggagggattgtatagctcgataaggggagaaaatgccacctgacgtggcgacacgtcataaaaaatctgagagaggtacaaaaaaaagaggcgccttagttcactattttattagcgcaactgctgctggcaaaggcttccggtttggctttaaaggcaaagcccatacccaggatatagcccattgcttcccgcaaggccaggttgcttttgaactgagggttcgtattgatgtctgcatgcacttccatgtctacatcatattctgtaaacaggtcacacaattcatacgcaatttcaatactcttcgctacttctaccagcatgcgctctttgatagaatagcggtcttttgttttttcattgtgaataaacataaatccgccgtggccttcccgcaggaatactatcaccgtagcgaattccgtatctactccttttacctgggaatcagtaccaatgcacactttcaggcgaaacccctttgcggtttcacgaacgatggcttgtcttacttcttcctttaccggaaggtggataacctctccattaaatcttctccattgcatacatgtataattaagggtgaacatgcgtatttgggttatgctataatgcctgcctgctgaagtaattccatgcgctaattgggtcaacaatatgggatgcgttcattggggaataacagcaatatttacgaatatacgaaaaagctgttagcaatagccaacagctgtacattaaaaaaataagaagattcagaaaataaaacggctagaactgccccgtactaagcattacaagggtacatgcttccaccggctgaatattatgctccctggcaatatcttccagttcgggattttctgctcccgggttaaagatgatacggcggggttgcaactgcaaaatataatcataatattctttctgtgccgccgggttcaggtacatggtaaccgtatctactttttcgagcggtggatgcgcggtaatcacgggcgtatcaccaatggcggccgcccgtttgccgatcgccactaccgggtgccctttggctttgagccggttcacggccaggttgctgtatctttccgggttgggcgatgcgcccagtaccacggtgagctttttatcgttattgggttccatatagctaatttacggaattcaccacaagtgataagcgctccggggcagatgcgcgaggatatcgctgcatgcccccgcaagctccgggaattgaaaagtaaagccctccctggtggccctggcaggcagcacccacctgctttttaacaaaagttctgcttctgtgccaatcagcatggcacccgcttttaataaaggaacaggtgccggcaatccaaaccggtaccccgcagcgttgcgcagcgttttcataaataccttgttggtaaccgggtggggcgccgtacaattaaacaccccgcttaaagcatcgttttcgtatagccatgccaccatcctgcacacatcggtgatgtggatccaggtatacatctgtcgcccgctgccctggtggccacctaaaccggcttttataaggttgaggtagggctgcattacgccgccgggtttccagccaagtgtaatgcctatacgcaatattattttccgtgtatgcggtagtgtaatgctatcgaacgattgctcccatcgtttacatacctgtacagagaagtcattttctatctctccgttaaattcatccatcggccggtcttccgcatgacggtatatggtggcgctgccggcgttgatccatactttgggtggatttttcagcgtaagtatagcagctcccaatgccctggtggcattaaccctgctatttacaatcgcctgtttattggattcgttgtaccggcagttcacactcttgccggtgaggttaatgagcagatcggtatgctccatcgcttccacccagtttcccggatgttccccatcccattgctcataacggatacgccccgaagaaggacgtgcatgtcgcgtaaggataataatatcgttatccgcaccaaaatattcagcgaagctgctgcctataaagccggtgcccgcagcaataacaatacgtttattttgcataaaataaagttaaaccggggtggaagtagccctgctatggagggtaacaatacatctccgtatagttaatcccgttacagacaatatcagcgccggcagcacaatataaaaactggcgtaaaccagccatccgtaaatattgaaaaaatcgatagatctgaatacccgtaacttgtttgcctgtacgaggagaaataagattcctataatagagaacagtacgcactggagttttcgtagcatcctgtcatcaggagctgttttccttagtataaaattgataacgcctgcagagaattgccaggccaggaggatgaaagtaagatatggcggcagggagaatttggaaaaaacaacaagatgagtaatatcaatcgcgcaaataacagtcaggagcccttgaacaatgccatctactatataatatagcttcatctttcttttttatttgtttggaactttcagaaataaatgaaagtatgacccaaaaaaaattacttaatgagttttatcaggctgctgtagaaccagttttcttccgatttaataaatgcactgatcgtcttatccgtttgctgggcaaacttggtgatattggaaatagaatccttaaaagctttcatttccttatctttcggatcaccttccgcctgttgcagctgtaacagcactttcatgataggatccagttcgcgcttctttctttcgcgggcgatatacgtagccaccttccagatatctttctctgctacaaaaaattcttttctttctcccgggatgaggatacgttccaccaacccccagttaatgagttcccgcacattcatattggtatttccacgggaaatgttcagttcctccatgatatcatcggcactcaacgggtcgggcattaccagcagtaaagcgtgaatctgggccatcgtacggttaataccccattgggcgcctaatgaaccccaggtttgaataaactgcgcctttgcttccactaaattcatgtaggttattattttatagcgtttgacaatttacaaggccaaatgtatatcaagtttttgaactttcaaaagctaatgaaacattttaccggtgaatgacggggcatacagccgtcttccgggcacaaaaaaaggcgaagtatacactccgccttttcgtatagctattacaattagtttataccagcattgttaccgggttttccaggaaccctttcagggtagccaggaaacgtgcgcctaccgctccgtccacacttctgtgatcgcagctcagggtcagtttcataatgttggctgtttttatctggcctttctccaccaccgcagtttcagtgatattacctaccgccaggatcgctgaatccggtggattgatgatcgccgtgaattcgtcgatacccagcatacccaggttggagatactgaaggtattgccgctgaattcctgtggttgcaactttttgtttttggctttgtcgtacaggcctttcgcatcagtggcaatctggctgagtgttttctgatctgcaaagcggattaccggaacaatcaaaccttcttcaatagccaccgcagaaccgatgtgtatatgctggttctgacggataaaatcgcccatccagctgctgttcactgccggatgctgacgcagtgccatggcagaagccttgatcaccatatcgttgaaggaaatcttaacaggggaaatttcgttgatggatttgcgcgcttctatcgccttatccatattcacatctattttcaggtagaagtgaggagcgctaaacttgctttcgctgaggcgtttagcaattacctggcgcattttggtcagcggaatatctgtgaagccttcctggccggcaggtacaaacgccggagcagcaggcgctgcgccgctttgtgctgccggagccgccttggctgcaggaacatagctatctacgtcttttttgataatacggccaccgtcaccagaaccaggaacctggctgatatcgatgcctttttcctctgccagcttcttagccagcggagatgctttcacacggccatcggcgctggtggttgcagcaggagccggagttgccgccggagcagcagtcgtgccattctgtgatggggcagcagcaggtgcggatggagctgatgctgccggggcagcgccttcagcagccaggatcgcatctacattagtcccctgtttgcccacaatggctataatgccgtttattttggccgcttcgccttccttcacacctatatataataaggtaccgtcggcataacccattacttccatggtcgctttatccgtttccacttcagccagtacatcgtcattcttcacaacgtcgcctacctttttgttccaggcaactattttaccttctgtcatagtatcgctcaggagcggcatacggataacagtagcatttttcagcgcttcttttaatgcagcgtcatcagccggtgcagcagcagccggagcagcctgtggtgcaggtgcagcaggtgcagcattagcggcaggcgccggggcagcagcagctgttttaccttcaccttccagcagggaagtgtaatcttctccgggtttacctacaatggcaatgatcccgtttacctttgctgcctttcctttttcaacacctatataaaggagggttccttctacgtaacccatcacttccatagtggctttatccgtttccacttcagcaattacatcgtctgcctttactgtatcgcccacctttttatgccattccgcaatcaccccttccgtcatcgtatcactcaaaaggggcattctgataacttctgccatagtgctttattcaaaattttgttcaaacctacatgtttttgcgcaaaaacgcaaagaaggaattgtaaactgtttaaaaatgtctgtctatcgttaatatttaatcagcgcaatcacgctagaagtctaactccatgttcagccggtctttcaactctttcaccagcgggtatttttccgccatctgctggaattgctcccggctggaaagcggcgccggacctatatcctgggtctgctgactctcatccagctgcagggtgagcacaatggccggattgttaaatttcttcttcagaaactcagcaatcacgagcttttcttcttccataaaccggaattgcacaatgttccggctcacaattcccacctccatagtgcccagcagtttcagttgcgccagctgcaaattgcttaccaccgtcattttgttggcctgccggtacagatcaataaattcgtcccagtacacatggatcgctcccatcgtaagcggggtcgactgcacatgggtggttccctgctgtttggcagccatcgcttctttcatggcagccagccctgttagtttgctggccggagcagcagcggttgtaccagctgcggaggtgccgccggccgcaggtgtgacggtggcaggtgcgggcgttgcagatacagggctggttgccggctgactggccacaggcgccgttgccggttcgtgggtagcagttgaatgcccattggaaggtattggctgtgcaggagcaacgaataccggtgtgggcggtggcgcaggtgctgccacaggggccgctgctgtcacaggaaccgctacgggagccgtttgctgcggagcagactgaaccggcgtatctaccgttaaacgtggtcccggcactatgccgatactctccgtagtagccggattcccggtaatggttttagcagttaccggctgggctacaggggcccgcaacttctgcgggggagaaccatcagctaccagctttttttttgacacttccccgttactgtcatcactgaccagggttactgcctgttgcagaaaacatagcttgatcagcgccatctccacatgcagccgcttgttacgcgccatgcggtagttgatctccgtttcattcagcaggtgaagggcagtgatcaggtaagcaggactcacctggcccgacaactgtttatatcgttctttcaggttaccggaaacctccaccaggtgaagggccttgtcttctttacataacagcaggttacgcaaaaattccgcccacccgttcaggaaattatccccttcaaaacctttctgtaaaatttcatcaaatatcagcagggcattggctacgtcctgttgaagcacagacgccattacccggaaaaaataatcgtaatcaagaatattcaggtgctccagcgtattctggtaagtaagatgcccgctcgtaaagctcacaatcttatccagcgtactcagggaatcacgcatacagccatctgttttctgcgctaccaggtgcagggcatctgtttcagcctggatatgctccttgttacatatctcctgcaaatggtctaccgtgtcctgtatggtaatacgtttgaagtcgaagatctggcaacggctcaggatcgttggtaatattttatgcttctccgtagtggccaggataaaaatcgcataggatggcggctcctccagggtcttcaggaaagcattgaaagctgaggaactaagcatgtgtacctcatctattatatagatcttgtattttcccgcctgtggcgcaaaacgcacctgctccaccagggtacggatatcatctaccgagttgttggaagcagcatccagctcatgaatgttgaaggaactgccctcattaaacgacttgcaggaatgacactcattacaggcttccccatccggctgcagattttcgcagttaatggttttggccaggatacgcgcacaggtggttttccctactccgcgaggcccgcaaaacaggaaggcatgcgccagctggttattgcggatggcatttttgagagtggtggtaatatgtgcctgtcctactacagttgaaaagttctgtggacggtatttacgggctgatacgataaaattctccatatgactgctacgctttcgcgagcgccgaaaatacgcacaaattcagtaagagaaaaatgcacaacaggaacagcgcttcaaacggggtacgctcccggttctaaggttaaaataaattccagatatgatttttttagtaatatgattccgttgttgaaatgttccatcatcgctgaactgatttcatgtaactcctggatagccacatagtcggggatcatatcctgcataaaagtgcaatcatgctccctgaatcttttcagcttttcctccatcccttcgggaaaactcccgaacaacgcaccctgctgaatgttttccgtcatcatccggaaaccccagcactcggccgacagctcatcaaaaagcgccggcagcgattccatatcctgttcgccggaattaaacaacaggctgatacaatgaatgatccggatcacctgctcattcaactgttggccggtttgctgatactgcaggatctgggtgtatttctctttaagcagggccgccttagccggactttgctgcatggcaacggtataatgataccggaaggcctgctgatcatgacactgcagccacgcctcttcggacgtaacctgcgcagataacatccgggccagctgctttgcccgcgcggcactgtatttctgtccgtcaaattcaaaataactggtctgaaactgcccgctgctgatagcctgcaacgtttccgcatcctgacggtcacggtaaaaagcccgcatcctcataataatatcaggatgataaagcgcctgtaaactgccggcggttatttcctccggtggcaacagccgggtaaactcctcactaatgccgcagaatggccggttatcataataatcattaaatgctttcggatattcgtataaccggtgccgttgcgaaagctcttcaatgtaggcggcaggagtgatctccgtaaatgtttcgtcactgttatgtaccgtgaaattatatatcagcgaagtcatgtgctgctgcacattttccggctcattaaacaggttccaggcactcaggctgaccggcttacaggaaacattcgccgctaaataatgcgcctcccgcgcttccctggaaagatgcgaagtccactgctcccgcagctgcacccggctcttcagaaaagtatggaaataattgtcggtgataaccggtaatccggcagcatccactgtgagatggttttgtgaagcatagtaacggatcatggcccgctgcgccgtaaaaatattggcaaaccgcagcgttctttctgcaagatccggtaccttatgaaaacaatggtccaggcagtatccgcccatttccagccgccgtaaaccgctgatagctgtttctgtactggtaagactcacagctactgtatctgcatgatattccatctccctgcttaattccaggtattgccggttaatgatcgcatatatcttccgcaatacatactgcattccgttcagtatcctcgtagtaatatgcgcaaagaaacttaacaggctgctgccactgctccagcgggcctctatttcatcccaccgttcattttcatatagcatattatacaacatcttattcaatgcatagatgtagctgcccagtttcatactacgctgcgagaaatgtgcaaactcatacgccagcaacatcttaaattcgctcacgtttacactgttaattaaccccaaacctatttcgaggtttttccccaccggccagaataaactcagaaaactggaatgatagaataccgtagtatgcatgtccggcacaataaatactttcttcggaaaactgatgcgcgtgtccttcaccagctgcgtaataaaatcaaataaacggggatgatgatcccggaagatctgcatacggtaagggttacccgcagaacgtttgttgaaaagaaatttaatgagaaaaaacaataccatcccacccagtaaaatgaaactgagtccgatgatgccggtgctccaggccggataagcgcggaataacataatccctcccgacacacaggccacagccagcacaacggttgccaatagcagtaccacgtagagaataaagaacaacaccacgcagctgacggctttcgttatctgttgcctgaatagtaacgtgggctgaataagtgccagatccgcgttatcagggcactcagggtataagttggtcataacaaaacatcaggttagatacgattgtaacagcaaaagagatttaaatgttacataatattcataaacttatatactcccccaatgctcccatatattcatatgagagatgtatataccccgctccggcggattattttttatgccaggatcggatgccttttatatggagccgagcggtcaaataaatagcgataggtggcgagcctgcgggttggcgtagcaccaagcccctcggccacattctgcattctcggattaaaatcaccaatccactgcatttcataatcttcataatgagacatgccgctctgaattaatttcgccccttctacaatcatataagcatccacgcccttcccctggaattcaggaattataccaaatataattcccaccatctttttgcagtaaccggtttgctttaaccacaggaacttcagcttttgtaacaagccaaatttcccgttcatatgttttatatactggttcagatccggtaaattcagccagatggcaataggatcgtcgttgtgataaacgaaccacgctatcttttcgtccatcaacggcttcatctgcttaaacagcgccagcacctgcgctttccccatttcctttccacccatgtgctgcgcccatgccttgttatacacaatgctgaatgcctcggcaaaccgcggcagatcattcttccggatatgcaccgccctgaaagccggatcagcttcaatagctgcatgccggataaagaatttcggcagcagctggtcactaaccctcattccataacaaagttggtggaagaaaagttgaaaaccatactgctcaaataaacggatgtaatagggagggttgaaattcatgcagtataatggctcatgaaacccttctgtaagcaatccccaccagttattgcgctccccgaaattaataggaccatccattgctcccatgcctttttcctgcagccattgtttggccgtatcaaaaagcaggttggctgcttcctgttgatctatacaatcaaagaaacccacaccgcctaccaggcactcatctccttttgtcttatatttcttgttagtaaaagccgcaatcctgccggctaaccggcctttgtcatcttttaaaatccatctgatacactccccatgacggaatgccttgttcttttcaggatcgaaaacagtattaatatctttatccagcggccttatccaaccaggtacatttttatttaaattcacatgcacgtcgataaattgccgggcggtttgttcattatttacaataatcagctgcattgaaaccatttgtacaaatgtaataaaaatgcattggcattattttttctctttccttcgatatgaaaagaacttatgtttatcccgccatactcctgttgctcatcgtggtatttaccctgggctattgtcagcaacaacggcaagtgcgcaaagtgctgtccgaaaatcagcgcctgtggaacgaaaaccgtgatctgcgtaaaagtctggatcaatccggggcagtttcccggcaaataaccgatcaccaggaactccgccaaagggtggccggccagtttattgaacgcagggcttattaccggcgaaactggcaacagttcattgcggttactgccggcgattaccgcacagggctgctgggagggatcaaagacctggatattatcgtaagaaatcaaacagaatacccgctggataatgtagtagtcagcgtttcctacatgcgcaacaacaacgaagtttttaaaacagaacggtataccatcagtaatattccggagaaaggtacccgcagcattgcagcctccaacagccgcaaaggcagcaaagtagcggtaaaactgatcagcattaccagccagccaatgaacttctgctgggctgccgataaacctgcccccgccggcaatcccgatccgttcgaatgcgtaccatccgttaaaaatacaccggcgccaccggcacaggataatcagtaacttcgtcgcatgatccggctaatacccaccaccatcgctaatgaagcgaccagggatttatatgaagaagcatttcccgaagaggaaagaagaccctggaaccagcaggtgcagctggtcgcatccgggaaactgcagctattgcatattcaccgcgaagacgcatttgccggatttattttctactggaatcttcctgattttagctttatagaacattttgctattcatcccggtacaaggggaggaggcgccggtacgcaggtaatgcagctgatggaagcgcaactgaacggaattgtactggaagtggaaccgcctgtaacggaacaggctatacgtagaattaaattttatgaacgactcggctaccaggcgtttgctgaatcctatcaccagcctccatatcatccgcactatccgccgctggaactgcgcctgatgcagaaaggactagcgcccgctgctgccatgtttccaaatataaaggaacagctgtataaatacgtttataacaaataaaaaaagtacgaatgatatacaaggcattaatgatgtaatctcacaaacatctttgccgctgttatcattcgtactttcgttatgtcaaaagaggtttatcctacacgtgaaggacgttccccctgttgtctgggttgctcctgttgccgttgctgttgttgttgctgctgttgctgttctctttgtattctttgctgttgttgctgctgctgttgttgctgttgtctctgttgctgttgttgctgtaccctctgctgttgttgctgttgctccctttgaaccctttgttgctgttgttgctgctgttgctgttgttgttgctgagccctctgctgttgttgctgttgctccctttgtaccctttgctgttgttgttgttgctgctgttgctgttgctgctgaatcctctgttgttgttgctgttggtcccgctgtactctctgttgctgttgttgttgttgctgctgttgaactctctgttgttgctgtaactgctgttgctgttgttgttgctggatcctttgctgttgctgttgttcagcagttctgtctggtgttactctcgatggcctgttaaagttacccggggtattgttattacccggattcgcattattagccggatttgccggctgggtagtagttccctgccttactcttcctccgttgttatatggaggtatatttccggtattgttatttccaggctgattcgcttctccgggacgtacccggttaccaccattgttattattattacccggttgagtagtattgcccggtgtaacacggcccggacgattgctgttgttattatctactgcctgcaccggtcttgtacggtctacttcacgtcctctctggatagctgcggcatccgggcggtatatgcgcaactggttattctctagtcttcccccggttcccggtctgttggtattttccactctcactggtcgtactgcctggccggaataccgttgtacttcgttggcactcggaccggtatatactcttcttcctccgtaattattagtgttgttgataacagtggtgttgttaatgatcgtaacgttcctgctgttattaacgtagtagttgttgatccgcggactgttaatgtactgtcttggtacaaatgcccagtaatcagccggtgcattataagaatattgcggactcattggcgcccatccataatagtcaccaccggttctccagctaacccatgccggaccccagtcgtaacccggtacccacatccagccctggaaatcgtcatataaccagcgaccgtagtggaaggctgcccaaccccacgcgtaatcagatacccaggtccagccatagtcagtgtatacccagtgcccgtttgtatagtaaggtctgaaatcacggcccgcattagggatccacaccctgtcgtatccggggtaacttacccagcggccgtaaggactcaattcatcataaaaagaaatcgatccgctcacctgcacctgcggtccgccggagtaggatgagccatattgatcatcatatccgggtgcatacgttgatgcacaactgctgatgaatgaacctataaataaaagtgatattcctgtgtgttttaataaactgttcataactcctgttttttagtcctgataggtattgttgtttgtaagactctggagatgtaatgaatgctgcgtaaaattgtgtttatatcgacaagcattttttaatggtctgtgaataaaagtatagaaggcggaatcattttaaattgttaaaggattatgttaaaatttttataacgctttgctgcagttacagcgtcatatatatcattagacaaaaatggttccaatttcgcaaccgctgtaagagcttgcattacagccggtaacagaagcatatgcggaataataaaacattcctgtaatattgcaacagctcacttaatcaaagatggcttcctttttcagtattcatcatattttctttaccacactgggatatccggtcagttatgtggagtttataggcacggtcaccggcttgttatgcgtatggctggccgcaagagatcatatccttacctggccggtggggttggtcaacgtgagttgcttctttgtattgttctggcaattgcaattgtatgcagatatgttcctgcaggtatacttctttgccaccggggtttatggatggctcttctggtacaggaagcaaccggaaaatgaacccgtgtatgcattgcagccccgtcatcgctggcggctgggaatggccgccttgctgttgtcggcagctaccggctatgttatcagccagctgcacctgtggtggcctcacgtatttgaacatcctgcagcatggccctacaccgactcgctggtggcggttttaagtgtgatcgccaatatcctgctggctaaaaggatctgggaaaactggctgctatgggtaaccgtagatgcaatagctacctatatttattttcagaaagatgtaaagtttcttggaatagaatactttattttgctcatcattgccgccatgggactggcaaaatggttgaaaacatataaacaacaacttaccaataaataaccctatgcttacttttaaacaaaaaatccgtcgtatagcccttacatttatagccatttttgtattgatgttcctctgcaggatcgggtatggttacctctataaaggccgccagcaggaagcatccggtgaaaatgattttttatccggtgtaatgaggcaacagaaaaattatgcatctgaaaaaataaaagcctttaacccgcagaacaatgcaccggatatggtgtccggcaatcagaagtatgaaaaagtagccaatgtacgggcgaaatcatcgcagttttcggaagatgaaaaactgctgcatggcaccattaaaaaatttgatgccattgtacagtacgagcagcaatccggcaacagcgggaaccgccagatacaactgctgataggcgtttcgcctcaaaagttcgattcgttttacaaggcaacacaagggatcggagaaataaaatctaccgaaataaccaaaacagataaaacaagcgaataccgtaaactcaatgcccaaaaggcttccctcgaaaattcactggcttattttaatgaactgaaaaagaaagacggcaaaatagaagactttatccagctgcataaccagatctatgaagtagaaaaggaactgcagggcctgggcgtggaactcggcaacttcgcagaagaaaatgaattttgtaccgtgcagttctctatgtatgaaggcgccgcggttaaaggcattgcttttattacccgtgtgaaagtggcgctggaatggactatcaagtactatgcagtgctggtagcggccattttctttgccgcaggaagcgcctggtttttattgaagctgtgggagctggtgaatggctggatcctgtctgctaaaaagaattaaaataaaagaagctgtctcataaataaatgaggcagctttttcattttaggctttaaggatggttttatccacaatttgcagttgaaaaaaagggaagttgtaagtgtttacgcaccagaagttattgtgt

SEQ ID NO: 14 - DNA, 243886 bp, Chitinophaga pinensis
  source 1..243886: mol_type = genomic DNA
gcttgctaaagcaagctgacattaactatttattctcttaaaaaacacctgatcatcataatgattattaggccatcttttggctaaaacaaagaagctgtctcaattaattatgagacagcttcttaattattattaagaaaatctaaaaatcaggaaaaaatccaaaagtaaaaatccagctaatcagtataatcagcgtaatcctgagccaagacaaaatccgctctgagcctctgcccattcgaggccacccgccagttgccggttgctgaattcgatgtggattacacggcggttacgaccgttgctgctgcgtccggaggcatgcatcagtaaaggctgcatgatcatcacgctgcctttgtttacgcggcagctaacatccggtgtttcgttcaggttaatactgtctgcccggtaaacacctttgacgtgtgagcctggcagtacttttaatgcgccgttctgttcatctgtatcgtcgaggtgaatgcggagggtatagatgctttccaggatgtctgttggcggctgtactgcgaattggccgggtttcacggtccaggggccgtagccggctacggagagcttctctgttacggaaatagtgaggtcctggtgccaggcaacaaaccagttggattgcccgggcttatcaaaataaatggatttaacaggcacatgctgttcgccaaacagctccctgataatttgcctgatacctggtgtaaatatcagcggggtgatggcaggaacctcctgcaaaaaacaacggatggcaaagagatcgttggttttccggaatagaggaccggtaggatccacgctgtcgatcaaagcaatcatttccccgatggcactttccgaaaatataccgggaatcaccgtatatccgtccctgcttaattccagcctgtgttgtgtgatggcgtcgttcgtcatgtttcaattattcttttgcaaattacgcgaattttgtcttggctcaggattacgctgattatactgattacctggattttgtttttttggattttataaaggattaagggagatagcagcggatatattcgctgctatctcccttaattattattttaagaaaatctaaaaatccaaaaaaaatccaaaagtaaaaatccagctaatcagtataatcagcgtaatcctgagccaagacaaaatccgcgttatttaatcagcgtaatactccctttaaactcgaatttctcgccgccttcgcacacggtctgcatggagtaaatataagtgcccattggcgcttccttgttgccgctacggccgtcccaaccggaggaaggcgagttgatagcgaagtgggtgttctcaaatacaagggtgccccagcggtcgtagatgcgcagccactcaatttcttttacaccttttccttttggatagatgcgttcatttcggccatcatgattgggggtgaaggcgtttggcataaaaacggcgccctggttgcagagaatgtgcagcactacttcgtcggcagctttgcagccatatacgttttctacttctacccggtattttgtcgtgaaatcaggcagtgccaggacccgtgcacaggtggcgcaatccaggaattccgcaggtgtccagcgccagcggattacatcattgctggcgtgggctgccaggtatacagggatgcccgccataatttcacgatctacgccagcatttacggttggggcaggatttacttttacggtaagggaagctttatcggagaaacaattgtctttgtcgaacccggttacctcatacacgtattgccccctggcgttgagcgtggctacaggcgcaggggaggagggcttgtcgattccggtgccggtccacgtataataatccgtgcccgatacctgtagcggcaatttatcaccgagacataaaacagtatcaggcgtagcctgtatcttaaagggctgtactacgcgtattgctacttcatcgttattgctacagccgttgttgtcggttacctttacctggtaggtggtggttgccaatggtgcggccgtaggggtagcgatggtgggatcgtttagtccggtggtaggggtccattcataggtgccgccgccgccggcgtgtaatacggtggtgttaccaagacaaataaaatctgcgggggcgctggcattgacgtctggtaagggtaaaatattcagtggatgtattacttcgtctgcgcagccgtctttgctggtaacggtgagctttacctgcaccaggccgggctgcgaataagacaaggccgctggttgctgcacatcactggtggtattattacccaaatcccagctccaggtaacgtcattcgttttggtaacgctgccactgaaggtaaccggcacgtccttgcacgctttatcgggcgcgctgatggcagctaacggcttcgggtatacgtttaccggtactgttacggtttgtgtgcaaccgtatttagtggtggccgtcatgccgaagatgtattcgccggttttgtccaggtgaaataccggtgtggtagtattgatatccgttggagtgagtgcggcatcataggtccaggtataagctggtgtaatacccagttcatctgcagaatagctattaaacgcaggcgcaaaagtaagcgttcctgcatcgcatatttttgcgggagaaggattcagcttaatatccagctgatctattaccaccgggtgatccaggaaggcgctgcctttacaaccggcatcatctttcagtaatagccgtggtttataaatgccaggttcggtgaaatgatgttttatttcgagcgacgtggtttgttcaacgttaccatccgtaaagtcccagctgaaggtagttgcattttccggcttgatggtaaaggtgatctctttttccaggcaaccgccgtcggcgctggttgcgatggtggcgtacggcccggtaacgatcactatctcgctgtattcatcttcagtgccggcttctccgtatacctttaattttacggtataatggccggattctgtgtaggtatgtacgggatcactttgattagaggtaccgccatcaccaaaatcccaggagctgttcagatagttgagggaccggttactaaaacggaatatcataggagcgcattttccgccgtttacaaattctgatgtgtaaacaaaacttgcggcaacagatgccactttgatatttttggttacctcgtccgtacagccgttattgtcatttacttttatagttacaggatatgttcctttattgggataattatgggttacatcctgcatggcattggaagtattattgtctccaaaattccatgttaccatagagatattgccacccacttcactcgaggtgttgcggaaaaatacgtctgtaccgggttttactatatagttatctgcttcaaaatcggctatggggccattcacctggatatacctgccatcaaatgtattcctgcaaccttctttatccgtaatagtaacggagggctggtaatagccggatttgttataggtatgtttgaagggaggggttgtaaacgtctgcggagtgcttccgtccctgaagtcccattcccattttacaattccactgctgttactgacatttgaattatcagtaaagctcatttcggtgccgcggcaggaatagggaacgggaaaattataatctgcaacagcgccgcgtacgtttacatcaatcgaattactggtgtctacacagccgagatcattgataccaattacccttacgcgatatttaccgggttccatgatgtaataaccaaacgactgggaagaattattgtgaaaattgctaagatcgtttaattgccagtagtaaccagctacatcataataggaaggatcagctttagtaatggtggtggtcagcgcctcgccggcgcataatatggttttatcagtagtgatttcaatcggggatttagtatatatacgcgccattacttctttaaaagtggtgcaattgcccgctgttgtagtaagtttaataatataggtgccggttttttggtaatagtgtgagatcttattgctgctcaccgtataagcagtatcctgcccgtcgccccattcccatttccagccggtggcgcccagagaaccatcggtcacggtgattacattccggttcgcacaatccacatcgtctatcgtaaaccgcgggaagggatcaacagtagtgatgtatgcctttttggtaagcgtagcagggcaaccgccgttccatacggtaagtgttacatcatatgcaccgggttcactgtattcatgttgagtgcttttatggccatctcctgcgccgtctccaaattcccagaaccaggcatcggcaacatcagatttgtcgttaaaggtaaccatagaattcccacaaacgataggtgcattgggagaactgaaatctaccactggttttttaaataccctgacgtcgttgtaaacttttattctgcctgtacagcctgccgtggtggtatattgaagatatgtttcgaagatgccggattttttaaaaatgtggtttggtgtggcttcatgggacaccgggctgccatccccaaaatcccattcatattttgtaatgggatcattatagttgccaatagcggtaaagccggacgacatgccttcgcaaccactgtcattataggcgatggcagatatttttgtagtataaaccgtcaccgcactgtagctgttcatagcgcaaccgttgctgctggtgccggtcaacacaatttggtaagcgccttctgcctggtaaatatgagaagggttttgttcggtggaactttgtccgtccccaaaatcccatttccagctgctggcgccggttaaattgtctttgaatttgacggtagccggtaccgtgcaggtcggaggactttctatcagcagattccctgtgggagcgggattaataaccgcttttttctctactacttctttacagcttccatagttggcggttagccgtaccgtaatagtgccggcactgccatagggcatataggtggcgttgtcgaagttgccgtaagcgttttgtccattaaattcccataaggtgctgtttggagtaaccccgctaaaactggcattaaaggtggcatattcgttagaacacataagcgccggaacaataatgtcggtaccatagttggcgacgttgatatcgtttacttcttttgtatcactgcatcctctttcattggtaaccgtgagcttaatgctgtgctgccctttgttgaaagtatgtttggcgggatctttttgagtactgctgccaccatcatcaaattcccatttatacgaaagggtccccggacccgtagaagtgtttttaaagaacacatcggccggaccactgcacaaggttttttctgttacagtaaaatcagcatttatagcaggggctacatctactgccttatccagtactttgaaattcgtgcagccatagctgtcagttacactgagtactacactgtaaattcctggtttgctgtaaatgtgatcaactacgccgctgccgttctgtaaaacttcgccgtcgccaaaatcccagctgaagttttgcagggtaccttccgctgtggatttatccgtgaacgtagtcgtaaacggtacgcatcctttgccggaagacacactgaagtttaccgccggctttgcccttactgcgatatagtttgttttaacggctgttttcgtactgccatctccgaaggttacttttagtgatacagtatattttcctgtttttacataggtggcgccgggattttttttggtagaagtagttccattcccgaagtcccacagccaggcggtggggttaccggtagacaggtcggtgaaactggtaatgagcgattcacaatcgctggtggcggaagcagaaaagtcggcgttttgttgcgccaacgcacataaactgataacaaaacatagtacaagggatacaacaaatttgcatcggacagggaaacggtacatcggacgtataggtataagccctaaaaataggcttttccgcggatatttgctttgcctggcgtgtcttgaatattatgttttcgctatacgattaatgcttaattttaaaggtcttaaaagcagcgttttatgtcacatttgtttagccctctgcaattgagggaagttacgttccggaacaggataacggtgtcgcctatgtgtgaatattcttctaccgatggatttgccaccaactggcacctggtgcatcttggaagccgggcagtgggtggcgcgggactggtgctcacggaggccgcagccgtatcccccgaaggccgtatttccattcacgacctgggtatctggaaagatgagcacatacctatgctgcaggaaatcacctcatttatttccgcgcagggcgccgttcctggtattcagctggcgcatgccggcaggaaagccagcacactaagaccgtgggaaggcagccgcgccctgcccgcagaagacggtgggtggcaggtggtagcgcccagcgccattcctttcaacgacgtatatcctatgccggtagcactcacggaaacaggcatacgtaaagtgaaagatgattttaaggccgccgctgtccgggcacagaaggccggcttccaggtaatagaaatacacggtgcgcatggttatctcctgcacaactttttatctccccttagtaatcaacgtacagatgaatatggaggcagttttgaaaacaggatacggttgctggtagaaacaatagaaaccgtacgggaagtgtggccggagcaatatcctttgttgttgcgtatttcggctaccgactgggcggaaggtggatggaacccggaggaagctgtaaagctggcggcaattgtaaaagggaagggggtagacctggtagattgttcttccggcggactggccgcacatcagcaaattaaagtgggacctttataccagactccttttgcagagaaaatcaggaaggaagccggtgttgccaccggtgcagtaggattaattaccacagcagaagaagcagaatctattattgccgaggggcgtgcagatatggtattgatggcgcgtgaaatgctgcgtgatccatatttcccgttgagggcggcccatgaactgggggctgagatcaaatggccggtgcaatacgaacgggcaaaacgaagaaaatagcagtcagccgttagcaatttctgctaacggctaaccaccaaaaaactatttcagtatcgcttcaatagcgtccagttcttcttttgtaaaggcggtatttttcagcgtatccaggttgttgtccagctgagcaacagaactggcgccgatcaatacggtggtaatccgtttgtctttcaggatccaggccagcgccatctgggcgagggactggccgcgttgttgcgccaatacattcagctttttaactttctcaattctttcaggcgttacttcaccttcctgcagaaatcctgttggtttgctggcgcgtgagccggccgggataccattcaggtaacggtctgtcagtaatccctgtgccaggggagagaagggaatgcaacccacgccgttggcttccagtacatccaacagtccgccttctatccagcgttcaaacatactgtatttgggctgatgtatgaggcagggcgtaccaagcgattttaatatctctacagctacttttgtttgctcggcagtatagttggaaagtcccacatacagcgccttgccctgttgcacaatgctatgcagcgctcccattgtttcctcaacaggggtagccggatccgggcgatgagaataaaaaatgtccacatattcgagctgcatgcggcgtaaactctggtccaggctggaaacaaggtatttacgggatccccagtcgccataaggaccaggccacatggtataacctgctttagtagaaatgatcagttcatcccgcaggtgcccggtgaaatcctgtttcaatatcctgccgaaattctcctccgcactaccaggtaaaggcccgtagttattggcgaggtcaaaatgagtgatacccttatcaaaagcgttatgaataatactgcgtccgttctcaaaattatcaacagagccgaaattgtgccataaacccagtgatacggcaggcagctgtaaaccgctcttaccgcacctgttgtaggtcatattgttatacctgtctgcagcgggtgtgtaatgcatggaattttaattttagggagacaagatagaaaaataaagcggattttgtcttggctcaggattacgctgattttactgattacctggattttattcttttggattttataaaggattaagggagatagaagcgggtattcgctcttatctcccttaactattattatacgaaaatctaaaaaatcaaaaaaaatcaaaaagtaaaaatccaggtaatcagtaaaatcagcgtaatcctgagccaagacaacatccgctttagctcagttcctccaccggtacgcgcggagcagtttcctgcttcagcttattgctttccttcagtttggctggaaccgggcgtatttcccagacgattcccaggaaacccagtgttttgatcacataataggtgatatcaaattcccaccagtaaaagccctgtctggctgcactctggtagtagtggtggttgttatgccagccttctcccagggtgatcagcgccaggatagcactgttgcgggactcatccccggtataatatctcttattaccaattttgtgcataagagagttaatggtaaaagtaccatgatataacagtacggtgctcaggaaaaacccgatcagcaaagtagataacccggcggaccagtcgaaccaaccagtaccatttactttattgcccacaaaatacactgctattgccagtaccactgccggtatcatatgccatttattcagccacaacaattcttttgctttgtggtccttgatcaggtcgaaacgggtgggcttgtattccgggcccatgatccagccgatatgcgcgtaccagaatccgtaaacattcgctgaatgcggatcttccggggtatcgctgtgtttgtggtgaatacggtgattggctgaccaccataaggcgcccttctgtaaactgctttgcgcacctcccgccaggataaactggaagaaccgcgacgttttaaatgcacggtgcgagaaataacggtgataaccagccgttacaaaaaacatacgtactacatacagtacaccgcacaatatccagtcaaaagctgttgtaccggtgaaaaatgccagtaagggcaccgcgtgaatgcccatgaagtctgcctggtgccaccagttaggtggctgtctttcttgcttgatcgccttattcattccacaaagataatttccgtcttttattaaataaatgatttaaatcatttggacaaagttaagtgcttttccccggtttttgcgcgcctatattccggcgaacattttacaaccggatgtgttagagagaaacgtagtactatcctttcatcacgttaaagtaattattatgtcacaattcatttcggctatcaggaacaatgtgaagtattggtggttgtacctgctcaacgggatcatattcctcatagcaggttgtgttgttttcgccaatcccttcagcagctacgtattgctcagtatattcttcagtgtcacccttttcgtgacagggatctttgaaatagcttttgcagccggcaaccgcagggggcaccacgggtggggatggtcgctggcctcaggtatcatagatgtggtgataggctttatcctgatgctgtatccatcggtaagtatggctgtgatcccgcttttcctggctttctggtttttgttcaaaggtatcagtctcattggattctctatccagcttcaaacagataaggtgcctaactggggctggctgctggtgggaggaatcgggcttattattatcgctatctttattctcgataaccccgcactcggtgtggctactgtactcggactgatggccgctgccttctggggaaccggtatcctcagcattatcttcgctttccgtctcaaacatgttaaaaaagaattaaaagaacacggcctttaaaaaaagatacgccgtagaagctgttactgcgaaccacaaagtaattcaccactttgccgttcgctgtaacagctttatactgtcggcattttctgtatattcggtgctgctaaatctattctcttccgatgaaaatcaacagaatctatgctatcgcgtccttgttattatgcaccgggatgcagcaggtaatgggccagacagtatctaaatatgatgcgcatgaggctttttccccgctattctatcctgctcccggtaacgaataccgcagtgcaggcggacaaccaggtccgaaatactggcagaacgcagcagattataaactggccgttacactcgacacggcgcaacatcgtataagcggctccgtagtcattacctataaaaataacagcccggaccaactgccctttttatggctgcagctggaccagaacatttaccgggaagattcccgcggcagcgctaccgtagcggcttccggcgaacgatttgctaaccggagcttcacacagggctttgagttgaaaagcgtaaacgtagttgccaacggcaaatctgcctccgccaattacctggtaaatgatacccgtatgcaggtgaagctggcagatgcccttaaaacaggcgcctccgtgcaactgaaaatagattacgcctataccatcccggaatatgggaccgaccgtaccggccgcctgcgcaccgccaacggatggatctacgaaatagcacagtggtacccacgtatggccgtgtatgacgatgtactcggatggaataatataccctacctgggcgcgtccgagttttatcttgaatacggcaacttcgattataccatcacagctcccgccagcctgctgataggaggctccgggcaactgctgaatgaagcgcaggtgctgtcgccgaaggaaatgagccggctggccaaagcgcgcaacagcgatgaaaccgtgtatatccgcgacagtgcagatgtaaaaaacaataccgccaaaggaaaccgtacctggcatttcgtatgtaaaaatacccgtgacgtagcctggggcgcctccgcggcgttcatctgggacgccgcgcgcattaacctgcccggtggcaaaaaggcactggcgcaatcactttacccggtagaagttgccagcaaaaatggctggggcagatccaccgaatatgtgaaagggtgtatcgaacactactcagataaatggtacgtttatacttacccggtagccaccaacgtagcaggtattgtaggtggaatggaatatcccggtattgttttctgtaactggaagtccaccaagggcggcctctggggcgttacagaccacgagttcggacacaactggttccccatgatcgtgggctccaacgaacgtaaatacgcctggatggatgaaggcttcaacaccttcattaacggtatttccactaaaaatttcaacaacggagaatatgctgctcgtcaaagtatgcagagagcagcccccatgctgttttccgccaatgcggaagccattatgaataccccggatgttatcggtctcaattacaatggcatcgcggcttattataaacccgcagcaggactgaatcttctcaggaatgaaatcctgggtccggaacgtttcgattatgcattccgggaatacattaagcgctgggcatttaaacaccctacaccgtgggactttttcagaagtattgaaaacgccgcgggtgaagaccttagctggttctggcgcggctggttttttaatacctggaaactcgaccaggcagtaaaagatgtgaaatatgtaaagaacgatcctgcccagggcgcgctcatcaccattcagaacctggaacaacttcccatgccggtagtgctggcagtaacagatgctaatggtaaaacagataccgttcacctgccggtggaagtatggcaacgcggcaacaactggactttccgctatccttccactactaagcttaccagcgtgatcattgatcccgcaggcaatttccccgatatcaatcctgcaaataacagctggaaagcagacaccggtaaacctgtacccgacggtactacgggaacggctatactaaaaaaatacattgatgccataggcggcgccgataagctgaatagcataaaagacctgttgctggaagaagatggagatattgcaggaacagctattgaacgcagtgtgcaggtgaaacaacccgataaaatgctgcaggtggtaagcgttccggtgaataagttaattgcctataagttgcttatcaatggcaataatgtaagtatggcccgcatggggcaggaggtgccgctttcagcggcggacaaggctatcctgaaggataaaaacagcctgtttcccgaactgcaataccttaaccatgccggcgatgttaagctggaactggcgccgctgaccaccgatgtcaataatgcaagcgcctatgttattggtgtggctacttccaacggggcattgctgcgcaactactacgatgtgaaaacgggcctgaaagtacgcactgtttccctgccgggacaggaaggcaatgaaaaggaaaccactactgattacactgattaccgcaacgtgaatggtgtacaactgccgtttaccattactaccaatacaggcggttatgatgcggtgatgaaagtgaaaaaggcggctattaacagtgggctgggagatgatatatttaaataattgccggcaggccactcccttacaggcggcataaaggtggcatacttgtcttaaagttaatatcttcgcggcagtactaacgtcatgaacgaatgaaacaactccggccggtaatgtttgtgggtacggcttccgatgtaggcaaaagcgtaatcaccgcaggattttgccgtattttcaaacaggatggatatgctcctgcgccttttaaggcccagaatatgtcgctcaacagctacgctacccccgatggactggaaataggccgtgcgcaggctgttcaggcagaagctgccggggtgcaatgccacaccgatatgaaccccgtgttgttgaagcctaccagtgaccgcaacgcgcaactggtgctgcacggcaaaccagctggtaatcagtcggcctgggaatactttatggaagacgataaacgcgcgctctttgaagaagtgaaaggcgcttttgaccgtttgtcgcagcgattcaatcctttggtaatggaaggggcaggcagtatttcagagctgaacctgcgtgcaaaagatatcacgaatatgcggatcgcgctgcatgcaggagcagcggtgtacctgatcgcggatattgaccgcggcggtatttttggcagcgtatatgggactatcgccctgttgccgccggaagaaaaggcgttgatcaaaggaattatcatcaataaattccgtggcgatatccggttgtttgaagacgggcgggcgatgctggaaagcattaccggcgtaccagtaaccggtgtgctgccttactatcacgatattcatattgaagaagaggatgcggtttcattgcagcttaaacagaaacggtttgccgccggtcagataaatatagctatcgtactgctgcggcatatgtccaacttcaccgacttcaatgcgctggaaaaagatgagcgcgtaaatatattttatacagataatccggcagaactgtcggccgcagatattatcatcctgccgggcagtaaaaatacgattgccgacctggtctccatcaggaataacggtaccgctgccgcaataacggaagcgtataaacgaaataaagcagtgatcggtatttgcggtggctaccagatgatgggacagcaggtagcggatcctgatggtgtggaaggccctgccggcagcataccggggcttggaatattgccagttgccactgtgcttacaaaagaaaagatcaccaggcaaagaagtttttattaccgggatcagccgaaagtatgtgaaggatatgaaattcatatgggagataccaccgccgcagtggcttccccgctgaacacgtttacagatggcggcacagacgggtatttcctccggactaactgctggggtacttacctgcatggcatcctcgataacgacactgtgatcaacgatctgctggcgcattgcgggaaacccgcagtagtaaaggagttcgattaccgccggtttaaggaggaacaatataacaaactggcaacacacatccgtgaacatctggacattccggctgtttataaggcactggaattataataatattgcattatgatacaaggacacggtgacgatggttacctgtttgcccaacaggtgaaagctgatttcagctccaacgtatggtatggtggtttacaggaaggattgaaggagcacctgaggaataaagtaacgggtatagatcattacccggacgcaggtggctcaaagctgcaggccatgctcgaaaaccaggaggctctccccgccggcagtatcctggttaccaacggtggcacagaggccatttacctggtggcacaggcatttacaggcgccactaccacggtggtagtgcctactttttcggagtatgcagatgcgtgtaagctgtatgggcaccaggtgctgtacctgcaatgggataagctcacaccgggtaccgtgttcagcagcgacctggtatttatctgcaatcctaacaatcctacagggcaggcattggatgaaacagccctgcaacaactcatcgcccataataagcatacggtgttcatcattgacgaagcctatatacagtttacactaaatgccgctaccatgctgccgttcctgcaccggttaccaaatgtgctggtgctgagatccatgactaaaacctgttgtatcccgggcttacggctggggtatatggcaggaaggaaacaactgctggaccgtgtcagggctttccggatgccatggtcggtgaatagcctggcactggatgccggctattatatcgtggaacacccggagcagtttaccattgcgaccgacagcctgttgcaggaaacttttcatttgtgggagagtatccgtaagatgcccgagtacaaagtatatgcatcgcatacgcattattttttgtttgaaacattaaccggtaccgccgctacattgaaagcatggctgatggagaagtatggcctgctgatccgggatgcttccaatttctacggactggaagccgggcattgccgggttgcctgccgcaatgccgctgacaatcaattactgactactgctttgcgccaatggaccctgtattaaaattcgtattgccgctactgttagggtatatcgccgacctgctgctgggagatccccgcagttggccgcatcctgtgaaagtttatggctggctgatcagccggggcacacgctggctgaacaggggaggcgcccggttctggaagggggccttgctcacggttaccttgtgcgtagcagtatatataagtttttattttacgcttatagtactatcggggtggccggtagtgtactatggattcagtgcagtgtttgtttttttcgcgctggctaacaaaagcctgctacaggaaggcaaagaagtatttgcagctttacaccacgaaggagtggaggccggccgcaggcggttgtcgtggatagttggaagggataccggtcatctttcacctgatcagatccgcatcgcggtatttgaatcgatgtctgagaacctgagcgatggggtagtagcgccgctgtttttttacgctgtactggggctgcccggcatgatgttgtataaaatgattaataccctggattccatgataggctataagaacaaggaatacctgtattttggacgcttcgctgcgcgcctggatgatgtagccaattttatcccggcccgtatcacggcgctgctgatgatcctcctgtatggcagcagccgtgcctggcattttatgattaaatacggaccggcacacagcagccccaattcaggatatccggaagctgcactggcaggtatcctggattgccgcttcggtggtcccaacctctaccagggagtagtggtaaataaaccttacatcggtgaaaatgaacgcagtattgaacatggagaattcagcaaggtaatgtaccttaatcaggcagttactttcgtgatgatcatcagcattattgcagtaaaatattattttatatggacagcacagcggtaaaccccggacaggaaagaaacgaaaggatcagtattttaagctgtggctggctgggaaagcccctggcactgcacctgcaagccgcaggttattccgtaaaaggagcccgcaccagcatggcaggcgtacaggagctgcaggcccttggcctggaagcgtatacggtggtattgtctgaagacgtgctgaccggccccgatgccttctgggatgccgacatactgatcgtaaatatcccgccgcggaaagaaagaggcaaagatgcacatgtatcagaaatagcgctgttgcgcagttttatagccacaacgcccatcagcaaagttatctttgtgagctccacttctgtatataaagacatcaacggcctggtaacagaagaaaatgaagaaatccctgacacgcccaacgggatggcgctgcgggaagccgaaagcctcctgctggagtcagacgcatttgataccaccgtattgcgcttcggcgggctcattggctacgaccggctgccggatcagcgccggatcatggaaggccggaaagccaacggccagcccatgaatgtaatccaccgcgacgactgcatcggtattatccggcaggtgatagaaaagaagatgtggggagaagtattcaacgcctgcgccagcggacacccgcaacgcagccattattacaaggcagctgcgcaatacctcggcatccagatgccacgcagattacccgccgaagaggaaccctataaaattgtaggttccagtaaactgagaaacgtgctgggatatagttttctgtatgatgatccgctacaggtgtttaataatatcaatgtttaaggtaccaacacctgtccatccgggggcaaaatgagacatagtgcatggggagtgcatggggagtgcattggaagtgcattggaagtgcattggaagtgcattaggagtccatgctgacagcattaataccgcatggtttatccaaggtatacgcaggtttgaagcatggcagaagtatcccggaagtaacacatatataagcattctccatacctccccgccggagggcgcatccccgccttgtaaaaaaaattgtttacatgtgttaaattcactatattgtagtagtacctgctttatgccaacaggaggtaccgctcaactataaaatattattcaacctaaacctgatcaaaaccgtgaatctgctgctccttagccttttgtttgccctggcattatgggcgatgatctccatgtacaggagtcgtaatcgcaaaaaggccgaattgcttttacctgtaagatctgcgagtatcataaaaattcatagttacaagtctttcggtatcattgctaccatccgctttaaatacgacctgacccctcagattggcgaccggttgcatgaagaaggcaatatctaccagatcaccggcgtggtaacgcccgatccggtacaggaacaacccaaagatacctgggattgccgtcttgtaaaaatctaaaaaatggagtatctcaaagtatcttggcttcatcattttgaagacgaaccggtatacctatacagcgagatagattcgcagcgtttcgaaaacaggaaaattgaaatctacccggatggaagcttcggcatcgcctgcagcaattttcatttcggcggcaccgccttatccgatcaggtgatgcccggcctggaagaaatcatggaagacaggcaatttattcctgaactaatttccaaggcagaatttgaactgatctggaatcaatatttttattttttgtcctgacatagctggtccgtggtttgcgtaagttctttagaaaaaagaatcttatgaacgcatttatgattaaaacttccggaggccgcttttacgtaaaaccctcttcagctgaacgctttctggtagacgtagacggagaagaggtaatgatggagaaagacgaagacggatatgtacgtgcaccgggcgctacagacaatggccgtcgtttaaacatgggactgctgaacaacattgcagaccagatcgcggttcagacggcgtaaaaattccacagattggggttacgggtgttcctcaaaacctgtaaggtatttgtcgatatactgcgacttcgttttggatttgtactgcataacaaagcgcggatgttccagcgggacaatcgccctgaaaaatttctccttttcatttaatgcctgcaggaacgcggcattcttccctgtccccatacaatagcatacctcacgactgatattccactgcaattgcgcttttaaactgctcacaataaaaggataggcggcttttgttaaagcggcgctgtcgtagtaattgtaatttatttccttcccgccaggttgaagggaggtaaatccgagcggacaaacagagctgatataaaactgctggtaaaactttttcaccccgccataggcgtctattacatcatatacaaatacagaggagggctcgtgcgttttaagcccggtaatttcaatgccgcacttgtcccacatacgtttagtatccgtaaaaggtacgccggtagatcccgatcccagccggccggggttaatgcccaggatcagttggcgtggctgtttgtcgttataaaattttttatagaactgtgtcatgatatccatgatatcggggccttcccggaaagggttcatcacacgtatacctgcgggcaacttgcccgggaaatgcagctggctgttgaagctaatgatctgatcggcgatagtcattccgcaatttacgccatttgatgatgcctggtaattttttccaggatgtcttcttcgcggtaaggcttcatgatgtaatcatttaaacctgaacgaagatacagctcaatatcatcgtccataacattaccggtaatggcaataatggttacggaggctttcttcttgtcaggtaattcccggatcatattggtcagcatcagtccatcaatgccggggaggtcaatgtcggtcagtacaaaatcgaatgcttcacgatggtatacttccagtgcttcttctgctgaagaaacaatcaggtaagaagcctgcattctgtccagcatcagggccagcagtttctggttgaggatactgtcctctactaccagtaaccggatacccgccggaatagttgcgtttgtagatgtattattcaccgggacaataatttttttggtaacaggtgatggggtcatcagcttatacctgatttcaaaataaaaagtggagccctttcctgcgaggctttccacatgtatctttccgttgtgcaggtcgatgatcttcttggaaatatgtaatcccaatccgcttcccttatgataatggttatttccctgggaaaaggcctcgaaaactaaaggtagttctttatgcgaaatacctacacccgtatcttttacgcttacctgtaataagttgttgtcacgtatatgcgcggttaccgtaataccgcccttttctgtgaacttaatggcattggctaccaggttaatcaacacctgtttcaggcggaaggcatcgcccaccacaattaaagtgctggggaagtagatgtttacctccagcgtgagcgacttcatggctgcctgtatggccagcgtattgcatacttcttcaatagcggtacggggagcaaacttctcttctcttaatatgggttctgcagattccatccgcgtgtagtcgagtacgttattcaccacctgtagcagcatttctgcagagtgacgtatagccgccaccgtttcgggcgttgtatcgcgttccagcaggtgcgtatagccgagcaccgactgtaccggtgtgcgtatttcatgactgatcgtcgctgcaaagtcgcttttctgttgtgcaaacttttcagcctgttgcttggctcttagcaacgccaggtcgtagcggtataaacggacaataccatatataataatcgctgccagtaacaggatgagcggaatctcccagtagttgtgcttatccagcttgtagagggaatgatcgatatcgtgacccaattgcagccgccgcttatcggtttccgccacgatgtcctgtttcaggttcgccatgaggtgaagcaattcagagaacagccgctcgttggcaataacgagggcgtattctttttgcttcaggttattatgactttcggtggcatcttttataaacttattataggcggcctggatctttgacagctgatcttttgaaaaggctttgccatcctttggtgtgtcgtattgaacgattttcacctgctggctggtttgctgtacctgcgatttattgctgatcgcatctttgatgcggcccagtagtttcttgcggccctttgcagtggccgtttccgtagttataatcgtgtcggcctttatgttgggcgccggtattttaatattactcaactgctgcagggggagggggtgggtggcagtgtcccatacctgcgatagctgcagcaatgaatctacgtataggcgtgtctgtaggtacagctgcgacttctttactttatccgccagcagcgcatgcatctgcttttcatttttagcggagctcacggcgctgtccaggtgcgcagtaatgctgctcaactggcccacataagcattcaggtaatgcttgtcgtaagtgagcgtatatacacggaagttattgtctgctgcgtacaacagttgcactgcctggtcaatatgacctacatcagttttagtagctatcaggtctttaacaacaatgcttaactgtgctgactctttttttcttaaagagataatcatgaaaaaggtcatcaaaacaatcaccattatcgttagcacagcataacgtacaaaggtctttttttcgtgggttgtatacattgttacatatgattgggacgtcggcgtggtggcaaaaccgcgacgaaaataatgattttacgttccctaactaatagataatcaatgaaaaactaaaagaataggtatgtattttctgctgagtttcctatgtataattatatttaatacattatatatttttacctattaaaactttcatatgggtgcaaactttaaggttttaatattggtatataaaatatgtattatattttagggagaagataaagttcccttttccttttgtattattgttgctgtaatacctgcttttgatgaaaaactgttttcttaccggtctgttactcctcgtatgcttgccttttgtttttggtcaacctgtttcaccggacccgcattacaaattttacaaaggaaccagtgccctgcaggacaggatcttttacctgtttacattgctggagcgtgtgcctggtgtgacgcagctgataaataaggatagcacccttaccgcattgcgggatgaatacacacagcgtataacccatcccgtgagtagcggtgattttaccgctccgttgcagtttgccggcagcaccatcagtgaagtgagcagcgcttttattactttattacagcaacatccaaaggaaatggaacaactggtaagtgaaatgcgcagcagtggcttattccagttgtatgccgggaaaacggacccggtattgctctcccttgcctggaaggatgccgccgatggcgtgaactatatcctcaatgcctatacgaacggaaaaggactccgctacccggtgattgattcggccacttattacgtgatgtcgcctgcctataaggcaatggtacaacgtgtaattgaagatgcggggaaaaagaagccggacttgtttttccagccgtcgctgcacgtggccctggaattactgacgctgaaccgccgcgatgaagccgtgcgttatgaaccattatctgataccaaccgggatgcgtataaacaaataaagaaaacagactggaacaaatatccgtactccgccatgcttatcctgggcgcaagcccggtagcaaaggaggccatcagtgaaaccggtaaaagccgctgccgtaccggtgcggaattataccgcaaaggaatggcgccctttattattgtatccggtggtcatgtaagaccggtaggtacccaatattccgaagcggtggaaatgaggaaatacctggtacatgaactgaagatccctgcgtcggcggtgatggtagacccttatgcccgccacactaccaccaacgtgcgtaatgccgtgaggatcgtgtggcagagtggcataccggccggtaaaagaatgatgtgcgtgtctgatgtgatgcacgttgcctacgtgaacagcccgatgttcacccaacgttgcaccacagagttaggatatatgcctgcggcagatatcaaacaggccgacctttactttttatcattcctgccggatctgcggtcgctgcaggtaaatgtgtttgatccattggacccctgaaataaaatatctcatccatttattcgtctactttataaacacatccttattatgtctgattcatctatccagcccttatatacaatcctcggtgcaggaggtattattgctaacgaactggcagccgaactggtgcgtcatcagaaacgggtacgcctcgtaagccggtcgccaaaatccattgaaggcatcaccgacctggtgccggccgatattaccgatgccgctcaaacaaagaacgccgtaaaaggtagtgccatcgtatttcttacagccggtctccaatataatatcaaagtatggtctgatgcatggccaaagatcatgaccaatgtaattaatgcctgcaaggaagccggtgcgaagctcattttcttcgacaacgtatattcttacgggttagtaaacggacctatgaaagaagatacgccgtatcatccctccagtaagaaaggaacgatccgtgcggccattgcagcccagttaatgaacgaggtaaaggccggtggccttacggctaccattgcaagggcggccgacttctacggacccggcgcagataaaaccggcttcctgaacctgctgatcatcgataagttccggaagaacagcaatgccatgtggcttggaaaagacgatcagacacatagctatacctttacgccggatgctgccaaaggattgtaccttctttcacaggacgatagttcctggaaccaggtatggcacctgccgaccgccaacccggcgccggacggcaacggatatataaatataattgccacccagatgggggtgaaacctaaatatatgaagctgggcagttttatgctgaccctctcgggattgtttgacactaccatccgggaaatgaaggaaatgctgtaccagagtaactatccttatatcttcgactctacaaagtttgaacaacactttaaggtgaaacctacttcttatgaagaaggaatccgtttaacactggcacataaataatagtctactgatttagtaggaaaataaatttggaagttattttttctgtcttatctttgcaccagttctttaaatagcttatcaagaaaggaggagggacatggcccgacgataccttagcaaccatcactgtgcaaacagtgaaaggtgctgcatccatcccggtttacggaccaggaaagataagtcagatcaatagttttacatgatattattcttacgataatagaaaactcatctggctcccaggtgagttttttttatgctcccaccttttttgatatgctcatttaacggacctgtttaaccaatttttcatcaaactaaaaatcaaacaaagatgagcactatcactgaactgatccattctattcccgtagatccgcaaacaggcgccattgcagttcctatttaccagacatctacttttgtgcaaacagcacccggtgtaaataaaggatacgattatgcgcggtcaaataatcctacccgtgaaaccgcagaaaagatcattgcgaaactggaaggcggcgctactgcatctgcttttgccagcggcctggcagcaatcgacgcggtaatcaagctcctgaaatcaggcgatgaaattgtagcggtagatgatatttacggcggcgctttccggctgtttaataaagtatatgagaagtttggtatcaaagtaaactatgtagatacctccgatacgcaggcggtattcaacgccatcacaccggccacgcgcctgatctggctggaaacgcccactaatccaacgctgaagatttcagatattgcggctataggccgcattgcaaaagcgcataactgtttgttttgtgtagacaatacctttgcctcccctgtgctgcaaaagcccttgcagctgggcgccgacctggtgatccacagtgctaccaagtacctgggcggccacagcgacctgattgcgggcgtggtagtggctaaaacattacaactgggagaggagattaaattttatcagaatgcctgcggcgctattctttccccgttcgacagcttcctgctgatacgtggtattgaaacattgcacttgcgtattaagcaacatggtattaatgcgcaggccctggcggaatacctggaaaaacacccggcagtagaaaaagtgttttacccgggattgccatcgcatccgggccacgagctggcaaagcagcagagtaaagggtttggaggaattatatcttttaccttgaaagatgacagggccgaagcggcaactgcgtttgttactgctacgcattactttaaactggcagaaagcctgggaggcatcaaaagtttattgtgtcatcctgcggccatgacccataaatccattcccgcagaaaagagaagagcggcaggcgtaagcgatagcctgatccgtttatcagtaggacttgaagaaaccgctgatctgctggccgacctggagcaggcgtttacgaaactgccggcgcccgcccccgcagaaaacgtgttgtcagcatagcagcaacattgtcgcccgtcgcattgaggattgtagccagcggatctaccagcgtgcctataatcatcagcggcgggagcgcttctatgggaaacccgtagatgctcatcaccagcagttcgccaatatagccgccattaggaataccgccttccacaatgctggctataacggtaacgcctagtgccattaaaatgatggggacgctgtcgaagccctttccgaacatggcaaacaccacggccatttttatgatggaagaaatgctggagccatctttatgcagggtagcgcccaatggcactaccacgttgccgatatcgcgtggaacgcccatccgctctactgcctggagattagccggaatagtggcaatactgctgccggtaccaaccgcggtaagggtgggtacaatattgttcttccagaaaatttttatacccggtataccaccggcaacaaatgcgtacgcgctgaagccaacaataaaatatacaacgccaaagccatagtaaataccgagggagtgtgcataggtaccaaatagttgcggccctacagtgcccacctggtaagcgaagtaggcgcccagcccgatagggcccaatttcatgataagcgtaaggatatctttcatcacctcgttgcccgactgcagaaatccgcggaaagcagcgcctttctctcccgtacgcatggctgccaaacctaccaggccggagaaaatcaggaacggcagcatatttttacgcgacagcagctcataaaattcattcacagtgaggagccgtactgcctgctcgccccagttgcccggctgttccaggttcacatcttttgtaagcgttacctgctggtggatgggaaatatccatacggccacaatagtaagaaaggcggagatgagaacggtgcaaaggaataccagcgacatcacaccgagaatacggcccagcttatgccccgcctctatattggcaatggcggacgagatcgcaaaaaataccagtggtatgatggctgtaaacagcaggttcagaaatacatcgcccagtggtttgataacggctacacgctcacccaatataagcccggcaatactgccggcaatgatgcctgccagtaaccagaacatactactgtacgttttgaggaatcccatacctgaagtttatgatttacaagataaccaaatgtatctgttcggtgaacaatctgccatgattattgtttatggtgttagcgaaccaatataattatcatgaaaagctggatgctatgtttgttgcttcccctgttcgctctgcaggaacgaacttacaccatcggagaggtgatgcgcaatgcccggcaactgcacaacgacagcatcgctgttaaggtgaccggttacatcaccaaaaagctgcgtggcaataattatctttttgaagaccgtaccgccgaaatccaggtggacatagacccgaagttcctcccgcaacggccgttcagcgaccgggaagtgatcactattaaggcgctggtggaatacgaagtcgacaagcccattactttaaaggtaaaccagcaggtaagcaacgattaacggctacggctatatgattttggctacaaacatatagatgctcctcatacttgccaggatcacaatgatcgccaccgctaccataatagttttagcagaaattttattggatacttttgccgcaataggagaggcgatggcgctacctataacgaggccgagtacggcatcccagtgtacgtgatacaacaccgttacaaaagtgagggaactgagcatagcgataaaaaagcgggtagcctttaccgtgcccagcgaaaagcggggatgccggccgccggcaatcagggacgacaatacaatagaaccccagccgccgccaccgatagcgtctataaatccgccaccgaagcccagcaggcctattcgcttaatttttttagctgcgtgttttttgcgctgcgcgttaatggctctcatcaggatgacggtgccgaggatcagcgtatacagcgataccaccggtttggtgtattgtgcgtaatgttccagcgacgataagaggtaagcccctatcacagcaccggcaatacccggtaatatgagtagtttaaacagttttttgttgacatttcccatccgcatatgcatccagccggcaatgccgcagctgaggatttccgaaatatgcaccgccgtactcgccgatgcaggcggaatgcccatcgacagggaaaaagtagtggaagtaatgccgtaagacatgccgatggcgccgtcgatcatggcgaagataaatcctgctatgaggaaatagtaaaaagtaggaggtacgtcttctacatacgtgcggaaatcgggcgattgccaccacgccacacccaggataacgcccagtatgaggatgcctgctataccataaatccagcgctgttttctaaagttgacgctttcctgcggcgttgcagcatttgattcgtttgtgctcggagctgcgggtgcagcaagggtagtaagttctttctccattttttaataatgtgccagccttaattccccacaaaatacataaactctatgaaataagtagactgcttggaaaaaattgcatatcagaaaggtaaaatcccgaatatatctcccggaattttaatttataatctgtaattcttcaaaatacccgaacgtataaaaattgatttacctatatttggggttgcgaaccaatttaacaactacatgctttggcaactcttctggacaattatattagtattattaaacggattctttgttgcggcagaatttgccattgttaaagtacgttcctcccaaatcaacagtaaaggcggtttgaccggcaaaagagctactgccgccgccaaaagcatcctcaataacctggacgggtacctggccgctacacagctgggaattaccctggcttcactgggacttggctgggtgggtgaatcggtgatgacggccatcgtgctccggttgatggaaagtcttggtgttaccatttcaatggccgctacccatgtaattgccgtagccgttgctttcactattattaccatcctgcatatcgttttcggggaactggctcccaaatcaatggccatccgtaaaccgctgcccaccacgctggtggtggccatcccgctgcgggcgctgtttgtgatcttccgtccttttatatggctgctcaacgggctggccaacagtattctccgccttatgggtattaaaccggccggggaatcggaaatccattcggaagaagaactgaagctgatcatttctgaaagccaggaaggcggcgctatcgaggaaaccgaacgggaactgatccagaacgtatttatgttcgacgacagccgcgtaaaggaaatcctcacccaccgtaaagacatatcctccctcgacatcaacctgcccctggatcaactgatagaccaggtgatcagggacggctactccaggtatcccgtatccagcggttcgctggatgaactaaaaggggtggtgtataccaaagatgtggtgaaaggcgtacatgaaaaaacattgcataacattaaggatatcatgaagccggtattttatgtgccggacagtatgaaaataaaagacctgctgcgtaccttccagggacaacgcctgcaaatggcggtagtgaccaacgaatttggcgatacagagggaattgttaccatggaagatatcctggaggaactggtaggcgacatacaggatgaacatgatcatgaaacgccgattgtagagcaaaaagatgataattttattgtagatgcgcatgaatacctggcagatatcaatgaattattaccccatcctttgccggaaagtgaacattatgaaaccctttcgggtttaatcaactacatccacggaaatattccgagggaaggagaagtgatcatcattgaaaattatgaagtactgatcctgaaaatgttccgcagctccgtggaaaaagccagattaaaactgatccgataaaataatttttatggagaagaagatcctccacgtcctcgaaggacgcgaaaaacatattacagatacagaagtcgtaagacaatcactgcctaccatgcagttccggtttgccaacccgtttattgtggtgcatcatatgccggcaaagtattttgcgccgggatcgccggaagacaggctgcatccgcatcctcaccgcgggtttgcaccggttacctttatgctgcaggggcagggatatcaccgcgataatgccggtaatgccatgactgttaccgccggcgacgtacaatggatgtttgccgggaaaggtattttgcatagtgaaggcccgtcggaggaatttctgaagaaagggggcaactatgaactattgcagctctggtttaatgtaccagcagcgcataaagcagaagatccctggtaccagtatatcaaaggaacagaaatgcccgcagtggcggtaaaagaaggcgtgcacctcacgctggtaggcggcgattatgaaggtaaaacagggccgttaaaaaactttacgcccatcaccgccatctggggaaatgtggaagcaggaaaagccgtaacgcttacggctacacgtggatactggacgttgttgtatgtagtggatgggaaaatagaagtgaatggaaccgctgtatcaggttatcacctggtggtatttgataaggatgatgagcaaccggacattcatatttcagcacttgaaaatacccgcctgttatacctttgcgcggaaccgatcaatgaacctattgctgcaaaagataattttgtaatgaacactgcggaagaaacggagcaggcaatacaggattataagaatgggctatttggtaccctcgaacaataaaaaggaggggagattcccctccgctaaaaatcatctgaataaagtatctcttttctgtggccaggaagtatctcctttcttatcttttttcttcttgtgtttcatgacggtatccattggcttaggtggaaaagtgtcctgtgcaaatacttcaatctgatcaatctgagctggctttaccggagccgcctgtgctttgtccggagtacccctgaagaaaaagaggagggtaagcgtgcctataaggccgatggtagctggtaggtttttcataaaaaaataaatttgttcaggtattaataagcagatatcatgcgccctttccagcggcagagcactgttgatgtaagctgctgacaatatttcagttatcttatcgttgcgttatttattcccgtttttactgtggatattgcacgtcaaacagtggagtgacagacacgttatcccatactgtatacccctatggacggccggaagaacgtgaggcactgcttttgtggcggttaagatattgttcaccaaaaatttatcttatgaaaggcaccagaaatgagaacacccggcaaagtaaacaacagtctttttccaatatgccgcgtcccgaaatcagggataatcttgacagcaggaaaaatgaagaacaggattataaaggcagcgataccacgcacaacagtaaagacaccaaagctaacaaacataaaaagcattgatgacaggcagttccggccgctaaccggcggccgggcttttaaatcagcagcatatggatcatatacttttcaggttatcgctgttagcggtggtaatttgcaccgcatgtaacagcccgatgcagaatgagcaggagcgggcagccaaagattcggccaatgccccggttcagggcgtgccggaagaaaaatcggaaagcatctcgttagatactacatatggcgactaccgcatttcggcgattgcctctggtaccggcagtatgcgggatcttattctggcggtaggcagcaaaaaggattctacacaggcagacagtaccattgagcatgacgtgaaagggcagctgaaaaatatgatgatcgcagacctggatggaaacggtaaaccggaactttacctgcaaatgttatcggagggtaccggccggtttggtaagatctatgcttttgaaataggacggcctaaggttacaaggattaataccttctccctggataccatgcagcaaaaggattacaggggacaggatacattttttataaaagagaaaacgctggtacgtacttttccggcgttcagggaaggtgatcccgatgcgttaactgcaaacaccaaagggattatcatttatcacctgcaaaaggcaggcgacaccctgaagctggtgccggcgaaataaaagctattgcagccataccaggctgcaatagcttttttacaattatttattgtactgaataccttctttatcccagcgggtatagaagtattgcagtgcatcggagaactgtgtgaagtttttattggcgggaatggtccacccgtcttctgcataagccgccaggcggggaaatacctggtggttcattgtttttacatccggaatccattcaccccacatctggcagccactgcccagtattttgctgtggaacttcggatcaaggccttcggggatgggatcaaagctgtaggctttttccaatgatatttccttgtagctgtaatccaggtaagtcatggcgtgataggaattgattacgtcgtatcctttagacaccgcatcggtgatcagtttcagctcccctttccagaattgcacaatggtaccggctgcgagtttttccgtagcggaaacatctttgctatcagtgaactcatgcagctttgtgcccatgatttcgttccatccggccatacggcgttttttgcttgccaggtagttggagatattgttggtgaaagcaatctgcaggtcggcaggagagccaagctgatgcgctttcatgaaggcatttacaccggcatctgctttccactggtcgtattttacttcgtcgccgccgatatggatcactttagaggggaagagggtgatcacttcctgcaacacatcttccaggaaggcgatcactttgggatcagacacattgaaaacgtcgtaatgcacaccgaatttacccggaaccctgataggcgtgtgggtggtgccaagccagggataggctgcaatggccgcgctggaatggcccggcatttctatttcaggaacaatggtgatgtgcctgtctgccgcgtatttgataatgtctttaatctgttcctgcgtataaaacccttcgtggggtttgccgtcgtatactttgctgttccaggtaccggattgggtggaatcgcgtttgctgccgacagtggtaagcaggggatattttttgatttcaatacgccagccctggtcgtcggtgaggtgccagtggaaaacgttcattttcagcagtgccatttcatccaggaggtgttttacagtttcgccgcctttgaagtagcggccctcatccagcatgaatgccctccagccaaagcggggcttgtctttgatggacacggcattaatcgtatatgcgctgccgttggcggtaatgagttggcgtaaagactgtataccataaaacacgccggttgaagttgctgcggtgatggtgatgttatcaggcgttacctgcagctggtagccttccttgcctaattccttctccagttttgcgtccagggagaagcggatgtagttgtttttggcagcaggtttcagtgtgagagagagtccatatgcttcctgtaatgcctgttgcagctggttggcctcgccggcgcacttgcctggaatgatggcagtggcgccggataaagagaacgtgccggacaatgtttttacttccgacggctgcggaataatattgattgcctgcaggggcatggtacttaccgacagcagcagcaggccggccaatgccagtgtggagcgtagttttaacatacgtagatttttattgttcacttggttaaggtgaaaaaatacaataaaatcccgtgatttaaaagaactgcgccattaaccttcctgttccatataaccgcttggtaatccgttttccatagaggcgtcgccatagtcgtattctaccgcataattttgcggcagggttacgggcctgtccagttgaggaaacaccggctgcgccttgaatgtatctttccattgctgcagggtagctgtatccaggtgaatgggatgcaatatccttacctgcgcattttccggaagggtaagggagtcgccggtaagcgtccgtggcgtgatgttttcatcgcagtagaaggcggtgatcagctgatcgccttcatcgaataacgcccagacaagccttgtggcgaaaacggacatcaccgggttgtgccggaatacggcctgccatttttcggcgctccattttctttgttcttccaggaaaagttccagtcgctgtgtttgtactttgatggtatcggccatttcctttggcagtgctttgaaagcattcctgatttccctgggagtggctacgggaatggctttcaggcgacggcccttatcattaatgtaagccggtttaaagttactgtcgaggaatgcgcggtatgtttcgcctttcacttcaaaggaccggtacagtccatcgaagccaaaatcaggcactattgaatcgatcagctcctgcagcgttaaacctctttctgtggccgtcagctccagcgcccggagggctgcagcgcctactactgctttacggaagcggtacctgcgtgagaagaattccacttcgcggagcgctttattgctgccatgcagggccagcgcgcccacgccgtgttccgccattttgaggcgtttggtggtaatccagagctgtatgtcttcccgcagggtatcggccagcaggtcgtctcccagcagggcggtgagcgtcatgaggtactttagcttcaggtcgccgccctggtcggcatatgctttatagagtgcgcgggcaaagtcgccgctgcgggaccggtcgatcaaacgcagcagtggtttggcttccacgtcggcgtgtacttccgttaccctcgacatgcggtaaatcaggaagcgcatcatgtcggtggtcatcaccgtaccatccagcaggtagagcggcggcaaggctttgtcgtccagccatttctctgccggtttggagagtttgtgtcttttctttgcaaacatcaccagcctggtaacgagcaccaggtcgtcggtatctgtgagggtatgtcctcccagtgtttccagcatcaggtcacgtgcatcgtcgtttacttccttgtggagcgcctgttgcagcagttcgcgggcatgctcatggtcgagtttagacaggatctgtacggcggttaagcgttgatcggctttcttatgccccagtaattccgccgctctttccagcgcccgcgggtgttccgccagtatcacggcaacgagcgtacgaactgatttcagtttatgcagggtgtatggccagagctgatctatatacagtgccttgtccagctgggagagtaccgggagtattgttctggcgtcgtaatcattttccagtgcgtgcagcagcatgggtgctgcctgttcctgtaactcgtctgccagcacctggaaggcttcggggtggagcgaacgtttttgagcaagcaggtcagcaagataaggaacggctgcggggcggtcgaggtgcagcaagccgcgcactgccagcacgccggggggcatattgttgggcggtatgttccctgttacctttgagtaccccgattccggtgtgtatgagccggtaacctgcctttccaggtaatcgtaggctgctttcagcagccgttggttatatttttcgggaagatgaccggcgagaagataataaccactgacggcggcggcataatcgggcagtgcagccagttgcgtggttgttttttcgatcagcggttcatacttgcccgggttgttttgcagtaatacgcgggacacggcctgttgatccggaaggtattccggcagcaggaggatgttttccaggtattccatttcccggtccgggtgtcctttggtaaggagccggaagaagagggagttccatccttttttacgccaggtgtttacataggcgttgatcacatgtggttccgcacttttgatcaggtcctgcagaaatttgcgcaggggcgtgaatttcagcggtgcaaggtcgaagttattgccgtccctggaatagctgatcatgagagagccgatttcttccggtgtgcaaccccgttgctgtaggtagctggtaaaatagctgaaccgcagtacaatggaagaggaggttccgggcatgtccatcatcggaatgatggttgtcaggaaggtttccctgcattcgttccaggtgatcggtggtgaaatcagctttagtatgagccggtcgttgtcgtcccagtggtcgggaatttgcagcagggagatgaaatgtcccatttgccgggcggtttcagcggtgggaaataccggtgtttcataggtgtgccctgtaaggaaatctaccccggactgtatagcgcctgcgatgttttcatagtcattcagttgtttcagtttttcaacaagaggtagtatagtttcctttttgtatggcataagggtatagatagattcagattattttttcagcacaatatcttcttttgctgcccattgtgcaacatcctgtttgctcaatgcgcaggccatcatctccggaaacttgtccggggagcaggcgaatacgggtattccgaggtttgccaggaattgggcattctcgtgatcgtagctgggggcgccttcatcgttcagcgccagcagtacgattacctgtacacctgctgctgcaagttcggtaaagcgtttccgcatatttttttcatctcctccttcaaagagatcggtgatcagtaccagtacggtgtctgccggtttggtgatgatctgtgcgcagtatttcagtgcggcatggatatctgtacctccgcccagttgtacgccgaacagcagttccaccgggtcctgcaattcttctgtaaggtctgccacggcggtatcaaaaaccaccatctgtgtttttagcgccgggatagaagccattacagccccaaagataccagaataaacgacagaggtacccattgatccgctttgatccaggcataataccacttctttcagcgccgaccgtttgcggccgtacccgatcagtgtttcagggataatggttttatactccggttgatagtgttgcagatttttccggatggtgaggggccagttcacctcgttatgccgtgggcgccggttgcgtgcactgcggtttaagctgccggtgatggcttgctgggtaggttgcgccagtttccgcatcagttcatccactacttttttcactacctgccgggcggtgtctttggttttttccgggataaccttgctcaaagtcatcagggtggccaccatgtgtacatcgggttctatgttttccagcatctctttttcgaagagcatctgggtgaggttcaggcgtttgagggcatcttgttgcattacctgcaccacagaggcgggaaagtagctcctgatatcgcccagccagcggcttacgtttggagaggatggtcctaatcctccctgcctggtgctgtcgtacagtgcttccagtgttttgtccaactgcaggtccgttttatttaacgggaaggaggtaccgtcattctgggatccacccagtacgagccgccacctgcgaacctgttcttcatgctccatccggtaataatttagcgtctttaaatcccagcagctgcatcactacggggatgccccgggcgccccggtcatgatctatatcccctgtggcagctgtttttatgctggttccatttccgccgtgtttcactttgtcgcccagtttttttcgttccggggcggtaaagttagaaaaggtgcggcgtaataacggcaatacctgtatgaaaatatcattttccagttgggaaacccaattatgcaccatgtcccacagctcttcatccaggagcagcagggtaccgctgcccctgaggaagccctccagccaggcggccgccagtgcaggcggattggctactgacatggatacactgaaagcttttaccaatgtttcccccgtcattattttgccgtcgaagaggagccgtgaagcgtagccggctatcatgggggccgattgcgcgttgcgggaaatggccagcagcgtttcctgccaggaggtggtgagggcattatcctgtatgaggttaatggcgtcgttcatggcaaagaagagatccagcagcgggagtgcggcatcatcggcaacggcggtgcaggcagcgggtaagctgatgcagatgcggcctatcatgctttcggtgatattgctgaccagcgccgcatctgttttgcgcacgttgccatagcggctgatatttaccagtgagggaattacttccatcagctggagcacatcgccggaggcggcagcgaggttgttgatccggtggatcaatacttccactacagcggggagttctgcagggatggctgattccagcattttacatacctgctgaagagtgccggtattattggcggtgttggtaacaaagctggtagcggcttctgctacggtatttccccaactgcctttttcgatgatatcaatggaaaaggcggggtcccattgcaggcgccattgttctttgaaggtacctttcccggatacctcgaaacgttttccccagtatatttccagcagttgcaggcggtggaggaaaatacttctttccaggtccgtgtctttccgcaggtcgagggtatagtctttaaagtcagctgtttgcggcagccttagttttttctgccaccgggaaatatcggcctggagtggaggcgtaggcacttctgcgggtactttcccgatccggttgcgtacaatcagctcatcacggatcagttgcatgaggatactttccccgttgcagagcacactgagggtggcctcgttgagttcttccaatccgggtctgggataatgacggagggcagccaatgcgttggccaggcgtactgcttccattacgtgcgccacggaggtatcctgttgctgctccctgaagagctttgctaccagcgccatccagcgggtaccatcatcggcagggtattcccagatgtgttcgtaccatcccggtgagggaatgccggcgccatagccgctttcataactgaggcgactatacgtccatggtatccaggtgcattccacttttactttggggaggcctttcagcaggtcgttatcatctttttgtttgggcatggtttgcagcgccggtgcgtgccaggcgccgcatatgacggctatccgctggaacatttccttttctgcctggcggatgcacttccgcatccaggcttcacggagggcttctttccggtcgtaccgccgggggagttcttcccggagggcgtgcatggcgtcatgcaccgcctcaaatacctgttcctgtccgaggcggtattcaaacatatgttcccaccagcgttcgctatcgtcgtatccggcggcatgggccaggtgggcgaccgggtcttgtggtgatggcgggagaaattccaggtccagttcttccgcattgaatgctttcgtggaagcattcaatgcggagttcagttccgcgggaggcatgtcttcccctggtgttgtattttcagcttcttctttttgagcttcctctttttgagcgccggctgctctttttgccgcggcttcgttttccatgccgaatacatgggccaggggaaggtccataaagcgggcgtggatgcggtgggttttggcatacagcatggcctgccattccggtgagaaggccgcaaatggatagaagcaggctttctgcggactatccggctgataagccaggatggccacgggtggttgcagctcttcatgaccggtccattgcagcaaggcatctgcttccggtggtccttcgatcagcacaatatccggttgcagctcttccaggaaagcttttacattcctggctgagccagggccgtggtgccggatacctaatatatgtacggacatacgtcgatcattattaacaaatgaatggagtgccagcagttcggcacctcccggaaattatactgaaagtaatttctaaacaaacataatgtaataaacacattatgatttacttatgaaattactattaaagtaaaaactaaagcagtaaagcaggagttttcacgttgtatcacgctttatagccttcataaaggtggacttgatacggcgtatgcccggctttgacccttagtaagggtggacttgatacgcttcatccccgctttaaaggcggacctgaaccttacctgctgctaagcgaggtcacggcaggcgcggtacacatctttccaatcctcccgtgtttttaccactgtttcgagatattcctgccaaaccagtttatcctgaacgggatctttcactacagcgccgatgatgccggcggccagatccgcagcattgagggtaccatcgccgaaccaggcggccagggtgagaccattattcaccacagaaatggcttcagcagtgctgagagtaccgccgggcgatttcagtttggttttgccatcgagggtaacgccgttgcggagttcgcggaagatggtaacgatgcggcggatttcttccaccgcaggcttttctgccggcaggtccatcgttttttcaaagctttccactcttcttcttacaatatcaatttcttcttccatagaatccggaacaggcaagataacggtattgaagcgacgtttcagcgcactggataattcatttacgcctttatcgcggttgttggcggtagcaatgatattgaatcctttggtagcctgtacttccgtattcagttcaggaatgggaagcgttttttccgacaggatagtgatgagggtatcctgcacatcggcgccgatgcgggtgagttcttctatgcgggcaattttgccttcctgcatcgcgcgcatcaccggggtttccaccagggcattccgggtagggccttcggccagcaggcgggcgtagttccatccatagcgcacactttcttcgctggtaccggcggtaccctgaatgatgagcgtggaatcgccgctgatggctgcggcgaggtgttcgctcacccaacttttggcggtgccgggcaaaccatacagcagcagggccctgtcggtggcgagggtagccacggctatttccatgaggcgtttgctgccaatatatttaggggtgacttcaaaaccgttcttcagtttcccgccgatcaggtaagtaactaccgcttgtggcggcagtaaccagttttgcggacgcttccctgcgtcgtcttttttcagttcttccagctcctgtgcgtacagttgttcggcgtggtaacgtaaaatgtctgacatggtatgttgattaatgtgtttggattaaagtgattgtatctggctttttgcctggagcagccggcccaggtgaactttgatattattccagtacccggtgtgataggcctccacgggtgtgatatcatccagggtggcggcaatggccacgggtatctgccggatatgattattcatgaattgctgattgtaggtgtaaggctgtgtggccgcatatttgaagatccgggtacacagcgggaggctccattcttcctggttgttgcaggcgtactggataatagagtccgggtgttcatcaaagaacttttcactgaactgctgttgttgttccggtggtagcagggggatgatatctatataaaaagtttcgctgtgctccataaaggaaacggcgcgcgctttgtcttcaaaccaggcaatagccagcaccagcgcagggataaagggtttcagcgattcctgcagctggaagagagcgatgaccctttccgtattccggttaaaatgttcttcccagcgagccgggtgtacgaagctgatcagctggcagaggatgtgtgtttcatccgtaatgcttttatcgttgctgagtttttcgatgccgctctggaagatgctgtcgtccgttatttccgggagcgctacggttacctgaccgtattcatcgagttgtatggcgccggctacgatctgccagtatttttcatggagggaggagccgggcagttttttcaggatgcgggtggcggtgtcttttacctgtttacttttttcggtgagcagcgattccagccagggaatgtctgcgggatgggcaggttgttccagtacggagagcagttccgttttcacggtagcgctttctttaggccaggattgctccagccaggtgcgcgccattacgggatcggttgcacgcaactccttcagcgcttcaaaacgctgtgcggtggcgccgttctgccatctgtcttcgatggtatccgctacgcgtgaaaagttccagtcggggttaaagtgcccgagccattccgcacgttgtccgcccgtagcagcgatcaatgcgcgcaatgatttattccgccagcctttgtcgagcatcacgggcagttgcgccggtggcaggagtacattggctttggcgcagtattcgagccatagctggagcagctggatgctttcggtttccagtacctgttgcagtactcttatggcggcgggcttgcagtaaagttttgtttccggcgggcacactttcatgggtgctacgttggcggtaacgggttgcgtgccgctcaggcggtagttatagagcactgctgccagttgcaggaacttatcttctttatctgtgtgttcgcctgtcaggatggtatgggccgcctgttgcagggggccgttcataccggtgctgtctaccggttttttagcggtgcccagtaaggcggtattaatgagttgatgccagtgctccattataatattttatattcctgttcatgccaaacgccaatgggttcatattgggtttctttaccggtaactgccatgtggaggggtgttcccccgctcagcgccagcagtttccaggtgtgctggaaagtttttttcacggccatgagttgctgacggctgtcctgtagccaccattgatccgcgtgccaaacaggggtaaggtctgcgatcgtatatacctggtcgttatacacgggcaatacttcattgatggcggtttgcgcggttactacttcctgccatccggcatagccgctgaaggtgtggtttgccggcaccgttacctgttgtttgatcagtgcgcgcagcggtgctgcggaaggataaaataccagttccgcattgatggcgctgccgggagtgagggtattggcgatggtgctttgtccgcgtacataaaactgcagtatcagtgcgggacgtttggtatttatgccgtatagccagtagcgttccaccacgaggtggtcttcttccgtggtttgttttcccagtacctgccaggtgtcggtgataccgttttgttccttcagttcttcctgtgaggtagaaaaaccggcgagggtgcggatatcctgccggagtgctggtgggaggtcgctgaggtgctgatagccctgtataacgaggtaaatgcgtgtgagctgggtgataaaaacggattgccatccgtcgtggaagtagctgatgtctgccagttcgcgcatcatggcggcgaggccgggggcctgtgcatctaccatgcggcggatcatattttcgaagaaagccggatctttttcgggcatgtccatgataccgttgcgcacgagatcttttatccagcggagaagttctgcggcgccgtcgcttactttctgcatgcgtgcctgttgccttttggcctgggcggaggtatctggctgcttctctgttgaagtggcggatgtatttttcttctcttctttttcggcgcgtttggcgagccattcgcttacccaggacggtggtgtttcttcctggaaggaagcccgttgcctggagtagagcaacagcaggcccagtccgtgtttacagggaaacttacggctggggcaactgcatttgaatgccatgttgccggtatctatctgtgtctggtatggtttgctgccgctgccctggcattcgccccataacgctatatcgctgacgcctttactaacccatttagccggattagccagatccttcccggatttacgggaagattcatcaggcgccatagcaagcacttgttcgtcggataggttcaatggattaacgatttaaagcgcaaagtaaataattccataaaataaaaaaccaaatatcaggtaacactacgcagtgtatctgatatttggttttagtatgtaagtattgtgttgttttacagaaagccgagttccagtttagcttcttcgctcatcatttcttttgtccaggggggatcaaaagtaaggtgcacatccacatcggaaacgccttctatatttcttattttttcatctacttcccggataatatcgccggctacggggcagccgggagcggtaagggtcatatcgataccgatcctgttattttccttgatctttacttcgtataccagtccaagttcccatatgttcaccgggatttccgggtcgaatacggttttgagctgtgcttctatctgttctcttaatattgcttcactcattgctgattaattttagcctggtaggcgatggcgtacagcttcatttgtttgagcatactcagcaacccgttggagcgggtgggggagagatggctgctcaagccgatggcatcgataaaataaatatctgctgcggcaatttcctgtggcgtatgaccggaaagtacatagatcatcaggcttacgaggcctttggtgataacggcatcgctgtcgccggtaaaaaaaagtttcccgtctttcagctctgtatgcagccacacgcgtgactggcagcctttgatgagattgtccggcgttttaaattcttctgagatgagcggtaattccttacccagctggatgatatattcgtatttatcttcccagctgcccatcaccgaaaaatcggatattatttcttcctgtatttcctgaatcgtcatattcacctgtttacaaaagcatggcggcggctctttttatgccggttaccagtttgtctatttcttctttggtattatagaaagaaagggatgcacgcacggtacccgggattttaaagatatccatcagtggttcggtgcagtggtgtcctgttcttacggcgatgccttgctgatccagcagttcacccatatcaaacgggtggatgttgtgtaccaggaaggagatggcgccgcttctttctgtggcgtctccgataaaacgaatgccatcgatctggcgtagttcctgcatggcatattccatcagctcttcttcccattgctggattttggagatcccggtttgctgcaggtattcgatagccgcgcccaatgcgatgccaccggcaatgttgggggtaccggcttcaaatttatacggcagttcgttatagattgttttttcgaaagtaacggttttgatcatatcgccgccgccctggtaggggggcagtttattgagccattcttttttgccatagagtacgccggtgccggtagggccataaattttatggccggagaaagccaggaaatccacgtcgagcgcctgcacatcgatactgatatgctggattgcctgtgcggcatcgagcagtactggtatattgcgtgcatgcgccagcgttataatgtcctgtaccgggtttatggttcccatggtattggaaacgtaggtaacggctactattttcacggaatcatccagcatggctttgtatgcgtccatccggagttcgccgcggtcgttgataggaattaccttgagtgtggcgccggtttcttcgcaggctatctgccagggcactatattactatggtgttccatggcggaaatgatgacgctgtcgcccggctgaaggaagcggcggctcatggtattggctaccaggttgatgccggcggtggtacctgcggtgaagattacttcatgcgggtctgcggcattgatataacctgcaatggtgatgcgggctttttcgtatgcgttggtagctacctggctcaggtgatgtacaccccggtgcacattgctgttatattcttcgtaatagcgggcttccgtgtctattacaacctgtggtttctgcgtggtagctccgttgtcgaagtataccagcggtttaccatgtacctgttgctgcaggataggaaaatcctttctgatctgctttacgtccaggccgtcggttatgatgttagcaatatgttccatcgtaaaattagttattcatgatctccgcaatctgcgtctgcaggaaatgttgcagggcaggcaccttcactgcatctgtgatgtcgtgggagaaggcgtttaccatcagtgcttttgccgcatcttcgccaataccgcgtgagcggaggtagaacatggactcttcactgaactgaccggcagtaaaaccgtggctgcattttacgtcgtcggcataaatttccagctgaggctgtgaattgatgtccgctttggtaccgagcaggaggttattgttctgctggaaagcatttgttttctgtgcttcctggtgtacaaggatcttgccggtaaatacgccgttggcgttatcgagcagtacgcctttgtacagttcgttgctgttgcagtccggcatgatgtgatccataaaggtatggttatctacatgctggtgtttgctggcaatatataaaccgttcagattagtttcggtatgactgccattcagggccacgctcaggttgttacgggtgaaaggggtgtttggcagggtgaaattaaaatggtggtaacggctgtctttgtgttgctgtgcagcggtggtatgtacttcccggaagctttcagcgccctgttgtacattataatgccacagttctgcattttccagtaccacggtttccagtacactgttcgcaaaagcgatggtggcggtttccgggtgaatggaagtttcgatgatggtggcggcagcgtttctgttcaggatccacaggtggcgtggctgaatgaaggcatgcgctgtacaggagtaaacgtttactacatgtatgggtttatcgaccacggtgttggcggccagttcgatatacaggccatcggcgaagagggctgtattaagctgtgccaatgattctgcggccaggtggtgctgttcattgaaataagtaacaaagcctggtgcggtggtatgggcactcatggcgcccacggtgatacctttgccttgcggcagggtagactgatccgcctgcaggtggccatttaccagcacaatgcggtagcagtccagttcaggaatagcggtgctgtttactacttcttccgcaacgggggaagcagtggtaagcagttcataaggaaactctttcaggtagcgctgaatattcgtgtagcgccatgcttccgttttcagcgtaggcaagcctatcgcagagaaacgctccagcgccttgcggcggatgtcctgcagcgtatcggtagcgagggagggagcctgtgccgacagtgcatttacatcttctgttaacgcctggtaaaatggcaatatcatatcgcttgtcatagttctttttatacagattctttcaaatgtaattcctctttcagccagtcgtatcctctttcttcgagttccagtgccagttctttggtaccggttttaataatacggccgttgtataatacatgcacaaagtcaggtatgatatactccagcaggcgttgatagtgagtaatcactacgaaagatttttctgcatcgcgtaatttgtttacaccatttgaaacaatacgcagtgcatcgatatccagtccggaatctgtttcatccaatatggcgagctgtgggttcagcatagcgagttggaaaatttcgttacgtttcttttcgccaccgctgaatccttcgttcagggaacggttcatcaggttggagtgaaaatcgaccagttgttgtttttctttggtcagcttcaggaattccctggcttcgagggccgggagacctttatacgccctgatttcgttcagtgcggttttgaggaagttgaggttggaaacacctggaatttctacggggtattgaaaagcgaggaaaacaccttcgcgggcgcgttcttccggagccatatccagcagatttttgccgttgaaccaaacttcaccttcggtgacagtgtagttatcacgtcccgccagaacagaagccagtgagcttttgccggaaccgttaggtcccatgatagcgtgcatttctcctttgtttatttcgagattaatgcctttcagaatttttttcccttctacttctgcgtgcagatttttaatcgtcagcatgattgttttatttcgttctgtatgtattaattggataatgagttatccaacgcttccttcaagtgtaatagataataatttttgcgcttctactgcaaactccatcgggagctggttcagtacttccttcacatagccgtttacgatcagggcaactgccttttcgctgtcgatgccacgttggttcaggtagaagatctggtcttccccgattttcgaagtggtggcttcgtgttcgatcatggctgttttgttccttgattcgatatacgggaaggtgtgggagccgcattggttaccgatgagcagggaatcgcactgggtaaagttacgtgcgttatcggcacgtggcccaacggataccaggccgcggtagctgttatcgcctctgccggcggaaatacctttggagatgatgcggcttttggtgcctttgccgatgtggtggatcttggtaccggtatcagcgatctgtttgttacggactactgccacggagtaaaattcaccttcggagtggtcgccctgcaggattacgctgggatatttccaggtaatagcggagccggtttctacctgtgtccaggagatcttactggcagcgcctttgcagatgcctcttttggtaacgaagttatagataccgcctttaccgtctttatcaccgggataccagttttgtacggtagagtattttatttcagcctgttcgagtgctatcagttccactactgcggcgtgcagttgattttcatcacgcatgggagcggtgcagccttcgagatagcttacgtagctgttgtcgtctgcgatgatcagggtacgttcaaattgtccggtgttctgtgcgttgatacggaagtaagtgctcagttccatcgggcatcgtacgcctttgggaatgtaaacgaaggaaccatcggaaaatacggcggcgttgagtgctgcaaagatgttatccgtatggggaaccacgctgcccaggtatttctttaccaggtcggggtgttcctgtactgcttcaccgaaagagcagaagataacgcccatttctttcagtttccctttgaaagtggtggctacggaaacgctgtcaaaaacggcatccacggctacaccggtaagggctttctgttcattcaggggaatacccagttttgcgaaggtagccagcagttccggatctacttcatccaggctgttgagctgtattttcttctttggtgcggcataataggaaagtgcctgcagatcaagtttaggcatttcaaagtgctgccatttcgggaattccattttcttaaacgcggcaaatcccttcaggcgccattccagcagccattcgggctcattcttcttcgccgaaataaaacggatgatatcttcattcagccccggaggagctatatccatttcaatatcggtgctaaagccaaactcgtactccttattggctatatcatcaattatttcgttactgttgatcatacaagtttaatatttaaaccgcaaagctttcgccgcagctacacgttctggttgcatttggattattaaagtagaggccttttccgttgagtccatcagaatagtccagttctgtaccatacagatacaggaggcttttcatttgtactactacttttacgcctttatcttcaaaaatctggtcgccttcttcttcggttgcttcaaatttcatcacatattcaagaccagagcagccaccaccttttacgcctacccgtacaaaggtgcccggcgcatgatgttctttttccatcagcgcttttatatattctcctgctttttctgaaacggttatcatactcagaatttgttttaattagctatttaccggtttcccggcctatccttatctgtttatccttcaataccagccactacatgcgatttagccgcacacagtaactgcaccatcgtatccagtttatttttatagaactcagtgaacccccgggtttcggggtcatacaggttgtctttcaaaatgggcagggaatatggtaaaacccacgcccttagtgcctttgccactgcatccatcgcatttataccctgcatggcctgggtgccgtccgcccaggacagcaaagctacaacctttcctgttaaataaggacgctggttcttgcttgtcatctcgagccagtccaggcaatttttcatggcgccggtcatgctgccatgatataaaggagtcatccagatatgcaggtccgccttacaaaaagctttgcacatggcgtctactgcgggtggtttcgttcctgcttccgcctgggagaaaaaggggatctgggcgttacccagactaaagatctccggggaaaatcctttctcttttaactgttccgtcagatacaccgccagctggtttgctgtggcataaggacggtcatctatcgcaccattaaatatcaggacgttcattaatatttaacttttagagatttaaatgattatgagattaaattttgatgaaggatctcataaactcaccaaaatcccaaaatcttttttttagctttcacaaaaataccgatatttgagaataaaacaagtaagaacttggaaaattatccaatacgaaccaagaatgctgccgaacggtttttgacgttgctcaagacccggggaccgctgtctgcagctgaattggccaacgaattgggtattaccggagagggcgccaggcttcaactgcttaaactggcagaagaaggattggtgcagtcggaaagtgcttccaaaggcgtaggacgcccagttttaatatggagtcttacccccctgggtaatgcccgtttccctgacacacataccgaactcacccttcagctgatccagaccattaaaacggtattgggaaaggaagcgctcgataatgtggtgaacgcccgggaaaaaagccagctggaaaaatacagcagtgccctggaaggtgtaaacggtattgaaaaccggctcacctcgtttgcggccatccgctccggcgaagggtacctggcggaatggaaaaaagaaggcgatacgtattactttatagagaatcactgtcccatttgctgcgccgccacagaatgcgacaatatctgtacttccgaaatgcgcacgtttgtgagcatactcggggagaaaatgaatgtgtcgcggatggagcatattatcaacggcgcccgccgttgtgtgtataagatagaggcggagtagcggaggttgtctttctcaggattacgctgattttactgattacctggatttttacttttggattttataaaggattaagggagataggagcggatatattcgcttttatctcccttaattattattaaaaaaatcaaagaaatctaaaaaaatccaaaagtaaaaatccaggtaatcagtaaaatcagcgtaatcctgagaaagacaaaatccgcgtgagactgttatttcaggatgagcaccagggtgccggcgatgatgaggctggcgccgatggcggttttcagggtgagtgtttcgtgaaggaagatagcggagaggagaatggtgagcgccacactgagcttatccacgggggctacctgcgatactttgccgatctggagcgctttgaaataaaagatccaggaacaaccggtagcgataccggataagatgagaaagagcagtgcgtgtttggacagggcgccggcgcctttatattcccctcttgcaaacacaatggcccaggccaataccaatataacgagggttctgatggcggtagccaggttggaagggatgtccgctaccccaattttggccaggatagcggttaaggccgcgaagaaagcggatagtaatgcataaaaccaccacataattttccttttacggtttgtaagttatcccggaaaactgaaggaatgttgtagccggaatcagatctttatacctaaaatttttaaacttctttccactccatccagtaccgcaatttccggcaggtgcgcccattcttcaaaacccatattcagaaacagtttcagactgggttcgttgtgcgcaaaaataaaacccagcagtgtttgtacgccaaattccggcgctacggtaatggcatgttgcagtatttttttgcctaatcccttgccacgcatcgtttcatcgagatagatgcttacttctactgtgccgtcgtaggccggccggccgtaaaacgactgaaagctcatccatcccacattactgccgttgtcgtctatcatccacaggggacggagggtattgttgtgcgcatgaaaccagggtagccggctttcaacagtaacaggtgaggtgtcggcagtcaccattctgctggcgatagtggtgttataaatttcaacgatccttggcaggtcggcttctgtagcatgccggaattgtaagctcatgatataataattagaaaatagattcgcgtgtatgttcgtgtcttagaagactgtaaagttctgcatttacgaattttcctttttcaaaaaaggcatctcttaaaaaaccttcgtagcggaatcccagccggcttaacagcttggacgacgcctggttttccgggtccacaaaggcttcaatgcggttgaactgcaattcttcatagccataactgagcatggcgcttatcgcttctttcataatgcctttgccccagtagatgggtttcaggtcgtaaccgatttccgctttgaaatgtgttttgttgattttgtgatacccgcaggtgcctatcagttcatcctttccggccagtgtgatggcccatcgcatgccttcttccttttccaggctttgacggaaaaactgtataatatgggtggcttcactgatattggaaaatgaatcaatgtccatatattttgtgacggcatcatccgaaaaatgcctgaacagggcggcggtatctttttcgtctattggtctcagtaccaggttgccggtatttaaaacgggtaaatgcatgatacggttgccggtttaggttggggcaaagctaacagatattgcgaaaatgtccataggaaccttgattttaatcccgctttaatgcctgcccgggtaaacaatgctacttttgcaggggttattgcttataattttttgatatgaaaatactggttatagaagatgaagtaaaagtgggcgctttcatcaaacgcgggctggaagagcaccatcaccatgtggatgtgcatacggatggcattaccggtcagcaggcggcgctggaacacgactatgatctcattttactggacctgatgttgccgggtataaacggaacggctatatgtaaaaaactgcgtgcgctggaaatcagtatccctgtattgatgcttaccgcgttaaatgccacggaggatattgtagaaggactcaatgccggggctgatgattatctcgccaagccttttcatttttcagagctgatggcacgtatcaatgcgttgtcgagacggaaaagccacttccacgaggagcctgcggtgcttaggtttgcggatcttcaactggatacccattccaaaactgccagccgggatggacaggaaattgtgcttacagcgaaagagtatgcgttgctggagctgctgctccgtaataccggaagggtgctgtcccgggcgcttatttcagaagccgtgtggggactcgagtttgacacaggcaccaataccattgatgtatatgttaattatctccggaataaaattgaaaaaggctttaccggtgaaaagctgatccataccgtagttgggatgggttatgtgatgaaacagaaataagcttatgaagatccggcaccggctatcgctgcagtttactttgatttcaggtattattcttacggttgttttcgtactgatatacctgttatctgcccaatacatccggaacagtttttataagctgttgcagatgcgtgcgctggtaactgcgcaggtgtaccttgaaaaagacgagctgacgaagaagaaatttcttgaaatagaaaagagctaccgggaacggatacccgatgaatccagtaatatttacgatcagcacaaccaggcggtgttcattgaaaaaacgaggtataactggccggtgtcgctgctggaaaccatccgtcaccaggaagtgtaccggttcgttttccgggaagagtcgggcctggggatttattatcccgataaccagggcgattttgtagtgatagtaaccgcgcgtaatacggcgggcatccagcagctgcaatatcttttgtggatactggtcgtgatgtttttggttgccctgctgatcaccttcctgatggggcagtggtacgccagcagggcgctcgaacctattaaaagcatcaaccggcaggtgcaaaagatccgctccaacaacctgcacctgcgcgtgcagcaaggattaaataaagatgaaatagatgaactggctgctaatttcaatggactgttgcaacacctggaacaggcttttgatatgcagcgttcttttgcatctaatgcctcccacgagttacgtacaccattaactactattatcggggagatagaagtaacacttcagaacagccgtagcccggaagaatatgtacaaacgctgggtacgctgctcggtgaatcggagaaactgaagatcattacggatggactgttgcagcttacacgggtggatgccaaccttacagaagccaacagcgagctgatccggatggacgagttattgtgggacctggcggaatactggcgtcataaatcgccgccgttgcagctgcacgtacaactcagcggtatgccagacgatgctgctttgctttgcatccgtggtaaccgttcgctgatagcattggcgttgcaaaacatcctccgtaatgcatttaaattttcgtataaccgtgacgttagttgccggctttcctatagcgacagtggtatcagcctgtctgtaagcgaccgtggtattggtattgcggcagctgataccgaaaagatctttatgccgctgtaccgggcagataatgcgcattccttcgaggggtatggcattggcttatccatgacgcaaaagattctgtacctgcataaggcctccatcacggtgagcagcgtgttagggcagggaaccacctttaatattttctttcctccggccggtaaatggctgtaaaggttttgttagtccggaccgctgcggcaacgacgatatttatggtttagtctttcttcaccactttcaccttctttactttcggtttggattcatcgccaagcaaaatagcccagggggtcatctcttcgatattctgacaaataattttaataatagcgatggtcggaatggcaaggaacatgccggggatgccccataacatattgcccagtaccaccccaatgatggtgatcaatgcgttgatcttcaccttggaacccacaatgctggggaaaagcacgttactgtcgagtacatgaatgaggaacagggcaatgcccgcctgcaatgcctgtataggcgtacccgtagccagtgttaccaggatgataaggatggcggccgttaagatccctacataaggaatgatattaaagatagcggccattacgcccagcaggatggcgtatttaataccaagaataaagaacagggcggtattgagaacggctactatcaccatttctatcatcaggccgcctacatagcttttaatgatggtgcgggtgctggcgatgacggtgagtaatttttcgcggtgctgttcctggaagatcttgatcaggaaagataccagtaacctgcggtagaagaggataaagaaagcatacaggaatacaaatacaacgaataccagcagggaggaaagcgacaggaatgtttgactgatgaagctggtggcggttccgagggtacccatcatcgctttttccacgtagctcatttgtgtgctggaattgatatgaaacttagtattgatccaatcttgggtggaatctatcaccagcatgagcttttgttccagttgcgggaaatcggagatgaaggcttccatttgtttggcgagtaggagcattatcagcaggatggcgatgataaacagcaataccgctatgatggctgccatcccccggggcaggcgccatttttccagctgatggacaacgggcagcagcatgatggcaatgagcatggcaaacatcaacggaacgatgataccactgccaacatgagctatatagatgataaggataatcgaaaacagggtaaaagtgagacgggcagtaaacggtagtttgatctcgttcatagaggtagtgcttttatcaaagatattaaaaatcaaagtgtataacattagaatgctgattatacatttgttacggtgaaaaggttgcagttgcgcaccgcttttattattttacggacatgcccgtaaaaattcaagcgttatgaaaaaactgtttgcccttttgctgctcgtttgcggcagtggatccctttcctttgcaaaacccctgccggctgacaccttacctgtccgcggtttttgtatagcggcgcccagggcggaaggactggctccgttcctgagatttatcgatacagaactggcgccccggcacatcaacaccctggtgctgcgcgttgattttaattaccagtttaagtcgcacccggaactgcgtgatgccggtgggttaaccgaacagcaggtaaaacagctggtgcaaacctgccgtaagcataatatccggctgattccgcagatcaacctgctgggacaccagtcgtgggcgggtacaactaccaacctgctgaaggtgtatcctgattttgatgaaacgccgtgggtaaaaatgccggcgaaatatgtatggccaaatgcagatggattgtattgcaaaagttattgcccgttgcatccgggggtacataaagttgtgtttgagttggtggatgagatctgtgatgtatttgagagcaccgcttttcatgccggcatggatgaagtattttatattggcgaggataaatgtccgcgttgcggcggccgggacaaggccgaattatttgccggggaggtatggacgatccggaatcacctggcgcagcaggggcgtgagctgtggatgtggggcgaccggttgctggatggcaagctgacggggttaggcgcctgggaggcgagtatgaacaatacacaccgggcggtggacctggttccgaaggatgtggtgatttgcgactggcactacgagcgtccggataaaacgccggtatacctggcgatgaagggattatcggtgattacgtgtccgtggaggatgccggctaatgcgaagctgcaactgaaggatatgtatgattaccgggcgagtgccaccaaagaaatgaaaccccgtttccagggaatgatgcaaacggtttggtcggatgccgccgggttcctggatgagttttatggaacgggcaagccgcagaaagataccgtgaatacgagcgccaattgtttccgggctgtatttactaaatagataaaagaataaacggaatgacatcattggtcattccgttttctttttaataatgttttttgagcagcggaataaatatttcagagtattgagggccgtcgagcgaaatgaagaagtggttcccgctcattttgaaaattccttccttacagttcatgctgataaaattatacatcggcatacctgctgtggcgaagtccattggcaccggcagtttgaggtagttgccacctgctatccgttttgtggcgagataggagtggtttttcgtcagctggatatgcgcgtttattgcagccgttggaatcaacagtccagcgaacatagacagcttttcatagttggttaccggtacggcgtcgagggtacctgtaatgatcctgctttgtggcagatcgtataatgtctgcatctttttaaacagactatgataggtgttcatgcgggcgatcatttcagtgatcgggtcctggccccgtgaaatgaaggagtagtacaggatgctgtccggcattctgattttctcacagcgatcataattgaacaattcctggaatgcttcactacctacagctgcggtgatggttttagtgatctgcagggtcctgttttcattgggcaggatgatgatgcggcggaaatctttgggactttctttaaagtgtagtttaaaggctttgctgaaagccgcggtggtggcgtatccgcaatactcgcttatttcaccgatgttatagccactgtgccggagcaggcctgcgccgagttccaggcggtgtcttttaacatagtgccagaatggttctcccatgtaattcacaaagttgtgatagaagtaggagtaggagatgccgaggcgttctgccacatctctgatattaaagggatcacttacgtgatcatctgcataagataacccttgtaaagcaaaattttcaagttgttctttggtcaaaagggcggccataaaatatgagggattttagttgattttcattggatccggtacatgctgatttacatcctggataagcagatcgctacgtgaacattatccctaatttaatttttttatgattaccggagaagtaaatttcaggatcattttattaagttgattttcaatatgatatattttgtatttagcatataaatttataatatgtagaaaaattgttgcctggaaggaggttccggaggagaaaaaaaacagaaaaagctaaaatggacaaaccgttaattacgggaatgaatatctttaacagtcatgttatgtttggatcatcagtcgggcattcccatagttttatagccattaaatgattttgtcctatcaatcctgttatggagttgcggccttcgcaacaccatttgccggtggtttagcatagttgattgatttgattgtataaccttttatgttatggtagccgtcatcattgttttagcgttattgttgctgctgggttgggccatcctgtaccaccatttcagggccctgcgggtagctaatattaacctggtaaaacaggcgcagaaagaggcttcgttgcagttccagctgcgtgaggccagggaaaaatacaataagctggaagagaagctcagaaaggtacaatatgagctgcataatggaaaacaaaaagagagtcagcgctgaaaataacatccacctggtattgatgtcattgttttcgggtttgccaatatttagttaggtttgctggcatgcaggtagtttttcagattacatccggtgagcgggatgcacaattgtctatgctcgggcagctcaataatcttcttcattataccaacgaacgtcaaacacgtgtagccatagaggtggtagtacatggtcatgcctggaatttactgctgccggagggccaccctttccccgaaaagatagcgtccctgcagggccggtcggtccgtttccttatttgccaaaataccttgaacagccgtcagctggcagcggatcagctgtttccctttgtggaagtggtgcctgcagccatagcgcaccttatagaaaggcaacaggagggatgggcctatataagatgttagtttaattgtttatgagttaattggtttattagtttatttttacatttttaaagtaaagtgccgggaatagcggttgaaagtttgggagggcggcaccaaataaaaattgcagtaataacgttaaatggatgcacgaataataaggactaacctcttaaacttaaatacattgaaattctccaaatctaccggaatactgttgttattcatggcagttccctttttcacctttgcgcaggactggcatgtcggcgcttttgcaggtatcagcaactacagcggggatcttacccagcaaagggtggatatgaaatatacccggccggcgcttggcttgctggtgagaaaggatattaaccgttacctcactatccgtggctcttttacctggggaattgctaccggcgccgacagcaccaactcttccaaagacctggtggcccgtaaccttagtttccggaccaatatttttgaaggcagcctgattggtgaaatcaacttttttgatctcgacgaaaaagggtttacgccttatgtgtttgtgggtgtaggtggttttggttttgatcccacttctaaagaccagtcgggcaaccgggtacggcttcgtcccctcggtaccgaaggacagggattaccgcagtatcctacccgtcagccttacgacctgttttccttttcctttccgtttggagcgggtgtaaaggcaatcatcaatgataaatggacacttggatttgagataggacttcgtgctactaccacagactatatggatgatgtgagcactaactatgttgatcagaataccttgctgacctaccgtggccaaaaggcggtagatatggcttaccgtggcgatgaagtaaccggcaaagtggcgccgggaacatatcctgcagatggtgctatccgtggttctgacaagcataacgactggtatgcgttttccgggttcaccattacttaccgtttgggtggtggcagtggctggggtaaacaaaaagctacccggtgcccgatactgagaccgtaatcagctgatattcacactatttaatactttatttatccttttaatcccggcatcccgccgggattttttttattggcatagttgttgaatttatgagttcaaacaggtactaatgcagccaccagcttatggcggatcgcagaatcacaaatcgcggagagagtaatgaatcaacagccgcaagaaaataagttggtgtgcaactgcctgttttaactaacgaaaaagaagtgccatgaggaagtttttaaatatagcttcagtgatgttgataacaggttcaatgagcctttctgcacaacaaaggccgcctgcaccaccactgccacccaggccaccggctccggcacatttaccacatccgccggcgccaccagtaccaccgggattgccaaggcctccaacgcctccgcatcaccggccaccggctccgccaacaccaccgcatcatcataaaaaaccgtataaaaagcattacaagaaaccgcgtaagccccggagatattcttttatcgcatatccgggttccacttatgttgttacagatgccagttttgcccggtatgcgggttaacattaacaacacaccacaactattatttgccaaccgatcttgaactaaaaaccaaagaaacatgaaaaaagtactgctgttgatgctgcttattggcggcactgtgctcaccacgtatgcacaaaggggacatggacgtggccacggatatggacatgggcgcggacatgaccgttatgatgatgaccgctgggaaagatgtgagcgacccaggagagtgtatgtacgcgacaggtatgactatgactgctaccctcgtcaaagagtggtatacgccagaccggcttattaccccgctgtaatacctgttcccgtgccagccccggtacgctactacccatcaaggccaagggccgtattccacgcgggtgttaccatcgtgaactgataactgaaaatggaataaatgagatgcctcccatatttaaaatggggggcattttttattgcggtgcgggatggttacttttgttgattggtaataagattcaaacatggcatataaaaatctcagacactttatagacacgctggaacaggcaggagaactggtacgtataaaaacttatgtggatcctaaactggaaatcgctgaaataacagacagggtcagcaaatcgccggatggcggcaaagccctgctgtttgaaaataccggtaccgacttccccgtgctgattaattccatgggcagctacaagcgtatgtgcctggcgctgggcgtgagtgaactggacgatgtggccggtgaaattgaaaatctctttaaattattatccaaaccaaaggaaagtatacttgataaactggccctgctgccaaagctcggacagtttgcttcctggatgcccaaagtagtaagtggaaaaggcagttgccaggaagtggtaatggccaacccggacctcagcaaattgccggtgcttacctgctggcctaaggacggtggtccttttatcaccctgcccgtaatccataccaaagacccgcttaccggcacccgcaacgtaggcatgtaccgtatgcaggtatttgaaaaagatatgaccggtatgcactggcataaacataaggtatccgccaaacacttcatggaatacaagaagctgaataagcgtatgcccgttgccgtagtattgggcggagatcccgtttatacttactctgctaccgccccgctgccggaaaacgtagatgaatatatgctggccggctttctccgcaagaagaaagtagagctggtaaagtgtatcacccaaccggatatagaagtgccggcagatgccgattttgtgattgaaggttatgtagaaccggctgaagacctcatctgggaaggccctttcggtgatcataccgggtattactcactggccgactggtaccctaaatttcatgttaccgctatcacgcaccgcaaagacgccgtatatccgtcgacgatagtaggcattccgccgcaggaagatgcctggataggcaaagccaccgaacgtattttcctggcgccgattaaaatgacactcgtgcctgaaatcattaatatggaaatgccggtggaaggcgtgttccataacctggtgattgcacagataaaaaaagactatgccggccaggcgcagaaagtgatgaacgctatgtggggcgccggccagatgatgtttaacaagatcctggtggtaacagacgacggcacaaagatcaccgactataagcagctggcacagtatgtcttccaacacctgaaccctgctgctgatatatacctcagccaggggccgatggacgtactggatcactcctgttccaagatgggctttggcggtaaaatgtgtatcgatggtacccgcaaatacgaagaagagcaggacaccacctttatatctgttccggcgccgcggcagctggatacagccgccatcatgcagcagttcccggaaatcaaaggcatcaacgcttcgctgctgccactggatatttcctgtatcctggtggcagtggaaaaggcccgtccttcgcatgtacgggagctgaatgagcagctgtacaccttaccggcactggcgggcattaaaatgatccttttcgtagagcataccgtggatgtaagcgatctggcttctgcgttatggcgtttctgcaataacctggaccctaaacgcgacagctttattgtccgtatcccttccggggaacccggtaaatatattggcggcattggtatggacggcaccctgaaaaccaggctgctggacaattttgagcgcgactggcccaatatcattgtggccgacgatgccactatccggaaagtggataccaaatggcctgagctgggtatcggacctttactgacttctccttctctcaaatacaaacaacagatttatggtgaagaagcggtggtacaacagtagttacctgctgctgatcctgttactggccggcagcctgcgggcagccggccaggtaagtgctgccgacttccgtttcctggataagctggaaggcacctggaagatgaacacccgcaaaagcaccatcgtggaaacctggagccgggtcaatgactctacctggaaagggaaaacctggcgggtagtaggagcggacagcgccctgcaacaatccatgcagctggtgagaagaggaaccggcatcttttatattccagcctatgaagggcaggacaaacccgccaccatacacctgaaactgcgggttttaaaagccattggttttgttgcagaagacctgaacaacgatttccccaaaaaaatcacctaccgttttaaagacgccaaacacctcgacgcccgcgtggaaggcatgcgggacggcaccaccgaggaatacattttccagtataccttctccccggagtaaagtttcccgattgcgtaaatgattttcccgcttcgagaaagcggagtgcatggctgtacctacttttgtgtaacacacacacgatacacagcaccaagatattctcaataaagcaataatttgagttggtcgtacaagtaatgccgcgcctgttcacagggagcggcttttttgtgcggagggagggcggcgccttcggcgccttttgtcttggagcaggattacgctgattatgttgattacgctgattttcccaccttttgtttagatttttttagggaaggatgggaatgatttttctgcattttatttgattagaaaaattttcctggtattgtgataaaaaaaatgggagatagaaacagacatctctgtttctatcccccaaaatatttaaaataaaatgtgggaaaatcaatctaatctctccccaaaaaaatctaaaacaaaaggtgggaaaatcagcgtaatcaacataatcagcgtaatcctgctccaagacaaaaggcgccgaaggcgccgccctccctccgctacttatgaatctccgatgtgaagttgaattgaatgtcagggttgttggtgcgctcggtgttaaggtaccattccgattgcgccaggtatacgatatggccgtccttgtcctccacgatgttggaggatttgaagcggatgaattcctcgattttctctttcggaccggtgagccagcaggccttgtagaaaggcagggtattgaactggcaggcggcgccatattcctggagcaggcggtactggattacttcgaactgcaggtcgcccacacagccgatgattttgcggttgccaccgtgctgcgtaaataactgtgccacgccttcgtctgtaagctggcggatacctttttccagctgttttgttttcagtggatctttgttcaccagttccttaaacagttcaggagagaagcttgggataccggtgatgtaaaagttttcaccttccgtaagggtgtcgccgatcttgaagttgccggtatcaaacagccctaccacgtcgccggggtaggcatcgtctactacgttcttttcgcgggcgaggaagctgtaagggttgctgaacctaacgtctttgtctaaacgaacatggtgatagaatttattcctttcgaatttaccggagcaaacgcggaggaaggcgatacggtcgcggtgacgcggatcgaggttagcatggattttaaaaatgaatccactgaacttatcttcgtttacgtctacttcgcgggtggtagcggtgcggttacgcggaatgggcgcgatgtccacaaaggtatccagcaggtctttcacgccgaagttgttgacggcgctgccaaagaaaacgggcgccagtttaccggcgaggtactcttccctgttgaaggtatcgtacacgccttcgatcagttccacgtcgccacgcagctgtgcggcatctttttcattgaagtgttcatcgatgtagctgctgctgagatctgtgagcggtactacgtcttcgtctgttgctttcttgttgggaaggaaggccacgaggcttttatcgtacaggttgtaaacgcctttgaagtcgctgcccatattgataggccagctgaggggtcttacccggatgttaagtttttcttccagttcatccaggaggtcgaacgggtatttaccatcgcggtccattttgttgacgaagatgatcacgggcgtatcgcgcatgcggcatacttccatgagtctttccgtttgttcttccactcctttcacgcagtcgatcaccagtaccacgctgtctacggcagtcagcgtacgataggtatcttccgcaaagtccttgtgaccgggggtatccaggaggttaacgaggatatcgcggtattcgaaggtcataacggaagtggctacggagatacctctttgcctttcaatttccatgaaatccgaagtggtgtgcttctttattttattggacttcaccgcaccggctgtttgaatagcgccgccaaacaggaggaatttctctgtcagcgtagttttaccggcatccgggtgagcgatgatagcaaaggattttcttttactgatttcgttagcgtacttcataaatatccgaaaaatggcagcaaaggtaactaaattttttgtccggctatatttcgtgtttattggcgctgcccgtgccgataaatccgctaaatttggaatatgatagcaacccttaaaatattatggaatagtttcaaaatggcgatgcaggagctgcgggtaaataagctgcgcacttttttatcgttgtttggaattaccattggcatcttctgtatcatcgcggtatttacgctcaccggtagcctggaacacaatatcagaaaggatctggctgacctgggcgacgatgtggtatatatgcagaagtggccctggggcggtaatggggaatatccgtggtggaaatatatgaaccgtccggagccggagtataaggacctgaaacctatacaggataaggtgcagagcgccagttttgcttcatttaattttgaatcgggcaataagaaggtggaatatggggatgattatatggatggcgtgacgatgatggcggtgacgaacgactttgaccagatacagaccttacagatcctggacggccgtttctttgccaacagtgaaagtaacagcggcaccaatgtggcgatcctgggctttactatctgggatggacttttcccttcgccggaagcggctatgggcaaggtggtgaaagtagcggggagggatgtaaagatcatcggggtgttgaagaagaagggagaaagcatgattggcgggatcgggtacgacaatgccattatactgccttaccggtttgcccgtacggtagtggatgagcgccggtttgcggacccatatatcctgataaaggccaaacccggtgtaagtatggatcagctgaaagatgagctgaaaggggtggtgcgcgcgtctcaccggttaaggccgaaggaagaggatgatttttcattgaatgaaatcagtaccgccaacgacagtttgaacgcgatgtttgctgcgatcaatatgggtgggggaatgattgccatctttgcgctgatagtgggggcttttggtattgccaatattatgtttgtaaccgtaaaggagcgcaccaacatcatagggctgaaaaaagccataggagcgcgacggggcattatcctgatggagtttttgctggaagcggtgagtttgtgtttgttgggaggaacttttggcttgctgctggtttatcttcttacagtaattattaatctgtctggtacctttgagatggtgctgtctgcgggttctgtgatattcgggttgagcatatctgccctggtagggttgctggcaggctttattcctgcttatacggccagcaagctggatccggtggtagccatccgcagcaactaaacaggcatacgtaacaggcaacagcttagctgttgtacaggcggggttttcccgccttttttattaattttgcgccttatgtcggttaaaatattagctatagagtcgtcctgtgatgatacaggagcagcagtcattgtagacgggcaggtgttatccaatcatattgccggtcagaaggtacatgagcaatacgggggcgtggtgccggagctggcttcccgcgcgcaccaggagaacatagtgcctgtagtggatattgcgctgagaaccgcaggtgtgaagcgggaggagctaagtgcgattgcttttacccaatcgcccggattgatcggttcactgctggtaggcagttgctttgccaaatcgatggcgatggcgctggatattcccctgataggcgtgcatcatatgcaggcgcatgtactggctaactttatagatgatcccaagccggactttccttttttatgcttaaccgtgtctggtggtcatacccagatcgttttatgtgaaagtccgcttagcatgcgggtaattggtgaaacgctggatgatgctgccggagaggcttttgataaaagtgccaaaatattgggtttgccctatcccggcggcccgttgatagataaatatgcgcagacgggcaatccggcgcgctttaagttccccgagccccggatacccggtctgaacttcagtttcagcggattaaaaacggctattctttatttcctgcaggagaaccagcagaaagatcctgcctttattgcgcaaaacctgcctgatatctgtgcctccatccagcaccgtattgtgagtatattactgaacaaggtggtgaaggcagctgaagaaacaggtatccgcgatattgccattgccggcggcgtgagcgccaacagtggtttgcgcactgctttaacggaatatggccggcaacaccaatggcggacatttattcccaaattcgaatattgtacagataatgcgggtatgattgccattacagcttactataaatacctggcgggtgactttgcgtcactggatgcggtgcctactgcgagagccgctttttaatttcattaacaaggttggctaaaaacgaactgctaattgctaaaatcctattctaaatcaatagtatatcggtttagctttaagtcgtgctttaggatcgccttcggcgatgttaaattgtcttggagcaggattacgctgattgtactgatttattgatttttacattacttattatctatgaagagaatttttagcattttactggcacttattgcggtgggaaagtttgcggtagcacaggaacctgtggcgcaaacggagtggaagaatcagaagtattccatgtttatacactggggcgctatttattccacgctgggaggcgtttgggagggtaagcccgttacgaagggatatagtgaacagatacaggcgcatgccggtatttacagtgatacgtatggagacgtggccaaacagtttcaccccgaacaatggaatgctgactcaattgtgcggctggcaaaggcggcgggtatgaaatcggtggtaatgacttccaagcatcatgatggtttttgcatgtttcatactgcgtatacagattataatgtagtggatgcaacgcctttcaaacgggatgtgctgaaagaattatcggatgcgtgccacaggcatgggttgaagttcgggatgtatttttctttgatcgactggcattttccacaggcgtatcctatttccagcagtaatagcgatcctattacccccgagcatcatgaattcaataagaagcaggtaacggagctgatgaccaactatggcccggtatccgagatctggtttgatatgggatcactgacagcgcatcaaagcagggaccttgctgatattgtgcatcgtttgcagccgggttgtatggtgagtggccgtttgggaaatgatgccggtgatttttgtgtaatgggagataaccagtatcctgactataagattgcttccgcatggcaaacgcctgcttccgtgtatgatgaaacatggggctatcgcagctggcaggagcatggcaaggcggaagacaaggcgcatgaaaaactggaggggctgattaaagtggtaagccgtggcggaaactacctgctgaatattggcccgcgtggcgacggttcggtggtggactttgaaaaagaggtgctgctgttaaacggcgcctggctgaaactcaatggtgaagctatttacagcgctgctgccaacccgtttgatactaccttcgcctggggcgaagtgactacgaagcccggaaaattgtatctgcatttactgcagcagccggaacatggcactattatcttaccaggactgaacagtaagatcagccaggtaaccttattgagcaatggaaagaaagtacccgttaaaatatctgccaaagatggtaacacctatctccggttacccgcagattttaagctcgcagataaagacattgcggtgctggcagttgcctgcaaaggacctgtagcgattacaccggttcacttattacatcatgctacgcgtttgagcagggataatgctacgccgttattcagcttctccggtattgattatgaaagctattaccgcagtgaggtgggtgagtcgtgggcatttaccacaccgcgccctgctgcgttggagctggtgtatagcgatgcagagaaaggcaaacgaattttgctgacactgaatggcagcaccagggaagtgttgctggatggtggtgttaccagtccgctgaaaaatgatccggcttccctgcagtggggaccaatgtacagcgcgggtcctttctggtccggtattgatggcacgcatggaagtgtgaaagatattgatccgtccaaaccctggcccaataaggataatgctgcgtggacactgcacagtgactggaagaatgatgcacctattacattaaccgcagataaaagtgtggccagttatattttacaggagatcacggcgccgaaagccggtgattacctggtaggttttaatagcggagatggtattgcagtatatctgaacggggaagagcagttattgcacaataacccggaaaggggaggtacgcaatcggaagtgttattattatctttgaaagaaggaaagaatcagctggtggccaaattctacaatcgctttgcaaagcaggcagtagtgggcatcagccgtaatgtaccacaggtgttatatgttcagcagttgccgcaacgtacaggcggcagcggtaaagtagaaaactgcgtgatcaggcaggccaacccggtatctgtgcaccgtaatttacggatgcctaacctggcggtggtgttagattcaaaataaagatggcaaatacattttttaaatttaaacagtttacggttcaccaggggcattgcgccatgaaagtttgtacagatgcctgtatacaaggggctttcacagcgcagtacctggcggacaacgatataacggcgccggctatactggatttaggcgccggtaccggcctgctgagtcttatgctggcgcagcaggtagatgctgaaatcacagcggtggaactggacgccggagccgctcaccaggccatagagaattttgaagaatcgccctgggcgaaccgtttaaccctaacccggcaggatatacgaaaactggatgggttagtgaagtatgactttattatcagcaatccacccttttatgagcgtgcgttgaagagtgggcaggcggagaaagaccaggccatgcatgccaccaacctgagctaccaggaattgattgcggcagtggaccagcaattggcggcgtcgggagagttgtcggtgttgctgccttatactgcttttgaaggtttccgggtattggcgctggcagcagggtttcatttgaagcaggcgttgtatatccggcagagtgtgaaccatggctttttccggaccgtgggtattttttcgaggaagccggtgaatactgtgatcagcgaactttccgtgtatgatgcggagcgtgtatatacgcctggatttatcgccttattacggccatattatttatacctgtagattttttgtattttggcactctatttatcctgatatgcttcgagtagccagaatttgtttggtgtttttattgttgcccgttattgtgcatgcccagaaagagatcaatatctggtactttggatataatgccgggcttaacttcaacactacccctgccaccgttcttactgatggacgaacttacacccgcgaaggggtagccaccatttgtgatggcgccaccgggaaattacttttttatacagagggatctaccgtttggaatgcccaacatggcattatgcccaatggaactggtctcatgggcgacccatccagtgtgcagtcgggtattgccgtaccatttccgggacatccggggcagtattacctgtttactacaatgaccaataaagggttccgttataatatactggatatggcgctggataacggtaaaggtgatatcattccttccaccaagaataccccgttgctgagtaatagtcagagtacggagaaaatggcggctacccggcattgtaacgggagggactattgggtagtaacgcattccgccaatagcgcaacctttcatgtatacctgctttcccccgccggattatctgctgccactacttatacaactggtgcagttattcatccgggaggctgggaagaaaccggtcatatcaagttttcgcctgacggcggcactatggtgcattccctgggatctatccgtcagggcgccatgagcgtagtagatttgctgaagtttaataacagcacaggcgtgatcagtcctccttttgcttcgctcaatattattttcccacttggtattgaatttactatcagcgggaagctgctgtatgtagtgagcatgaactatctgaattggggtaagttataccagtatgatttgacggcgcccaacatcaatgcttcccagcaaacaatagtcaccaatacggatgatatccagatgggcggacttcagatggggcctgacgggcatatttatatggggtatgagcagggatactacgggggataccggtatgtgggtatgatccataacccggaggtgaggggtgtaggttgtaattttgaacgggatgcgatagatatggagcctcccggcaccgggcaacacagaacttctgtatcttttcccacatttgtaaatagctttctttattttcctgcggactttactgcatcggacctctgtagtcgtagccctgttttcaggctgaataatgaagtagatgtaacgagtatattgtgggattttggagatggaactacttctgccgacctgtcgccccggcatacatatgccatcgaaaaaaaatataccgtaaaagtaaaggtaacgcgtcgatgcagtactgatgagaaaatacaggatatcatccttggcagtaagacagaggaaagtgttgcaaaaagtatttgcagtaacgtcacttatacgctgccggatggcagggaagtgagtaccgccggcgtttacgttagtacgctgaaaagattgagcaatggttgcgacagcattattaatactaccttaaaaatattgccggtatatcagttgacggagaaagtgactatctgcagtggacaggagtaccagttgcctgatggaagaaaggtaaacagttccggcagctatacatcttccctgaaaacttaccagggctgcgatagtatcattaccactgagctgtatgtgccggagaagaactatctgcaggatgctgttatttgtgagggagataattaccgcttaccggatgggaaggtggtgaccgctgcaggctcctataatagtattcttacgtcctcgttgggctgcgacagcattattatcacaacattggtagtaaatcccgtttatgctgccgcggaatccattagcatttgcgatggcgatacttaccgcttgccggatggccggactgtaagtgttacaggacagtatacttcccgtttcaagagtgataaaggatgtgacagtcttattgttaccgatctgcaaatgctaccccgttataatattgcgaagacagctattacctgtgagggagaaccttatatattaccggacgggcggtcagtgagggtttccggtacgtatgtatcttcgttcgcttcttatcatggatgtgatagcattattaccacccggcttactgtaatgcctgtttacagccaggaaaaatatgataccatttgcaatggacaattttatacgttgcctgacggcagaagtgtgagcagtaccgggcgttatgtgagcgcattgtttactaccagtggctgcgatagtacggttattgtgtacctggcattaaaagagaagccgcaggtaacgcttgtccctgaagtgtgcttgttttccggccggccaaccgttataacgttggttccgggatacgacaaatatgaatggcagagcggattttccgggaatgtttacgccatccgttacccgggtatttaccgggtggctgtttccaatgaatgcggtgtggttaacctgcaaacgttggtgaaggaatgtgcttctgacttgtatgtccctaatgcatttacgccgaatggtgatgggctgaatgatgtgttcaggcttcgtcagccgaacggacaggtattgctggagtttaggatatttgaccgttggggcgtggaaatattttccacgactaacctgttgcagggatgggatggtacatataaagggcagttgcaaccggtgggagcctatgtatatttcatccgttataagaacattgatgggatagaaaaacagctgaaaggcgctgttaacctgttgctatagcgctccttttgcatagtcttcgaggtaagcatacctttcggttagtttgccattagcgacgatcgttgcattactgatcatctcgctgtttgtttgcagtagctcatcaaaaacatatttcatcagctggtccccgaaatactgcgaggcatcccgaggcagttcgttggggagattgcttacgcacatcatgtctaccgttccggggagatagggttctgtttgttccatcttatcttttgtaacgccgtacacggggctttcgatagtactgtcgccgaggttgcagggaatggagccgttggtatcgtctgtgatatcggcgatgacctgtatgcggaagttttcttttttcagatcatctggctggaagagcggcgggattttctggtcccagtagatcccgttcatgagtatatcacttacggtcacatagggaaggaagcggcattcgtatgcttccggatgtgcgtggaagtcggcccggctgtatgttttatcatctttccgcagatagagttcgcctgcttttagttgagtatataccgggtatgaataggtattgatcaggtattcttccggcggaagatatttaatgccgagcaggcccatgatttccagtgcgccggcggctacgcgtccggagccggtgattactattttcagcggaggcagtttgatgccgaagtaatgattgatgagttcctggaagtcgtggcacgtgtgcactcttttaaaatgaaaggactgtgttttttccccgtatgccatcaggccgttatgcgcgcctacgatacctgcaaagaagccgaagcccaggattcgttgtccgtcggggtgtacgaggcattcataatctatcagtgtgatatttttttccaggatggtttgcagcatgtgttgattatgcggctgtttctttttggtgtggctgaagaagaggtatgtttttcctgcgatcagttcatcggtgggaacttctttgatgcccagcagggtggtgcagtgggagaggtcctcctgcagcgggacgcctgctttttcgtattcatcgtctttgaagcatcgtaacggggatggttgtacgtagatttgtacctgtggaaaatgttgcatgatccattggcattgtttgggtgtaaaagctaccctgttatcatgcgggtgtttttcttccctgataagtccgatgtgtatcttgttttccatctttgaatttagggtattttagtcatttgtgaactcctgaaacgccctgtttatgcggggtgcgaaatttttatatacaaaaatgtaaaaattatttgcagattaaataagagtttctatatttgcatcccgcaattgacgcggcgaagttcattagtaagattgcccagatggcggaattggtagacgcgctagactcaaaatcttgttttcgaaagggagtgcaggttcgattcctgttctgggcacccaaaaggcttgtaagtaattgacttacaagccttttttatgagtgtcaaatttcccggctagcaaccttcaatacagcatttgctgaacgttaagcacgcactttaacttcgcctaactaaaacatcgcaattgaactaaagtggtcatttaaacttttcagttagtattgtccaattttttgccagaaataatttctcttcacacggtgtctgctcattaccggtataatactactgccggtactcataaaggcgattgtgcgcatcataaacttgttcaaccattagtcgccagctttcgttataatggttaaattatatgaggtcgcaaaccggaccggtcatgcacagcgtgttaacgatagactcggggaaaacgcaatattttatatggaacggtactaaaaagatgctgacctttaaattaaccctgtcggacacagttggctttgagggatttgacttccaatcctatcatttaccgcagatccaggcgtatgctgcgcctgttccaaatgataacccgctgaaaacgcatttggattcggctgtccactacggcaccatcgactttatgcttacacatcatttagtaggcctgtcgatcggcgtggttagcaacggtcataaacatttttacaattatggtaccgtggagaaaggcaaaactcagctgcccacttcgcgcactgggcttccgcagttactgcgccgtcttgcccgataaaaagaccggtatgatctggctctcaaaccggtcagaccttgccgacgatgaaatcgcagtaatggtcgatcagatattgtctgccgctaagcaatagtctaaattcggattgatctatccaaagggtggatatggcttttggggcttgttcaattaaatataatccttgataacctgaaatgaggagttgccttcttcatcaaaaatctgtttcccgcaatcctgacacacatcgtcggttatcttttcgccccgttttacctgccagatattcatactgccacagtcgcagttcacggtataaagcacctcgccacttaaactgccgaatgcagtaaatctccagacaggatctgattgctttttcaatccggcagcatcactttgctttatcaaaccaatatagtaactgtcattcccgatatctaataaaacaaccgttaaaccggtctttttttgttgtgcctgaaaacttttcaacaggaggggtacgctgtctccggcattgatactttccttcctgacagcatctcttagtttaccatatggagtttcaatgtcaatacttgttccgggtaacaggaccgctgccctgccctgaaggaatttgccgatctggaactcgtgttcttctcccttccaatccacctgtagcaatatgccgtgatccaacagataggcgagtaaatcctcatggctggtaaacgattgctgtaccatagcctcctgttctttaagatccatgagcaattgactggatttcatattcatattgttatgcgctttttttttgttgtgtcagtctttccccttcctgaactcaggtctattttaattcattttttgcgtcggggctaatcattttaaactgttctatatcctcaccatgcgacaggataattgattctgtatacatgacttttcttaaacaggtaaatagattataaaggcgcatcaaggtaacctataagggatgctgaatacagcaatatactaattgtttcgaaatgaatcaagttgttttcaaacaagggataaatgtcttcaggtggtactgttatgggtttcaaagctgcaagaattgccgcctggcacatcatcgacatgattaattgggttatatcttagcgcacggaaagaaacagttccccggttccaacatcctcctcacggcgacggtcatcaccccaatatcacctcaaaataaaaaattgtcattttgacaataattactattatgcactctgaatgatgagaatagaccttaatcatgtaggacatggggtaaattcgtagttcagccagtcaaccaggtcataataagaagatagaaggaattgtcggtaattcttgtgtactattttcaatttcacgggatgagaaaatttgtaatgcactgtttgctgcttattgcagcaacgttccacacaccgggttcccaggcccgggataatcgttatcatgttatatcatacctgggcatagaacagggtttatcgaataacgctgtgcgctgtgtgttccaggatcacaaaggatttatgtggtttggcacctatgatgggctgaacaggtacgatggtaacgtatttaaggtattccgcaacaggttcaacgacagcagttcactggtaaataactgggtattcacgattaacgaggatttgcagtataaactgtggataggcacgcgtcagggacttaacatatacgatcaggtaaccgggaaattcagcagtgtacgttaccaggtaaccggtacaacaagatatgagccgatcacggcagttgtgcgcgatattaaaaaagatgcgaaaggaaatatgttgattgggacagagggactcggcctgctgttttgccccgccggaacctatactgctataccgttgccattggatgctgatggggtgcgcctcgtttcatatgatgcaggagccattgaggtggccgctaacggcgatgtatggttgtttgtgcaggggaaaggattgtgccgcatggataaaagcgctgcccgggttagtttgattaacggaactaatccgacgggcgactgtataaaagccgacagggacctgctttggataggtacaccaaatggactgcagaaatactccattcccgataaccaataccaggagagctatacggaagaaaacggaaaactctcttacaacaaagtatccggcctgttcctcgacaaatgcggcaagctgtggattgccactaatggaggaggcataaatatcattcatacaaaagacggaacggtagcggagagcatcccctcgggcaatagcaactatacgcttgcaagtggctcagtaagcgcaatttatgaagatgcggatggtagaaagtggatcggaacactaaggggaggcgttaacatcattgatcctaaaaaagacaggtttcagtctttcctccacgacccactaaacaagaacagtcttgtcagcaatttcattttcaccttctgcgaagagggcgacggaaccatctgggtaggtacagatggtggtgggctaagcaggtggcagcgaaaagcaggattgttcactaacttcgttcatcaggcaggtgtacctgcatctctcagcgataattttgtaacaaatgtgcgatgcgacaatgagcagcatatctgggtttctactttctggggaggcatcaaccggtttgacaaaaaaacaaatagcttccggcattaccgcctgttttataataacacccaaaaagagagtaaaactgtttacctgtataaagacaacaagaatacgctatgggctggaacctttggcagaggttcattatataagggcgcactgtataaatatgacaggcagcaggattctttcagactctttgacgacaggatcagggatctgtttacgatgaacgaggaccggtccgggcaactgtgggcggggaatcttcgcagcctgataaagattgaccctcaaaacaaaatgcatacctcctatacgctgggcaacccggtaagagccattcatgaagacagtaaagggcgtttctggatcggtaccgaaggaggaggcctgattttatttgatcgtgcgcacggtaaaatactggaacgctatactaccgccgaagggctttgcaacaatgcagtactcaatatcctggaagacgaagccggagacctgtggctaagtactttttatggcctctccaggttcaatgccacccggaaaaattttaccaatttctaccagggcgatggcctttccagtaaccagtttaattacaatgcagcgctacggcttaactcgggcgaattgatgtttggaggaattaaagggctgaacatcttccggccatcaaatattatagcatcaggcgaaaagcccagaatgcttttcaccgatatccatattaacaatatgcctgttgggcagcgaccaggctacattgccaaacggctgggtgacgacatacggaaagtccgggtgccctaccgcgatgccgtcttttctttcgacttcaccgcgctggattattctacttccgataagatctcctatgcctactatatggatggctgggataaaaactgggtccaggccgggaatacaagaactgccacctatacacatcttgcggcgggtcattacacattccgggtaaaaagcaccagcgcagaaggtcagtggatcagtaacgaaataagcctggagataatagtattgcctccctggtatgacacctggtgggcatatttgctatacctgttcatggtactggcagtgacggccatttatattacctataaaacaaaacaacgcaggctcaggtaccaggttgccatggcaaatttgaatacggagaaagaaagggaactcaatgaaaagaagatcgccttttttaccaacgtatcacatgagttccgcacaccgctcacgctcattattaatcctgtgaaggacctgatgacagagcaggagcccggcggaaagcaccatcgggagctgactaccatataccggagtgcccgccggctgttacggttgctggatcaattgctgttgttcaggaaggcagacagtgatatagaccggttgaagccagcccgttttaatttcacggaattatgccaggaggtattccagtactttgaacagcaggcccagtcggccagtcagcactattcatttgtttgcgaaagcgaggcgctatggatatccggtgacagggagaagctggagatagcgttattcaatttgttatcgaatgccttaaaatatacccctgccggtggcagcattgaaatgaaactcgtttgtgccggcgaccaggtggaaataaccattgcggacactggttatggaatatgtgccgacagcgcccatcacgtatttgagaagttctacaggtcggagggcaatggtcatacacaacaaccgggattcggtattggcctgtacctggtaaaacagtttatagcgctgcacggcggcaacgtcaattttgaaagcgaagagggcaagggcactgtcttcaaagttgttttgccccgtagtacagaggaggtttatcccgaccctccccatagtgttcccgttgaccgaaccagttttttgaccacaatggcagatgaagagcccgaagaaatactggacggaccgtctgacgaggaagcgaccggtaccataataacggccaaacaaaccatgttgatagtagatgatgacgcggagatacgccaatacatttcaggcatgttccgctcagcatttaacatagaggaagccggcaatgggaaagagggcctggaaaaggcaatagccatgctaccggacgtggtggtcagcgatatcaggatggagacgatgtcagggctggagctctgcaaagaaatcaaacagcatgcattgctgaatcatatcccggttatcctgctcacgggctcctcctctgaagagggaaagctggaaagcgcggaagttggcagcgactattacatcaccaagccatttgacaaggagttgttagcggcagctgtgcagggggtactgcagatgagggataacctgcgtaattattttctgaacgaagtgactctccgtaagaatgattttaaagtgtcaggtcaatataaggagtttgtcgaaaaatgtattgcaatagtggaggctaacctcgataatgatgaattcaatataaaggtactggccagggaaattggcatgagccactcttcggtttataaaaagatccggcaggtttccggggagtcgctgagagggttcgtacgttttatacggctcaggaaggccgctgagctgatgataaatacaagtctgaatgtcaatgaaataggtttccaggtcggcattaatgacgttaaatttttccgtggacagttcaacaaggtatttggcgtgaatccttccgaatatataaggcgttaccggaaggtattcgaagataaatacaaccttgaacagacagatacacggaaaaagagggcaggtcgaaagaaagtctgacccccggatatgttaaccccggttaccccttcccggcaaatccgcccggggaggggtaaattctccctaaatttcacactacacccccctttttatgcgaatactcccccttatagttgggagtgcttggtgtttactttgcatactggccagtaatacttatcaatcaaaattgaatttacccgttatgacaatcattctacgttttatgaatcaccagcgtgatttatccctgattttttgtcagtaaaaaacagtacaaaagctttatcaagatttattatccacgttcaacgccactaaaaaaactggtatgcgtaaaatcagactattaccaacatgtgccgccatcctcggaacaatgttattactattaattgtaaactccttgccggcacaggttaaaaccgggagaaccgtttccggcaaagtggtaaatgccgaaacgggcgagccattaattggcgccaccattttggttaaaggactcaaggtgggaacaaccgccgaccaaaatggactcttctccctgccggtatccacctcttcctccacactgaccgtaagttacctgaattttgaaaagctggaagtgcctgtcacagcaggtttcctggatataaaactcaagcctgccggaaatatcgacgaagtgatagtcgttggctatgccaaacaaaagaaggctaccctcactggcgcggtagaacaggtatccggcaaaatatttgaaagccgggcggtcaccaacatcgccctggcactccaggggcaaacgccgggcctgctggttacaagaagttctccccgcccgggcaacgaagggatttccatgcgtatccgcggcgcctcctctgtaaatgggagtgatccgctgattgtagtagatggcgtgcctgttctcaacaattactcttttcagaacctcaatccggatgatattgaaagtatctctgtgctgaaagatggatctgcggccatatacggatcccgtgcagccaatggggtgatacttgttactaccaaaagaggcaagggcaaactcaaagtagactacaacggcaatatgcgtttcgttacaaacggtatcaccggttattcaccctccatgcaggaatatgccaccatgtgggtggaagccaacaaagaggaaaccgttcccaactggtgggtatggggcgaagataacgtgaagaaaatgcaacagggcgttgaaggcgcgtatccactgtatggtaccgagttctatatatacaatgccaacaggattaaggaaatgtttgcgccaagatattcctatcagcataatctgagtatttccaacagtacagaaaagtcgtcctatcgcctgtctttcggctatgcagataaccagggtaatctggctaccgcctacgacggacagaaacaatacaacgccaggtttaattacgactacaacctgacaaaggacctgaaactggaaaccaatatcagcctgatcgatgcaaaaaccagcgagcctgctgtaggattggataataccctctatgcatatgatatgccgttcttccccgcaaagaatccctatggcaactggtttgctacctttaacggtatcgatggcggcgccaacaggaatgcagcagctatgagcgcagccggcgggcgaaacaacaggaattcactgacaggcagagtggatgtaaaggcaacctaccagatcacaaaagacctgtcgatggaaggcctggtttctcttcagaacgagcggttcaaccaggagcgttacgtattaccggtgcagttatacaactggtataacgtacctaccggtattggtcttaacacaggaggaaccaataatacttattatacctatgcctggcagggtacctaccaatactattcaggattactgcgttacgataaaaccctcgccacgaaacaccatattgcagcaatggccggtatcaacgccgaaaagaataatgcacagtgggtgtcggcccagcgtataggctttaccgatatgggcgtgtatgacatcggcctggcgtctaccaccacccaaaccaattcggggtctaaaagtctgaatggccgctattcttatcttggccgcctcaattataactatgcggaaaaatacctgttggagttagtgggaagaagagatggtaattccaggtttgcccccggctataaattcaaaaactttggtaccgtgcagttgggatgggtatttaccaacgaaggttttatggaaagatttaactccattctaagttttggtaagatccgtgctacctacggcaccaccggtaatgaagcatccgggctgggtgcattcgactatttgtctaccgtcaatatcggaacaacggcattgggatctcccgttacgcagcagcagtcgaccggacttaataataatggcctgatcagctataacagaacatgggagaaagtaaagcagcagaatatcggagtggacctgaacttcctgtccaacaggctgtcgaccaacgtagattacttcgtaaaagaaaatatcggcatgctgatagacgtaacctatccctccgtgctgggtggatcggctccgaaaacgaacagcggcaggttcaaaaccaaaggatgggagtttatactctcgtggaaagactcgaaaaaagacttcagttacagtgccacatttaatatcagcaataccaatacagtggttagcggcgtggaagggagagatagttatggccccggaagaaacgatattgtgaatggttatccgtatcagtcgtggttcgttttcaaaacagacggttacttccgcgatcaggctgatgtagacgcttattatgccgcctatggaggcagtactttgctggcgaatatgcctcagaacaatcaggcggttgcattgcgtcccggcgacacgaaaagggtagatgtagccggtacgaaaaatattaccaacatcggaaatgaaaaaagttcgctggtgtacgcaggcgacggcacacctcatctcacctttggccttaacctcggcgcctcctggaaaggtattgatatcttcaccactttccagggacagcttaaacagaatatgatgcgtaatggctatatggcttatccatttggcgcagtatacactaaccagaaccctgtattccttggtaaaacctggaccaccagcaacccggaagcgatgtacccgcgtttaacggtgaatccaacccgtgcgggctggaattatgccaataatgattttatgctgcaaaacaaccgttatatccggttgaaatcactcatactcggttatacgctgccacaacgatggactgaaaaagcaaaactgaacagggtccgtgtatacttctccggtaacgacctatgggaatcgacttccattaaagacggatttgatcctgaaatgggagaggcttccatcaacagtggctatccattcggaagaacctggtcctttggtttaaacctgggattataaggtattcatctttcatactggaacttataaaaactgaactcatgaaatctatacttaataatattatcatagggagcctttgtttgggaatggttgcctgccagaagaattttattgacctggaaccgaatgcccagtttacggacgcagtatattttaagaagccgtcggatttcaaagacttcgccacagggttctatggtcaattacccggatggaattttggttccatggacaatggctctgacctttccgccaatacaaatggcaatggctcagacatcggcactggtactattgctgttggcagcaccaattggaattacaatggtataagaagttgtaatatcctgttatcaaaggcagctgcgtataccggtggcggtgaaatcggccagtatgtttcagaagcctatttttttcgtgcattcgcttacttcaacctgcttaaactctatggtggggtgcccattgtaacaacggtactgggtgtggagtcgcctgaactctacgacaagcgcagcagccgctaccaggtagtttcccagatattagctgaccttgatttggctattgcaggattgcctaccgagcagaatatcggtactgccgataaaggcagaataagtaagtggggcgccatggcgctgaaggcgcaggtggaactatatgaagctacctgggaaaaatatgtaggcaaggcgccggatggcgatggcagcagcgttggcgcaggcactgcgggatacgatcctgccaatgccggcaaatacctcaatgaggccgtgagcctttgccagcagataatggacaacggcggttatgagttgtggaacaagaacagcgattcaaaaatggccaattcaagttcctggtatttattcaatcttgaagatgaaggcagtaaccctggaggttacaataagcaatccaataaggaatttatcctctataccgtgtacgactatacgctgcggcaatccggcatcaacatcacctggaccgtagggcagttataccccagccgcaagtttgtggatatggcggtttgtacagacggtttgccaccggcaaagtcatccctgttccagggataccatacggctgccgctgagtttcaaaaccgtgacctgcgtttactgaactacctgtatgcttccgctacagcgccggcaaccgtaacgctggacttcggcggcctgggatccagcggctatggcaacaacaaatatggtgtttacggtttcggcggccgcaggactgatcgtactgaatcggccaactggcctgtcatccgccttgcggaagtatacctcacgtatgcggaagcgctggtagaattgaatggaaacatgtcagacggacagttagacgcatccatcaataaactgcgtgaccgtgccggcgtagcccatctcaccaatgcactggtggctgcaaacggcctggatatcaaggaagagatcaggagggaacgtactgtggagttgtatcgtgaaggtaaacgctttgacgatctgaaacgttggggcatactggaggcgtcactgaatccgtcgcggcttggtagggtagtaggggatgcttcttatgaaacaccgtttaaagatgccgcaggcaatccaacggctgcctataaaccatccacctatgtgtttggagaggaaaccgcggcaacaccggccggtatgttgaaatgtgtggtggtcgccagttcgcgtaataacagtgttgcaaagagacattacctgtacccggttcccacctcgcagatgatcttaaataaaaatctgctgcagaacccgggttattaaaaacattcaattcacaattaacagcgcgcattttatatgactagcaatatttttaaaaacctgttcctgccgggaatgatattggttgccggcatatttctccctgcctgtgaaaaggatgcacaattcagggaatttaattatcctgctcccgtggtgacagacttctcacctaaacagggatatgcattgtccaatgtaacgatagacgggcaggatttcggggaagtggttggtgcagtgaaagtatattttggtaacgtgcgtgcagatactgtgagaagcgttaccggcaataagattgtagtgcaggtccctccaaaaggcattaccggtgtagtcaccgttgagatatttggcaagcgcgattccataccgcaggtatttaccttcaaagcctctgccctactgatttctatgagtaaggataaagcacaggcaggcgatgaaattacgctcacaggaaataacttcggaacagataaatccctcgttcatgtgtttgttggtgcaaaggaggcagaagtgctgagcgttgcatcggaacaggtaaaattcaaggtgccggatgcgcttcccggatccgtaacactggttgttgatggtcagcgcctcattggacaatacctgctgataaacgcggagaagcttaccggtatactgtttggacattcaggctcctggtccaataacccggccaccatgattcctgctgctgtagacggtaatctgaatacctacatagatggacctaccgcaaccggttatgttggatacgatatgggagaagggaaagcggcattactgaaatcggtacgttacgtacccaggagcggcaatgccgcccggatggtgggcggacagataagagcagccaatgatccgtcactgtccgactatgtggtactttataccattgccgctgcaccgcctaatggtgtgtatacggatgcgcaaatttcaactgtcaatagttatcgctatatctattattactctccggcaggcaactgtaacatagcggaaattgaattttacggcaagtaattttattagtgttttcaattttacaatgatgaatttcgatcggatattgacgaagctaaccggtattattatttgtgtgttgttttcagcagtatgtatggcacagcagcagcaattggtggcttatcctttccccgcaccagaggcgggaaatcctgcgcataacgcggattttatggtgaaggtaaggcagcaaggcggcaagtggcaggacttatatgagtataatgtaaaggtagatgaggtacgcggagttaatcatcatgtggaaaacgcttccatggcagcctttgatttttcgggagaagtagaagttgccatcaccagcaacagggcaccaatacgacaggtggcaatacggccgctttcatacgggataggtcataagctggtaaacaatacgatttatttccgcctgcttcaaccgaagcatctttccattgaaatcaacggagataaatttcataatcttcatttgtttgccaatcctgtacaggcaactgtcccggatccgaaagcaaaaaatgttatttatttcggtccgggtatccacgtaatccaaggcggggtgctgaaggtgccgtctggaaaatatgtgtacctcgccggtggtgctgtaataaagggccattttgtggtggatagtgtacgggatgtgaaaataggcggcagaggtattattgattctcccgggcaggaaggggtgaaaatttcgcattcaaaaaatgtactgctggagggtattatcctcacacaatgcccggtgggtagttcagatagcgtgatagtcaggaatgtaaaaagcatcagcgcttacaaatggggtgacggcatgaatgtatttgccagcaataatgtattgtatgatggtgttttttgccgcaactcagatgattgcagtaccgtatacgccacaagaaagggttttgtgggtggctgccggaatatagtcatgcaacattccacactctgggcagatgttgctcatcccattcatattggtctccatggaaatacgccgcatccggatacgatccaaaatgtgcgttataccgacatcgatatcctggagcaccgggaaatgcaggtggactaccagggatgcatggccatcaatgcgggcgataataatcttgtgagagatgtatcctttgaagatatccgcatagagaatatcaggtgcggccagttggtgcatctgcagatcccgtttaataagaaatactgcacagcgcctggcgagggcatagaaaatatactattcaaaaatataacctacaacggcgataacccggaactttctattattaccggctacagcgaagggcgaagggtcaggaacgttgtattcgaaaacctgaaaattaatggaacactcatgtccgataatatgaagggaaaaccaggatggtataaaacagcagatatggcgcggatgtttgtaggtgagtttgtagatagcctggtattcaggaaaacagaataggggccgtggcgaaataccctgctgaagccactcttttccggaataacctacaattaattttataaattgataaaaattgaaaatgagtcaaagattcttttggttgaaatcacttggaatgctgggcctcacacttcttttgcagtatgggcaactagctgcacaaaaagtatactccattgtatctcccggtagaacaacagtgttggaattacaggctgaagaggggaagctcagctatcagctcttttttaaagggaaagcaattactaacaggtctgcacttgagattacggttgatggcgtgtctttaagcacggcaaaaatcagccggtatgacaagcctgcattgcaccgggaatcttttgcaagcccgttgggcgagcaggactctttgtataacaattaccggcaggcaaaattgtttctgaaaaccaatagcggtaaccaggtaaggctcgatttcagggtgatggacagtagtgttgcattccgttatgccgtatctgttgctgacgccgtaccgcatcagctccgggagttgactaccttctctttcccatcttctccactcatctatcaatacaaccaggagtctgtttttacgccgaccttggtggataccttccacactactacggatttgccggttacgctcctggcagatagaaattattgccagcttggagaggccgcgaaccttcattacacgaaagtggaactggcccgtggagttgatggaaataccctggcggtaaagtttcctcgtgataccgctgtactgtttagcaaacaaattgaaacaccatggagaacgttgagtgtagccggttctgctattgcgctggctcattgccgcaccttgaatttgaagctggcagatgcgcctgcaccaggcgatttatcgtggatcaggcccgggaaacttatccgtgcacagctgaatacccaaagcggactggattgtattgattttgcagtaaagcatcattttcaatatatcatgtttgatgcaggctggtatggtgcggagttccgttcgtcttccgatccctgccaggtaatcccggcgattgatatgccgaaggtgatagcatatggcaaggaaaaaaatattggggttatcctgtatgtaaattacgtagggctgaaaagcaaactggataccattctcccgctttataagcaatggggtgtagcaggtattaaattcggtttcgtggatggccttagccaggcgggtctcagctggctgtcgcaggccattaaaaaagtccagcattatggttttgtactgaacatacacgataattacaaacctactggtcttagccggacctacccggcgttattgacgcaggaaggcataagaggagatgaaaacagccctgatgcttttcataatactacgctgccatttacgcgctttttcgccggagctgctgattttacctattgtttcccgaattcgaagaatagtttttcaaaaaatataaaagtttcgaaagcccagcagctggcgctcagtgtggtttactacagcccgctgcaggccgttttctggtatggccagcccaacgactatatcaacgatgaagagatcgcgttctacgactatgtacctactacctggaatgaatcgcattacctgtcgggagatatcggaaagggtatagcagtggcgaggagaaaaggagatacctggtaccttggttgtgcagccggcccgcaggattgggaaactatgctggacctttcttttctccggcctggcattacttatactgccactatttatgaagatggcgataatcaagtcatcaataagcgaaccgttacgctcaacaataccgacaagctgccggtaaagcttttagcgaaaggcggacaggccatcattttcagatcaggcgccaacaaccccgaaaaataaaaatcgaatagatgatgagtcgcacgaaaaatgtgatactaataatcgtatcatttgtggcatgcatattattgttttatgataccgtttccgcacaggcgcctgcttttttacaccctggcctgctgcatagccaggctgatttacagcgcatgagaaacggcgtggcacagcaacggtcacccatatacgaaggttacctggttttcggggaaagtcctttttcacattatgattacaagataaagggaccgctgacgaccgtgggcagaaatccgggcattggccagtccgactacgacagtgatgccaatgccgcttatcagaatgcgctgatgtgggccatcaccggtgataaacgccatgccgaaacagcgatccgcatcattgacgcatggagtaatacactgaaggcggttaccggaaaagacgctgtactgatggccggcctgggcccatttaagatggttaacgccgcagagattataagacacagtaatgcggggtggccggaagatgccgcgaagcgtacagagaaacattttcgccaggtgatttatcctgttcttgcggagtttgcgccttttgcaaatggcaactgggacgatgccgcgcttaaaacggtgatggggatagggattttctgcaatgaccgtgaaatttttgaaacggcagtccgctactatgtaaacggatgggggaatggaagccttactcactatataattaacgacaccggccaggtacaggaaacaggaagggatcaggcccacacgcagctcggcattggcatgctggccgaatgctgcgaaatggcctggcaccagggactgaacctatatgcctatgctgacaaccgtttattaaaaggatttgaatacaccgcaaaatataacctggggtataacgatatcccctatacgccaatgcctgaccgcacaggtaaatacagccatatgcgtccatcggaggtggcacggggtaatctgcgtgctgtatttgaacaggtgtataatcactatgtacacaggatggggatagaggcgccgtttacaaaagcggcggctgataaactccggcctgaaggccccggtaatccgggggcagatcatccagggtatggtaccttattttattccattgatccgggagagggaaacaggcatgcacaaaatattgtcattgaaagtcctgccgggctggtattgacagcaacgcctgatgcaagtacgctgagctgggttggtctggtagatgcttcgtcttacataatcaaacgggcagataaaaaaaatggtccgtatctaacaataggaacttctacgggaaatttcttcccggatgatcatgtaaaaaaaggagttgtatactattatactgttgcagggataagtaatggaaaagaatcagccgcatcaatccctgtatctctagcgggcggagggcttcccggcggctggcgtaacagtgatatcggaaatacaggaaaggccggttacgcacagtatgatggcaatctgctcaggatagaggcagggggcgtatttacagacaccttgcaggaagctttcaattatacctacaggaagctgttaagaaatgaggagatgattgtcggggtgtgtccgcagccgagttcacagtttacaacggtaggactgatgatcaggtccgggctggagcccgacagtccttttgccgcgctgatgttgtaccctggtaaaacaaaggaaatagaagtgcctgcatggatgatgcagttcctgcaacggaaggctcccggaattaatgcatctgttattgcaagggaactattaacaccgccggcggtaacctacggccgcctgacaggaagttactggttaaagcttaagcgatcaggcaataccataacaggttccggatcctacgatggtataaaatggcagcaattggcatctgtagaatggcgcgctgaccagccggtactgattggtgtggctgcggcctccaatatttcaaataccacaacggtacgtgttcgcctgcattaaaacccaaagaaggatgaaggtaagtttcgcaattgtaatatttcttctcattgcatcccggtctgctgcgcaggcttggcagtggcgtattctggtagataatattatttccggtgagacgaaagcacctccgcaggcatttctctggatacctgagaactgtaaaaagttaaaggcggtagtttgggggcagcataacatgacggaagaaacggtgctggaacatcctgcattccgtaaaacattggctgaacttggggtgggagaaatatgggttacccctattactacgcagatgttcgatttcaccaaaaatgcacctgcagattttgagatgatgatgaaccggctggcagaggtatccggatacacggagctaaaaacaatttctgttattcctatcggccattctgcccaggccagttttccctggaactttgcggcatggaatccgtcacgaacactggcagtaatatcccttcatggcgatgcgccgcttacaacgctaaccggtagcggcaaggccaatccggattggggcaacagggatataaatggtgtgccttctctttttatcatgggggaatatgagtggtgggaagaccggattgtcccggcattctcctacatacaatcacatccgcgtagcgtcatctccttatttgcagatgccggtcacggtcattttgatgcatcagatgccttagtcgattatctctccttgtttatacgcaaagcgatgaaattccgttggcgtgcaaggggtttacatccggtgcagccggaggagggatggttggtggacagatggcacagggatagtttgcctaacgccgctgcggcgcctttcaaagcatatgccggaaacaggcaatctgcttcatgggtatttgaccggcaaatggccgatgccaccgaacagtattaccgcatggcaagaggaaaacagcaacagttcatcgggtttatgcaggatggcaagccgctaatacctggtaaatctcatgctgtatatgccctggacatccatccgctaagcgatggcacttttcatatcagcgcattttttagcgattccaccagaaccaggcaagttgctcaacatgcttcaacggcgctgcaaattaatcgtatatgcggccccgttaagaagatagatgacaccactttcagattggatttttaccgtatgggctttaataataccaagagaagcaacgatatctggctggtagcggagaataaaggagatgatacgtttaagagcgctgtacagcagctgaatattaagataccgctaccgcaaactaccggcgaagcgcagcagatacatttcaaatcactgccggatcagcgaaaggggataaaaggtctgccactggcggcacaggcgacttcggggttgccggtgagttattatgtaaaggaaggtcccgcatatattgacaacaataagctggtttttacaagcgtgccgccacgtgcaaagatgccgttaaaagttactgtggtggcctggcagtatggcattacaggaacgttccagtcggcagtacctgttgaacagtcgttctacattcgtgctgttgaaactgtcctaccagcgaaaaccggaaggacccattagggaatggagaaaactattctattttgttctctttaatcagattggccatattagcattgaaggacaccagatcacgacccaattttgtgaaaaattccaggtcagcattttctacgctgataatagctttttgtaagatcttttcccctgtagccgtaagcctgatcgttttggccctcgtgtccgtcggatgctcgtgacgggtaataaactttttatcttccagtgttcttaacaccttcgataccatcatcctgtccgcattcccctggtttgcaatatcgatctgtgttacggcatcgctctccctggaaagccaggccagtgcacagagcagtatgaactgggtatgcgtcaggtccagaggatctaaaacacgctttagttttctctgccataacatggtcagctgtcccagcaaatagcccggactgtcctctggctttttaaaatgaaactcaatctttttgggcatagtttttttgtagcatctgtgaagaaatcagttcaaaatcgtgccggttgatctcgaagaaaccaaaacggaatggatagccccagcttttcttgttttggataaaatccagccggggaattaacggcaaaatagaaacatcctcacctggcaaaaattcaatattacgccttgatgggcaaaagttctcagacacccggatctcatagatttcatcatccataacctttcctatcgcggtaaattcctggcaggcctcgggttttcccagtgtctgctttcccgaataatagataatgaaatcatccttacgcatccttttcaaaggtgatgcctttccatggcaggtttgggcaatcccttctgcgatgccggttttgacatggtctttcgatgccacgatgatccagtatttcatatccctgttcatatcgaaatgattagtttgattttagaaaggtgatgttgtatccgtcggggtctttagcaacgaggattttcccgaaaggtgttgcctggaccgggcctaacaggggcacattctttgctgataaccgggcttgcagctcctctatttcctcatcgattgcgaaccagagtgaagcgccgatgcccagttcttttccttccaggttaccgatgggtgttctgatggcaaaacttgcttcgcctttgttatatttaaaaatacaggcccctgggttggatattcctgcttcttcaaaccctagtttggtggtgtaaaattctttcgaggtttcaaggtctctgacttgaagggatgcaaattctaattttctcattgtgtatgtgtattgttgtcgcaaatatagtatatacgacaacaatgtgcaaattttattatgattggtgtaataaacgacgtgggaatccctactatgacattgacgctcaccaaaaatggcattaaaatggcgggccttccggtatgaaaaatacatttcttgtctttattatcactctggctgctatagccattgcggacaaagcagatggacaaagcccgtccacaaatatcactgatactgttttggaaaacaaacgaaaggacatcgattcgcttgataaaaagcttttcgaggtgctaggggcaagagaacgggttgtccgtgagataggtgtttataaagcccggcatgatattgctcccttacaggccgcccgctttcaaaaggtgctggaaagagggattgaggcgggtaagaaagaaggactgtcggccgaattcgtcactgaaatgctcaatgccatccataaagaaagtctgcggatagaggaggccatttcagatgataagccctaaagcgatggtgcctgtctaatctcccccgccttttaaacaaagcataatgcgccttttaaacaaaacaagctatcttctttaaaccgaattttggttcatcaaaacaatacgagatgaacacgaactcaagtaaagaaaaattggtgctggttaccggtggcactgggtttattgcagtgcattgcattgctcaattattaaatgccggttaccatgtaagagcgacattgcgttctctggaccgtgaggacaccgtgagagccatgttgcgcgaaggcggcgctgacgctggtgaccggctaaatttcgtgcaggccgatcttgcttcagatgccaactggagtaaagcagtaagtgattgcacctacgttttgcatgtggcttcacctactccaaaagttaattacaaacatgaggatgaaatgattattccggcgcgagaaggtatactgcgtgtattgcgcacagccaaagatgccagggtaaaacgtgtagtgctgacctccgccatcggagcggttgtttacggacatcctaaccaaacagcacccttcgatgaaaatacctggacgaatacagcaaatgcaccagcctatcaaaaatcaaaaactctggcggaaagagcggcctgggacttcatcaaaacggaaggaaacgggctggaacttgctgttattaatccggtaacggttatgggtccggtactaggacctgattattcgcattccattcacctgatcaaaaatctcctgaccggaaagatgccgggttgccctaagatcaactcgtgtttcgtagatgtgcgtgatgtggcggacctgcacctgcgtgcaatggaaaatcctgcagcaaacggtgagcgttttattgccactgccggcgaaagtatctggttggtggctgtggcaaaaatattaaaagagaaccttggtgctgctgccgataaagttaaagtgaaagaattgcccaatactttgttacgtattgccgcgttgaaagacccgatggttaaatcgatgatcccgctgttgggtaaagtgatgaacgtaaccagcgcaaaggccattcgtcagctcggctggtctccgcgccctgcagaggaagcgatactggccgctgcacaaagcctgatccgtttgcaattactcgatcaataaagctaactttataccgatggaagtagccgaagtatttattgcctgcaagaaagaggcccattacagccgtgagctaattttaccgcaaccagcgctggtacatatagtttccggcgaaatgaggattgttactgcggaacgtcactatcagttttttgcaggcgatacaatcttgttaccccgtaaccaattgggcaggatgagcaaactccctttggcggggcagccctgcatcgccatatcagtagtgttccgtaaagaaaagctacagcaatattatacggagaatcagttggccacttcacaacgccatggtgcggagctcatggttttaggagaacatcccttattgaaaagtttattcaattctttacaaccttactttgagctggccgatgctttgccggaggacatcgctgccttaaaagtcgaggaagccattcgtgtactccgggtaattgaccctcaggtggatctgctcttggggcattttgaagagcccggcaaactggacctggttagtttcatggagcaaaactattgtttcaatcttccgctggagaaatttggttatctgaccggcagaagcctgactacctttaaaaaagatttcagaaaagctttcaacagcacacccggcaaatggctcacccaaaaacgcctggaactggcacattaccagatctctgaaaaaaaacgaaagccatccgaggtttacctcgatgcaggtttcgaggatctttcccatttttcctatgcgtttaaaaaacatttcggatacagccccggcagtttgtagaatagcgatgctttattaactaccttactaaacgaagtgctatgagttatgaaatattattaatccagggcgcgggccttgtaaccacagaagaagaacaggtaattgcagacgccctgaaggctgaacttggcaatgagttcaggattatatacccgcctattccggatgctgacaatcccagttatcaggcctgggacgctgttttaacggccagcctggaaaacttatcgggaaaggttatcctgctcggccactcgttaggagcctctgtaatattaaagcatttttcccaggagccggttgcggataaaataataggaatgatcctgttcggtgttccctattggaaggatcagaactgggatgtttcggaatatgttatagaagatgattttgcaggtaatcttaacaagctggataatatttatttttattactcaacagacgatgaggtgattccccgtcagcaatttgaaacttaccaaaagttaatgccacaggcaaattacagggtgttttcaggtatggatcattcttatcacagggcaataccgtacatggttgcagacatcaaggatttggcaacaaaagcgcaggaagaaaggtagtcactgaataaaagagcagcgctttgaaaaaggcgctgctcttttattaattaatattcctggaagtcataatacgaaacggggccgccgtttacagccacctgtacataggtgtttgcattgtctgccgcattacaataaaccggggtcgatggtgtaaggaatccatatccgttcgcggaatatactatgtaactgccggaagaaacatacaaataattgctcgaccagcttaagccggatacagggccattgccaaaggcatagatgaaattccaggcgaaagccggcgccttcacgccagggatggaaactgtttgttttaacgcggaagtggctttcatgctaaaaccgcagctaagaatgatggctgcggtcaaaagtagagtccttttgctcataagataacatttagaggttaatgtgattaaactttctaaaagttaaaaagactttctttaaccggttcatcaatttgtatcataatgttgacaatttgtatcattatagaggatagaggttgcaacggagtggtcgatcttatcatgatgcgtaagcgtccgaataaaacattttctgaaattaacttaagtgaaaaaaaaactgctgatattcccccagctttgcctaaaaatattcaattatgggaatatcacctttaggcatctttcatactattattggtgtggtagccattatcgcaggactggcatccttttttaaatttggaaaaatcagcctggctcactggtcaggcaaggtttactttctcggaacactggttacatccctgaccgcgctgggcatctccaggcatggagggttcaatcccgggcatggacttagtttgttggtgattgcattgataggcatttcatatttcctgtttaaaagaaaacaggaaagtaaaaaagcgcgttactgggagaacttttgtttttcattcagctttttcctttctatgatcccaactgtcaacgaaactttaacaaggattccgctgcatcacccgttggcaagcggaccgggcgaccctgtggttggcagaacgctgttagtggtactggtattatttattgcgggcgctgtttatcagtttatcaaacagaaaaaattcaacaaatctgccggaatacggtaacttattatacattagtagaaaattgatgcagataaatgattactactgatgaaacttatttattaagacaggtaataagagaattttcaggactgacagaggaggatctctctgttagtcttgctttttggcataaacggaaaattgcaaaaggagatttttataacaagcaaaatgttgtttgtaaagatttgggaattgtggtcaagggaatgttcagagtttattattatgaccctaaaaccgatgaggaaagaaacatttttttcttttccgagcatcaatttattgtttctttcagaagttttatttttcagtatccctgtgtctactatatagaagcattggaggatgcagagatcctgtgcctgaattaccccgatctgcaggatttatacgcatctcataaaggatgggagaaatttgggagaattcttgcagagcatttttttaatcattctcagggaaggacagaagaactgctgtttttaacccatgaacaaaggtatctgaatttactacaagaacatcccaacattgtgcagcgtgtaccttcgtttcatattgcttcttatttaggtatcaaaaatcaatcgctgagccgcataaagaagcggatttcggaaaagaagaataatgacaaagcaaatataggctaattccgatttagatagaaagggacgtggaaccagggaggttatttagagctactcaatggattcttaataacgcttactgaatcctcactattgctcacaatagccagcccttcattaaactgcccggcttcggtaaattgtggtggtatgatccatttaccttttgtgtcaatataaccccataaatcatcttgtcttaccgccagtagcccttcgctaaaattgccttcagtgccggtaatacgtttacctgcggcataaaggagcagtttgcctgtttctgtgaaattgctgtccaataagtaaaggaagccctctttgctgtcacccgcctttccacgtatgatgccccaaagaggcccgccatcgtaatctggcggcaacctgtcaaaacggggagctaaccttattgtgcctttcttatccactaatccatagtgcccatctgcaaggaacctggcgatgccttttttaaatattgttacatcatttatattgttggcaagggtaaacaaggtattacctttcttatcaattattgcatggtattcgtctccttcgttttggttccctgttttttttgttcctgttactaccgccacgctatctgaaaaataaaaggtattgctatactgataggggatcaccaaccggccggcagtatccgcaaatccgtgacggaaattgttatctttatctgcctggaaaacttccagcaggccttctttaaacatatagggcatactggtaggttcggcttttatactttccgccgtaaatattattttgccattagtgttgatacaggcccagcctttacctcctggaatccacacaatggcgcgtccacaggaaaaaggtcttgtatccttatatcctggttcaataaccagttttcctgttttattaatataaccatagagatcagcacccgctggtactaccgacgcgaagccttcactaaacggggatgacagattatattgggcgggtattttccactcacctgcggcattgataaaaccatatagtccatctctttttgtttttacgctcaggagtccctcactcataggttgtatccggctaaactgtcccggtgggatggcatattccatttcctgcgcgcacgaagtaaaataaaaaaagctgcttattagcagcgatactatcttcaatagattattttggttcatcaattatttcattttgatggtttctgcaagcgtatattgatattggctttttaaaagtagtacagttttaccggcagataaatacctgaaagcaggtatttattgtagcccgtgttatggttacttttagatttaaaacacaacgaccatcttgtgaaaaaacttatgagtcacgtatttttttatcgggataatgaatagcagatttttgatttcttttttcttgttgatgcttgcatcaccccttatttatgcccaggcatacaagggcgttgtagaaaaattttacggtgccctgggaaagcgggattttgacagtgcctatgcgttgtgtaccgggcctcaatggggcaccctgcaacaatttgccgattcaggcagttacggcggtattaatcatgttatcctgtcgtctgttacttataaaagacagcgcgacactaaaaacatggaagcaaaagtagatgtggtagtaaaagacccggtgaacggtgacggaaggtatatccagaactttgtgctggtagagaaagaacacaaatggtttatccggagtaccagcctgttacaaactgacagggcagaaaaaggctggaaccttaaattaatagaccagcccgggttggacaaagcgacggtgaataattttataaaacctgtatacgatactgtgaaaaccgatgcggctgttaataaaaagagcgctcaacgcattgttaacgatccccggttttttcaaactcctggtggcgtatatgcggtagtagtggtggagaatcccgggcgggagcagggcattcttagctacggctggtgcgatgtctttgtttttgagcaaaaagatcaacaatggcagatgacagattttaaactacatgcgggaggtggcggtatgtacggcaattccggaggatttaagaagttgcttcaggccgggactaatgtggtagctttggtaatcgccggtgggcaaatgcatatgggagatctggtggaacaagatgacattattgcgatggaagccggtaaattatacaacctgacttctgtcgtggtccatcatagctatggtgattttgggtcgtcgcatgatgaaaagagcctgaaaatatgcaacgaaagaaactatttgtttatcaaatcagaaaagaaaaattacgacctgaaaattatacgcagcagttgtcttgtctctaaaaaggaaacgaaaacagacagcgtcattattccctggattgataagaactatagttttccggaagcgctgatgcatgaaccggaagcaaattaaatttaagaagagattatgaaaaagataaaggcgattgcagttgtcattttattgttactaggcagaagtacctttgcccaaagctttagtcttgaaaatttaaggcagatgaataaaatgagtatggacgctttcaggatagagatggaggataagcagaagtttgtttttgctaataaaagaatgccgccggaggagccgtatacataccacgcttatgaactgaaaaaggagggtggaacattaactatggaaaaaatattgtattctgacaggcctaatacaataacctacaacactatctataaaaatgacctggaaaccattcagcaacaattattgagagaggggtataaggtgaagtcgaccagtaaagtattcggcaacacggtacaaattacagattatacgctgaatggaatggaagtgcaactggttgtaccgatggccggtaatggtatgcgttatggcattaccgtgcgttagctttagcaatatgtaactttatgcaggataaaaacgtttaataaaaaaatgcaaccctatgagatttatctactgtattttagctgcagcattgttagtagcggcctgtaagaaagacaggaaaaagacaaccgcctgtaatgtggaaaatcctgtggcgaatctaccctggctgaaacatgccatcgacagctttgtgtcgcttaagcagggcggcagtgtaacactggtcagctacaggggagaggattacatcaatatccaacagaacataatttcctgctggccctgtgggttgcatacctgcgccgggaagcgcttattttatcccggcgacagcgcattgatcagcgacattgcaaggaatggcgagccgaaggtgatccatacttttggggagtaagatggggttcccaaccctgaaaccattcatttattaccaggaattttaccatttcttgctccttccagtgataagcgagcgggttggacagcacctgcttcagtcatgcctgatccctgcgtattccctgcgttatctatacggttaccatgcactccccatggacttccaatgggcttcccatgcacttcccatacactccccatacactatgccccaaccatttccggcaaaatgtgacaaaaagcggcaaaagcggcgggtttgtttttacgtgtgcctgccggtaaagaacttcgcatagtacctggttgatcaacaggagcagcttaacaggcatagctacctaaattgcctttcttctaacgaaaatactttactatgagcaaacaagatggattgctgcaatttactggcccactcgaaaatttatcattttataaaaccaaacatggttacgtggtcagaaaaagatccggtgtgccgggcgcccgggtagccacagaccctgccttccagcgcagcagggaaaatagttgggaatttggccgggccggaagggccgggaaactgctccgcaccgctttccgtaatatgataaggaacgcagccgatggtggcgttacaccccgcctcctccgggaattcctgaaggtgataaaagcggatgcgatcagtgagcgcggatggcgcaacgtggtggatggcgatataaaaatcatggagcattttgaattcaatacagcgcgcgtgatgagtacttctttttatgcacccttaacggcggctatcgatcgcgataccggcaagggaaccgttgtaataccgcccttcctgccggcaaaggaggtgcaggctccgcacggcgcaacacatgtcatcattacctgcggagtgagtgcgattgattttgccggagcgcgttttgaaagtgacgaggtaagtagtgctccattgctgctggatagccgctttactgcgccgttgacgcttaccgtcagtatttcgccgcacagtcctttcccgttgttcctggcgctcagcattgagtttgtgcagatggtgaatgaacggccgtacccattgtcggacggggcatacagctccatgaagatgatggtggtatctgctccgggtttggaaagattacttcaccagtaaaatgcttcctttgaattcaaatttctctccgttttcgcagatggtttgcatgtaataaatatagcttccaaaagcggccgctgtattgtttatccggccatcccaaccggcagaaggtgcgttgatctggaaatgtgttttttcaaataccagttttccccagcgatcatagatgcgcaggtattcaatttcttttacgccttttcccttaggataaatgcggtcgttttgaccatcctggttgggcgtaaatgcgttaggcataaaaacggcggactggttacacaggacgtgtaccgtaacatcatctgttgctttgcagccatagcggttttccacttctacggaatagatggtggtaagattaggaatcacctgtatgctgccacagccagggcaattgagatcctgttgtggcgtccacttatagctgactacatcattacttgcggcagcagtcaaatgcacaggagtgcccgcgggaacattccggtcggggcctgcatttaccgatgggtggggcgctacggttacctgcagggatgatttatcggagaagcatcctttgctgtcatagcctgttacggtgtaggtatagttgcctgtattcgttaatgtagccgtggtagcatctgtattgggatttgccaggccgctgccttcccatttgtaatagtctgcaccggaagcgtataatggcaatactgcgccaagacacagtgaggtatccggtgtggccgttaccttaaagggttggattacggccagcgtcaattgatctgtattaacgcatccgttgctgtctgttactttcacgtggtacgtggtattggtatcaggacttgccgcggggttggcggtgaacgggttgctgagccctgttacgggtgtccactcataactggtgccgccggaagcctgtagtacagtagtattatgtaaacagataaattcactcagtgaagtggcctttgcattaggtaaaggttgcacgttgagcaggtggtgggccgtatctgtacagccgtctttattggcaacaataagcgatacatccacaggaccaggctgagagaacacttgttgcggaggtttattgccggcaggggtttgcccgttatgaaagttccattcccaggtgaggccattgtcgttgacagcactgccggtgaagctgaccggagattccacacagactttatcaggtccggcaatgctggctacaggcttcgtatacacgtttacgttggtagttactgtttgtttacaaccataggcggtagtggtggtaagactaaagtcatacttacccggtgcggggataaagaaggatggggtggccgtagtttcattggagggtaccaatgtgggatgaaaatcccattgataggtagccggcttccctaattgatcaatcgaaaaactgttgaatacaggattaaaagtaaccgttcctttaccacaaaggatagcgggcgtggatgataactgcacgtcgagtttgtcaataacaatcgggttgcgcagcagtgcactgcccctgcaaccggcagagtcagtgaggagcagcctcggttgatagatgcctggcgttttaaaaacatgcgtcactacctggtcgttagtatgaaggataataccatctgtaaaatcccagctgaaatcctgtgtacccttgctaaccacattaaaccggatctccttttccaggcagccgccgtcagaactggcaattatagcggcataggggccttttacttctatggtatcaatgtactgatctgttacgccagcttcgccccgggcggttagtatcacttcataacgtccgggttccgtataggtatgaatgggatccgcttctgtagaagtggtgccgtcgccaaaactccaatggctggaaatatagctgagggaagtattggtaaagaagaagatcataggtgcgcaactgccgccattagcaaaaataccgctataggtaaaggctgcaccaacagcagacactcttacctgtttcctggcactgtcttcacaaccattgttatcctttacgcgcagtattacctgatgggttcccgacagtgtgtagttatttaccactgttccggtggcggcagaagtatgcccgtctccaaagttccagttcacactggtaatagtgccgccggtttcactggatttgttatagaagaatacatctgtacctggtttaacaagataactgctggcgtcgaatacagcatgagggccttttacctggagggtgttgtcataaccatagcttacgcaaccctctttatctgttaccttcagcatcgggttgtaattgcccggctgcttgtaggtatgcacgaaaggtccttttgtaaaggtggctaccggggtgccatcgccgaaatcccattgccattgactgatacctgcactgtatttcgtagtggtaacatccgtgaaagtgagttcggtgccggcgcattttgcggccggcagtttaaacccggcaacaggtccgcgaacgtttacgggtataatgttactgaggtctatacagccctgcaggttttcggctgataattgtatcagttttttacccggaggaagatttttgtagatgaatgtttgctggttgtcgggatcgctctggtcgatgccatctgccagccatttgtagcctgaggttttatatatagcagggttgtagctggtgatagccgcgttcagcaactcattgctgcataaagtagttttatctgtactgatgactacaggagaaggagcgatcacggttaccatcaatccttgatgggtggtacagtgactgtctttcgtagtcagcactacctggtaagtaccgctgcccgggtaaacgtgtgttaaagtagcggtagccttactataggccgtatcggtaccgtcgccccaattccattcccaggattccgctcctaaggaatgatcctcgaaaacgatagcagtgcgtttgttacagtccaccggccttaccgcataccgggggaatggagtagtagcagtaatgtattcctttttcgcaatagtatcatagcaggtgtgattacccactatcagctgcacgtcatacgttccggggcgttgatagctatgcgtggtgtttttgccggcggcggcggctccatctccaaagtcccagcgccagctgtcgccaatatctgactggtctttaaatgcagcgggattattaccgcatattttcggcgcatcaggtgaaacgaagtcaggaaccggttttttatatacttctaccttattcactgtctctacctttcccgtgcagccattgacggtagtataggttaagtaaaccgtatagatgcctgcgtcactatattgatgggcaggagttgccaatgctgatgcgggactaccatcgccaaaatcccatagataggttttaatgacgtctgcattgttggtagcggcgctgaagctggccgttagtccttcgcaaccgctgttgttttttgctgctgcggttatttttacgggagatatatcgaagctgctgctggtggtagccatacagccatccttgctggtggttagcaatgtagtggtgtagttaccctctgcagcataggtatgtgcggggtgttgcgtggtagcggtttgcccgtcgccaaagtcccatttccatgcagcggcggcaggggcgttgccggtgaacgtggcggtagccggcaggttacagaaaagcgggacggttacggcgatgttggctgccggtgatggcttaacatccagtgttttctctgctacatccacacatttgccgtaggtagcggttagtttaatatgtaacggaccagtagcaggcggggtgtaggtggtagtattatccgggttgtttaaagccggttgaccgttgatctcccaggctacttggagctgaccggtagtagcaaatacaccgctgtaaatgcccggcgtattggaacaaacaggagatggaaaggtgaaatcggtagtataggcggctacgttaatatcggctgcttttttaaccgagctgcaacgcagttcgttggtcaccgtcagggtaactgaatgaaggcccttgctggtaaaggtatgtgtgccgggatcttttaaagaagaagagcttccatcgtcaaaggtccagttataggccagttggccgggaccggtggaggtattggtgagctgcacaatggcgggtgcgctgcagaatattttatcggcgaccgtaaaaccggccacaataggaggggatacccttaccagtgtatctaccaatttaaagctggtgcattgatagctgttggtaacaatgagtgttacgggatattttcctgcctgctgataagtatgtgtgctggtgctgccagtgccggtagttccatctccgtagtcccaggtataagtgagcagggtgccgcttaccgggtctgatttatctgtgaaggtggtttgcaaaggcgcgcagccggttacattggtagccgtgaagtccactttgggcttagatcttactgtaataaatcctgttttggtaatggtagaagattgtccggctgcatccttcacggtgagggacacggtatacacacccggcttgacataggtagccccggggtgctgttcagtagaggtataaccgttaccaaagtcccattgccaggatataggctgacctgtcgatttatcactaaatgttgttagtagcagttcgcaatcactggttgatgaagcattgaaatctgctttgatttgtgctgttactcccgaaaaaataaaacaatccgctaatagcaataaaagtagtgatggacccaatttaagcttggtgaggctaaaaaggttcattcatagatatgttatgtaccctgaaattacggtattaacagcaatgtaccataatgttttaaagttattttatcttcatagatatatgcacaaaaactaccgtatatcttccctgggcgaccgggctgttatcatcgaatgggaacaacagattggcggggatattcatggccaggtgatgcaggccttccggcggctacgggagctgcatcagctttacatcctggaccttatcccggcctatgcctcgctgacggtggtatatgatgcggtggtgctgtatcgtcaacagcatagttacggcggtgaaaagatccgggaattgattgcggcaacgctggacggggccgcggaaatcactgccggcccgccaccccgcctgctggagatccctgtatgctatcatccttccctaggacctgacctgcatgcgatggcggagagcaagaaagtttccccggagcatatcatcgaactgcatacggcacaaacctacacggtgtacatgctgggatttctgcccggctttccctacatgggcagcgttcacgacttgctggttatgccccggttaaagcagccccggctcagggtaccggcaggaagtgtaggtattgccggtgcacaaaccggtatttatccgcaggaatcgccggggggctggaatattattggtcgtacccctttgcggctgtttgacgccgctgcggaaaccccttgttattgcgaacctggcgaccaggtgaagtttatgccggtatcactggaagatttccgggagatgacccattatatttgacacattaagaccaaaaaacattgatacaggtaatacaacaaggattgctggataccatccaggatgcagggcggtacggttatcagcacctgggcattaaccccggaggggctatggatcgggttgcacttgcagttgccaacagcctggtgggaaacgacattaccgaagcggctattgaactgcattttccggcatctgctttcctgtttgatacagaagccatgatatccttatccggcgctgatttcggggcaatcgtcaacggcaggcccctcgatattaaccggccggtgctggtcagtaaacaaacggtgctgcgttttaacaagcctgtttccggtgcgcggtgctacctggcagtacggggaggattggcattgacgccctggctgggaagctacagcacccatttaaaggcaggcgccggcgggtttgatggccggccgctgaaaaaaaatgaccgcctccacctacggtcaggcaatatttccccgtcatggttccagggcaaagagtttgtagcgttgccatggaccgctgatgtaagccatctttataccagaaacggcattatacatacattgccgggcagtcaatggaacctggtatccgaagatacccgtcagcaatttaccaacactgccttctccttaacggaacaaagcgaccggatgggattccggttaaccggaccagccctggctaccgagccgcgggaggaacagctatctgccggcaccaccaggggcaccatccagttattgccggacggacaactcattatactgatggccgaccatcaaacgaccggtgggtatgggcggctggcgcacgtgataacagcggacatgccttccctttcgcaacgcatgccataccaggagattcatttcagcatgaccgaggaaaaaaaggcgtctgccttgttgtggaaacaggagcaggacttgctctttcttcaaaatgcctgtaaattacgactggaggaatggctgcaacagcaggctgtttaatcatcatcactatgcattatatagatctcaactgcgacatgggagagggtttggacaacgattccgctattatgccttttatcagcagcgccaatattgcctgcggctaccacgccggcaatcatgatacgatgctgcgtacggcaacgctggcgctcgaaaataacgtggctattggcgcccacccggggtttgcagataaagaacatttcggcagaacagaacagcagctttcagatcatgcattgtatgaattgattaccacacaactgtatgccatgcaattggtttgcaaatcgctcgataccactatgcgacatgtaaaggcacatggtgcattgtataacatggcggctaagtctcccgcaatggcgcgcgtgattgttaaagcagtgaaagatgtggactcccggctttgttttttcggtctcagtaacagctggcttattaccgccgccagggaggccggactgaaaacagccagcgaagtatttgccgacaggacctaccaggacgacggttctctcactccgcgcacacaacccaatgcgcttattgaaaaagaggagcaggtaatagcccaggtgttgcagatggtcgccgaccaaaaggtaactaccgttaacgggcatacgattccgatgacggctgaaaccatctgtattcacggcgatggcgcacatgctgtcgaatttgcgcgcaccatccatgctgcattacatcatcatcaattaactatacaacggccttgagtaaacaaaaatcttccgtgctgctgggcgcagcctttctcatggctacttccgccattggtcccggtttcctgacacaaacaacggtatttacgcagcagctggcggcgtctttcggatttgtaatattgatatcggtgttgctggatatcggtgcgcaactgaatatctggcgtatcctcactgtttccgggtaccgcgcgcaggatcttgccaacgcgttgttgccgggtctgggttatgtgctggcggcattagtggtaacaggcggactggcctttaacattgccaacataggtggctgtggattggggttacaggtactcaccggtatggatactgtttatggtgcgttgctgagttgtggtatcgcgctgtttattttctggatgaaggaggccggcaatgtgctggatcagtttacgcgctggcttggtatcctgatggtgctgctcacgttgtacgtggccatcagttcccatccgccaatggtggaggcggtgcggcaaagcgtatggcccgcagtgattaataccaaagccattgttacccttgtgggcggaaccgttggtggttacattagttttgccggcgcacaccggctgctggacgctggtgtaagtggaacaacacaggtacggttcgttaaccgcagtgcagtaagcggcattgttattaccgccatcatgcgcgttttattgttcctggcggcattgggtattatcacacagggcgcggtgcttgacagtggtaatcctccggcatctgtattccggatcgcggcaggggagatcggttaccgtttctttggtatcgtaatgtggagcgctgctattacttctgtggtaggtgcggcgtatacttctgtttcctttctgaaaacatttcatccttttattgcggcgaacgagcgttggtttatcagcgtttttatacttttttccactgttgtttttgtaatagccggcaaccccgtgcagctgttgctgatggcaggcgcgcttaatggccttatattgccggtggcgcttgcagtagtgctggtggcggcaggcagcgcaaggttattgcaacattaccggcatcctgtgtggatgcagctggcggggtggctggtggtgcttgttatgggataccttggcggtgttacgattgcggattggttgaagtgatcaccccggcaggtgtagataagttgaccaatgttgaatatatgttatgattaaatattggtttgaacattcggaggaatctattattttgcgttatgctttctttataccatttttgaaattcgttccttacctggaaaagtaatgtgttgcccataaagttgtaacaatgttaacggtttcactataataattcaatccctatgaccagagttttccttagtttttttattttgttatgtgtatggtttcctgtaaaagcccaaacaggtacatacagtacattaaatttcccgaacacctacaccaatacaatcactaccgggttctatgctagcaacttcaggtccgggtttattcatcagagcagtgcttctatcaattttggcctgactggtttaaaggccagcttattcagattccgctggctcgcccatgataatggtgcaatagattatgcaaccgatgcagaccaggttatgtcattggataactatggcaacctgaacctgaaagggacgttcacggccaatggtaatgtggggataggaatggcacctaccaccgacaagctcgcgatagatatgggaaccacgagaggaggcgtaaactttttgagcgatggagacgccaacgcatacatggatttaaaattcactgtaaaaactaccaccggtattgcaactggtaaaccctttctctgggaagcgtctttaaggaaggatggttactttagcggagatgctaccgggcctacgctggaattttacgcagtgaggcaaggttcgggatattatgcgccgttattgttcaaatccaatggagatattatcctggccggcgctcagaatgctaccaatggaaatgtaggcatcggcaccaacgatacgaagggatacaaactggctgtgaatggcgacgcgatttttaccaggataaaggtaaaggcctataccgcctggcctgattttgtgtttgcaccggattatgatttaccggctttgtctgacgtagatgcctttattaaacaacataaacatttgccggatatgccttcagaaaaagaggtaaaagagcaggggcaggatttgggtgagatgaacaggaaactactgcagaaggtggaggagttaaccttgtatattcttaaacaggatgagcagctaaaacggcatgaacaggagattctgaagttaaaatcggctgttgaaaaacgttagttgaaaaggcagcaattaaagccaggtaatcgtttagagatacccggctttaaccagtttttttacaccctgtattgtctaaccagcctttccgtttgtccgcttcacctcaaattacctggactattccttcttcctgttacaactttgtgtcattgataacgtaaaccaaaaatctcatgacacagaaaactgtaacaacaatttattggataggaaccgtgctcacttccttgtggtttggagcaagcggattttttgaaatcaccggaaatccaattgtatggggaataacgcagcaattgggatacccctcacattttatatacctgcttggtattttcaagctgtctggtgtagtcgttcttttaactcctggcaagttgctccggttaaaggaatgggtgtttgccgggatcttctttgatatcatttttgcctttgcttcaaaactaagcgtacttgggttaccggcaaccgtagatgctgttgtggcgtttataatggtaagtgtaacttatacgatgttccggaagatgtacccgggtttaaatgctgagttttaaggcgtacgggctttgccatgagcggtaagaatttaaagccatttgcattaaaaagagaaagcgggtgtctcagagtaattctgaggcacccgcttttattctgaggggaaattgataaattagcatgctgctgttacttagccaatctattctgcgccgaaaaaggagtatctgtatggagaaaatgaatcccaccatgaaagttttattagccattatggtgatggcacaagctgttttaggaactattttatatagaaattttacccggtttaaagcagagatgcatagtattcatgaaaataagctgtcaggtattattaccgcctatgaatttcagggaagaggttcttatgatctgacaattgttgataaaggcgtttcgaaagtaataccttgccctgcctttggaaggtctattaagtcaattaaaatcggggactccatttataaggcatcgttttcagactcagcctatattttcaggaaggaaagcaacggcgagtaccggtttaatatagcgacgacaatcagcttctaaatcagcaggtataagatgtttaaaaacaagaaggcgtctcaaaaataattgagacgctttcattccttttggatgagcgtaattacagggaagcccgcgttaccgctttaatagctcctgtttccccatgttggatcataccaatcagttcccactcctgtgtattaaaatcgccgggtaaattaacctgcacagtgccctgcttggccccgaggccgaatgagtgaaggtctcgtactatctgcacatgtgaaagcatgcggccttcgttttctcccctggttactttactgacagcacgtttttgcactgtggctatcagcaggcggctgttgccggcatcgcctgtaaattcgtaagcaagacttgccttgccggattgcagttgcccttttatattcagggtttgttcagcagcgctggccaaagcgtcgcctactgcgttagttactgcagcttcatctgatcctatgcaggatgatttgccgttcaccaccagctgcggcgtatatacctggctgtttagctgttcactgtattgatattgccgctttgaaaaccgggaatcactgaatatatctttccagccaaggcggttccagtaatccacatggtaggccagaatatagatgggcttatttccggcttcgtcctggatacgcgctaacagggcatcagcaggtggacaactggagcatccctccgaggtgaacagctccagcacggcaaagccgttgccggccggagctgtttttttgtgagtggtattcctgtttgcacataccgcggaaaccagtgtgaatgccattgcggcgcctatcgccgacatcattattgttttcatcttttgaatttttattttattcaaaagtaccggctgctgatggcttaagtaagcaaaaaagccaccaggtggacatttttggctttcaaccgggaatatatggccgggagaaaaatgaggttaacgttcttccatccagctgagaaagctatgggatttttctttatttacaagcagtttttctggtgtttcaataaccagttttacataaagtttgcggagaaaatagggctccacctctttgatggccttgaaattaataaggtactggcggttaaggcgaaaaaactgaagggaagataccgactgtgtgatctggtccagtgattggctgatgacatactgctgcttatcaaaacacataatccaggtggcgtcatggcgtatataaaagaacgcaatgtcttccacatttatcgtcttgtacttttggttttgaaagataagaaagctggtcttgccgctgggaggcgccaattttgaaagcaggtcattgaggtcaggaactgttttctgctggaagaaatttttcagttcatccaccttccgcaatgcgtcctgtatatcctgtttggaaaagggcttcagcacataatccactccattatttttaaaagcgtcaagactatattcatcataagccgtgcaaaatatcacggggcaggtgatttttacagacttaaatatttcgaagcaaagaccgtcggccagctggatatccatgaagataaggtcgggcatgggaccctcagacaacgcgctgacggaacttgccacactctgatactggccggtaattttatcgccgggttttaattcaagtataatattcgcaagtgatttagctgttttaagttcgtcttcaatgatgataatgttcatgaataagcggaagtttgatttgaaaaactttttcgtcggcaacaatatcaatatgctggttcagcaggtgctgatatctcaggtcaatattttttaatcccacaccaagagaatgttgttctcctgttttctgctggacctggttctctacaattattttgtcatcttcctcatagatcctgatacgcaatggcttctccagggaaacgatattgtgtttgatacaattttcaaccagtaactgcaacgtgaaaggaggaatcagcgttttcaatgtgccggggctaagcgtgctctcaaaggtaaagccatcctcgaaccgcgctttctgcagaaagagataggcattgagtatttccatttcttcactcacatggatcaggtcaagtttgcggctttcgagcgtaaaccggtaaaagttggacagcttgatgataaagtcaacagattcctgttcaccgctttctaccatagccttcaacgtattcaggctgttgaacaggaagtgcgggttcacctgctgcttcaatagttcatactgcgcgctgagattatcacttttaatacgttccagttccatcgtcacatgctggttttcataattctgctgcagcaggtgcaggaacatataaaataccaggttgataaggatacctcttacctccaccatcagcatcacaggcccaaaattaatatgcgacaggatcaactgctgtatgcaggcaaggcccagcatcactaccagaccaaataacaggctgcttatcagttttgaatacgaaatgctctgcttccggggagcatcggactgccgggagagcatgaaaatattgaagtaccacatcagcacggcgaaggtggctgttatacctgcattaacagctgcttccgctaagtgaaaatggtgctcggcaatttgcggcacggacgacaacagtccgagaacaatggagctgacccatatcgttgcatgtgatattttaaaccctgttttttccatctgtaagaaatcaatctaaatgctaaattaaaaatattgatttttaacttaccatttaggaaagttagttgccctcttttattcccgccggtaagcatcaaggggaaaccgagggtctgtgggaaaatatatcgttgatccggacggctgcatctactttgttgcctgcgctattgaccggccagtggccacgttctagttgataagtcagtttgtccgcatcaccggataccatttccacggtttgaacttcgccattgatataactgccgtaccagtatttattatcggcctgtttgtaggtcaccagccggaatacttcaccgggggtatgtttttcgtaaccggcaagcgcagattgctgtgcggcggtattgccatacaacacagacattgtttgtttttgcctgttggcaaaggatgtgatcacatgcaggtttcctgcatcaaacatctcccttgccggcttgggtgcgttatcgactaaaggaaggttgaatacataatcattcgcactggctattttatggcaattgaaacaggtggtattaaacataggtgtgctgccataaggcttcaacgctgttccgttgaattttgcgaagccccagccctcactatccgcgaagcgctggttgtctttggtcatgatctgtacactgtttaaagagcccgggatgatgtcaccgttcttttcctcaatgctgttccacactacttttacgatggtgctgccttccgggaaaggattgatccggttatcgcggatggcttttgcggcaagggcattgccatacactacccggatactgtggttgtcgaaccggttggtggtactgatcacctgccattcccggtagccgggcgtataggctactccgttagcagcaaccgggttctccattgagagaagggattgttgccggaattgttggaactcccgggcggcttcactgataatggttgtatcgtgatattttgaggggctgatatccgttacatattcctttaaaacagtgatatcttttgcagaaagcctggattgtggatgtgtagcagtataagtgctcaatggcatttttcctgtcagcaccatattcaccatttcccagaggcgtccttgctggtcggccgacgagagtgtatcccaggtggaaaaattaaaccgggaccttgcttccgtaacgtcggcagctaccagccatgaaaccggcgcaatatgatcataccagctaagcttagtttcattggagtggcagtcgtaacaggcacgtttaagaatgcccagtacttcctccggcgcttttatgggcgccgtaaccgcgtggttttgaaccggctgacgaatgaattgcatggcggttaccattaaaataaacagggctattaccaggccggatctggttttccagaaagataacttcataaattatttttttactgagatgtatttccaatgtcaggcatagctgctcgcctcgataatcgctttggcgaatgcttccggcgcttcctgcggaaggttgtggccggctcctttgatgatgcggtgcacgtgtttgccggtaaacatgcgggcatacgctgaaccatcaccggcgggaacaacgccgtcagcatcgccatccagcgtaaccgatggaaccgtaataactggtgctgcagccagttgcttttcaatggcgtcgtattgttcttcgccgggttctatgcccagccgccagcggtaattatgaataacaatggcaacatagtcggggttattgaaagaggctgcagacaacttataagtggcatcatcaaaatcccatttgggagaaacatttttccagatcagccggttgaagtcgtaccaattggcggtataccccagttttccacggtcggtagcaaagtaatactggtaccaccatccccattctgctttaggaggcaagggctgtttattttttgccaggttgttaatgagatagccgttaacagaaaccattgcattacagcgttccggccatagtgccgcgataatattggcggtgcgcgctccccagtcgaacccgccgatgatcgccttttttatatggagtgcgtccatcagcgagatgatatcatttgctactgccgcctgctgcccgttcctgaatgtgccggcagaaaggaactgtgtggtgccatgaccacgcaggtgaggcacgatcacccggtagccttcagcagccagtatggccgatacttttgcatagctgtgaatatcataaggccatccgtgcaggaggataacgggctggccatttgccgggccggcttcagcgtagccaacatccaacagcccggccctgacctgtttgatgtcctgaaaggacacaggggcctgactagcttttttgtccctttgacccgtagtggccaatgcctgcaggggtgagagtttggttgctgcgaaagttaaagcagcagcgcttaaaaaatgtctgcggttaaatttttttgtcggttccataatgcattcctgcagatgcttttgtgctcccaggcgaaacaaaggtaccagccggaccaggtaacgggaaccggttttagggtgagttagacaaaatgggggctcatttagacatatggttggccggatggggtaacctttatcacgctgtttactcaatattaaaataacggaatacctccttagtgatcaggcggcagttttcagtaagttctgtgagggtgcaataccggacaaccaatacctcgtgtggtgtatcatcgaggtttacgaggctcatccgcaggaggatgctttcaatgacgatgctgccatgcagggagtcgaagagcgcccgcgccctgctgcggtcttccccgatatagaaccggcagtattccgtatagccggcctgtaccctcatgtcgacgataatacaatagcctttcaccatatattaacggagattttaatgaatgcttaaaatgctttccctgcacccggcaaagggtataccaggcggtatctgccggaaattttttcaggaaaatgacattttttcaattcatctttctccttctatacccagctttagtaaaacattacgggtaatccggtcgcagcgggttaaatgaaaatggtagacatgatctttcatataggcggtcagatcttccctgagcatggccttagccctgttcaggcgtacctttacattgttttcttcaatggccagtgtttcggaggtttcccggacagacatttcctcgatttcgcgcagcataaaaaccagccggtatttttccggcaggcgggtaatggcgtcttgcagtatctggttcaattccttattcgctaaatctctggccggagttttcatgtctatgaatttatctgaaggtaactgactaaaagggaggttatttttacgtttcagttcgtaacactggttgagcataatccgtgtaagccaggtgccaaatgaagcgcggtgttgaaattgtgacaggtgacaataagcattgagataggtattttgcatggcatcttcagttgcgggatcattttccaggatagacatgccaatccggtacagccgctggttataccggctgatgattacactgaacatcttcttttcacctgccagtattctttctattgcttcccggtcaggaacctgtgcggctattgcttctttttgtatggtcatgttatttagatgaagtaagaggagaaaggttacagaaaattactattgatttcctgtaacctttttgtcaatagcctctctaattaatacactaaacatatgtatcatggcaaccataaaacagcttcaaagcaccttacgcctgacctttggcattgtgcccattgtagccgggctggacaaattcactaacctgcttacccactgggaaaactacctgggcagtaatgcagatatgctcccgtttgccgccgccaccttcatgaaaatcgtgggtattattgaaattgccgccgggatacttgtattggtgcgtcccctggtcggcgcgtacgttgtaatggcctggctgatatgcattgcactgcaattgcttcttggcggtcagtacttcgatgtggcggtcagggacctggtgatggcaatcggcgcctatacgctggctcaactcacaaaaatgaaggaagcacattcgtaaaggaccggttaaccggcacgccgctggttaaccggttacagttttctgaagtccgacggcctcgcatgcaggaatcccctgaatgtatcgctgaaggaattgatgctgctgtaacctaccgcaaaagctatttcattgataggcttacttgtttttaagatcatttcaatagcttttgtcattcttattgttttaagaaattgcaaaaatgaaattttaaggttagcctgaaataaccgggagagggagcgttccccgatattaaattgcttactgatgctggtcagtgtatgctttttcccgatatttttttccaggtaatcaatgatatcctgcatctgttcattgttggtagcaggcaaaactatagggagcgatttcctgcttttttcaggaaggatctttttcagtgctaccaggaattcaaagttgggatccgtgttatcaacatgttttccatcccaccgctccgtgtaattgatcatctggatcactaattcgctggcagggtaaattcccagcctgttataaaaaggatccctggtatcatcgtgggcgtaaaaatagagcgaccgcagcacagtggctttatagccgatccgcagtatgtgcggcattccctgcggaatccagaagtaatgcctggctggaactatataagtaaggctttcaacggtaatataggcgattcctccctccacataacttaattgccccttattatgccggtgcagagggatcagtttttccgatttctcgtgcatgacaaaaacggaatttttctttttctctatatccggtaatgaagcaattaagcccataagattatttgaaatgtaaaataataaggtgagagaacaaaagtagcatttgtccggaatcatgaaaatattgactaatacggtgaaattaacaatagctcagcttgtagggaaataaccttaaattagcgctctgacagatcatatgagcgtatccattaccaccttacagcagttattatttgacctggccggcgtgctgccggccgacaccgcgccgttatttgccatgacgcggcaggtaaagctggcggccaacgaaacgtatatccatgagggtgataccgaacgccgtcttgcttttatagaacagggcatcatgcgggcctatattattaaggataatggcgatgaagccaccttgtttctgcgctgggaaaagcaatttatcgcttcgcatgatactatcattcaccggcagccttcccgttttatataccgtgcactggagccggtcacattgctggaaatagattatgatgtgttggaagaagtactgaaaacgcacccggaatatgaaccgctgcggaatttcttcctgatgcgcatgttgtccgagtcgttaaaaatcatggaatcttttgtcacgctgtcgccggaagagcggtaccgtaacctgctgacagagcgtttcgacctggtgaaccgggtgcccgataaatatattgcttccatgctgggcatcacacccgtgtcgttaagccgtatccgcaaacggatgcttgataaggggaagggataaattatcctttgttaagcagcgaaattatcttttgttaactacatctgccatagcggttctctaattttgagagataaatttctcaaggccatggaaccgatcattgaagctaccgttaagatctttagcatgtctgccctccggtattttgtgttggcgggtattccttttacattattctacctgctgttaccagacaggtttaaacatttcaagatccagcagaagctggcatcaaagaaagattttctccgggagatctggtattccatgcaaagcacgctggtgtttaccgccattacgattatactgctgtttacgccggtgaggcagtataccatgatctataccgatatacaggcgttcccggtgtggtacatcggcgtaagcctggtggggagtctcgttatacacgatacgtatttctattggatgcatcgcctgctgcatcataagcagctgtttaagcgcacccacctggtacatcaccagagcatcaatccttctccctggacttcctacagttttcatttcctggaagcggtgttggaaggcggagtgctggtggtgattacgagcgtaatgcctatgcatccggttacagtgctgttgttcaccgtatccgggtttattatcaatgtatatggccatctcggctatgaactgatgccacgcgggttccggcatacctggttgtttgaagtgttcaatacgtctgttcaccacaacctgcatcacaaaaagttcaggggtaattatgggttgtatttccgggtgtgggacagggcgatgggaacagagcaccccgactatgtgaaggagtatgatcagctgcaggagcgaaggtttggggagaagacagtatggagtaattaaacaaatatttttaaaagcggatggtttaccatccgcttttttttaaccgaaattttttttcactgtagaaatatcgcagtggaaccggatagttttgttcctgcgcgaaataaccatataaccatataccacgatttttgtaagaacctttaacccaggggaagcaaacgcccctttttcttaatttctaactattattctatgaagcccaaacacgctcccgtggagcaaaactatgcgtatgaaaatccggaaaattttatggtacagggagagcaatggcgctacgaccgctcggccactgttatctctcttttcaatcagcaggctgtacttaacccggatcgcactgcggtggtattcgactcagctgtagtcagctacgacaccctacaccggcgatctaaccagatggcgcattacctgctggagcagggggtaaagccaggtgatattataccggtatggatcgacaggtccgttgaatggctggtagcagtaactggcatcttaaaaacgggtgcggcatatgtgcccattgatccgtcctatccgcttaaacgggtacaggtgatactggaagacaccggaaccagctgcgtgatcacgaccagtaaacatacattaccggatgccggtaagtatcactatgtgatgctggattcgctggacagtcttgatgaatggccagatgccctgccggaggtaccggtgaccgccgatgaccgggcatatatcatctatacttccggttctaccggaatgccaaagggcgtgatggtggcgcaccggtctttacaacacctggtaacctggcatcagcaacggtttgaggtaactgcaaacgaccgggttaccctggtggcgggaattgcttttgatatttctgtttgggagatatggactgcacttactaccggcgctacgctggtgatagccagcaacgaagaaagaacggatgcagcagcgctgttgcagttctataccaggcatggtatcacgcatgcttttgttcccaccgtgctggcgccggaagtagtagcactcagccgctctgttccccatcttcacctgcgctacctgtttaccggcggagaaaaactgaagccagtacgcacacatggcctggattatcaactggtggattattatggtcctactgaatacagcattttcgctacctgccggattgtgcgcgatgaaaacggggagtatgtaccgtccatcgggcaaccggttgccaatacacaggcatatattttaaaccaacacctgcagcccgtgcctgcaggtggtattggggaactctatctcggcggggaaggactggcactgggatattggaacagacccgcgcaaactgcagcatcatttattgaccatccgtttatacctggtgcgcgtttgtataaaaccggtgatctcgtctccttattgccgtcgggtgaattaactttttcagggcgggtcgataaccaggtgaagatccgtgggttcaggatagaactgggggagatagaaaaagtgctgctgccaatcgatggtatcaaagacgttgctgtgattacacgcgacgatgaaaaacagcataaatatattgttgcttttttagtgaaaaactgggaagcagcagcgccggaaatcgcggccatcagggcggtgctaaaagaggcgctgccaggctacatgatcccttcgcaatttattttcctggataaaatcctcgtaacccccaatgggaaaacggaccaggcgaggttatcgcagctggccgctgcctatgaagaagaagcagtgtatgaaccgccggtaacagatatggaaataacggttgctgctatctgggaaagtgtattggggcggaaggccatcaacaacacggataacttctttgatatcggaggcaactctgttcgggtagcgccggtagtaactgcgttggggagaaggttgtctttgaaagtatatatgagagatgtataccagttcccggtgctgaaagacctggcgcaaaccctgacggcccggcaggcacaggcggataccattgtgatggaggaagacgtggaaccctatgtagcattacagcaggatgtgtacctgaaacccggcactgttatccgtaaggattttgacattataaggcttcaaaacccgggggcaatattactcaccggcgttaccggttttgtaggcattcacctgctgaaagacctgctgctggcttccaatgcaaaggtatactgtcttatcagggccagtaacgaatattacgcgatggaacggatcaatggatacctgaacaattatcacatccacctcgatgaatcgctgcgccagcgtattataccggtaacgggcgatttctccaaaccggatatgggattaacggaaaccgggtttaaggaattagctgataccattgatgtgatttatcattcgggcagttccgtcaatttcatcgaaccttattcgtatatgaagtcggccaacgtggaagggctaagggaaattatttcctttgcagctgccggtaaaacaaaatgcctggtattgctgtccactatttctgtatacagctgggggcatgtgttcacgcataaaaccgtgatgaaggaaacagatgatattggccagaacctgctggcggtgagcaaagatatcggctatgtaagaagcaagtgggtgatggaaggcatcgcagatcttgcggctgcgcagggattgccggtaattacctaccggcttggctatgcgatgtgccatagcgaaaccggcgccagcgcaccttaccagtggtgggccggattggtaaaaaactgtgttgagtttaatgcgtatcctgcattaaaggagttaagggaaggcctgattacggtagattacatgacaaaggccatcgcttatatttcaaaaaaggagacagccctgggtctaaaatttaacctgattgccagcccggaaacgaaccttacgttgcagcagttttttgacctcttgaataaatactattcttttgatctgcgtggcctgccatataaagaatggagaaagatatgggaagatgatcctgccaacaggttgtatgcgctcaccagtttgttcaaagacaatatgcacgaggggctgtctaccgtagagttgtaccaggatacctacatttgggataacacccatgtggctactttcctggaggggagtggtatagcggaacctgtgtttgataaggaattactggatcgttatctgcgatacctgggtgtgttgccggggctctattcagaaaaggcgatttatcagcagtgatttataaaagatgcccgccaggaacaaccggcgggcatctttattatattattttaatgtccagagacctgggctgccgggctttctttcatctgttgcttttttaagcaaggtatcgccgggagagaggttgccaaatatttcaatgcctgcatctaccgtcatgccctggcgtacgtccacccattctgcctggccctggtgtactctaatcacaaacttcctttcctgcgtagtggctacggctgcaaatggcacgatgaaggaagtagtgccgcgttccagcggcagctttacatatgcaaacgatcctgctttaagtaagtgatcactgttatctacctggaactcccacaactccgtgcgggtgccgggatcgatggtttcagacttacgggtgagcgtagctttaaagcgctgggtagggtaggcatctacgcgaaagtcgatgttttttgacgggcttgcggcagcggtgtatatctcgggcacggctgcacgaagacgcagcgtgcggttattctgaacggtgagcagcatggcgttggtgcctacgagcgcaccgggatcggctttacgcgcggtaatgatgccatcaaaaggcgcggtgatatacaggtagccggaaacttccttgtaggactgcgattgtttgctggcggcaatgtaagtggagctgtcggccagcatcagattgcggcttcgctcgaggtctaccggggcaacgatgcccggtgttttcgcctgtgatgccctgtagaggcgctcataattatccctgctggacgcccatttcgctttggcggattgtaaagcagcttcggattccgccaggcggctgttgatttccggggcttcaattactgccagtgtttgtcctttttttacgcggtcacccaggtccactttcatgctgcgcacaaagccctgtactttggcaaataattcagcggtttcgtaggggatgagttctgccggtaattcaattgtttttttaacagtgtcctgcttcaataagaataccggcacggtatccgctgcggcactgtcatttttatgctccggttgctgcgctgcgttgccgcaggctgccagtgttataaccaaactgataaacgcgaaagatcgcatatgattaaatttattttttaagattgtttgtcgtgatgaatactgtttacatcatccggatctaaagataccgccacaaatttccttcttccaacgatcagctggtacacctgcggcaggaaaaataatacgctgatggctgaaaataaaaggcctccgatcactgcgatgcccagtggtgcggtttgatcgcctccttcggagaggcctgctgccattgggatcatgcctgctatcattgcgacgctggtcatcacgatgggacgcaggcgtgtttccgctgcgcggagatgacctgcctcgatcccttctttccggttatactctgcaccggtaataaagagcacggcgtttgcaatggccacgcccaccgccatgatggcgcccatatacgactggatattcagcgtgttaccggtaataaaaaggaacagcagggaacctgctaccaccgcgggtataatggacaaggttgccagtgccacgcggaacgattgaaagtaaaccgtcatcagcaggaagatcacgacgatagcgatcaacagtccaaactgcaggctggtaagcgtttgctgtaacagttgtggttgtccgcgaagcaggatctttgctccattgggcagtttacccatgccggaaatgatgccgtttattttattaaacacggttccggcgtcctgccggtggatgtttgcggtgatggtgatataacgttgctgattgaggcggtcgtattcaccggcaacaacggtgcgtttccacgtggctatttcactgaggtagtgggtgtttccaatgccgccggagatcggaattgcttccagttgcgcggtgctgttcatccggtattcggggtattgcacctgcacctggtaggcggttccggtcgatttatcgagccagtaattaggcgacgtaaagcggctggaggaagtagcggtaacaacagagcgggcggcctgttcgccggagatgccgagctgtccggcttttacgcggtctatttccagcctgatggccgggtaatccagcggtgtggcaatttgcagatcccgcagcgaaggaatggccgacagctgatgtaccagttgctgcgctgttttcctgccctctgcgaggttgcggtttaccacagctatttctatggggttcgtgctgccgaggttcagcacctgttccacgatgtcgcccggttcaaatgaaaccgtggctttcggaatttcttttgcaacggctgcgcgtaatttctcccggaaaacagctatcggaatcacatctttattcaactttatttttgttactgattcatgcgggccaccggtccacagatgaatgtagtttacggggaagctggacggctgtgtgccaataaaggcagaagtgatgtcggtgttccctttgccggcaatgctgtcggacagtcgcaacagtttcctggtagcatcttctgtacgttcaaaacgggtgcctacgggcatgcgtaaacgaacttgtgtttggccgctgtcggtttgcgggaagagttccgtgccggtaaaatagaacaacactcccacgagcagcaatgacactaccaggaacagggtggtaagccatccaaagccggtttgaaagcgttggccggtgttggtataccgctgttgcaggcgatggtaaaagccggtgttctgttgggtttgatgatcctttagcaaccagttggccgctaccggcacaaaagtttgcgatagcaggaaagaagctatcatggcgaagcctactgccagtgataaaggcaggaacatggctttgggcacgccgttcataaacagggaggggacaaataccgcgaggatgctcaggaggatcagcagttttggcgccgctatttcccggcaggcatctgcaatggcgcgtgctttatttttacccgcttcctggtgccggtgaatattttcaatggttaccgtggcttcatctaccaggatgcctactgatagggccagtcctcccagggtcatgatattaatggtttgaccggcgaggtataacagtgtggctgccgaaagtaatgccagcgggatggtcataaccacgatgagcgcgctgcgcctgtcgcccaggaaaaaccataccatcaggccggtgagcagtgcgccgagtccgccttcaaacaacaggcttttcagggagttgatcacgtatccggactggtcaaattcgtaggttacttttatatcttccgggatggccgcctgcatatcaggcagtgccgcttttacccgttgcactacctcccaggtggaagcgtcggcgcgttttgttacggggatataaacagagcgtttaccattgaccagcgcatagctggttgttacatcagatcccagcgtaacgttggcaatatctttcacatataccgccggtcctgcgccggattgcagcggcgtgttctgcaggtcctgtaatgtttcgatcacgctgttttgcggcgtgatgtaagtggtatcgccgatgcgcacattgcccgcaggagaaatagtattgtacttcgcgatggtttgtaccacctggtccggtgagaggttatgcccgcgcagtttttccgggtctatggtgatcagtactgttttctggttaccaccaaacggcggtggggcagatacgcctggcagtgttgaaaacataggccgcacgcggaacagcgccagatctgatatttctcccagcgagcggctgtcggagctgaatacgagttgtcccaccggcacgctgccagcatcaaagcgcgtaataaatggtggcacggtaccgggaggcataaatgccctggacctgttcacatagcctactacttctgccattgcctggctcatatcagtgccttcattaaattctattttgatgagggccgcgccttgtatacttttcgactccacgtatttaacgccggtgatgtatagaaagtggtattcataataagaagtaacaaaaccttctacctgctcgggcgacaaccccccgtaaggctgggcaacatataccacgggcagtccgaggcgcgggaatatatccaccctggcattgcggatggagaggaaggaaaaaaagaggatggcaataacagctaccagtatggtgacgggatgccttaatgccgaaatgattagtttcataaagaatggatcgttatttcagtttatctgtaaaaacattcaggttgccatttgccgtagccagttccagtaaagcatgccatgcctggaggaatgcaccggcttcacctgtttccgctttcagcagttcatattgtccctgcatcaggcgtgtaaaatctaccagtccgctttcgtagctgagtttcagtccgtcgaaagcataccgtgctgcctgcgattgtattaacgcctggcgtgcaatcagcaggttctggtcgtaattaaactgtgcggtttcctgttgcttttgcaggttcagttttacctggtccagttgtgcttcatcggattttaacagtgaccggtattgttttttctgaagatttacctgtgaaaactgtagtatcgggaagctaagctggataccggcgccatagttcttatgggaaagcgaccagccgtcggccttattgatattaccggcagcatccacacctgagccgcgggcataggcatttgcccagagatccagtttggggcgccatgcgcgtccggcttctttcagtgctgcttcacttacttctttttttgtttgataatattggaaagaaggatgtgctgtaaggttggtggtagtatcggcgccggaggggaactggtttatcagcgatgtatctgccagtaaaatatcatccggtttacccggcaggtctgccaggcggctgagttcagtgagttgtgcatagtattgccgttgagccgtcatcaggtccatccgggcctgtgccagcaccgactggaactgtgtggtatcaatgccggggcgtagtccctgttgagccagcaccagcgattgctgcaggccggcctgggtgcgttcaatattcgactggtagctcagtagtaatttctgcaggtacaccgcatccaggtaagtggatatagctaagtactgctggcggaaaagcgcttcattgtaatagctgcctgccagtttatattgagcaatggctttttcaacggcggcctggcgctggccgaaggtgagcgggttccattttaccagggcggttaatgccgtaccgggaacggggtcgtaggtattcccggcagatggagggccgctgatcggtaaaaacaaaccgggataactcatgccggtaatattgttgtaggtggcatatcctgcctggtatcctgcggtaagctccggcatcagtgaattccgggccatacgcacattgtattgcgcggcctgggattgttgttccgatgctttcacctgtggctgcgattgtaccagtgatagtaactctttgatgcggatagttctttgctgtgctataccagataatgacagcgtgatgaaacagccgctgatcagcatctttttatggtaaacgttcatttatcaaactgtttaaaagtatggtgccggtctttctggtgggaattctcccgttaagatattacaatcattggatatttttcagcaaaagtccgatgcctgctgctgccaggatgatcaacggctccggtacttttttaaatcgccatattatcaccaccgtaataatggcgatagcgatggtataggcatcggttaaagaccttttacccagcacaatcactgcgcccgagatagcgccgatagcggcggcggtaacgccatctacaaatgctttgataccgggatgtttcccgtatttcctgaaatagggcgccggtacaactgtaaagatataagagggaaagaaggtgcccaatgcagctatgcaggcgccggcaaagccggccaccaggaaaccaatgaatgctacggtgatcactacaggtccgggcgtgatcatggcaacagctacggcgtccataaactgttgctcattcagccacgcatgttccttcactacgccgccataaaggaatggaacgatggccaggccgctgccgaaaaccagtgcgcctgctttcgtaaaatacagcaggagttgccagagggtgttgcccgatgtagtaagagaagcattgaacaggagaggaaatgataacgatttgataagatctgccggcttctttttcaggaaggatattttcttcccgggggatttcaaccaccagtaaataatacccgccccgaggaaaagccatatgttttcattttctttccaaatggtgtaagcagctgtaaggagatagatgcctgtcagccatttatctgcgccgattgatttacgtgttagcttccaggcgctcatagcgatgatgcctatgacggccgctcccacgccatagaatacggcctgcatccaggggattccctgccattgggtatagatgtaacccaatatcactacgatgatgaacgatggcagcacaaatgccagtccggccagtgtagcgccgaggatgcggtaatggacatacccgatataaatgcccagctgggccgccagtggtccgggggcgagttgggccagtgccaggccttctttataatcttcttcagtgatccatttgcgttgctctaccaggtcgcggtgcatatagccggccagtgccacggggcctccaaagcccaaggcgcccaggcggagaaaataaagcactagctgttgaagcgtataagaaggtgtggtattctgatccatgcagctcaatttgggtgcaaagtgcggcaatggggtagtaaaaaatagaacgaaaacgaaggtttggtatggattttactttttcctgaagtttttttgggtgggtagcaaggacttttaaatcgttgacaaataagatgctttcaaaaaggtgagtatcacacttaaaagtgtacatgccaataacaatgttatggtcctgcaaatttgcataaaaatttacacatgcaaagcaggatgaaacgcaccctttatttattggcgttaggggtatttggtattgctaccacagagtttggcgtagttggcatattgccgcagatagcctcccattttcagatcacagcagataaggctggttggctgttgagtgctttcgcactggtaattgccgtattcgggccgtttatgaccttattgttttcgggcgtggaccggaagaaagcgatggtgtttgtattgatggtttttacgatctcgaatatcctgtcggcgctggcaactaatttccctttattgttgtttgcgagaatattacccgcatttttgcaccctgtattctggtctattgccttgtctgccgcagcgggagcagtacctgcagcagattcgcccaaagcagtgggaattgtttttggcggctttaccatagcgagtgtattgggcgtgccattgtccacattcatagcggatgtttttaactggcaggcctcctttgctttatgcgccatagtaaatggattttccctgcttggtttatgcttatggttgtcgccgatgccggtaagtgtaaaggcaacctttggtgaccaggtaaagattttaaagaaaccggtattatggatacaattgctgctggcttgtttaatggtatctgctatgtacgcgagctatggttacctggctgtttatctgaacagcatcaccagaatgaatggccgcgaaatcagtgttatgttgcttattttcggagtcgcgggcgttggcggcaactgggtggccggcaaaatgttgagcaggaatatttcacttaccactattatgtttattttgttgctatcgctggcgcacctgttgttgtatgtagccggcggtttttttatcccgatggtgatggttattattgtgtggggatttattcataccggtggtttcctgatcagtaatatcaatgtcacttccgcggcgccggagtcaccggagtttgtcaacagtatttttacttcctgtggtaatttggcggttactataggcgccacgctgggaggtatgactattgccagggcaggggtacagtatgtagcgtatacgagtattgttttgctggggctggccggggtggtatggggtttttccaggtggtggcaggggagatgaggtatagtcacactacccaagcacttccgtcaaatttttccgcagatgctatagtaaatagcattattggtactacaggagatataaaattaaaatcttgaaattaacatggggacttatgatagtcattgaaaattatttgagaaaagcaaatatcaaaggaggggtgaacggacggcttttggaaacgaaagattttttttcccttgagaatgacaaacttgtacaagataatgttgagtggtttaaagatgggcatctgatgtatattccgggagctttaataatatcagttaatggactgagggttttggattttaaggattgggattatccatattggatatatgggcagttgtgtgactttcttgacgaaattaatgcaggtaaaggttttaaattaccatatttagaatcagatagttgtatagatgtaacgccattaaacagggaactttgcctattgagttatctgtcaaatgggaacgtgctatcaagaattgattgcaaaaagaacgacttatataaagcctttcttaatggagctttacaggcctttcggatcgttgatgaacatagaggaaagaatagctcaaaagatatttcagcgttagaaagttgtttgaccaaattagcaagtacacccgaataataatcatttgctattgcttatattttatcgagctttaagggttatcaataatatgtttgttttttgttcacttgtaggttttattttttttagatgaggctatttccaaagaagtgaagagaagtggatgtaatagaacatcagcccgatacagtgcgtattcttgtggattgaatgaaattgaagtaagaaagaaatgtcattttaatcggataggacgatatctgtataatgtgccaaatgacacattgggtcaagaatcaactgattctacgcatttggtgggtggtgattatctttcagcctgattctacgtttcacgctaatagattggttccttttttagaagatacagtaggtgtttgggatgcagggacatgtggatttgaaagctctggcaaattgcgatttaaacacacaccagtcgtcatagacttctcgccgtacaatgagaatgattcaatgtttgccattattggatctaatggaaaagatggaagaccacactattattggtttaaaaagcaacccggtcactgaccgggttgtttagttatgtgcaaacctcacgacggcaaccgaaaattgtaggtaacaacccgatcatcaaccagtcaattcaatgctccccgcaatcctcattcctctccctcctccaaatactccctgtaagctttcgtcgccacagcattaagcttcgtcttatccactacattcttcccctccatccaatacataaacacgggctcaaaattaattttagcaggatccacggaataaggtccgttcaaaacatattcccagtcgtcgctgccatcagttttgaaacggtacaatatcagcgatacggtaggttgtacctttacacgggacacctgttcaatggccgtcacggtatagtcgtcgctcaggtaattggcgatgtaactgcgccccagaagctcctgggtaagcagaggacggatgtatgccaactgtttttgttgctttaattccccgatgaacgaatagcctgcactataatccgagagaatattgcggaggattttatcgtttactttgacgccccggcttattaacccgcgtgcgccaagggcacagagcgacattgtggtatctgccaggagttcgtggaagctttcagtggcggaagcaggcattcccggtagagcaagtatccggcctgtatacagcaagtcgttttcccaataccagctgctgtctgaatcggcctggcggcttttccatttttgcagctgctgcttaaatagttgtgttgtgcccggcaggagacgttcaggtttatattgactgaaccggggagcgtaccataaagagtcatcgctggtgtatgcggtaaaggcatacaggaaagtttccgagcggccggcaagattaatcatggcagggaggtacttttcatacagactatcattcctgaatgaaaaagcaaaaatattccggggaaacggcgtattggcgggcagctcgggagccaggcgcagaaaggtgaggacagccgaatctgaaggaatgccgtttataaagcgcagtatatttttgcgttgctgaatgctctctgtggccgcaaatagtttctcggctgcatgtacgacggtatcaccggttgcactttccaatgaaagcagcaaccgcacctttgcattgctggcgcctgtatctgcaggaaaaggtttgtttaatgcacttataataggtccaatatccgagctgtcgggatgcaggttgttcaggtagtcactggcttgatagaatactgatgtatcggaactttgcagatccttcaacagcatggatagcttcttctgctgcaggtggagggtatctgcccgttcccggctgcccggatgaaaagaagcaaagtattgctgggcatatcctgtggcagccagttcttccggtacaattgctgacaaccggtaaatggtatggccggcaatcaccgccttccggtaaaaccgcaagccggtattccgccgtttcagatcaacttcgtatacagataaaccatcctgcgaatatttccggctgcccatcacaacaaaggtcgtgtctatgctatgtatgtaagttttcagaagactgtcaggcttgttgtgataataaggagcatacttttctatctctatcaggtatgtcgaaagagaagcactatccatggatgtataatagttggcattaacaaacgatgattcatattgttgttcgagaggtccaccggtaaacttatctggtccggctactataaagctgctgtctgcaggtgcaaaagttacgaccggggctcgcggctgtaaaggaagaatatgaaagccgtagaggaaatgttgccagtagctgctatctgtgtgagcagcatcataggttgtcagcaggcaatatgccaaattccccctgggaatataatgtaagcgggaaataaagccattgttatgctgataggtaagctggtatagtggaagaccattcttttccgttaaaacagagtcggtcagctgtaatgtgctgtcctgctgcaatatcgatgtccgcaggtctttcagcacctgtctgtcatcagtattataatatcccctttgcattttttctacacgcagcacataagagatattatgagcgttatccaatgcagaatacacttcttcgggccgcatgcctttcttattaccaatattcatgtgattatgctcagatggcagaagcgcagaaaatcccagttgaggctgatacagcgtatcatatttggtttcaggccgaacaatatcgtagaaacgcaccgaccggaaaaagtcctttctgctactgctgtctgcttcctccgagctgtgcataaatagaaacgccctgttgttgataatgaaaacccgtacatagaaaggcaggttcttctgcagcaggatggcctctgtgcctgccatgttgcggtaggtgataggataggatttttgcaataccgcatcatcctgcgctgccatgttcgcgatcatagattgcaccagctggctccggtccattgccagttggggaatgtccatcgaaaaggcaaatcctgcttccacatcgttacctccgacgaacattttgccgtttacaccgggcaaaggatataccacaggcacacccggtaacacaatgctgtaaccatttgccatcctgttcagcgagtatcctttcaggctgtccagctgttgacgctggcgacgtgtttcgccggtgaacttggcgcttaccggggtaacagtatatcctttttcacgaagtaaggataacatgcctttttcaccaggtaaatgggcgacgcctaccgcggcgaaaatgctgtttttgttgagcattgaaacaagattgctcaccatttccttgttccggacttccaggctgggaccatcctcaggatctccccaactattcacgagctttgatatcttctgcagatcgccctcataatacaggtctgcgagttcattgagatgggttacccgtgcttcgagccggtcggttctgtctttcgcatcagcctggccggcgggctggtagccaatactccacaggaatatttccttttgtgcttccgaaacatccgcgctcataacacccagctggttttgtatcctttcgaggctatgcaccggtttattaagcctggtcgctttctgatgtaaccagccatccaggaaaatgttttccggtttttggttaggaccggcatttttattgagttccccttcttcatccacgagcagtttttcgagaaaccataagcgtttcagcttcagttgctcaaggggagaacccgtcttttcccttaccaggctgtctacgtagtggtactcctcgttgttcagtaagtgacgcatatggttaacggtatcctgcaaggggcctccgggcgacaacatgtacgccagcattgaatccatatccacttccatggcaaaagctgaggcgttacgtaatgctgtaagcacggagtcactaaactcaaacacgcgcctgtcagtaaggtgcatagtgccaaagaggtacgagggggcatgcaggccggggccatcaatgcgccaaagcagttgataatttgccctgttgttggattgggcatgtaaaaaggctgtttgcataagcagggctaacagcagggttattgctacgggtacaaaatgcccggcattttgaggccggcgccgggtacaggaattaaacatggcgcaaatgtaataatgttgcagcatgtttaaaatcgaataaaagttgtatttagaagatgctatttctatcaccgtgccacataaataataagtccccggccaacagccggggacttattattcaatccccatcaatacaacgtcctcatactcgctgcatcaaatggcttcaactgatcaaactgctgctccctcaccttcttcacccagttaggatcgtgcaaaattgaccggccaaccgccacgaggtcaaaatcgccccgttcgaagcgacgttccagttcgcgcatatccgtaaccacgtctgagttctcaccggagaaggcgcccattacatcgccggagaggcctacagagccgacagtaatggtaggctgaccgctcacttttttaatccagccggcgaggttcagatcggacccttcaaactggggttcccagtatctcctttgcgaagcatggaaaatgtctacacctgcatctgcgagtggaatgatccagtcttccatttcttttggattgtgcgccagctttgcgttataatcggtggctttccattgtgatacacggaggatgatcaccaggtcgggacctgctgcagcccttatggcttttacgatggcggttgcaaagcggcttctttctttgatggttttgccgccgtagtcgtcggtgcgtgaattggttttgtcccagaagaattcgtcgatgaggtagccatgtgcgccatggagttctatggcgtcgaacccggcttctttggccgatttggcggcgttggcaaatgcggcgatagtggcttcaatatcgcttaccgacatggtggaagggttttctattggtgcagccggcgtccatccgctcatgccgggagcgtcaccggtatgccatagttgtggggcaataacgccctgttgtgcatgaacgtggtccactacatttttccatgctgacagtgcggcggttccataaaaattgggaatgtctttttcattcttcgaggctggccggtcgatgacggtgccttcggtgaggatcaaccccacttctccggcagcgcggcgcgcgtaataatcagctactgcctgggtgggtatgccatccggcgacgccgcgcgtgtcatgggcgccatcacaaaacggtttttcaggtgaagacctctgtattgaaacggtgtaaaaaatgatgcgtaattcattgaatatttcttttacgcaaagcaacaaccaaatgcttaattttacagcggctttggagcaataccagttaccttaaggtaagtacaaatgaaagataagatattaacgaaatacagcgattgcccgatcaaacggtcaaaatcaatcatcggatcacggtggaaacctattattatttacgcattacgtaaccgtaaaatgcgcttcggtcaactgcatgctattataggcgatgtatctgcaaaggtgtttgcgcaatgtttaaaggaactggaagcagaggagattattcttcgtgaaacatatacagatactcaggcacatgtggagtacagccttacatcaaaaggagagggacttgtgccgattattgtatccctgctgcagtgggaatggaataactacgaagtaacgcctgtataaagccgacatattagtaattattaccctgttttaatgtttggcagaagctgtctgtgccagaaattcctgttcccatctttcccatatatcccgaaaatccctgccagccaatgttttcactgctctctgccggtgtgtaataatttataattatagctaatgcgaatttatttataaaataataatatttgttactaatttatgcagcaaaatagatggccattgcctttgggagacctggcttttttctagccatataaattatattccacgatatgatttatataaaagaagagatatgaatataccagatgctgaattagtagtgcggttacaaaaccacgaagtaagcgcctttgatagtttgtattggaagtatcacggcgctgtataccggaatattttcaagtttgtgaaagatgatgtggttacagaagatattctccaggatgttttcgcacgcctgtgggaaaaacggcaggatatcgagccagaccagtctgtgagcggctggctgtttgtgatcagctttaatatgtgtgtgtcttttgtaaggaaaaagctgcgtgaacaggctttccacaaaaatatcttccaaaccgatacggatgatgcggtagccattgagcgcaaaaatatcgatgaggaacaatatcatttactggaacaggcgatttcaaaactatctcctaaaaaaagaaccatcgtaacccgctgtaaactggaaggtaaaacctatgaagaagtagccaatgaactgaacatctcccgtaatacagtaaaagaacacctgtctgccgccatgatcaagctaaacgactatatgcagcgcaacggcgatcagaaatacattgtgctcctgatgctgttcctgagctaccctgattcataagcagataaacctatttcatattatcttttaattaatattttgttttttcaaaaaaagttcaaaaacgacccacccatttttattaactgcgcgtatttagattaaaccatcacgctagtgcccaacagaaaggaatatctcaaacagctgttaagtaaagatcaatggactgccacagagcaggagtggatggtagaatacctggataccaatgatttttcagaactggaaacagtagccgccgaatattttgaggccgacctcctaacggcaaagcatatattagataaacgcctgtcggacaggatgttgaataaccttcataagcgtataggcgttgcagatagttctttcaaaggaatcttccggttgtttaaatataaagcagcagcggccgccgccgtactgttactggcaggagccgcctggtacatgctactgcacgaccgcgtaaagcaaaaagtgtttgccaccacatcagaacggcaaaccgtgaaactgcccgacggttcagtggtacacctggagaaaggctccagcattacctacccggaagtgtttgataaaaaaaatcgtgaagtaatattaaaaggagaagctttcttcgaaatcaaccacgatgcaaagcacccttttatcatctcctcttcgctgatcaatactaccgtattaggtacctcctttaacatggaagtacacgaaggcaataccgccagggtagtagtggtatcaggaatggtgcaggtgaatacccgtgaaggcaaaccgcataaaaacggccaactggtactaacagccaacaaaaccgcggtatacaacccggcctcgcaggacctgttgttacaggacggaacagaagatgccaaattctttgcccagaaaacgagtggcaaatttatttacaaaggagatccgttgtcaaaagtggcaacagacctgcagcgatattacaatgtgccggtaataaccgaccaaagatcggcacagtgcaggttttacggatcatttaatacagtggacgatttagaaaaagcacttgcgttaattgctttttcattagatgccagagtcaaaaaagataatatcaataaaggatatatcatcgttggtggaaattgtaagtaaaataacgaccgctatatcgttaaccaaactatatttcaaatgagaaactgctatcaacaaagctgaaccaaaatttaagagaatagaaatttcagtctggtatactatcctggtggccttttagcctgaaagaacttcatgctggttagttaactagtgatcacgaaaactgatcacagggccacctgttgccaatacttaccgtgaataaaccgtagaattattttcaaccaaactaaactgtacatgatacaagtaatacccttaccgcccggctaatatattgccatgatatagttgattgaaaaacaccctgcttacgcagaaggccctttattgcccggttttgtccaaaaaccggaacggggaacctatggccgaacgaaaccaataaaaaacaattatgttcagaagaaaactatcattcatctattgcttactgctcctgctggcagtaacgcaagcccacgccggcaacggtttgcaggacgctcttgataaaaaaattacgatcgaactaaagaatgtcatccttaaagacgcactggaaaaaataggcagcctcgcagaagtttcctttgtatatgtaggcaatgaagccctggatgtgaataaggtaagcgtaaatgcacacaacgagaaagtaggcgacctgcttaataaactgcttacgccctattccctttcctatagcgtgatgtacgaccgcgtagtaatcaaacacgacagcggcaaaaaactgaatcaactaacggtaacgaatacactactaaagctcaacgttcctgttacagatgtaaaaggagtggtgaccaatgaaaagaaggaactcttacccggcgtaagcatcatgatcaaaggaacttcccgcggagtgactaccaacgataaaggcgtatttgaactgaagaagatcgccaacgatgctatactggtatttaattttaccgggtataaaacagaagaaatcagcgtggcggaattcagaagcggcacgcttaccatcatactgaaagaaaaacctacccgcctccaggaagtggtggtaaccggtttccagagcatcgataaatctaaattctccggcgccgctacccggctgaaaggagaagatgtgaggatcgatggtatgacagatgttagtcgcatgctggaaggtaaagtagccggcgttgccatccagaatgtatccggtaccttcggctccgcccccaaagtgcgcatccgcggtgctacctctattaatggcgacaacaagccattatgggtggtagacggcgtagtactggaagacgtggtaaatatttccaatgatcagctttccagcggcgatcccaccactctactcggttccgcagttgccggcctcaactccaacgatatcgaaagcttcgacattctgaaagatgccgcagctgctgcgttatatggcgcccgcgccatgaacggggtagtcgtaattaccactaaaaaaggtcgtgcaggcaagcccgttattaactacagcggcaacttcagtacgcagctgaaacccaactacaataacttcaatatcatgaactccggtcagcagatgtctgtactggcagaactggaaagaaaaggaatccttaactcagatatcctttcacgcgctgatatcggcgtattcggaaagttatatgaacaactggatgcagatggaaatggcaacttcccggtagaaaacgatccgcaaagtaagaaggcttttttactgcgttacgcgaaagccaataccgactggttcggactgctcttccgcaacaacttcgtacaggaacattcgctcagcatttcttccggtacggataaatcacaatcttatttttctaccagcttttacagtgataacggctggaccctcgcggataaagtaacccgttacacactgaactaccgcaatacctacaaactctcagaccggttatctgccggattttcctcactggcttctgtgcgccgtcagaaagcgcccggcgcccttacccgcagcagtaaccctgtggaaggacaatacgaccgcgatttcgatattaacccattcagctactcgctgaatacaagccgtacacttactgcctatgatcaaaatggacaattggaatacttcagaagaaactatgctcccttcaatatcatcaatgaactgaaaaataattacctcgacctgaacatgatggatttgcgcctgcagggcgacctgactttcaagctgacaaaaaatatccgctacgaatttaccggtgctatcaggtatgtaaaatcatcccgtgaacaccagattgcagagaatgccaacatggccaatgcttaccgcgctgccggtaatgctaccatcgcggaaaggaataaattcctttaccgcgatccggaaaatcccgatgcacaaccggtaattgttttgcccgccggcggtttctataaccgtacggaagaccagctgctgaactatgatttccgcaatggcctcaactactccgacaccttcgcccagaaacataatatcaacgtattggtaggtcagcaggtaaaatatgccgaccgccagaacgcttccaataccggctacggttaccaatacgataatggcggcgccactttcactgactaccgcattctcaaacaaaccattgaaagtaacttcccttactttggcatgagcagggactatgatcgcttcgccgctttctatgctaccggcacctatgcctataacaacaagtataactttacagccaccggccgctacgatggttccaaccgcctcggacaatcccgtaaggcaagatggctgcccacctggagcgtagccggttcctggaacatcgacagggagccttttgcggccagtatccgccagctggactatctcacgctgcgtgccagctacggcttaaccgccagcatgggacccgccaccaattcaaacatcgtataccagaccgttaataccaacaggcctcacctcacagaagtggagtcagtgatccgcctgtcgcacctgcagaatgatgaactcacctgggaaaaattatataccaccaacatcggtgttgacggaggctttttcaatggtcgcctcaacttcagcatagacgcttacacccgtaaaagctttgacctgatcagccgcatcaaaacttccggtatcggcggtgaaatgtttaaggcggccaactatgccgatatggattcaaaaggggtggaagtgatgataggcggagatgtgttccgtagtaaagactggggctggaaatcgaacgttacgctcggatacagcgtcaataaaatcaccaatgcaaaaaatatccccggtattttcgacctggtggtggcagaaggtggtaacaccgaaggctatcctgtgcacagccttttttccctgcaatacaccgggcttgatcctaaatcaggctctccggtgtttatcaaccaggacggtgctgtcagcggcgatgtaaacctgcaatcattaaatacagcccacctggtatacgaaggtccggttgatccaccggttaccggcgggttctccaatactttccgctataaagcgctatcactgaatgtatttttcacttaccagtttggaaataaaatccgcctgtacccggctttcaaaacttcctattcagacctcgatgcgatgcctaaagagttttatgaccgctgggtaatgccgggagatgaaagcaaaacaggtgttccctctatgctggatgcttttgagcagatattgctgagaggcgctcacccttacaataactataactactctaccgaaagagtggcgaaaggagatttcatccgcctgaaaacagtgtcacttacttaccagctgccgggtgtaatcatcaaacgcgcaggattaagcaatgtggctgtaagcgctgctgccattaatccatggctgatctatgccgatgaaaagctgcagggtcaggatcccgagtttttcaacgctggtggcgtggcacagcctatccagaaacaattcactttttcattgaaagtaggtatttaaaaagaagcactatgtcaatgtactatataacctccgcgaataaacgaaaaataaagcctgccatcatcggggcatttgcactgatggcccttgtcaccggagggtgtaaaaaatacctggaacaggtaccagacagtacctggacagatctcagctcgccagtaaaggtgagcaagctgctgggaactgcttatccgcaggccagttacatcacgatgtgtgaagccatgtcagataatgtgggcgacaagggagtgggagagtactaccgccctaacggtgacgcctatctgtttaacgacattcaatggatagaggaagactctccggaagcttactggagggcttgctacactgctatcgccgcagccaaccaggcgctggttgcctgtgaaaaggccgccgatccggccgcttatacccgtcagcggggcgaagcgctgctggcaagagcctatgcccactttatgctggtaaatatttttgccaaaacctacgatgcggctaccgctgcaaacgatccgggaataccatacgtaacagtaccggaaaccgtggtaatgaaacaatacgaacgcaaaacagtggcgtatgtgtatgacatggtggagaaagacctgctctccgggttgccgctgatcagtgacgacgcctacagcgtaccccgtttccattttaaccgcagcgctgcttatgccttcgccacccggttctacctgtataaaaaagattacgcgaaagtagtagcctatgccgacaatactttttcaaacaatgatgtggcctccaacatgcgcctgtggaataccacatatggcagcatgtcgccggcgcagatctttgatatttatgccaatgccaacgaaaaagccaacctgctgatcgtggaagcgccttcgctgtggggccgcaatgcgggccggctccggtatgacctcgacttccagcatgaagcgctcatcctgggcaggaatgttaccggcggcgtttggtcctacccgttatactactacggctcacaggattattttgtgccaaagctctctgagtactttgtaaagaactccgtgaatgctaccattggtcagccctacgtaatgacaccgctgttcaccacggaagaagtattgtttaaccgtgcagaggccaatgtgtatctcaacaacaccagcgccgtactaaaagatcttaacctgtttgccagcaaacgtatccggaattataatgcctccctgcataatatttccctggctgctatgcagaatttctacggtatcagcgatgcgagaacggtttgtatccgcaccatccttgacttcaagcgtgcggagtatgtgcaggaaggccagcgctggttcgatctgcagcggtataagatccccgtggtgcacaccacccgcgaaggaaaagtactggagctgaaagccgatgataaccgccgcctgttccagataccggcgtcggccactacctcaggaatagcattgaatccaagataataatagcgatagtaccaaaattaatacatacacaaatgaaagcattcttactcatcatccctctttgcttgctgatggcctgcagcaaaaaagaagacctgggcaatgtggaagatattcccggcctcggcggagatacctgggccgcttctccattggataaatggctgcacgatacccttaccgtgccttttaatattgccgtgaaatataaatgggaccagttcgagtttgaactcaacaaaacattggtaccccctaaagaagagaaaataatcccggtgatgtcggccatccggcaggtatggatggacacctacattgcggaagcgggcgctctcttctttaaaaagtattgccccaagtattttattctctccggaagcgccagctggaatgaaaacggcaccatcacccttggcaccgcagaaggcggccggaaggtagtgttgtacctggtaaacgatttcctcacaaagtcgatggaaggctacaaaccttccgactccgccaacgtgaaacagatgttccatgtcatagaacatgagttcggacacatcctgcaccaaacagtgatgtacccggtggagttcaaacgcatctgcgcgggtttttacaccggtaactggaacaacatctccgatatggccgctcgccgcgatggctttgtaacgccctacgcgatgtcggcctttgacgaggactttgtggaaatggtatctaccatgctggtagaaggaaagcagggctttgatgccatcgtgaacagtatcccggaaggaaccagcatcaacggcgtaaccaaagcagaggcgcagtcgaggctgcgccagaaggaggcaatggtagtcagctatttcctcaccgtatggcatatcaatttttatagccttcaaacccgtaccaggaaagaaattaatcagttactctattaaaacgaaagactccggaggagtaaaaataatagtatgagaaataatctgatctgcttattcttcatcatcaccgggatgtttgcctgtaaaaaggaaacagatccgctgtttgataaatcaccggacgaacgtatcaatgatacattggcacggtaccagcaggtgctcacaacggcgccttatggctggaaagctttcgtatatcctgccggcgttccgggcagtgtatttggcttttactttagtttctctgatgctaaccgggtgcagatgttttccgacttcgatgcccccagcacgggaaccatgcgcgaaagcagctggcgactgaaagcattgcagcaaccctgcctgctgtttgatacctattcctacctgcatgtgctttccgatccggatgctggtcagaatggcggccaatacggccagggccttggctccgattttgaatttgctattaatggcgccgcgggcgataccgtttggctgaccggccgtttccatggcagtaaagccatattggtgaaagctacgcagcaggataaggataattatttccagcaccgtattaatcgctccatcgatagcatcggcgctatacttacttatttccacaagtttaccacaggcggcaaccggtatgatatcagtatcaatccctacctgcaccaggtaaattttacctggatctccaacggcaaggtaaaacaggcttctaccggttacgtatacacggcaacaggtatttccctgatgccggcatttaccgacagcaccatcactattaatagtttcgaccaggtgaagtgggaaaatggcgccattactttcacggtaaacggtaaacccgcagccatcacggaaacggtaacgccattggcgattgatgcagcagctcccaaaagatggtaccggtacgcgttgcagaacgaaagctactgggctacctattatggcttccatgtaaatggaaaggacgacgcctgcggtatcaccggcctgccagcttatgctttcctcacttactatccccagatagacggccccggtacttccctggacttactcggttttgttgtgaagcaggaaacgggcgaaaatgtgatctcttatggtcccggctacgacgcacccacctttacttcggatggcaggatcatttttaatgataacggcttatatggcaagttgcccgccgacagaaccgctatcaataaaacgaggtcgctgatggccgatccgatgggcttttacctggtacaaaccagctcccttacctacgacatggtaagcgcccgggatggtaaatcatggatcaactggcagggattctaaatgcattcaaccaaaattcaaataacctcatatgagaaattgtactgttcattatctatataaaacaacattacttgtaggagtattgctgatgctggcctgccggttgtcggcacaaacggatatcggcattggtcaaagcacttccggtaacaccaacacgggatatccgtgcccgttacaggattactatgaaggcaccaggacgcaatacctgtaccgcgcttcagagctgcatgccgcaggaatgaatgccggtgttatcagcggactgaaatacaaggtgctcaacctcaacggcgccgatacgatcgagcagtataccataaaaattggcactactactgatacggcgctggacaatagcacctgggtacccattaccaaccaggtattgggtccggttaattatctgccgaaaacaggtgtcaatgtttttccttttggctctgcttttttctggaatggcacagataacatcgtagtggaaatatgtaacggtgcgcctgattcagataacaatgttacctatacgaataacccggaagtaccgtatacaacaggacttccttttaacgcgtcacatacctaccgctccgacggactgaattatttgtgcggtaccaccagcaccactaataccggtaccatgaccacccgcccggatgtgatcttttcctggacgcccgctgtggcctgtaccggtacgcccgctgcaggaactgctaccgccagttcatcaaccgtttgtatgaacgggcaggtaaccatcaccttgtccggcactactattgcctccggtattaaatatcaatggcagaaatccactgataatactacctggaccaatattcccaacgatactaccaaccgcctggtaactacacaaccggctactacttactatcgctgtaacataacctgtgtcgcttccagtaccactgttacctccaatgcggtaacagttacttctccgcaggcggtgtcaggcgtcttcaatattaataaggccctgcctaccggtggtaacaactttgcctccttcaatgatgcctataattttattaagtgtggtatcaacaatgccgttgtatttaacgtggctcccggcagtggcccgtacaacgaacaactgctgatcacaccggtaccaggtgcctctgctaccaataccattacctttaacggtaacggcaacacgcttacatttgcgggtacctcttcagcgccggcagtgatccggttgtcggacgccgactattttacttttagcaacctggtgattaaaaccagtggcgccagcaacggatggggtgtacatctgatcaacgatgcagattataacacaataaagaactgtacattcctgctggattctaccgccagttccaccagtaacgcaggtatcgttatcagcagctcgcttacttcagctactactaccggagaggcgaaatgtgatttcaatatcttctctgataatattatcaatggcggttactatggaattgcattaaccggcagcaatacttttgcaaatggtaataataaagttaccggtaataagattagcaatttctacagctatggtatctatgtaaccggctcttttaatacgctgatagaaaataataccatcagccggccggcccgtaccggtgtaggcaccttctacggtatctatttcacgaatctcagtacaaaggcaaacgttacccgtaatatcatcagcaatccttttggaggagcgcctaacagcaccagcgcggcttacggcatttatttcagcagcaccgatgcactcgcacagctggaaaacgtagtaagcaataaccttatgtataattatacgggtaagggagatgcttatggtatttacaactcaggatccgacaacgtttggtattaccataataccattgcgctggatggaactgccactacaggtactacctataccgcccgcggcttttatcagacatccaaggcagacggtatcgaatttttaaataacctcattgctgtaacacgtggtggtggcggcagcaagtattgcatatactttgctgcaaccaacggtactattcatgccaacaggaatgattactacctggctgccgccggtggcaccagcaatgtaggctactttggcgctaacaatgcggcgttgctcgattggcaaaccgcttctgcacaagatagcaactcggtaagttccaatccgctgtttgtatctgtcagcaccggtaactatcagccggcgaatgcttctatcgataacaaaggtgtaccggtaaatattactgtagatattaataatgcagtaagaagtacctccacgcctgatattggtgcatatgagtttacgccgggtccctgcattaatccaccgctggcaggtaatgcacaggtaagcccatccgtgatttgtgtgaaccggaaagtggcgttatcactcacagataattctatcgggctcggacaaacctaccagtggcagcggtcagctaccgctacgggtacgtacaccaacattggcaatgtgcttaccaacccggatacagtgatcacagcggttataacgtcttattatcgtgtagccgttacgtgtagtggtaacaccgtgtactcacaaccaatactccttactgtaaaccaggcattcccaggtggcggctataccattaataaaaatgcaccagccagcgccaccaacttcatcagctttaacgctgccaaagcggcaatggaatgcggtatacaaggccctgtggtaatgaatgtagtagctggttccggtccttacctggagcagctgatcctcgactctattgcaggcgcctctgccattaacaccatcacctttaacggtaacggcaatacgataaaatttgcacctaccgatgataatgaaagggccgtgataaagttgcgtggtgctgatcatattaccttcgacagcctaaccatagacgctaccagcgatgattatggctatggtgtgcagatgctcaataacgctgatagcaatactatccgccgctgcaacctcatcatagatcaaacaggtacctacaatgagtttgccggtatcgtgatcaatggtagtgaatccagtccaaccaccggttccaacaacgattgtgatggcaatatcatcacaaaaaacaccattaccggcgggtataacggtgtgcttatctatggcgctactgcttctatccccacacgtaatactatcagttacaatatcataaaagacttttatgaaacaggtattacggtaagctataccactaataccctgatagatcataatgatatttccaggccgggccgcgacaatgacagctactccctgtatggtatcagcgttgaaaacaaagcagctgatgtggtggtgagcaataaccgtatccataacctgttgggcggtgcaccaggcagtacttctactgtttatggaatggagttctcttatgcagatgcaaccgccactaacccggcgaaagttttcaataacgtgatctatgatttccgtggtcagggtacgcagtatggattctccaactacagcgccgactatgtctactattatcacaatacaattgcgctgaatgatcttaagagtacctcttctgatgaagctaccggcttctatcagtcgggtactgctacaggtatccagttctttgataatattcttgatgtaagcaggtccggtaaaggaaacaggagaggtttgagcataggcaccagcacggtgcttacgtccaattacaatgatatttatgtaaaaagcaattttaatacagcttatataggcggtaactatcctacacttgcagcatggactgccgccactaagctggacagcaactctttgtctatccaacctgtgtttgcagatcctgttgccggtaactacgcaacggttatctctccactggataacaccggtaagccggtaggcattactaccgatatccttggtgtaaccaggagtactaccaaaccagacatgggcgcttacgaagtgagcgtgcctaattgcagcaaaccagtggtaccgggtacttccaccgtattcccgcttacaccggtgtgcatgggtaccgatattaagctggatcttaccggcaacagcacgggtggcacacaaacctaccagtggcagcgttctaccaccgctgcaggtccatgggtaattgtcagcgattcacaatatgtgagcgtatttaatactaccattggagtagaaaactactaccgctgcttaatcatatgcggaggcaccgacagcgcttattctaccgtggtaaaggctaacctgaacccgccattgctggcaggcacctataccattaaccctgctgcgcctaccagtcttactaacttccagtcgttcagcagcgctgtatccaaactggaatgcggtatagccggtcccgttaccttccttgcaaaggcaggtacctatacagagcaggtcaccatgcatcatatccccggcgcttctgcggtaaacagggtaaccttccaaagtgaagccaacagcgcagctgctgtaacgcttacctacgccggtacatctgcattgaattatgtattgcagctggatagcgtagactatgttacctggagagctattaccattaaaccggcaggcaccaccaacgcaagggcagtggtgtatgccaatgcatcttcgtacgacagcatcgctaactgcgccattccgctgccggttagcaccagcaccggtactgccgtgagcggtgtgtatgccgatgaatgtatcggcactggtaacgtgatcaccggtaataccatcaccaacgggtcgaatggcgtttactgggaaggcagttacagcgccgttgcacgcggacttgtactggatagcaatattgtagataaaccatattcaaacggcttgtatgttgagtacgcagatagtgtgatgatccggcgcaaccaggtgaacctgggtggtaacatggcagctgatgcctatggtatccatacagataacaccaacggctactcgatttcagccaacaacattaaggtaaccaataccaccgatgatgttcacggaatatacctttactacgcgactgctgatgccggcgtaaaaggcattgtatccggaaacaggattactgcaagaggaaatattaccggggaagtccgtggactggaactttaccaggcagatggggctaccatctccaataacgtgatcagtgttaaagccaatggtgtgaatgcgtacggtatttatagtgaaagcagttccaacctcagctactacaataactcggtactgaacagctccactaccaccggcgataactatgctgcatacttcaggcatacggcgtcttactatggtaatatcaaagtaaagaataacatttttgcttcagataccagcggtatcgccatgtatatcgcgaacccgctttacatgaagagcgattataacacactgtatacaaaaggtaccgtgctggtgaaacagcttacccctgcgggcagctatgctacattgcatgactacatcacagcggatacactggatataaattcaattgtatacaaacctgcatttacagatgataccacgctgcaaccagccattgcaaagcccgatgtatgggctatccatggccgtggtgtgcagatagaaggtaatgacaaagacatcaacggcgttgccagggcggttaaactcaccgacggcgcgccggatatgggcgcttacgaattcctgcccacttccgtgccaccggtgctcccggcattcccggctacaccggctcccggcgttacccaaacatttatgtttggtacggacacggtaacaaaaattacctggaacccgggtacggcgatacccaataacatagcggtaagacgctactccggtattaagccgccaaacctggctacaggcagggactttatgtatttctacaccgatgtggatgtaacaccggccaatggtcagtataactttaacatcgatcagttctatatcgatccgtggcagggttatatcaggcgccagaaggatatccggatgggccgcacagacagtgccaatgcatggatcgtggattcgctgagccatgtatatgatatcccgaatgtgatcagggatagcgctgtacacttcctggataaattcaccggtctcaatggcggcacggctacttctcaattgctccagccggccgacagctccaaccgcggtacccgcttctgggtaggttatggtcaccaccagttcttcaccggggacaactcgcagaacatggtgctgtacctcaatgcacaggattcttctaacgtaaccgtgcgtattaatggcaccagctgggaaagagtgtatcacattccggccaacaaaaccatcactacggagataataccaaagagtggtctgaacgatgcccgcctgatagaggaaggattatcagataaaggtatcagcattgaaagtgatgtgcctattgttgcctatgcgcatatttatggcagcgcctcttccggcgccaccatgctgctgccggtaggtacctatggttatgaatatgctacactatcgtccaggcagaattacagcacagacacctattcctggttctatgtaatagcagactatgataatacaaaagtggagatcacaccttctgtgcccacgctggccggtaaacctgccaatacaacgtttacggttacactgaataaaggagaagtgtaccaggtgctgggcgctatgatgcctggcggtggcagcgaaggatacgacttgtctggtagccacatcaggtctgtcatcaatgaagatggaaaatgctacccgatggcggtgttctccggtagcagccgtaccggtattggttgcggcatcgaaacgggtggatcgggcgataacctgatccagcagaacttcccgtcgcaggcgtggggcagaaagtatcttactgcacctacctctaccagtggatcggccagttctttcatgaccaacatttatcgtgtgctggtgaaagatcctgctaccgtagtgaaaataaacggcgccacattgacgggactgatcaacaacaggttctaccagtttgaaagcagcactgccgataatattgaagccaatcagccggtgatggtagcgcaatatatgtcgtccagcggcagctgtcccaataccagcggcaacggcgatccggaaatgatttacctgagcccggtagaacagggtatcaaaaaggtaggactgtaccgcaatacacaggagtctattactgttaattatcttaccctcatcatacctacgggaggtgtatcctccctgctgatcgacggcagcgctactttcgatcatacgtatccgcatcctaacgcgaccggatatacggtagtagtgaagcgctggccggcagcacctgcacagtgtacggtaaccagcgactctgccttcaccgccgttacctacggcctcggcagcgtggaaagctacggctacaacgcgggtaccctggtgaagaatctgaacatcctgccttcatttaacaacgtaatgaacaacagtggtcagaacaacacctacacctgcgctaaaacaccattccgcttctctatgctgataccagtgaagccaacagcgattacctggaaattcagccaggtagcaagccttgcacctaaaactgatatcgtgcagaataacccggtgccagtggattctatcatcagcaacgaacggaagtactatcgctttacggtgccggctgattacatcttcagcaaaccaggcttgtatgaagtgcctatcctgatttcacatccggatattgaaagctgcagcaacagttttgaaagcatcctgcagataaaggtaatccctgcgccagtggttgacttcagcgttgactataccggctgcctgaacgacggcgccttgtttaaaggtaccgccactaccagcaacggggttgctatcagcacctggaaatggagctttgccgattctacagtatcgtctgcaaaagataccctgaagtatttcagatacccgggtgtgaaagaagtgaaactgagcattgtagcggcagagggttgcgtaggggatactaccaaagaagtggaagtgtatgcgcctgcgctggcacaacttgtgaaagactctatgaccgtatgtaacggcacggatgttaccctgtctgccaggaatcctgaacccggcgtattgtacaactggtacgatgctccaacaggcggtaccctgctgcataccggcaacgactacacgattaacaacattgccgccgatggtaattactacctggaaacactcacacacggatgccccggactgtcacgcgctaaagccattgtacatgtattgccggttctggaaacaccggtagttacggtagacagcgtaggcgtaaacatgatccgcttcaaatggaaggcggttgccaatgccaccggttacgaagtatccctggatggcggtaccagctggacattgccaacttccggcagggaaggactggtgcatatcgttagcgggttacaaccggtgcaaacagtgaaactgattgtgcgcgcgaaaggttgtgaagacaaggcatcactgccggctgaaggtaaaaccttgcctgacggcatctatattccgaatacgttcacacctaacaatgatggccggaacgatgtactactcgtgtatggttacattatcaagcagctgcacatcaccatttttgaccagtggggtgaaaaagtattcgaatccaacaatcagtctgttggctgggatggcaactacaaaggaaaggcattgccctccggtgtatacatctatgtatgtcatctgacccttacagacggaagtaaaacagagaagaaaggagttattaacctgatccgctaaaaacagttgtatgaaaaaagtaagcatagagaagttgttactgttagtcattggatgttggatgttgcattggccttgtgccaatgcaactatccggcccatgcgccaggatatcgacagccttttaatgttgcagcgatctgtgaaggtatatcccaacccggtcgtttcttccctcaccatacagtcacgcaaatcaattcaacagctgatactctatgcgatggatggcaaaaccatcaagcgtgtagcggttaccggtaaaaataaccagctggatgtacaggatatccagcggggagcctatatgctgaataccatttttgcagatggcacaacgacgtcgaagatgatcatcaaacaataatcatttcaatatgaaaaattgaaaaagatgtcaaccaaattactatacataaagcgactttgcattgccatatccctgaccctgtttcagttcgtagccgatgttgcatacgcccagaatctttccaataaagggaaagatttctgggtgggctacggacaccaccagttcatggagatggggcaaagcaacagccaggaaatgatcctgtacctgagtgcagaacagcctgccaccgttacagtgagcattaccggcaccacctggacgcgcacgtataacatcccggcgaataccgttattgcttctgacctgatccctaaatcgggcgctatagatgcaagactgtattccctgccgccttcttttggcggcaccggaggcgagggcgttttcacggggaagtctattcacatacaaagtaacgtgcctattgttgcctatgcgcatatttatggcagcgcctcttccggggctactatgctgatgccggaagaaacttggggttattcctacatttctgtgaacagtatgcagaactatgcggacgattgtttctcgtggatgtttgttattgcgaaccagaataataccgtggtggaaattacaccttcggtattaacccgtaacggacgccctgccggcgtacctttcaccgttacgctgaaccgcggggatatctaccagctggtaggcgcttcgctgggcagtggcgccggccgggagctgaccggcactactattaaatcgatcggcaacccaatgggacagtgttatcccgtggccgtgtattccggcagcagccgtacggccatcacctgcaataactccagcagcagcggcgataataacatccagcagatctttccgttccaggcgtggggtaaacgttatctcaccgcgcccacctctgaagatgatttgccgtcgaccctccagtataatatttataaagtagtggtaaaagatcccgccaccattgtaaaaagaaatggcgtaacactcaccggcctgatctccaattcttactacgagtttgttagcaataccgccgattatatagagtcagataagcccgtgctggtggcgcagtttatgtcgtcttccggggcctgcggcaataccggcggactgggagatccggaaatggtatacctgagccctatagaacaagccatcaagcggattggtttttaccggaacgaccgggagtttatagaaaccaactatctcaccatgatcattcctacggcaggtattccctcgctcaggattgatggcagccccctgtttgacttctcttacccgcaccctaacctgaacggttacacggtggtgatcaaaagatggccggctgcgcctgcacaatgtattgtgagcagcgactccgccttcaccgcagttacatacggcctgggcagcgtggaaagctatggctacaatgccggtacgctgatcaataacctcaatgctgtaggctctattcacaacagttatgatacttctaaaacatccaatgattttacctgtaccaacacccccgtgcaattgtccattttaatggcgtacaagcctacaaaaatggtgtggcggctcagcaccctgggcacagcgattacgcctaacgcagacgtaacggttaatgcaccggtaagcaccggtacggtactgatcaatgggatcacttattataaatactcattgcccggcacttaccagttcagcgcaataggagagtatgatatcccggtcatgtccacgcatccgagcattgaaaactgtaacaataccgaaaaggtgggattcacggtattggtgaaaggaaagccgcgtgcggtaatgacttatacctataccgggtgttcgctggatacggtttactttaagggagatacaagcctgaaggatccgctgatcgaccgttggcagtgggagttcccgggagcagtgaaggatagtggcatccaggtaggaaaagtatttcctgtggggaatgctgcggtaaagctaacggtgatttcaagggatggctgtgtgggagatacttccttccaggtagccgcagcggccaaaccggtggcatcctttacaacagatgctgctgccttatgcgaaggcggagtattgaagatgaccgataactccacttacggaggtacggcgcctttaaaatcgtggtattggaattttggaaatgattctgtgctgaacgctgtcaccaacgcggtacaaacgattacttacaaagatcataatacctacaccataaaacacgtggtgaaagtaagtaacctctgtgtgagcgacaccatttcaaaaacggttaccgtgtacgccaaacccaacccgctttttgcttatcccggcgactgcctgccggtaggtggcctggtacagtttaccagcggtgcagtggtacccgatgcgcaaaccatcagcacacacgcctggaacttcggggatgctaatgcaacaactgctaacccgaatacctcggtggcgaaagatcccacgcatgcctatacgaagtttggcacttatgctattaaatatagtgtaactaccgataaaggctgtacgaaggatactacggtaacggctacctttaaactgaaaccacaactggcttatgctgccctgaacggggtttgcgtaaacatgcccggcaccattgccataggcaaagctactgtacaaaatggcgtaactggtaaaggttactaccgtggtccggctacggattcaacaggcaatttcacccctgccaccgcaggcgcaggtacgcataccatctggtatgtgtttactaccagcagcggctgtaccgattccatttccaccaccatggtagtgtatcctaaacctgcagctgcttttacagctaccgccaatttgtgtcttggacagaatactgttttcactgaccagtctgccatctccgtaggaaccatcaccaactggaaatgggacctgggcaatggtacgctgagaaacaacaccaacaacaatccgtttaccatcacttaccagaaagacagcagctacctcgtgaagctggtggcggtgagtgatcataattgtatcagtgataccgctaaagccatagtggccgtacatgaattgccggtaacagattttgcactgcctgccaaggtatgtatgccggatggaaccgctgcgtttaccaatctcactacggcgagggacaagtcgtccctttcttaccagtggaacttcggcgacggtggtgcaggatcggcggcaaaagaccctacctggcagtataaagcctttggaccgtttaacgtgaagctggtggctactaccgcttatggttgtaaagattcggccactaaaacattaagcgccttctttggccagccggtggcatcctttaaagtaacgccggataccctttgccagggcgccgacaatgtgtttacggatcaaagtacagatcctaccggaagcattaataaatgggagtggagctttggcgatggcaccacctccacggaacaacacccggtaaagaaatatactgcacctggtgaatacagcgtgcagttgcaggtagcaaatcagtcgggttgcggatcatctgcctatagcagcaaggtgattgtatacctccagccggtgatagatgccggaccatcctttgttgtgccgcagggtactatcgtgagctttaagccggtggccaacgattcggtgaacctcactttcgcatgggaccctgctgccgacttccccgatcctacggtgttgtcgccggtaattcctgccatgcacgatgccacctacacacttactgctatcggcaaacacagttgtatggctcgtgacgctatgacggtgaaagtattaaaaccagttgcaccgccaaatgccttctctccaaacggagatggtgttaatgacacctggattatcaccaacctgtctgattatgcagaaagcaccgtggaaatatttaaccgctacggacaaaggatataccattccaccggttataatgtaccatgggacggcagattcaaaggtaatcagctgccaatggccacttactattatgtaatcaggctccgggcgggtatggcgcctatcaccggctatgtaactattatcaggtaaagtaaatcattcacataaaaccgtattgtaaatgagaacgatcattgcaaccttattcatctttgctgccactgtatgctccggtacccggttaatggcgcaaaccgatccccacttttcacagtactacgtatatccgtcgtggttaaatcctgcgcttacaggcgtatttgatggcgactaccgcgtggcggccatttaccgcacgcagtgggggaatatcagcccgtttaaaacatacggtgtaagcggggaaatacccaccgcaaagaatattaatataggcgccagcgtattaaatcaaactgccggcgatggcggttacaattatacaacggcttatgtaagcgcggcctataccggcgtgaaactcgatgcttcccattatcaccagttaaacttcggcttgcagctgggctttatccagcgtaggtttgacccttcgaagctcacctatggcgaacaatggaatcctgttaccggctacaaccccggtaacccggtatcggatgtacttacccgtaactcggcagcctcctttgatgccggcgcaggggcattgtattatgacgctacccccgggaagaactttaatatttatggcggcttctccgttatgcatcttaccaaaccacaggaccagttcagcgccaaaggtgatgcccgtttcccgatgcgctttaatgtacacggcggcgtgaagttaaccctgtcggaaatactcagcattacgcccaacttcctgttcatgcagcagggccctgcacaggaaaaaatgatcggcgcctatggccagctgaatgcagcggcgggaacggatttcctgctcggtgtaaactaccggtacaaagatgcagtgactacacacgcgggatttatttataagaatatgatgctcggcgccagctatgatatcaatacatctgatctcagcaaaatggcacatggctccaacagctttgaaatatcccttacgttcattggccgcagatcggtaagaacaccggatgtagaatttgtttgtccacgattgtaatcaacttttaaaagcaacaggatctcatgaaaaaaataatatttacttccgcattgctgttatcgggtatgatgtcgtttgcacaatttacctataactatctcaaagcggcagatcagtactacagtaaagaagactacaattcagcggctacctactatgaaaagtacctgggctcccgtaccaaaacggtgaagccggatacttacaaaccttatgcggccgtgtcggtggtaaagaataaaacagtaaaggtaagcagcgaacagctggcggtgtataagctggcagagagctaccgcaacctgcataactatggtaaggcagcgccttactacgaatccgtgatggaactggataaagctggtttcccattggcgccatactactacgcagtttccctgcgggcattggctaagtatgaagaggcgacccaggcgttcaaaaatttcctggacagctacacggctaatgataaattcacggaagcggctaaacgcgaattgcagaacctggcatttattaccgcccagttgaataaaaaagatctgtcggagtacagcgtaaagaaggcgcctgctgcgttaaataccactggcgccagctatgcgccgttgtggagtaacggtagtaccctcatctttacttctacccggcccgacagttcgtttcagaaaaatcatacttatatcaatcgtttatataccgccagctatgaagccgggcaggtatctgatattcacctgttaaagctcgatcagccggaagggctgcaccagggcgctgcatgcctgtcgcccaacggggagttactattccttacccgctggcacatggatcatggcaaaaaggtatcggccatttatgtgtcccgtaaaaacggtgataactggagcgagcccgtggtgatggatgcgctggtaaattcggcgggtaataatacccagcaaccatatttactggaagatggtaaaacattgttgtacgccagcgacagggccgatggctacggtggtttcgacttatggtatgcctcccttgatgaatccggaaagcccttgcaaacagccaacctgggagaagtaatcaacactgccggtaatgagcaggcgccattctatcatgcggctaccaaaacgctgatcttttcggcagataaccgtgtgggcatgggtggatacgacttcttctccagcaaaggaaatgtaggtacctggaaagcgccggtaaacatgggttacccggtgaactccgtgaaagacgatatttattttaccagcagaagcaataataaaaacctgctggatgatgtactgctgggcactgaccgtgcagcagaatgctgcctggaattgttctttgtacataagaaccgtccgccaaaacggttgagcggcatcatagtatcctgcgacagtaacacgccgctggcgggtgctgccgtaaacgtgatagatactatcagtaacaaagtggtatacacgcacactacggccgccgatggcagctatgcttttaccgtggaagactttttgccattaaaagcagtggctaacgcagatggttatacgactaatgcccggcagataactgttccgcaggacgaagacactactgccatgacagtaccggtattgtgcctgacgaagctggttacaccggaagcgccggtggtgctggaaaacgtgtactacgatttcaacaaggctacgttacaggaaggttcattcccttcattggataagcttgcggaactgcttgctgccaatcctgatatgcacatagaactgagcgcgcataccgacagtaaaggtaaacccgcgtttaaccaacgcctgtctgaagcccgtgcgaaaacctgcgtggaatatctcgtcagcaaaggcattgatcgctccaggcttacttatataggttatggcgatacacagccggtagcgcccaacacccaggaagatggtagtgataacccggaaggaagacaaaagaacaggagaacggcatttaccatcattaaaaagtaacagcccggctgtttaacccaaaatcactgatccatgaaaaacattgtgctcacaggtttgcttgttttgctggtgcatgttacccatgcgcagcaacagccacattacacgcagtatatcatgaatcctttcatcatcaacccggcattggcgggtattgaaaactactgggacctgcgcttcagtcaccggcatcagtgggtaggtatgaaaggtgcaccggtaaccacgtatatgaccctgcaggggcctttgcgtaaatcggattacagtaccgcgtcgcctaccggttttgacccggaagggaataatccccgcggaaaaggctactggcaggattacaccacgccgcctccgcatcccggagtagggctcaccgtgctgaacgacaaaaccggtccgcttaaccgcttttccattacgggggcatatgcgcatcacattaacctatctcccagaaccagcgtcagcgccggtatcggtataggtatgcagcaggtgagtctggatgccagcagggtggaattctttgatccttccgatccggtgctgggcaccagcaccggtatactgaacaaatggaagccggaagtaaacgccggactgtggctgtactcagcagattattttgccggtatctctgtgcagaatattatcccgcagcaaatcgggttcgacaatggcaaagtagtgggcgactctgtttacagcggcaaactggtaccgcatttattctttactaccggctaccggttatggataaacgatgatctgaatgtgatgccgtcggtaatgctgaaaatgatcaccgccatgccattcagtgtggatgttaacgccaggtttatgtaccgcgaccggctctggctgggggcttcttacaggataaacgacggggtggctgctatgtttggggtcaacatcagctcgcagtttaacattggttactcttacgactatacggcatcttccctgaatacagtgagccggggtactcatgaaatcatgatcggtttcctgctgggtaacaagtatggagatacctgtccccgtaacgtatggtaacggctgtcaattttttcatcttttcatttaataaataaaaacaaaaacaaaacaattgtcattatgaaacaggttacacgctttatgccctatgcattgatcactgcggttgtattattttttgctgcctgctccaaagacggagaccagggtcctgccggtcctgctggccctgcgggtccttcgggtgtgcccggtgctaccggtcccaaaggcgattcaggtgcgcccggtagtgcgaatgttatttattctgcctggaaggatgtggcctttgcgcctgcagataccatctttaatcagaatggtacaattaacaccatcatatatggcgccagcctggatgctccgaagttaacagctcccttactggccaatgcatctatcaacgtctatatcaatctcggtactgctgccaattctttcgtacaggcgttaccgtatgtggatgaatatggttacctggtaaggtttgtagcctctgtcggcgccatcgacctgcttgcgaatgcacctatcagcaccactgctacggataaacgttatcaatacaggtatgtaattattcccggtggcgtgtctgcaagatctgcagcaggcatcgactggaatgattacagccaggtgaaaaaatatttaaatctcaaggactaggttggctaatacaaccaccagtatataaaagggctgccttattcagggtggcccccatttgaaatcatttattgaccaaaatttacgaaaccgtgtatgaacccatatagtgaccttacggatcaggagttgatccgcctgtatatttcaggaaataacccggcttttaccgcattggtataccgccataagaacaggatctttactactattgttttacttgtgagagacagaagcctggcggaagatatcttccaggaagtatttataaaaatagtgaacgctttacaatcgggccactatgtcgataacagccggttcctggcatgggcggtaaggattgcccataacgcctgtatcagccatttcaggaaaaccaatcaacggcaaagcaccatcgttacctacaacgatgacctgggcgattacatggaagtcacggaacacagccaggaataccgcatgatccgtgccgaggtaaccgaagaagtaaacaggatgctggaccgcctgcccggactgcaacgcgaagccctgatcctgcggtattacgccgacctgagttataaggagatggcgcaaaccatcggtatcagcattaatacagcgctgggaagggtacggtatgcactgatgaatttaaggaaacaggccggggttgaaaacctggtggcggtataattctgcgggttaaactaaatgttgaaagccgggtgtttttcgttaatttcagtcagccggaataacgaaaatacaactcccatgtatacccgaaataatccccaggaacgtaaattccgcagcaatgccgatcacatagctggcagaaatggtatctcccaaaatgcgcctgtacagagaaaatttatatatgagggtactgaagaagagcccaccatcactgatatgatagcttttaatccggaactgtttgagcagcactatggcttaatacaggtcatgatgcgcgaatccgaaatatatccgctggagaaaggaaaggagaaggaggctattgagcgttacattagtgaatttaagagtaaggataacggaggcctgccgaagatcatccattttatctggataggggcttccatgcctggatccgggaaaacaaatgtacttgcctggaagaaaagaaatcccactgcgaagatctggttatggtctgacagccgctggcgcgaccggactaacagtatacagaatggttttgcggatatggcggcctgggcaggagaacatgaaataaccataaaggatatctcggctgatgccagcgtctttacagaacattataagaaggaggcaggttatattaaaagggcacccactgatacaaatgatacatggaccaactttggcactgcgtccgatctggcgcgttacagcattctcagcaagtatggcggcatctattcagatagcgatcttggtttcagggagaataccgggcagcatgaatcggggagtagctccccgcaggcagaacagcccgatatttttgaagaagtaaaaaagaagatctataaaacaggcatgcttacccataacaggacagaagcaaaaaaggctgccaatgacctgatcgcagcattgcctggtgcggagaatataggacttattaacgctaatgcggagaagaagctgaatgcgctatatcaagacggggagaggcttaaagagtatcctgacctggaggggggattatttagcgcccggggattagaaacaatgggctccaccggtcctgagggaatgagagaagcgttaagaaccaacagcaggacaagaggggttcccggtagtatccctgtcggaaatagaaagtatttcagtgaagcaatggaaaataaaatatcagcagacgatctctccattaaagtcccttcgctggcggtaagcgattttgaaggaagtgatatgtcctggctaaagtaacgcctatacaatcttcccgtctttcccaaattccttgcggatgcccgccagcagatccttttgccggatggttttatcaccccgtttcaatgccatcaggcaactgtaccgcacaacgttaataatagtaccgccggtcatttcgtatttacgcgcagtgtcttccaggttcactttatcttccagcgctatatgtgaaggaaaggattgttcccatatgcgtaaccgttgttccggccctggcatagagaaatagatcatcgattgaaaacgacgggcaaaagcttcgtcgatattggctttcaggttagtggccaggattaccacgcccggaaaatcttccacgcgctgtaacaggtaagccacttcctggttggcataacggtcgttggacgaagaggtttgtgtgcgttttccaaacaacgcgtctgcttcatcaaagaatagaatccattgctggttgatggccttgtcaaatacctgtgcgaggttcttttctgtttcaccaataaattttgataccaccagcgataagtcgatccggtatacatccatgttgaacgttttacccaggaggcaggcagtgagcgacttccccgttcccggcggtccgtaaaaaagactgcggaagccaggctttattttgtggctcatgccccagtcgtgcagcagggtggtgccatgttctatccatgtccggatgtcttctacttcttccatcgcatgcggttccagtaccaggtcctgccactccataccggtttcaatacgcttggcaggaaactgcgtattataatcaggacggtaggaaacgccttctgtaaacaggctgagatactcggtcgacaagctcagggtgccgcttagcagcggctcatcgccggcggggttgagtttgaggatttgatgtttggcaaagaaatgatcggggctaaaataccggatcatgttaaaccgttgctgcaagccatccgccgtcagcaggaacgcggctgtttccccggttggtaaaaagccgccgtgcatctgtcctttaataccaccaaattctgtgaagcccctgtcataggtggcgttctttacaaagaaaatgtccagcaactgtggttgtatatgcgggatcagcgcgagcagcagtataatccgctccgcatgcgacatgccatagtgttttataatctgtgcgtacacagatggatcttccgagagatccggtattggcgggtattccaccactgtttgctggaagtattgttgcatccgtgcttccgtcagtagccggaaccactccagttccttctccaatgcagctgcgttggctgctattaactgtatgcccattctgtatatattgttttttccatccacggggtcttgatcatgccaatgccccacggtaaggtttgaagtatcatgtcgtagccccgttcttctacccgcagccaccagtcatcatctttttgccatagtgcgccgtcgcgctgcaggaaggccgcctggaaaccttctacggaggagttgttcattttctcccagcgctggattactactttcaacagttcctcgcagagttgtttttcttccgcggtcagcagtatttctgcgggcaccggttcttccagtggtaaggcgcacagtattttattgagcgccaattcatgttctgcatgtatttcctttccgtttaccatatactgaagcaggtgtacggcacgatgttgtgcttcccggtttataaaaccttcgtcgttcaccaggccgatccgcttgaagccaaacggaataaaaggatgcagtatgatcaggccggcgttaccggtataaatggtatccaatggttgcttcttcactttagcccagctgtcgggctcgtgaggcggtgtttccagcggatgcgccgttgccgtagcggtagccgggtttattgtctggaggcggtccttttcgtaaaggctttcccgtaacaacgcccggtgacggctggctgtaatgtttaattgcgcttcctgctgcaataccggtactacatgccgtatatgcgtgtacgatagcgacgccggttgttgcgcgctttttaccagccggctgaccagtatttccgcaatacccggggtggtcatatttataaaatcgaggaaacgggtagcgtagctgcgcgcgtcatatacatgtatatgtgcgcccagcagtaacaggtgaaaccgccggaatacctgttgcagctgtattttctcctggctgccgggaagcagtgattccagcagctgttgcaactcgtgcaaggcatccgtggtgttggctgtccagccgaggggaacatcctgtacaatgtcaaggaacgattcttcgtcgaggtgctgcgccatttgttctatcagtgcaggatgctgcagtattttactgtagaataacctgcgttcctgccggctgcgctgcttataaaagcggacggccttccgcaggtcggtgatgctgccctggtgactgttaccggctgtttcctgtaacaggagcaggctgtcctgtaccgcgtatatatccagggtttgccgtatatggctgtcgggcacccccgcgtagaaggagaacaacccatatacctgtagcctggccgccagttgttgccggtagctggtaaagagctgatgaaggatggcaggagcggcgttgaataaaaggaccacggctgctttgatgatttcgttggtcgctgataatggcaacgaacccagtttttccggcagccggtagcgtgtaaggtataccgttagcagctgccgcgcttcttccagcacttgctgttgctgatgttccacggtaatggaagggtagcgctgcatgcgctgtaataacgaccggaaggccaccgccggttgatagatcctgctgctgctgccttccgcaaagaagctgcctcctgcgatggttttctccagccagggttgcagtaacgcctgtaccggttcaatatgcggttccagctgaagaaacagctcctccagttgccggaatagttgcggcgatggggtgatgctttcctgtaatagcttcatgtgttcttcatgatattcgtatagccattgcagtaaccttgcggcataggctgaagagacattgcccgctgccggaggtaattgcccggtggtcaggaattgttgcagccagcgggtgatctcttccggtgaggctgttatctgtgcgggtaaacgttctgcctcctgcagggaaagagcggatgcgggcatggtccatgcctgcaaatcattggccagcaccgtattcccggaaaggtgattaataacgggcagcagctgttgcagcaggaagcggatcatgtgcggtgctgccaccggcgtttccgaccacgcgggcaggaacaggtgttgcagtaacacctctttgctgatccgccggtaacgcgtggcggcgagcgattgccagatggcttgcaggataaactgctccggcggcagggtgctaaccgtcacaaattgttgcacggcggttaacagcgtatatacgttgtcgtatacttcttccgcggcggcgctcataccgctgcttttcagcaaccggaaaaacaccgcgggctttacgcctgccaccagccggtacatagctgccggtagggtggcggcgtattcgagtatcgtcagcgtttgatccggatgctgatcagccagctgttccagtaagctgttaagggagtagtgcgcatatatttttccccaccacgacatactgccataggtgagcaggtgcaggatcacatcgcggagcaatagccgttttgtaagcgtgtccccggtaaaggaagccgcagcaatggtatcagctgcccagttctttatctcccttaaatacccggtttgctccaccgccacttcattggtttgcataagttcatgccacctgccggcagcggtttgatgctgcaataccagctgcagcatttgtttcagggaggcggcggcatggtaaccggtattgttaaacatcagttgcagggacgcaggtgtaacacccggagcccaccagggaatagcgccatatagcagataatagcggagtacattgatttgttccccggtgtctgccattaattttttgtaagatggatcaccgccggcaaccagttttcgttgaggcgaaacggttagttcgttatagaggtctttgatatagttacccaatcctgtttctggtaaggaagatttgtaacgccacaacgcttcataaaacaactccaggatggtttcataggaaaggttgaaatgccccgccagcttcagcaggttgctgcgtacaaattctttgcggttaaagttgctgccccgttccataatgagataggtgagcataaataaccacaccgctttttccagttcactggtttctgtatggagtaattgttgctgctgttgcagcaacagtatttcccggctgccggcaataataaacagcgcttccgccggttccagcacctgtacgatggcctgtaatacatcaacggaaaattgccacacaattcgctcccgtacgctttgactccggccaatgctgcggataaaaccagccagtttccccggggaagtttttgataactgtaaaatgatgtctcccggttgcgcgcgttcagcggtagtggcccaccagggcatcacaccctgcaacaggaaaaagctcatcagttccagctgccggtcttcgcctttccttatggtaatatccccgctaacgccatgctgcgtgcccgcctgttgatgatacagcagatcagtaagcgcctgttgcaaagccgctaatatctttgttggcagctcggcttccaggtctttgaaaggaatggtccctatgttcagtaccagcccgtcgatagaagccatcatgtcggcggggatcagttgttgcagcaaatcatccgtaccattgctgatgctttgccggaaaagcgtactcactttatcctgcaaggcaaaagccctggacctcgaatcgtaggtgatatcaaagctgtatcgccggatgatgtgtgcttccatttatacggtaactacatgttgagaaaatgcgggatcttttacaatgaacgccagtaaagcagcggtggcagatggccggtcgccttctccgcgcatggctttgagccaatcgaaataccgggattcaaatgcctgcatggcgctgatacccagccagtcgaagttcatgcggaattgtacaggtgtatgttcccggaacagtccttcggtaaaattcctgaactccttatactggaagcgtgccggccatgaagggaaaataatgctcatgccgaatttaaagaaggcttcctgcaacatttcggactcgccgtgttttacataaggcaccacacgtacctgccggtgctgcccggttttcatttgcctgatcagcaacagcagatccagcattgttttttcaacggcaaccttatggtcaggagacgtgaaatgtgctgctgttaacagttccggcgtatcgccacgatagaaatatattttgtaatactgctgcagctgttgccagctgccataagcatcctgttcattcagggcagccgccagcggggccacgttttccagctgcgcttcccgctcttcaagggtgagccattgtgcatgttgcagcagcagtttattggatctgctgtaaatacggaaaccaaaactcttgtctgtgtaggcaggcttcagcaacaggtgttccagcaggtaacatccttccgattctgtgctgatctgtttcaggtgccgcatcgtttctttttgcgcctgcatagcttcttcatgcgtgttttcccgggttatcacctgccacaacgcatgtgcagcctgacggtataccaccaggtacacatcttcttccccatcgtatacgatgcggtaattggccggatccagtccgtaacgcagcagcgacaccgactgacggccatagtcatatttcttgccggtaatgatttcgccggaagtgctttcagcgatgttcactttcagcagttcatctttcactttgtattccttcaccaggtgaacatgaatatgtggctcggaaggttggctcacggatactttccagttgctgctatcaaatacggcggtaagccgctttcttttttccggacgcacatgaagcaacttatgcagaatggtttcatagcctgacaaactaccttcgttaaaaatatcttcgcggtagttgaacgaacggttgcggttagcgctgagtgcgggcaggtcacgaaggatggatgctttccattccagctccggactgatccgggagggaggcgcatcgcggtcataggtttgttcatagaaagtaaccgggtatttcagtaacaccaggttgaagcgggccatcaggtgatccagtatcgtgttcttacgttgctggtattctttatccggttctgctgcttcctgcatatttttaatataggggttcccgttatcattgatgaaatcctcccaggatacgggtgatttctgatgggtaaatgctttcagcaatgaggccacatgcggcacgttgtacagcggttgtgtagcgtaggtagcagctggcacctgttgcaggaaaggcgaaaacaggttgccgatgttgcttagctgcgcgaggtagttggccagcaactgttcaaaaaagagcaggtaagcctttagctgtttagcctgtgcctggcggagggcgggagcatctttttcgaggccttcatgcccgatgccataaatcgccggaaagtgatgctgaagggaatagtactggcccaagttgcggtatattcctttcagtggtttgggagcttcggcattttgatgaccagtaaatttcctgcgggctactgtttttacctgctcgtacatattgaggaagccggcatcgcggaggttgtattcaaatttgtcgctcgatatttttatctcgtgcttttcgcttatcatttccaggtaagggtagtggccttctttgatctgcaccggttttgcctggaagttaccgttttcatccgcgaggtaaatagcttttactttcattacgccgggtacttctgaaacacttttcatcaggtcggccggatcggcggtttgtttgcggggatgcagatcgctgttcgctacgaaacctttcttcagcaagggacctgcatacatttcttccggtgtgtgaccattgatatacatttcggcggcgggtacaaatcttaccggcgggtgcattgtcatttcaaaagcattgcacatcagggcgaggatctgctggggctcatgcctgctgtctacaaaaatttcggccttaatgaaaatctcctgtggttgcaatactactgctggttcaaagtcttccccgatgttccggtacgattgcaggagatgatctgtttgtgcggccagcagctgtacctggtctgcattggcttccatgttccgggcaattgcatcttccacctgtataaatacccggtatacgccctttgtacacccggatggatggatggtttgtacgggttcaatccatacattttccaggtcgtctatttcatccagcaccagtttgcggtagtcgttcaccgtcacgggcgcggaggtaagcatttctgctctccggaaaaaggagtgttgcaaaggatcaatgtcgccctttttatctgccagtatttcttctattgggaacgccgtgcgatatgccggatcagtgattgcatagcatagctgttgcaggatggttacgccgggatcatgcaggttgtagtcggtccattcggtaccggacagctcctgcacgcgggcaatggcttccttcattaaaagatcataatccattgcaggggcaatggatttgtctctgttgatctgaacgggactatcggacatatgacagcattaatagtaatattcatccggcataaacagctcgtcgctccatagccgggtgatgttataaaagatttccacaccatcgccatagttgctgttggaacgtaattgcagcgcgtagttatgcgtggtgcctttccagcgcagtttgatcttattccagaaaaagccgtagtgggcgcagcgctggctgatccggttatgtgatccgccgtatgccgcgagtgccgtggcgtgaagcaatgctaccctgccggcgcctttccggccggttctggccatcacttcaaatgcctggcagttatccatcgattcgagaatgggatgccatttgccgtttgccggaacggcgcctgctttaaaagttcctacgcgtccctgcatacctgcaaagccgtttacatccactttaaaacgggggtcactttttttcccgaccccgaggttaccgttcatatgaaaaaagaagctcttcccgggtccggtctggtcatcttccccggtgccgggtttcaggcgaagggcaggaaagtcctgttcatctttttccatacagaaaaaaggttccaggtcatcagtggcgcggtaaaaggataccagccgcttggagtcgccgagcgtagataccagcaagccattgtcttcatcttttgaaaaaccatcttcctgtttattgatggtagaatctatcaggtagccgaagtggttttctgttggcattacgccgtttctgaaatattgtttgagctcatcccgcccgtatacttttttactttgttgcgtatccatatataagcaatttattttaagagatgaatagttactggtatgaccggtcagggtggaagtatagagatggtcagcatctcttcatcggttgcgtgatccggtcgttggtccgttggcgttataacatgatggtcgttgcctataatgagttcgttgctgatcttcaacgcatcgatgcccaatggttccggttctttgtattcgggcgagtgcagcacggtgatgaggtgttctttcgacgggaccagcacggcttgcggcaacgaaggcgtaacctgctgaaggccgcctatggcggtatctgtacaataggccgttaccataccggtatcttcatcttttgtatagtaaaaatgcacgagggaaaagccggtgatatattccacataaggctgccggttgatataattcagtagctcagatttgtacaaggtgctgcctatctttaaatgggaagaaggatcaaacaaccagggacaaagatatttctggatatccagctgcagctgttgcaggtggctgttctggttgttttcagatggatccctgaacatgatgctgcacactactttcacgctttcatacaccgggttacggatcgataaacggacaaagggagatatatgctgttgcataaaggtttgaatgcggcaaagggtgtccaggtctactttgggttccgggctgataaacaggccgctgtccgattgccgcggaaccaccacaatgcttacatcttcgtccctggcgccgggtagcgcagtgatgcattttacaatcagtatctccggaaaagcttccagtaatacctgcgcaatatccagtgctgtaacgggccgttgcttgtgccgtagtctttcacttacccgtgtataaaatttactttcggattctgttttacggcccccgaaagaaggaaataactgccagatcgcctggatggttcggatatctttttttgttttttttatcgtcaggggtgggagcgttaatactttttcgagcgaaccgccaattccttcaaacacccgctccacggttacggcattaggaaagataccaatcacccttggcgtaatgcattcgtgggaaggggtggaaatcctgatccaccaggtaccgggtgtatggatagtgttattgggattgataccgtgtggaacacggatctttacaataccactccgcgaaaggttatttgtattgtctgataaaagacacatgctttcaaagggataccatttgttatttgccaggtaatgccagttgagcggggtaagattggtagtggtgtcggtgaaatatttatcttccagttgaaacaacagcgacagctcttctccgggtttcagttcgttaaaaccaatgtagaggtgaccggcttcgttgaataccggaagcagggaaaagtcattggcgccgttgccgggataaatgccctcatttccaaatacgcccgcatggtgtacttccatggtttctccaggtatggctacttttcccggctttaatgactcggaatgttccagtgtatagttgacggcaatggcctttaccaccggcacgtaaggaggcgacggcagcggttttttccgcatcgggtgtttggcgttgtataaaattacttccggaaagatgagtgtgtacaactgatgcccgaatgtttcggagggggccgacagctccagcctgacggcgccctgcttgtaagccgtgccgccgcgctttacttccttatccattttcatcccgttagggaaactgattttattgaagtcggcgtctttaatcaatgaggtatcggccaggtacagatcgccttctttgtcgcggcgcgtatcgaaaagccggaactgttcctggttgccacgttcgggcagaaatacgccgttgttaatactactaaggcccaccttataagagttgttggtcatattccccgggtaggcggcgaagtaactatcgaacccgtttatatttttgggaagatccagccattccagttttatgctgaagtctttcgtatacttattaaaaacattgctgttggaaatatcgagaaaagagcctactgccggcatgggtccgaatatcctgaaggagctgtatgcgttcagttcccctacgttattatccagttttaccgcccggaagccggttactttagccgttaccgttacccggtccagtaccagttgacggagaaaggagtaggggtggtggaagctgttattgttcagcaatactttcaggagcggcaatgccgatgtaatattatcgccatgtacatcggggctgaatacggtgaaagcggcttcgctgctgcgtagcaggaagttgatgacaatagcgttatctgcctgctctgcggcgctgcaccgcacgttataatgtttaatgggctcccatcctgtgggagtggtgtagtatagcaggaatgcggcagacatcagttcactgttaatgatagcggcacttctgccggtaacggcagaaaaattctgaaggtatttaatcaactccgtatagccggcagcgttaaaatgaagtcttacctgtacagaccgcgcaccttctgtaaggtatagtgtaggcgatccgatcataaagccgatcgaggtattctccatggtacgtaccgattgcgacaggtcgtgctgatcttctcccagcaagggccacgtcaccggcggggcggtgagggcggcaaaagccgccggtggtatcaccgggtgagtagcatgataaatagctgcttcgcagatgttattggtttgcagcgaccgcgcagcgatctggaggtaattactgatatacagggtgtgtatggcggtaatggtggtggcatgtaccttgagcggatcccgcagccggtattgcaacggttctttcctggcagcgctgggcgcaagcactatttctcctttatccagcgtgaggctgttcacctgcggggcgggcgtgaccaggatatgtactttgtccggtaccgcatgcaggggttccatacccagtatggtgcggtaataataatccagatgccgtttgggtatttcgttgatctggtcctgcaggtatttataaagctccgtaaatgccatcagcagccccatatgcggcgtatgtttccgttcccggagctgattcttcaggtagtaggcggaagcgctggaagtctggtaaaatttcgtccgcagtgtatcgtaaatttcgttcagcgaaaaaaatccgctgaagatgtcttcgctttcggtgatactgtttgaaatgcccgggaacagcgcctgcaaccgcgctgtggtagtgacgccgcggagggtatgatgcctggctgtttcataaggaaacaattgttttacctgtagttcataccggtttaacttcatcgtttcatcttccaccacctgaattacctgttgtatgtaatgccggatcacctgctgtttatccgagaggaataatttctgcagggcatccatgagttcaatggcaatgtcgtaaagcagggagaagaagccggcggtatgtttaaaaagactggcttcatttcctgctttgcccatcgcttcccgcaggaagagatatttttcttcataggcggtgaactggaggttggagcaggtgatgagcataatcaccaggtctgcctgaaaaaactcctgccagtcgccatccggctgatcctggaaattataatagttaaactggctggcgagcgcggtcagctgcgccagcaggtcaaaggtacttttgtcgtctacttttacataggcaggttgcaatgcatccagttgccgttccaactggctgacgccatcctgtatattttcaaagtagttattcatctcgtgctgatgttggtaccttccaggaagtagaacggatacaccaggttatgccgggtattggtagaaatcaccgtatagttgatctgaacgtacacggtgccgctttccattgtctggtcaacaatctgacagtccaccagtttgatccgtggttcgtattccagcaatgcatgatagatgaggtggttcagttccccggaaaaccgggagtctactacttcaaataccatcttgcggatattacagccgaaatccggcagcatgatgcgttcgccgggaatggtgctgagaatgatgcggatgctttcttcaatatccgccacatcagacaccatcaataccgaggcgttgggtttgtcgaaggaaggagggaagctccagcctgttcctaaaaatgatttgatatcttttgccattgttaacctcctattaataccgttggacatcctaatgcaattacgccgccgtgggcggtggtgtcgcccatacgtaccgcaggtcttccgcctatgagcacggtgaacgatcccatgatggcagaatcaggcggtcccacacaggtacacaggtcgcccattacggaggcgggcatgccgccgattaaaacagtgggcatacccggtcctactatggggccacccacatgcggaatagggggtagtccaggtgtaatgagcgggcatacatgcatatctgtgatccttgcggcgggttgtcccataatttattttttatcgttttaattaatcattactacgcctccctgtatgatggtggcagcagaagaagagagggtggcagaggtgttaccagtggcgctgagcgtggtgtcggccgacattgacagtgtggcgccgctcatttccagtgcggtagtggcggcaacattcaccgacatgccattcagtttgagctgccccgtggcctgcaatgtaaggtcgctggcgctttttatggtaacgcctgccggcgccatagtaatgctgttactgctctggtcctggatcactatttcctgcgatgtgtcgttcagtgccacgctgttgcctcccggtgtaatcacggtgatgatcttgttctcatcatcaaaactaattttgagctgactctttgtatacagcgccttgatgtaattgttattatctgcgggaattaccggcggcgttttcattttgccatataaggagccgatgatcaccgggtaacgcggatcattttcaataaaagctactactacttcatcgcctacttccgggaaaaatatggcgcctgcactggcggtggcatagaaagtagacagccgggcccaggtgccttgctgaccggtagcggtactggccagcatcacctgcacgcggtactctgcggcagggtcctcagaaatggcgactacggtgcccagctgaagtccttgtatagccggcagctgcccgtttgccggggagtaggaaaaattttccctttcataaataggtttgctgttcaacccaaactttgcgttggtattccaaacgccttccttgagggtatgtgttacggcccacacgtaggcgttgccgttaaagcgtgcgcccacgccggctaaggtgatcaatgtgttgggccatacggtggcgttgcccatgaaggatacctgcccgctgatggattccagccgcatacggagcagggtgctgttggcccatgattgcaaagtttcctgcgccagcggcgaattggataccagctgcagcggcgtttgatgcagcgcggaagccagtgtggtggcttccaggttaccttgcgcattcagtcccggttccgtggcggtagcggtaatcatggccaatgtttgcgggtcccatgcggcagcggtgagagaaggtacctgtttctcggcgcttacagaagcgttgaagctgatcagcgattcaccgaaagctacagataccaccggctctccgcttactaccggaggggcggccactattttgggacctaccagtgataccacgaagccgttaaactccgcacgtgataacaggaaatcccaatcggtacaaaatttctgaaacaccagttcgttgagtgcgctggtactttgtatatctccactcaaactgttattactaacagtcgtggacatgatgtcgctatctgtttgattgatgaacactgcatcttttttggtgatggtcatctgcacggcgctgtgcttacaggtgacgatcaggtggaaaccctggtcggtggcctgtatggactgcttcaccaccacgccggtgaaaatcagttcttcaccggtattgccatatccggcagtaatggtgatggtgttcccgggcaaaaagctgtcgctgtcactggcggggaaatcgccgatcacgcctgtagatgctttcgctgtagtgccatcagacaacatgatttctgcataggagatccggttcagttcatgatgtattgttacagatatgacagggtacgtgtattgcacagcggtgccgtttgccgtgatggtatactgcagggtaggatctgctatattgataggtacaactgctgccatgggaatttatttctttagcggggggaaatagagtccgtcgccgggtttaatatcatggatactattcaaaccatttaccctggccacttccatataataaccgggttcaccgtaaatacgataggtcattaacggcagggtatcgccggccagtacggtccgcatatgtgtaaggtccggggatgacacaccggattcttttattttcgttgcaaaggctaccgactctattacagtgagtttgatcactgcacgcaaagccacgccggtagtgctgaacaggctgtacttgatgttgatgttcttacatacgcctgtaaagttggtatttccccaggtgatgcgcaggtagttgggacggtggtctgttccctggtagttatacgcgatgttcatcactttttcgatataggcgtctactgttaatccgccgggaatagggattacgccggttccatccaccagcagttcgaggtcgaagttgcccgactccatgctgctgaaaatttgtgtaggcgctactgcgccctgctcatctgtgtttttataattgatggtatagttgagcgtataattgtccgggttgattacggcggatacgctgtcgatcaattccgtagcttccggatctgcatagcctgccagtaataatttcgtgggtcctcctgtagggttcatcttgcgggtaagttctctatggtagtaattaatttatccatgcattcccttactatcttatctttcagggcttgcaggtctttaacgccggtatggcctgttgcctgcgagggatgttcttctatggtgactttgatcaccagttctcttatttccaaaggcataactaactgatttgttgaaaatagtcatagcatagttccagggtctccagggcaataacgctttcctgcgctttgaattctgatactttcaatgctacgggataagcatttacaaattgccatgaagcaaccagtccgcggtttgcattcatcaggcttactactactgctacgggcgagaaggtaaaaagattaatactgttctgcgcccagcgtatcagcggagagccggtgagcatgcctcttttgagcaccaggttgccatattttggcgcctgcggaaggcgatggataaacctgttttctcctccttcttttacttccagtggcgtaatggtagcggttagtccgcttacttcctggaagctgccttcattgctgccggtgattcccggcaccattaccctgaaataaaatcccaccggcggataaaagggcgtttgggccgacgagggcggtggtggtggaataggcatgacaatttatttgaagccgtgaataagcggagtaacggataacgaagtcattcctgcggcttcgctacccgttgtccgtttttatttggttaaatgcagtccttcatgcgctacttccatggtttccactgccacttcattggcatcggatttcatatcggtaaccgtcattttacagggaaacgcattggtcagtgtccagttcatcgccgtttgaccggtttcatccagtaaactgattacaatggtggaacgcttgatggtattcattttgatgagatcataattatcccacagggtagtatctcctttgaagatacctttcttcagggtgatattattgaacttggcgatccccggcatttttactaccgagtatacaggattactgccgccgcggtattctattacctgtgtttcagaagtaagcccggttacttcctggaatatgatctctttgccatcccacatgactttgaaagaaaactttaccataggccaggtggcctgtgattgggtggagccgtcatctgccataattgcaagttttaaaagttattgaatagattttttagttgtggattaagattcctgcatttgctgctggaaggtgatgatgataaattcagcaggacgtgtaagcgctacttttacggtgatcagcatcctgccttccaggatgtcctggggtgtcatagtagcaccaagacctacctgtacatcaaaagcctgctccggtgcggcgccggccagtgcaccctgtttccagaggttttgcaggaagttgttgatcatgctttttaccgtgatccaggtagtggcatcattggattcaaacacataagcgcgggtagccagttttacagattgctcaatcatgatgagcgtgcgccgcacgttgatataacgccagtcgagactattgccatccaatgttctggcgccccataccagggttcctacgcctgtaaatggcctgatcacattgatagactttcctgccatgatatccacgttgagatttttttgttcctcaccggagatgttaaccgtgggggcggttaccatgctcaccgatacattggcaggggctttccacacgccgcgtgaattatctatcagggtatagatgcccgctaatgctccacttggtggcagttcattcatctgcgcacgcacttcctcgaggatatgcacgtaggtaggactggcagccttcagcgactgatggaaattctttttggtatttttatcaggtgtggcgttggtcttaaatttggtgatgatctgcgcagccgctggttcgggtaataatttttccaggtctacgctggcatccaggttttcaaagtccacttcatccggctgcacaatagtagttttcagccagggatgatacgctgcgccgtagttgagcgagttaacgccgatctgttcccggaacacgcccactacatcttccagtacgtccgatggtttttgttttaccaggtcgaagataccgaagcggctttgcatgttggcgcaatgctgtaatacctgtgagtacaccgtagtataggcatctgctcccagtgcaatgatgtcgggcattacaatcagcgtgggttcagcttctttttccagcagggtaaatacattgggcttggtgtccgagccaatgaaatcatctgctgcaatggtaacaccgtctgctccactgccataggtgccaaccgacaggatgtagcagaggcttccgccgttgccgaagaaaagccgcatactgttgtagaagtaggccgtgttattgtctttaatctgcaccacggtcggcttcccgttgatgttaaaggtttcctgcttcaccttgggatctgcgtccgccagcgtgaatttaggtttgaactcactgccgaagtattccaggtactctgcgaaagacgtgatcctggtgggcttgtggataagggatttaccattcctttctgctttctgcgtatagcctatgaacacaggcactgcagtttccacagcggtaatggaactggggaacgcatttttctcctcaatataaaccccaggggtcatgaaggttgatgccatattaggtgattttttgtttagtataaaaatatttccgagtacgtttttccattggtataccacgatcttcctgcagcagatatcctgttgacttccggcgacgggagcggggagatgatgattttgtgtttgttgtcttcctccgatagccggtttgccaatttgaatatgtcaggagtcctatccgaaagttggatagggtcatttgataccagtaccggtacgttattccgctcaggcagcgctgccagcaatggctcgctgaaacaggaaattccgctgttgttgaggattaccgggtgtggcagcgctgccagctgttcactcatcaggtagtagcaccagtgggtgctccgggcctgaaacctgatctcatagttatcctgtagggagtcattcagcatcaatgtcagcaatccgaacggttttgtaaaaaagggttccgtcagcgtatctgttccgtacaggtctgctgcatcagcatatggatgccggtgtaaaacgcctggtgcattagcggcatcattgccaaacataaagcattgggtagtaatgctgccggcatcaatagcagtatagttataaaacagcggatctttcaggattacttcaaaggttagcatggtattgtcctgcagtaagtcgctcctggtgcgctttccagcgcccagtgtgttgtatagcaacaggaacccggatgcctgttgtttaagcatcagatctgcattcagtaactgttttccggtagcggcagacatgcggatgcctatgccttcgtaggatagcgcctggaaaaaatcatgacgatagcggatagtagtcagtatttcatattgctgtttcattcaagtttttaaaactagctaaggataacatttatctcgccggtaacatttctccggcagtgcccgcaacggctggcctgtattctttgatgatggaatcgtcgaacgtaagcatgcgcaccttgtacaaaacggatggcatgtacttggcgcccagcgtagcccacatgttgtttagcctgtcggctccgggactttccagttcaaaggcaagcttgctgatgccggcatctaacgcaggtgtattctgtgcggtaaaggtatttttcgactgaaaaaaggcgacggtgtaggaaagaaatcttaaagcctgcgcgtagttattgctgctgaagtaagcagaaaataatacatagaggttcacggataccgctgctgcagaggtattgtacatgccggcgccggtatttgaaacggatgttcttgctgtctctttttcaacattgacaagcgttacaagcattttgttttcgccctgtatcgctacggaaccatcctggtttacaataccggaaagtatcactttatcttcgttgatctgtaattttcgcttcaggttattgttaatatcttctgtaacacagctaagggcctcatagatcattggaatggtatttaattcttatcgcgagatgtatactgtcctgtaaattgtccgggctgaaaaaggtgttcgttattttgagaaatgaaaatgagttttcatgttgatatcgcaatataaattcaaaaaagcgatttatttatttttatttgaaaaaatatttttctatcttttattatcttaagcatcctgatgaatcccgctcaaaaaataaccgccctcataattgcattcctcgttttttttcattgcgatagcaccgtatacggcaacagcaggagtgtgcgccattatttccaggagtcgccagttaaattaccaaagccaccaaagccgccaccagcgcctaaattgccgaagccgccaaagctgccatcggatactgccgccaacactaagctcatacaacggattttaaaagcctttcgttttcgatataatgctcacgcgcgcgagcgcgcccgcgttttatatgttatcaaccaaacgttaacagattcactggtagttagtaaggatgacatacggaaattaaacgaggcattaaccaaaacagaaaaccagcaatttgattcgctgatgtcactgctcaatgccattgcattaagtcatgcttcgcaggctgcaaatccgccggctgataccagcagtaaaaaaccggtgcaggaacccgatagtgcggtgcccggaactgatcttgacgccctggtggataagatgatgcccatcctgcagaagaagagtgaggaacaggaaacagaaaataccaaagccgctcatcttaccgctatccgctcattgtacggacggccaccggaccaggtagatacattgcggctgagcgatagtgcgggcgcgcgttacctgctccggctttcacaaaaagtaaatgtaatgggtatccagccatactggatggagcagggatatacgacgtacaattttaatgcgctgagtacttacagtttcctcggatacctggttgatggccagactggccgtatccagccagcctttcagcaggatgaagtgaagtctgtgggcgatgcgctgtcggcaggatgcaacctgcagtttctttttcttgataaaaaaagcagtaacatactcgcccttctcaaaaataaaaatgcacaggcaacgttttcggatagccttgcccgtttgttggtgcagcaaaaagcagatggggttactatctattttcaggcactgcccggtaatcaacgtgccgctttcagcagctttatcattgggctttccggtgcgttgaaaagtgtaaataagaactttaaaattaatgtagttgtacctccgtacgacccttcctataactacgatctgcgtgcactccacagttatgtcgattactttatcattgattttacacaggcgggcggcgaaacggcaggaccgcttgctccgctggatggcaatgcgtcaaagtctttgacaggcgctgtttcacgttacctgcaaggcgacattccgcctgcacaactttccttgttattgccttactacggcgccgtatggaaaaaaggaagagatggcaacccggatgttttcagtcgctatgttagctacagcgatatccgcaagcagtacccttcggatactgtggccatcttcgatgaaaccaccgctactttttttatagaagtaaaagatcagtatggcgtagtaaaggaggagatctggtttgatgatggcatcagcatgtcgatgaagtatgactttgtaatgaagaatgagctaggtggcatcgcaatatggacattgggcgccgataacggcaccacagacctgtgggatgcattggtagataaatttgtggtaacagacacgcttgttcttgatacggtatcactgtatccccccatcccgcagcatctcacgttctggcagcgcataaaaagagaattgagcatatacgctatactgttcaaagatccgtgcagcgtggatgcctcgcagtatgaaggggatgtttactttatttatttcaccatcggcttttttattttagtgctgatggcgggtgcggtgtacttttattttgtaaaaacacaaggggacgactggaagtggcgaaaaaaattattgatactattaattgtactcatcctgcttacggtggtcagtggctttatggcgctttttctaaataaggaaataccctttgtagggatcagcagcgtaccaggtcagtgtcacagtgtgccgctaatgagtgtgctggccatactgggtattggttttgtgctgggattattgatcatgcacttcttcctgcaaccattttttaaagatgatgatgtgccgtagagcgtaggttgtctttctcaggattacgctgattttactgattacctggatttttactttttggattttataaaggattaagggagatagaagcggatatcgctcttatctcccttaattattatttttaagaaaatctaaaaatctaaaaaaatccaaatgtaaaaatccaggtaatcagtaaaatcagcgtaatcctgagaaagacaaaattcgcgtttacttcttattccaccacactggctggctgatatacgtcgggctgctggcagtagggtctgcattcagtacctgtgtgctgttgtaattgatttcatagctgggtaccgcaaagcggcgtggccaatcggtttgggccgggtaatacaacgtgttaacatgcgcgggacgtttaaaccctttataaacgccggttgtttcgttatagtttccggcggcgtcggtgcagtagtttaaccggcgcaggtctgcccagttttccggggagtacgacaacgcaatgtatttctggatcatgatattgctgagtgtgagcaatgccggcagctgcactacggagctgctgttgaggaatgcgtcgatcgttccggctgggatgtccagcagttccatatgtgcgcggataccggctttataggctgttaatgcttctgtgtttttagcctgcttaataagaatttccgcttcaataaaacgcagttccgcattggtaaacaataatcctttagcgcctctttttgtgtaccaggtaccggtggattgtatacggtcggtggtggttggcgcatacggtgttttacgcaggatcacataaatggaatccttgttggagaacgtattattagtcgtactgtaggtgtatgacaatggaccggtattggtaataccggaagtcatgtctacgccctgtgtgcggtgcagtacgccgttccggtcagccatgcttggaatgagcaggtctactcttggatcttccatattattgatgcctgtaggagcgccggtgtagttattggtgaggtagtccatgtacagtttggtgatcctggcggtggtagctgtattcgtgtactgtaatgcttctttggcagaagaggtgactgttggaccttcatctacatattgcatcacggcgctttggtctttcgactgtgcgccttttgaagcggcatccagtacggcctgtgcgttgaagccgggcaatgcggaggtgtggttcaaccagcgtgcttttaagccgtaggccaggcggatccatttgtcggtgctgccgttgttgaggatatctcctttggccagcggaggcgcagtaggtccctgtgttttctgcaggtccgcaatggcttcatccagcagtgccagcactttttcctgaacgtaggatgcctggtcaaattttggcgtgatagtggtgggatcgtcgaactggtcatatggcagcatgccgtatacatctgcgagggtgccaaagccccatgctttcatgattttggcggcgccgatataatgatacgcctgtactttttctgcggcggtgatgagtggcgccacgtttacggcggtatttacataccagcattgccacggccattgtatgttggtgctgttggatacccaggcagtaagattgtagttacttccgccgctgacgtatacggaagcgagttgttgtgagagataggctgcccgggtgccggtgctttcatatgcatcgcagaactgggcgatgagtggcggcagccgttgttcggcggtgggtacagatgaattggcgctattgggattgtcgttgatgtccacccatttcttacaggaggcaagtgcaaacgacaggctgatgataaagagtatttttttcattttccgcacgtttagaatttaagatttaaaccaatggcaaatcctgctgtggcaggtaccccgcaatagtcgatgcctgaagagccggagcctattacgccggcgccggcagtactggtttcaggatccatgccggagtagttggtcagcagtaaaaggttggtgccggtagcggttactgtggcatccctcagccagcgtgcgccgctaagccatgttctgggaagtgagtaggagagggaaacagaacggagtctcatccagtttactttttccaggaagaaaggcgcgttctttacatacacatcgcggtagtatttctccgactgcaccactgttttcgttaccggttcaaattttcctgtggtgggatttttagctacaccgctgaaggaaatttcgctgttcctgttttcggtgcgttcgctcaggccataggaggtcagcaggtagtcggtgccgttaaacacatctccacccaccctgaaatcccagaggaaggaaaagttaaattgcttataggtaaaactgttgttcaaccctccgagaaagtcaggctcacggttacctatatacgtagtaagggcggtggtaggaatcgggtagccggtgttccagtcgagcagcaggttgccgttttcatctttctgccatacggagccgcttacgcccataaacacgccaccatcaaaggatgcagcctggcctactgcaaggtgcacatcagttacatacaggataggcagggagcccggcagggattttaccacgccgttgttatgcgacgcgttgagcattacctcccagctgaaatcttttttctttatcggcgtggcgttaatggatatttcaatacccttgttttcaatggtaccggtattcacagagctgaggatataaccggtggcgttgcttacgcggggcgtgaggatctggtcgcggctggtggtaacataccaggtgaaatcaaatccgagccggccgttgaggaaacgcatttcggtaccaaattctgtggaggtagttgtttccggtttcaggttatcgtttcctctcgaccagtagttgcggaagccgccgccaatagtaagttcaggcccgaacaggtaagtgttggtctggtaggtaggagcgtctttacccacctgcgcccaggaagcacgcagcttaccaaagctcaggatattgtttttggggatcagctccgtaaacaccaggcttccgcttaatgaagggtaaaagaacgattggttctgagatggcagggtagaggcaatgtcgttacgaccggtagcgctcaggaatacaatgttcttgtatgacaagcgcaggtcgccatagaagccggctaaccgtctgcggctgattccctggctgatgtactggttttccttggcagcattgttaatgctgataaaggtgggtatctggaaactttctgcacgggcagaattggattttgtgtagctgtcttctgtagtagtacccagcagcaggctggcatcccagtctttatgaaaggttttgtggaagttcagcatcaggttggagtttacataattgtagttccggtctgtttccgacagcattcctttctgccagccttctttgacactggagccgggggaaattaaattacgcagctgcgtgtagtagttgtctatgcccaggcggtaggtagcgtcaaaccagctggttacttttacatttacataagcagaaccgataaagcggttggttttatccgactgcgggttacggttaatgatccagtaaggattgtcgatgtcggtatccagcggaatatccggcagcagccggtgcttggagccatctgcgttcagccatactttcatatcatcgttccgtggccaggccacaatgctttccatataaccggaaccgccggaggcccataagccgcttccggtaagtgttttctgcgtttcactccgcgcataggtagcatttacgccaaacgtaaaaatgccgatcttctgttcgccgttaaaccgcacggtagaacggttgaagtctgtggaaggcactacacctgactggttgaggttagacccggagagataaaagttgccggtggcagtacctcctgaaatggtgaagctgttatcaaacgcattggctgtctggaagaagtctttcatgttatcatagatcttctcgcccgggtcaaatttatttccccacgacatcgccgtctgatcggtaaaggtgccgttataattggagccttgtttatagatactttgctgtttgggcagccggtttacccagttggtaatatagcggctggtaacggagccggctacatttccggtggtaccttttttggtggtgatcacgatagcgccggcagcagcacggagaccataaagcgcagccgcagcggggcctttcaggacggaaatggactcaatatcttcggggttgatatccatggcgcggttactataagtagtgctctggttgatagatccatcgaaggcgctgttgtcgccctgcccggtggagttgtccattggcataccatcaatgataaacagcggctggttgtttccttccagggaggtacctccgcggataataattgaggcagacgcgccgggtgcgccaccggagttggtgatgttcaggcctgcaattttaccgttgagggaattcaccaggttaggatccttgtttttcagcagttcagccgatttgatgtcctgcacggcataacccagtgcttttttctcttttttgatacccataccggtaacgatcacctgttcaagcgaactggcgctcgtcagcattttcacgtcgattgtcgggcttttcccggtaggaatgctctggctttcataaccgataaaagaaaattccaggacttctcccggagttaccgcaatgcggtaatgccctgtagcattggtttgtgtattacggttgctacctttgattctgacggtgacgccaggcaggggattaccatcatcggctaacacaatgccggtaatgagtttttgctcctgtgcataagcaatgttgggtaacatcaggaataccagcgataatatcgccaataaccggagaggatttctcatgttctgttgttttaaatgaagcttgatatttggttgaaactatacgcgtgtttaggtttacaggttgttacaggatcttgtttacaaataggtacgaactacgattttggttaaactacatagtacgggtaactaaaaatgacgattctctataagcataaactttcactaaggtaatggcaaaaaacattcagagttaatattaaattcacctgttttctatttggtatttaagatgatggttaaataaaagtcctttgggtcacggttatttcccggatgcttcatccatgggtcaaacatgggtatatcatggatcatccatgcggttttaatactgttcgcatgcactccccatggacttcccatgcactccccatgcactccccatggactccccatgcactatgtccgatttgggggcggcggagcccggattaaaatgatacccgatatcagtataaccgggcatcctgctcatattgatagaacccaatacagtactggaaaaaaaaggtaacgccatccaaaaaagcagggtactttatcctgctgatctgtgtaatccttgtaatgattcgcattatttttattttcgttttctccctgcccttttttgcaatggcgcagcaacagcaagcagataccacaaaacccagaaagttaaaggaggtaagggtaaaggcacgctggcagaacaggcatgcggcgttaaataagcaatatgtcatccgggaggaattcagggccattgaacattatacttttgatctccgggaccccatcaaccccggcagggaatactttgtgctggattttctgaaccgggagttgccgcccgggtggcaatccagcagcgtgctttcctgctcctccggggtacaatatttcatagacgagaatgaagtgcctgcggccatagtggccatgcgcccgctgtcggatttcgcctacgcaaaagtattccaggatttacatccgccgtgtccgtgtattgtattatacaccaggaagggggaagatctgaagcgtaaataacagggtgcgacctctcacctgaactgctttttcaactttgcaaaatattccttaacggccccggctttatctttttttatcttctttccaagttcccttcgcggacaatttacattgtattttgccccccaatccattatttcaatgatgatgggcaacaggtctattccttttggcgtaagactgtaaaggaacttcgacttattcgccggtgatacccgctttaacaggataccttctgcttccagcacgctcagcctgttcgacaggatattggtggcgatcttttcttccgactccaggaactcactgtaagacaatttccccctgagcataatgtccctgatgatcagcagcgaccaccggtctccaaaaacatccagcgagcaactgatggggcaatccgacctgactttttccatactgaatgattttaaaaagtacttgcaatttacaataactttattatttttacttgcaaaatgcaataactaagattgcaattcctgattctttaaaaatagaaaaaaatggaaacctccacgtcaacaaaacaattactcgaaatttattacaatggctttgccaggaaagaaggatgggagacagtcatctccgacgactttaaattcaccggcggcgatatgacaaaaacggcgcctgctgttggaaaaacagcgtatatagaagtgattaaaagattttcacgggcattcaaaacaatgcgggtgaaggaaatgatcatagacggtgaaaatgcctgtgtaatcggaaattacgattttatatttcccgacggagtaagcatcaatggcgatgtagcggagatctggaaggcaaagaacggaaaactggatgcactgaccatattctttgatacgcttacttttgacaagcatatccccaaataaattttatggcctacagtgaaaagctggcggataagatccggcaggcactcgcacaactgcccaatgttgaagagaagaaaatgtttggcaggattgcgtttatggtgaataataaaatgtgcctgacagcaggccccggccagatgatgtgccgtattgaccccggtattcatgaagaagcgataaaaaaagaaggctgccgtacagtgatcatgaaaggacgggagtacaaaggatttgtatatgtaaatgaagagcatcttaaaacgaaaagagattttaattactggttaacacttgcccttgaatttaataagcaggaaaatacaccggtaaagggtaagaaataaagtcgctatagatggttaccagggcaacctggagcaggaggggcaagcggtttcccgccggcaaggcaaattttttgataagaaaaaaaggactaaatttaccttgtacagggaacttaatgaaaaaagaaaatgagctaaatagtgaacaagcgctcttccggcttattgctgaaggggatgaaccggcctttaaagcgctttttgaatgctaccgcttgcgtttattcgcattcgctctccagttcactcattccagaaccgatgcagaggaggtagtgcaggatgtgttcctgaaaatctggaaaaacaggttaaaccttgccaatatccagcttccacaaaagtatatctataccatgacgcgcaaccaggtgtttgatcatctctcacgggtggcaaggaataagcgtttgcatgaacaggtatgggcaaatatccatgaaagcggcgattacaccgagcaggcagtgctggcagctgaaacggccaatatcgttcaaaaggcggttaacggtctttccagccgcaagcagtccatctactacctcagccgccgggaagggttaagtaaccaggaaatagctgtgcaactgggcatttccgtgcctaccgttaaaaattccctcgtggagatcctccgttatatcaggacctatatgagcaaccagtacgaatcctccgtcctgatcataggcttcctgctctctttctttctataggaaaattttttttgcattcaaccggtacggttgcctttattaacagtctatatactggaggaagtatttccccctcacgttttatgacagaaaaggtaattcccgcttatgacaggctgcagtacctgttacagcaatatacacgaaagcgctgtactcctgaagaaatgcaggagttgttccggtacctggaaaaccccgcggtgagggagctgttcaataatatagtggataaagattttgaagctcccggagttgcggaggacggtgaggagatcgattgggagttcatgtataataagattgtcctgggggaggctcctgctaaaagaatcaggatcttcaatcttttgaaaattgctgctgccgtattaatcctggtttcagcaggctgggcatggtcgcattttgctgcccgccgtgcggcgcccgttttagtgcatgtgcaacctcagggagatgcattgcctgcggcgaataaggccgtactgatactggcagacggtaacaccgtgaatctcgacagtgccggcagcggggctattacccggcagggtactgttaacctgagcaaggcgccggggcatctttcctacgccgcagcaacaaacggatccggtaatcctatatataacaaggtggcaacgccccgtggcggcatctttaaacttactttatccgatggcaccaacgtatggttgaacagtgcctcttctatccgcttccccgttgctttttcagacaaggaacgcaccgtggaagttaccggggaagtatattttgaagtggcaaagcaggtggtaaaaggcaacccggttccttttttctgtaaagccgggaacatggaggtggcggtgctgggtacacattttaatatcaacgcctataataatgaaacggatataaaaactacgttgctcgaaggcgccgtcaaaataaaacagggtgcaaatacaaaactgttgcaacccggacaacaatcccttgttggaaaagacggtcagattgcgctttctgatcatgtaaatatggacgaagtaatgggctggaagaacggctattttgtttttgaagaagcaaatatcggccagatcatgcgggaggtggaaagatggtataacctcgacgtggaatatgacggcccgctaccagacggccgttataacggacggatatcccgtgccaccaaagtatcgcaggtgatgaaggtattagaattaagtggcatcaacttcagaattacaggaaataaaatcatcattaagtcccgatagcacaaattaatatcaaccaaaagctatgtcagcgagagttttcataatgtactcaggatagtcatggtcctgatccacctacttattgtaatagttcaataaaatgccgcttcatgtgcgagatgaagcggcggcgcctgaactaaacggaattcctttgtcagaaattttcatttaacatccaaacaaccaaaagtatgaaattgcaggcttttcggaaagaaaaattcccccgtccggaggggaacagcttaacgatcccttttaattggaaaaaaataaaaaaactgctatttatgaagctagcggtcctgttaatcattgtcagtacgggaatatcggccagcgcccattcccagacagtgacgctgaatgagcgcaacctgtcgcttaaacggatcttttcattgattgaaaaacaaaccgggtattctttctggtatgatgttaacctgctgaaagaagccaggaaagtagacatccgggtagacaaggcctcattgccggaagtgatggagctgagtttaaaagggcagccatttcattacagcattgtcgataatgtgattgttgttagcaggaatgcccctgatccagccgccgcagcgccgctgcgggtggaggtttccggtaaggtaaccgatgaaaacggcgcgccgttgccgggcgtatccatccaggtgaaaggaacaaaacaaggcgtgagtaccgacgcaggaggaaatttttctctcaacgtgcctgataatgcttcccatacccttattttctcttttatcgggatggtgacacaggaagtgccgttgaatggcaatacaaaactcaggattgtacttaaagccgctatcgagcaaaaacaggaagtagtggtgattggttacgggtccgttaagaaaagaaatgtaaccggtgccgtatcttctgtaaaaactgccgagttgaatacagctgcttccaccaatgtggtacaggcgctggccggccgcgctgcgggcgtatctgccatccagagcagcggacagccaggcgccggcgttaacctgcagataagaagtaatccatcgtacgcttccccgggagcattgtacgtggtagatggagttatcattaacgataacgccgcggaaccttcgtcagacacccggtatggcagctccggcgttgaccggtcgccccttaattttattaaccccaatgatattgaatcgatcgacttcctgaaagacgcttcggctacttcgatctatggcgccagggccggcgccggtgtggtgctcatcactaccaaacagggtaaaggagataagccgcatattgagtacagcggaagctacgctttccaggatatcatcaggttttatgatatcctgaatacgaaagaatatatggagcaacgtaacaaaatagggctggaacaatggatgctgactaacaaggttgcgccgtatggcagcaccgatccgggcacagttacgccgtatattccaaagtatacacaatcacaaatagataccactgctttattacccagtgcaatagatgcgatcacccggaaaggctataccaagcagcataatatttccctctccggcgccagcaataaaacgcgttactatgtatccggcaattacctggatcagcagggcgtgctggagcactctgcgtttacgcggtataatggaaggatcagtcttgaccagggagttggcgaaaacataaaagtgggtgtaaacgtgatcgcttccggttccaatgccatcaacgccaacgtgggcacacaggcaaatgaatattccggcatggtgctatccgcattttattacccggccaatatgcccctgagagatgcagcgggtaactatctcatcaacccggactaccagaactcaccgaacccgctgtctttcctggatattacagattacaccaaaagcagccgcctgcttacttccggctatgcggaatggacaatcatccccggcctgaaagctaaaatgaattacagctatgatcagtcctccgggaaacggtatgcctatctccctaaaacctttctctatggtgcacgcgcaggcggacaggcatctatcaacgaaaataactctgtctccaaaatttcagaagttacactcaactacaataaaagcttcggggaaaaacacaatatccaggcactggccggacattcttaccaggtaagtgattgggatggtttaggactttataacgaccggttcccgaccgataactttctttttaataacatcgggtacggtaccgcgccaagacccggcgtaagctcttacagaaatcctacccgtatctggaaatcatattttggcaggattatttatgattttgcagataagtatatcctcacagccagcatcagaagggacggcgcctccaattttgcacccaacaaaaagtggggcacattccccggcatttccgctgcctggataatctctgaagaaaatttcctgaaaaataatctcccggtgatcagcttcctgaagttaagggcaggctatggcaccaccggtaacagtgacatcggtggcagcgccttctcctattataccgccaacagctcttatgtgtttggaggtaccagcctgcctggtgtgtcgcttagccagctgagtaacgataacctgagctgggaaacacaaagggatgtgaacgtaggattggatttccagttgttcagtaacagggtaggaggttcattcgactatttcaacagaacgattgtgaacctgctgcaaagcgtaccgctgacttcggacttcccggtatcgagcgtggcgggtaacgctggcgaaacacgcagccgcggatgggatgcaagcctgaatacaaaaaatattatcagcaaaacagcgggaggttttaactggtccaccacgatcaacctgtcgcattactataattcctgggtgaagagatccccggatgcattaagatcgctggcaaaatatattgcccccgatggtccgttcaatgggctctatcgttacgtcagcgatgggatctataaaggagataaagccgcacctgccagcatgccgggcatcctgccgggtggaattattgtgaaagacctgaacggctacgacgatgcaggtaatcttaccggtaaacccgatggcaaaatttcctctgccgaccaggtgctggtgggcatcgacggtccgcgctacagttttggattcaacaacagtttcagctatcaaaattttgacctgagcattttcatgtatggctttatccagaagaaatataattctgactatgcgtctgcattcagtacttatgcgcagctgggacaatttggctggaatgtgctgagcattgccaaagacaggtggtcgtacgataatgtgaatgcgaagtatcccaccggtctcaatgatccttatgccagctacgccgccaactcggactattggctggaaaatgccagcttcctgagatgcagggatattaccctgggctatactttcggcggaaaaatgattgccaaacagaacgtattgagcggcttacggatatatgccaatgttcagaatccttttatcattacttcttacaggggaattgatcctgaattgcagaactacctggcatatcccatgtcccgctcttacactattggtctgaatgccaagttctagcctctttattcattttaaaaggaacagcaatgaaacgtccaaataactacagatacgctttactgataatttttcttttctccctggccagcttttcctgtgaaaaggggctggaagaaaaaacatacgaccgttattcttcctccaccttttttctgaatgccgaagatgtaaaagcggcggttaccggtatgtatgccggtatgctcaatgcaggattttacgggggaggctggggcgccgccaatgaaggctggaatgcccagagcagcttcaccacagatgaactggtgtgttcctggggctgggatggctggcgtaagtttaaccagctgaatttttcggaagatttttcccaactgttaaatcattataatggcctgatgccggtgatttctgaaatagccattgacatcgacaaaatacaaggcgtgcagatggatgaaaccctgaaaaacaggtatatcgcagagctgaaggcattgcgcgcccattactcctggattctctataattgctatggccctgtgcctatccgcctggatgcgaaggaagcagcaaatccttcagcacaacctattccccggcccgatgccgcatggatggtagcacagatagaaaaagattacaaggaaggatttgaggggttacccaaggccagtgaactggcagcctccgattatggcaggtttacaaaggatatctgtctcatgggcctgatgaaattatacctgcatgaaaagaactgggcatcggttatcagtactggtaaacagctgcaaacatatggtcatggcctgcagagtaactataaagatattttcactttcgccaacaaaggaaatatccaggaagtaatactggctatcccgtgcaggttcgacgcatcggtcaataataacctgtggctggccatgtgtatgccgggtaattatgtagatcccgaaggacttaccattacacaatggggtggttataagatgccctggaaagcctacgacaaatttgatcagcaggataaacgcctgagcgttttgctggccaaatggcctacttccggcggcgctatattcgacgcccgtgcaaataattatattggcgccattcccatgaagtatggccctgatcccggcgctatcagtgaagcacagggaacggatattattgtgtggagatatgcagatgtgttgctgatgctggcagaagccattaacgaaacccagggccctgtgcaggaagcctgtgacctggtgaacgcggtgagaacccgcgcaggcgtggctacctaccagcctggtcaattcacgaaggataccttcaggaagaagatcatggatgaaaggttctttgaactgtggtgtgaaggaagccgccgggaagatatgatccggtggggaacctttgtacagcatgcgaaagaggaaggctccatatttgcaaagccggaatttgtgttgtacccgttgccccggaaggtaatcgacgaatccaaaggtgttatcaagcaaaataatggatactaaaattaaagtgacggacctggccttggcctggtccgttactttattattgctctgtggctgcgcagggaagcagccggatcaccggcgcgatatcgcaaaaagatattgcgcttcctgtcatttgtttcctgaaccggcactgctgccggcgcatatctggatggatggcgtgctgccggcgatgggcgcctttgcggatatttataaggaccgcagcggcgaatataagatgctgccgccggcattgcagcacctgcgtgatccggccatagcgcctatgagaacatttattcctttggacgactggaaggaaattgtggcctggtatgccgcatcggcgccagcagaaattgcgcagccggtatttcctgttcctgtgtccggcaacaacttcctgctgaaattaccgccaaaaaaatcggcgtcttttacatcttgcatttattatgatgaaaaagcaaagctgctgtttcaatcagatattaataagcgtatcctccgtgtttttgacccggcattgcagcaggtggacagtcttgataacagcacagtggtggatgtagcgcctgtgggcgaagggcgttacctgctcacgcacattggaagtcttaatcccggtggagtaacgaggaatggcgcggtggaggaaattgccatcaaagacaataagattatacagcgaaaaattttatgcgaccagctttaccggccggtacaatcgctcctgctggatgatgagctgctggtatgcgagtttggttttatggaagggggattgtctctatttaccaaagccggtaaaaaggtgatcgttaatcttcccggtgctgaaaaaatgtatatagaagatattgatggagatggtaaaaaagatatttgggtattgtttgcacaggggaatgaaggcatcttccagttgctcaacaaaggaaacggtaactttgaaataaaggaggtattgcgattcccgccttcctatggcgctacctatttccagctggccgatatggatggcgatggcaaacgggatatcatttttacctgtggcgacaatgcggatcagtcgcccgtactgaagccctatcatggcgtctatattttcaggaacacgggcaatgcctggcgccaggtattcttccagccgctgtatggctgctataaggcagtgccggcggatctggaccacgacggtcgcccggaccttgttgctatcagcttcttcgctgattatgcgcagcatcccgacctggcgctgacctgcctgctgcaaaaaaaggatggacagtttgaattacataccgataaacaggtggctggcatgggccggtgggtatgtatggatgttaaagattttaatggcgatggcaagccggatatcctcgccggaaatatggctgcaaagccggggaatgataagtctttgatgaattactggatgaatggtcctgaatttattatctgggagaaccggtattaaatgtgtttattcaatgccttattcacgatgcgaaaaaccaggtaggaaaatgtgccaccgataacagaggcaatcacatcttttacgtcaaaagtccgcccgggcatccacaactggcaaacttcatatagcgtgagtccagccaccagcgaaaaaataaggctgacaactttccggtcgtcgacaggaaaccttatcaccatgtatcccagaaaaaagaccaccaccgccaggaagtttggcagggaatccgctatgtaaaaggtgctaatatgatgcttgaataagtaaggtctgagtttcagctcttcatagagtgtgaataggagtgcaatggaaagaagaataatgtatacgttttttttgttcatgggatgaaatcataaataacaaaatgcaaagcaggttcaaaataaaacgaaaattttgtaacttccttacaaataaccatttccatgaaggccgcgtcatcaccggatacgttaaccagttcgcatgcagccgctaaccaggtggcagcctacggcattgcgatgccggcggtggtaaaccgggaggcggcgccacaggaggaaatccccactgcagaagtaccgtttaatggagaactgacggagccattgctgatcgatatggacggcgatggcgaagatgaactgcatacgctgatcatggacaccgcagacgggcagctgtggctgcattcagacaaagaaacactggaactttttctaaggcggaagcgcagcaaacacgccaggcatatgacgccggatatcgctaaactgctgaacgatattgaggcgttggcgaagaaggtgcatgtgaatacctatggcactaccaaggcgactaacagagtcagtaagaagaccggtttaccaaaaaaatctcagcacgtggcggccacaaaggcggagcgcattatcgcagtagtacaattaagagagatcgccggattgctaaagcagctaaacgcgaagtcggttgatgtgatgaaaaaggtacggccaccatctcataaagaaaaatcatccgttcatacaacggtcgacggggatactttttgtaaggaagtggtgatgcacccattgagcctgttgcccagggatgacggtgtgacgggaagtgctcctacgggtgaatcaaaactattcacagcgctcaacaaaaagatcacgtatatacgtggtcatatgctgaatgatcacctgcatggaccaggtactaacgataacctggttcctatatccaccccgtttaatagtttgatgaagacaacggtggaggcgaaaaccaaagaagccgtgaatgccaacaataaagtagtgaggtttgaagtggaaacactcgaatggggcgcatacaaagggttttttaaaggcactttcctggaggagaacaaacttcccgctaagttcagatttcttgttcaacagctggagcgggatcccacaaaagatggcagtgaaatcggccactggaaactggccgctaaaagcccggtattcagtgaaacactggtgcataccataccaaccagcaaagaaaccaagagcggaacaatggcgctggtaccggaaacatttatacctgggtattacttttctgctgccggaacattaaaagaagtgccaccggattatcatctttcagggaaatattttgttaacggatccagattcgactatctttttgaaccgtttgggctggataaaagtgcactgttttctaaggagtacgacctggagatcaccacagcatttaagatgccggccggttatgaactaatactgatacctcagaagccgatagcatttattcatgataataatatacattccacgacaacaccagaaggccaatcgtttcttatcgccaaaaaaacagagcaggcggctaatgaagcagcatatgcggtgaagatagaagaagtaaggaaagcaaaggaagatgagaaactggcactggaaaagaaaaagacacccaagccggagtataaagtcaaaaccgtggcagaacttaagaaagagcgctggttacgggagctgggaccagcgttcaaaagggaagtggagaagtataccctggaacttaaccccgaatttgggaaacgttttgcggttatgcaggaagaaatcctgagcagaacggttgaagagtggaagaaagatccgcagttgggtgaaaagaaactggaggatttgctggctcccctgaaagcgcaaattgtaaagaacaagagcgcattactcattgaacaaggtaaagctgattttgtgctggggctgctgaacgaattaaatgccacgatcagctcgcaataccggcctaagttaaccgaagactggcggaaaaggaagttcgatgcagcagcaaaagatattttcgacatgtataaaaaattctggcgggaaaatcaggcgaaattggatctgaacaaccgggaggtgctgcttaagtccgcctatggaaaactcgacatagcactgaaggaagcccaaacagccgcacctataaaacgtaaatccgaaacagacctgaaaacagaggataccggcgatgaaaaggacaagaagcctaaaatccttccaggaccatttgttcctaatacgaatgtaacaacatctccgcagcgggatataccccgtttccagccgcaatccccgcctgtcagtgcaccaacactgaccgttgccgaccgggagacggccgacgagttgctggcgttggtagccagcgtggcgcatgttgatccggcactgctaccccagatgggaatgttaacagagagtatccaggagttcctccgtggacccaatgcgcaaacttgggagaatgtgtaccggatcctggaaaaatgtaagtcagtaaagggggtggagcttcacttattggattggatcaggatgtgggagtcgatgagtataagatcgacctgacacaggattttttatcatcgatacggaccctttcattcttcatcaatatacgcctggaactttttctgaacatcctccgtgaaataataataaccatactcctcgtttgcctccacataatcctgcaaatgcattttatcagcaggcatgattccctctttcataatggtaaaaacatgtgctccttttataccgtaggcaattccggtgtaagaaatcaggttgataagttcttcaaattcaaaaccggtatgctggcttccgtcaatattaaacaccgcccagttgacgtcgtcatgcacggcgatgtattgcgatttgaggaattctattgcggcgtattcaggcgccagtatccatttgctaaaatcaccgcaggtgaagaataagccatcttgattattggtaataaccttacaaaagttgaaagacagatgttcaagacgttcgggtaactccttaataatagccgttatcggctcatcggtaattggacgcagatcttctattaaatcaaagtcaaaatccagcaccagtcccagcgggtatttaaacaatccttgtttatcattcttactcattaaaaatgcgtgtccccaggtttcaatgatgtcagtataatcagccagtaagatttctccactggaagatagtaaaacattatgcgcctgatatggatgttttaaaacctcgaatataacaacctcttcattaaaattttcagcatgataaatagctctccctttaacaaaggcaggatcgaatctgccgagaaaaacaaactgaccggagaatattaaatggctgccggcgccttcctcttcgatggtgtaaaacgtttcatcgtcggaaactttaatttcatgattataatcaaaaggcagcattactttgtcatcagcatttattaccccgtattttccattcaatccggccgaccagtaacttcccaaaggcgttaaggaggagaggtcatcgtaacgcggcgggagcttgatgttgccgttcgattgtatcaggccatacttgccctctaagttcactactgcatatccgccgtcaaatccataggcgtcgttataaaccggctgtacaaccattttcccggatttatggatatagccgtacttcccgtcttttgctacaacggcgagttcttcttcttcatcgaaaccatagaactcgtcataaatcgcttccgccaatatctcccccttcttatcttttaatccccaaagtccgttttcttcaaaaatatctgtatccccggtatctgcctgttcatagatatacctgaatccataatcataaccagggtaattcagcaaggacctgaaatcggagaaccccagcatcaccccgcctgcaaatgcagcaggggttaaaagcgaaatatcatctgcgtctattgcacgggtgatgacattgttgttataggctatcaccgtcaacaggtcattggcttgctgctgatgactttcatcgctcatgttaaaaacgtcccaggcatctacatgaatgtaaggctgacttaaattatccaggtaccggaacattttttctttggcaatcgtaaaattttctatatcatctatcagtgctgactggtgattttcgataaaattataaaaccgtttaatgttttggattcccttttctgcattataataaagaccaaaattttctggatcggtatgcgtgttataaatattacccgccacaaaaccttcgtcaatcagcaggggttgcagcagcagcggcacttcgtatccccattccattaccattacatcggtatcctgaacaacagccggggaagaaatattatagaggtaagctctgtgagacataatgaataatttcagacggaagataaatcaaatgcagataaaaaaatgcgccctgtatacatttgtatacagggcgcagaaaagcactataacgtgcaaggctatatttttatcatggtttaaattcgagccagtccagtgtaaacaaatgctggtccggttgctgatctttgctgaacacgaagtagaggtcatttttaccggcaggtgcttccactggtgcggttacttctataaatttatcccagttgccggtggctttgtatgccagcttgctgatcactggtccgttcacgctgccagtatgaatttccagcacggcatccttgtcgagggatgaataccggtaagtgactttatgaatacctttcagatcaatatccctgaatacaaagaacgatttgttatgaatagccccaaggtgatcagatgaacggtctatgttgttaacggagtccgcatcttctccctgtacgcggagggagcgaaggagcagcagtccgctgccgctgagcggggaggcgttgccgccgccatctgtataggtggctgccagtacataggtgccatacttttccttacccaggtgatccttcagtgctacgctgccggaggcgggcaagctgcctgccgcctgtggcgcggacagcgtgaggatgtattttacaatttgtccggcttcgtcaacagacagctgcggatgtgccgccatagagtgttctccccaaacgccgccgccgcctttaatgatcttggcagcaagataggctggtgctttagggtctttctcatagcgtttggctacctgtgtaaaggcagggcctacggaggctttatctacctggtgacacgccttgcaatcgctgctttccatcagcaacttgccaggatgcgccggtaccgtggtaatgagctgatgtcctttctctgctttcgctttgctgcgtggaatgtaatgcaggccaatcatcagttgctcgttattgatggccggatcttccttatccgtcactgtaacggcataatgcagcgggctgttttcaaaatagaaggtagtgttatcggttgtgctaacctttacttccggtacggtgttacctacgcggatggttagggtatcggtgctgctggcgccttccggatccgttattttcaggatggcatggtacacgccattcttttcatacgtgtgcacaggtgaggaatcagttaccgcagcggtttcatcgccaaaatgccattcgtatttaagtgcctgtccttcatcaaaatcatagctctttttgctgctgaagtttactttcatgggggcagtgccggcggtatcagcagtggcaatagctgctaccggtgcgcggttgccaccgttataggaaatgcgtaccagtcgcgcatcgtcgttgtcgataccatatacggagccatactcgagtatgtacaggtcgccgcctttaccaatggccatgtctatcgggcgcctgaaatcgccgttggttttcatgaaaggttccatcgatttaaagtgctgctggctgtccagtcgcacggcatatacccagttacgcatccagtcgtaaataaataaggcgttatcataccatgcaggcaaaccggtaggggaggcagttgcttcattataatggaatactggtccggccattgcgcagcggccgccgttgcccagttgagggaatacggcagaggaatcgtacggataccagatcatggccttttgtgcgggtggcaatactttcagcccggagttattgggtgaattgtttaccggcgcttctgctttgaaaggtgcgccgatggttttggtagcgaaatcatattgcgggtatactttattatcacctactacaaatggccatccgaagttgcctggtttttttgcctggttgatttcgtcgtatccgcgcgggccctggtcgccgtcctggcctgcatccggacctacctcgccccagtaaacaatgccggtggcagtgtcaacggacatgcggtaaggattgcggcagcccatcgcgtatatctcagggcgtgtgccggcggtgcctttgggaaagaggttaccggcaggaacggtgtagctgccatccggttcgggatggatacgcagcacttttccacggaggtcgttggtattgccggcggagcgttcggcgtcaaaagtaatgcggccgggaatagtgtctatcggcgcataaccgttggaagcgaaaggcaccgtgttatcgccggtggaaataaagaggttgccgttgcggtcccagtcgagcgaaccacccgtatgcgcgctcacttccagttccagcgggatggtgagcaataccttttcggaagccaacaccagggagtctttgccttccagcgtaaagcgggatacgtgttgcgctgcgggaagcttattgggcgtatagtaaaaatagatgtaatgatttttgtcgaagtccgggtcaagtgtaacacccagcaacccgttaccaaatccttccttcgtatcggggagtaccgggaatgtatatacgactttggtggcctgtgtggccgggtcgtagtgatacaatttaccgctgcgttcaataaaatacacgctgccattacctgctaccgccagttccatcggctcgttgaggtcgttggaaagaatggttttggtaaaacggttgtcttccggggctttggtagccttgcttttggcagggtggtcgccgcatccctgtataattaatgtcaatccgacaataaacagggccggaagtctctgcgtgcatagcctgaacagttcactcatgtgatgtgattatggatttgatttgcgggacacaaaataatagaatattattttttatttccttaaaaatggatgaaaggaaataaccacatcgttttgaggatcagggaatattggctaatttaatatcagattggaagaggaagttgtcattttgcgctgtgcttccgtatatttgagacccacattattcaagctggtaaatggaaaagatggatctgaacgaatttaagcaatctttacaggagacacacccacctaaatatgtcgacatataccttgaatccctttggtacgaagggaaaggtaactggaaaaaggcgcacgacctggtagacgatctgccgggaccggatgctgcaagggtacatgcttacctgcacagggtagaaggagatcaggcaaatgctgactattggtaccgccgggcaggcaccaccaggccttctggtacacaggaagaagaatgggaacaattagttacccagtatttaaaataaccggcaactgacggttaccgattgccaatttagcgtgtacattttacatttgtcattgattattaggctataaaaaagcactaatttgtttattatttgtatattccgcgtggcgttagatcaacaaatattagacaatcagttattttagttttttagcggagtatgcggaaatttatccttttactatttttatctgtttatctgattacaaatgctggttatgcgcagtcctacggattacgcttttccagtcatgaagtggtgcaggaaaggagaacaacgctgaacttaacttcatccggtccgctgtgtttcaaaaagaacggggaaatatcattcgatctgaacttccttccttataaagaaacttatttcggatacgtattaaggatcatcgccgccaacaaccagaacatagacctggtatataaccagaaagaaagaacctttaacttcctcataggcgaaagcttttcacgtgcatttgccattgattcagccgccctcttcggcgggtggacgcatatcactattcacctcgacctcgggcgtaatgaagccgctatttcggtcaatgataaatttatcgccaaaggtcctgcaaagctaggcaacccggcatgtacccgcgtgttctttggcgccaatacctacgaaggttttcaaacagtggatattccacccatgaaccttcgtaatatagtggtgaaagaaggcgcccaaaccaggtacaactggccgctctccgaaaacgatggcagtaacgccaccgacctgcaggaaggtaaaactgccgagatccgcaatgccaactggataggtcccaaacaccgcaactggagcctgctccagagctgggaaattaatggtacccccagtgtggctttcgaccgggagaaagaagtgctctatattgtatcttccgattcactatataatatttcgtttaaaaatgagcagcaacacggcatccgcctggcgcaacgcctcgatagcctcatgccggggaaccagtcggtgttcaacccatttcttcataagctctttaacttttatatagaccaaaaaaaagcagggtcttatgattccctcaaccggaaatgggatatcagctacacaccagacctgcttaccgtttactggcaagccaataaatttgtctcccaacaggatacttccctttatatcctctgcggatacggacaaatgcaatataaaaataccgtacagcgatatcattttgccaataagaagtgggactccgtacccaccaccggcgaaaggctcattccccggtacctcgccgccaccggcgctaccagcaatggagatactgcttatatcctgggcggctacggcagcaacagcgggaaccaggtagtaaacccccgccattactacgatctcatggccttccacgtgaaagatcactcctttcataaagtgttccagctggaagaaccgcccgtgcagttctgctttgccaacagcctggtcatcgatccaaatacccagaattattatgccctcatcttccccgacgataaatttaataccagcctgcagctcgtggaaggctcgctgaaagcaccacggttaaagccactggccaataccatcccttactcttttcatgatatcaaatcgttcgcagatctctattactgccgcgacagtaaaaagctggtcgccgtaacgctctatacttccaaagacaatatcacggaagtaaaggtgtacacgctggaattcccgcccgacgcggtagtggcagataaatccggtctcccggaatttttcgcctggtacccgctgctgctcattcccgtagtcgccgccggcctgttcttattcctgcgccgccgcagaaagatcatgccaccaccttcagttgttgtgtcgccggtaccagcaactgcaacaccgcttcctccgctgcccgtggtaatacccgaaacggttaccgatgaaacggcaccggaagaaatcatcgctgaaaaaaaaggaaacatctatttttttggtccgtttgaagtactggacaaagaagggcaggacgttaccaaattcttcacgccgctgctcaaagaattattcctgctgatagccatcaataccatccgttcaggaaaaggtatttcatccgaccggctctatgccaccctctggcgcgataagtccagcaaggaagcacagaacaaccgctccgtgaatatggtaaagctcaaagccatcctcgacaagctgggcgcctgtgccttcgtaaaagaagctgaccgctggagcctccaatactccaccgccgatatcgacatggacctggccgggttccagcaactgctgcactcgccccgtccactgcaggaacaacatgtaagggatctgttgaagatcctccatcgtggctctttcctgcccgacaccaactacacctggctggaagatatccagtccgaaatctccggcataaccctcgacatcctcacagaggccgccaaccagttcaaatcagatccggaactcctcgttgaaatcgcggaccgcatcttcctcttcgaccccgtgaatgaagaagccctccgcatgaagtgcagcagcctcgtgtcgctggggcgccattccctcgccaaaacggccttcaacaagttcgcgaaggaatatctccacatgtatggggaggagttcccgcagtcgttcacggactactcagggtagcgggattagagcggattttgtctttctcactgattacgctgattatattgatttttaggatttgatcacgttgggattttaaaggattttgggagatataagcggatattggcttctgttttcctgattattattattattattattattatcgttaaaatcaaacattatcaaatcagcgcaatcggcgttaatcaacctaatcctgcaccaagtcaatttaaaatcgccgaaggcgatctacgctaatatttccgcttatatctccccaaatccttttaaaatcccaacgtgatcaaatcctaaaaatcaataaaatcagcgtaatcagtgagaaagacaaaatccgctctaatcccgctaactttttttcgcattagtgcattattagtgctgccgttaaggcccgccgtataaattgcattgaaatgaataagacaaggttccacgactatggcactcaggccgttttattacgaaaaaaaaggatgctggtgattaaaatcatcagcattctttttccttttttaattatcggtggagtggaagggggattgcggttatttaattacggccacaacctggcgctttttattacctctccgcaaaacagcaattactaccaactcaaccccgcagcttccctgaaatatttttccaatacggaaatcgctaccaaaggcaatagtgaattatttaagaaagtaaaagacacaggtaccctccgcatttttgtattaggtgaatccactacgatcgggtatccctattttcataatggctcctttcaccgttggctgcaataccgcctcatgcattcctgcccggagaaacgcctcgaaatcattaatctttcactaacgggcgttaattcctatacagtagagggttttacaaaagaattattgccttatcagccggatgcggtacttatttataccgggcataatgagtattatggctgcctgggcaccggcagcaccgacaaaattgccggcaaccctttcctgatccacctggtgctgaagctcggggagttccggattacccagctcatggccaacgcgctccataaaatttccaggctaacaccggccagcccggatggcgccggcaaaacccgcatggaaatgatggtggcagcacaacagatccctttcggatcagcgatgtacgaaagaggcattgcccagttcacggccaacatggataataccctgcacatgctggaccaggcaaatgttccggtgttcatcagcaacctggtgtctgctgaaaaagacctgttcccatttgttagcataccacccgacagcataaagtaccagggcttcaacaccgcatacctacagggtgagggggcgatggccaatggggattccgctgcagccctgcaatatttcatggccgcggaaaacagctaccaggcgcatgccggctgcaactattacctgggactactgaccctgcacaacggcgatagcgccgctgccaaaacgtatttcgacaaagccagggacctcgatgcccttcgtttccgggcgccatccaaactgaataaagtgatgctggagctatgcagcaaatataagaacgcgcacctggtagatgccaatgcggcttttgaagctgcgagtgccggccgtattatcggtaatgggctgatcctcgaacatgtacatcctaacctgaaaggctatgcgctcctgtcggatgtgttttataataccatgaaagcacagggacttttcaagccgttgccggaaacggaaatgagctttgcccggttgcagcaaaccatgcccattacggttatcgacagcttatccggcgcttataagatcgctaatcttaaaagaagctggccgtttagtaaaacgcatgttgatgatactatgctgattgccagtgcagaagaacagcttgcttatgaagttgctttcaggaaaacatcctgggccgcggcgctgcaacagctttataatgcctacaatcaaaacggcgattttgcaaacgccgctaccattgtggcggcatgggtacaggagcatcctaccgaagcgggatactacgaggaagccggtaattactatggtaagctggatcatactgcggaagccatcttctactttaaaaaagtatttgacatgtcgccttcctttgaggtggccaggacgctttttgtgctttacctgaaacaggataacgccaccggagcattgccttacctgaattatgccatcgatcataacgaacggcgcttaaacctgttgcccgtaaaagattgcctgttgcaggtcctggagctgcaaacaaaggcggcgagggagccggcaaatataggtttgcttaaccagattgcgggactgtactaccggatgggcaataaagagggcgccgtgctgtatgtagaaaaagtattgcaagtctcgccaggcaaccgggatgcactcaccatgcaaagtcaactcaaaaaagtatagccatgtggaaacggttcacccatattacgctgcagcaatgcatagaatccggccaggtggctgtggcggcgctactggcggcggccctgtatttccgtgatttcaggctggtaaccattgccttgctgctgttgctcatcacattgctggcgccccggcttttttatccgctggcggtgatctggttgggcatcggaaaagttttgggagaagtaaacatccgcattcttctgacccttgtttttatactggtggtagtacctgtgggcttatggcggaagtggcggggcaaagatactttacagctacgcgggtttaagaaggagaaaggatcggtgatggttacacgtaatcatgtatatacgaaagaagatttactgcatacattttaaaacgatcatcattttcacgtcatggaatttctgcatgaactgttctattttttaagaacccgtaaaaaattctggctgcttccgctgatcatcgtgctgttgttattggcatcgctggtagccctgaccagtgcttccgcgctggcgccttttatttatgccatattttaacggctttgaggaaaattatcctgggtatatcggcattttatcacgacagtgcagctgcgctgatcatcgatgggcgcattgttgcggccgcacaggaagaacgttttacgcgcattaagcaggatgctgctttcccggcgcaggccattaaatatgtattgtctgaagtgggtatctcctttgatgagctaacggcggtggcgttttatgacaaaccgctgctgaaatttgaacggttgctggaaacgtatcacgcttttgtaccacgtggctggcgcagctttatcactgctatgccggtgtggatgaaggagaaagtgtttatgaagaaaatgctccgccaccagttccgcacactgggagctacggtaaaagtgccattgtatttcccagaacatcatttatctcatgctgccagcgctttttacccgtcgccttttgagtcggccgccattctcaccgttgatggcgtaggggagtgggctaccactaccatttgttatggcgccggtaacgatatcaaaattttaagggaactgcgatttccgcattcacccggcttattatatgctgcattcacttatttcctcggctttaaagtaaacagcggcgaatataaattaatggggctgtcgccctacggactggctgatgccccgcaaaccattgccttccgggaaaagatcctgtcaacgttggtggatatacgaaacgatggttccatcctgctgaacatggattattttgaatttgccaccgggttgaaaatgacggctacgccactatgggaagccttatttggttttccccgccgggagccggaatcagctatcacgcaggagcacatgaacctggcgctggctattcagcaggttaccgaacaaattgtagtgacgctggcacgtacggcgaaagccattacgggcagcaatcacctggtgatggcaggcggtgtagcgcttaattgtgtggccaatcataaaataaaagctgccggtatttttgaggatatctggatacagcctgctgccggtgatgccggcggcgcattgggcgctgcatacgccgcttatcatattggtatggagcaggcccgtgttttttttccgggagatgatggcatgcagggcgcatttctcggccccgcttatggcgacgccgatatccggaagctgctggcccgctatgcagcggtggctgttcatcagccggacttcgtcgcactcacgcaggaagtgagcgcccacctggccggcggaaaagtagtgggctggtaccacgaccggatggagtttggtccccgcgcactcggcaaccggagcatcctcgccgatccacggcaggcggccatgcagcagcaactcaacacgaaaataaaattccgtgagagcttccgcccctttgcacccgcagtactggcagaagatgcgcaccactattttaatgacgccactacttctccctatatgttatttaccaccacattaaaagatgcgctgcgcacaaatacaccagcagatgccaccgcctccatttatgagcggctgcatctgcaacgctccaccatccctgcggtgacacacctcgatcattccgccaggatacaaaccgtacatcgtacgcttcatccaaagttatggcaacttattaattgttttaaagaactaacgggttgcagtgtgttgatcaatacctcttttaatataaggggagagccggtagtaaacacgccggaagatgcgtggcttgcttttatgcgaacagaaatggattacctggtaatggggaattatatttttgatcgccgccagcaaccagcgttgccgccggagttgttcaaatcctttgaaagggattaatagcttcttcttaaaaagaaaattaaaaaaaatacagcattaatatggctgttagttcattattagcgctgctgttaggccgccggcgcttacttgcattcattattctcttatcaatcgaaatatcgttcgcgttatgaaaagattactattgctgatgctcctcgcatcgggcctgctgcaggcctatgcacaaaagcagttgacaaagggtaaagtgctggatgaaaccggccaaccactacccggagcaaccgttagagtaaaaggtaccaacatctcaagccccaccaatgcacagggcgaattccagattgctaccggcgaaaccgcttccccggtactggtgatttcctatatcggctacctttcacaggaggtgacggtaaccggcggcgacttatccgtcactttaaaaacggatgccagatccctcaatgatatcgtagtagtcgggtatggcacacagaagaaaagcgacgtaaccggcgctaccagttcggtgaaagccgtggaaattgccaaacgtcctttagtaagagtagaacaggctttacagggaactacttccggcgtaacggtgcaaagcaacagtggtcagccgggtaaaggcatcagtgtaaggatccgcggcgccagttccatcaccggcagtaacgacccgttatacgtcattgatggttacattggcggcaacctggagtccatcgctcccggcgatattgaaagcatggaaatcctgaaggatgcttccgctaccgccatctacggttcccgcggatctaacggcgtggtaatggtaactaccaaaaccggtaaatcaggaaaaccccgcgtggatgcaagcgcctggataagcaaagcttctttgccaaagaaactaaacctgatgaacgcctacgaatttgcgcagcaggtaaataaaaaaggcgatgttgccggaacgggccatccgtttaccgatgcgcaactcgcagaactgcagaaaaatcccggtggcaccgactggcaggatgaactgacccgcaagccattgacacaaaactaccaggtaggcgtgtccggtggttctgaaaatgtaaagtattatttctcttacaaccacctggatcagccaggtttgctgatcaactccggctataaaagaaatacgctgcgcgcgaatgtggatgtgaagctgaacagcaaaatggacctgaaagtaaatattacaggtttgttgccggaatcacacaacacggatttctccggtgatatcgttgatccgttctcgcagtccagtatgtgggatcctaccagcccggtaagaaatgcagctggtgattatatcagccagtctaatttcgcatccctcgctaaaaacccggtgcaaaatatcatgagccgttcggtagatggaaaaacgtctaacctgactgctaccggcgttttcacctatcgtatcatcgatcaccttacctttacttccaataacagctatgagctgcagaaccagcaaacgcaatccgtttttcctccgggaacaaacgaagcgtttaacggtaacgactatgcgaaaatggagaatagccggtacaggagctggcagaactccaacttcctgacctataacaaccgcttcaggaatcattccctcacggtcaccgcgctcgtggaacaggcttccaaaaccaatacaaacaccattgcgcaggctaataaattatctacctacagcctcggctactggaaccttggattgggtaaaacccagtcgaccagcagcggttactgggcagatgcgctcatctcttatatgggaagggtaaactatgcctttaaagataaatacctgttaaccgtttctgttcgtacagatggatcttcccacctggtagagaagtactccacattccccgcagttgcattaggatgggctgtagacaaagaagggtttatggcagattcaaaagtgataaccggtttgaaactccgcgccagctacgggcaaacgggtaaccaggcagtacctgcctattctaccattgcccagatcggtacggccctgccttactacttcgatggtactacttcaagcgtaaataccccgctgggaacaccggtagccactacgcttcagtgggaaaagaacgctacctatgatgtaggattggacatggaattctggcgtggccgcttaaccttcaccgcagatgcctataataaaaaagtatccgacctgctgtatgccaccgataaccctttttactatggcggcggaagctttcagcgtaatatcggcagcgtaaggaataccggcctggaattcagcgtaggcggtatgccggttgttggaaaagacttcaagtggaccagtaacttcaatatctccttcaacaggaacgaagtattggatctgggaggtcaggacaatatcattgtaaatggtatcggctctgcacaacaaggcgtatccatcatcaaagtaggggaaccgctcggtaccttctatggttataaatacctgggcacctggaaaaatgaagaaaaaacagaagccgctacatacggcaagaagcccggagatacaaaatatgctgacctcgatggcgatcataaactttccggcggcgatcttactacgatcggtaatggtatgcctaaatattacttcggtttcatcaatgatttctcttacaagaactggagcctgaacgttatgttccagggcacgcacggcaaccagatgtattcctttacccaggcctatacaatgggcggactgggagatgcacgcgatgccaccaacgcgcaactcctcgatatgtggacgcctgaaaaacagacagacgttcccgtctatggtaaccagaacgaaataaaaagcagccgttatgtatacgatgccagctatatcaaactgaaaaatatttccctcacttataccattcctgcatcactgctgagcaggatacatgcacgcagcctggatgtttacatcagcgcccagaatatctggaccatcaccaactaccctggctacgatccggaagtaaccaacgccaccaatgccattacacaaggtttggaaacaggtacgatacctaaccccaaaacctatacgattggtgtaagacttggtttataattgacatagcgtataagtaaggattctgtttttctaaaaaattactattatgaacaaaaaatatttcctccctttagcgatggcagcaatgatcggtgcatcatcctgcgtgaagctgacggaagatccaagagcaacactcactcccggcaattacttcaatacacaaaatgaactggatggcgctgtaacctctgctttcagggcgctcgccgtagatggtgcatggggtttcaccagtaaaatgaccagttacttcggctccgatgatttaacaacgcaccctgcttccaacaaagcagactcgcgggaatttgaccggctccagggtaccaccaccaactccagtatgagagccgagtgggaaggcccgtggaataccatttatcaggcaaacaacgtgattgccaattttgaaaaagtaaccgccaccaccaatgaagcgattcagcaacgcacgtatgccggcggacaggcatacttcctccggggactgtgttatttctacctcgtaagaacatttggtgcattgcctattgttaccggtccggcagatattaccgtaacaccggccagggaagaacctgcaaaagtatacgaactgatcatcgccgatctgaaaaaggcggctgacatgctgcccgataaatggaccggcgcagacgtaggcagacccggcgcattgtccgcaagagccgtgctggcaaacgtatacctcaccatggcaggctggcccgttaaccaaaattccaattacgcgctggctgccacggaagcaaaagccgtaatggacgccgggaaatacgacctgatgcccgactacctcgatgtattcaaaaccaataacaatattgaatcggtattcggactgcaatataatgtaggcggccagttgcctaaccgttcctttggcgctacctgtattcctgatgatgaaggtggatgggatgatttctttccggaaatcaactacttcaaggatgcaccggtttgtaaacgtaccgatcaaacattccacacacaaatcaaaagcaataaaatcggtgtagtaaaatgggatgatccgagaacggctacccaccatccttactataacaaattccgttatggcgcaggtgatggtatcgttgaaacgcctacacaggtggtgagctttaacgccagtaccaataaaaccactgatatcgttcgctttgcagaaacattgctcacctatgcggaagcttctgccatggctgccaacaccgtttctgatgaagcctatgaagcgctgaacagggtgagacggcgcgccggtttgcccaacatcgtaaaaggtttaacggcagtggctttccgtgattcagtagtcaatgaacgcaaatatgaatttgccggggaattcggacaacgctggttcgatatcgttcgcttgcagttgctgccaaaagtaattgcgcgccgcgatccgaatgagttcaaggatctcccgttgaatcctgctgcggttgccaacccgggtcctaagtatattgctccgatcccgttcagagatctgaacctgagcccgggatggacacaaaacccgacatactaaacactttttgatttggcctataaatagtttaatcatgccttgtgcatgattaaactattttgttaattcgttctgtagccaatgaggaattctcccagcgcataaattttagtgaatgaaaaaaacaaactggaagctgtacagccttctgttgctgacaccttttgtatgcttatccggccgcgcgcatgcagcggtgtatgatactatccccggcgtaaagccatccatcgacctgattgacccaaccataggaaacgtaggtcagctgctggagcctacccggcccaccgtgcagttgccgaaccagctgatccggtttacgccgcagcggaaagactttatggatgaccagatctccgactttccattgaacgtggtatcacaccggctcgggcaggtgttttccctgaaacccgccaccggcaagctgtcggaaaatgactggcaaacccggatggcttacgaccataacctggaaaccaaccggccctggtactattctacctggctgctggatgaagaagtaaacgtggaatttactgccggtaaaaaagcaggctactaccgtttccgttttcctgccggtaaagaaaaatcgctgttgtttggtacctataacgatggtgaggctgcttacaccttcctgcccaataaggtaatgaccggcatggaaacttataacggctatgtaaaagtatacctgtacggcgttttcagtgaagccggtacacccggtgtagcagaacagggacagttgagcaacaataaaaatattgctggtaaaggaatcaaagcatttatcagtttccctgccgctataaaggaagttactttcaaatacgctatcagttacatcagcgcagaacaggcaaagaaaagttatgaagaagaaatcagtaagaaagattttgacgccgtagccgccaatggaaaaaaagcctgggcagatgtcatgaaccaggtgaaggtaaaaggtggtacgctggcgcaacaacgttctttttatacggccttataccgttgctatgaaagggccgtggatattacagaagacgggcagtattacagtggttatgataaacagatccacaaagacaaccgtcctttttatgtagatgactggacctgggacacctacctggcactgcatccgctgagaatgatcctggaccctgcaaaggaagaagacatgctgcaatcgtttgtacacatgtacgagcaaagtggctggctgcctaccttccccgtgttgtttggcgatcacgcctgcatgaacgggttccattcttccgtagtaatgctggacgcacaccggaaagggttgaaaaattttgatattgggaaagcctatgagggcatgcggaaaaatgcgacggacgctactatgcttccgtggcgcaatggtcctaaaacagcgctcgacgacgtgtatcacaacaaaggttattttcctgcattgcgcatcggcgaaaaagaaaccgagccagcggtgcatccttttgaaaaaagacaggcagtagccgttaccctaggcggcagctacgacgactgggcattgtccgagctggctggtgatttgaataagaaagatgaccagcgtttgtttgcaccaagagcgaagaattataaaaatctatggaacgccgataaacaatttttcctgccgaaagatggtaacggggaatggatcgatatcaacgtaaagtatgacggcggtattggtggtcgcgatttctacgacgaaaataacggctggacctacctctggcaggtacaacaggatatccccggcctcatcagcctgatgggtggaaaagatgcgtttgaaaaaagactggatcagttgttccgtgaaccgctggatatgtcgcgttacgctttctggagtaagttcccggatgccaccggtcttgtaggacaatactccatgggtaatgaaccaagctttcatattccgtacctgtacaactacaccggcgctccttggaaaacgcagcagcgtatccgtttcctgctcgatacctggtttaaggataacatctttggtattcccggtgatgaagacggcggcggaatgtcggccttcgtcgtattttcctccatgggcttttacccggtaacacccggtattccggaatataccattggcagccccgtgtttgaaaatataagcatcgcattgcccaacaagaaacagtttaccgtagtggcgcacaacagctccgtggtaaataaatatattcaacaggcaaagttcaacggcaaacctttgaacaaacctacgtttacacatcagcagttaactgatggcggaacgctggagctgttcatgggcccgaagcctaacaagagctggggcgtacagtaattaggcgctaagaagtttactggttttggtgaaccggtaacaatgatgaagacaaaagaaaggccgtctcttaatgaggcggtctttttttatgctgatatcttggctgtaaaccggcggcgccttattatcttcgcagctgacatggcatcttacatcgttactttgcaacttgaacggaacgccgctgcattctttaaccagatgcgccggcagtattatcctgctcatgccaacgaggtgcacgcacatcttactttattttaccgcctgccggcggatgaaccacaaatcattacttcccttgcggcgatggttgcgcggccgtcttttttattgcaggtaagtgaactgaaacggtataccaacggtattgcctatacgctcatgtccacagaactacaggcattgcatgaagccctgcaaatgcaatgggaaccctggctgattccgcgcgaccggcagccattacggccgcatatcactattatgaaccaggtaacggcttttaaagcgcagcaggcgcatgaacaattggcggccagcttccggccctttgaagtaaccgctacgggcatacaggtgtggcggtatttaaaaggcccctggaaactggcaggggaatatcctttcctcacataaaaaagccttcccgaattaccggaaaggctttcttacttcattcatcgtcttatcgttgttaaataattctattcacgtgtttgatcttaacaaccacctcgtaggttccttcctggaaaatctggaactggaaccgggggttcacgttatagattttttcgttggtaggtgcataccctggatccacggttacaaactggcttgggatacgataatagatcaggtatccgtacacactttgtaataagggaaacggcgtggtttcaaagttgcagaccatgctcgtatctgttttctccagcggatgaaactgtgcataggtctggaaatcactacggtcgcccctgcggatgatctctcccttggccgggttaaagtagcggccgttctggtcggcgatcttcaggataatattggtgccttcatcggagatcttccggatggtaacggtgggcacgcccaggtcgccactggtagtggtaccgtctttaaaccaggcagcgccgccgtcgcccacatgataaggcggctcgtctatcagcgtgaaggtggcaatgtttttatactgtttgctgccgttctgattggaggcctctatatcaaattcgtaggtgcccagcggtactttgatggaagtgccgtaaaaagtaaaggcgccggtatgctcgttgaattcaaagcagggggtgtttactttttgtctttttttattcagtaattctaccgtggtatctttttccggatcaaatttcccgatccactcatagcgctcataattagtgaacacggagtcggcatgggtgtgtttcaccgcatcgcggatatccaggagcttgtacactaccggtgcgctggaaccatcgttgctcacggggttggtggattgtacctggccgcgttttattttaatcggattatcgatgtagcgtatctggttgctgagaaaaccgttttccacttttgagcaaccgtacatagctgccgaaacagccatcaccagggcgccgaatatttttatatttcttttcatgatcattgcgtaagggtgaaaactcagttaaacgtatccgcgaaataggtgaatgtgtgtttgttattcagcacatgcagtattccgttggtagtaagtataccggtagtctgacagcgtgcttgcaggtattgctctggtatggtattagccaggtcggcatctgttacgggaacaggatggccgggttttgcaatcagcttggtcaggtagaggtataccgggtattgcgtgaatacgcttccgtcggtataatccccgctgggaatgccctgtaccaggcgcagttccccgtcgtttgccctgtatagctttcctgttttggtagctttgtctaaaggaatcaggtctttgaaaagataagcccgtaaagaatctctcattgctccaaaatccagggagtcgaaagtaaagatatagttaggatctgttctctgcgtgcgttccatttcctgccgtaaatccaggtagttggtgatatcatagtcagtgatggcaaagaaggttccggtagcatttacttcttccttcaaacctgttttatcgatcatcaacacaacggtatcaaaaagcggatttgttttcaggtaatcataagtagtcatgtttacatgcggatcatgcaaactgccgccgatcgtgtaatccttcttacaggaaaataaaaccacggccatcaaagcgatgaaagagagatatattttatgtttcatacagctgattttaatgggttagagtttacctctccagtaaggagtttgagtaagggtgaaatcgtctttaaacattgttggatcaatgggccataaccagccgccgttttcaaactgatcgcctgggaaatgctcattgtacgtagtcagttttttattacgcaccaggtcgtaataagcgtggccttcgtagaagagctcccggaggcgttcttcgaggatggtagtggcgaggtcttcaccagcgccggcataatcgtccagtcctgcacgttcgcgtaccctgttaagcaggggcagtgcatcgccatccttacccagtttactcagcgcctcagccctcagcagcaggatatccgccagccggaagatggtgaggttgttggtcatgcggggatcttttttggtagaaccatccgcataagcaatattggaaaacttgatgatctgtccctggttaccgccaagtccgtagaagaagtttttgaaacggatatctttatcggcatcataaattgacaggtagttttcattcaccggccattcgatatatccttttccatcgataaacggcatcatcagcgtaacgcctgcaccgccattggtggccagggaaattccttctgactgtccgtcgttgatattgatctcaaaaataccttcctgtgttttaccgataaatactttcatgtaattggcagaatcgatcagcgcataaccaccgttggtgattacttcattcgctgctgcttcacagccggcgtaatcgcctttccatgccaggatatgtgcctgcagggcaaatgcagcgcctttattggctcttaccgcccgttcagattcatcttcataaccaaaatccaggttttgtttagccacttccaggtcggccaggcattgtttccaaacactgtcggccgggcttctcgggatattcttcgcggtagacacatccaggtccggttccagtttcaatggcacatctccccagatcctgctcatatagaagtaggtaaaggcgcgaaggaagtaagcttcgccgatcacgtgccgtttgttattgatatccgtgaatttgctgtcgtcgatacccggtactttattgatgatcaggtttacctgttggagcagctggtagtactgctgccagttccagttgttgccacccacgttcaggccaacaaactgaccattcgaaatattgtagttgccgttatcccggccgccgtcgatactcagttcgccggatacaatgtccccgtatttatgccaggaattatcacggatcaggatattacgcaggatggcataagctccggcgagcgatgttttggcatctgtttccgtagaaaaataagcgctggtaaaagtggagttatgcggttccaggtccagtattttggagcaggacgacaccagggaagctgcagaaataacagcagctgcataagcgatatataagcgttgttttttcatgattttcttttttatggttaaaggctaagatccagtcccagggtgaactttctgggaatgggataaccactgccgctatatactccaaaggcatccacctgctcagggtcagggatatttttagattgtttgaagatataaaggttgtcggccagcgcatagatccttaaacgtctgaagtgaattttatccagtatttcctgcttgaaagagtaggagagggatacgtttttcacacggaagtaggcgccgctttcgatccaggcagaacttaccatggcgtatttgtagtgggtaccgtttacggaactgagacttggatagtccgccttatcgcccggatttctccagtagttgatgttgctcaggtcgggcatggaatgggtggacagggagtgatagggatcgggatcgccatcatccgtaggtaccagctgggaaagctttccggcgaggtagtcgttgaatactttacggcccgccgtgaaagtacagaacacatacagcgtgaaattcttgtagctgaaggtattaccaaaaccgccggttactttagggttggggttaccagccgggatgtaatcggtgttatcgaggataccgtcgccgttggagtcctgccagatcgggtcgccacctctgaatggataaccgtagaaactgagcggtaatccgctggctttatttaccggtacatctgcatcggtaaagtagatgcctgttttgttaaatacattgtaagagttcagtggttgtccctggcggagcaggtatttatcgagataaatatcacggccgccgttcggcagggaggtaatcaggttgtcgttatgcgcgaggtttaacaacgcctgccactggaattttgaagatggcttcaggatattggcaatgaactgtacttccacaccggtgttgcgtatgccgatggcgttggcggtgaggatggagtaaccggtggttacaggtacattcaggttaaagataccgccgttggtatttttaatgtaagcatctgcaacaacattaaacctgccgttatataaggttatatccaaacccaggttactttgtgtactcttttcccagctcaggttattgttggtaagacctttgtcgaagtcgagcgatacggccggaataccgttataggcaaagccatagttgtttcctgtagcaggattggtactgccggggaaatcacctgcaccgatacggtaagtattataagagaggtagttgtcgccaccatccggttgacggccggcaacgccataactggcgcgtaatttcaacaggcttagccagctgctggcagattttagtgccggttcgtcgctgattacccagccaccagatacggaagggaaataaccccagcggttatttttaccaaaacgggaggaggcatctgcggtgattacagcggataacaggtaacgttctttatagccgtagttggctctcaggaaaagcgactggataccgctctgtaacaggtcggagcgggtatcggccaggtttttattgagcacggtaacggtacggatctggtcattcggtatgccgatggcgctggactgtgtagcccggtattcccagtactctgtattctgacccgccaggaagttgaacgagtgattggtgttcagcgtggtggtatactggagcgtattgctcattaagtagttgttcgatttatcaacaaagctggtcgccttaccggttccgtctctccttacagcaccaggggtataagagtccatccggctgttggtttgcgtaaaggagatcaccgtggtgaagttaaatttactggagatcttccactcgatgatcgggctgatagacaggttatcattactgttctgatctgtgccgctggtggtattaccgaaaatgaagtctttgttggcattgctcatatacagcagcgaggtaggtaatgcgttggatgcatagtacccgccgttgaaaggaccgtagccgccggagagatcattgatggatcttgggcggtctattttcgagtaacggatctgtgtattgatctgtacattgggagagaggttcaagccggtgctgctgctgaagctgtaacgctttaagcctgatttccggatgataccatcttcgctgtagtagttgaggccgtagcggtagttgatcaggttattaccaccggaaatggaaaggtcgtagttgtcgacccggccggtttgatacataccaccctggtaatcgttggcgttattgaaggccggattcaggctgtcggtcagcacctgcgggatatttctcagggtgccccagtcgccgtaatggttgatcaggtccattttagcccggcgttcttccgcgcctatcagtactttatccagttgcggcatttcagtgaaaccatgataggtagcgaaatcaattttgggtttaccggagatccctctttttgttttgatgatgatgacaccgcctgcgcctcttgatccgtagatcgcggcagcagaggcatctttcaggatatcgatgctttgaatatcgttgatggaaataccggccattacgtcggtgttggtaccggagccgtaattgatggcggcaatgtcttccgtggtttgcggtacgccgtcgataacgtaaaggggcccgctcaatgcgcgggccaaactggctttcccggaattgctggtaaagtcgctgttgatgttgcggcttacggcggtattaccacgcattaccacgttgctccttacgccgggttcaccggaatagttctgcacatccaggccgggtgcgcgtccctgcagcaaggcgtcgaaagtaggggtgggcacatccagtaatgtttttggattaatggaagtaacggcggcggtaactgttttacgggaggtttcctggtacccgataaccaccacatctttcaacatttttttgtctaccggtaaagttacgttcagatgcgcattagcttcctttaccattaccgagtaaggaagatagcccatcatgctgaaggtaagcgtactgccagggttcattttgagtgtgtagccaccatccgtgttggtgatagcgcctgctttgctgtctgaaatgcttacagatacgcccggcaacgggttgccgtctgaaccatcctttactgtgcctgatacggtgatctgtgtggaggcagattttacctgtgcggtacctctcaggcataggaaggtgaggcagaacgttaataacataacagcgccgttacggctgttttgtgtaaaattaacagtcatgtaaattgatttgaaactgatgaatgatactggaatgctgattacccagttgttattatgatattggttgacgtattatacccggaataaatgatgtaaaacgtattctctgttgttgactaattttgatttgacaaataccatcgtcgcttccgatgacaaaattttggtctgataaactcctttttttgttactaatttgaattttggtctgataaattcttatattgctaaatcgattttctgattaaatcacaggtctcagaatgtgaggatgaaattagtatgaacaggaaaaataacttgttaatgaaatttaaaagattgtaaacaatcttaaaaagaagcaggtctggccgcggtctgtatctccctgcaggtaaacaaaaacagtgaatttcctcttcccgtttccggggtatagatatataatttaaaaatattatatttatggttgtaataaactatctaacccgaaattatacctatgaaacaacgctacttatttgtcggcatcctgctgaccattttcagtatccacagcttcgcccaggaggcagtcaacccgggaagcagggccaaggcagctgccgtatttaccaaaatcctcaacgacgccgctgccatatatccgccggagttatcttatctcacggaggcgggtgcgaaaatcgagtcttctttccgcgtgagcgaagatggtatcctgtcggtaactttccgttacccggtggaaaccagttatagcctttaccgccttagtgcgccggtgagctccattaaaggtgtgttttatgattattatatcgggctggaatttgacggcccggttgtacacatagcggagagcgacaaaggcagccgggagctgaaggaaaacaatacactggcgctttttcacatcgccaaacccggcgacgggccacccggcgaaaagctgaaagtcaggatagaacaggcattacaggcgttccgggagaattacaagtaaatggttcctcagaaag

SEQ ID NO: 15 - DNA, 188935 bp, Chitinophaga pinensis
  source 1..188935: mol_type = genomic DNA
ttgctaaagcaagctgacattaactatttattctcttaaaaaacacctgatcatcataatgattattaggccatcttttggctaaaacaaagaagctgtctcaattaattatgagacagcttcttttcttccataaatatgatctgttattacttgatttctcctaccatgtttgcgggtactacccattcatcaaattcagccggggttacataacccagtttcacggccatttctttaagggtagttccttccttgtgggctttctgcgcaatttcggctgctttgtagtagccaattttggtgttcagtgccgttaccagcatcagggaattttccacatgttttttgatattggcttcaataggttcgatgccttctgcgcatttatcgttgaagcttacgcagccgtcgccgataaggcgtgcagagtgcaggaagttgaagatcattaccggcttaaatacgttcagttcaaagtgtccgttggaaccgccgatactgatagtaacatcgttacccattacctgggcagcaatcatggtgagggcttcgcactgggttggattcactttgcccggcatgatagacgatcccggttcattgtcgggaatatgaatttcgccgatacccgcgcgtgggccggagctcagcatgcgtatgtcgttggctatcttcattaaacttaccgccactgttttcagcgcaccatgtgcttctacgatggcatcgtgtgctgcgagggcttcaaatttattttctgctgtaataaaaggcaacccggttaacagggcgatattctttgccacattttcagaatagccttttggcgtattgatgccggtgcctactgcagtgccacccaatgccagctcgctcaggtgagccagtgaattgttgatggctttcaggccgtgattcagctgggctacatagccgctgatttcctgcccgagagtaagcggggtggcatccataaaatgggtacggccaattttcactacgtttttaaacgcttctgcctttttcgccagcgtgtcgcggagctttgtgatgccgggaatggtaacttcctgcagcattttgtaagcagcgatgtgcatagcagtagggaaggtgtcgttggaagactgtgacttgttcacatcatcgttgggatgaacaaatttgtctttatcagtaagctgaccgccatgaattacgtgggcgcggtaagccaccacttcgtttacgttcatgttagactgggtaccggagcctgtttgccatactaccagcggaaactgatcgtccagtttaccttccaggatttcatcgcaaacctggccaatcagatcacttttttctttgggcagtacgcctgcttcgaggttagtgatagctgccgctttcttcaggtaagcgaatgccttgataatttccttcggcattttgttgatatcctgcgcgatcttgaaattttcaatggagcgctgtgtttgagcgccataataggcatttacaggcactttaacctcgcccattgtgtctttctctattctgaattccatgacttaaacttttaaggctacaaaagtacggctttacgggttgggctgcaagctattccccggtaaaattcgcctgtcttttctgaataaaggcggcagcgccttcctgcagatcttttgtagcgaagcaggccccgaactccttcagttccagctcaaagccgtccatgtccttatccagtgcggcattagcgcatttaatcacgcgggctactgccagcggcgcttttgtttgtattttttgtaagatggatttcgctttgggcagcaattcttcgagctttaaaacatggttcaccaatccccaggcctgtgcttctgtggcattgatcatgtccccggtgagcatcagttccagggctttcccctttcctatgagctgcgtaagacgctgtgtaccgccataacccggaatgagcccgaggtttacttccggctggccaaactttgcgttgtcgctggcaatccggaaatggcaggccatcgccagttcacagcccccgcccagtgcaaagccgtttacggcggcaatgatgggcttagggctgctttctatacgctggaaaattacgtgccctttcttggccagttcttctccttgtttatctgataaagtaagaaactcgctgatatctgcacctgccacaaaagctttttcacctgcaccggtaataatggcgcccttgatttcccggttgctgtatatttcatctaccgccaatgccaggtcggccagcacctgctggttgagggcattcagcttttccgggcggttgatcgtaatcgtgaggatattgttttccaattgtgtgcttaacgtctgatacatgtgccgtattttagtttatcaatattaagcaatattcaataacctaacgaatcagcccgatagccgcctcccctcattttggtgataaccgctatcgacaaaaaaaaccggaaccaattttacaattagttccggtttgctaaaaatagcggatatatttcttaatagttcacttcaaactctgctttgccatttttcatcttcatatagtgtcttttcttctttactttaaaataatcgataccgctgaagttataattgagcgtaacgaacatcatatttgcttctaagtttttatacggataaacggaattaccgtctttatcttttgttttaaagtctttattaaagaaattctgcgggtagtattgcactttcagtccgaagccggggttaatgcggaacccggcaaaaaaggagggcatcagcagcggtgtacggtcgctgaaccattcattgaacttatggactttatcgccatctacaaattgtttctctttataattaacggccaggtctatttctccaccggcaaaaaagaagaagctgccggaagtcacatcacctatctttatccccagcggaacaccaagggtatacacccgctgtttaagcttcagagagtcggtaggtttggagatcagaccaatatttttgatattgatgcccgtaaaaactccaaagtttttagagaaatctttattaaagttagagccaacattaagaaagagggtaaaccgggggatattgcgcagatgctccccgttttctttcatagaagcaaaggacagcagggggccgtcgccaccgtgggttacgtataccccttcccggtgtttgggatattttccgaaaatgatggaaaaaacggttttcccggtagtagtatcgggggcagcagcattggctgaatcttttttctcctgggcaaatacattacaacacaacatcaacagtaacaggaataacgggcacaacttacatttcataaaaacgggtgttatggtttttagatatttggtggactatttccattaaagacgacccggtttagaaaatgttacggcaacagggaaatatttttaaaaatccctatgactggccacccagctggtgatatactcggaaatatctttggtgttggtgccgggagggaacagttttcctactcccatttcctgcagtgtttccatatcggcatcggggataatgccgccaccggtcagcagtacgtcgttcatacccttttccttcatctgggcaatgatcttggggaatacggtcatatgggcgccggagaggatactgataccaatagcatccacgtcttcctgcagggctgcattcaccaccatttccggggtttggcgtaaaccggtatatattacctccattccggcatcccgcagtgctgccgcaattacttttgcgcccctgtcgtggccatccaggcccactttagctaccaatacacgaacaggacgatttaacgggttgaccataccattatcatattaaggaagtaaatgtacgaaaaagcagaaagcttaagctctcggcttttttgtacatttgccgtccaagataaaatcattatgagcgaagaaagatccctcaactttatagaacaaattgttgaagaagacatagcgaacggcgttaacgacggaagggtactgacccgttttccgccagaacctaatggctacctgcatataggtcatgccaaatccatagtgctgaactttggactggcccagaaatacaatggaaaaaccaatctccgctttgatgataccaacccggtaacagaagatactgaatacgtggattccattaaagaggatatccgctggctgggatttgagtgggaaaaggaattgtatgcctctgactattttgaacagctttacgcatttgccgtaaaaatgatagaaaaaggactggcctatgtagaagatgccagcgccgatgaaattgccgcagccaaaggtacccccaccgtacccggtacgcccacgccggccagaagccgctctgcagcggaaaacctggacctgtttgagcggatgcgcaaaggcgaattcaaagacggggaaaaaacactccgcgccaaaggagacctggcttcccccaatatgcacatgcgcgacccgctcatgtatcgcattaaacatgcccatcaccaccgtaccggcgacaaatggtgcatctacccgatgtatgattttgcgcacggacagagcgatagcatcgaacatattacccattccatctgtacgctggagttcatcccgcaccgcccgctgtacgactggttcatcaaagaactggagatcttccctagccgccagtacgagtttgcgcgtttaaacctcacctatacggtgatgagtaaacgaaaactgaaacaactggtggaagaaggtcatgtaagcggatgggacgatccccgcatgcctaccatcagtggtctgcgccgtcgcggctacaccgccgccagcatccgccagctctgcgaacgcgtaggtgtacagaaacgtgacaacatgattgaactcagcctgctggaattctgtatccgcgaagagctgaacagaaccgccaaccgcgtaatggcagtgctggacccggtaaagctggtgatcaccaattacccggaaggacaggtagaagaaatggctgccgataataacccggaagatgaaaacgctggctcccgcaccctgcctttcagcaataccctgtacattgagcgggaagacttcatggaggcgcctcctaaaaagttcttccggctcggtcccggcctgatggtacggctgaaaaatgcctatatcatcaaaggcgaaagctttgagaaagatgccgatggcaatatcactaccatttacgccacgtacctgcccgaaagcaaaagtggcggcgaccagagcggcttaaccgttaaaggtaccattcactgggtaagcgcagcacatgccgctaccgctgaagtgcggatctacgaccgcctgtttaccgcggaaaatccgcaggcagaggaagccgacttcaaaacgctcatcaacccggattcgctgcacatcatcaaacaggcgtatgtggaaccaggactgctgcaggctgccccgggtgaacgattccagttcctgcgcaaaggctactttgtggtggataaagacagcacgccggaaaaaatagtgttcaaccggaccgtaacactgaaagatgcctgggcaaaagaaagcgccaaagggaaataaatatttttttaaaaaaagtgaaggccgggcagttactgtccggcctttttatgtgtataattatatgtatttttatttacagtaaatcactttatatggctaaaaccaatatagacttagacgataagctgatcaaagaagcgatgaagcttaacaagggtaaaaccaaagaggaagttataaacgaggcgctgaggaagtatattttaggtatgaatcagcgtaaatttttagacctgaagggaaagattgaatgggaaggagatttaaacgaaatgcgaggtaaataatgcgaccactactcttcgacacatccgtttggattgatgctttacggcggaaggaaacaccacaaaccaacctgttaactcattacatcgataatgattttgaaattccgcttattcccattgttgttcaggagtgcctgcaaggaataagagatgataaccagcatcagaaagtaaaggaaacattccgccgttttacaagactggaaatagcgcctatggcagccgctatgggcgcctcctccttattccgttcactccgcaaaaaaggtattactattcgcaaaagcaacgattgcgtaattgctttttatgccatgagctttgacctggaagtggtgcacaacgacagcgactttgagctgatcagcacgcactcggaattaaaaacatggaaaaataactaaggctaagcgactcacgtcgcttagccttcatttatttgaaactactaacaattctacttaaacgctgccagtccctttgcaatcctgttacgggtttccgctacaccgagcgtggccacgatatcaaatacaggagggccgaatttaccgccggtcagcataatgcggaacggcagttgtacatctcccattttaagattcttttcagcagccagcgctttgaaggcagtttccaaatcggctgcagcagctgcagataacgattccagctgttcagaccaggtatggaaaaatgcttctttatctgcattccattttggttttacagcagcttcatcatggctgtcagggttttggaagaagaaaaatccgtgatcccatatttcattcacaaaatagcagcgctcctttaccaggccagcaacggtagccacataagcaggatcggcggtaacacctttttcatccagcaccggctggaacaaggctgccaggctttcattgtctttgtggtgaatatactggtggttaaaccatttggctttttcaaaatcgaatttagcacccgccttatgcacgcgctccagggagaacttttggatcaactcctccagggagaaaatttcctgttcggtaccatcattccagcccagcatcaccagcatattaataaatgcttccggcaggaaaccgcgttcacggaagcctttcgttacttctttgctcacggggtcagtccagttcatggcgtatacggggaagcctaaacgatcgccgtcacgtttgctcagtttaccattgccatccggtttcaggatcagtggaagatgcgcccattgcggcatatccgcttcccaacccaggaatttccaaagcaggagatgtaccggcgccgaaggaagccattcttctccgcggaaggcatgggttattttcatgagataatcgtccaccaccacagcaaggtgataggtaggcataccatctgctttcagcaaaactttatcatctacctgcgaagtatggaaggtaacttctccgcgaaccaggtctgtaaaagtaacttcttcattggcaggcatatttatacggataacatgtggcgtatccttcgccagcaggtcctgtacttcagcatcggagagcgtaagggaattacgcattttggcccttacaatatggttgtattgcggagaaggattctccggcgttttcaggcgctcacgcatactttccagttcttcgggggtatcgaaggcgtagtatgcatggccggcttttaccagctgttccgcatattgacggtataagtgcttgcgctcactctgacggtaaggagcaaacggtccgcctgcttccgggctttcatcaggaataaggccacaccaacgcaaacattcattgatatactcttccgcgccgggaacgtaacgggtttggtctgtgtcttctatacgcagcacaaaatcgccgttatgctgcttcgcaaacaaatagttgaacaatacagtgcgtacacctccaagatgtaagccaccagtaggactgggcgcaaaacgcactcttacttttttgtgatccataggccgcaaagataaggatttagcttttaggtggaagttattgccagggagataattgggagattaaaattttttaatacgaagccctgctaacagacattaagtatattgcaatactaaagctcatcgctaaaaagccaaaggctatatgttctatcttactaaaactcccggcatcctgaaagccttatacaaaagctgtgtctggaatctgtccccggcagggaataaggtatatcttacttttgatgatggtccgcatccgcaggcaacgccctttgtgctcgagcaactggcaaagttcaatgccaaagctacttttttctgtataggaaaaaatgtactggagcatcccgctatctatcagcagatactggaagcagggcatactaccggcaatcatacccaaaaccatttgaacggatggaaaaccaataccggaaaatatattgagaatgtgctggaagcagcaaaatatattgcctccccattgttcagacctccctatggcaggatcactcccttccagatccgtcagatcaggaataagataccgggcgctaaaattattatgtgggacattctcagcggcgattttgatacgcaaatcaacggggaagcctgtgtgcagaatgtagtattcaagttgcagccgggatctattgtggtttttcacgacagcgccaaagcctgggaccggctggagtatgcgctgccacgggtactggagtattgcaggaagcaaaaatttgaagtagccgctatactataataactgttgctgataaactcatttatcagcaacagttaagaggttttataatttaatctctttggttttatctcccacagtaatcgtaatgggatcggtacatttaccattaccataatcaattaccccggttactttatcaaattcaaccttcagttttcctttaacgaagtgctggcagtcaaatattttcaccagtgcctcctgtgttgtaaaagtgcccgtaacaccaattacaggtcctttttcataagaaatgctggctgttccctctacggtaaacacatcatcagaaggatttaacaacggtgttaccgggtcaaaacctgctgtttgcttaatggttttcttactggcgtagttgattacaatggtatcgctgagcgttacttttccgttagttaactcggtggtatactggataccggttgttgcgctgtagctcacgccactgatggtaaagcggccttctactgattttccattgagtttataaccaaccggctccaccaggatgattgaagcaggattaaataacggaccgctgaaagtaacattcaatatgccgctgcggaatacgccatacctgtcgaggcatgatgtgccaaaattgatcactacttttttcggccatttatcagggctcgtaacatcctgcagttctgctaccgggcagccagtggaggctgtattggccagcgcattgtttacgttatctgccttgcgggcggtaaacaaaccctgcgtaatagctacttccgccactgtttcaaacagtccgctgtacatagcactggcagccgcctcgtgttgcgaagcagcaatggtattgttatctgattgattattcggtgcggtatctgtggttacttccttcttacaggcaaagaaaatggtgactaccgccacgctggtgaaggtccacgccagcacacgattggtactgaaatagcttttcatagtttaggttttattagcaattaggtttttcggtctttacctttacagaaataaagataccgtttaaatattaaagaaattacaaatttaataaaataattattatgctttggatagatacccacacgcacctttattctgaagaatttgaggccgaccgggacgaaatggtagcgcgggccatagcagcgggggtagataaactgttgttgccgaatatagacgagagttccattgaagggatgctggcgctggaagccaggtatcccggtcatatttatgccatgatgggaatacacccctgttatgtaaaggaggccgtagatgagcagctggacctggtaagagcctggttacagcagcggcctttccgggcgatcggggaaataggactggatttttactgggataaatccctgctcattcagcaatacaaggctttccaggagcaactgatgctggcgcgggagtatgggttgcccgtatccattcacagccgggaagctacacgggaatgtatcaacgaagtaaaggcattgcaggatggccgtttaagcggtgtttttcactgtttttcaggcaccctggaagaagctaaggaaatcattgacctgggcttttacctgggcataggcggggtagttaccttcaagaagtccggtttggataagctgctgggagaaatagacctggcgcatatcgtgatggaaacagatgcaccctatctggcgccggttccttatcgcggtaaacgcaatgaaagtgcttacctcccgctggcaggtgaaaaggtggcagatataaaaaatctaaaaatagcagacgttgcagctataacaagcagcaatgcccggaaattattcaaaatgctctaactgtttagtgaatacctttgcaggcaatggctactagcacaatgagtaaaattctgataatttacacgggcggtactgtaggtatgatctacgacgataaaaccaaagcactgcgcccgatcggcttcaatgaaataaggaataatttaccggaactataccggatgggcatcgatttttatgtgtacgcatttaatccgcctattgattcatcagacatgcagccggagatatgggtggaactggccagtataattgaagaccggtacgaccggtacgatggttttgtaattctgcacggatccgatacaatggccttcacggcgtccgccctgagcttcatgctggaaaacctgtcgaagcccgttatcttaaccggctcccagcttcccatcgggaaaatacgtacagatgccaaagagaacatcattacagcgatggaaatagcctgcagcaggcataatggcactgccatctctatggtacctgaagtatgtatttactttgacttctccctgttcagaggcaaccgttcaaaaaaatataatgcggaaaaatttgaggccttctataccatgaactatcctcagcttgcggaagccggcattgatattaaattcaagcatcagtttattttaccgccgcctacacaaccactgaaggtgcataaggaactggaaacaaatatcaccgtactgaaattattcccgggcattaccaggagagctgtagaagccacactgggtgtatccggtttgaaaggtgtgatcatggaaacctttggcagtggcaacaccaacacacagccctggtttattgagagcataaaaaaagtgattgatcatggcgccattgtagtagacattacccagtgtgatggcggctctgtggagttaggcaaatatgaaaccagtcagcatttagtggaaattggtgtagtgagcgggcatgatatgacctttgaagcagcagtcaccaaactgatgttcgtattgggtcagggcctctctgtagaagatgcaaagacaatgctggaaacatccctgcggggcgaactaacgccaatcgaagtatactaaatacctttttaacggaagcttatacaagcgggagatacattcagttgtactttcgcttttttttattttgaatatttaaggtaattttaaacatcaccaaattctcttcccctattttctattcaccacaaaattcattattctatgggagtttccttatcacagaaatgcattgctgaattcttcggcacttttgtcctggtatttatgggttgcggcagtgccgtgttagccggtacgcacgtagggtttctaggtatcgcttttgcatttggtttatcagtagtaaccatggcgtacgctgtaggccacatctccggatgtcatttgaatccggctattactatttccctgtggtctacaggcaaaatatccggcaaagatgcgggcggatatattgtagcacagatcatcggaggtattgttgctgctgcactcctgtattttattgcacagggaaaagcagattacagtcttgctgctaatggccttggcgccaatggtgtggaagatggctcaccagaccattattcactgatcagtggattgattgctgaaatcgttcttaccgccattttcctggtggtagttcatggcagcaccagtaaaaacaacggcaacagcgcatttgccggactggcaataggtctctgccttaccatgatccatattgtaggcatcccggttacaggggtatctgtgaaccccgcaaggagcatcggaccggctctgtttgttggtggcgccgccctttcccatttgtgggtgttcctcgtaggacccattgtaggcgggcttttaggcggaggaatatggaagctgtacgataagaattaaacttttttttgaaatataaactaaaggattatctttgcaaccctgaattggaaaatcaacccttcctttgtattcaggcaaagataatcacggagaagtgcaggagtggttgaactggcacgcctggaaagtgtgtataggtgaaagcctatcaagggttcgaatcccttcttctccgcaagctttaaagctctggtaacgcaagttatcagggcttttttgttttgcttatctacttaaaaatagtgctgtaatttcgtgtgggatatttcattttttctaaaatggaaagtatctttagacttccacaataagatattcctttatttgaagaaaaagtataattagtcattgttttaacgagagttgtgaacccataatccatacaatctattatttgtcaaaattttcaacccttatatttaaattctcaaacacattttatctatgaaaaaaaaatggcttatagcgttatcgctaagtgtactgttttatgcctgtagcaaagacaacaccaatgaaagaccagacacccgtcaggtacaaattccattcaaagtaagcgttgctgagtttataaaaaaagtgcagcagctacccagcgcttccggcagaatggctccttcgtcaatttttgcaaaagattcaacgcttaatacagcggtttctgatatttacttttttgcctttaaaaataatggagacagaattagttatatacatcaaagatccaccgatgctgattttggcgttatttcagattcattaccaagtggagaatgtacaatagccctgattgcttccagtgattctctgataataagtgatgaattacgtaacgctggtataaatcttaatgcagattataacaacaatactatattagctgcgttcccggatatcttttacaaaaagatgcaaattacagttggacccgacactaccgcaaacaacttcagtttatctctggaacgcatcatggcttctttggaagtaaatattacagatgctcctgctattagagctgattcaaatataaccgtcaacgtaagatctgaaaacacctattttgagattttttcggcctgggcatatacagggattcctatgcaactgaaaattccccaaagaactcagcatttatttagcgaactgattatgaatacaagtgaagaaatcaggatagatatcaattatccagacaaagtaacaaatacgatgttaactaaaacaattggtcctattacacttactaaaaatacaaaaacaatactgactggtagtttatatcccgcaataccaccggtaactaatgtcaatagtggattcagtgttagtattaatagtatatggaatccagctcagacaattgatttttaatctgtttactacaactattcagtgcaaaatcttctgaacaagctttaaagcgctggtagcttaagttgccagcgttttaaggcttttatcccaaaaagtttttcgtcgaaacaaacctgttgtcttgcagctacgaactaacttcggcaatcaagcccggctagcttcatccctcatagttctcacgccatcatccgcgacaaaataacccggtccacataaaacgttccgaaaggaataatacacgccagtaaaactttccaggtagttgtactgaatttccacttataggcaattcctacactcagggtattcaggataaagaacaggaataatattccgtgcacggggcctattgcctttaccagggaggcatcatgatatacatacttcagcggtactgccactccaatcagtatcagcagggaaatcccttctaaaaaggcgatcagccgcaatcttccgatttttgtattaaagaacttcagcatagttaaaatggtcttatatatggccggttcgccagcggtgagaacggccacggtattgcaatgaaaataataataagcgcgagggaaaaccaaatggtcatagtacggaacctgccagcatcggtattttgccgtttggctaccgatgaaccaatggttataaaaacgatggcgatggtcatcagcacaatatgtattaacccgaaaaacaggaaatcaaattgccggatggcttcatggaaatgagacctgaaataagccaccacagggctcttgaagtacaggatgtaaccaatcgccagctggatatgtgcaatggtggcggtaccatgtcttaccagatcatcctgccgggtaaatacttctttgcggctccatccgcgtatgccacggtatacagcgtataaaaggcttagtactactgcccagcggaataatgaatgtatgaataacaaaaagaaatacatgcccgcaaagctctgacgaaaagcaacgggctgttaggacaaataagggttgttttaggacaattcaatcttcctgcggaaatcagtaggggtaataccttcatactttttaaagagccgggtgaagtacgactgatccccgaaacccacttcccccgctacttcgctgatggtgagatcactttgacttaacaatacttttgcttccagcacgatggcctcgtcgatccaccgcgcaggtgatttaccggtaaccgctttcactgatttgtttaaatgattgggggaaatattcagcagggatgcataatccgttaccaggtgccgcgaccggacattggtaaataccagctccttaaaacgattggtggtattgacggctgccgtttgatgactgcccgtcagcggcttgtaaagcagctttacttcgcatagtaatgtgatcaggtatggctggataatttccaggtgctgcagcccgttccggctgtaatcaaataacaggcgtttgaaaagatgtaccacaaaccccgcggtttgcctgtcgagactgatccttggattgccccatacccttaaaaaatcaaatgctctcagcggctcttgtgtattgtatttgccggtaaggatatcagtatggaaattacacagatatcccttgttcacttccccgcttttaaaggaaaaaacctgtcccgccggtacaaacaacatttcatttttgtggatggtatacaattcactgccaatttttatacttgcttctccactggtaataaacaggcagctatggttggtagacctggaagccggtactgactgcgttaccagccggtacatctcttccactttcactataaaaaacttatcaaaatcgggtcttaagatgttatcaagctccttcttaggttgcataaacctggcagtaaatgaaccaggaccatatacccttattccctttctcgctggcatgatcaattttcttttaccctgaaggtaaaaaattatgcgcttcccggcaggcccatattatgcgggcctggcgagggagtaacacaacagccccgtcagatcatcttccttttccagttcttctctcaatgcgtgatcgatttcaaagtgatgacgttcgaggagcttaatggatttttcatttttgtcagcggggagagctgcaattttttgaagatgcaattgctcaaatccaaactttatgaccaccggtatcacttcctgcataatgccttttccaaagaaggcagagcgaagctcgtagccaatttcagcccggccggattcaggtactatgttccagcaacagatagtaccaacgagttggtcgctttctttgtcgataattatccagtacaacgatttgtgggctgcaatgcctgcctgaagcttttcaataaattgccgggcctctgctactgtagtggtggcagcccggttcaggaactggttcacacgcgggtccgacctgagagcagcaatggcttcatcatcactcaaggcaggagccctcaaaataaatcgttcggaaacgagcgtcggaaaggggttaaaattaagtaccagcatacagttaaaataatcattattcagttgctatacttatcaacaggcatatctttttaaatatacaggtacaacccgcatgtaacaggtgttcatgcgggttgttcttttttaaaaagatgtacaacggctagcgctatgcaggccagggattctggtaagtggagttatttaatttcacctccctcgaagacaaggtcagctgtatttgcaggggttgctcattggcggaattaaacgtctcttcgtattctacgcaataggcgtctgtaaacttcagctctttgagcctcgacatggaatcccgccggaaaaaggtgatactgccgtttttcgtctgggtgttggaaatcatccagtcaaacaaactggtttcaccggcagactcgatcagcaggttaatagtgcctcctttggggcgggcggcaggtttcccgttatgatctgtattttgggtaaatgaaaacctgcattccaggatgttcatttcttccccgtcgatgttgagaacagctttaaaagacataattaatctggttaacaggtccgttgcaaggcacaacagacaggcacaaaaatatggtatacagaatgaaaatacacatttctgtttacatgccgaaaaattgagggttatttttgaaggaagccaatggatcccgcagggatggcccttccagccagttgttgatatacggtttaataactatataagatcaaatgcctgggcaaaactggtcaggtcgtagctcgactgtgccccaatcttcgctttgatatttcgccggtgcgtaacggcggtcttttcggagatccccgccttttcggcaatttcactggcgctgagtccgagggccagcagccgcaggatttccttttcccttttggtaagggaagcaaaaatatgctggttgcggcgcaggaagttattttcttccagcaggcggtttaccttgctggtaacgtgatgcagcggatcaatgggaatggcgcaggtaataacgtgtgtgggaagccctccggcatcccgcataaatacccgcgtagagcccagatgccaggtccagtcccgcgacgcagtggttcgtacctgctggaaaaaggtgaccgttatattggcttccgccggtgcgtccagcatgttgatgatctttggcaggtaatccgctacatcgtgtgggttaaagaaggtgtcgtaatacccggcgcccatttcccgtaaagcctccagcgtaatatcgagttcccggcagccccgtggcgacatatactccacgtagctctttaccacattcattacaattaccactaccggaagctcctgatcaatggcccttaaagcgttcagcttctcttccagccctgatccgtcattattaaatgcagcgtgctcaatcatgtacctgatataaaatcgtgtataggaatcctctgtgatgttggttgactacttacttcagtgctctttcggcaacaaatgtagtgaaaataagaaagggtccctcacaaagaagagacccttttttggggatagaaaatacggtgattgactaaatcaggtggatgactttatatagaataatgtgaaatcagattactttcacaaagatatgttaaagctaaagggaaacaaatacctacatgtgagtatttttaaaaaataaatgaccttcctatcatgaaagccagtccggaacatttcctccaaagcctttcgcacattgctccccttagcgatgaagcaagggaactatttgcaacacatactacttcacaaatagtaaaaaagggtgactatctactgcgtgaaggacaacgctgccaacacatatggctcattgaaaccggtgcctgcagagcctttcaacatcacaatgaaaaagagatcaataccagcttctactttgaaaatacattcctcactaacctgaacagcctgcgaaacaacgttacggccgattacaatatacaagctattgaagccggcaccatatggaaatggcataaggacaatctgttttcactctatcagcagtcatccgaaatcaccgcctttggccgccagtggctggaacacctgttcattgaacaggaaaaacataaccaatggcttaaaagacacaatcccgaagaacggtaccagtccatactaactacgcaacccgaactcctgcaacgtgtatctcttacacaactcagctcttatctcggcatctcgcgggaaaccctcagccgcatccgccgccgcctgccctgaacccattatgtgacgtttgacacaattgctttatagctggccttctacctttacggtataaaactaacggtcatgactatacaagaacagaaagatttcatcggacactacattgccaccatctggaaccagggcgataccagtcgtttggagcaattcctgcatccggattatgtggatcattccttgccgcctgcgctgcccggcaatgctaccggcctgaaacaatggattgcattaacgcatgaatccttccaccccgaaaccattatagaagaacaggtagccgaacccgggaagtgtatcataaaagtaaccatgcgcatgaaacacattggattatggcggggaataagccctaccggcttaacagtaagcattcctggctatcgttgctttcgattgcaggacaaccggatcgcggagcactggggtttaatagatggaaatgcacttgaaagaaaacttgctccaaagtcttaagtactccgtatgcccgtacccgttataatcgtttactaagaatggagcttatggtcgcctgccgcagggggacaagcccctgccggaaagcaacaccattggtaaaactgagtaataaaacgtgaaagtggaacggaaaaatgcaacagtccatctgtaaaaagatccgtattaatacagtaagcaataaaaatccaggtgttacggccggctatgttcccttccggaaccattgtaaaatcaactatccgcgcatccggatcgttgatttcaacagccagctccttccggtaatattcgtcctcccccttacaacaccacgccggccataaacacctggaaataatattattcttcccctggaaatgtttctatacaaaaatgccttttattcacacatctgcttaatacttttttatcttttaattatactttgataatcaaattcatgatataataagtgtaataataacacctatatactcaaatcgcccggcagttaatactataaggaaaaaagtaaaaattgtattttacgcccgataaccttatttttataatgcttttttagcaaccaggtcataaaaatcaacaaccagtacttacattccacgtcaggattccggtgtgttataaaaactgcgctcattatgaagagtaaattattaagggaaatcactcctcttacgcaaagtgattgctttacgttgtttgcccgtgagaaaaaagtgttcgatttcccgttgcattaccacgacgaatttgaattaaactttatccagtatgccagtggggccaaacggatcatcggggatcatattgaagagataagcgaccttgagctggtactggtagggcccaacctgcaacatggctggtttgccaataaccatgaaggaggcagcgttaaggaaatcaccatccagttccaccgcgatctgtttgatgataaattcctgcagcgcaaccagatgaatttcatcaaaaacatgtttgaacgttctctgcggggaatcctcttttctaccgaaaccacccagcagatcatgcaccgcctgatccggttgccgcaacagcaaggcttcgattccgtcctggaactgatgtctattttgcacgacctgtctatcagccggaatatgcgcatcctgtctgattccactttcggcaacacggaaaccttctcctacaatagccgccgcgtggaaaagatcatgacctacctgaatgccaattacgataaaaacatttcactgggggaagccgccaggctcgctgccatgacggaggtagccttcagccgctttttcaaggccaaaatcggtaaaacctttgtggataccctcatagaaatcaggctgggacacgcttcccggctattaatagaaaccacacacacagtaaatgaaatcgcctataagtgcggttttaataatatctccaacttcaaccgcatctttaaaaagaaaaaagattgtacacccaaggaattcaggctggcttatacctcttcagggacgcggactttcgtttaacgcggattttgtcttggctcaggattacgctgattttactgattacctggatttttacttttggatttttttggattttcagatttataatgtaataattaagggagataagagcgaatatccgcttctatctcccctaatcctttataaatccaaaagtaaaaatccaggtaatcagtaaaatcagcgtaatcctgagccaagacaaaatccgcttagcaggtaaattgtaatagcgacatgtaaaaaaaaaggtattactggccactgtaccggtttatatgccccgttttgcatatatataagggttaaatcctccaaaaatgccggtaaaagcgtaactttgcggcttcatgcagacttctactttattaaagcctaattgctacgtaaatgatgccgggtttgactggttgtatcctgaaagaatacagcaactatcaagaaggcactggacgccactcagtatcgctaaagcagcggcccgtttcctcgcaaatgaaccagggaaaaaaattctggacatcggcagcggtgtcggaaaattttgcctggtaggcgcccgcttttacccgggaaccaatttttacggcattgagcaacgggaagagctttatcagcacgcacttgaagcaaaggctgccacgcaaatcaggaatgtgagctttattcacggcaattttacgcaggaggatttttctgcgtatgacggtttttacttctataattctttctttgaaaacctggtagatcaggatcagatagataacaacgtagaatattcaacaagtttatataattattacagccgctttttatttaaaaaactggaaagcagtgcaagcggtacaagactggtaacataccacagtcttgaagatgaagtacctccctgttatcagatggtggatgcttctacggatttaatgctaaaaatgtggatcagaagataggactaagtaatacaaaaattaatacaatgactgcagacgaacatgctttagagaccatagcacaattaggcgccataacagattaccagcaggctgaccagttactggaaaccataaaaaaggaacatgctgctttatataaagaaatcttcacctccctccaggaaaaaatagaaagtttgtcaccattggaatgtaacagcttacagtggagcatttaccggtatgccttgatgcacatacgtaaatgcacggcattggaaccagcctgctaatcaggcgctgatagccagctttttgccaatggcagccaccacggcttccggcgaaaattcttcctgcaaatacaggtcaacaaaatcgtaactgatttccagtgaaggcgcaataagatatgccgccggcacaggtacgtctgcattaacaccggaaacaaagccccagatcgggtctgattccctgtaaatgcctgctttcctggctatgcggaactgtgcgtcgtgcactacatcaaatggcaacacctccggataaaccgatgtaaactgcttcttatcctcgctggacaataccagcaaacgggcgccggcagccactatggccgcatggctttctttcaatcgttccatcagctgatcagcgtaattgttccaatgccaggaataaaacaccactaccagcggctgcaaagtaagactgtgcaatgatgcgccggaatgggcattattcagcagcggaccagcgttgatcacacgcgcttcttcaataaaaaattcaggaaaaaagctgcctgattttaacgggttaattttttccctgttccttacaggactggggaagttttccggtgtgggctgcggtaagtaatcggcgtatctatacaatgatgacatattaaaggcttttataatggctgataaaatggccgctgttataggtttggtgaatatcttttgctttcgtaaaacaaagatagggagaatattttaattaccctactattcctatagactattaggattataaattctaaataactggttcctaatagctttgagaggaaaatatttttccgggagatgaaaacaggggtatttaagtccggcgccaaacattcaaagcgtgtacccgttattgttataaagttatagcaaccaggggcgcccatctttaaaaaaaacgataaaaacgtgccaggataaacccggatgacataatttacagcgaagccataaaagaataaatattgacatatgctgctgaaacacagactatcactcggccagatcttttcctttacctggaaggtagaccttatgttgctgggatgttgtaccctggtatattttctcgactcacgctggctggcagcacatattaacatccctatagccgtatctaccgtactgggtaccgccatcgccttctttatcggcttcaataacaaccaggcttacgaccgctggtgggaagcccgtaaaatatggggcgcactggtaaacgactcccgcacctggagccggtccatgctcaactatccctccccggacgctacgcccgaaaccaaagccctcatccgtcacatgatttaccggcacctcgcctttatttatgcgctcaaaaccgttctccgcaaacggcccgacgactactacacccgctaccttaccacagaagaaattgaagaagtacaaaaacaaagtaatatccccaatgccatcctgaacctgcagacccgcgacttacagcaactccgggcctccggcagcatcgatggcttcacttttatagaactgaaccagatcctggtaaaacactgcgactgcatgggccagtcggaacggatcaggaacaccgtattccctcccagctatgtatattttacgcagatgtttatctggttttacgttatcatgaatacactgatgatgacggaatccatcggcgcatgggccattcctttcggatggatgttcggcttcgtattccatgtaacccacctgaacggcatcaccctcatggacccgtttgattttcagccactcgctattccgctcgacagcatcgcccggaccattgaaatcaacgttatccagctgctgggagatgaaccggtacccgcaccggtattgccgcgacaggaaggtttgtacgtaatgtaagcccatagcgaaacgtatttactttgtaatacgtaattccttatttttacacctatgacgtatgaccaattatgtaatctatatgcccagtcagttaccctcaagatactacgggcacgtagcgcgccaatgatgttgtcattttttcattacacattcaaggaaaaaaatcatactaccatttccaatgtggaactggtaacccgcttgtccgactacctcggcgtaaccggctaccgggccgcagatgatgaaatagacgctaccagcctgctggaacacgacgatgtgaaggccaggaaatatatcgatcaatggagcaataaaggctttctccgcaaatatcccgacgacgacggactggatatccatgagctgagcagcgacatggaaaaagtaatgcactgggtatccaccctccagaaaagagaatttgttggcacagaaagccgcttcaaagacatcttctccaaactcaaagagctgattgaccagagcaataaagacccggaacaaaggatccaggaactggagaaaaagaaatatgaaatagaacaggaaataaaagcgatcaccatcaccggtaaagtacaggtgtttgatgatacccagataaaggaaagattttacgacgtcaatcgcatgtcgcgcgaactcctgagcgatttcaaagaagtggaacaaaactttgaacagatcacccaggaaatttatcgcaaacaaagcgaaaaagatatcgcgaaaggcgcactgctggcgtataccctcgactccttcgaagcgctccgccagaaagaccaggggaaaagcttctactccttctggcagttcctcatggatgaaaacaaacaagaggaaatgcgggagctgatcgaaaaactttatctcctcctggaagaccggaacatcgaatataaaaatgaccgcttcttaaaaaaactcaaacaatttcttcatgcctccggcaaaaaggtaattgacgccaataaaaaactgagcgataaactcagccgcgtgctcagcgaaaataatcttacggatcaccgcaaagcaatggagcttatcaacgatatccggcagctggcgttccaatcgctcgagaacccaccaggggaggaattttttatagagatagaaagcgatccagaaatagacctcctcgaccgctgggatatggcggaagagaagaaacccaacgttgaagtggaattccccgaaggaatgggtggtaccgaatttgacgacaacgacctgaacgcattatttaaccattttaacatagaccgcgccctgctggaagatcgcatttccacacaactgcaaaataaaaaacaggtaagcctgaaagaactggtagaaatttatggcgccgaaaaagggctcactgaactcattacctatttttccatcgcgagccagtcggcacaccatattatcctggaaaccccggacccggtgatgctgggcagccgcaccatcaatatgccgatggtgctgttcacaaattcacaaaactaatatcatggccgagaaaaatatatctccctttgcacacgtgtttctaaaactcatgcagggacctgtatacgaagaagataaatcttactggaaagacctgcttggatggcaaacagagctcagcaaatacctgcagcaaaccggtctccaactggtggtaaacgaagccgacggatttgcacgtatcgtgcaaccggaagcagatgaaaccaacgaaaaaccactgcctcgcctcatgcgcaaatcacggcttacctacgaagccacgctgctgtgcattgtgctccgtgaagccctcgatgaatttgatatccagggcaatggcacccgtctttttatgacacaaaaagaaatcaaagaaagactcgcgctcttctttaaagaacgacacaacaaatccaaactactgaaagatctcaataaacccatcaacagcctcttaaatgtaggcgtgctgaaaatgacccgggaggacgctgccaacaaggaactgcatcaatacgaggtaaaaagaatcatcaaagcactggtaaataacgagaaactggaagaaataaaatcaaaattaaacctgcatgtccaccctgttcaatagtgattcaaaagaaagtggattccggttgcaatattttgaaatatacaactggggaaccttccacaataaaatatatcgtgtcaataccaacggtaatacctccctgctcaccggcgcaaacggtagcggtaaaactaccctgatcgatgcgctcttaacactgctggtgcccgccgggaaaagattctataaccaatcgtccggaacagaacaacgccgcgacagaggagaagaatcctatttctggggctactacggtaaaaccttctccgaagaatcgcagcagtccaaaacggaccagctccgtcataaggaaaacaacccttactcagtactgctggcctacttctacaacgccgctaccatgcaccagatcacactggcgcaggttagatggtactccggggaaatgaaacggcaatacatcgtttcgccgcataaacttaatatcaacgatcacttcggcaacgggaaatttgatgtaaaaggcgactggaaaaaaagactgcgcctcgaatttcccaaaacagaaatcaccgacagctttaaagaatacgcagccctgttcagcaacatcttcggactgcgaagcgaaaaagccctgtctctctttaaccaaaccgttggtatcaaagtactcggcgatctgaacacatttatccgcggacagatgctggaagaaacagacagcgaaaacgaattcctgaaactgcgcgaaaactatgatagtttactcaccagtcatcgtgccattcagaaagatgaaacccagctgaaactgctggaacctatcatcgaaaaccgcgcggcctggcagcaattacaagacaggaaccgggagttgcaaatgctccaggatatcctgccctcctggtttaataaacaggaaaaagatatcctggaaagagaactggaatctttacagaaagaacaacaggcaactacccgcagtcttaccaatatcaatgagcaactccagtcgctgcacctccgcaaagacgagctgatagcccagaaagccaataacagcgtagatgaacaactgcgctctatcgaaaaatccatccattacgagcaaaaagccatggaggccaaacgtaataagatggaagaatacaatatgctcacagaccggctggagctcgcacccaatccggatgaacagcagttccatgaaaatattgcaggcgctgaacagatgaaaacagcgcacgataaacaactggaaacattacaggaagaaatttttcatcacaaaagcagcctcgccgcagaaaggacacaggtatcaaagctggaagaagaaatagattccttcctgcaccggaaaaataatatcccttatgagctgatccgtatccgtcagcagctggcaaatatgctggatatccaggaagatgacctgccttttgccggtgaactgatcaaagtaaaagatgcagagatccattgggaaagcgccatcgaaaaagtattgcacaacttcggcctgcgcctcctggtacccgaagaatatatcctggacatcaaccgctacatcaattccaataacctgcaaacccgcctcgtataccacaaagtagaagaggagagttataccatgttgcggatgccttctgaaaaagaaagcctgctgcaaaaaatagatatcaaacccggcaccatcttcaaggaatggttacagaaccagctgctcgatcagttcgattatacctgtaccgacgacatgactgtattcaaccgttgccggaaagcagtaacttccaacggactaacgcggcaggctacacgccatgaaaaagatgatcgccctaaccgttcccagaaaaataattatgtgctgggatggaacaacaaaaacaaattgcgcctgttaaaagaagaacaggatgaatgcaacaagaatattgaaacgctgcagcatagcatttcccagctggaagacagcaggaaagccattgccaatatcaatgcgctgctgaacgcattgctgtcgctgcgtaactacagtgaaatcaactggcagatccatgccggcgtcattgaatcatttgcacgcgaaaaagcaacgctgctcaaaaccagcgataaataccaggtgatctgtgatcagctggacgatattaccgggcaaatacaaggcaaggaaaaagagaaagaaggcaccctccaggaaaaaggccgcctggacgataaagccgcggagaaactgcgccacttcaatcaactgaaggtcaataaactggacgacgtttccctgcaatacgtgctggaataccttacagatctgtcgctgaccgaaccggcggaaacaacccttgagctggcatcttaccggaaacgggcagatgataacatgaaggcaaccatgcacgacgcgatgcgtctgaccgcggaaaaagaagctgaaatcacccggcagctggcagcatttgtgatgccgccaaaatccatccacgataccttccctgactggctcggtgatgttacagacctgcagccgcatgtgaaatacctcgacgaatttacctcgctctatgagcggattaaattccagcggctcattgaacataaagaacgcttccgtaaatacatggacaccagcatgctcaatgccatcaccaactaccgggcatggatatacggacaggaagacctgatacgcgaagtaatggaagacctgaacgaacctttacgcaacatcaccttcaataaaaatccggatacctatctccagctggaatgccgccatgtacgtgatgtggagatccggaacttcaaggaaaaactcagcaacgcagtaccggattcttataaatatcaacttgaaaaagatgaagcctatggcgatcagctgtttgaaaatatcaaactgctcatcaccgagttacaacaaaacgaagcatggcgccgcaaagtaacggatgtacgcaactggctcgacttcggcgcaaaagaattctatgtggccgacaacaaggcattcaaatattacgaggatacggctagtctttccggtggcgaaaaagcacagttcacctacaccatcctgggagccgccattgcctaccagtttggcatcaatgaagccaaccgtcaacaccgcagcctgcgcttcatcacagtagatgaagccttcagcaaactggaccctgaaaagagtcactacctcatggaatattgcggacaactgaacctgcagctactggtagtaacgccactggacaaactgaatatcgcagaaccatatatccatgcgtgtcattttgtagcaaataaaaacaaacgcgactccgtggtatacaacttcacgatggaagaataccgcgacaggaagaaagagttcgaatccatggcggcaatgtcctaagcgaaggttgtctttctcaggattacgctgattatactgattaactggatttttactttttggattttataaaggattaagggagatataagcggatatattcgcttttatctcccttaattattaaatctaaaaatcttaaaaaatccaaaaagtaaaatcagtaaaatcagcgtaatcctgagaaagacaaccttcgcttaggacattgccgccagagcgggtgctggttggcattgcggctcccgtcccatttgtttgcggccccattcgctcagcagggtaatgaagggtagtagttcactgcccgtatccgttagttggtattccacgcggggcggcacctccaggtatacatggcgggtaaccaggtcgtcgtcctccagttcacgcagcacttgtgtgagcattttaggggttataccggtcatgatccggcgtagttctccatatcttttcaccccgtttctcaggtggtaaataacacgtcctttatgcttcccgccaatccgttggaaagcgtaatcaaccgcgcagatcgtgtcagcatgaatattttttccggatttcttcatttttttggcattgattatcagcaatagtatccatctggtacctacattcccaaatggtgcatacttgtcttatatgaagttagggagcaattttgtgaaagaaaaaaatagttcttatgaaagcaatacaacaagtagccttcggactggaaagtttacagctcaaagaaatacccactcccatagccggccccggtgaagtactggtaaaaatagaggccgcagcactcaattacctcgatgtagccctcgctaccggcacttacagcaaggaattaccgctgccccgcattcccacttccgatggcgccggtgtagtagccgccatcggtgataacgttaccaaatggcaaccgggcgatcgggtggctattcattacaaccagctctggcagcatggcctggccaccgccggtaccaatcatatcagaaccggtgtaagcacgcccggcctgctggcagaatatgcagtaatccctgaatatgcactggtacgcactcctgccaatttaaccagcgtggaagccgctacattgcctgttgccggcgttaccgcatggacaggcctgatgggctatgctggtatcaaagcagggcaaaccgtacttacacaaggcaccggcggcgtctccctttttaccatgcaaatcgcattggcagcaggcgcgaaggtgattgccaccagcagtcatccggataaactgaagaaattacaggagctgggcgcccacgaagtaatcgattataaaaaatatcccaactggcatgaagaagtaaaacgtatcacgggcggggaaggtgtacatgctaccttggatattgccggcgccgccaccatcgttaattctgttaagtcggtaggcttcaatggctttgtgggcctggtaggcttcattgaaggcgcacagctgccggtagacctgtttacagttgtaggcagctatatccggctgcagggctactctgtaggcagcctgaaaagtttccaggagctggctgccgcaatagcaataaatgatatccatccggtaatagacagcgtattccctgtaagcgaggcgcaggaagcattcaggtatatgggcggcggtaattatttcgggaaagtagtaatagaaatgaagtaaagtggtgaacatataaacgtcctgcgcatcggcaggacgttataccaagtaaaccattacactaaaattattgtttcaagatagtaaaaacaagttgaaaagcgggttatttccttgttaaggtgatgataacattatatttttatcaatacatgacaaacatcagtttcatggatatcttcacctgctacctttgcatcaataattgaacattatgccttcagtagaaatactatccagaatacagtttgcctttaccattgccttccattacatctatcctccgctgagtatagggctgggactgtgcctcgtgatcatggagggcctgtacctcagaaccggtttgtcgctttacaaggacattacacgatattggattaaaatatttgcattgatcttcggtatcggcgtagccaccggcattgtaatggaatttgaattcggcactaactgggctacttattcacattacgtaggcgacattttcggaagtgcgctggcagcggaaggcatctttgcatttgcgatggaatctgccttcctgggcgtattattgtttggctggaaccgcgttcacaagggcgtacatttcttttctacgtgtatggtggcgctgggctctatcttttctgcattgtggatcgttattgccaattcctggcagcaaacgccaaccggttaccgcatagaagggcatgatctgcaggcgcgtgcagtagttactgatttctgggagatggtgtttaacccttcttcggtcgacaggttctcacatgtgattattggttcttttctcgccggctctttcctggtgatgagcgttgccgcctggtatgtacttaaaaaccgctttgccaaacatgcacaggctatgtttaaagtaggcctgggcgtagctgtaattgctgcgctgatgcagcttttcaccggtcaccgttccgctcactatgtaagcaaatatcaacccgctaaactggctgctatggaagggcactacgatagttctgcagtagcgcccatgtatattgtgggttgggtagataataaaaatgaaaaaacaaccggcataaaaattccgggaggcctttctttccttacgcatggcagcttctccgccccggtagaaggtctcagagccacgcccaaggcagacaggcccggcgcagtgaactttgtattccagatgtatcatttgatgattacgatcggcatgatactcataggacttacgctgctggccgttttctttttatggagaaagaaactgtttaaccagcgctggctgatgatcatatttgcatgggcggtactgctgccgcaaatagccaaccaggtaggctggtatgccgcggaagtaggacgccagccctgggtggtgtacaaactgctgcgcacatctgatgcactgtcgcgtaaagtaaccgcagaccaggtaatgttctcgctgatattatttacgctggtatatatgttgctgtttacgctgttcatctatctgctaacgcggaaaatacagcacggaccagatgtttcagagaatgctgaaattgaatacgacggctattatcacgataatataacttaccatcccactaaattataactcatggaaacaattctcggactggatcttcccacctggtggtttttagtgattggcggattgatcactggttatggtgtgctggatggcttcgacctgggtgctggtgccttgcacctgttttttaaaaaagaagaaagccggcgcctggtgctgaatgcgataggaccggtatgggatggaaatgaggtatggctggtaattgccggcggggccttgtttgccggctttccgctggtatacggcgtggtactgtctaccttctacattccctttatgttattcctcgtagccctcatcttccgggctatttcaatagaattcagaagtaaggaaacctggctatggtggcgcaaaatgtgggatatcagttatacagtgtccagcaccggtattacgctgctgctgggattggtactgggcaacctcattcacggtctcccgattaataaggaacatgaatttaccggtacgctgctcaccttttttaatccttatgcgatactgattgcttttaccaccttatcgctgttcatgctgcatggttctatttacctggtaatgaaaacggaaaacaggctgtacaccaggcttacggtgatagtgaacaactgcagcaagttcttcattctttgctttattctaacgtcaatggctacccttatttatgtgccgcacatgacgttccagtttaaatcgcatccgcagctgttcctgctgcccatgctggcggtactgatcctgctgaatatcaaaaggaatgtggatgcacgcagatattataccgccttcctctattcttctattatcactgcctgtttgcttatcctcttcgcggtaggcctgtatcccaacattgtgatatctactactgatcctgcttatagtatcagcatttatgcagcggcgtcttctgttaaatcgttgaaaattatgctgctcattgcagccataggcaccccgatggtaattggatatactactttcttattctggacattccggggtaaagtgaagctgaacgaaatgagttattagatattagctattggctaaaaaaacaggtccccgcaagaaattgcagggacttaccatttaacctatattctgtactgtagcattgtgttgatgatctcccgaaagtcgccagttatcattttcccgtatcctatcttttatcaggagagatgtatttaagacggcctgctttgataaaagtttaaccggtttaaaaaaatttctgaaaataattccgggaagccgaaattagtacccagaattgatcacttccatgaatcgtatcgaccggcttaccgccattctcatacaactacagggtaaaaaaatagtaaaggccgcggagatttccgaccgctttaacattagcttaagaacggtgtacagggatgtaaaagccctgcaggaagccggcgtgcccattggtgcagaagcgggtaccggttattatatcgtggaaggctatcacctgccccctgtgatgttttccaaagaagaggcagccgcactcctgaccggggaaaaactgatggaacaattcagtgaccacagtaaccggaaacagtttagtcttgctatggaaaagatccgttccgtactccgtggaacagaaaaggactacctcgaatcactggatgaaaacatcgccgtattgaggtaccggcctgtagtagcggatgcggcggagttccccaaccggttcctttccgatattcagcaagccctgggcatgaaccaggtgatcagtatggagtacttttccttccaggaagaagtggccacacgcagggaagtagaaccaataggtatttttcatagcagcgccaactggcacctgatcgccttctgcaagctccggcagggctaccgcgacttccgggtagaccgtatccgtaaattaaccgtgctgcctgccacttataagaaaaacaagcatctttctttgcaggattacctggaacagcagcgcagccggaacagcgaaaatacctatctcgtaaaaatagcgctggacaacgatatgttgcggtatgtaagggaacagaagtattactatggccttatggacgaaaaagtggtgggcgataaaacagagcttacattcctccaggcctccctgggccatttcgccaggtggttgattatgtttggcaaccgggtggaagtactgcagccccaggagctcaaaaccgctatcggagatcttgtaacagaactccacggacattatttataaatccggaaatgctgctgacataaggttgtcactcccaggctgttcttttgtattgtgatcaaaaacaatacaaatatgaaaaagctcagcaattgctatgtattcctgttcgatggctactccgactgggaacccgcgctggccatgtatggcctgggaagcttcacagataccaacatcgttaccttttcctttaccggcgaacccgttacttccggcgggcagctaaagatacaaccccgtgcaagtcttgatgaggcattgaaagcggatatcgacctgctgatacttcctggaggtgcggccatggaaaatgattccaatgctgcaatcattccacttgttaaacaactgctggcacagcaaaaaacagtcgcggctatctgcggcgccactgtgctgctggggcagcacggcttcctggacaacattgcccataccagcaatcaccctgaagtgctaaagcaacaggcccctgcttataaaggcgccggaaaatacctggatgaacccgcagtagctgataagcagatcataaccgccagcggtactgcaatgacagcctttgccaaagctatctatcagcattttaatttactggagatagaacccctgaagttttggtttggcttctttgatcattcggctgttcttccggagatgttatctgcggcgccctttcatttcttctatcagcgttacgaaactaattatgccggtatgctgtcgctcgtacgcaccgctattaaagacgtgtaccgggaggccatcaacgccggactggaaatatgcggcgcccccgaatggcactaccgcaacttcgacggaaaaccagataccgtattcaccctggatatcggcctgccggtaacggccgtgcaaacagttacagcgccgtggcaatgcgaaacactgcccgccttcaactgcgtaagcatgcagcacaaaggcccctgggaacagctcatcactacctacgggcagttatttaccggtatcggtatactgggtatggaggtaaccggctatacgcgggaacaatacctccggtataattttgaacaaccggcgcagaatatcaccaacatacagattgggttacgctagccggcgtaaacatcccctggcactccccgggggattttaactcttaaaacaatgaaagtctatatcatcatgggatggctgctgctcatcacctttgcatttgatatacaattaacatttaaaaatatgagtaaactggatttaacaaaggaattcaaacagtactatactgccgcgttagtacctgaactggttaccatagaaaagggactgtttgtaactatcacaggcaaaggggatcccaatggtcccatgtttagtgaagtaacggcagcgttgtatgcagtggcatatggtattaagttcagcagcaagcaaaagggccgcgactttaccgtgagcaagctggaaggtttctggtgggtaaacgttaataccgcagatccgctgcaggtatcccgagatcaatggcactacgaactggccatcaggatgccggacgacatcacccgccagcagttttccgaagcagtgcttgctgcagagaaaaagaagaagtctgtttttatcaggcaggtggatttaaagcatatagaagaggggctgagtgttcagctgatgcatattggtccttatagtgaagagccggtatcattgaaaaagatggaggagttcatgcttcagcaggggttgcgcatgaatgggcggcatcatgaaatttacctgtcggatttcaggaaaacggcgccggaaaagctgaaaacgatattaagacacccggtaagtaagtagctgatgatgggcggagcacatcttaccaaaaacagttagtcggttaacccgagttgtataatggcttgttgtgcagcgatctggctggcatcttttttattgaaggctttgccgctgcaaatgagttcgccatctactacagcccctacggtgaagatgcgccggccgttgtccatctgttcttcgaggagttcgaattccagtgttttgccatttttattggcccagccgtataatttgttcttgtggttcatttccacggtttccagcagttccatgtctatataaggcatgataatgcgtttatgcacaaactgttgggttttattatagccgcggtcgaggtatacagcacctacgagggcttcgagggtgttgccgaatatctggcttattttgaggaagctgttgtatttgtcgtagatggtgagctttcttaagcccattttgatggcaatgtcgttcaattgttgccggttaacgatcttggagcgcatctcggttaaatatccttctgttttatagggatattttttaaagagatagtcacccacaatggcgccgagaatagcgtcaccgaggtattccagcctttcgttgctttctaggaatttttctttactggaacgatggctcagggccacttcataaagggcaaagttaccaggcgggaagcccagcaggttgtgcagctctttatataagtgcctttttttggaaacaagtcgatataaaaaacctggcagtaaactcacacaatcaagatcaaggaacaaattttttgaaaatcacggaagcattatgtccgccaaacccgaaggtgttggacaatgcagcgtttacttctctcctttgtgcgatattaaaagtaaaattcagcttcgggtctaactgcgggtcgtcagtgaagtggttgatcgtaggaggaactatgccatcgaggatagacataattacggctatggattcaacggcgccggcagccccgagtaagtgccctgtcatggattttgtagagctgatgttcatttgataggcatgctcttcaaaaacgcgctgaatggcttttacttcggcaatatctcccaacggagtggaagtaccgtgaacgttgatgtaatcgatttcgttggcctgcattccggcatctgccaaagcgttccgcattacatttaaagcgcctagtccttccggatgtggggctgtgatgtgatatgcatctgctgtagcgccgccgccggctaactctgcgtatatcctggcgcctctttcctgtgcgtgttctaacgactccagtatcagtgcgccagctccttcgcccatcacaaaaccatcgcggtcaagatcaaagggtctggaagcagttttgggatcttcattcctttctgacagggccttcatggcgttgaagccaccaacacaaggctcgttgatcacattttccgatccgccggtaaccaccatatcggttttgccgtaacggatactgtacatcgcctcaatgatagcattggtagcagatgcgcaggctgatacaacggaaaagttgggccccctgaaaccgtgacggatagaaatatagccggcagcgatatcaagaataagccttggaattagaaaaggactgaagcggggcgtaccatcccctgtatggaaatctctcagctcgtgactgaaattgatcatacctccaacaccagtaccccatatcactccaacacgatcagcattgatcttgtctttattgatattggcgtctagtatcgcctgatctgcggcaattacagccgtctgtgtaaaggggtccattttacgggcctcttttttgtccaggtagttagcaggatcaaaatttttcagttcgcaagcaaaacgggttttgaacttggaagcatcaaattgcttgatataatccgcgccggatacaccgttcgtcaatccgtgccagaaatcggccacagtattgccgagcggtgtaagagcgcctaaacctgtaacgacaactcgtcttggttgcattaaaacaattctgattaggaggattattttacatgttcttccaggtaagcaactgcctggccaacagtagtaatagtttcagcttgttcgtcaggaatggagatgttgaattctttttcgaattccataatcagttctaccgtatccaaagagtcagcgcctaagtcattggtgaagctggcttcaggagttacctcggcttcgtcaacgcccaatttgtcaatgatgatctttttaactcttgatgcaatgtctgacataattttaagtgtttttggtttaaaacttgactgcaaaaatataatttttattgaattgccaacagatagcccgaattttaaggacgctctaacctggccaatctcaccaaacccaatacagtaaacatattcatagctttgttaataaaagaatttatatatttttgatactggctggattacagatttgcatattttaccacaaaagtcgcctttttcgggacaattacgccattctctgaaatccaaaacatataaatcttaaaatatctccattcaaccggctatttagccacttatctaaagcattaacgctatttaacagttgccgggagcattcagcctcctcaatgcgtaaatttgtccggcttgtgagatagtatcccttcaggagcctgtttctctgttatgaatcagtagcaaaagttagaaaaacacatataaataagatatggccatcaccaaaaagaccgttcgcacaatagttatattggccgcagccggtatcgtcatttacctcgcttttaagaaaatatccggcaaaaaatcagccggagagccggccgctgccgcatccggcgcaaaaggaggcgcttcccggctgctgcttaccgatgcctggattgttaaaacatcccggctcgatcaatctattgaagcaagcggcaccttgcagagcaatgaagaagtagaagtgaaaccggaaattaatggccgcatcacacacctttattttaaagaaggaaccactgtaagaaaaggagatctgctggttaaactgtatgacgaagacctcagagcacagcttcagaagctcaaattacagcagcaactggccaaaacaaccctggaacgccaggaaaacctccttaaaataaatggaatcagccaacaggacgtagatgtgacccgcaaccaggtaagcgcctacggagccgatatggagtatacccaaacccagttgcagaaaacagaactacgcgctcccttcagcggtaagctcggtttacgcaacgtaagcgaaggcgccatcgtgtcgtcccttaccattattaccaccctccagcaaatagatccgctgaaaatggacttctccgtggccgagaaataccgcaacgccatcaaaaatggcgaccaggtcaacttcctggtatccggtgacaataaagaatataaaggcagcatttatgccatcgatccgaaaatagatcttaccacccgtactgtaaagctccgtgctatcgttcctaataataacggtatcctgttccccggctcctttgccaaagtgaaaattttgctgaaagacctcccggatgctatgttgataccgtcacaggccgttattcccggtacccgtgataaaaaagtaattattgccgataaaggccaggccaagtttgtaacagtagaaacaggcatcagaaccgaaagcagtgtacagatcaccagtggcctacaacctggtgacacggttattaccactggtattctccagctgaaaccaggcatgcagttgaagtacaataagatacaataatagttttcccaacggcactaccaccggcagcatcgctgccaacaggaaagcccggcagaaaacctgaaaataattatcatgagtttaccttcattatctctcaaacgccccgtatttgctatcgtgatgaatatcattatcgtgatattcggcctggtgggctttacttttctgggggtaagggatttcccggcgatcgatccgcctgtcgtgaacgtacgcacctcgtatgcaggcgctaactccgatatcatcgaaacacagatcaccgaaccactggaaaaacagatcaatggtatcgcagggatcaaaaatatttcttccagcagcagccagggaagcagcaacatcaccgtggaatttgaactgggagaagacctggaaggcgcgaccaacgatgtgcgtgataaagtatcacaggcgctgcgccagctgccacccgatattgatgctccacccgtagtatccaagcaggacgccaactccgaccccatcatctccatgacggtgcagagcaacacccgcaaccagctggaagtaaccgaatacgcctccaacgtactcctggaaaaactgcaaaccattcccggcgtaagcgccatacagatatggggagaaaaaaaatacgccatgcgtatctggatggaccctgccaggttatcgtcctacagccttacccccggcgatgtacaggccgccctgttacgcgaaaacgtggaactgccctccggcaaaattgccggcaacgccaccgactttaccgtacgtaccttcggacggctggtatctgaagacgatttcaacggcctgatcattaaaaatgtaaacggcagcgagatacgcatccgcgacatcggccaggcagtgctgggacctgaaaacgaagaaaccgtgctgaaagaatccggcagcccgatgattgcactcgccctcatcccgcagcccggatccaactatgtagccattgcagaagaattctataaaagattcgaacaactgaaaaaagatatcccggaagattattccgtaaatattgcaatggataacacccgcttcatcaaacaatcgatcgatgaagtagaagaaactctcatagtagcactggtactcgtaattattattgtatacctgttcttccgcgactggctcatggcgctccgtccgctgatagatatccccgtatctttaatcggcgccttctttattatgtacgcctgcggctttaccattaacatcctcaccctgctggccattgtactggccaccggtctggtagtggatgatggtattgtggtaacagaaaatatttataagaagatagaacagggaatgcctcgtatgagggctgcacgcgaaggatctgaagaaatattctttgccgtaatcgctacgtcgatcacactggcctttgtattcttaccgatcatcttcctccagggcttcgtgggacaactgttccgtgaatttggcatcgtggtggccggcgcagtaatcatctctgcctttgtatcactcacgttaacgcctgtactaaacgtaaagctgggccgtaaaacacatacccattcctggttttataccaaaacggaacctttcttccgctggatggaagacggatacagaaaatcgctggaatcgtttatgcgtatccgttgggtagccggactaatcatcgtcggctgcctggcaatgatttacttcctctttaaaacgttgcagtcggaactggcgccactggaagaccgcagcactttccgcctgtctattaccactccggagggcaccgcattcgattacatggataattatgtggacaagcttactaagttcatgatggactctattcctgaaaagaagatcatcctgagcgtaacttctcccggcttcagtgggtccggtgcggtaaacaccgcctttgccaacgtaatgctcacagagccgcacgatcgaacccgctcccagaaagatatcgtgaatatggtaaaccggagcatgaacaagtttccggagggtaaagtttttgccatcgaatcccagactatccaggtaggccgccgcgcgggattgccggtgtcttttgtgttggaacatatcaacttcgacagtcttaccagggtgctgcccaagtttatggaagaagtgggcaacagccctgttttccagggaacggatgtggacctgaaattcaataaaccggaactgcgcatacatattaaccgcgataaagcaacacaactcggcgtatctgtacaggatatatcctccacactgcagctggcactgagtaacctccgctatggttattttatcaggaatggtaaacaataccaggtaatgggacaggtgttccgcgccgaccgtgatgatccaatggatctgcaaaacctttatgtacgtaactcacgtggcgaagcgatacagctcgataacgtggtaagtatagaagaagaaaccagtccgccgatcatttatcactttaaccgttacaaatccgctacggtgtcagcaggattggcgccgggcaaaactattggcgatggtatcaccgaaatgtaccggatctataataaactgcaaaatgaaagtgtgctgaatgaatcctttaataccgccttgtccggttcctcccgcgactatgcggaaagcggctccaatactatgtttgcattaggactggcattggtactcatttacctggtattagccgcacagtttgaaagctgggtggatccgctgatcatcatgttaacggtaccgctggcatttgctggagcgttgctgtcgctatgggtatttgaccaaacctggaatatcttttcgcagatcggtgtaattatgctgatagggctggtaacgaagaatggtatcctgatcgtggaatttgccaaccatcagcgtgataccgggatggcaaaagccgatgccgtaatccatgcctcctcgatgcgtttacgtcctatcctgatgacgagcctcgctatggcgctgggtgcattgccgattgcgatgtcgctcggcgctgccgccaccagccgcattccgctgggaatcgttatagtgggtggaatcatcttttcactggtgttaactttatttgtaattccggcgatgtataccttcctgtcgcgcagaggcagaaataataatactgacgaggaagacgaaatggcaaacaatgaggaagcacaggtagcagcagcacatgcctgataataacagatttgaatgatcacgattatgctatttatgatgaaaaatataaagaagtgtttcttcttattcctgttactcctaagtgcgggtgcgttaaaggcacagcaacaggtgcttacccttgaacaggcaatagatgtggcgctgaaaaacaactttgatatccgcctggccaggaatacagctgaactgtctgctaacgactacgcctatgcgaattttgcatttgtaccgcgcgtgaatgctactgcaggtactacctggaatagcaccgctaccaaacaggagtttgtaaacggtaccaaacgcgataccagcggcatcaagggcaacaatctcactggcaacgtaaccctcagctggacgttgtttgacggtttaaagatgttcgctacacgcaataaaatagcatctatccgcgacctaggggaactggccataaaagaccaggtgcagaattccatctccactatcatcggcggatactataacattgtacaacaaaagcaacagttgaaagccctggcagagcagatgtccatctccgaagaacgggtaaaattgtctgacgccaaattcagtacaggtctcgcgcccaaaacggatttgctgcaatcaaaagtagacctgaatgcgcagaaggcattatacatccgccagcaaacgctgatagaacaaagtaaagccctgctgaaccagttgatggccgtacccgccggcgctaccggatatgacgtggtagattccattccgcttaacagcgggctatccttttcggtgctgcaacaaaacattgctaacaacaataccgctattaaagtacagcaacagaatgtgaatatttctgccctgacggtcagggagcgtaaagcagattacttcccggttatctccttcaattcaggatataattataacaggaatacctccaatgctgcatctaacgcattcagtccccgtttcagccggaatgccgttttcaactacggcttcaccgctgctatccctatcttcaatggatttaatgtaaaaagacaggtgcaaaatgcgcggatcgactttgatttccagaatatcacattggataacgtaagatcccaggtagacctgtcgctcaacaacgcgttcaaagactacgaatactataaaaaacaagtgtcgctggaagaagaaacaaacgatcttgccagagagaatgcgatggttgcgctggagcgcttcaaacaaggcgtatctaccattcttgaagtaaaaatagcgcaacaaagcctggaagattcctattaccggcttatacaggcgcgttataataccaagcttgcggaaacggagctgggtcgcctgaacggcgcattgctgcaatagattatttttttatatcagaagcggataagtaagggagatatatcctgcttatccgcttctttttttgatcttatcatcaactgtacgggcatgaacaggcacttgtatcattaacgaacacattaaataatagacaatataaaaaggattaccactcaaagctgattcgtccggcatgattttgcaaatatctccaccggattataaaacacgatacacatgttacgttacattatgcttactttaagcggcattatctgctttacctacatatgtacagcccaggagctgcgggtggtaaaccgcgcaatggtcagtgactccattatccatttgaacgaagcgccaagcgcaggaatagcctggattaaaaataaacaatttgccagtggcactattgagtttgatgtaaaaggaaagaatgttttgcaacagagttttgtaggtattgctttccatggcgtaaacgattctacttatgacgccatttatttcagaccgttcaatttccaggttcctgaagccggcagaagagggcacgcggtgcaatacatttcacttcccggaaacgactggccatttttaagagaacaataccccggaaaatatgagcatgaagtaaatccttccacagatcccaacaaatggtttcatgtaaagatagtagtaactgatacggaagcaagtacctatctgaatggcgaaagatgcttaacagttacattactcggcaaacaaaaaacaggaatgattggttactgggttggtaacggctccggcggggactggaagaatctgaaactaaattaagattgttgattgataagttagaagtcgggctttgagaacatgtgttcttaaagccttttttatttggtgtttagtcacatagaaaagtgcgaagcttagtttcgacataaatcccttctgaaaaggtgtctacaggatatactacttccatctctgtataggcatctttggggatgcaaagatgaagaatgttaagtcttaccagaagttcatgggcagcgtcagcgtcactgctaacaagctcctgctgttctttaagaatctgtagcatctcattgtaatctttctctgtcatcttataaatttatcaaccaggaaaatcagatctcgtcaaaccttttagggccggtatttcttaatggaacccgaccttgccagtgtatgtccttcacagggttaaaatagcctctgatacaattaggattccggacgcagatctgtatgtggtttttatccttaaatcccgcgttagggtaaagctcattaccttccatgaaaacacttctcacagaatcgtagggtattaaattcttcatttgtctgtcgatatgcaggttctcaattactgcacaatcgagatttcttaacaataaatcctgtgatcctcgtgccggcatattcacgggtagcgttcttttatcattaacaacagctttgaacaatgcatgataggattcacgtacaaggtttaaacatgttgcatccagcaaatcaagacagaacttcagatcaataactgctcccaataccgccggtgagcggattactttatttcccggaggattacaggcataatcatatgcccgttcataactgttctcccagaaatagcagccacttcccagccaatcatatggcttactgctgggactcattctaatactccctctcactaatgcgtctcgtacgtcttcttcacaaccgtgaaaaccaagcaccaatccaggccgtgttgcgtgaatcatttccatgatagattaacatgaacaataaatcatagaaccagactataactgaatgaatagatcagtttaacctgccctttgcaacatacatttactatagatggaacacctgttgttgtgaaagtatttccggtaataaaccagcgaacaacgtcacaatttattattttttccggataaaataaacacaggtaaaaaatactttcgtttgctacactaaaacgaaatctcaggaaaggcaatgttgatatgagttgtatcaaaatgatactaaaaataaattttgaaaaatgaaaagataaaaataatttttaggtaggaatcttaattaatttttcatcaattaaaattaattgcataatttagttttcacgtttgttatcaacaataacttcaagttaactcctcaccaaaacatatcctcaactctttcaactcatttagtcatggcactgtatacaaaaacaaccatatcagtagacgaacaacagttcagtcaattcaacttcctgcacctgaaacaatacatggaccagcaccacgaatttgagatagggatacaatacgattggctatcacaatacggatcgaatgcggttgcagcaggcaggtcgttactgggaaaagaaatcagcatctgtatccggcctgtcgaatccctgggaacatttaaccagttgctgtttaatggtatcattacaggagtccacgccggaaaagaaaataatggcaataccggcagctgcatacttcatggcaacagtcctaccatattgctttcaggtaatccacatatgcaatcttatgagcaactggccttatcatccattgtaaacaccgtcatgaaaaactgttatccctttgctgcgcatccgcaggtgaatcccaatttcacacaaccgctgaagtatattgtacaatacaaagaaaccggattcgactttcttcagcggctttctcagcgttttggagaacatttcttctacaatgggcagcaaattattttcggtcagtacagctccccaaaaaacgacctggtacatcagaaagacctgattgatttccagctggaatataaagtttcacccatccatcaaacgtttcaaacatatgaatacaggttacataatatagtagcggaagatagttgtaatgcagccttcggcaacatgaaccatcactcgtatcacgcgggatcagtgagcaggaaactgtatccttataaaaccagctataaagtaccacatgtatttggcaagaatgccgccgcagaactttctgcatttaccaatcgcttctataaaggacgaatagcagaattggttttcataaaaggcagtagcaggaataccggtctgtgtatcggaaacattattgacgtaaaggaacagctatccgcccgtgaagatcatggtgaatttatacttacaaggctggaacaccattgtaatgggaatggcgactattacaatacatttgaaggtattccggccgatatagcagtacctgctatgaacctgaaaaacatgccatattgcgaagcccagagcgccttagtaacggataacaatgaccccaaaggtcttggacgcgtccgggtaaaatttaactggcagcagggaagtacgccctggatcagacttcatcaaccgcatggcggaatcaataaaggtttttactttattcctgaaataaatgaagaggtatgggtagatttcgaaggcggtaaccctgaagcaccatacgttaccggctgtgcgtacaacggaaaagcaactgctgccttcggggatccaatgaataacattaaagcaattaaaacacgtagtggccacatgatccgcctcgacgatacagatggcaacgaaaatattatcatcaccgataaaggtggcaacatgatcacgatggatacccagggacagaacatttcaatttcggcgcccgaaagaataaacctaaccgccaaaaatatcgacgttaatgccactgaaaatatcaatataaatgccgggagtaacatcaaccactccgcagggatggatattcttcaacaggcaggtaactgtctttatcaatatacggtgaacgattatcaattaaccgcaaccaatatcacaaaaatagcgatggaaaatatcaacctgcaggcgagagaaatagataaacatgcggaagaaataaacatcgacagctccaaagaaaacatgcagataagctcaggaaagtcagtcaatataaagagtacagaaaagtcaaaactattctaaaacaccaacaaatgcgagatacccccacaggaggcatgctgattgtctgcaaaaaatatatagaaacagggaagagcattcgttggcatagttcaggagaactgtttcttcattccggcaaatcagtaatcatcaacggcaaacagaagggtgtaaaattccataaaatatcatcagacattcataatcctgaaaaataaaattgcattaaaaagatggctgataaacacgttgtggtgcaaggagcattatgcagatgtaatttcggtaatgctcccgctaaaatacaggtttccgcaaatgcagaatacatgaacgacgtcagtggaaactccaaaccagctgcaggttccaatgagataggcaatcccttcatgccaggcacatttggaatgtgcatgttaacccacaagccttgcacgcctaacatcattcaatgggacaatgtattgcccggcgttacactttcgaacggagggaaaatactaacagaaaaaagcactgctgtttgcgcggcagccggggctccttgtgtttgtattatccatcacggtcaaacagcttatgtagctgaggatagcattgcggaaaatgaatccgctattataccggcgctaaatcccctagttgccagccgtttgaagtgcagggaagttcctgccatacgcacaattaccttatgtattgaaaaacgtaaccctgcggcaatctttaccagtgaaaagaaggaggaggtttccgtcaggatcatggagccgttattgtttgaggttgaaagctattataatcatgtgatcccggacgaatcagcggtacaatggaaagtactcaatcttcacaatgacggcaacgatgtggtgttaatcgaatcatccggctcacggttaacattttcattcgatgcatccgggcactacagggtacaggccttcggaaaagaacaaacagatagcgatgccttcattgatctatatgcgaataacaacacgcttaaagaggaattcatcattagtgaaacaccttataagtcaggctacctgcaaagtggaactccggtttgtgcagaagctgtatacaagataactcccccaactgaagcagaaagagcgctggtgtctatgcaagtaaccgataacagcaaaaacataattgccatatccgataatgataaaatctggttcacgcccaccaacgcatctgccacttacgttgtttcagccatcatgcgtacgggtatacatccgcaacagatccgcaaagaaatccatacccaaaacaacggggccatatcagtgagcaacggggcgtcaacacatgtggtaaggccccgcacaaatatgaatttccacgtttcacaaatgctgcatactaaactgccaccagtacctccagcagctattcaatggttgttaaacggccggccagtaggcatagggctccacattacaatcaatggcgatgttcatcttatacttcccggaaagtatacagtagaagtacgtgtaaatatcatggagggggagcgtaataatattcaacaagcctattggcactttgaagtaaaaaacaatgaagtattaaagatgctggtgccgggagatagtaccaactggatcgttggaaggtattatactgtttttgcgcaaacactaatggattatgaggaaacactcgatggccctgttttctggaatccctatggagctcataccaataagatatcaactgcatcagcttcacaggaaggaagcttcatgatcagtgcccgtctgggaaattcccggaaaacgctcagtatcagtgccataaaagccacgctcacacgttggtgttttacggatgagcaattaatttatagaccatcggctggttggcaggagatagtccgtatagttatcagtagccatgaagcggcaaatgaaaagataccgcttcacctgttgcagataaatcctgcaaactgcattcatcatgtaaaggatctgggagaggtggctttcaatacggatggactattgcaactcgatgttagcataaatagcctgaaaccattattaactaataccagtttcgaatgggatacatttcgcctgttgttcgcaatacctttgtctgctaattgcatccggtttgctgaaatgaaaaccattacctgtgaaggaacagcatactgggtgccgcaaaagcaaagcaacaaacgtatgcaggaaaagggagggtacctggagctcaataacaaacgacgtgtagtatctgtacactttcacgatcagcgtaaatatcctgcctataaagtttacaaatacggacagaaattcagcatgctcgtacaaaccgctaaccttgccggagaggaattatcctttcagatatgggaaaaccggtatcagggaaaagataaacattggttcagcggcaggttgcatataaatgaatatggaaccgcaaatgcaacaatagattcaaaccagctgaaagcggggaatacactggaagatagttttctccgctgcttctatgcagtaataaagtcttctccggataactatttctatccacatgagatagcggataaaaatatcctgaaccctgataatatcagttactaccagcatataaaactatccaactggtttgataattttataaacaggcattccagggcaaatgcaccggtagtactgggcgagcaacttgaaataaatgagcttgactccaggtgtccggcatgcgaagagatgattacgatagaacagctggctaaaatattccctcatgcaacaacctcctcattgcagattgcagccgccacttacaacaggtttatggaacaaaccggtatgaatacctgctggaataaggcacactttttcgcccaggtggctatagaaagcggtggatgtttgaatgttaaagaaggagaaagcttcaactggtattgggaagacctgggaaagaactttcccccattcagaacagcggcaggtaaaataaaagcgaaagcatgggggagagcgataagaaaaccggctcgtcctggcgtaacaaaagaaaaccaacggcatattgctgattatgtatacggtcccgattcggtaaaggggaaatcattgggcaacatacaaccgggagatggatggaaattccgaggcaggggactgatccagcttaccggccgggaagcttatacttatgcaaacaagtttacccggaaagaaaaggccgatattcttcttcaaccagacctggtagccacagatataaaaattgccgtactatcttcaatggctttctggaaatggaagggattgcagcttgctgctaatggcaatacagaagtaaccgctaaaataagcaaggtagtaggcctggatgcgatttcaaatggcaagagttcacatgctgaaaagaaacatttcttcgacacaaattcatctgtcttattccaggtaaacaactgccggcatcgaaaaatatccgaaggtgcattgaacaggtatattgtcaaaatagatgccttcagctacacactggtggaacaaaatgttacttccaatcaatacaaatacgacctgtacaacgccggtacacatattaaaacattcttgctgcaaaaaaacagatacggcctgctgccattccccgaaactggtcccaactggggaagatacggcaccagggatggaggagatgataattatatagctcctgatattgccgctcctttgtttggattcttctattcgttaccacagaatggctacacagatacactttattataacgatatctccgccggagacaaacggaacataggtcataaaggacatattaatgggaacgacattgatatcaggtaccccggaagctcaaacaggaaaggatctgtattatggacggaagcgatggagacatatggcagcgaaaaagaatttctgaaagtgttggagaagctactcaacattgccactaaatgggaatttagaaacaatttcgcttataacaaacgtattaataatacgcttggcagttctacaatcgcacatcaagatcattttcatctcggtctcaggaaaaaaataaaaaaatgagaacagtaaatttaatactgatagtctttatacttagcaatgtaagctgtcaaaacacccagcagcaaccagtacaaagcattggaaagaataacgttatcaaaaaagaaaaaatgtacaccatgaatatagacgccattaaacgacacatagaatggcaatcccacatagaatcaacggaggacggaatacctgcaagctatacgtatacagagcaagatgttaatatcgctttacctattattgctcaaggtttaaaagacaaagggtttaaacagctcagcgatagttcttttaataaagcgctgaccgatatatttggaaaaatacttagtcgtaaaaatgacggagtcaggtttcataacaaattcaatactattattgaagaaggatacgaaaaagaagatgaatatgactatacaatcgagaatatcttcgtttccatagaatacaaatttatctcctgggttcctctattaggggatttcattgaatttgaagataacaacagttataaaattgatctccatccaaaaataatctcacgcaacaaatacctcttcaacaacagccaatcagatcttgcctatcttctcgccgaagatacgctcttcctcaaaacactggtcaaatcattcggctataccaaagaagaaaagataaatacgctggctatgaacgattacctggatctcgacaataatcacatgcctacagtaggcgagatcatctttgtaaaaaacgcagaaggtgtgttagaaataaagcaggaattactacaatggatttcggatcatacccgtgtcaatgataacgccttgcttcgggcgctggagcaatacgcctattctttatatagcaataccagtaacgacatattcgctaataatccctttgaaacattttcgctggatgaaaaaagaaaaattgtggcctatatcgccaatatttatgaaccacttcagcaccagcttatgcctaaaaatccaggtatatggccgggttcatcggtactggaaaatatgcttaacgaagacaaagggctggaggattttctcaaacaacatcgctatttttcattgccggccttaaaacaggaattggaaccagctgattaaaattcgtgggttcgccgtcagcataccacatggtaaaaacataaatattaaaaaaattcatagcagatataaacaattacgccggagataactctccggcgtaacattatttaaggttctttcttttctatctttcgcttctgatattcttcaaacgattgttttatataaagtaacagatcgtagtctgaagcggaatttaaaaactggtatcccggcctgtatttatacataaacgaatccagttccgggctctgtagcttggtcattcttcccaccagttcaggagagtagcgatagtcgatgaacttctccttctcccaataaaccagctgttcatgaaactgctcttttcttttacgcactttacttggcactagataacttaaagccgtaatagggtttgccggcaaggttttaagtacatccatcgcccccggcttacggtaatcaaagtatcgtccatattcatctctcagcgccatagaatcgttacggtagttcttaccccggatatttaccccctgcaattcaaacaaccgcttctgcatatatacatcctgggaagctgacattcccggaacaagcaacattttaggtgtatagctcaacatggaaaattcaagggtatctcccggcagtgcctcaatataaaaacggccattttcattacttaatgtgcccgtcattgtcctcttgttaacaatagaaacaaaaggcaatcccgttttggaatcctgatccgccaccataccggacaaacgcacctgtgcgaaggttccctgcatgttaatgaaaaagaaaaaaaacagtgctccgatatatgctgtaatacgaatcatgaatatactaatccttcaaatttaatgttccacccgcaaatgaaaagttaaaaaacgggagaaatatgagtgctcagcagcaaaattattaattatcaacattataaatatccctctaatcacttatttttacggttatcacccattattgtgtaaaagtcatgccacagaaaatcatctttgctacccaacattatcagtatctgaaaaacaggatcctctcaattgcaggctccacctgggaaaatggggaattagacatacgtgatttccccgatggggagcattatcaccgcattttgagtaatgtcagcaacaaagaagtgattttgctcggtggcactatcgacgataaagaaacgctggaactatatgatctggccagcggttgtatccagctgggagcttattccctgaccatcatcattcctttttttggatattctactatggaacgcgccgtaaaatatggcgaaattgtaaaggccaaaacacgcgctgtattgttttcgtctttacccaatacctcccgtggtaacaggatcgtaatgattgatcttcatgtggatggtattacctggtattttgaaaacgatgttcgcccggtgcatttatatgcaaaggaatttgtaatgaatacggccatggagctcgcagccggagagccttttgtgctggccagcacggatgcgggcagggctaaatgggtagaatcccttgccaacgacctgcatgtaccggcggctttcgcgttcaaacgccgcctttccggcgatgaaacagctattactgccattagcgccgatgtaaaagacaaaacagtgatcatctacgatgacatgatccgcaccggcggatctctgatccatgccgcacaatcttatcgtgatgccggtgccggaaatatcttcgttatcaccacccacggcatctttgcaggaaatggcttcgaaaaaatcaagcaatcaggtctcattaaaaaggtagtctgcacagatacccatcccaatgccatcaccatcaacgacgatatgttgcttgttaaatcagtcgaccagctgatcgtcaattattttcagtcacagcactcctgattcctgttggcaggctatttgtcatccagacacttgtgaaccatgcagcggtaattcctgaaattgaaatggcataaatcggccatctgcaaatctgacaaatcattatgcttgattttcgtatactcgaatacggtagttgcgactaccacaccatgattgaccttcgtagcgaggtgcttcgaaaaccattggggcttacgttttcagccgaacaattacaaaaagaaatcaatgatattttcattgccggctttacacaagggaacgatcatgaaatactcgccggttgttgtattctcactcctgtcagtgaaaacacagtacagttaagacaaatggcagtgtcgccccgcctgcagggcaaaggaataggcagagaaattgtggtattcgcggaacaatatgcacgtagcaacggctttgatgaattaaccatgcacgcccggaaagaagccacgggattctatcagaaactgggctataaaatctgtggagaagaatttacagaggtgggcattccgcactacgaaatgaggaaaaacctgaattaattattttttatttttttgcttctgcaacccattgtagaaggcgttttgattgtattgttatattgatggataaccaatataacaacagacagcataggaatcctgtcaaaaaattttgtaaccaaatctttcataatacgatgagaagccatgtactagcctggtcggggctgtgctatgcctttttctgctatacctccagcagcgcatacgcaaaacccgaagggtatctcacagcaaaacagctgcaagctgataccaccgttccggtagtgattaaacccgctgctgctgataccagtgttaaacctaaacaggataccactgctccggtagtcattaaacctgctgctaccgattccactgttaaaccgaaacaggatacttccaaaccagtaaccgataccgccaaaacggctgtagtaaaacctaaagaggataccgcactcatccttcccccggactcagctacggccaaaagcgaagttggaaaattccagcttacaggaacagtgaaagatgataaaggaactcctattcccggcgccgttatccggaataaaacatctaaactaaacgcacagtcagacccaactggtcaatacaccattaaggcggccgtacgcgatactatactcgtcacagctcctactttcggtgaacagtctatcccggtagaaaaaagaggtgaactcgatgttaccctggttccctccaatgctaccaaaaaagttttgggagaagtagtagtcacggccctcggcattaaaaagaatccccgctccgtaggttatgccatacaggaagtaagcggtaatgccgtacaggaagcaaaagaagtaaactttgtaaacgcccttacaggaaaagttcccggtgtgcaaatcagctctaacacaggttccatgggcggtgccagcaaaatcaccatccgtggggtaaaatccatcctgggtgataacaatgccttctttgtactggatggtgtaccgatgatcaataacgtaacaaacgatcccggacagcaaaacggtggcggcggttacgactacggtagccctatgcaggatatcaacccggaagacattgaaaacatctctgtcctcaaaggcgcagctgcaaccgccctctacggaagccgcggtgccaacggcgttctccagataaccaccaagaaacgcccggataccgaaaaaggaatcggggttacctatagcctcaacgcccaggtagaccaggtagctgtactccccgattatcaaaatacttacggcggcggtagtgcaggaaaatttgataccctctattacaatcagcatccggaaggcttcctcaatgaacaaagcgctacctacgacgacaacaacggcaaaggacgctacgacctgatgccacaatatgcagtggatgaatcatgggggcccaaactgaacggacaaataattcgcccttattggtcatgggataaggataaaaaaaatccatacttcggcaaaactgatacctggtcaccacatccaaataatgtaaaagacttctataaaacaggttttacacttaccaacaatatatcaatggcaggcagcgacgataaaggaagtttccgcttgtcgtatggtaacatggatcaaaccttcgtactccccaatgccaccaacaaaagaaacaatctctctttcaatggtagctatgaattaacaaagggagtaaaagccgtagcctccatgaactacacctccttaaaagtaaaaggccgtccaggtaccggctttaccggtcccaatcctacattgcagttcacgatgtatggtcagcgccagctcgatctggaaatggagaaaagatacaagtacgatgacggttcccagatcacctggaaccgccggtcatgggacgatccaactgtttcctccagcaatggaccatactggaaccgttatatggattacgaaacagatagccgcaacaggctcttcggatctgccggactggatatagacgccacaaaatggctctccttctccggtcgcgtattcatggacgactatagtacactcgaagaagaaagaacagcaaaagattatgcaataggaggatatatcaaacgcgtgagaagtaaccgcgaaatgaactatcagttaacagcagatatcaaaaaagatttcggtaccgacttccagctgaatgcaacagttggtggaaacgtgatgcatcgtaaatggaccgttaccggcggaagcgtcgtgggtggattgatcactaaagatgtgtacaacctgctcaactctgcgcaacccgctcaggccattgatcagtactacgaaaaacagatcaactccgtctttgctaccgccaacctgggatataagaacctgctgttcctcgacctcacgggtcgtagcgactggtcctctaccctggtaaaaggtaataaccaatatttctatccatcggcttccctttcctttgttttctcagacctgttgaaagaatggaaatggctgtcatttggtaaattaagaggtagcctcgctgcggtaggtaatgatgccgatccgtaccggatttacaacacatacgacttcattcctcctttcggcagcaatccggttatccagttctctccaacattatacaacgaagacctgaaacctgaacgtaccacggaagtggaaacaggcgtggaattgaaattcctggataaccgtgttggtgttgatttcacctactacagacgcgttaccaaggatcagatcatcacactggcactgcctacagctaccggtttcacaggagcctacgtaaatggtggtagcgtggaaaataaaggtattgaaatagggctgaacctgaaccccatccgcctgaaaaatggcttccgttgggatatcagcgccaacctcgcacgcaaccggaacaaggtgctcaacctggatattgcacagtacaatacatcactggacttcctgacaatcggcaccgaccgccgtacacagaaggtatcggtggtaggacaagtaggagagccgctgggaactatccgcggtaccgattatacttaccttaacggccagaaagtagtagatgcgctcggacgttatgtgcccagtgaaatcaaacctatcggtaacgcctatcccgactatgtaggcggtgttaccaacacctttacttataaaggtatttacctgtctgcactggttgatttccaacacggcggcgatttcttttcctatactaacctatacggaaataaatccggtctgctggaaaccactgtagaaaatggtatccgtgaaaatggtatcgtcgttccgggcgttacagcagatggccacgccaatacaacaaacatcagtgcacaggatcacttcaattacaacggtggaaatgtgatcagcaaggccaacctgtatgatgccagctatatctacctgagagaggcaaaaatcggctacaatctgccggaatcatggtataagaaaataggagcccaggccgcccgcctttctctctatggccgtaacctctggttaattaaatcaaatgcgccgaatgtagatccatccaatatcctcaattccgcttccaatgtgcagggaattgaaggtggtgcgctgccatcactccggtcttatggattaaacctgaatgtatcattctaaattttgtgaagatgactaaaaagatttttaaatatagcagcatcctgttcttgttggcttcactggcagttaccagctgtaaaaagttggatgatatgaacactgatccaaccaggccaactaccgcttcgccggcaaacctgctcacgggcgcccagaaaagcacgatggacatgctttacagcggattacaaaacggtttcatcgccatgaactatgcacaattctggactggaaactccaggacaaatgatagccagttcaatctcgatgaaggtaataatgccgccttctggaatacattataccgtatctcgttgcataatcttgatgacctggttaaacaaaacgcggctaacccggggctgcccggcgcgactaaccagagtgccatcgcaaaaatcacaagcgcctggatctaccagatcctggcagatacctacggaaatattccatatacaaaaaccttccagggtagcagtaatattacccctcaatacgatgatgcccaaaccatttataactccctgctcgacaccctgcaggcgcagataaatgtgctggacacatcacagattagctttgaaaccggggatattatttataacggagatgtagaaaaatggaagaaactggcaaattcgctgatgctcagattggccatccgcatggtagacgccaacccacaaaaagccaaacagatcattgaagcgcactatcaggatgcccttagcgataacagtgacaatgccgagttcgaatacctgaatgcagcacccaacaaattcccttataatgactctgaacgcgatatcatcgacttttctgtaagcgccaccctggtggattatatgaaaagtgtaaatgatccccgcctcagcatttacgcccggccttcagccattagcgataccatcaaaggtatgccttacggctcgtccgcttcaaatccggacaggcttcctatagacaactactcctttcccggcacacaaatatatagcgccacaatgccaggcattctaatgggatatgcagaagtagagtttatcctggcggaagctgctgccagaggcatgaatgtgggcgatgatgcggctacgcactatgcaaaaggcatcaccgcttctatcagctactggcgtacacttaccaacaacacagatatcacggatgctgctatcgaggcatatatagcgaaagtaccttacgtagccgccgactggagaaatgtgatcggtacgcaaaaatggctcgcgctttatccgcagggcttccaggcatggtttgaaagaaccaggcttcattttagcaaaccaggcggacaaccattattcatagctccggtatccggttcactggatcccagcgttacaatggtgccctacaggttaacttacctgcagaccgagcaaacacagaataaggccagctacgaaaaagccgcttccgacatcggtggcgacacaaaaggcaccaaactgtggtataacaaattctgatacaacaatcaactatagctaaacaacaatctaccggcgcctgcatctgcaggcgctttctttttttataccgatttatttatctttaaccccacctatattcaacgatcatgaggaaagtactgctaacaatggccctgctggctattgtccgtttggtatcagcacaggaaacaacacatgcctaccagaattggtatacttatttcggcaccatgaaaattaacagtaaatgggcggtgccttttgatgtgcagttacgcatcagggatggtatcagtaacaaaggtcagctgctcatgcgcggcggtctgcaatattcccttaccaaacaggatcatattttactgggatatgcatatgtgcccacttacaatgccaccagcaatacatggctgcctgaacaacgcatctttgaacaatacatccataaagcaaaaaaactggatatgacccaccgggtacggctggaacaacgctgggtatcccaaccgtcagctcccggagatccgcatgctatcggtaattggaaatatggtaaccgcgcccgctatttcaaccgcacacaactacccatccttcataaaaaagcagccaccccgttttacgtggccctacaggacgaaatctttttaaatctctggggaaatgatatcagcaacctgctgttcgatcagaatcgcttcctggttgcttttggatatcagttcaatcctaatctcaaagcagatataggctatatgaaccagctggtccaggttacgtcaggcgctaaaaccatgaaccatatcctgcatttcagcgtgttccagaatattaacctgtaacgcagaaagtcttaccggtaattactaaacttcgatttgagtatgcccgcgaaattgcggtaggcctcctctgtctggaaagcactggtgggaatgagaaagaaagttttcttatcacgatagaggaagaagaatttttcagtttccactaccctggaaaaattgctccagctgatattacgcggatgatcactcccccgggtggtaatcaataatccctcgtcagaatacttgagatgtatactgtctttaaaagtagccgccttattgtaaatggaaacaggtaaaaggtaccagaatacccagccaagcaccagtatcatgataacaataccagtaagcgcaccggtggtcaccacgctaaaaaaataacctgttaaagtagcaagtaataagatgataagggtattgcggaagactttaatctcgcctcttcgcataaaatgatagcgcaatgcatgcaacacatcccctttatcgtagttaaactctaaatgcattatcgcctggcaaaactattttatctgttaactgaaatcgacatcggattatccatttcatcacgcacagtaacaggtgcttccttcttccggctgcgttttacattagacagatcgtcctcgctgaatccggggaagttcttcttgatgaacagaaaatattgctgcaaggtttttggatctaccttgaaaggaaaagccatttccttaccactccctttgaggaagtcgtttgtatttaatttagtctcgttttgtaaataccacttgtataagtccacaatagctttctccaactctgcttcatccactttctcagttgtctctacccgcggaaacattaacacaaactcttctacccttacaggcttggcattattcgtgtttttggcgttattacggttgtcgttgttgtctccgtttttatcaccattattatccccgtttttgaaaccagtgctggcatttgctgatgcggctgcggccaaaactaccaacagcataaacaacagctttttcataaggcgtcaaattttcgagtttaaaaatacaattatattttgagatttctagtagattccaaaatatgcgtaaaaacccctgaaaaaaacaaaagcaatgggcgaaccattgctttcgagagtcatttacagtgcatgatgaatcatgcggtgtaggaatatttggtttttcataggacagtaaccataataaaaattaatacaataacaaatataataaaattatatcgtgagttaggggaaagattaaatattagaaatatattaatatttctgcacgtttttaaaaaagatgcaattagattgatctttttagaaaaatatcaaatgaaaaaaatatgttgtaaagaatcaggacctaaatattgcctggataaagagaagaaaaacaggtgttttttgaaaaaagtaagggcgcctagaaaagcgccctcaatttgttactatcctatgaaaaccctatttgaatacaaaggtaagggcatgttatttttctttgaaattttagagcctaaataacatatcattaacaagaagttgtaacatcaatcagctgcaacccatgctggtaccgcaattcaaacatttatagcaagtacccgaacgcaccgtgatatgtccacaggtattacatgccggcgcatcactttgcatacttttcaggtaatcctgcgtaccactttcctgctgaaatgctgtagccgcctgcatcctgggaatacgcggagcagcttgcccactattgtttacctttcctggcaatggaaccggcgcctcctcatccgcatccccttcacccgtattaccaggtgaatccagcacatgtaccaggtcggtacggcccaggtactcatatcctaacaccctgaaaatataatcgattagcgaggtggccgatttaatattgggatgatctaccattccggccggctcaaaccgcgtgaagacaaacttatctacaaactcttccaacggaaccccgtattgcaatccaacagaaacggcaatggcaaaacagttcatcaaactccgtaaagtagagccctctttcgccagatcaataaatatttcgcccaacgtaccatcgttgtactctccggtacgcacaaaaattacctggccacctacatttgccttttgcgtaaacccaccccgtttggatggcaaactttgccgctccacaatcctcgacaactggcgctttaaggtggtgtccctgctggccagcatccgtttgttcacttcctccagcaactcatcaatcgtcagctgctgcaggtcctgcccggcagccacctcgttcaccggctccgctttcttccttttatcactcttattgcttaaaggctgacttaacttactaccatcccggtacaaagcacaggctttcaacccaagttgccagctgagcttgtaagcatccgcaatttcttccacagccgcctcattcggcaggttaatggttttggaaatagcccctgaaataaaaggttgcaccgccgccatcatcctgatgtgaccatgcgcatgtatataccgctctccatgctttccacatttattggcgcagtcaaatacaggtaaatgagcatctttcaggtaaggagccccctccaccgtcattgttccgcacacataatcattcgccgcttctatctgctcatccgtaaatcctaaagcatgtaacaggctgaactcaagactgtaataatcctccgccttaaaccctaaccgctgcaaacactcttctcccaatgtataaacattaaatacaaacgatatatcaaaggaagaagaaacggcggtatccagctttttcagctcttcccccataaatcctttctcactcagcgactgatgattaatataaggcgcccccgcaaaattgccggttccttttgcataatccacaatcgcctttatttcgtgggaagaatagcccaggttttgtaacgccgtaggaatagactggttaataatcttaaaatagccgccaccagacagctttttgaatttcaccaatgcaaaatcaggctccacgccggtagtgtcacaatccatcaccaggccaatagtgccggtaggtgcaatcaccgtcgcctgtgcattccggtaaccatattgctcacccagcttcactgcctcgtcccatgccttggtggccgatttcagcaggtaatccgcgcaataccgtgcatcaatgcccctgggctttatctccagtccatcatacgcatcagaggcatcgtatgcggccgcccggtgattccgcatcacccgcaacatatcttcccggttctcttcataccggggaaaggcgcccagatgtgcagccatctccgcagaagttttataggcaatccccgtcataatagcggatatcgctcctgatatgccacgcgcttcctcgctgtcgtaggcaatgccgctcaccatcagcatagagcccaggttggcataacccagccccagcgtgcggtattcataactaagctgtgccacttctttagaggggaactgtgccatcagcacagaaatctccagcaccactgtccataacctcacggtgtactcaaagccgggaacatcaaacaggttactttcatcatcgaaaaagcgccggaggttcacggacgccagattacaggctgtattatcgaggaacatatattctgaacacggattagaggcgttaatacgcccgccctgcggacaggtatgccactcattgatagtcgtgtcatattgcgtacccggatctgcacaacgccaggcagcataagtaatctgatcccataaatcctttgcttttaccgtttttgtagttttgccggtactcctggctttgagttcccattcgccatcttccaccaacacccggaaaaaagaattcggtacccggacagaattattggagttctggccagataccgttttatatgcatctccttcataatcagaagaatagccagctgcaatcaacgctgccaccttcttttcttcctctactttccagtttacaaattccataatctccgggtgatcaagatccaggcacaccatttttgcggccctcctggtggtgccacccgacttaattgctcccgcggcccggtccccgatcttcagaaaactcattaatccactggaagttccgccaccactgagcttttccccatctccccggatatgcgaaaaattagtacccacaccggaaccgtatttgaagatgcgggcttcccgcatccataaatccataattccaccctcattcaccaggtcatcgtttacacttaaaataaaacaggcatgaggctgaggccgctcgtaagcagaagtagacttttccaggttgccggtattttgctccacatagtaatgcccctgtggcttgcctttaataccatagctctcaaataagccggtattaaaccattggggggagttaggcacacacgactggttgagcatactgtaggtcagctcttcatagaaaatccgggcatcttccgcggaagcgaaatagccatatctttcaccccaggcacgccagcagttggccatacgatgcaccacctgtttcaccgaagtttccctccctgaagtgccatcagcctgcggcacccctgctttgcggaaatatttctgcgccaggatgtcggtagcaatctgcgaccaggcagccggtacttccacgttattcatttcaaatactacatcgccaccgggattccggatcacagaagagcggagttcgtaggcaaactgatcgtatggactcacaccttctttggtaaaatggcgggtaaacgcaagcccattcttactattgactggattttccatgcccgtaaatttttcttagatgatataaatgagttagtatagcggagtactctaaaattaattttaaaatgcctggagcggcccatttattttgcacagattgtggataattgcgcaaacagtttgccaacacgtttgttataaagccaaaaagaaatccggcttaaaatttgtcattaacaaaacgtttacagttgcgttacacataatccgctaggtatcatgaagttcatgaatagaaaatgaattgaatgcatatttatttagcaatgtgtgttattaataaaaatattatacatttgcgacaaccggaacaatgcgctattgatgtacaataacatatacacttcgttcatcgaaagaaaggctaaaaaggaaaaggcattcgcggttttaattgacccggataaggtaacacctgccggcatcatagagattgctgataaatgcactgctgccaaagttgattatatcttccttggaggtagtctggtgatctctgatcaccttgatgaatgcgtacaacagctgaaagccagctgcaacattcccgttgtattatttcccggaagcccttcccaggtatcaaaatatgctgatgccttactctatctgtctgtaatttccggcagaaaccctgaattactgattggacagcatgtggtatctgccgctgctgtgaagaaaagcggactggaagtaatttccaccggttacatggtaatcgacggcggagcacccactacagtttcttatatcagcaacaccatgcctatcccggcagacaaggcagatattgccatgtgtaccgcaatagcaggggaaatgctgggaatgaaagtgatttatatggatgccggcagcggcgcccgtgtacctatcacagaaagtatgatcagcagggtggccagccaggtacaggctcctattattgtaggaggaggtataagagatgcagaaaaagcttacctgaattgtaaagcaggcgcggatatcctcgtagtaggcaacgccattgagaaagacctttctctcattaaggaactggcagacgccgtgcattctgttcctgtaaaagcctaaagatatagcataaaatataaaacgaatgacagcaggagacagcaggagatctgctgtctcctgctgtcattcgttttattagctgaccgctaaatacttacaggctcatcatctccttaaacttcactgcctgcctgcggcttacttcaattttttcgcccccgcgcatttccagcaacaagccgccattaaagtaagtatcaattttctcaatcatccgcagattcacaatatgtttacggtttgcacggaaaaaagtacgctcgtccagtctttcttccagtgcattcaatgatttgaggatcaaaggcttgttggtttcaaaataaacccgcgcatagttacccacactttcaaaaagccggatttcctgcagcttcacaaaccagcacctgtcgccgtctttcacaaaaacctggtcattttcagacaataaattacggataccaccagatgccgccaaacggtccttctcatcctgctgatgcagtttatggatcgcatctgccagccgctttggctctaccggtttcaacaggtagtccagtgcattgtactcaaatgctttcagcgcatactcatcatatgcagtagtgaaaatcacctgcggcgttttctccagctctgccagcaaatcaaaacctgttttatcaggcatctggatatccaggaacagtaagtcaggatgaagcgtttctatcttctctataccatccttcgcgttcacagcttcccccaccaccactatttccgggtgatctgccagtaattttttcaattcacttctggccaggcgttcatcatctattatcaatgcttttttcattggcaatatgaagtttggttgatgatttaattgatttaaaaataatagctataaccagttaatccggctacagcagtttataacaagtgatttagagcaagggcatcactacagtagcttccaccgtttgctcatctttattcctgatttcaaaagaagccctgctgccaaacaaaaggctcaaccgctgccgggtgctctgtaatccaaagccatgcccgttcatattgttttctataatctgaccggtattttcaatggtaattacatgctgcatacccttcagggaagaatgaatataaaccgagcctccccggatgatccgggaaatcccatgcttaatggcattttccaccaacgtttgcaacatcatcggtggtacctgtaactccagcgtatccgggtcaatctcatacttaacactcaaacgctcctcaaaccggatatgttccaatgcaaggtaatcctttactatattcaattcgttttccagactcaccgtttccgccttctccgtttgcatagagctccgcaggatattggaaagctctgtgatggcagttcttgcccgctgtgggttttcatctaccagcgcccggatactgttcagcgcattaaaaataaagtgtggattcagctgcgctttaatcgttttcaactccagctccttcacagtagtctccagctttaactgatccacctgcgaccgccggttcctttcaatgtaatgccatatgaaatatagaaaccaccagatggtagtgatcaggaaagatcctacaatccccacctggatgggcgtatccgataagtgtaacaggtatattccaaaaaagtaatatccaatatacgacaccagccccgaccccgtcattaacccgataaacagcagaatctggttctcaaaattataattcacccaggcaaaccgatggatcaggttgcggaaaagatgagtggcgataaaaccgaataacacaaaaattaccagattcagataataagccgcgtccggagacgttttcctgtaaacagaaaaggcgaagaaaacattgatcagaaaatatgccgaccaccccaatatctggcaccaccaatatttgtttatttgtttaaacattcaatcaaattagtaaacttcacctatattccaaaaataccctacagcgcccccagcagaaacctaaatgttataaatggtgaatcaaaaaaggtaaatggcagatggctgtatctgaatggtgaaatatcacagaactgtcctattttcctgtcatccttacactatttaccacatatttttatgtatttttgttacttcatataaaccctgagcccaattatgaatataaaggcaggtcaactgttgagccagatagaatatcccgctgatttgcgaaagctgaataaagaacagcttcaccaggtatgtgaggagctgcgtcaatacattattgacgtggtaagtgtgcatggtggccacttcgcggccagtctcggtgttgtggagctaacagtcgctttgcattacgtttttaataccccctacgatcaactggtatgggacgtgggccatcaggcctatggccataaaattctcaccggtcgccgggaaacatttcctaccaacaggaaatataaaggactcagcggatttcctaaaagagatgaaagccgttacgacactttcggcgtaggacattcatccacttccatctctgccgcgttaggcatggcaatggcttcccactacaaaggcgaattcgaccgccagcatattgcagtaatcggcgatggcgccatgacagcaggtatggctttcgaagccctcaaccacgccggtgtggcaaacgccaacgtgctcattatactgaacgataactgcatgtccatagatcctaatgtgggcgcgctgaaagaatatctcacagatatcaccacttcccccacctataacaaggtaagggatgatgtgtggaacctgctgggcaaattaccggtaggaaagaaatttacccgcgacatggcctccaaactggaagccagcctcaaaggtgtagtgtcaaaatccagcaacctcttcgaagcactgaagatgcgctactttggtcccattgatggacacaacatcaccaaactggccgataccctgcaggacctgaaagatattcccggtccgaaattgctgcacatcgttaccaccaaaggtaaaggctatgcactcgcagaaaaggaccaaaccacctggcacgcaccaggtctcttcgataaaattaccggcgaaatattcaaaaaaccggtcaccagcccgcaacctcctaaataccaggacgtttttggccataccattattgaactcgcagaacaaaacgataaaattatcggtatcaccccagcgatgccttccggctcttccctcaaatttatgatggagaaaatgccgcaaagagccttcgacgtgggcatctgcgaacaacacgccgttaccctctctgccggcatggcaacgcagggcatgcgcgttttctgtaacatctactcctctttcttccaacgtgccttcgatcaggctgtacatgacgtagccatccaaaaactgccggtgatattctgcctcgacagggcaggactcgtaggagaagatggacctacccatcatggcgcctacgatattgcttacatgcgcagtatccccaatgtgatcatcagcgcacccatgaatgaggaagaaatgcgcaacctgatgtacagcgcacaactgccggaaaatgatatgccttatgtaatccgctatccacgcggacaaggcgtaatgccggagtggcgtacgccgtttaaagccattaaagcaggtaccggccggaaaatccgcgacggaaaagatatcgcgatcctctccctcggacacaccggtaacttcgtggctgaagcatgtaaagaactgattggagatggcctgcaacccgctcactacgatatgcgttttgtaaaaccactggatgaagcaatgctgcacgatatcttccagtcgttcgacaaaataattaccgtagaagatggtacaattgtaggtggcttcggtagcgcagtcatcgaattcatggctaacaacaactataaagcaaccgttaaaaggttgggcatacccgatagaattgtggaacatggcaagccggacgaattataccgcgaatgtggttatgatgccgccggcattgcacgcactaccagggatatgttgaaagaaaaaattaccgtcactatttaataaaagaatttagttatttagctacctgaatatttaatttccacaggaattgaatattcaggtagctaaacttttttataccatgtactttcagctcaggataacggagatcatacgcgaaacacccggtacttatacttataagctggaaaatacatcgccggagccactggaatatctggccggacaattcctcacctttctcattacgctcaacaacaaagaatacaggcgctcttattcttttagctccacaccaggtgtagatccctttctgtcggtaacgatccgcgaaaaagaaaacggcgagatatcccgccatcttatccatacctggaaagtaaatgatatcgttactgcactggagccctccggccgcttcacttacgaaaagtcagatactgcagaaagagacattttcctgctggccgcaggaagcggtataacacccgtattctcgctgctgaaacatatattaacaacggagccgcacgcgcatgttaaactgatttacagcaacgctgcgcccgaaacaaccatcttctatgaagcgttgctggcgtggcaaaaacgttacccgcatcaactggaatgtatctggcttttcagcaatgatccggatagtcaccatacctacagaaggctcaacaatattttactggagcaactggtgaacacgcatatccgttatcaccgggagcatgcacagttctttctctgcggtcctcccgattatatgcgcaccatcctgcttacgctcacctttatgggcttccgggaatcacaactccataaggaaaactttgtagtgaatacagatgcacggattgccaaaacaccgttaccgcaggatcacgatccgaaacaggtaatcatccgctatcgcaatgcagagtataagctcgctgttcccgcgaatcaaaccatccttagctacgccctcgccaatgaagtattactaccttatagttgcaagggcggtgtatgcggttcctgcacagcgcagtgtgtgagcggcaaagtatggatgccggtaaacgaagtactaacggataaagaactggccgaagggcttatacttacctgcgtcggatatccggcaagtaatgaaataatactagaattataaaatcatataatataaaaaatattatcaatcataacgatctgatattattttttggattgctaaaattttagctaaattatgtggaaaatcaggtgatgcggaataccccaatcccaataaagcttacttgcttatcgcttctgattgttgttatcattattaacagctacctcctgtttaaaaacggtttccagcattcttcattattattgtcactcagcatactaacgctttgcagtgtatgtgccctgctgatcgtcgccacattcttatcagacaaacgtccccttcagttcgaacatctctttaatgaatatcccatccccatgtggatctacgaaaaagccacgatgcgctttttgtctgttaacaatgccgcggtagaaaaatatggttatagcagaaaagaatttctggatctaacgttattggatatacggaatgaagaagatataccactgttggtagaaaatgccgcggagcggtgtaatggagatgaatacaggggcatctggaaacaccgtaaaaaagatggcaccaatttttttgtggagatatactcgcttcctgcagtatattttggtaaaaatgcccgcttcatcatggccagggatgtggatgcacaggtgaaagccaccagagaagcgcgtgaactgggtatccgctatgaattacttgcacaggcaaccaacgacgcggtatacgacaaaaacctcctgacaaacgttgttacctggaaccacggcctgcataatcttttcctctataacaaccatgatgaaaccgacctggtgcaatggtggcagaataatattcacccggcagatcatgccaggatcgttacttcacttgatgcctgcaaactggcacacctgaattactggtcggaagaataccgctttaaatgcgcagatggcagccataaatatgtggtggaccgggcattcatcatgtacgaaaacaatatcccccatcgcatgataggcatgatacaggatatcgacaagctcgtaaaacaagccaggcaactggaagaacaaaatgaaacactcagggaaattgcctggatcaattctcacgaaatacgcaggccggtagtatctatactcagcatcgcagacttatttgataaaagcaatcaggacctgcatctcaacacccagctcatggaatggctgcatgaatccacccttcagctggatgaaatcattcataaaattgagcataaagtaaaagccctccaatagctatacctcacaaggtataaactggttgaagtcttcctttagtgataaatataatttccggaaaatctccatacggtgctgtatggtttgaaagtcatcaataggacggtcgtcatgcaccacggttaccggcgtgttggccactcttttagcgcattgcttgatgtcatgatgcatttcatcagctacttcgcgctggcgcagtaaacggttttcaaaatgttcaacctgtgtcattatatccctggaggctttgctgagggcgatctgttccaaccgctcccgcatcatttttacttcagttcttacttcgtttacttcttctttccaggaattcaactgctggtgcagttcttcagtgggagttgtgatttccatggtgtattgatttatcaatttaaatgatgattaaaaaactattcatcataccaaacgctgttgtcaatatccatattaatttaccagaaaagacctcttccaaggtacaatctttttctattcaacccctcacttttgcacttctttttacagataaatgccaaactcaggaaaaaaagccatcgcctccaggatgccgccggcgcccggccgctgtgcctgcaatacgtgcgtcattcctgcagtgcgcgctattaattcgggctccgaatcacctactaccacacctttaaatccggtttcatacatggaataatcattcatagagtccccggctaccagcacattctgatgcggcaatgccagcacttgcaacagctgtttcaaggtaaagcctttgttcacaccggaaggtaatatgtcgaggtattttccggcagataaaatcaggtcacattgcagcgatgccgcaatttcacgggcgccttcaatatctgtactatcatcataatagtaagaacaccggtattgctgatgtgcttcctggtgcagtaatcccttcactgttttcaatgtttccctcacgtgatcaccgggccatttggccgcaatgtgcgactgcaccggctctaccgccgttagcgtaggcaaatgggtaacagtggcgcctacgtcgcaaataatatattcgggccgcggtaaattattattttccagtaacgataatacactgcgtatgccccgcccggttacaaacaccagctgtatatctttctgctgctgcaataaactatatagttgttccttatctgccgttgtacctcctaaaaatgtaccgtccagatctgtagctaataacatgtgtcctggttgctttaatgatttcaatgaatacggatgccgataaaaatataaaaaaaagaccagccgtaacgactgatcttcttttagatataatgggttagtatataacgatgtgattagttcagcattggtacatctatcagcaaaaactctgccggtttgattacctcaatacttactttgttatattcagataacccgatcgcatcacgtgttgttaatgtttctccatctatattcaattcaccactgagcaaaaacaggtaggttcccatgttggtggccttagcggtaatgtccagtgttttgcccgcttcatatttacccagcgtaaaccaggcatcctggtttaaccacaggccattggcttctttatccggtgaaatcaccacctgtaaagcgttttcacgcgcggcaggatcaaatgtttgctggtcgtaacggggcgttacgttcctttcttttggaattacccagatctgcaggaaactcacttcttccgttttagatgcattaaattcagagtgcactacacctgttccggcactcataatctgtacatcatttttacggatcacttctttattacccgtgttatcgctatgggccagttcaccatccaacacaatagatacaatctccatattatcatgcgggtgggcgccaaaacccattccgccttttacggcatcatcatttaacacacgcagtgcgccaaagtggatcctgttaggatcgtagtagttagcaaagctgaaagtatgatgacttttcagccaaccatgattggcgtatcccctggtatctgcgcgatgaataactttcttcataactaaatctcctttgttttaacactacaaatatcgctataaacgaaggggggaagaatggatcatatgttgaaaaaagtggacaaaaaaatacggatctttctatacagtagccgtttaaaaaacggcatgcatatgaaaaatccgtaaaagctgtaacgatgcctggtagctatttacaccagtttcgcatctgtagtaatagtagcattcagcaccttgcttaccgggcagttagcctcagcatccgctacaaattcagcgaatttggcagcgtccaggccctctacgctggcagttacttccaggtggctggtagtaatagcaccgttatctaaagtaatagtgcatttggtatcaatgttaccgggagtaaaacctgcgccagtgatcacaaagctcagcttcatggtaaaacaaccggcgtgggctgctgcaatcagttcttcagggttagtaccaataccatcttcaaaacggctgctgaaagagtactgggtcttgtttaatacagttgactgggaagttaaagtgcctttaccttctttaccggtaccttgccaattggcagatgcaaatcttttcatgtttaattttttattttttccagttagaaaaatcagtgcggaggcccaaattacaaattaatcggcaataaaaaacgccggagcttcctggaacgtaaaagcacataaaaaaagccgcacagtttcctgcgcggctatacatggttcctgtcaattgattcctatattctttctattaatattgctatagcctgttacagatcctgacctgcaacaggcaagtgccatattattgttgctttaccatttgtacactggccaacagctttacttcatcactcagcaataatccgccggtttcagtagtagcgtggaaagtaagaccaaaatctttacggttaattttaccgctcagttcaaatcctgctttagtctggccataaggatccaccacttcgccgccaaactcaacattcagctctacggggcgggtattatcccggatggttaaatcacctaccagtttaaatgtatctgcatctattttctttacttctttagacacgaatgtgagctttggatacttttctgcttcaaagaaatctcctgcctgcaggtgagcatcacgctgcgcattctgtgtggaaatactgttgatgtctgcttcaaatgtgatattggcagtgctgaaatcattatcaacagtttgcatggtaccatcaaatttggcaaactgaccggttacggtcgtaatcatcaggtgcttgattttaaattgtacatcactgtgtgacggatcaattttccaggttgtcatatagctttgtttttttagtattattaaatgtttaattagtttaaaactcccattttaccggcgttaaaatcatctatcgccgttctgatttcatcttcggtattcatcacaaacggaccgtaagcaaaaatgggttcatcaatcggttcgccactcagcaccaccatagcagtgtctttcagcgcggtgatgattacttcggtaccctctttttcaaagagagcggtttccactcctttgagtgactggccattcacatcagcttctccctggaatacgacggctgccgtgttaaaattttccggtatgcttaaagtgattttatcatcttttttaagatgaatatcataaacattcactggggaaaaagtactggcggcgcctttcacaccatcatactcacctgcaatcactctcacatatccttctgcacttacctttaccacaggaatttctgctttggtaaggttctgataggagggaggattatttttaaatgctttaggaagatttacccataactgggcaaactccaccttcccgccttgtttactgaatgcttcactgtatttttcttcatgtaagatgccgctggcagctgtcatccactgcacatcaccgggaaacaacaaaccacgactaccggtagaatcccggtgttccagttcgccctggtatacgatggtaacggtttcaaagcctttgtgcggatgttcgccaacacctttgggtcttacactcggtgggatgtaattgggagctgcatagtccatcatgataaaaggactgatcctgttaccttcagaacgggttccgcccggtaaggtgctctgcaccctgaatccatcgcctaccatgtgtggtgcggctgcaattacgatctggcttacatgtttttgtgttttcatattatttgcctccttaagacaacacaaaagtacatgttacaacatcggttaagaatggataaaacactcctagtgatggactttttttaaaattccggaaaattcagacggaagggcctacagatgtgcgggaagcctctttaaattcagaagggctctggttggtatacttcttaaaaaagcggctgaagtagtgcggatcatcaaaacccagcttataggctatctctttggcggtaaggtctgtattgtacaaataccgctgcgcttccaggatcacccggttgcggatatgttctccggcggtaataccggataattgcttgctgatttcattcagcagcacgggtttgatatgtaaaaggccggcgtaatcagatacggtttttaattcctggtatttttcctctatcaggtttttgaatttcaggaagatggaactattatgcgctgcatgctgttcaggggtaatggctacattttctccctttatgcgggaagccaataccaggaaataacgcagcaggccgtgcagggccatttcatattcaggttcacgcagggttaactccttcatcatcaggcgaacaatggcgtcaatatctttctcctgttcatcatcaatatgaattacgctgctgaactggttattgaaaaacaaccctgaattgatgccggatacctgcgtctgatcctttaaacacatgaaagcatcgcggaaggcgatcatgtatccgtctattttatcggttgcctgcaggttatgcacctggccgggagccacaaaaaaaagcgtgttcttttttacctcatgcgtcaccgcatcaatggtatgcagcagtttacctttcttaatccagtaaatggtgtagaagtcgtgccggtgaggtacgccgatctgatcaaaaaaagagttacctaattcacaaagaccagacaccacaaatcccggatctacatgtgagtactccggtaaggaaacaatcccgatattttcacgtttctcagccatctattaaggttcctgctgtttcttcctccctttcggaaggatcaatgtattcaataataaagttattcctgccttcgcccaccataatccccatatgcttcatttgcaccagttccagcatactgaggaacaggaaaatggcatgcacacggtctttacagtgatcgaatattttttcaaaagataaagtacgctctgctcgtgccagctcttccatatacatcctggagccctccattgtataatcgtacttgtataccacgtgctggggcttgttatcgcgttctttcatgcgctgaatcaccttctcaaaggtttttgtcagcttgaagagtgtgagggtttgcacttcagtaccttcactggtcacttccccgatttcggccagttcctttgcaatatttccacgttttacagacagcatacggtctgcttccatttctgccagttccgcggccgccagcttgtaacgcttatattccaggattttgtctatcagctccatccgcggatcaatttcatttccctgctcatccagttccttgcgcggcaacagcatctttgctttgatacgcatcagggtagacacaaagagaataaattcactggccagctctatattcaacgtttcaatatgatgaatatagtccaggaaatcctgcgtgagggtattgatagggatattgtagatatccagctcatcacgttcaatgaagaacagcagcaggtcgaaaggaccttcaaattgcggtaatttgatcttatagacaggtgcttgttcgctcacgtaatgtttttaaagattttttataaaaagatatcgcacaattgcccggagtcattaaatgcccggttagataaccggtttcctgtctccatgccgctgtgcgatatcaaaaataacaaaattccggcgaatcagaacttggcagcaaagccaatcccgatcacctgttttatctgtagccggggacccatcacaccggtttctttattctcaaatacttttacatcatcatcatatatcatatctacggtcagcagggcagaaatccacttgtttaccttcagttccaatgcgttggtaaaaaacacgtctatgttccccgggttgtgcctgtaatcggaaaataaatccagccggcctttataagtcatgttttttgcaaaggtctttatatagttggcagagaggtaagcgcctatttcatatttaaaatgcgaccctgtatccactccgtaagcgccctgtttagagagtacgtcatccattacaaacacaaaacgggaagtaattggcgacaggaataaagaaaatgaattatccggtttataatcaaaacccggcgacaccagcacgtaagcaggagagaagaattttgaggacaactgcggcgtagtatccgaaggatacaaataaccattggtgaactgggtacgtaaattcaccaaaccgcttaaataccagtttttgccaatctcatagccatatttggaagtaaggtcaatgcggtcgtcatttttccgtcctcccaaactggtggtattaatatagccataagccaggtcggcgatgttgtcccaggaatgttttcctttcttataaaacgcccagccaaaaagattggacccgatagagaaagcaaaattatcaccgcccgcagcccagttactcaaggatccctggttgatatttacattaatgttcatcccctttctccacaatttgggaatggtgtcattagggtcttttttgatcttaccggcagcttcttctctcgacttcttcatccagtcattttgcgcgtgtaccgccgtaaacagtagcatacagcaggcaatggataaagtaaattttttcatcaatttgtgtttaaatgagtacgtaataagtcaccccactttttccggaaggaaaaatggaatggtaagggtatttctaaaaatttttatctggattttttcagttcatcacggatttccatgagtagtttttcctgggtagacagttcagccggggctggggcttcttcttttttcttggtaagcttattcataaatttcaccagcaggaaaatacagaaggcgataatcaggaaatcaatcacactttgtataaaagcgccataagcaaataccgctatgcctttagctttcgcatcagccagtgtggccacgtctcccttacttgtgtctaatacataaaagacgtcgttaaaattctttccccgggtaaataatccgatgataggcatcaggatattatctaccagggatgtaacaatctttccaaacgcaccacctataatcacacccactgcaagatccattacattgcctttcatggcaaactccttaaactctttgatgaacgacataatgcaaggtttttattggttaaaataagtgaacaaaattaaagcataatacccgaacacgttaattattaagctattatttctttaaccggggatatttcatctttaatgatttcagtgtatccctcaacgttagcgcaatcaggtattccttataccagttctgatctgccggaacaatcagccagggcacatagttacagtggttaattgcatcttcataaacatccatatatttattccacagctttgattctgtcaggtcattttcgttatatttccacatcttgcgggggtcttctgtccgttctacaaggcgttgctgctgggcttcctgtgatacatgcaggtaacattttatgatgtgcgtattattatgaaccgtcagcaatttctcaaaatcgttgatggcttccatccgcttaaaggccatcttatcgtcgatccacttgtgtacgcgttgtataagaatatcttcgtaatgtgagcggttaaacacctggatcatgcctttacccggcgcatgctgatgtatcctccataaaaaatcgtgttctgattcctcggggctgggtgctttgaaagagtggaccgtgcagccctgcggatttaaggtaccggtaacgtttttgattacgccgtctttcccgctggcgtccattccctgtactaccagcaatacacagtgtttatgctgtgcatacagcaggttttggagttcatccagctcctccagaatttcccgggttaccgcctttattgtttctttatccagctttttgggagccgatgtactgatagcagacaatttgattttacccatgtagcgtattcttataaataaatttaacaaaatcgggacagaagtgttgcgttatcatgatttatattttgctgaatatgaaggatacctgcacctttgtactcgaaaaacaacagctatgcaccaacgtttcgcccattggggagtgtttctcctgttatcactcacatggggcagctcctttatattgatgaaaataggcctggaatcatttacttcgtaccaggtggccagtttaagactggcggctgccggcgtagccctctcaccttttttaccaaaggcattcaggcaaacgcccgtaaataagcttccccttattatactttccggcatcctgggcaacggtatcccggcttttctattttgccttgcagaaacagaaatcgacagctccctggcgggtatccttaatgccttaacgccgttaatggccctgctttccggtatcattatctttaaaagtccatttaaaaaagcgcagctcaccggcattttcgtagggctggccggggtagtattactgttcgctgccaaaggcatcaatacaaatggccactggtattatgcgctgctggtaatcctggctacagtaagctatggcgtaaatatcagcatggtacatcataagctgcagggcttcagttctctgcagctgggatctctggctatgttcttttgtgccgtgttcacatttccgattctgtggtacagtaacttctttccacagttttcccaaccggatgcgccctggcgctcactttccgcaggcctggtactgggtgtgatgggaaccggcgtggcagctgtgctctttttcctgctcatcaaaagagcggggtctatgctggcctctatggtagcatatgcgttaccgttagtagccgtgggatggggcttgctggcacatgaaacaattaccttgattcaggtgggaagcatgggcattattttgttgggggtgtatctcgtaaacagggccaacagggtgtctacagcaaaataaggcatgctgcccaccactaaaaggagcggagatattaacaggatcggtatccgttaatatctccgctacaatattttcaggctatactttttaaatagccataatttctttctcttttacttcgcaatgcttatcgatcagcgtaatgtgcttgtcggttaattgctggatatcggcttccgcatccttggcagtatcttcgcttaaaccgtctttctgtaactttttaactgcttcaatagcatccctgcggatatttctgatggctacctttgcctgttcaccttcgttattcacctttttcacaaattcttttctgcgttcttcggttaatggcggaaggaataaacggatgataaccccgtcgttttgaggattgagaccaatattagatgcaataatggctctttcaataggctgcagcatatttttttcccagggctgaatggttagggtgcgggcgtctgcaatgcttacattagcaacctggttcagtgcagttggtgcaccataatagtcaacaaaaataccatccagtatttgcggattggctttcccggctctgatttttgtaagttccgattccaggtgcccgatagctttcttcatcgagtccgctgcttcatcaatgataagcgttagatcatcttgcataacataaatagttaagtgcgtgcaaacctacaggttttcttttaatcgtcaaagtaacgccctgataatggaagtagaaatgcttacaaataaccacaacaaaaggattatttatcttgcaatacaccctctgttgtaacacgcaatattttggtggcttcttttgctgttgccactgctggctgtattaccggctctggaatagccttcaccgccagtttcttccggcgtgccaggtacaatacccctgtaaaaaaggtagcagaacctattacaaccattagcagccaggtagcgcccattccctgtaacacaaatgcaccaacgatataggtagcattgattgctacagaaaccagcgtggtttgcctgtgattgagcttcaggtccagcaggtaatgatggatatggttcctgtcggcagagaaaggagatcttccctgtaacatacgaaccgcaaatacgcgtaaggtgtcaaataaaggtacgatcaggatagcaaatgctacagctggtgtagccccgataggcatcttaccggcaggattgccagccacatcaataaatttcagtaccagcaccgcatttaccaggcctatcagtaaggatcccgtatctcccataaaaatacgggcaggagaaatgttatatataaggaaactggctaatccacccgccaatgcgaagcctattacggcataagtgatttcacccacatgcaggaaataagcaccaagcacggcactcaccaacaatccgatgctaccggcatggccatctacgccgtctatcagattgaaagcattgattaccacaataaaagtaaaataagtcagcatcaggctgatattcggaggcatggcataaattcccatgaagccatacatgctggttatctgaagattgccgaggtaaataatagcgaaagatgccgccagctgcccgattaatttctttaacggagacaaccctacgatatcatccttcatgcccaccatgaaaatgataaagaacgccgccatcatgtattgaaatggcgaattggctaacgcgggtacgcagatagccgtggcaattataaatccggagaaaaaaccgattcctcccagcgttggtatacgctgtttatgcgtctttctttcgtccggttcgtcgtataagtgctttaattccgccactctgatcagtattggaatagaaaaataggtaacaacaaaacttaggacggtagcaattaatacattctccattagtggggcttaattgtgcaaagatattaatttcaacgaaatatgaaaagaaacgttaaaaaaatcaacttttttaatactttgagatcgcaaaaaaaacattcaacagccacaaaatctacgaaattctattagttttgcggcacaaaaattaacaactatcatgccacagctcaaagatattgctactcaggtaaggagagatattgtacggatggtacatggcgttcaaagcggtcaccccggaggttcattaggttgcgccgacttcctgactgccttgtatttcaaggtaatggatcataaaccggaaccttttgatatggatggtaaaaaccaggacctgtttttcctgtccaatggccacatttccccggtgttctatagcgcacttgcccgttccggctatttccccgtacaggaactgagcactttccgtaagctgaactcccgcctgcaaggccaccctaccacccatgaacacttaccgggcgtacgcattgcttccggctccctgggccagggcatgagtgtggcaatcggcgctgcgcttgcaaaaaaactcaataacgataaaaacctcgtattctccctgcacggagatggcgaactggaagaaggacaaatctgggaatctgtaatgtttgctcctcatcataaagtagataaccttatcatcactgttgatctgaacggtcagcaaattgatgggactactgatgatgttgccggccttggcgacgtgggcgccaaattcgaggtattcggatggctcgtacttcacatgaatggtaatgatatggatgatgttgttgccacactggaaaaagctaaaagccttaccggtcagggtaaaccaattgccatcatcatgaaaaccgttatgggtcagggtgttgacttcatggaaggtcaccacgaatggcacggtatcgcccccagcgacgaccagctggccaaagcactggctcagttaccggaaactttaggtgactactaatagcagttactcattaagatattaaaaaaagaggcgcatgaattcatgcgcctcttttttttaatatcttaatgagtccatatcaggttgccttcaaggtaatcgcttccaccgctgcccttctcgccggataccagctggcagccacgcctatcacaataatcgtaacaaacaccaacccaaaatctgccgcatgcatactcacagggtatgaatccaccaggaaagaagtcccctccagcttaataatcccaaaatgctgctgcaacaaacaaaaggtgattcccagcccaaagcccagcaccgttccaataccggcaataatcaatccttcggccaggaaaatgcgcataatcagcgacttacgtgctcccatcgccttcaggatcgtaatatctttctgtttttcaattaccagcatatataacgacccaatcatgttaaaagcggcaatgatcataataaaactaagtatcacatatactgcccacttctctgtttgcatgatggcatatagcgactgattctgctcataccgggtttgcaccttataccggccgcccagcaacttttccagttgcactttcagcacattatcgtttatccctgcccgtgtcccgatttccagcgacgacatctcatcggcccccatctgcaacaggccccgtaaaaattcaatgtttgtaataacatacttactgttgaactcctgctgaattgcaaaagttccggcgggatataaaacgccgttgttcagcgcatcctccggggtcacaaaagcatttacattcctgcggggaagatatacggttacaggtgcaatgctatgcaccacatccacgcccagcgcaccttccagctccaatcccagcactgcccggtaggccacactgtcgccggtgtcaaaacgtccgcggataatattgctttttacatcggtaacatagttataactgctgtccactcccttcaatacggcaatcgtaggctcgtcaccgtaacggagtactgccttctcttcaattacccgggagaaatgggctacacccggcaccgctgctatttgctgcagctgcgcaggcgtaaggataattgttttaccggtaaccggcgcaattttcactgcagggtaaaaagaggaataaagggattttaccaggccctcaaagccattgaacacgctcagtatcacaatcagggcgccagcgccaactgcaattgccaccacacttacccaggcaatgatattgatagcattggtagattttttggcccggaagtaacgggaagcaaattgccaaaccatgtatttgtagaattacgaatgaagaataaagaatccgtaacccttatttcttgccatccttgatattggcgtcatcttccttgattttcttgaataactcttccatcttaaacacgtaatcaagtgtatcatccaaaaagaagctcaactcggggatcctgcgcaattgtttgcctaatcctattcccagtaacttcttgatctcacccattctttccttgatccgctccagcatctccgaaggggctttgatctggaacatactcaggtataccttcgcctccagcaggtctggggtcatcttcacggcagcaacagatatcattcccccttccactacattaaatcccaaccgctgaaaaataccactcagctcctgctgcacaagttgtcctatttgtttctgccttttagtttcctgcatctcattcagttttaatcgttagtaaaacagtctgcgtacgataataacataattaccccgccccgccaaaccataaccggctgccagcagcccgtcagttgcgaaattaaccatttccgggaaagaatagccgcatttacaccccctcataccttaattatgctatttttgccagcaagttaaacagactaccaggaatgaagacattcaagcgattactaagatttgccacgcctttgcaccattatctgccggaatatgttatatatacctttataggtatcatattcggtatggtcaattttgctatgctgatcccgttactgaccgttattttcaaccaggtgggcgaaattccacaggcactccctgaaccacatttcaccttttctatcaattattttatagatctgttcaactattatttctacaactttatcagggccagcggctccaaacaaagcgccctgtacttcgtttgtgcagtgataggcgtgtgtatcgtaattgccaacttcggtcgctacatgagcgccagggtaatggtacgccttaaaatgaccgtactctcccggctacgtatacgcctctatgaaaagtttacgcagcaatcactgtcattttacagcgatcagcaaaaaggagatttgctttcttccatgaccaacgatgtacaggaaatagaaaacagcgtaatcaatgccatacaaacactgttgcgcgacccgttcattataatcggctacttcgcggcactgttctatctttccgtaaaactcaccctgttcacgattgtattttttcctatctccggcctgctgatatcttatgtatccaagaaattaaaattaaaaggaaaattcagccaagacctgttaggaaaaattctttcggtaacagaagaaacacttagcggtatccggatcatacaatccttcacagcagagcgtttcatgaaaaataaatttggcgaggtaaacaaccggtttgtgaaagtgagcaaatcgatgtacaaccagcgcgaactcgcttctcctatttctgaaatattaggcgtgatcgttattgtaatcctggtaatttatggaggcagcctggtattatccggcagcgaactgcttaccggcgccactttcatgacatacctcgttttctattcacagatcatgcagccggcaaaaaatgtatctacttccattaccacgatacaaaaaggaatggtagccagtgaaaggattttcaaaatactggacgccccggtaaccatccacgaaaagccgaatgcacgcgctgtgagcgggtttaacagcagcgtggaatacgatgatgtttcctttaaatacgaacagcaatatgtgctgaaacacatccggcttactattaataagggacagatgatagcgctggtaggccgcagtggtgcaggaaaatccacgatggcagatattttaccacgcttctatgatgtaaatgagggcgcaattcgtatagacggcaccgatatacgcgacctgaaagtgcatgatctccgcagcctgatcggcgttgtatcacaggaagccattctctttaatgatacagtgctgaacaatattgcttttggtcagcccaatgccgacagggacgctataatcaccgctgcaaagattgccaatgcgcatgaatttattgaacacctggacaacggttatgataccattatcggcgaccgtgggctgaaactcagcgggggccagcgtcagcggcttaccattgcacgtgccatcttcaaaaatccgcctatcctcatattggatgaagccacttccgcactcgataccgagtccgaaaaactggtgcaggctgcactggataaactcatgcaaaaccgcaccactattgtgattgcccaccggttgagcactatacaacatgccagtgaaatcattgtaatggatcacggtgaaatcaaagaacgtggtacgcacgacgcattgctgaaacaacacggcatctatcacaaactggtggaaatgcaggaatttaaatagataatcactaacgttaaagaatatacgtaaatgtggcacgttccgctcaaaagtggaacgtgcccgtttaaccagtctccgcatggctttcggtaacattttcttcttatcgaaaacccgtaataggtatggtttttgttattgaagcgccctgacaatgccaacaccagctctttgcagcacttattttttaacctttaacatagcgaactcctatgatatctatcgtaattcctgtattaaacgaaggtgctaccatacgccaggttattaaaaccgtaaagaaaacgtcccggaaaattgagatcattgtagtagacgataattctacagataacacagtggaagaggcgatgaaagaacatgtgagagtgattaccagcagccagcgcgggaagggaatatctatgcgtgaaggtatgatggctgccaaacacgatattattgcctatgttgatggcgacatcctgacttaccccgacaatattatagacctattaactggtcctatcgaaaaagacgaagccgacttcgtcaaatcctactttgaaaggcaggcaggcagggtcacccaattggtggccaagccactgctgagtatattattccccgagattgctcatttccagcaaccgctcagcgggatgattgctgcgcgcaaatcattcctttcccgtgtgcattttgagaacgattatggcgtggatatcggtctgctgatagatatgcatcacctgggcgcccgtatcacagaagcaaatatcggaaaggtggaaaatgccatgcaaacctgggaacagctgagcaaaatgtcgagagaagtatcccgcactattctccgcaaagcggaaaatataccacaggaaaatcttgaaacactgggcaacattaacctgatacgggagcaaatggagtattccatcctcgagtctattgataaactgcagaagatggtcatctttaacctggaccatgccgtgtttacacaagactacatgcaatgggctgcagtggccttcggacaggaggaagggctacaggaaattgaatcttccgggcatgatccggtaactacattacatttaaaagccacgctttttgaagggcgcaatattgcagaattactggaagtagcggatgctattccattggtacccggcatccgcgaaatagtgcgtgaactgaaaaaaaggggttatgctgttggtctgatcaccgacggttttggtaccgtagcccgtcatatcaagaatcagctgggaatggatttcgtatttgccaataagctgcacctggttaacagcgtggctaccggcgagtttactattgcagactactttatgaaaggagaggaatactcccggagtaatatgtttccctacatcgcgcagcagtatcatattaatacacagaatatcatttatgtgggagatggaaaacgcgacagcaaattattatcagaggccggcatcggcgttgctttttgtccacagtatccgggcaatgttgtagaaaaggttgccgataaaattatcagcggcttatcattagcgcccctgttggatattgcgcaggcgagcccggcgaagtttggcattaaattgccggctatcagtaaaaagcaggcgcgtacaattggagtaggcagcctgataggtttggctggagctgggttaatttacttcgctgtgcgacaaatacgtaataaaaaagagatggccacctgttgatgatattcattcagctataaaggaaaaggcgcagcggataaccgctgcgccttttctgtcttaattagtactaagactatttacttttagccagtttagcttcaatgctcaatgtagcgtgaggaactgccctgaggcgtgctttatctatgagtttaccggttacgcggcaaataccataggttttgttttcaatacgcatcattgctttttccaggtgatcaatgaactggatctgacggctggccatctggttcagttgctctctttcctgggagccgctgccatcttccatactcatgtatttgttctctgtatcgtcggtaccggcctcgtctttacgggtgatcaggccttgcagatagatgagctcctttttagctgattccagcttcttttggatcaattctctaaactcctgcaggtctgaatcactatatctgtatataggaccagtaggttgtgccggttgatccagcactgacttggtgaattcaggttgataagttaccagggtagcttttccaccttttttctcagatttttcagttttttcgggtttttcggatctttccgcctttactgacttttcagccttaacaacaggcttttcggctgctttttttgtggattctttctccttagcaacttctaccttagtatctgctttctttactgccatcgttttaagttctttttcttctgacttagaaataaatggtttctctttttcagcggaaacacttttcgttaccacttgctgctttacagcaggctcttttttaacggtcgatttcgcaggtacagcaactttcttgacggatgatgttttactgtttggtaaggcagaggcctttttcactgcttttttaggcgccggagcgacttttttggcagtgcttttagctaccacggcttttccggctgctggttttgctgctgctttaggggccgcctttttaggggctgcttttgcagctgctttttttggagcaggcgccgctttctttaccggagcaggtttaacagctttcttcgctggtgatgcctttgccacagtctttttagccggagctgctttctgggtcgttttactagcaaccttcttttttgttgccatgggggattagctttttttgttaactaatacattaaatttaaggtcatttacctctatttctgtaccatcttgtaatcgctccactaattccaggctatctgccaaaatttccgtgcaaatataatcattatagttcacaatggccgacttgagcgtgtctacactttcaatcgttacgtcaattctgtcagtcaaagcaaaatcactatccttacggatcttttgtatccggtttaccagttccctggcattaccttcgtcttgcaactgtggagtaatagtaatgtcgagcgctaccgttaaggcgcctttattagctactgtccatcccggaatgtcttcggaaatgatttcaacgtcagagagttggatttgcaactgctctccctctacaaccaggttgaaatggccgtcgcgctcaatggtggtaatttctgcctctgtaaacgcgctgattgcggctgctacagatttcatctttgctcccattttaccaccgagggacttgaagttaggcttaatctttttcttgataaaaccctccgtttccgtaagataatcaatccctttgacattaacttcactttttatcaggtcggctaccatttctatttgctccttcatcctgccatttgccaccggaattaaaatcttctgcagaggctggcgaactttaatgttcacctttttacgcaaggataataccagcgaggaaatatcctgcgccagctgcattctttcttccagatcaaggtctaccgcaccctcatttatcacgggaaaatcagtgtggtggatggaagcagccttgctacggccactcacactgttcaggttgttaaacaaccaatcggtgaaaaatggggaaaccggggccatcaattgtgcaattttttccaaacattcgtataatgtctggtaagcactaatcttatcatgctcgtattctcccttccagaaccggcggcggcataaccgcacataccagttactcagctgctcatccacaaaccgctccactgctctgcctgcctgcgtaggctcgtaatcgtcaaagctgctggtcacgtcttttaccagggtgttcaacacggaaataatccatcggtcaatttccgggcgttcttctaaaggaatgtatgcttccttgaaagtaaacttatcaagattggcgtacatagcaaagaagttatatgtattgtacagggtaccgaacaacttgcgctgcgcttcccctataccttttacatcgaactttaaactatcccagggcgaagcattggtgatcaggtaccaacgggtggcatctgccccaaacttttcaatggtctcaaacgggtttaccacattgcccaggcgtttactcattttctgccctttcgcatccagcactaatccattggaaactactgttttatacgctacgctatcaaaaagcatcacacccagggcgtgtaaagtatagaaccagccacgggtttgatctactccctccgcaataaaatcagcggggaaagcctgtcctttatctatcagttccttattctcaaaagggtaatgccactgcgcatacggcatcgcgccactgtcaaaccaaacgtctaccaaatcaggctcacgacgcattggtttacctgacgggctcaccaggataatatcatccacatatggcttgtgtaaatccaggataccttcatggagataagacttattcacatctccacccaatacctggttcgctttgcggatttcggcattcagttcctcaataccaccgatacagatctcgtccttgccatcttcagtacgccagataggcagcggcgtaccccagtaacggctgcggctgaggttccagtcgaccatattttccagccagttgccaaaacgaccagtaccggtggaagccggcttccagttgatcgttttattcagctccaccattctgtcttttaccgcagtagtctttataaaccatgcatccagcgggtaatacaacactggtttatcagtacgccagcaatgcggataagtatgttcgtacttttctactttaaatgcacggttctccttcttcagtttcacagcgatatccacgtctacatctttgtaatcgggatcatctttataattctttacatatctgcctgaaaattcacccacattctcggtaaacttaccggtccggtctaccagtgttaaaatgcctataccatatttcttacccacccggttatcatcagcaccaaaagcaggcgcagtatgaacgataccagtaccatcttccgtggtaacaaaatcaccgaggagtacccggaacggatcgccttcttccggctgggtaaatggcaataactgttcgtaacggatattttcaagctgactgcccttaaagctggtcagtatcttccatggaattactttatcgccttcctgataagctgcaaagtcagcgttttccccttctgctttgaaatatttgcctaacagcacttttgccattatcacatttaccggcaggtgagtataagggttaaaagtatttaccaatacatattctatattagcccccactgttaaacccaggttggatggcaaagtccagggagtggtcgtccaggccaggaaaaacacctcatctgaacccgcagcatcaaaaaggaattgggaattacttgccttttgggctttaaacatcgccactaccgtagtatcctttacatccttataagtgccgggctggttcagttcatgggaactcaagccggtaccagccgcgggcgagtaaggttggatgcttacacttttatacaggaatccttttttataaagcgtttgaagacaccaccagagtgtttcaatatagttattctcaaaagtgatatacggatttttcaggtctacccaataccccattttcagggtcaggtcatcccacatatctttatatttcaatacctcccggcggcaggtatcattatattcagcaacagaaatctttttacctatgtcttctttggtaatccctaaagttttttcaacacccaattccaccggcaaaccatgggtatcccatccgcctttacgctttacctggtaaccgcgcatcgttttataacgacataccaggtcttttaatgtacgtgaaataacatggtgaatgccgggtaagccattggcgcttggaggtccttcataaaatacaaaaggagtggcgccttcgcgcacgtccacacttttttcaaaagcctggtgctgctcccagtgttgcagtatatctttctctatctgaggtaaattcaactggctatattcctgatatttgctggacataaaacaattccccgccctttgatgttatttagacaataattgattaaaattgtgcgaagttaagaaaatacgctggctcctaaatagccatctttgctaaaaaccatgctttttgaatattttttattgttttttttgtaatttgcaataaagaatacagaagctgcgtttttggcattgttttagctaacttgccaggaagaattagaaaaacctagtagttaattttagcccaacggaaaaaaccatatcgagtatgaaaaagttgacgttaatattttgcgcggttctattcacttccggcataacttttgcacagcaaaaaaaatcagttaaaaaaacaaagatagttgccaaagcggtgcaagcacctgaggcagttaagagttcttttgatcagaattttgcgggaacagcggctgctaagtggacaaagacaagtgcgggacattggacagcaagtttccaaaaagacaatataaatacaattgcagagtatgatgcagatggcaaatgggttgccacaagaagcgcatatgatgctcaaaaccttccggaatcagtggctggtacactgaaaacaaaatatccggcggcaaccataaaagatggctggaaaattgagagatcagatgtagctgcatactacaaaatcaatattcaggataacggtacggacaaggcagtgttgctgaatgaagctggtaccatcactgaataacacaaacaagtatttcataggtatagggataaataggacagaccctgctcttttgggcggggttttttatttgttatgactcctcacttctgtttttgcaggctatcatttcccaacatgtgaatttttcccaacggtagaacctgcaaattccacaaccacatatcagcaggttgctttatccaaacaaaaaaagtcgcccgcagaagcgaacgactttataaaatctggtagaaacttttctggcatattgcacttcaatggtgtttgatattcatgcaagtatgatttatggctttacttactttgccagccaagcttcttccaaggtcaaatctgataaggaagcttataggaaacgcaaatggatatctgcctatcgtgttacaaagaaacacctatattttatcttccattttccaaatcgggaaaacaaatgatcgaaaagggaaaataccagctcatttgcccggcttcaaacctcttttcagggcccgggaaacggtaaaccaataaaaccgggctagcgatccccggtagaaatacttcaaaacccacttatattcaccctggaaatgtaatacagacataggttgcacccttccgtcgatggacctacaatacaccgtctctccctttaaagtgatcgccttcctgtcgccaaaggactggtaaacgccgttttcgctgtaaacagccgaaatgttatggtcaatgcccagtgaattaccgatggcattggagttcaggtagggaattctcttctcttttacccacatatagagcagggtcatatctgaaatagccgttcttcctatcttttcctgctgcatttcgtaatgcctggccaggaaatgatcctgcttatttctctcataggtttccagcaggtaatcagtaaaactattgatcagcgctttattccagaacgaaaaatgtggcgaaatctggtgttcgctgccttctccgtaaaacccttcactccctataaatatgccttgcagcgatgtatcttcccggatgtgctgcaggttgtttaccaggtaaatgtctgagtcggaaagaataaaagcatcctcacttttatgggcttccgcaatggcgaaataacgggcgaaacaacttacttcaaacccaaacgaattgacactataatgttcataaagagacaggaatttctcatacctggcgttgcctttcaacctatcaggaccaagtactgtaatgttcaggcttaaacgccgagcttttcgttcatataattttaaatagatgagatccctgttttcatatatatagatgtcattcaacatgtgtgctgttttatcatctgctatgagtttgaacagatgattaaagattatatgaagatagttaggttatttaacgcagaagcacttcaccttacggaaaaatcatagaagtgacgtagaaagaaaggagaagctgttgtttagcgcagcaacagctcacagggtttcagcccggtgtgctttttaaaggcagtggagaagtgggaaatgcaggaataccccatcagcatagctacttcagaaacagacatccccttttcatataaaagccccttggccttttccattctctctttctggaagtaatcatatatggtggtgccgtacatggctttgaagcctttcttcaggtaacattcgttcatggctacccggcgggccaggtccctgatggtaataggagagtccagctgctccaggaggataccccgggcattctctattttttcacggtcttccaggtgggtgaggaagcggcaaccatagcgttcgtcggtgtcgttctgcataaactggtcggagctgtatagtaacaggtccagcgcccggctttgcaggaatatatttttcagcatgccctcgtaatcgtgatgtaccattgtttccagtacggattttgacttcgtacagggctggatggttttcacgaaaggtttgcgggactgattttcaaataaggaaaaggtagtggtacccttttgcagcgattgaatgaatgcaggctggaagcgaacggtgataagatctacagatggcaccctgtcattgcaggcttccttctttccttctgaacaaagctgatcggtacaggaagggtttttacaatacttgctgccggcaacgcaataccggagctctatggcggcagattgcccccttttggccggctggtaaatgaccatcgccacatcttcaacaggtaacggcttatcgtaagtaaaacgttgtaaggtaaaatcaagacagtcaggtactgacacactatcctgctccgccagctgtaactggtcgctcatcgcgggctgcggaatggccaaagacaatatttcctgtatttctttcactttatctgtttttaaacgccgtgctgttatagaagtcacaaatttagtgattcgttttttaaacaaatacgttttgacaatacagttacaaacacaactatccttctccccttaaaacagcgatttacttggtataaatttcgtatatcctttagggatggcaaaaaatggctttaatatccgcagactggtaaaaatcatactcattgtagccggtatacttaccctgctggtagtgggtacaggctggtatctcaatcaacactggaataagttgttgaaacgggagcttcagggctatgtgaccgatttgtcggacagtttgtataccgttaagttcaaagacctgcacctggacgtactttccggcagtgtcactatcgacaaagccagtatgacggccgattctgcggtatatcagcgcctgctggcacaacaaagggcgccggccgatatttacaccatcagcgttgaccggctggaactcaggtactttaagccgtggcgttacttctttgggaagcatctcaacgcaggaatccttactgtaacgggtcccagtattatcctggatcaaaatgctaccgtaaaagataccagtaccccgaaaacggcctaccagaatatctcggccaaaatgaaatccattttcataggcaaactggtactggacagcaccaatttcaaatatatttttacccggaaagattcttcccgggtgatccatcaattccacaatctgagggtccggatcaatgatttcctgatagactcggttgccctggacgaccccacccgttttttatacgcccgcaattacgaaatcgggatgaaggactatatgaaccggacgcgggatagtctttactggatgtatatccgcggaatacggtacgatgcggcggaacgtaccctgcacgtgggccggtttgaactgcaaccccgttatgataaaacggccttccagaaaaaaacaggcgtgcagcaagaccggtttgaagtggtgtttaatgatataagtctgcgcaatcttaatccccgcctgttattacaggaacaacagatctgggccgaccgggtaaatattcagaatggcagattagatatttacaggaaccgtatgatgcctatgcctcccggcaataaactgggccaatatccacaccagttgctggcaaagctggatgttcccataaatatagatacgcttaccggcaataatgttgatatcagatatacggaattgagcccggttaccgaacaaaccgggtatatcaatttcagtcatgtacatggtttattccgcaacatcaccaatatcgatagcctggtggccaaaaacaggcacctcacggccgaccttgacgcggtatttatgaaaagcggtaaactcaccgcccgttttgattttgtgctgaacgacaagggtggccggtttggcgtttccggccggctgagtaatatgaacggcaaagatctgaatgtaattacccagccaatggggaagatcgaaatcaggtcgtgcgatatccaggacctgacctttaatatcaatggaggtgagcgaagcgccagtggccatgtaaaactgctgtaccaaaaccttaaaattgccgttttaaagcaaaataaggatcatgatgggtttaaacgcaaaggactcatcagcctggtggctaatgcattggtaatcaagtcagaaaacccatccaaagacgaaaaaccccgcacggccgatgttacctatacccgagacatcaagaagtctttttttaacctggtgtggaaaactttatttacaggcgtaaaagacattgctggtgctggaaatctctagtggaaaaaatggtggatcctcaccacataaaaacagcccttcttttgtggaaatgaggcttatttttcgtacatttgcatgattgtctaccgattttatttctaatagattttacaccaacatatgagcgaagaattagtgcaagcacccagccccagcagcaacggatatgatgcagggagtatacaggtattggaaggactggaagccgttaggaagcgtccggccatgtatatcggcgatattggcgtcaagggtctccaccaccttgtttatgaggtagtagataactctatcgatgaagcattggccgggtactgcaaaaatattgatgttaccatcctggaagataactccatccgtgtaaaggatgatggccgtggtattccaaccggcatcattcccaaggagggtcgttctgccctggaagtagtaatgacagtactccacgccggcggtaaatttgacaagaacacctacaaggtgtccggaggtttgcatggtgtgggtgtgagttgcgtgaacgcattgagcgacaggctttatgtaaccgtagaacgtgaaggcaaattatttgaacaggaatttcaccgtggcgccccacagtatcctgcacgtgaaataggtaccagtgaagtaaccggaaccaccattcactttaaacccgatggtgagatttttaaagataccacctacaaccgcgaaatccttgccggtcgtttacgtgagctgtcttacctgaaccgcaaaatcaagattactttaaccgacgaacgtgaaaaagatgaagaaggcaacttcttctctgaaattttctacagtgaaggtggtatccgcgagtttatacagatgctcgacaaaaatggccgccgtaacccgatattgctgaatcctatttatgtagaagtacatgaaccggtttcaaatgtagcagtagaagttgcgctggtatataacgacgcattcagtgaaaacattttctcctacgtaaataatatcaacaccattgaaggaggtacacacgtagccggtttccgccgcgctattacccgtgtatttaaatcttatggtgataaaaataaaatgtttgagaagtcgaagatcgaagttaccggcgacgacttccgtgaaggactgagcgctattatcagcgtgaaagttcctgaaccgcaatttgaaggacaaaccaaaaccaagctcggtaactccgatgtgatgggtgtggtagacagttctgttgctgcagtactggaggcattcctggaagaaaatccacgcgaagccaaaaccatcatcaacaaagtagtattggcggctcaggcccgtgaagctgcccgtaaagcacgtcagctggtacaacgcaaaagcgtaatgaccggtagcggcttaccaggtaaactggccgattgctccgataacgatcctaccaaatgtgaactgtatcttgtcgaaggagactccgcaggtggtacagccaaacagggacgtaaccgtaactaccaggccatcctgccgctccgtggtaaaatcctcaacgtggaaaaagcaatggagcacaagatctacgaggataatgaaatcaaaaacatctttaccgctttgggcgttaccatcggtacagaagaagatgataaagcactgaacctttccaaactgcgctatcacaagctcattatcatgacggatgccgacgtggatggtagtcacattgccacactgatcctgaccttcgttttccgttatatgaaagcaatggtggaacagggctacgtgtacattgcacaaccacctctgtacctcgtgaagaaaggtaaagaacaaacttacgcctggacagaagaacagcgtaaagaagcgacccaaaggctcgctggcggcggtaaggaagacagcgtaaccattcagcgttataaaggtttgggtgagatgaacgcagaacagctgtgggatactaccatgaacccggaacaccgtaccctgaaacaggtaaccattgaaagcgctgctgaagcagaccgcgtattcagtatgctgatgggtgatgaagttcctccacgcagggcgttcatcgaatcacatgcgaagtatgctaagattgatgcttaattacgtatatacgttatagttataaacaaaaaatcctgccgtttcagcggcaggattttttgtttatcttctgaaaataatctctttatccttctctcgtaagaatataatttgccagcacctggtacaggaacacacctatcagcaaagcggtaaccactatattaaaggcatcattaatgatgaatgccagcacagtgcccaatacgcccagcagcgccagtcccgccgtataccatgtaataatccggcggttctttttgctttccggtatataaaatcctgccgcaggcagcaacatgatgccactgcaaagacacaatgccagcaatccctgcaagtgagtaaacagaaacgccacacctgccgttaacgacacgcacaacaggatccccactacattagacacctgtgtttgctccttactaagtgcatacctgccgtatggattgaggcgcaggaacaggttgctcaccggcgtaatcagccaggtagaaagcgccaggaatgccaacagcacgtacaccgggaagaacacctggctggcgatctgcgtcaatataaaaatggcgatgataatgatccattgcgtacgggctttttgccgcgccatgaaaaaagcgtagttcaggaactgccggtacagccagtaccgcgctttcatcgcctgcaccataccttggcgcgcccattcattattaggatccagtttcaatgactccctgaaatgctccagcgacttacggtgatcaccggcttccagccacttctgcccgaggttggcgtgggtataagcattctcaggattgtgctccagtgcttcatgcaggttggaaaaagcttcttccttttttcccagccggaacaaggcatgggaacggagattaaggcaggcttcatcttccgggctaatagccaatccttcttccgccttgtgaagtgcggcttcatattctttcctcgacaacaaaatctggctccacatagcaaaataattcacccggtagggatttatagctactgcattactgatggtcctgatagcttcattaaactgattttttgcaaaagcaatcctggacaacaggtacaggaaacgatcatcgtatggagcaaagctgagggtattgcttgctatttgtgttgcttctgcggtgttgcctgtttccaggtagcagatcgccagcaggtacaatccgtcggtatcatgggcattggtgctcaggtgctgacgtaaagcagcaaaggcatcttggaagcggccttgttgaactaaaatctgagcgcgctgaattaatacagccataaacgttatttcttaatatccaggtatttcaatacatcatcataaagaccggtttcatttgaatacagcgcataattacgggcagtattaaaccattcccttgtggtgggtttatgtattttagcggcttttaataattctttctgtgtaataggttgcggtacgcctttttgcagggcttccagcagtttttcttctatcgcaatatctacaattgctttgaggtcggcgccggagtaacccggagtggcctttgcgagcgcgttgtaattaatatcgcttacgggtttattgcgtaactgcagcttcaggatttcttccctgccttccgtttccggtggcgccacaaaaatgatccggtcgaaacggcccggacggcggaatgcgggatcaaggctccatggagcgttggtagcgccgataatgagaatattttcattgctggcggcaataccatccatttctgcgaggaactggtttataatatgcgttgcgcccgactgccggagtgccgcacggttggcgcctaaagcatctacctcatcaaaaaacaaaacacagggcttactctgacgggcaagctcaaacaggctatgcagatttttttcgctggtacccacccacatatccagcacatcatgaatgcctacgttgataaattctgcctgtatttgcccggctgtagctttagccaggtaggttttaccacatcccggggggccatacagtaaaatgccgccaccggctttttttccataggctttataaagatcagggaactgcagaggcttgatgatcttcagatctatttcctgtttttctctttccataccgcctacatctgaaaaattaatttcaggtttttccagcatgaacaggctctcgctttcttcctcttcctcatcttctccgttaaaagaaacggagggttgctgggctacccggaaaagcccgtctaacgcttcatcacggaagcccggatttatttgcagtaaatgctggtatatttcctttgccggcggcatagattgttccttcaccaggatacggcaatgcagcaacagcgcatcgaaatgatccggttcacggttctccagttgctccaggactacaatggcagcggaatatttgtgctgatgataaaaagtgcgcgccagcccaagctgagcagcggtattggatgacgacagttccagtactttcctgtattgttcttctgcggcgatatattcataatcctgcagcagtacctgcgccagatgcatacgtaaaggcacattctccggcgaaaactgcaccgcctcctgtaattgctttattacttccgatgacataatgtgcttctgtttaattattcagtaaccccgtaataatacgcaattcggccgcaaaaaaagtgttaattgtgcctaaatccccacgcatatgaaaaatacacttggcagggtagtaatactgatccacaactacgatgaggctgctgctttttatgaaagcaaactgggcttccataagttgtatgataccaccacaaacggacaaaggtacctgcatatggcgccgtcgcccggtgaaaccaccggtatctggctgctgcaggcaatgggcgcagaacaggaagcgctggtaggcaagcaggcaggagaacaaccgttcctggttttatatactgactccttcaaggattatcatcaacagttggtgaataagagcgtcaccatttgccgtgcaccggtgaatacacccgaagccaccttcctgcatttcctggatttatacggcaatgaaatcattctggtgcaacttgccgggaagaaacaatgaaccagcccttatctatatatattttatttaattaataaatatttatatatattgcaggcctattatccctatgccaacagaacctaaccagtatcctatgtcaaattaaattaattgccggctgcacagaaagcggccggcactggtttcgttcatcaacaacggcatgcctaaacttaatgttatgagaatgaaattcttaatggttgccgttattgccgctttaggaacagtgctttgttcctgtgataaaaaaaatgagaccacaccggtcagcagcttctcctttaaaatggacggtgttcaataccagtccaacgccacagaggcatacctcactgataccgtatacgccggcaaaaagaccttggtagtagatggtgttaccaataacttcggccatcatatggaactgatgatcacctttccggattccctgaaagccggtacttatatagaagatgtagaaatgtcgctgatgaatatccaggaaaaagagccgggttacctgagtaaaaatatcaaagtaattataacgagcattaatagtaaacacgcggagggaacattctccggtgtattaataagtggtgaaacagaaaaacctttaacggacgggacttttaaagtcgggatttactaaacacatttgatgaactttctcacatgcccctcctttaaaggcggggctttttacttcgtaggcacgttaaggttatattatattgtttgttgtttaccctgggttaacaattaattcctatctcaattttagcgactgttaacattgaaatcaaacaaatgcctcgtttctgatagtatttaaacacaaaaagactatcaatagctccgtttcaggatgttttatgcacttcttaacaattccgtaataatctgttaacattctggttgcatcagactgtttcctttgcacctgtaaatacttacaaaacagtttatgaaatcattctttacgctattagctagcttcattgtaattctatgttacagcgcgaacgcacaggtgaccacttccgttatatcgggtaaagtatccgatccgggtggacaggccattcccggcgttacagtagtaatagtaaataacagcaccggcgccaaatcaggcgtacaaacaaacactgatggccgttataatctgcctaacctgaatccaggcggtccttacactatcactgtttcattcattggatataagaaagaagtaaaatcagatgttaacctcggactgggaaccaccagtttcaattttaaattacaggaagaatcaaccgcactgagtgaagtagtggtaacaggtaatgcgggtgcaggtaaatccggtaccagggtaggacaggagcaaattaaagcgctccccacactgagccgcagcctgcaggatcttaccaaagtaacaccacagagcaacaacaactccttcctgggtaccaactaccgttacaataacgtaactgtagatggcgccatcaataacgacgccattggctttagcccttcactgggcggacaaagcaacaccagcggtcagccgggcagcagcacccgtaccaatcccgtatcagtagatgcgatccaggatatacaggtattactggctccctttgatgtgaaagttggtaacttccttggtggtagcgtaaacgcagtaacgcgcagcggtaccaacgaagtacacggttccatctatggatttggccgcaatgcttcactggttggtaaaaacaacgctggcgacggttctaaattaccgagcgattttcatgagtaccaaaccggtgttcgtctcggcttccctatcatcaaaaacaaattgttcttcttcaccaatgaagaaattacccgccgcgtagatcccgtgatcctcggcgcaggctccgctgatggtggtggcatcttaacagaaaaagacgctgctgacatcaccgcactgatgaaaacatacggcgtagatccgggtacctcaggtaacaccagcatctattccaactccaataaatttttcaacaggatcgactggcatatcaatggaaagcaccagttgtctgttcgtaacaacaccatcacttctgaagctaccaacctggaacgcgatcagcaaaacttccgtttcaagggcattgacttcaaacaggtaaataaccagacttctactgtggctgaactgaaaagtaactttaacagcggtttctccaacagcctgatcctcggttattccaatgtacacgattacagggagccattgtcagatccggctacaccacagatccagatcaaaggaagaacaccaggttctaccatctttctgggtaccgaccgtgaagccagtatcttcaacatgaagcaaaaaacttttgaaataacagataacgttaccctgttcaaaggaaatcacacgattaccctgggtacacacaatgagttttacaacatcacctatggttttgtaaactcctggaatggccgtttagactacaacagtattgaagacttcctggctaacaatcccgcacgtgtacgtggtaactacaactacaccaacaactcccgtgattacatcatggctaatcctcctgctcaattcaaggcaaacctgctgagcgtttacggacaggatgagatccagttgtctgatcgtttcaggattacgccaggtatccgtttggattacacgggcattcccaacaaacagcctttgagtgataaaaccattaaatcaccggaagatcctaactacggtaacacttacagctatacgaaaccaaaggatatcaaaaacgacttcctgaataatgtgcagatctctccgcgcttaggtttcaactatgatattaaaggcgataacagcctggtactgcgtggcggttccggcttatttaccggccgtattcctttcgcatggatcggttatgcatattataacaatggcgttacttacggtgcctacgatcagagaagcagcaccaaaccatttgtcaacacgccgctgcctgcagcaaaaccatcacagaatggtatcgcagacttcgcgtctcagaatggcgtagatgttaaaaatgcagccggcgccacccaggtggatatgatcgacaacaacttcaaaatgccgcaggtatggagaagcagcctcgcattggattacacgacccacgaccagtggaagttctccattgaaggtatctataccaaggtaatcaaggatctgatgttccagcaggtgaacctggcggataatccaacttactttgcatacgatgtaaacaagcaacagcctatctacaccggttctaaaatcaatcctttatatactaacgcttacctgttatccaacaccgataaaggttaccgttacagcatcaccggtcaggtatccaaatcgttcccttttggtctgaacttcatggtggcttacacttacggccaggcaaaagatatcaccaatggtatccgcaactccatggaatcgaactggcagctgaaccaggcgctgaatcctaacaaccccggccttgcttactctaacttcgacatccgtaaccgtatcgtagctactgttgcttacaaacaggattggggcactaaaggcaaatgggtatctaacttctctgccttcttcaatacttcttccggaacaccgttctcttatggtttagtgaatgctaccatcaacggtacaccacagcaggtgagcctcacctacatcccgaaagatgtggctgaagcgactaacttctttacagataaagcaggcggaccaacagctgctcaacaggcgaatgatttcatgagctatgttaacagcaacagctacctgaatggccgtaaaggtcagtttactgaacgtaacggcggccgcacaccatggaacacccaggccgacttccgcttcgcgcaggactacaactttaaagccggtaaaaaggtacacaccatcacgttgacttacgacatcgtgaacgttactaacctgctgaacaaagactggggcattcaatacttcacgcccaacacctttaactctatggcgagcgttggtttgaatcctactggtaaagtagttaacaattatcctacttatactttcagcaaaccaggcactccttattcaaaagatttctttgcatcccgtcatcagatgcagctgggcctgagatatagcttctaattcagcttgtcttaataaaatgtaaaagaggttgttccatacggaacaacctcttttttgtattacatctccagtgtaattatttgatagcaaatactgctcttacttctgcacggatcttaatagttttgaaatcaatatcactcgctgcttcggcactatctgcagatttagccatgtagttagccattacgggacgaacatcagaatagttatctgtattcatttcctggatttcgatcacaccatctgttttgttaccaatagcggaaagcatatactccgctttttctttcgcggcctgtaaagcttttatttttacttctttacggtatgcttccattttgctggaagaataagaagctatccttgcattttcaataccttcagcatctactgcggcgaggatttcgttgattttatccagcttgcttaatttaagacggtattgtttacgcgccataaattccagcggatctttcttcttccttaaaatttcaaagttgttgccatatacattctcaatggtgaaatcggctttcggaattcccgcgtcagatacagctttctgcagttgtttttccagtgtgctgatgtctactttgttttttcctttgagatattctcttaaagagatgttgaaataaatttcatccggtgtgatttccatttctgcggatccgtttacttcaatcttttttaccggctgttgcttatctgtttgctgtgcaaaggtgctcagtgcaaaaaataatcctgctgctaataacattacctttttcatgtgtcgatgttttctattgttaaaaaaattagtgtttgttgttatttacaccctcatgatgcggggtttaaaagtgtttccacaaagggcgatttataaaattttgttaatgcaatagttacagaaatagaattatacatttcatattagttatgaaacgattacaaaggaattatgttacaggggaaagaattatttccggctatcggtcatggctttcaggaagtcgtacaggtcgttcatatgacggatacgggaagccaccaacataaagtttttaccaacctgttttagcttggcattgttggtacgggtttgtatatacgttaatatatgattgaacgtgggggattcgaagtaaggggaatccgggttgttgataaagtagcaacgcaggttttcttctttcagcatcattttttcgaagccgagctggatggccatccaacggcagcggatagctgtcagcaagtctttcaccggttccggcatagggccgaagcggtctatcatatcattggcaaaagcctgtagtttgccttcttctgtgatattatccaactcctggtaaaggtttagtctttcctggatgctttcaatataagtatcagggatcagtatttccaggtctgtatcaatggtacagtcgctcacgaaatctttcttctcttccagctgatctttaaacaggtcgcggaattcattttgtttcagttcgcggatggcttcatccaggattttctggtacatatcaaagccaatttcggccataaagccgctctgctcaccacccagcaggttaccagcgccacggatatcgagatcgcgcatagcgatctggaaaccgctgcccagctcactgtgctgttccagtgtttgcaggcgtttccggctatctgaaggcagcgtgctcataggcggcgccagcaggtaacagaaagcttttttattactgcggcccacgcgaccacgcagctgatgcaggtcactcaacccgaaatgatgggcgttattaatgatgatggtattggcgtttggaatatccaccccactttccacgatattggtacacaccagcacatcgtacttgcggtcaatgaaatcgaggatcacttcttccagttgatgtccttccagttgtccgtgtgccgtagcaatagacagatccgggcaaagtccctggatcaggccggccatttctttcaggccctttaccctgttgtggataaagtacacctgtccgcctctttcggcttcataataaatggcttcgcggatcaggtcctggttaaacacctgcacttctgtttcaatggcctggcggtttggcggcggcgtattgataacagagaggtcgcgggcgcccatcagtgaaaactggagcgtacgcggtataggcgttgccgttagtgtaagggtatctacgttgtgcttgatctgtttcagtttctctttggcagaaacaccgaatttttgttcttcatctactaccagcacgccgaggtctttaaacttcacttctttgcccagtaaagcatgcgtgccgataatgatatcgatctttccttcttcaaggcgcttaagcgtttcctttttttctttggaagatttgaacctgttgagatagtcaacggtgcagggaaagtctttcaggcggtcggcaaatgttttatagtgctggaatgcaaggatggtggtaggcaccagtacggcagcctgcttaccatctacaatagatttaaacgctgcgcggatggcgacttctgttttaccgaaacctacatctccgcacacgagccggtccatcggcgccggcgattccatgtcgcgtttcacatcggcggtagccttgctctgatccggcgtatcttcgtagatgaaagaggcttccagttctgtttgcagataggtatccggcgtatgcgcaaagccttgctgggctttacgtaccgcgtatagtttgatcaggtctttggcaatatcttttacctgcgttttggctttttccttcagcttatcccaggcatcgctgcccagtttatttactttaggttccacgccttctttgccggtgtatttactgattttatgcagggagttgatatttacatacaacaggtcgttgtttttgtaaatgatgcggatagcttcctgcattttaccccctacttcaattttctggagaccgctgtacatgcccacgccatgatcaatatgcgttacaaagtcgccagattgcagctcccgcaaggttttcatggtaatcgccttattcttgttgtaggcttgttttaccttgtatttatggaagcgctggaagatctggtgatcggtatagcaggccagtttcagcgaatgatcaatgaacccgctgctgatggcaaccgggatggggaagaatacaaaatctgctttaaggtcctcgaatatactgcgcaaacgttccagctgacgcgggttgtctgagaatataaagagggagtatttattgctgttatgtttaccgagatctttaatcagcagatcaaactgccggttaaacacgggttgttcctgtgtatcgaaggcgatgagctgaggctggtagccgttgtctgtcaaccaatctttattaccaaaaacaattgttggcttttgcagcagttgttccagtagtggggtggctttcacaaaatcctcttccttcagcaccatttcttcatcttcatccactttcactttctgaccggtgagcaggaaatcatccagccgctgttccatttgttctatcacgccttttacataggaaggatctttcatccatactacggtattggcgggcaggaattctgtgagtggtgttttgctgtggtctgccgcatgggtgtccatgttggcgattaaggttacctgtgtgagcctgcgttcactaagctgtgattccggatcaaacaggcggatagaatctatatcttctccaaataattcaatacggtagggcttttcgttaccaaaggaatagatatccaggatacctccccttacggcatactgaccgggttcatacacaaaatcggtggcgtgaaaaccccagccgatgagttgttccagcagcggatctactttcagtacatcgcctactttcagttgcaccatattggcgctgaaggcctgattcccggctactttctcccagagtgcttccggataggtgaccaggatctttttcctcacggtatccccggaaaatttcatgagcgcttccgtacggagcatactatggctgccgttgatttcatggaactgaccggctttcttaaatgagtcggggaaatagaaaatatccagtgcctggctgagttgctccaggtcgttatggaaataggctgcctcctctctatcgtttaagatgaagagatggtttgcatctgcatgcgcccaggtgctgactgccacaaaatttattgcgcttccactaatggaggagagctgaaagtattgtggggtgggtgattgaatccccttcaccagcgactgcagacgcgcatcacgttgaaatagttgtaatacagcctgtaaattcatgaagaatgcaaaggtacgaagatttaccgattttgagatttgatcagggaagatatttagagaagatacttccgcttttcataataaaaaaaacaaataagaagagatcccattagtagaatgccaaattttcgctatattcaataagaccaaactcaacttccatgctggacgtatggcataccggaatcgtaactaaattggtggatgaaacccacaatacgcgccgtttctggatacaggtaccggacatggaacggtttgatttcaaaccaggacaatttgtaaccctggaccttcctattcacgagaaaaagaacaaacgctggcgtagttattccattgcttcccatccggacggcaccaatgtaattgagctggtgatcgttttactggagggagggttggggagtacttacctgttcaatgaaataaaggaaggaagcgaactgttgctgcgtggtccacagggagttttcatactgcccgaacagttagacaaggaattattcctgatttgcacaggtaccggcatagcgccattccgttctatggcgcattacattcaactgcatggcgtaccgcatgcgcctattcaccttattttcggcgtccgctaccagcacgacctgctctatgcagctgagttagagcaattagcggcctctttacccaatttcaactacattcccactttatcgcgtgaagaaaactggagcggcaaaaaaggttatgtgcatgctgtttatgaagaactgctgcagaacaagcgtcctgccaacttctttctttgcggctggaaagccatgatcgacgaggctaagcaacggatacaagccatgggttacgaccggcatgatattcaccaggaattgtatggctaaaagcggtatcccattccaaattcaggaatagacagcggaaaagcatacctggaggaaatgatatttgtaaaccctcacttcgttaaagggctgcaacagttatatagtttcgtataggcataaagagtgcttatactaaatataacggttgtagcccttatcttttactagagaattttatttaataccagtgctttcacttcagacagcggaatgcgttcctgctccatgctgtcgcggtgacggatggtcactgtaccatcttcttttgtctgatgatcaatggttacgcagaaaggcgtaccaatggcatcctggcggcggtagcgtttaccgatggcatctttttcttcgtaaaaacaatagaatgcctgtttgcaatcattcatcagctctcttgccagttcgggtaaaccatcttttttcgtcagcgggaaaatggccagtttcacaggcgccagcttagcaggcaggcgaagtaccacgcggctatcttctttttccggtgtgctcagatcctcttctgcataagcattacagatggtcagcaggaacatacgatccaaaccgatagaagtttctatcacataaggaacatagttctgattgatttctgtgtcgaagtactgaatttttttcttgctgtattcctggtgttgtttcagatcaaaatcagtgcgggagtggataccttctacttctttgaagccgaatgggaactcgtattcaatgtccacagcggcatctgcatagtgcgctaatttgatgtgatctttaaaatgatattttgccggatcgatgccgaggctcaggtgccactgcatacgttcttctttccatttctcataccattcctgctgggtgccgggacgtacaaagaattgcatttccatctgctcaaattcgcgcatgcggaaaataaactggcgggctacaatttcatttctgaaagctttaccaatttgtgcaataccaaacggcactttcattctgccggttttctgcacgttgaggaagtttacgaagataccctgggccgtttccggacgcaggtatatttcgctggcttcatctgttacgctgcccagctgggtggagaacatcaggttaaactgacgtacatcggtccagttggaagtaccgcttactgtgcattttattttgttgctttctatcagtgttttgagacctgcaaaatcattttctttcagcagttcatccatctgcgccagaagggcattgccggcttcctgtggtaatgtttctgcataaccttcaatcaggtgatccacacggtaacgtttattgctatccttgttatcgatcatcgggtcgctgaaattatccacgtgtccggacgccttccaggtagtaggatgcataaagatggcagcatcgatccccacgatgttttcgtgcaactgggtcatgcttttccaccaataatccttaatgtttttcttcaattctgaaccgtactgaccgtagtcgtatacggcgctgagtccatcgtaaatttcgctggactgaaaaacaaaaccatattctttacaatgcgatatgatcgcctggaatttattctgatctgtagacatagtggcgcaaagataaagggctattttgaaaatacgtatgcgattattaaataatttataaactggtgattagccttcctggacgatctccggctcatgtggaatttcaatttgtttgatccaaaccgcataatcattgggataaatctgtgcaccgaaatattgtacgtaattgcgggtaaatacggccccaaaatacaggatggccgcggaatagtatacccacaacaatataataacaatggagccggcagcgccgtaggtagagcccaccctgctggcgcccagataataaccgatcgcaaatttaccgatcataaaaaggatggccgtggcaatagcgcccacccgtacgtctttccacttgatccgtgcatcgggcagcactttaaaaatgatggcaaacaatgtagcgatcaccacaaacggcactacaaagtcggccagggaaaagaggatacctgatgtaagcttacccggaagcaggttcaccaccagcgcggagaacaattccaccaaaccgttgatggccagtgataccagcaaaatgaaccccaggcttacaaccagtgaaaacgataacaacctgttcagtatcatccgtaacaagccattctttttaggtttggatttcagtcgccagatgaaatttatggagtcctggatttccgcgaataccccggtggcgccaatgatcagggtaatgaaccctaccatagtggcccagctcatatcaccggaaagagaggcgtttttaatcatggactgtatctgtatggcagcatcattgcctaccagcccgcggatctggccgtaaatatttccttcgatagcatccctgcccaggaacaggtcgcataaaaagataataatgatcagcatgggcgccacggaaaagatcgtataataggccagggcggcactgagcttcatcactttatcatctataaaatcaataccggattgcttcagtacctgccagatgattttaagcttgctcggttttttcatagcagcattttagtaacagtaaacaaaaagtatgcaggctgtattaagactttaatttagggttgttatgatgccgttgcgcatcacggatattcttcttttcaaaattcttttccagggctactgtcatatcaataccggtttgattggcaatacaaagcaacacccacatcacatcggccagttcatctgccagcagctttttattatcactttccttcgacgactgatccccatacttacgggccatgatacgggccacttcccctacttcttctgtaaggatggccatgttggtgagctcactgaaatagcgcacaccggtagtattgatccagttatcgattttttgctgggcttcctgaatggtcatgaattagtttttatttattaaagataatggattgactttattcccggttgtgtgaatctatgatgatcgtaacgggaccatcatttaacaacgccactttcatatcagccccgaaaataccgcgctgaatggtagtgcccatatcctgttccagttgcacgatcattttttcgtacagcggaatcgcaacatccggcttactggcacggatatacgaagggcggtttccctttttggtggaggcgtgcagggtgaactggctgacgagcagaatatcgccgtgaacatctttcacagatacattcatcactccttcatcgtcgttaaagatccggaggttcactattttagcactcagccactgaatatcttcttccgtatcgatatcttcaatacccagcagcaccagcaggccggtttggatttcaccggttacggccccgtctactgtaacagatgcggaactgacacgttgtataactgctctcatggatttttatttaacgccggaaaattaaggcaaatcgtttgtatctgtaacatattacaccccgtttgcgtttaacaggaaccaaaatcaatgttctatgacccgtatctgttacctgtttatcagcgtacttttatttacagcctgtaccacatcttccgagaaaaatccctgcgagggcatcgtgtgcgactatatggctcctgcctgtaaattcaaactggtagaagctggaaccggtcgcgatcttgtttatggtccctatgcccgcattcccgtagatagtatcaaaatactgatgcaggatactactataaaggttaaacaagtgatagatacacccagtaataccgccttgttatatttttatgtgctggggcctcaaaccctgcgggttggcaggccggctaaggttaccctggataaattgactttcctgtcaagatcagttggctgctgcggcacggagctatacagtttgcagttaaacgacaacccggttgcagtgccccgggattccgccggtgttttcctgatcccttatactttataaatgccgttataaaacgatgccgctgcattaaatgttaaaccagggaaaccgctgcccctggtaaaaacagcacgtattcgccgtaatttgtaataaattgcacttcctaaggcattttttatattataaattaaatcaagatgaatatcaatgtgacccccgaaatcacgttccgcacggcccgcagcggtggcagcggcggacaaaacgtgaataaggtggaaacgatggtggaaggctacttcgatatcatggcttctgcccttttaacccaggaacaaaaaacagtgctgacggagaagttatcgaaccgtatcaacgcagatggcctgctccaggtaaagtcgcagacggagcgcacccagctggggaacaaacaaacagtgatttccaaaatgaatgacctgatcaacaaagcgctgataccacgcaaaaagcgcgtacctacgcggccctccaaagctgctaaggaaaaacgcatccagtcgaaaaagaagcattccgataaaaagcagcaacggagagggggatttgagtaagccaggtcaccggtcaatcctcataaatccgcgattcgtaatccgtaattcgtaatttgcgtcaaaatatttgggaattgagtattaagaacctggcaggacaaacggtattttacggattgagtaacatagtgagcaaattgctcaattatttccttactcctttttatctgaccatcttaacccgtgcatcattcggggagatgtccaacgtatacgcctatataccgtttgccaatattgtgctgacttatggcatggaaacggcctttttccgtttcgccaaaaaggagaacaaagcccatgtactgggtacttccaccatttccctcttactttccactatcagcattaccattttactgttgttgttgcggtcgccggtcattaactcgtatgccggcgagctggcaggactgaatggccatcccacctattacacctatgtagtgctgttgatggcgtttgatgcgctcacagccattccttttgcgcaactgcggctggaaggacggcctatgagatatgctgccattcgtatagccggaatagttactaccatctttttcaatattttcttcctggtcatttgcccgaaactgtatgctgccggccatcactggttgccggatctccaaagcggcagcgaccagacggggtatatttacctgagcaacatgctgggcagcgccattacgctggtgctgtttcttccccagatccgcaaaatagaatggaggtttgataccggtttatggaaacaaatgatgcactatgcccttccgctgatcgttgtgggaatggcgggcatggttaatgaaacgttcgacagggcctggtttttaccgcagttcctgccaggcgataacatggaagccaaaaaagaagtcattgcgctgtacagcgccaactataaactggccatcctgattaccatgtttatacaggcattccggttaggagccgagccctttttctttaaacaggcggaaagcggcgatccgaggaaaatgtatgcacggatcatgaagctgtttgtgatcatgctttgcttcatgttcctgtttgtaagtctttacctgaatatctggaaggcgttcctccgggtaccgttctactaccaggggatgcgtattgtaccggtattgctgctggccaacatgttcctgggtatttattacaatctcacgatctggtttaagctcacggaccgcaccaaaacgggcgcggtgattaccatcattaccgccgtactggccttcctgctcaattactggtggataccggtgatgggctattatggcgctgcactggcaacgatggtatgttattttgtacaaatggtcatctgctatgtgtgggggcagaagtattaccccatcccttaccatcttcctaaactcattacctacatggggctggccgccggcatttactatatattcagctggctcaatgccacggtgctgtcgccgaaagacatttatgccctcaaaccccttccgctcgcagtggccacggctttctttctggcttatgcctggtttattttccgtatggagaagaaggagtttgcccgtttaccggtgatcgggaagtttattaaagtaggctaatccaccaggaaaggattgtgtttcttttcaaagcctatagtggtggctggtccgtggccggggaatacccttacctcatccggtaatacaaacatttgctcccggatgcttttcagcagggtggcatgattacctcccggcagatcggtacggccaatgctctggtaaaacaggacgtcgcccccaattacgaaatgctggcccgggcaataaaaggctacacttcccggagaatggccaggggtaaacaataccgttaactcatcggcgccaaaaagaatcttttccccttctgtaaggtaacggccggcctccggggagggatcaaaaggaatgttgtacatccccgccgcccgctgggaattgtccagtaccggctgttccagctcatgaaactccggacgcactttatacgtatctgatacgagcttattaccgaatatatgatcaaagtggcagtgcgtattcaataatcttataacatttaacccgtgcgtttgtatatattgtaataattcttttctttcgtcctgaaaataacaccctgggtctataattatacattccttttttccgttaataagcaggaaagtgttttcttgtagtggaccaaaagtgaattgttgtatttcaatcattgtaacccgatttttttaggctaattttaaaacagatcacaatattatcaatactttctgtatgaacagatttattaccaggttattattccacggtaccctattacttggaacgatagtatcccaggcccagaccaatacagtagaattcggacaaaatcgtgtgcaattcaagaacttcaagtggagatactatcaaagccggcatttcaacacctatttcgcccagaacgggctggaacttggtaagtatgcggcacaggtagccgaaaaggaattaccccagctggaacagttcatggaatccaaccccagacagcgtattaatattgtggtttacaactctttcggggaaatgaagcagtccaatatcggtattggcgtggattggcagaacacaggaggagtgaccaaactggtgggtaacaaaatgatcgtctatttcgacggtaaccatgaaaacctccgccgccagatccggcaggggattgcccgcatcatgctggaaacgctgctgtttggggaagatatcggcgaatttgccggtaatgctgccctgatcgacttcccgaaatggttcaccgatggctttattggctatgccgccgaaaactggaccgccaggcaggatgaggaactgaagctcatcatcatgtccggcaaatacagcaacttcaattccctcgcatatgaccatccccttttagccggccaggcgttctggtactatgtggaaagcaagtacggcaaagatgccgtgccttatctcatgtatatcacccgcattaaccgtggattgaaaaaaggctttgagcaggtacttaaccaaacgccgaagaaagccactaaagacttctttgtattttatcagaaaagattccaggaagataaccgcagaaggaaaacttctgccaaaggccgtactatcgtagcccaggaaattacgccgaaagccgactactaccgctttaacccgaatcctaaaaataattcctacgcagtagttgagtttaaaaaaggagtttaccgcgtacagatccaacttggctggaataagccaaaagtactgctgcatagcggtgtaatgcaactggccaaccaggtagatccaaactatccgcagatggcctggaacaccaaaggcaaccgcctggccgttgtgtacgagcacgaaggcaaaaccaaactgatgatctatgacctgatcacccgcacgactatacgccaggaactgaaccagtttgaccggatcatcgactttaaatacatgccggtacaggaaaataccctgttgttgtctgccgtgaaaaacggacacaccgacatctttacctataacattagcaactctaaaacagaccagatcaccaacgacgtgtacgatgacctggatccatcctttgccgcattccccggcaaaagcggtattctctattcttccaacaggcccggcccaaaaggaaggggcagcgatacttcactgctgaacaatcctttcaacatctttatggtggacaactggaacaggagctctgaaaagcagatcacccagctgaccgacctgcagtatggcaatgccaaactgcccatgcagtataacaccacccactttacctttgtttctgatgccaacggtatccgtaaccgttatgccggcttcttcaagtcgcaggcagatggcgtggattccctcttttatgtaggctctgaaatcctccataaccccgaccaggaagaactggattcagcgatggccgcctatggttctaccgccccggattcagtagaggcgatcactatcaccaaagattctacctatactttccctatttctaactatccttacggtatccaggaatcacggattaccggtgaaaagggagaagtatcggaagtagtgcagtatgcggatatcaaacggctgatgaagctgaaagtagatactgtggtgttgaaaaaaaggaatataacggcaaaaaataccaatttcaggaaagcccagatgcatgccgacagtttacgtttaggcctgcctacttacctggcgccgtcaaaagatacttccacacatcctaatttcttccagaacgagttcgggaatgagccggccgataccagcaacaacgctaatacggccaacgaaccggcgctgtttgaaaaaaggaaagaaaatgaatcgatccttaaaaaatcgaaactgttcccatataaattcaaattcgcttccgattacctgatcctgcaactggataactccatcctggtaaataaataccagccatttaccggtcctcccagcggtcctatccgccttaccgacccggtgaacgggttaatccgcattggagtaagcgatttgtttgaagatctgaaattcaacggcggcttccgtattccgtcttccctgcagggatcggaatacttctttacggccaattacctgaagaaacgcttcgactataaattcacttactaccgtaaagtggataagagcagtggatttgccatccgtgaccagtctggtaacgattccgcttttgttcctaccaaaatgatcaccaacatttaccagggcgaaatgaggtatcctttcgaccaggtgaggagtatccgtttatcagcaggtatacgtaccgataaactggtagtccagtcagagaacaaagaatcactgatagcgcctgattacaaggaaacgtatgctttaatgcgcctggaatacgtatacgacaatacgatcaacccggctattaatatctggaatggtacccgttataaaatttatggagaaaccaatgcacagctgaccaatggcggactgaatgagttattcaatccgggtctttccgccggcgcccagggcaggtttacctataacatgggagtagatatccgtcactatacaaagatttaccgcaactttatctgggctacacgttttgcaatggatatgtcgtggggaacacgtaaactgctgtattacctgggcggtatcgacaactggctgaaccctcagatcaacaccaggactccggtaaaccttagtgaaaactatgctttccagacccttgcgggtaacctgcgcggctacaaacagaatgcaaggaatggtaacaatgtgatgttgctgaacacagagctccgtttaccggtgtttgccactttcatcgacaaaccgatcaactctgcgttcctgcgcaatttccaggttacctctttcattgacataggtaccgcctggaataaaaagctgagctttaaagacgccaattatactacttatgacgatggtcagggtataaccacccgcatcaaagaaggcttcctcggacctttcgtaggtggttatggttttggtgctcgcaccaccattgccggctacttcctccgcgcagatgcaggctggcctgctgtagcgtttttcagaggcagtccgatctggtacttcggtatgggcgtcgacttttaaacggatcgccttcggcgatggaaattgtcttggagcaggattacgctgattatactgattgcactgatttgatcctgtttgatttttaaaagatttaggggagatagaagcggatatcgcttttatctcccctaattgttaaataaaatcccagaaaataaaatcagtgcaatcagtataatcagcgtaatcctgctccaagacaatttccatcgccgaaggcgatcctacgcgtgttgctttttcaccagcgggtacattaagctcaggaatattcccatacagacggtaaaagcccaggcatgccggttttccacgggatgcaggaaaatgtccctcatatctcccagcagcgtaagcgggtcttttacaatatcccagctgttatagcgaagataccggccaatatatacgcccattccgcataggaacattacagggaaagtaaataaccatgcaggccagcggctatgccggttgctccataatttctccatgctgcggatagacatatacccgaacatcatgccgttccaggcgaaagagaaaatcacaaacagatcaaaccacaatggcacgccgccatcaaataaatgaaacaggtccgtaaggatgtagggggcgttgggaataaacagcagccatactataaagcagccgtaccagttataccggtttttgatttgttccgggtgcttttccatccagccggtgatagcaaaaggaatgaaggccaggaaaaggttccagatcagtgatacccgcagatagctgccggtatgaactacacgacaaagaagcaacgccatactgaacagtacagatgtatacagggtgtattggtgccgcgaccggcctatacggtgttgtaataaacgaatggttctcatcaattgcatatggttacttttagtcaaattaaaatatagggaataaatacgacagccccgataataacggctgccacagccgctatcagtacagcgccggccgctacatccttgatgaacttcactttcggatgcagctgtggcgaaagatgatccattattttttcgataactgtattaagcatttctgtaatccacaccaatgtaatggcgaggatgatccaaatccattccggcgttgctattttataccagcaaccggctgccaccaccacgatggtagcgagggcgtgaatacgcgcatgtggctcactgcgcaggaaagcggcaataccactgaatgcgtatccgaagctggccaaccgtttgctgatataagagtttcccatgtttgtttttattgctggatattggtgtttttctgtcctaatttatcccatttgatggtggtgctgaaatacatgatcagggcgaggatgataaagagtcctaagcttcccatcagcagtgcctgatcttctgcactgataatcacgtaaatgaatccgtaaaggatggcaagcgtagccccgatgccggctgcaatgcggccgcttttaaaggcagcagccgtatacgcaataatcagacctattgtgagcacactggcaataagataagccatagtaaagttaatttgttctgaaatagagatgagcagggtataaaaaatacagagggctaacccgatgagggcatattgtaatggatgaagggcgcggcgttgtgatagctcaataaaataaaagacaaaaaaagttaacccaatgatcatgacggcatactttaccgcccgcatagacatctggtagctttcggcaggcatgaataacttaatcccgaaatcggcggaatggatgtcaaatttcttgccttcccagctttgcggatagttgcggttcaggtgttgtatctgccaggtagcggcaaagcctttatcgtccacccggcgggttttcggcgggaacgcttcatcgaatgcgggatcagtccagctggaattgatgcctaccatggttgttttaccaatgggagaaaaactgatccgtccggagccctttatccccagctccagggagaagctaccgcccagggcgccggcgtcgccggggacaaccgataccggggtttggataccattatcaaacaggtccttgctgaccaaaccggggttaaataaataggatttaccattccacatcatctgcacctggttgccaatgccccgcaaatcgctgatgccaatgagtactgacgcatgttcccaatctaaggcggaaggagggatattaagcgacaacagttcattgcggttaaaagtgccgctcagctgcaacctggcattgtacacggctacattgaaaataccgcggtgcagtttttcgggcaacagctctccgttgatccgtaaactatccggcaggaggtacacataggttgcttcgtcggttccggctttatacggaatggccagcactggtcctgtaatattctgttcgcctccccagcggctgccgatttcctgggtggcttcattttgccggtcgcggcgttcccagataatgttttgaatcatcgccgctggtacgagcagtaccagcgtcaatactgagatgatgatcgctttaatagcgtaggcgtagcggtcaaagaaagaaggagatccgtttgttgaaggttccatattttttatttttaaaagtactttgtatttcaaagtaaaaagacaaaaaaaatttatttagtgaatttgatcatatgctcaagcgccgcgatatggcctttgaaagctttttcgccagccgcggtaatagcataggtagtattggttttcctgccaataaagcccttatgcactttgagatacccgttctcttcaagtgtattgagatgcgatgccaggttaccatcggttacttccagcatctgtttgagatcgttgaaatttacttcctcgttcaccatcaatacactcataacgcccaggcgtatacggctctcgaaaatcttatttaagttacctatcgggttcatgcgattgattaaactgtccctttccgttcatatttccaccacatcagcgctccataaatgatgtgcagtaaaccgaaacctatagcccaaaaataaagaccatcgttcaaatagaaaagattaagtataccgagaacaacttcacagattcccaggtacctcacatcgggcaaagtatatttactggcattgatgatggccaacccataaaataccaggcaggtaggggctatcagtccttcctggtggttaaataataacccggctataaaagcgccgcccgccgccaaaggaatcgctgtgttgatcagcactttccgcgacgttaagtcccagatcggtaaattatttttcttcgccttgcgccaggtaaaaaaagttccggcgataagcgctgccgctaacacagaaaatcccaaaacaattaaccggtacttcagcactatgaaatctgaatgactatgtacaccggtagtgttccacctgaaataatattcattcagccacatattggcaataaatgcgccgatcaggccacagataccggcggagataccgcttaatccactcagcgaaatgaaacgactgctgcgttccatcattcgcttaatgtctgttaatgcctgcagatgttgttggtctgtcatacaaaaaagtactttgcaatacaaagctaatagaaaaatccgaatcacaaaatataattttttgttataactgcgttacctataggatactgactgtccagaatcgcaataaatgatataatattgttgtcagatatggttggctggaaaagaatattagcaataatcatcggcgtaagcggctggggttcgggtttgatggcgcagcagtacaaggttagtggagtggttagagacgcgcactcacaggaaatcattccgttcgccactcttcagtttgtgcgtacccaaacaggtatggttagcaacgcggaagggaaatacctcttcgaactaaatgttatcccatcagattcattgctggtcagggtaatgggatataacatccttaaattgccggttaacaaagatcagaaagaacaggtcatcaactttgaggtaacccgctcagatgtttccctgaaaacatacgaggtgaaagccaacgtcaactgggcactcattctcctgaaacaaatcgttaaacataaaccggagaataattataatcgcctcgataactacaaatacgaggtatataataagctggagctggacatgaagaatctcaacaaagagaaactcgggaaaaaccgcttcaccaaaccgtttgcgtttattcttgataacatagacagtacttctgaagacaaacctttcctacccattttcctcacggaaacattatcggattattatttccagtcgagcccccgcaaaacaaaagaaatcatcaaggccgcccgaacgtcgggaatagataatgaaagcgtgaccaaattcctgggagggatgtaccagaatgtaaatgtatacgacaacttcatcccggtattcgataaactgtttgtaagtcccattcaccacaacggcgccttctactacgattactccattgcagatacacaatacgtcaacagccagcggtttattaaactaaacttcacgcctaaacgcaaaggagaaaatacttttattggtgatatctgggtacatgataccacttacgccgtacaaaaaactacgctgtcggtaccccgggacgccaacatcaacttcgtccgcaaaatcagcatggtacaggaattccggcaattacccgatagctcctggttcctctataaagataaatttattgccgacttctgggcgccaagccccaagccggggaaaacgtttgacttcataggccgtaaaaccacgacttatgatgacgtaattacgaatgataccgctgctaccaacatcttcagtgataaaaaatatccggaaaatgtaatggtgctggatagcgcaagagcacggaaggattccttctggatggataaccgcccggaaaatctcagcaaaaatgaagaaggcatctacaaaatggtggatacccttcagaaaatgccgcttttccggagctattcaaatacaatccggttcctcgctaccggctataagccctttggccctattgaatggggaccttactattacctgttttcccaaaacaggctggaaggtttccgtttacgactggacctcggtaccaccccgcagttcaataaagatctgtacctgtacggttacctggcctatggcttcacggatcatgtatacaaggggaaaatgtcggcgctatggctgctgaaaagacatccgcgtacctatctgtatgcatctttcacaaaagacctggacaatggcacccactactatgatgaagtaggtacggataacatctttaccctcgccatccggaaaaatggggtaccgcagaaattcttaatggtgaatgaaaaacggtttgaatttttcaaagaatactacagcggtttttcccaccagatatcactcacacacaaacaggtaagaccattcgaaccgcttccaaccgctgctttttatccgaaagcgcccgatggccgcgatccgctgaccagcatggaggtagaactgaaattccgctatgccttccatgaacaattcctggaagggaattattaccggatcagcctgggtagcaaatatcccattgcagaactgaaatttgctgccggtataccaggcgtagccaacagcggacaaaaatatcaacgcctttcactcagcgtatcagattatgtaaaactgccacctttcggctctttttactataatgtttttggcggtaaaatttttggtacagtaccttatacttcgcttgaagtgcatcccggtaacgaaatttactactacaataagtatgctttcaacatgatgaaccgctttgaattcatcagtgatcaatatgcaggctttaacgtggagcataccattggtaatggtatcttcggttatattccactgattaaaaaactgaaatggcgccagttctggaccgccaaaggcgtaataggttccttatcggaatccaacaaacaactgaatctcaacaacggctttgcattcaaaacattacaaggtaatccttacctcgaactgggtacgggcatagaaaatatttttaaattcctgcgggtagattttatatggagagtaacaccggatgtgacaccgggagaacctgccaacaagcgttttggcgtattcggtagcttcaaattacagttttaacctgctgctcatgaaagatgtaacacataccccgctgtttgaatgcatcctgcggggagaaatagacggcagctcgtacgacctggaaaatgactatcaatgtatcaaaatgcaattggatggagcagagaaaaaattgcagctgaggtttattaatgatgattataaaatcattcttgagtttcatcaaactacgataacgtgcttcaccatcctgcctgaaaaaagcagcggcagtacctcgctgacaagcttctaccggggacaattcaagttcaataacaaccttcacgaaataacggcacaaggcaaatactattactatctatctttcctcggcaacgatgcgatagagctgtttgccaaacgtgttaccctatctttaagccggttgaattcctgaattaaactgtcattaaacatgatcagctgcttcgcagataatgctgcaggcccattttatttcttcgggcgtaatgatcaggggaggcacgatgcgcatacattctgcggcaaagaggaaccagtcggtgagcacacctttatcgatgcaataatcaattacctttttatttaccgggaaattttcaaattctactgcgatcatcaatcctaatgagcgtaccgatttaatagccggatgtttcaggtgttccaggaacaactgaccttttgcattcacttctttcaacagatcctggtccagcaatgcctggaagcctgcacggcctgcggcgcaatttacagggtggcctccaaacgtagtgatatggcctaacacagggttgttggtcaatgtccacatgatgtcgcgggaggcgatgaaagcgcctaatggcatgcccccgccgagtgctttaccaagcagtaatacatcgggtacaataccaaattgttcgaaagcccacaacgtaccgtttctcccaaaaccacactgaatttcatccagtataagcaaggcgccggtagccgaacatttttcgcgcagcgcgtgtagccattcccgttgtggcactattacgccgccttccgcctgcacactttctgcgatcacggcggcggtgtttccggtgatcagctccagcgacgcaaagttattatactccaggtgttgtatacccggcaacaaaggccggtaagcgttgcgccagtattcatcgccaaggatgctcagcgctccttgtgtagatccatgataactacggttaaaagcagcaatttccgtccggccggtataccgtttggccagtttcatggcgccttccacggcttcggctcctgaattggtaaaatatacacagtttaactgttccggaagatgctgggtgagcaggctggcaaaggccacctgcggcgattgtacaaactcaccatacaccagcaggtgcatatattgctgcgcctgttcctgtatggcctttacaacggcaggatggcaatgtcctacgttacatacactgataccggcaatcaggtcgagataccttttcccgtttacatcccacatatacatgccttccgctttcacgatctccaatgccagaggagcatcggaggtttgcgctacgtgctgcaaaaaaagttgcctgttgttcatatcactaactgctctgttctttgcgaagttagaaaacaactgctaattagtaattgttatatttgtaacataagcactaaaacatttaattatggcgcacattattccactgaacggagttactcctcaaattcctgaagactgttacattgcccccaatgctactatagtaggggatgtagtaatgggtaaaggttgcacgatatggttcaacgctgttgttcgcggcgatgtaaacagcatccgcctcggcgaaaatgtgaacgtacaggatggtgcagtgattcattgtacttatcagaaaaccaaaacgattgtaggcaataatgtgtctataggccataatgccattctgcatggctgtaccattgaggataatgtgctggtaggcatgggcgccattgttatggacaatgcccgtgtaagcagcaacagcatcattgctgccggcgccgttgtactgagcgacacgcatgtggaaccaggtaccatttacgccggtgtacccgcccgcaaagtaaaagatattgatatggccctcatcagcggggaaatcaaccgtatttcaaaaaactacagcatgtacgcttcctggtaccagaacgcagaggaagtaaaagtgccttagtaatcatcttacaaaaaaatgttatattgcaggcaaataccctcctatgaaaatactcatatgcctgctgacattgggaagcatcctgtttgccagctgttcatcgcagaaaacaggatgccctgcttccaactactacaccaaagatataaagcaacaaaaccgtaaggctggcaaacaaatgcggctgttttaaacctatcctatgcgcaaagtcatcccactggccctggtggccattatcatgtgctttactgcctgcagaacacaaaaaaaaggctgcccgcaacccaaacggaactggggggcagaaaaagtgctggacgaattaggcaaacccagaaaaggctgatcagtattgttcttcctcaatggtttccaggatggtagcatagctcacatacctgtctacatcaatatgcccttcctccacggctactttcaccgcacaaccgggctcattgatatgcaaacagttattaaactggcattgggcaatataaggttgcatttcaaggaaatagtgggagagttccggctttggaatatccacgatcccaaattccctgacgccgggggtatctatcaaacaaccgccaaaaggcaggtcgtacatttcagcagaagtagtagtgtgcaatcccttgccactccagccgctcactgctttggtccgcagatcgagaccgggcatcagtacattgatcagggaagatttacccaccccggaatgccccgccattaaggtggttttgtctttcaactgcgcccttaccgtatctaccccgttgccgttcgctgcagagatcagtaatacctggtagccgatactgctgtacagctcttccagttcctcaaatttttcgttttccttctctttataaatatcctgcttgttgaaaacaagtatcaccgggatatgataagctgctgctgtaaccaggaaacgatcaataaagccctgcgaagtgcgtggttcttttacggtacacaccagcatcgcctgatccatattagccgctacaatatgttttttatttttaccatgaggggaactgcgcactatataattcttccgggggcctatttccgttatcatggcatttttggcgttggcatcactgtcatcttccacaatttccactacgtcgcccacagcgataggattagtagaagtaatatcttcattctttttgaagatacctttcatcctcgcctggaatgtttcaccagtggccgttttaaccacataccagcttcccgttgatttatatactgttgcttgcataagatccccaaaggtaagcgaattttgttttatgggggagcgccttcggcgctggaaattgtcttggagcaggattacgctgattttactgattacactgatttgatcacttttgattttactttttgattttataaagatgaagggagatataagcggatatattcgctcgtatctcccttcatctttataaaatcaaaaagtaaaatcaaaacataatcaaatcaagctaatcagtaaaatcagcgtaatcctgctccaagacaatttccagcgccgaaggcgctatggcaggctcttgaaaagcgtataccgcagcacggtttccagcaggatgcaacctaaggcaatcatcgccagcaggaagaagtgttctgcaaaacgtttataggaagtgatttccacctttgttttttccagctggtcaatttcactgtagatgctcttcagatcgtttgtattggtggcccggaagtatttaccaccggtctcttttgaaatctttttcatcagtggttcgtcgatctgcacatcctgcatcaccatttgcacgctgccatcagacatgggcatgggaaacggcgctttaccaatagtacccacaccaatggtgtacacacggatcttaaatgccttggcaatttccagtgcggtgagcggatctacgagaccggtattattcaccccatctgtgaggaggatgatcactttacttttagcatgactgttacgcaggcggtctaccgaagtagcgagtcccataccgatggcggtaccatcctgcaacatgccgcttttcacctgcatgatctggtttttcagcaccgcatgatccgtagtgataggacattgtgtaaagctttccccggaaaacaccaccagtcctatacgatcgctgatgcgtttatccacgaaatcggaggccacttttttcgctgcctccatacggttgggctgcagatcttccgccagcatactgccggagatatcgatagccattacaatgtcgatgccttcactgtcgatgctttcagaagtgttggaagtttgtggtcttgccagtgctacaatgagtgcaattaccgccaggatacgcaacaccagtaacaggggtctgaaacgcactttccaggataccggcagtcctttcaaaccttcaatggaagataccatcattacactttgcctgcctctgcgccgtgcaaagtaccagtatatcaacaccggtaccagcagcagaagccacaggacaaccgggtaggcaaattcaatatttttccaggttgaaaaatccatcaatttttaattaagatccatgctgactttatgctttttcgagggtagcatcggtaccggtttcctcagccggacccgcttttggtttggtccactccaggatttcttcggctttccgcatacattcttcatgttcatctgccgttggttgcaatttggcaaactttgccagatccgcaatcgccaacagcgaacgcagtttgtccctttgctggttcagcttagtcaccggcttgatattctgcagtaattcctcactggtttgctccagcgcagcaatgctgaactgatgctcaaagtaggtacgcaggatatccgttaaccgggtatagtattgtttaatatcgccctgttgccataccttttcttccttcagcgctttcagctcctgtactgcaatttcgtatggggaaacggtaggcgtttgtataaccggcggcgtttttttacgggtacggagataccatatgagtccgccgatgatgagcacagctgcggcgcctataacgatatacagccagtagtcccagatgctccaggctacgccttttatttctttaattggtttgaatgctttagtggtatctactgctacggtgtttacatcaataccgataggcaatgtaatggcagaatcgggggtagcattggcgccgctgaaaacctcgaaacgcatggaaggaatatcccaatggccggagtcgaaactggtaagggtaaaagtctggtgaaggatgcgctgatcctggtttaccacggtatcaagattggagcgggttaccacctcaaaatgatccagtgaatcgggtaataccgggaagagcactttaaagttagcgtccttaaactgttgcgctgtcagcgtagcggtaagctgcagttttatctgctcaccgatcctgatactattggtatctgctttggcgattacatccacggcctgctgtgccagcagggagaaaggaaataacaaccccagtatgcaacataaaaacagacgccttatcacttgttgtttatacatgtttaatttgctctcctttaaatcttatgccctgttcaggaaaaatgtttgtaacgctttcacatagtcctcgtcggtacgtacgctcactaattctgcgccacttttcataaacgcatttttgcaatattgtgaatgctgcaggaattgctgctcataatactggcgtacgcggcggtcgttggtatcaacccattgcgtagcgcccgtttcagcgtctgctacctggatcagtcctaccggtggcaggtctttatcccgctggtcatatacctgcacccctactacatcatgccgttttgcggcgatgttcagtgcgtcctggtaatttccggataagaaatcgcttagcataaaaacgatgctgcgttttttggtagcattgttaaagaaacgcagggtttcttttatgttagttccttttcgtttaggcgtaaatgatagtagttcacggatgatgaaaagaatatgtgatttaccttttttaggagggatatatttctccatcccatcgctgaaaaagataacgcccaccttatcattatttttgatggcagaaaaagcgagtacagcgcacagttccgtgatcaggtcacgtttgtcctgctttttggtgccgaaggaagagctttcgctcatatccaccagcagcatcacggtaagttctctttcttcttcaaaaacctttacgaaaggatggttgaaccgtgctgttacattccagtcgatagatctcacatcatcaccaaactgatagtcccttacttcgctgaacgacataccccggcctttgaaggcgctatggtattcccccgcaaatatatggttggtaagccctttcgtcttaatctctatctgccttaccttttttaatatttcagccgtatccaatgggaaaaattttgagttgtgaattacgaataaatgcccggtccggcagcttttggctgctatggtacttctactgcgttcagtatttcactcaggatattttcgctggtaacgttttctgcttctgcttcataggttaaacctacgcggtgacgcataacgtcgaagcatatattacgtacatcttccgggatcacatagccgcgacgcttcatgaaagcgtaggctttggcagcccaggccaggttgatgctggctcttggcgaaccgccgtatgcgatgagcggtttcagtttattgagtttatattcttccggattacgggtggcaaaaacgatatcgaggatatatttttcgatcttctcatccatatacacttcccttaccagtttacgcgcttcgaggatatcggaaggctggataatgggacggatgggagccgagagttccgggttcaggttttgacggatgatctgtttttcttcttccttggtaggatagccaatcaccactttgagcatgaaacggtctacctgtgcttcgggcagggtgtaagtaccttcctgctcaatcgggttctgggtagccagtaccaggaagggctcgtccagtttgaaggtagtatcgccgatggtgatctgtctttcctgcatggcttccagcagggcgctctgtacttttgccggggcacggttgatttcatccgccaggataaagttggcgaagatggggcctctgcgtactacaaattcattcttttgctggttatagatcatggtacctatcacatccgcaggcaacaggtcaggcgtaaactggatacggctgaatttcgcgttgatagcggacgacagggacttgatagacaatgtttttgccagaccgggtacgccttccagcagtacgtggccctgggccagcaaaccgatgagcagtctctccaccatataacgctggccaacaattactttacctaactccattgtgagcaggtccacgaaggcgcttgcctggtgaatcttctcattcagttgccggatgtcggacgatgtattttccatgctaataatttttcaggtgtgctaaaataaacattctctggtcaaataaaacttatcactatgtgaatgggccgttaaaatgctgttaaacttgccactatggctcatttccggcaaataatcattctatgacgctgcctaaattaataaagccctgcatatttatataatatttttccctataacgtacctttgcggggaataagcgtctggcaaaaagccaacaatttaaaagcaacagtaatatggaagattttgagaagcgctggaaaccggtagaagatatgcttaccgaaagatttggtaaaaagcccaatatggaagccattcttttccttatcggcgtaaatgaaataaataatttaaagaagaaatataccaaagaacagaagcaggatctgatgcatgtggcagtatgtacgctgctgagccagagcggctactttgagctggatggctacgacgaagacggatggccgcatttcaaagagttacaacccgttccgaaaatggaaatgatggaacaggaaacctttctgaaagaacatgtaattgcttactttaccggtcacgaagaagcctaatacacttttatgaagaaactgctactgctgggtaccctgtttttgctgattgttaacctggcaactgccaaagaccggaaagtaaaagtaaccaccccttatggtaccatgatcatccggttatatgatcaaaccccgaaacaccgggataatttcatcaggctggccagacggcacttttacgacagcacgctgtttcaccgggttatccagacctttatgatccagggcggcgatccggattccaaacacgcccatgcgggcgatacattgggcaacggcgatgtggggtataccataccacctgagttccagctggacttattccaccgcaaaggcgcactgggagcagcccgggacgaccgtcccgataaggcttcttccggatgccagttttacatcgtgcagggcaaggtatttaccgatgagcaactggataagctggagcaaacaaggctcaaaggccgcaaaatcccaacagatcagcggcaggtatataaaacggaaggcggcagcccacacctcgatcaaaactatacggtgtttggccaggtaattaaaggcatggacgtgatcgataaaatcgccgcactaaaaaccgacagccacgacagaccattgcaggacgtacctgtgaagatccgtgtcataaagaaatggctgatcttctaaataaaaaaataccatgtccggagaaagtcaaaatttaagatagcttcccgtcaaaatcataatagtttctgtatttttacggctcaaaatcaaacttgatatgaattttccgtcaaatctgcgttacacaaaggatcacgaatggattttattagaaggtaacgtagctaccatcggtataactgaatttgcacaacgcgaattaggcgatatagttttcgttgatatcaattcattgagcaagccagtgaacgccgaagaagtttttggtacagtggaagcagtaaaaacagtatctgatctgtttatgcctgttgccggtaccgttagtgaagtgaatcctgcactggaggcttctccggaactggtaaaccaggatccttatggggaaggctggatggtgaaagtaactgttaacaacccggctgatgtggaagcactgctggatgctgctgcttaccaggcgctggtaggggaataattccgaccaaaataatcttttatataagaaaggacaacaggctacgttattgaacggtcagcctgttgtcctttttactggtagtactataacccgttcattaattaaaaaaggatcatgaaactcctgagatattatacgccagctattctatggatcatcctgatcctggttttgtgtaccctgccagggaaggacattccctccaactcattttttgataaaatccattttgacaaattcgttcacttcggcctgttcggaggcattgttttattcctgagcctcggcatctactggcaaaaaaaacacgtctctgcgggcacccttgtattgctggtgatttgtgctgcagggtatggccttgctatagaatttatccaggagtactgggctattggccgcagctttgatatgtttgacgtgctggccgacaccctgggtgctatcgccggcgtatgggtatttaaaattgtcagatccctgttcttcaaaaacgctgataaataaaaaatcccccctgtaaccaggggggaatgtatatctgcttatgagaaataagtattcttaatgttttttattactgttgaccagcttctttcttcgcgtcatttttcatcttatcatttgcgaagatagagaactcacaacgacggttggtagcgcggttagcgtctgaatcatttggcactttaggctgtgattcaccataccagaatccctgtatacggctcttagcaataccctgtgcttccagataagacattacactcttggttcttctttcagataaacccatgttgtactcatctgtacccttgtcgtcggtatgaccttccacacgtacataagtgtcaggatacttgttcaggataacagccagttgtttgatattgtcctgtgctacggcagacaggttagacttatcaaaaccaaataatacacctgcatcaaatgttacgttgataccttcacccacacgctctacggttgcatttggtacttccgtttttatttcctgcgcctgtttatccatttttttaccgatcaaagcaccaccagcaccgcctaatgcagcaccaataatagctcctaatgcagtattaccggctactttaccaattacagcaccagcggcagctccgccaccaacaccaattgcagcaccttttttagtattgtccatgccctgccaggttttacaactgaacaacatggttgcagacaagaccaaggctaccagaacattgatttttttcatcataataaatttagacatgaagggtttttagcattaattccgttgacaaaactaattgaaatcctgtatgcaaatagtttgccaacttgatttaacagtcacaacatattgataagtagaattaaataagcaataaaaaaattgcaggcataaatcacataacaataattgggcatgtaaaatgtaacgtgtacgactatataacaagcaaagtggtaaaaagattatccaagcagattttttaataatccgccgataccgccgccttcgccggcctgttgttgctgttgctgctgttgggcgccatttgataacaggctctttaaatcatccaggttcacctgtccgtcgccgtttttatccaaaccgccggaaagcccgcccagtataccgttcaggttaagtccctgtgcagaaccaccggtaagtgagttcaggataccatccaggctgaagctgctattgttgggatcctttgttttatttaccagggagcctaatacagttgggatcagggtagccgccagttgtgtagctgtacctttatccaggtggaatttctccaggagtgttccgataaaattgttggagatatttcctactacgggattagcggcggaagtatcgctgccggcgccacccagtaaagataacacgccttctgtgttaccactggccagttcctgttgcaaacccgttgcaatggaagaagtggctgcgcctattacggcttcattctgttcgttaggaatagcaggattgtttaccacagtaccctgggcattttcgcggacgaggtccattaattgctctaacatttgatgatgatttaggggaagaaaaaggttttccttagtgctacggcttgtgaccgctaactaaatgtaggatattttgtgtgattacgacttaacccggaggaaatttgtggaaagataacagcagggaaacacccgtcactttccacaaatttaaaaccggtgatcattaactgccctgcttcagcttttctgcgttttctgcaaattgaagggcatctatcatatctttaatatcgccattcataaaggcgtccatattatatacggtcataccaatacggtgatccgttacacgtccctgcggatagttataggtacgtattttagcagaccggtcgccggtagatacaaggcttttacgctgagaggcaatggcatcttcatgcttacgcaccgccgcttcgtatatacgggtacgtaacatcttcatagcaatttcacggttagagtgctggctgcgtccttcctggcactccactaccacaccggtggggatatgcgttaacctcaccgccgattcagttttatttacgtgctgaccacccgcaccggaggaacggaaggtatccattttaatatctgcttcccttacatccacatccacctcttcagcttccggcaatacagctacagtagccgccgacgtatgtacgcggcccgaagcttccgtagccggtacgcgttgcacccggtgtacgcctgattcaaatttcagggtaccatatacatcatctccatttacttccattactatttccttataaccacctgcagatccggcattttcacttagcaaactggtggtccagcctttgagctcacaaaaacggagatacatgcggaacaggtctcccgcaaaaagacttgcctcgtcaccgccggtaccggcacggatttcaaggatggcattcttttcatcctggggatcttttggtatcagcaggttacggatctctgcttccagggctgttttctgctcctgcaattcttccgtttcggctttagccagttcgcgcatctcatcgtcgccactgtccagtacttctttgttaaacgcaatattgtccagcaatttacggtaggcatcatatgccttcacgatcttttccaactgccggtattccttgctgagctgaccaaacttcttgttatcactaacaaccgccgggttggtaagcgccatcgatacctgctcgaaacgaccttttatagcttccagtttgtctatcataattatatttgacttttgagtaccctttccaaccggaaatgatactgccaatcgggttgcaaaattaacaccattaacttaattaaacagcaggtaattgaaacagatcaaattaaagggaaaagatatatttaacggtacgcatctgctgggtcccgggaaagtattgacactcactgaagatggcgtagtgacgggcattgtagccgaatccgatgccggccccggcgtcagggaactggacggaattctttgtccgggattcataaatacccattgtcacctggaattatcccatatgaaaggggtgattccggaaaaaaccggtctgcctgccttcctcacccaggtgatgcaaaccaggaaccaggcccccggcgattatgacgccattatagacagggccgagcaggaaatgtgggaaagcggcatttcggctgtaggcgatatctgcaacagtgccgccaccctcgtaaagaaacaacagggcaggatgtactaccatactttcgtggaatgcatgggtgtagcacctgcgggcgccggtagccgttatcagtatagtatggaagtattggcatcattccgggcaatcaacggcccgtatcacagctgctccattgtgccgcacgccccctattcggttagcaatgcgctgttttcattactggccggcacaccggacaatgcgcccgtatgtatccacaaccaggaaacaccggctgaaaatgaattgtatcagcacaaaacaggggagttcctttctttttaccagcacttcggaatggatatcagcggattccaaccaaccggcaccaacagcctggaagcttatcttccctatttctcccggaataaaatcctgctggtgcacaacacctttacctctgaagccgatatccggtttacacaacagcaacccgtggaaacctggtggtgcttttgcccgcaggcgaacctgtacatcgaaaaccgcttaccggatatccaacaattccggcagcagcaatgcaacatcacccttggtaccgacagcctcgcatccaatcaccgcctgtctatttgggaagaaataaaaaccatccgcctacattttccggaaattccgttggaagaaatactccaatgggctacatttaacggcgcaaacgccctgggcatacaaaacacctatggcagttttaccactggcagtaaaccgggtgtaatattgattaaccaggaaaccagcagaatcatttagctataactatgaacgaatttttgaacaaagtaattttagacaaccccgtacaggattacctgattttgatcggtgttttactgtttgtgtttattatcaaacggtatatttcaaagggactggccaccatcctgttcaggctggtccggcactggtcgccgcaaattgaagaaaaagactttatcagcctgttgctacgtccgctggaatatttcttcctgctgatcaccttcatgctgacgatcgaccgctttacatttccgcaggttctcaatgttcatgtttataacaaggcaacgctgcacgatgttaccaataccttactgagcctggcgttgagtatgagtattatctggatcatgctgcggctgatcgatttcatcgcactggtactggaaaagaaagccgatctcacagaagataaaaccgataaccagttcattattttcttccgggattttttcaaggccattatatttatcatgggcgccattgccttcatccgtatcctttttggtcccggcctggtagagaagatcatcgccggtttgggaataggtgctgctgccctcgcattggcagcaaaagaaagtatagaaaacctgattggctcctttattatcttctttgataaaccattccgtgtaggcgataacgttaaagtggattcctggcagggcactgtagaaaaaattggcttgcgcagcacgcgtatccgcacactggaaaagacttttgtcaccgtccccaacaaaaaaatggtagacagtatcctggataacctttcgctgcgtacccagcaacgggtagccttaaagctggaactgggtacagacacaccagcagacaccctgctgttgtttttacaagacgtgcggcaaatgctgaacaacaatcccaacgtactggaaaacccggtggtaaacctgaatgatttcaccaaagatacctacgtgatccagatcattttcaacacgtacattattgatggcacccagtataatgctttgagggaaacagtgaaccttggtgtgataaaactgatggaggcccgtgagctcaagttgcctactacctccacaacggttaccctgagcgacctgcgggcggagtagtgcggattttgtcttggctcaggattacgctgattttactgattagctggatttttactgttggatttttttagatttcttgattttcttaaaataattaagggagataaaagcgaatatccgcttctatctcccttaatcttttataaaatccaaaagtaaaaatccagctaatcagtaaaatcagcgtaatcctgagccaagacaaaatccgctattccttttccttcttcgtgctgctcagcaggatgcgggaaatgtcggcttctatggattctttgggcgcacctacgatgcggccttcttctttaccgtctttgaatacgatgatagtaggtaatttctttactttataatctaccggagcatctgtctgcagtttcttatctgctgcaaacattacgatctgttcgtcggggctgccgccggtgatcattactttatacagggctggtactacttcgcggctggtattgtcccaggtgcccatcaccactaccatgttgaagttagcgcggttggttttaatatagttcagcatattatcgttaggctggtagctgtttacacctttgtagaaccacgttgcggaggtgtcattcatcagtgttttcatatctatcttgcccttcagtactgtttcgttctgtgcccatgccagggatgagaataacaggccaccacccagtagtaatgttttcaatcgcataatgttgtttttataattgatctttcagttccgttaagaaaccacgtacctttagcaaagcctgtaccatttcaaaattacgggcagccagcttatgatcttctttcagtttttgcttggctccttcaattgtatattttctttcccgcagtaaatggtagattaatttaaggtggtgaatatcttcctgccggaaaaggcggtcgcctttccggttctttttgggttgcagtatatcaaactcattttcccaataacgtatcagcgacgtattcaccttaaacatggctgcaacctcactgatagaataatactgtttctccaataccaatttatccaattccataatcagatccgggtcctccgataactctttcaatgatttacgcccccgttttttcccaggtatggtggttgctacggcagctttcttgctgctggcctttgcttttactttaactggtcttgttaccgcagcttctgtgggatgcggtactccagatgtcgaaaaaaggtctagctggtgcatcgtagtaaaaaacgaggtgacaaatatcttttacaagatgaagttaagcttttagcttgtagcttgtaacattcccacctcattttttgggtttagacaagttacggaaagcccgcaactggctaaaaactataactttagtcaaacgactggttccctgacctggccattttgagcatgcggtcaaactgttccggggtaagatcattaaagaagaaatacacggggtccaccttgtctccgtttttaatgacttcgtagtggcagtgcggtccggtagatttaccggtgctgcctacccagcctaatacatcaccgcgttttaccgcctggccggccttcactttcatacggagcatgtgtccgtacagggttttatagccatatccatgtcgtacaatcacgtggttgccgtatcccacatcgctcaggctggcctcttcaatcacaccgtcgccggtagcatagatgggagtgccgctgggtgctgcaaagtcgagccccgcgtggtatttcatggtcttataaataggatcgatccggtacccgaaaccggaggcaatatgtttaaggtctttattggaaaccggctggatggcagggatagaggccagcatctgctgtttgttcttcaccatcttatcaatttcattgtaagatgcttcctgcgcttttacgcggttattgagttctttcagaagtacagccgtggaggcgataatctcgctgctggcaaaggattgcagctgggcggcttcttcttcccgctttactttacccatacgggtgctatccggaataggagaggcttcaaatatcacccggtaaatttcattgtcacggtcttccagctccgccagttttccctttacttccctcatccggccctgcaacgcatcatatttttctttcataccttccaggtcgcggcgaagtgatttctcctttggggagtctaccagccggtatgccacggaaagaaaaatagccccggtcacgatagccgcagacacaaaccccagtattctcaggatttttacccgcagggaaaccacgagcttctcgtattttaatgtttgggtattataaaaatatttaaccttcttcatgcaccagggtgtactttatgcgccatagtgcagtgaacgctatgacagccgatttatttcacgaggcacaaacttatggatgggtaatcattggcatttcttttcccactaaactatttttgccgggtaacacaacctgttttgcataatcatacaggtttcgatatttttgcactccctttaacacggcgggaaaataaggcgcacaaacctactgtaattagattaaaacatcaaccttttgattgtcaattttctaactacttcataaggacttgaaatacagctacaagcccctaaccggttatggcttataagatataaaatacatattaattcgtatcaatatttatgacagcatctgaaataagacagcaattcctggacttttttgcgtcaaaagggcaccagattgtcccatctgcccccatcgttattaaaaacgaccctaccctgatgttcaccaacgcgggcatgaaccagttcaaggattacttcctgggtaacagggttcctcccaataaaagggtggtagatacgcaaaagtgcctgcgggtaagcggcaagcacaacgacctggaagaagtgggtattgatacttaccaccataccatgtttgaaatgctcggtaactggagctttggcgactactttaaaaaagaagccattgcctggagttgggagctgctcacagaagtatataaaatccctaaagacaaactctatgtgactgttttccagggagatgaaaaagaaaacctgccaaaagaccaggaagcctacgacttctggaaagaacatatcgcggaagaccgtatcctgttgggtaataaaaaagataatttctgggagatgggcgataccggtccatgcggcccctgctcggaaatccacgtagattgccgccctgcagcagagaaaaacctggtagacggtaaaaccctcgtaaatgccgaccatccacaggtgattgaaatatggaacaacgtattcatgcagttcaaccgcctgaaagataaatccctggagccactgcctgcccaacacgtagatacaggcatgggcctggaacgcctcgtcagagtattgcaggataaaacctccaactatgacaccgacctgttcatgggcaccatccacaccacggaaggacttaccggtaaaaaatacgctggcactgatgataagaaagatgtagccttccgcgtaatcgcagatcacatccgcgcaatttcctttaccatcgccgacggacagctgccatccaataccggcgcaggctacgtgatccgtcgtattctccgcagggcggtacgttactacttctctttcctcgatgtgaaaaaacccctgctgcacgacctggtacccgtactggcggcacagttttcacatgtgttccctgaactgcaacaacaggcggacttcgtgaagaaagtagtgtttgaagaagaaaacaacttcctgcgcaccctggaaagtggtatccgccggatcgaagactatatcaaaaacgccaccaccaaaacagtagatggtcaaacagctttcgaattatacgacacctacggcttcccttatgaccttaccagcctgattgcctccgaaaatggcttcactgttgacaaagagggcttcgatgccgccatgaaacaacagaaagaccgctcccgcgccgccacagaattggatatgggcgattgggtagtactcgacgaaacgcctaactccgttttcgtaggttacgaacaactgaaaagcaccaccaaactgctgaagtaccggaccgtgaaagcaaaaggtaaagagcagttccagctggtactgggccaaacacccttctacgctgaaagtggcggacaggtaggtgataccggtaccctgcacttcggcgatgaggtaattcatgtaaccgataccaaaaaagaaaacaacctcaccatacatttcgcggataagctgccggcacagccaactgcaaccgtaaaggccgccgtagctaaagataaacgccacaatacagagcgtcatcactcggctacccacttactgcacgctgcactgcggcaggttttgggtacacacgtggcacagaaaggttcgctggtaaatgcggatgccctgcgcttcgacttctcccacttcgccaaagtaaccgacgaggaactggcgcagatagaagccattgtgaacgaaaaaatccgtgaaaacattccagtggtgatccgtgaacttccaaaggaggaagccctgaaactgggtgcgatggccctctttggcgagaaatacggcgataccgtacgcgtggtaattattgaccccgcctatagtgtggaactttgcggcggtacacatatcagctcaaccggcgaattaggccagtttaaatttgtttccgaaggagctgtggccgccggcgtgcgccgcgtggaagcagtaactggtgctaaagcagaagccttcgttaacgagcagttacagcaactgaaagaaattaaagctgccctgaaaaatccgaaagaactggtgaaatccatagaaaccctgatccaggacaaatcttccctggaaaaacaactggaaacactggaacaggaaaaggtacgggcaatggcagccactatacgccaccaggcggaaaacatcaatggagttaacttcctcggacaagtggtgaatgtaagcaacgcggagggactgaaacagctttctttccaactgaaaaacgatatcccggatcatgtactgctgtttattgccaatattggcggaaaagccagcgtggcgctcagtatagatgagaaactggtggcatccaaaggatgggaagcgccaaagatcattaaagaacacattgctccgctgataaaaggcggcggcggtggccagaaaacctttgctacagcaggcggacaggaaacagacaaactggaccaggtgattgctgcggtaaaaaaactgctcacaacttaaaataatgctcacagcataaaaatgagggctggctaaaaagtcaaattgggcttttaagccagccctttctattccaggacgtgactaacaccgtaaaccttttccaggatttaacacttatattgtaaactttaaacagggttatctaactaaagtgtaaacctttttcaggacgtgaccattctatccagggcggcatagtgtatggggagtgtatgggaagtgtatgataagtgtatcatgagtgtatgggaagtgtatggggaatgtatggggaatgtatggggagtacgacacatacgctactcctaagtatccgagaagtatcccagaagtatcggagaagtatcccggaagtaagggcggcaccttcttcaaataataaaaaaacaccctgtaaagcgtattctttttgccccaaaaccatagattttaactttttctttcctgacccaccctttaattttgccgcattagtttaaatttaatcaacaaaatacctaattaccatgaccaggttactgcaaatcctcaccatagcaggtttttcctgcttcactatgagcgcggtatctgcgcaaacgaaagattcttccaaaaatcagttgggagagttcgatgaaattgtgatcaaacacaaaggcaacaaagacggcaaagtgaccgtggaaattaaaaacggcgatgttttcatcaatggtcaaaaactggaccggtacgacaattccgatctctccgttttccgcaggaagatcacgccgcgggatggcaacaccatcacgtttgacagcaacagtttacagggaggcggctttgatttgtttaacgacaacgacggtgatgacgaaaatgacatagaaatgccggtgatgaataaagccattctcggtgtgatcactgaaaaagtagccgccagcggtgtaaccgtaaaatcagtagcaaaaggtactcccgcagataaagcaggaataaaaaccggcgatatcattacttctgtagatgataaaaagatcaatgaacccgcagaattatttgaagagatcggcaaacataaaccggcagacaaagtaacggtaacgtacatacgtaataccaaaacaaacaaagtggctgttaccctggatgaaagaaaggaaatagataatggctggactatgcacccacctttatctgcactgccgaagaacggaccgagatctttctctttcccaatgccacgcggcttccagggatttggcgacagttgggataataacgaaaaacttggcctccgcgtacaggatactgaaaaaaatgaaggcgcccaggtaatcgaggtggcgccttcctccgcagctgcagcagcaggtttccaaaaagatgatatcgtattggaacttgccggtataccggttaaaaacgccgcggagctgtctaaagcttaccgtgaaacacaagccaaagtaaaaggcgatgctccagcgaaaatccgccggaatggcgccgatcaaacgctgatcattaagttaccggtgaaactgaataaggcagatatataagcctacttcatcaccatcttcatcatcttcaatttatttttaaacggcgggtacttcatgggaacatccagccaggtagccgttttcagcattcctttctgatgggtaaaagtatcaaagctgtatttgccatgatactttcccatcccgctgtaaccggcgccaccaaagggtaattcgggattggtgagatgtaccagcgcattatttacacaacctccgccaaaccgcacctgctctatcagcgctttctccgtttttttactctttgtaaaaacatataatgccagtggataaggcaactgcttgatggcttgtatggcctgcggcaggccggtataagtaagtatgggcagcacggggccgaatatctcgtcctgcattaccgggtctgtccattccacatcttccagcagggtaggggctatataaagctgttcgcggttggtttgcccgccgtgtaatacatggccgtcgcccaggtagcctgccaccgtatcaaaccgcctggcattgataatacgcgcataatcgttgctgcgggagggatcttctccaaaaaattccgttatcgccgccttgagtgcggctaccagttcatctttcactttgtggtgtacgaggaggtaatccggcgccacacaggtttgaccggcattccagaacttaccccacactattcgtttagccgccaccgttacattcaccttttcatctaccacgcagggcgatttaccgcctaattccagcgtaaccggtgtgagatgcggcaccgccatttccaggatcttcttgcccaccgggatgcttccggtaaaaaatacatggtcgaaccggaaactcatcagggtaggaatcactgctgttccatctccctctactactgtaatataagccggatcaaaagtatcttttatcagggcagcggttaccgcggccgtatgcggcgccagctccgatggcttaataatagcgcagttgccgccggcaatggctcccagcaaaggactgagcagcaacataaacggataattccaggggccaatgatcagcgtaagccctaacggctgcttatacacccggctgctgctgggataggtaacaaaaggagaggtaaccagctccggctccatccactgcttcaacccttgcaggatataactgatttcttcatataaaaatcctatctcactaccataagattccagtggatgcttgtgcagatcagcatgcagggcagcggtaattttatcttcaaactttttaatcccgttctttaaacgctttagctgcgttttccggaaagaataagaaagtgtggcgccggagtcgaaataaacctgttgcgcctgataaagctgacttgcctgggccttgctgatcatagggaagaaattttgatgtgtatctcaatttagggatttattggcacccaatagcctgaaatcacggtattatttgaatatatttgtgggaatcagtacggaaaatgagcgatatatacagcaaatatgaaacagtgatcgggctggaagtgcacgcccagctgcttaccgaaagtaaattattttgcagcgacagcgcagcttttggcggcgctccaaatacgcatatcagtcccattaccatggggcacccgggtactttgccccgtatgaaccgtaaagcggccgaatatgccatcaaactgggtcttgcctgccattgtgaaattgaaaaggacaattattttgcccgtaagaattatttctacccggatcttccaaaaggataccaggtatctcaacatacggcgcctatctgtaaaggcggttatattaccattattacagatgcaggcacccgcaatgtacagctgaaccgcatccacctggaagaagatgccggtaaactcctgcacgaccaggaccccgacaacagctacgtggatttaaaccgcgcgggcgttcccctcgtggaaatagtaactgaaccggacatgcataacagcgaggaagcctacgcttatctcactgaaatgcgccgcctggtgcgctacctcggcgtatgtgatggtaacatggaagaaggcagcatgcgctgcgatgccaacatttcagttcgcccgaaaggcaccaccaccctgggtacaaaggtggaagtaaaaaacatgaactctatccgcaacgtaaagcgggctattgataacgaggtaaaaagacagatagatctcatagaagccggcggtaccctggtgcaggaaacacgcagctttgacgcctccaacggcagctctttttccctgcgctccaaagaagaagccaacgattaccgctacttcccggaaccagacctggcgccattcaggctaacagatgaattcatcaacagcgtgcgggccacactacctgcattaccggaagaactcatccgtaaatacaccaccgattttggcctgccggaatatgatgcgcgtgttatctgcgatgataaatccacggcagattattatgaaagtcttatcgccgttacctcgcaatacaaagccgccgccaactggatgctgggccctgttaaatcctggctgaatgaacattcggcggaaataagtcatttcccggtaacaccacaggcactggcggcgttgattacgcttaccgatgcaggaaaagtcagcttctccatcgcgtcttcccgcatattgccggaaatgatccaaacacccgcggatcatccgatggatatcgctacccggctgaatttattacaggatcataatgccgataacatttctcccattattgatgaggtgctggcaaaatatccggataaagtagctgcttttaaaggtggcaaaaaaggattgatgtcgttgttcgtgggagaagtgatgaagctgtccaaaggcaaggctgatccccggcttaccaacgaattgctggcagagaagctcaaaggctaaatagcattgaaaatatttatcctatattgagtggcttaggtcagatgaatgttcaaaaaataatagcatgaaaaaatacttattatggatttccgccgccgctttcctcgcaggatgcgccggacaaacggaaaaaggtgaatttaaaatagacgggcacctgaacaatttaccattgggtccggtattactggaagaactgacacttgacaatgtgaaagtggtagattctaccaatgtaaaggacgccagcggcaaattcacgctgaaaggaatggtagccgaacaggggctgtaccgtgtacgcttcgaaaacggcaaatttatattgctcgcactcgatgccggcgatatgaaaatagatggagatatagataaactggaagatgtaaagatcagcggctccgaaccaaccgccgaactgcaacagtttatgagcgatatcagcaaacagtctattgcactcacggaagaaatgcgcagcctggacagtctccatacaatactgcctgatagtgcattccagtctaaagtagctgccttccagaaaaaagaaaaagattttgaaaacggctttttcctgatggccgataaaacaaaaaatcctgctaccgcagtatttgccatcagccaggtaagaagcggagaagagattgttgcacacaaacaggtgatcaccaatcttgctacccgtttccctaaaaacacgctggtaaaaagtatgacagataaaatcctggaactggaaaagaaccagggcgcgggcgccgcaggcggtgatgcagccggtggtgaagaaccttctgctgtgaaagtaggccaggtagcacccgacttctcccttccggatccatccggcaaaatgatcagcctcagctctttccgcggtaaatatgtactggtggatttctgggccagctggtgcggtccatgccgccaggaaaacccgaatgtggtaaaagcttatcagcaatacaaaggaaaaaactttaccattctcggcgtatcactggataaaacgaaagataaatggcaggaagccatcaaagcagatggactggcctggaaccatgtaagcgatctcaaattctgggattccgcggtggtacctttatacggtcttaacgctattcctactaattttctgctggatccacagggaaaagtaattgcctccaacctgagaggacctgcgctggaagcgaagctgcaggaagtactgaaataagctatctatctccataaaaaaaactcaccggcattacaccggtgagtttttttattattgcaggtcaaggaaaagtttagtattgcggattctgcgcatttttcaacgctggattagcagagatttcagtagctggcagcggccagataaaccggtaatcagcatacttaatgctgccgtaaccagacggtgttaccggtctggttaccgtgttataattgctgccatcatctttcagatcatcgatgatcacctttgcagggataccacctgttccatactttgcatccagtgcaaggcgggtaatgtcgggccagcggcgtccttcgcctgcaaattctaccctgcgttcgtccaataccgcctggatcatgtcgagcggagcaatggtgatgcggttcggactgccttccggtaaagaacggttgcgaactgcgttgtataacttaaacgactgtacgatatttcctgcacgtgcatatgcctctgccgcattcagcagtacttctgcataacggatcatcggcgcccagtcggacttattcagataatcacggtatttataattgaagtagaagttctgcacgggtttgccgcctgatacagtcacctgctttacctgtaataaaacacgacgcatatcatcgcctgcccagaaagaggcgttgtacaaattagggctggtagctaccaggccgcggcctttctggtcagaagggccaaacatcgctgccagcgcaccattggaattaccgttggtgatggcactgttggcaatagagaaaatagattctgtgttattatctgcttttgtgaacgggccatccgggctgtcggtaagtttataacctttcaccgggctcacaaatggcgcactttgatctgcacccagctttgcggcttctgtgataacaccctgccaatcggccatatggagcttaattcttgttttcaaagcaatagccgctcctttagtagctctgctgataggattagcagtggtgggaagcaggttggtttctgcaaaatccaggtccgccaatattttggtataatcctcttttactgtaccacggcctattttcagggcttcctggatttgagctggtgtgcttacaggcatatccctgtaaggaatcccaacttgtgcacctgcaccatctgcatatgggcggctgaaatgaatgactgcttcatgatgtgccagtgcacgcagaaaacgggcttcaccttccagctgcaacgccttaccctgtgaaatcacgttattggcagcggctttccgcacaccatcaataagtgtattggcctggttgatcagcgcataaagatttacccacatctggacattattggcagaagtagggctgtaactgcctttataagtgatatcataaaacgtagccaggttcaccatatcctctccacgcatctcattttgctcaatggaagcagcaccgaagggataaccacggcccagggtataatcatcattataacttcccagcgcagctgtattatacataccatttgcagccagctcgatagtggatgaatccgaaaataccgcgtcttgtggcaaggcgttctttggtgataattcggtgtattttgaacaggacgcagcacccagtgataacaccagtaatcctgctgctactgctttcatgcttctgttatatttatatgccattgtatttctcatgttcattattttttataatcctacgttaataccaaaagtatagctgcggggaaccgggttggtgttgtaatccaaaccaggttgcgtgttagctcttgcatccacataagtatttaactcaggatcaagaccggaatactttgtaatgataaatgcgttctgcacctgcgcataaatccggatgctgctcagtttaattctttccagcattgctttaggcagggtataacccaggccgatgttctgtgcacggataaagctgccatcttccaggaaacggctgttaacattaccattctgcaggataaagttatctgcgcccaggtacagtttaggaacatctgttacctggccaggagtagtccatctgtttaaaacttctttaccgttgttcaggaacttctggttgttcaggccttcctggcgcgttacgctgtatactttattaccgccggagaaagaaaggaacaggttaaaatcgaaccctttgtaattaacggtattgttcaaaccaccataataggttggcgtagcattaccgaggatttttttgtcggaagatgataatgcttttgcagaagtagagatgtcctcaggctttgaagcattataggcatagtaaacacctttcgatgcatcgccctgtataatggagccgtcggcttttttccaaagcgggttaccatttgcaggattcacacccattgactcgtaaccataaaaagcacccatagattcacctacgcgggtaatgttatatggataaacgatatctgcattatctaccagtgcggtaattttattttttacaaaagagatgttgaaggaagtggtccaggagaaatcaccgcgctgaatattagtactgttcactgttagctcataacctttgttatacattttacccacgttagaataaaatacattcggtttggtagcacttggaacacctaatgacggcggcagcggagatgccaggatcatgttatcaatatcattcctgaaataatccgctgttactgtgatcctgtcgtggagtaacccgaggtccaggccaatgttcatttttttactggtttcaaaagtcaggtccgggttgtacacctggttgaaagcaatacccagtaaagatccgtatagtgctggtttgtaagtaccggcataagggtatgcaccgatatccacgttacctactttagcataaccgccacggatcttcaggttgctgatcaggtcggcgataccgccttcctggaagaaactttcctgtgaagctctccagcccacagaaacgcctggcaatgttacatcctgtttgccgataggcagggaggaaatagcatctctgcggagcgtggcagataccaggtagcggtctttgtagctgtagttagcccggataaagtacgattggaatgcgcgctccaccagtgttccgccaacagtttgagtaccggtgctattgtcgatgaggttatcagtaccaaagaaagggctgatcaggttagtaccctgcgcatagaaacttctttctcttgttttctgattttcggttccaattacagcgccaatattatgcgcaccgatcgttttgttatagcttaaagtatttacccagttataacggaaacttggaatagactgctggtagataaaaccgttggtaccacggccatcaccatggatagggttccagtactggtagtcctctccactcatatagtttacacctacctgcgttctcagatcaaaatctttcagaatttttacgctggcaaaagtattaccggtaaagttcaggtttttgttacggtagatgttatgatccagtacgtatttaatgttggtatagttatcagcgatagtggctttattggcgccactgccgagcgtattggtgttgctcaggttataggtgccatcattccactgtgcaggtacgttaggtaaagcacggatagcgttggaaagattgctggaaagcccgttctggctaacgttcaggccattgttggtaatgtgcgaaacaccggcatttacgcctacagttaccacattaaaagctttctgttccagtttcaggcgtacctggtacttgcgctgatcgttaccaaccaaaatacctttcatatcggtgtaccccagggaaacgtagtagttggtttgatcattggcgccgcttagcgacaaagcatggttctgttggaaccctgttctggtcactactttctgccaatcggtatcataaaaaccaccatcaggattgggtgtagggaaagcatccggtgcagctgctggcttggcgttcagctttttctcgttagcgatggttacaaattcatctgcattcagcagatcaaataatttggaaggcgtagctgcagccatccacatatcgtaggtgaggcgtggcctgccgcttttacctcttttggtggtcacaaggataacgccgttagcggccctggaaccatagatagcagtagcggcgccatctttcagcacttccatgctttcaatatcattcggattgatatctcccaacgggttgttggaggtgatcgtgctctggttgccggtgatataaggcactccgtcaattacatacagcggatcggtgccgctgctaatactgttggtaccacggatgcggatacgtgccggctggcccagaataccactggaaacggtagcctgtacgcctgctacctgtccggataactgacgatcgatgctggatgcagccacatttttcaatgtagctcctttgatgctggatacagaagccgtgaggtttttacgctcaatagtaccgtaaccaactactaccacttcgttcagtcctttaagatcggccgacaactgagcgttcacagtagatttgccggaaacacttacctgttgggcagtatatcctacaaaagaaaattcaatggcggcagctttttctcctacactgagcttaaactcaccattggaggcggtcatagtgccactggaagtaccaacaatttttacggtaacgccaggcaatggagatccatctttggagtctgtcaccttacctgtgatgaccctggtttggccaagcgcctgcagcgcggtaatagccgcaaataaccagagaaacaatcctttcttcataagcgattttgatttgaaaaaataaatgtaatacagacatgtccaggcatagcatggccatttagcacaagtgctattattatctaacagtaaagactaaacgaaacaatcgtattgcttttgcggcaaccttcgcaaagcacaattctacataagcattccaaaactcataagcaatcctaacattataaaaacaagtgaataagcgtacagtagtggcatgccactgaataaccagataattttatacagattgctgtaaacgggttgccaggtattttctgcggttacagaaaatacggttccgttactgcgtaaactgcagggtggcaactattgaatctcattaaattagatggaaaatctggctgtaagccgctccccataagcaaatattcccgttataaattcccgataagcaaaaaatgtattcgttgtttgttgtattggattacgctaaaatgaatcttgattcccgattttggcttcatgaaaattttcatgacgggagcaaatataagtaaacctttcaagtaaaaaataacattttagggggagtagaaaatgggcataaaaaaagcggttgtctcgaaaagagacaaccgctttctattattagttaaatgaagtactgattattgtttggtatcccaccaaacgcgatcagtaactttggcaggctgttctggttgcgcgtttgtttcattctctgatgctggatacacccatctgcgtggaacagttgtaataccctgataagcattctgtacaacagtcagcttagggaaattggttctgcgccagtcgttgtatgattcaagagacaggtagttagagatatatttctgtgtcatgatcacctcgtaagcattagcagcagtgagcttgcatttagctgccaaataggtcttaaacgctgtactatctgcgccaagtggtttcattccaaatcttgtgaaggttgcttgaactgcactgttcagaattggttgtgcagctacaaaaccagctgtcaggaaggtagcttctgccttaataaacagttgttcatcatatgtagccaaataaaccgattgatcagcagcagcaaaaaatttacctacagctgaaagtgaatcaatattaatctgctcgtcgcctattatcctgcctctataaccgcctcccaacaaagctgtgtctaccattacggataatctgggatcatttgttgatttcaataattgaatgaaagtagaggatactgcaacactaccccatttattattatcagtaaactgggaccaaggcgcctgcgctcctgatttgctttcgaatttcacgcccggattataactttcatcagggaaagcttttgtcaatgcagttaaagctgcctgtgcctgtgtggcagccactttaccaggtgcatatgttaaacgtaaagcaaaacgtgctttcaggaaataagcgaatgctgtccatttttcgggatcagaagcatatatcagatctttatcgccaactgatgcggaagcatcttctttagccagtagagcgatagcatcatccaacagcgtattaatactggtataaatgctttcctgtgaatcatacttcggcttaaagttttcaaagccggtaaatgcttgtgaataaggaattgcattccacaagtcagtagtaacagccaggttataagccattaatatttttcccataccagcggcatgtggatgatttgcggtagtagcctggtcctgcaggatcttcaggttattcaggatctggggatacatgtcaaaagaccaggtattatccacatcggaagctgttaccttataagtatcccactcgggtgcgggttgatcataacccaattgttgggtccagaaagcggcggttctggcaggataaccacccgcaatattaaatgcagtagttaattcggcgccgcccaccaacagggcatcagttacgtttgtggctgcagccgggtcatcgtttacatccaggaattttttacatcctgaaccccctaacattacacttcccgctataatggatataattatcttcttgttcatcattactcagtttagaaagttaacttcaaagttgcattgtaagatctggtgcttggtgaaacgtaatggtaaaaaccaccggagttactacctgctccataagtgctcaattcaggatctgaaccggtaaagtgtggggtgtagatccacaggttacgaccggcaacagaaaatactgctgctttaaatggagtacgttttaacaacttcggactaaaattataggccagtgtaacatttctcagttttacaaaggttgcatcctggatcaggttttcataagtatcaccccatgcctgccagtaagcctgatcagttttaatggatttggtattttgcttaccatcggcagttacaccgtcatataccattgatccgtcgcggctgctggtaagaccactggtaccgtagaaggtcatgtagtattcatcaaagttgatcacctgaccaccaaaacggccgtcgaaagtaaacgacaggttgatacctttataagatacactgttggttacaccaccaatccatcttggctgggtattaccaatatcaaaggaagttccatcttcctgggtaggataaccatcatcatcgatcaacagtttaccctggtcgtttctcatgtaacgtgaacctctgatagtaccataaggctgaccggccaccaggtatataccgggagtagtgaaaccacctatctggatagaagttacaccttctgtcaactcattgatcattgctttgttcctggagtagttagcagaaatattccagttgaaatcttttgatctgatcgggttggcatttaaagttacttccagacctttattggtgatcttaccggcattgattacagcctgggtataaccggaaccagcagatactgctgtctggaatatcaggtcggtactaaccttgttatagtaacttgcttccagaccaatacggttgtccaaccattttgtttccagacccacttcaaattccttaattttctctggtttcaggtcaggattacccaacacgttattcttggagaaaccatttacaccgttgaaaggaagatccagtgagccacgaagaccatcacccactaccgttttattgaaaggcgttgctaccttgtaaggaggtgcgtcattaccaatggcggtgtaagcaactctcactttaccaaatgataatactttgctgtcttttaatccttccagttcggagaatacaaatgcaccagtcacagaagggtagaagtaggaattattcttagccggcatggaagatgaccagtcatttctaccggttaatgttaaagataacatgcggttatattccaggattgcctgtccgtaaacactcacccttcttctatcgtagaaagatttggtggaggttacagactccgcactggtaatatcatagaaaccaggtacggataatcctacaccttttgaaaactggtcggtataatgttcagaaatgatattattacctaccattacagtcagatcgaatttatcaaattctttcctggcagtagcgtagaaatcgtggttaatttgcttgttgttaatgatttcattgtacatacgaccattggggaaaccaccgaaggagccgattgcttcatgaaatacacgttcatctgtataaatatccgcacctattctttcggttaatgttaaccaattcagtggattgtataccaggctgaagttaggaatgaagcgggatacattcagttgcaggccggtattagccgcggtccagaaagggttattagcactaaccttatacatattctgtgacttatctaccgggttttcatatggtaacaggttgtaacttaccggcgcattgtaaaggttagccaggtaagaagtaccaccactaccattaccttccagcaagcggtcgttacgtgagtcaatataactgataccagtagtcgcagttaacttatcagtaagatgggtagagaaatttgcgtaaaaggagttacggtaatagtcggtaccgggagccacaccttcctgtcttaaagaagagtaggacatcaggtaatttgacttttctgtagatccgttcaggctgatgttattatcccaggtagtacctgttttaaagaacgcgtcacgtggatcatagttaacagctggcttgccatccacctttaaggtatccattttggcaccccaggaacgggaagttttattgtttattccatcaaagaatacgccgttgttaccctgtgaccaacctgtctgaaattcaggcaataccactttgtcaatgttcacactggaacctactgtcaggctgaaagctttaccttttaaaccagcgccggttttcgtagtaatgattaccgcaccaccagctgccctggaaccatacaatgcggttgcagaagcgccacggagaatatttactgattcaatgatgttcggatcaatatcaatacctctgttgggagtagtaccccctgccagaaccggatcatcgtcagtgtcacctgcaccaatctggttgttatcaatcgggttaccgtccactacaaaaagtggctggttatttccggttaaagaggccgcaccacggataacgatacgggtaccaccaccgggaataccagaagtattactgatttgcacaccagcaattttaccctgcataccattcaggaagtttacttccttggattgcacgatatcatcaccttttacttcctgcgtagtataacccagggtgcgtttttcacgtttaatacccagcgcggtaactactacctcgctaagatctttattgtcggcgccaagagccacattgatagtgccttcggctccaacaggaatttccttggaagcatacccaataaaagaaaaaacaagcacggaacccgcaggagcttcgagtttgtaagtgccatcgttggtggttagggaacctttacctgtacctttaattccgacagatacaccagggagtccggagccgtctttagcatccgtaaccttgccgctgattaattttgtttgtgcataggcttgcacaacactgatggccacgagcaaccataagagtagtcctcttttcataagcaatttagatttgaaagatattgtcagttaactaataaaaatgggagtgctgtactcatttagccaaaggttattccgtaaatcgttttcctcataacccatccttccttattcgtattttctcaaagcaaattccagtttctctcctctgttctcttcctaactatatcagaaactgtttccggtatagattgaaatggcggttaaatcaacacaagcaccaacttaattaagattttgttctttagattctgttttagattctgatacgtatttgttaaatattgtttaaattctactgcaatataggaaatttaaaaaatactagtgcaaaactggcttttttttaaaatatccgttcccgatatatccaacacctgctggcctctgaggatcactattcaactaatagtatattaattataatatataattaattatcttatataccttttcatttaaaaagatgcctcacctagtactccttaaataaataatgggtatccggtccgcttcttcttatccagtagtctccggtgaaataaaaaaggtgccttcgctgaaggcacctttcaaatcatataataatactaattggaataaccctggttctgcaccatatttggatttgcatccatctcggcctgcggaatcgggaaagctacacgaaaatcatttgcttctgtaacccttgtactcagcgcattagcatctttgatattacgctgcccgttcttacggaacagatcagacataccaaaaccttcacccaccagttccaatcttctctgtttaataatctcagctttgatattggccacatcagtaaatggatccagtccacgtttcgctctcagcatattcacatcatccgtggctttctgcaggttgcccagctcagcataagcttctgcacgattcagcaacacctcacttattctcaggatctttacgtttacaagacccacctggccggtagcttcattacctgaaaatttcatcaggtagttactgccatcaagattctccaccagtgcattacgcgcatcttttggatccaacagttccataaagccatctgtgagcctgatatctccatacccacctaatttagcaggcacatacatataaccgaagttattggagccaccgccatccggtgtcagaaaacgcagggaaaagatttcttcagaaccggctgcatctaaattaaatgctttcgccacttcagacgcttcatataaaggatacttcccgatcagcttatctgcctcgtcaatagccagctgccagtcgcccttatacaggtaagcacggctaagcaaggctgttgctgcatccttcgtagcattaaacacattcgcgctgttgctctcagatttaccggcaggagcggtttgctgcgccactttcagatcgctgataatagccgcgtaagtttcagccagcgtactacgaccaggcttgaatgtaccgggtgcatccaccgctttggtcaccagggtaatcccggtgttaggctcatttacttttgctcctatattggtatatggtcttgtgtaccttctggccaggtcgaaattagccagtgcacgcagaaaataagcttctccgcggatcgcaccggttttttccgtttcaggcagtttatcaatcagcacattcgcctggtttaccaccctgtaagcattcaggaaggtatttgtttgtggcgccagcagcggtgtgtagttcaattggaattctgtaataaaccggttggagttctgggaagtaatcttcatatcattgccacccaggtctgttacgatcatgaagtcgcggccataatattccagcgcctgcatacgctcatacattccgtttgcaagaatacgtgcattcccttcagttacggcatcaccttcattcaatgatgactgtggattctgatccagcttggaacaagctgaaaacaaaccagccgtagccaatgctaatatggagagttttgaatatttcataattaaactaaatttttgttgttacttcattacagtcccacactaataccaaacgtgatcactcttgaagtaggataacggtaaaaatcggttcctgcattggtagtagccggagacgcagtgctggtcggagaaatagggttggtactcatatccggatcccatcctttatatcctgtcagcgtaaataagttctctgcctgtgcatatactcttaatccctgcattttcaatctgcttaaagtgttttttgggagattgtaacccagtgaaaggtttctcaaacgtacataggagatatcttccaggtaacgggtagaagaagcattagagttggtaccattgccccagataacttttggtctgtcagcaatatcgcctggcttttcccagtggctgccggcatcttttgcctgatttccggtagtgttgttaccatcgctttccaggaaagaacggttatagttgtacgctttatttccagcgctgaatgtgatgaatacagacaggtcgaaatccttgtaagagaatttattggtaaaaccgcctgtaattttaggcagcgcctggccaacatattttctcactgctgaattataatcggaagttggttttccatcagcgccttcccaggtggcagcaccggtagcaggatcaacgcccgcccaaaccggcatgtaccaggagccaaatggcatacctacttcaatccgctggcgggaacctgccgggataaattgctggccgcccagtgacagtaccctgtttttcagcgtagcaaaattcagatctgaagtccactggaagtttttagtagacaccgggataccacccactgttacttcaaagccctggttcagcatcttacccacgttcatcgtcattacatcaaaaccgctggtcatagataatggcagctgcatcagtaatgcggaagagcgcttgtcgtaatatcctacgctaccgtataaacgttttttcagtacactgatatccaatcccacatcatacaggttttgtttttcccagctcaatgccatgttgcctggttgcttcagataagcaactgatccgccatcataagcgcccacgaggctgtacagcggctgataaggataatcgcccaaaccttctgcgttacccatgatgccatagctggaacgcagtttcaggtcgttcagccaggatatatttttagtaaattcctcttctgtaatacgccatgcagcacctactgagtagaagttaccataacggttgtctttagggaaacgggaagaaccgtctcttctgaaactaccgcttaagaaatactttgatttatagtcataatctgctttcgcgagtataccctggaaagcgtaggaggtttcatcaccggccatgtcgaaatattgggaaccagcgtccggcacctgtgcctggccattagggaaaccattctttgcactatagttccacacacggttctggaaggagtattcattacctgccagtaagcggatactatgatctttacccaggttgaaattataagtcagcaattgctgggtagtatataacgccatgttggtattcacgttatacaggtaaccgccatagttacgtccatcgtaggaatccggagatgtccattgcttttcacggatgttggtcaactcggcattacccttcactacgaaacgtaacccgtcaataatgttgtagcccaatgcagcattaaaaactgtttgggtattattgctcctgttgtagttactgttcaccgtgctcacgaagttgcctccacgtaaaaccgggcggtaggaggaggggatatctgcgaaaccagcccaggaagtagtgcctggctgtccggcagtatatccgttataggggtttccgttctcatcacgggaagggataaacggagaatttgccagcgcacccatcaatggtgaagagtaactgttacctgcgcttgcacttctttgatctgtatagctgccgttcacctttacgctcaggtcaaatttctcattgaacttatgatccacgttcaaacggccactgtagcggctgaagtcggagccaatcaggataccctgctgcttgaaataatcgccggaagcatagaactgtgtcttttcatttccgccgcctgcgttgataccataagattgtgttttaccggtgcggaaggcctcgtctatccagttggtattgatatttgtcaggctgttcggacgattagccaggatctgttctgcagtgaaaagcggcgtgccatctttcttggtcgcattcttcatcgcctcgcgctgataagccagcagctcagtggaattcatcatgtcaattccgtgcgacaggtcctggaaaccatacttggcattgaaattaatcctgctctggcctttcttccccgttttggtggtaataactaccacaccgttagaaccgcgggaaccatacaatgaagttgcagacgcatctttcaggatggtcacgttttcaatgtcggcagggttcaggttcgcaattacatcctgggaaggagtattctgggtaaaatccccggaggaaatgattaccccatccactacatacagtgggctgttgctcgctgaaatagagccgataccacggatacgtacctccgttttcgcgccaggctgaccggagttagttgatacggcaacgccaggcgcattaccctggagcatctggtttacatccggcaacgcaacgttgttgatctttgcaccattgatactggatgccgcgatggtggagttgatcttcttctccatcgtgtaacccgttaccactacttcatccagacttttggaatctgttttcagttttacgttcaatgtggcagcagtacccaccggtacttctttggcctcatacccgataaatgatacgatcaatgtggcatttgcatctacctggatagtgtaagccccttccggattggtgacggttccttttgcggtgcccttaatctggatgttggcacccggaatagctgagccatctgtggcatcagtgactctccctgttactgtgcggctttgcgcatagacttgcccgcccagaaatagcacggacaagaggagaaataatactttcctcataagcatgattttgtttccttaaccttaaaaaataatcatcattatcaaggccatacgccttaattcaattggttcccgttaaataagcagtttggtgaaattgtaattggatacttaaagctggagcaggtataacggtacagtgatattgaccaaattaaacaattgagcagttctcttgcgatttattcaatgaataaacagcagaagcagtcaacttcttcctcataagcagtttccttagcaaattttcaaccagcctcaaatataataattcttaacaaaaagttaagcttggaaagttcccgataacgtttggataacatctttttaacgcctcattaacatataattattacaaattatctgtaagggcataaaaataaacaagcggcaagaataccgcctgtgctcatcaaccaaaatctaaatcgagattaaagttgccccgcataaatgcggggcgaatattttttatcaggaaagggtaagcggatatgtttttaacaactccagcaataccgtaaagagatcatcattacgatgattaaagcggtattcacactctttcagatgtaaataggcagtattccggttcagccccttgaacttagccaggcggtgcttggttagtccccagaaagcatctacatcatccatctgatgcgtatcagaagtctgacccagcctgtataaacggtactgacccaaatccaccaacccgttgaaccggcgcaaacgttctgtagccacctgcgtttccaatacggaacgaccgcgggtagccgcatgaatcatagaccggcttacgtctggaagaatttcggtgtgtaacctgtctgaggatctgcagatgccgaagattacgggcttaacaatccggtctacttccggttttaccgccaccagcgtgtcgctgtcgtggtcggaattaaggtcactttgccggggttcatacgttaacacgggaacaggcacaggatgctgcgtttcacagtatcgcgcaatctggtgtcgtagcttcttcaggtagctgttaatagttaccctgcttacaccgctgatattcgctatctgggtcgcagtaagatcatcggcaaacagccgcaggatctccttaaatttgcgctcggataaatgagcgccctttaagtacttatttttcatgaactatgtggttagaatggcgtactaaacctcatactttttcattataatcccacccctttttttacaagcggctataagtgtatgtgaatgctgtccactagatcatttcagcttctttttttgtccattttagctaaatatttagcatccactgcagtttgccggcactaaaaagccaccggggcaaccagcagcatgaaaaacatgccctgcttaccccggtggctcatatgattgtctttataaactattcctgatcgctgatccccagctcctttatgtcaatgtcctcctcctcgtccaacggcttccacagctctttcttcttcgctttcttcaacaatgccttttccatccacaacagtaaagccggcaaaatagtcagattcgtaaccattgccaccaccagggtcagggaagtaagccatcccaatgcctttgtaccaccaaatcccgagaaactgaaaatcataaagccggcaaacaggatagcagaggtataaataatactcagcccggtttcatggatcgtttgcttcaccgtagcactgatgtcaaaatcatgacgcggcaactcctgcttaaaattaaccaggaatcggatggtaacgtcgatggctataccaagcgctacactaaacaccaataccgtagatggtttcaacggaacgcctacccatcccatcacaccggccgtaaccaccagtggaatcacgttcgggatcaatgatatgatcagcatcctccaggaacggaacaggtacagcatacaaagcattatcaacacaaaagccaggataatactctccatcagcccgttaataatgaaacgggtaccttcctggaaaatcacactggtgccggtaaaagttactttgtaatgcgccgtatcaaaaatagcagttacctgcggctgcaatgaatccagcaacaacggcagcttctgcgatcctacatctttcatatttacactcaacctggccacctgcctggtgctgtccataaaggaagaaaccagtttggagaaagtagaagcgggtccggcagtattcccacccttcatgcgcaggtaaggcgccaggaagcctagatcaaactggttgggtaccgcaaagttggagctgtccccgttataatatgcctgcttggcaaatttaataccctctactaccgacaatggacggccaaaatcaggctgcgcagcaatcaactgtgtcagttcatccaacttattcagcgtctgcagatttattacaccattcttctttttcgtatccaccgcaatttccagtggcattacccctttgaaattcgtttccaggaatttcagatccgtatacaatttgtcggtatgcggaatatcgtccagcatatagcccacagactgcaaacgccccattcccactatggccgctatcaccagcaccaaacttactccgtatacccatgggcggtatttaaacaccagcgtggtcaggaaatcaagtattgccccaaagaaccggttatccaggtaagtagtatgcttgctcttaggcgcaggtaaataacttaaaacagagggcaggaaaataaaagagatcaggaagatgaacatgatattcaaccctgctactacaccaaactctttcaggatggcactgtttgtgaaacagaacaccccaaaaccaatagcagctgtaagattggtaaacagggtcactatccccatccgctgtatcatatgcaccaaagcccgtgttttattggcatccttggcgtattctgtatggtatttactcaggaagtatacacagttgggaatccctatcactactattaacgaaggtataagcccggtaagtaatgtaattttatatcccatcagtacgatggtagccactgaccagattacaccgatagccactacaatcatggacatcagtaccgcgccaaatgaacggaaaaacaggaacaggatcaaagcagttaacacgaaagagattttcaggaacagcttcagctcatccgctaccttaacggccatggctgtacgaataagcggcaggccactcaggcgtacttctgtatgctgcttttcctggaaggcattggccagcttcgtaatttcattcactacagccgtacgtttcggggaattaaatacatccttgttcacataaatagccatgaggtaagcatgggtatcggggttgtatagcagtcctttgtaaaaaaggagggtgtggaaaacacgggataaactatcgattaccacctggttggtcagatccccctggaaaagtaaattagcctccagcttctgtgtgctgtcgttcttcaccaggttgatagccatcggcacactcataatattctccactgcaaaaacattcttcatgtccttgttcagctgaacatagtccttgaaaaaatctgcctggaaaaatttatctgtttgcacggcaagcatcaacacattaccatctccgccaaatctcttcttaaaatcctggtactcaagaaatttaggattatcatggggtatggtggccacgtagtcgtatgacatttgtaccttgctggcaaaataacccatcacgccggtaccggcaagcagtagaacaagaagcaataatcgatattttagcacaaagcctgctaaacgttgccacataaggatttcctttttagtaatgggcgtaaaggtaattaaaatagctattagctgttaacaggcagcgatgagctgactccttttagctgccagctgttaggttttagcttttagccgttcaatcccttcgtttgtgtaacttgcattccggtttctttcacttaactgctaacagcaaaagccaggaaaaattgcttcacaaaacacgcggcatcgtattacgcacggtaaagtatggcgacaccagcctgatcgtgagtatatttactgaactcttcggggtacaatcgtatatggtaaacggcgcccgttcctccaaacccaaagctgccaaaggaaatctgctgcagccgggtaatatcctggaactggtggtatatcacaacgaaatcaaaaaccttcaacgcatttccgaatacaaactgggatatctgtacaactccgtacacctcaatgtggtaaaaaatacggtagccctttacatgatagagctcctccagaaatgcctgaagcaaccggagcaacaaaccgatctctatttctttacagaaaatatcctgcaactgctggacatctccggcctgccggtggtggcaaacctgcctttgtactttacgctgaaaatgggagagcacctgggtttccggctcaatggaagattttctgaatacaccccttacctggatttacaggaaggtaccttttccgatctgccaccacatcacgccaatcaccttgatacacagagcagcgaattaacagaccagctgtttcaatgcacggcagtagagcacctggcggcgattacaatgaataaagaaagaagaagaaaattactgtatgcgtacctggagtttttccggctgcacttacctgattttacagagatgcattccccgcctattttacacgagatcctggatgcctgatctgttggcccagcctggcggccttcgctccctcttcggtgaagaatttcagatccaccgtattcccatcaaaaacagcgtaggaaaaataattcagccagtcccccaggttgatatacctgctggcgccgggtaatggaatatcgaggggcagatgccggtgtccgtagatgaaataatcgaaatgttctttttgcagtatttctttactgtaaatggccagccactcattttccgttccaaggaaatgctccagctcctgcccggtagcagagcggcttttgcggctgaaataattggcaagggcaatgccccaggccgggtggatagcagaaaacatccaccggcaaaacgggttcctgaatacttttttcagcatcttataaccatgatcacccgggcctaagccatcaccatgaccgatataaaaccgtttattgccaatggtataggtttgcggctcataataaaccgggatgttcagctcttcctcaaaatacccgtccatccacatatcatggttaccaataaaaatagaaataccgattcctttgtcgcttagcgcggccagctttcccaaaatgcgggtatatcctttggggatcacatgcttgtattcaaaccagaaatcaaaaatatcacctaccaggaaaatatgctgcgcatcaggttccacctgctccagccattgcaaaagcagcttttcacgctccctgctggcggcaggattgggagcgccaagatgaaaatctgaggcaaaatatattttcttattggccggtaatgcaatatccattcttaaaattatgaagcttttagcttttaacggttagccttcagtggaagaagcgatacatcgctccggtactgaaagttaacagctaaagactaaaagccatttatttattcgtctactaaaaatacgtatacttctttgggaccatggatccctactaccagtgttttctcgatatcagcggtacgactgggccctgttgcaaaagatatggctgatgggatatcgttaccgtatttatctttcagcttattaagcgcatccttcaggtcaaataccaactggtgcgtgtaggctaccacgatatgcacaggcgcatataccggtaatgctctgccactgggttgtgcggaactcagcaccaatgttccggtgcgggctaccaggtattcacaatccgtgatggcggcatctgcttcgtgcatggtcccctggttgagtacaggtaaatcctgctggtggattgttttcagcagggcaggtgtctggcaaaacacattgtgccattctttgtgttcacaaagcgcacgaaggctttccatcaactcaccttttcctgtacagtaaacaaactttccctgcaaccgggtaaattcttctgcaaactttaattccaggctctcattctcggttctgaaaacagacgagttgccctccgaattcgggaagggcaactgtactgactgacttaacgcattccgtactctcttcagaatattttccttagcaggagaaatcttcatatcactatttacgcattagcaggtgatggagaaggattgatgatatctgacggatgtactccttcagtaggagcgccttctttacccagctggtgttctttgtgggtatcgtaaggacgtttaccgatcaatctttccaggtcggcctggtataaaacttcttttttcagcagttcttctgccagtgcctttacctgatccattttggatgtgagcaggtctttggttctaatataagcggtggcaatcagtttccttacttcatcatcaatcatcttggatgtttcttctgagtaaggtttggtaaatgactgatcactgtttggatcgtagaaagatacattaccaactttatcgttcataccatacacggttaccattgcatacgccatacgggtaattacctgcaggtcgttttgtgcgccggtagaaattttaccgaaaaccagttcctctaccgcacggccaccaagggtcatgcagatatcatcgagcaactgttcggtgttgtacagatattgttccttcggaagatattgtgcataaccaagcgcagctacaccacggggaacgatggttactttcaccagcgggttagcatgttccaggtgccagccacaaatagcgtgacctgcttcatggtaagcaattacttctttttcttccggagagatgattttgtttttcttttccagaccaccaattacacgatcaatcgcgtcattgaagtcgtccatttccacctgtgttttccctttacgcgcagcaatcagtgccgcctcgttacaaacgttggcgatatccgcaccggcgaagcctggcgtcatggaagccagttttttcacgtccaggttgggagaagttttgataggctttaagtgcacttcaaaaatagtttctcttccggccagatccggcttatcgatagagatctgacgatcgaaacggcccgggcgcagtaaagcgctgtccagtacatcagggcggttggtagcagccaggataatgataccactgtctgttccgaaaccatccatttctaccagtaactggttcagggtgttttcacgttcgtcgttactcatcattacgttcttgcctctggcacggccgatagcatcaatttcatcgataaagatgatacatggcgctttttcacgggcttgcttaaacaggtcacgtacacggctggcacctactcccacaaacaattccacaaagtcggaaccggacatggagaagaaaggcacctgagcctcgcctgccattgcctttgccaggagggttttaccggtacccggagggcctaccagcagggcgcctttggggattttacctcccagggcggtatattttttaggattcttcaggaaatccacaatttccattacttccaccttcgcttcgtccaaaccggctacatcgttgaacgtaatattcacacgggtacctttgtcgaacagcgtagctttagatttaccaatattgaagatgccgcccggaccaccactgccaccggcaggaccgcccatcttacgcatcagcaatatccacaaaccaatgatcaggataattggtaacagcaactggaaaataggctcaaaccagctctgacgctcatcataagagatctttacctggttttccaccggaacaccttcctgtgctttatctatatcctttttgaaactttcttcgctaccaattgaaaaacggaagtgaggaccggggttctctccgccaaatttacttttgttaacgtctttaaacttggcctctttaagatggtcatgttttatgtagacttctacatattttttatttacgacaaccagcttatcaacatctcccggtttcaggtaatccacctgaaattcctggaaactgatttctttggttggggatctcaaatcaaaaaagttcattgcgagcagggccacgccaataaaggcatatacccagtatatattgaacttcggtcctttcttaggtgatttctccgaacccttgttgaagttattgcctcctttttccataatcttacgctcctttacggatgtttattgcaatcagaataatatgaataattaaattctaaaacaactgttttgtttagctttctgtgtggtccatcctgtccgcgtcgctccacatttcttccagattatagaacttcctgttttcaggctggaaaatgtgaactactacattcacataatcaaccagaacccagttttgagaactaaatccttcgtgtttgtacggttcctctgaagtatgcttctccacttcctctgacacataatcagcaatggctttcacctgggtgccggaattggcttcacatattataaagaaatcggccacggcttcaggaatctggcgtagatccagggacacaatattttcccccttcttatcctgtatggcctttatgatggtggtaaaaatttcactttctctggtcaggcgttgctgcgccttctttctcgtgctcagaacggttaagggtgccaataaatctcgtttttgttaaaaataatctttaattgtcaaagttactaaacaagcagtaatataagatgtttaatatccgccgcggggggcctgaaaatgttaattaaataataaaatgaattacttttcgggccggatacagactaaaaaagattcatgtgataggacacccgttttatatattagacgaaatagacagcaccaataactatgccatggagcaggtaaattccggccaggtgacatcaggcacagcctggtttaccagcaaccaaacagccggaaaaggaacccgcgggaaacaatggctcgcccaacccggagatatcagcgccctcacaattgctctccaaccggctatgttaccgctttcaaggcaatttatgctcagcgtggcagtcgccctcggaaccaccgatttcttcacttcctatgccggcgacgaaacaatcatcaaatggccaaacgatatttactggcgtgacagaaaggcaggaggcatcctgattgagaatgtattgcgtggaaatatatggcaatatgccattatcgggatcggactcaacattaaccaggcttccttcccgcccgatctgcccaatgcagtttccctccggcaaattaccggcaagtcccgtgaggcggaaaccctggcaagagaactctgcactttcctcgataaaaggatccgtcaactgcaacccgccaattatgaaacgctgcttgctgaatatacctcccggttgttccgctggcaacaatcaggtttataccggaaagacggggaaatttttgaaggcatcatccgcgatgtattgcccgacggccatctctgcctggagaaaaacggcgaaatattaccacttggctttggcgaagtggagtttattattacccggtaaccggttacttccgggagtaaacgttttgctcttcatgcaaagcccgcttcagcgctgccggcaattccggcgaaaggtccgacaacagccaggcgccggcgccccataagtattccctggacaaggcatctttcattacaccggtttgcgtcaaccggcctatcattttcatataggcgccttccggcttcttaccgattttaacaatgtaacggatggtgtccatctccctgaaccaaaaaacgtaatccgcatccattgcattggctaatggaatattcctccccctgttatagtaattcaaagcaccggcctcgccgtagttgtcacagatcagcaaggtgtaacgtttatccgcgtccggcacctgctgccacgtttgccacgacatatccgccagttccctccagccaagcatatccgcaaagtcctggggaagggtatgatcttccccgtcttcccagcgcaataaacccagcgcctggaacttgcccgccttttcacggatctcaacaggcttcattaccgggaaaataacgttcgccagcagtccaaaaggcactacaatgagggccacccagagcaaacgcaggtaacgcgtccagtcgtgcgtgaaaatccgctcccaataaacactcccgaaagccagtaataccgggtataaaccaaccgaataataactttttgcccggaaataggtaaacaataacatggttagtgcgtaaatgccgattatcacccggtaagaccggaacgacggcgaaataattaatcctataaccgccgccaccacaataaaagcaccacccacaaagaactttaactgatctcccaaaaaagaaacccggcttacatgtaccagctggctttcacttaattccttcatatgatgcaataccggtatgccatgctgcaactgccagatgatgtttggaaaaatgatcaccacggctactcccattcctgcatacaggtatttattcctgaacactttccggtgtgcggacagcagcagcgccaccaccattcccaatacgaggaaaataatattgtacttgttaagcacgcccacacccgtaaccacgcccatccacaacaaccatttgttctcctgcgtttgcagaaactgcatcaggcaccagaacaaggccgtccacgccaggatatcaaaagaattgggctgatacagtatgttcatgcgggacaagcctgaacataaaaatgcaagcgccgccaatacctgcgcaaaccagccgccacccagcttttccaccattttccacatcagcaccatcgtgagcgcaccatacaacgcaggaaaaaatttcacccaaaaaaaattattccccaaccattgtatcagtaaagaattaaaggcagtaagcggcggcaccgataagtatcctgctgccagatgattggccatatccaggtgtaggtattcatcccggtgaagctcgtaatacgggctcaatactgcatattgaaaaaccatctttataataatgaatgataataacaaccataaagaagtggggcgataccctggttgtccggtagtgggatgtatcatatgcggtgacaaaaaaaattttaaccattaaaaaaaaacggaaatacctgctgatgttgcaatgtatttccgttatagattttaaaatttcttgttcagtggcatatgtggcaggctgctctacatagcgatcatcagggcttgatgataacaagattttggttgataaaggcgttaacaaattgtgaaattttttctgattaatcaaaaatgaaattgcaactatgtttcatttacgaaaacaagtccctgtcagtaaggctttacatggatttcaaaccagtaaaagttaacatacccgcaagaagtactgaaagattttaacatagaattgtttaaatttggtgtatgccttcaagtaaaaacaactccattacactcaggaccttcaatgacttcaacgacgatctgctattatacacgcaaaaggaggtaactcccaaagcgccgttaaatggtagttttacagtacatgaaagatctgattgcccttgcgtggatgaagtgagagccagcagacgggactattataagatcagtttctttaccaaaggttccggcattttcaccctcggtgatagccgttacgagatcgatagtcctgctttactttttattaatccatacgaattaaaaacatggcagcccacctcggaagagcaggaagggtataactgcctgttcaccgacctgttgtttgaagcacagcccaatcaccaggaaaacctgttacaacacccgcttttacagatgggcgcaaaagcggtattcactttaacaaatgaacaggtcgattatctcgagtccattttcagacaactggtaaaagaataccgggagaatgccgcctttaaacaggaagcgattcttatttacctgaaattgctgatgctggaagggaaacgcctgtctgcccaggtaaacgaacccaaacggcagctaacagccgcacaggcgcttgctcatcgctttacagacaagctggaaaaacaattcccgatcgaatttacgcataaccagttgtcactgaaaactgccaaggaatttgcacaggtattaaatacgcatcccaatcatttaaatgcgtgtgtgaaacaggctaccggtcgtaccgtgagcgaacatatccggcaaagaatgctgctggaagcgcgcctgttgctcatgcatactgactggcagattgctgaaattgcctggtgcctgggatttgaagatcctggtaactttacgcatttctttaaaaatcatagcggcgtttctccacatctctaccgggcgcagtaatgcttgatttttgcaattaatactttgcttcttacaattccggaacctgtacctgcatgtaaatttgtatcactaaaaattttaacaatgcagtacagaaaactaggtaaaacaggcgaatcaatttccgcaataggactgggttgcatgggcatgtcatttgcatatggcaatgcacaggattttaatgaaacagaatcactggctacgctggagctggcactcgatctgggcattaacttctgggataccgcagatatgtatggtcagggtgccaacgaaatcctgctgtcaaaaattctcgctactaaaagagataaagttttcctcgctactaaattcggattcagattcaatgacgatggcaccaactatttcgatggttccccgaagtatatgaaacaagcagtggaagacagtttgaaaagactgaaggtagatgtgattgatctttattacacccaccggatagatgaaaatattcctgtagaagaaacagtaggcgccatggctcaactggtaaaagaaggcaaggtgcgctatctcggattatcagaagctggtgtggagtctattaaaaaagcctacgcggttcatcccattgctgcgctgcaatcagaatactccttgtttacccgcgatgtggaagacggcattttggccactacccgcaaccttggcatcaccctggtagcctacagcccactgggaagaggcctttccaccggcgccatcaacaacaccgatgttttgaaagatggtgatttccgcaaaaacctgccccggttccagggagaaaattttgagcagaacttacaaaccgtaaacgcattggaagcttttgccaaagaaaaaggtattaccgctgcccagttatcgctgggatggttgttggcacaaggcgaagatatcgtgcctattccaggaacaaaacgcagaaaatacctgcaggaaaatgccgccgcagcggaggtgaatttatcctcagatgacctggcagccatcgatagcatcttacgcgataacgccatcgccggcacgcggtatacaccagggggaatgcgcctggtaaacaggtaggacgcggattttgtctttctcaggattacgctgattttactgatttttactttggattttataaaggattaagggagatagaagcggatattgtactgctccccaaagtttagacttttttgattaggcggcttgagttcgatattgtattggactcaagccatttagttttaatttgattctatcgttattataatattctatatattctcgaatgt

SEQ ID NO: 16 - DNA, 116909 bp, Chitinophaga pinensis
  source 1..116909: mol_type = genomic DNA
ggattacgggagatacaagcgaatatatccgcttgtatctcccgtaaatattattaatctaaaaatccaaaaaaaatccaaaagtaaaaatccagctaatcagcaaaatcagcgtaatcctgagaaagacaaactccgctctaatcgcgccacgcatcccgcaggaaacgcagccagttgccatgcatcacattgtcgatgtcttcagcgctgtagcctcttttggtgaggagtgcgggtagttgctgcatatcggcgattgtttcgaggtcgtaagggcattgctctttaccaaaggcgccgtcgaggtcggtgccaatgcctacatggagtgagttaccggcgatctggcagatatgatccatgtgatcgatcattttttccaggttacagcccatgctttcgggtgtggaggtaccacgaacccatccgggtaccatcatccaggcgtcgagggcgccaccgataactgcgcctttccggatgagcgttttgatcatgtcgtcgctgaactggcggttatgatttaccagggcgcggcagttattatgactggcccatacggctccgttaaataattccatggcgtcccaaaaggcgtcatcgcacagatgcgtggcgtcgaggatcatatggagccgttccatttcacggatcagctgtttaccttgttcattaagccggccggtggcatcggtaccgttggcataacgccccgggccgtagtgtgcggggcctatggcgcgcaatcctttattgtaggcctgttcgagatacttgaggtttacgatagagtcggctccttcgaggctgaggatgtagcctatgggctttttgtcgttgggcgtaccatcgttccacaatagcaggtgttgttccagtccttgtttatctttgatcatcaccatttctccggcgtcttccatcgctttataccaggccagctgcccctgcgtttgggcccaggcctgttcaggagagtgccatcccggcaacgggttatccggtgccacatagcggcctatctgggtggctactaccaacccgatgttacctttccgtagttcggggaatgccaccacccctttgccacggtcgggtttatcgttcatgccggcttctctcgcacggatggcggttaccggctgttgcaggtccctgttccattccagcgcattcatgctgagatctaaatgtgcatctattataaacatagttcgcagatatccaaatgtttaatacagttcaaacaaagcttctatttccacggggatattatccggcagggagccaaagcccacggcactcctcactcctacaccattttcttctccccacaccgcagcaaataattcgctgcagccattgatgatgtagggatgccgctcaaagtcgggtgtacagttgaccatgcccagcaccttgatcaccctttttactttatccagactgcccacatgcgttttaatggtagagagcatggttaatcctacctgtcttgctgccagcttgccttgctccatatccagcgcatctccaatccgtccgatgatcagtgatttatcatgctgtacaggaccatgaccggagagatacaggtatttgccatcgataaggcaaggcttataaacacccaatggcgatggggctggtggcagttccagtcccagggccgctaatttctcttctgcatgattgttttccataattgctgttttaatctgcttataaatgtaatattgtttccatgaccagcaatgataagaaaaaccttacaatcctcacaaagtagaaatttgttgcttacaaaagaaaaagccgtctgttaagacggctcctaatcttccattacctgacaccggaatccattttcatttaccagcatcattatttttccgggatgaaaattctctccttccacccgtaacactttatcacagtcttccagatcaaaattgattttactatccggaaaattacggagcagcagcgcaactatttctttcgcagctgctacccgttttacattcgttacgaatacttctaccattgtaataattttgattacatatatttcatcggctcgtatttcaacagccgcctccacaaggcaatttgcccgatacaattggcttcccggtaaatattaaaagtgagcaggtcccagagcgacattttcatgccgggaaattccagcacatgatccagttgttcatccgttacatttaccagtgctgtttttaacaacggggaaattttctgccagtcttttttaaaaatttcgagagatggatactgctgtgagtcctttattccctggaaatctttgaaaagatcattcgccgtagatgtggcttccacttttagcaaaccggccagttcgaaccgctgctgtaccaggctgccggcgagccatgcaacgtggttggcgggtgtgtccagtcttttatgcgcatcttcatcagtaattccatccagtacctttggaaaaaattctgtgtgcaggtcaaatagtggaaggatgccctgcatccgggtgcttacagtttccatataaattattttttttggttctcaaactaacggtaaggtacctcttaatttttgtccggatagatgctgatagagtcaatattagggggtatttgcgccaaattcgttatgtttgagtagataactaaaaactgaaaaccatatgctacagattgggatcctgcttatacgccactacaagcttttaagcctggctgccataacagatgtactggacaccgtcaataagatttactataaaaacggtgagcctgcacctttcagaataacattggtacatactccggaaacggaacacctggcagccgcctttccggattatgcgtcgcaacatacagatgcagcaggcgctttcaacctggtgctggtaccctcttttactacggatgatatccgccagtcgatcatagaaaaccgggcttatcttccctggatgcaacaacaatataaaaacggtgctgaaatcgccagcttttgtaccggcgcatttttattgggggcttccggtttactggatggcaaaatagccaccacccatgtagatgcctgcagggaattttccgtttctttcccggctgtgaacctgttatcggataaaacagttacccatgattccggcatttacacgagcggtggcgccacttctaccttccacctgctgcttcacctgctggaagttcattgcggcattgaaatagcgataaagaccgctaaaatttttgcggtggatatgggccgcgacaaacaatcttatttcagcacctttcagcctgcccgtaatcaccacgacgacctcgtagcctcagcgcagcaaaaaattgaaaccagctaccaggatgtgggtacgattgaagaaatgatcagggacatcccttccagcaggagaaatattgtgagaagatttaaacaggtaaccggtgtaacccctattgaatacctgcaatttacccggattgaagccgccaaaaaactcctggagcaaaccggccagcaaatggcggaagtcatctttaactcgggctacaacgatcccaaggcattcagaaaggtattccgcaaaacggtgggaatgaccccttctgaataccgggaaaagtttaacgccgccagatcataaattctgatccctgtcccagaaagccggaggctctatgccgagggcgcggagatatacatacccctgtccgcggtgatgaatttcattgtcgaaaatgtaaaacaggatgctgatggatttaccttcatactgtccaaaggcagtgatctctttttgaaatgcttccaccgggattttaggccaccattcgttgagtttctctgtaatcacatcccagagttgcagcagctccgctttggtagtaggggccaccgacacgccggcatctttcagcaatacatcgatacccagccattcgtcggtgacaacgccgtacacggacggaaaggccattccgcaaaactccattaccaaaacagaaaagggtcgcataccgcccacgctgaaggtgaacagctgatcttccgggaatgcttcgatcatccggcgggtcaatgcgcggtgaccctgccagtgtttcagtaactgatcaggcgtaataacggtggtagtagttgcggcagataaggtgttgttttccatgagtgttgtatttttttgtttacaatacaaaggaaacacagagttgtgacaaccctatgtcagtagccttaaaaaaaagtttgccgaaaatttctactcctttgaatcaccagccaaaatatgacctggcattgccataacagatatcctgtatgatctttcctacggcatcgatatcgtccgggatttcgccccgctctatttcttcaccgaacagatcgcagagcaggcgacggaaatactcgtgccgcggataggaaaggaagctgcgggaatccgtaagcatgcccacaaagcgggaaatcagtcccatattggagagtgcattcatttgtctcgtcatgccgtctttctgatccaggaaccaccaggcagcgccgaattgtattttccccgctacagaaccgtcgttgaagttgccggtcatggtagccatgagttcattatcggccggattcagattataaatgatcgtttttgccagtttatcctggctatccagtttgtcgaggaatttagccagcgcacgcgcctgggaaaaatcaccaatggagtcccagccggtatcgggtccaagctgccgcatcatgcgggaattattattccgcagcgcgccaagatggtattgctgcacccatcctgctttccagtccatgagcgccagttccagcagcaacgccgatttaaactgccggatttcggtgtaggtgagcgactgaccaccgcgtatcttcaaaaagatctgccggatatctttctccagaaaatcatctgcataaatttcctcaatcccgtgatcagacactttacagccatgcgcggcaaatacatcatgccggctttttaaggtctgtaacaggtcatcataggtgttgatgttgcaatttgctgcctgctccagtttttcgaggtagcggttatatacttccggcacctctacattcatggcctggtccgggcggaaagcaggaattacgggtatttcaaaaccctcctgtttcagctgccggtgatactgcaggttgtcggccggatcatcggtagtgcaaacgagcgatacgttcctgctgcgcagcaggttttgtacgctgtattccggcgtttgcagcagttgattgcaggtatcatagatctgccttgcggatgccggattcagtatatcggtgaccccgaaatagcgttgcagttccaggtgtgtccagtgatataaagggttacgcaaagtatggggcacggtggctgcccattgttcaaacttctcccaatccgtattatttccggtacagtaactttccggtacaccgttggtgcgcatagcgcgccatttataatgatctccgtatagccaagcctgtgtgatattctcaaaccttgtatccgcggctatctgcgcgggtggcaggtgacagtggtaatcaatgatgggcatatccctggcgtagtcgtgatagagcctttctgccgcatcgctattcaggaggaaattttcatccatgaatttttttctcatccgtaaaaatatttaagtattacaatgacacccctcttttccagggaataaaatcatcctggccgttaaggacagattttgcagtaatggcgccgctggccacctgtataacgtagtcgagtatacgttctcctgcttcagcaatggtttcttcaccgtctataatagtaccggtattaatatcaatgatatcattcattcgctggtacagctttgtattgctggacagtttgatcacgggtgcaatagggttgccggtgggcgttcccagccccgtggtaaacagtaccacgttagcgccgctgcccacttccgcagtagtggattctacatcgttaccgggcgtgcaaagcaggttcaatcccggcagctgcactttttcggggtaatccagtacggcggctacaggagaagtgccgccctttttggctgcccccgccgattttatggcatcggtaatcaggccatcttttatatttccgggagatggattcatatcaaacccggagcctgcttcttctgcacgctgctgataggtacgcatcaaccggataaaccgggtggcgtcttccacgctgcggcaccggtcgctcatttcctgttctactccgcagagttcggggaattcagcaaggatgacagagccgcccagggccgtcagcagatcggacgtatagccgatagcagggttggcagagataccggagaagccatccgagccgccgcactccagcccgatgcataacttgcttaatggcgccggctgccgggtacattgattggcgatcatcaggccggcaaacgtttgacggatggcatcagcgatcaactggctctctgcgcctgtttgctgctgatcaagtatatacagcggctttgaaaaaccggggtcgcgcttattgatttcgtcctgcaacatgctgatctgcgcattctggcaacccaggctcagcaccgtagcaccggcaacgttagcatgggtgatatatcctgccagcaggccgcacagggtttgcgcatcctggcggataccaccgcaaccgccatcatgtgtcaggaatttaatgccgtccacattttcaaatacgcggctatgctgcactcccggcgcctcttccgtatacacggtttcgaggatctgtgcagggcctgcgccggtttgctgctttgcggcaagtgaacgtgtgaaggcagcatacttacccgggcgggcatatcccagttccggcagcagcgcttctttcaatacttccacattcctgttttcacaaaacaccaatgggatcaccagccagtaattagccgtacctacgctcccatcggcacggtgataccccatgaaagtcttttgctgccagcgggaaacatccggtggttgccaggtggttttccgctgggcagccagctcgtagctgctagctgcatgatgcacattttccacagcaatcctgctgccggcactgatagtgcgctgcgcacgacccaccagcacaccgtacatgtaaatcgcatctccttcgttcatggacgccaccgcaaatttatgcttggcaggaatcttttcctgcatcgtatatacggcgccgttatattccaccatttcttccttttccagatcctgcagtgctaccagcacattatcgtgtggatgcacctttaatactttctgcttcatttatctgtccttgttttttttacgataccgttatttctcctgctattttttcaagataaacagctaccccctgttccattaacgctttcagcatcgtagttaccaactgtgcgaagccgggaatgacagtgaggttacagccccatatcgcctcgttgctgaaagaatttttcaccacttcctccggcgtatgctgctgccactgcgccgcataccaggcggcatgctcatccgtgatggtatagctactgccgccccgcataaataacgcatgcgcagcaaaaccgagcgctatcaacgcaggcacatgttctgtacgccggtgatattgcaacagcaccggcagtacccgcattttcaatttcgccgtatactgactgcaaatgcttaaccaccggtgttcgatagccgggttgcggaagcggtccagtacagcgccggcaaaacggatggccgcatcatttcgtatatggatatctgttatagcaggtataatttcatgcatcatcagtccttccatataggcagccattgcctcatcattcatggccgccttcaccgtatcgtgaccagccaggaaggccagtccgcagctaagcgtatgtgtgccattgagcaaccggagcttcagttcgcggaatacattgatgtcgggcgataataccaccccggcatctgcctcactgaaggataatatcttcttcacatgatcattgctggtttcaatggcccataagcggtatacttctgtcatgatcaggagatcatcttcataaccggttggcaggtaggccgcaccaggtacaatgcaatccaccaatgaattacaacagtagttactgttaacaagccagtgtacaaatccttcttccagctggttaaaggcgctcagctgcaacagtatttcccggagcctgctgccgttatccggtatcagttctgtaggaataatcaccattcctttggtggtatctcccttaaaatggtgataacggcgatacaggaaggccagcaatttaccggggaaggatgccggcggcgttgcatgaatactttcttccacatacacaatacctacttcggtggtattggatattactacctgcatatgcggactggcagcgcagtccataatatcgttccactgggtagcggctgtgagcaccctgctgatactggcattgataatattttccgataccgctttaccgccatcaatgccccggatacactgtgtataaaggttatcctgttcatcgaaagcagcggtactgcctttatctgttgacttcaccaccactaccctgccattaaacaatccctgtttattggctttatctatgaagaaaccgggcagtcctctcagcaatacgcctgttccaaattgcagcaccttttccggcagcgtaaagtattcttccgccggaacctgcagcccatcattttcgtgcagccgtgccagtaattctttagaaagtttcatatccgcattatttagtcatcatttccatttcgttggcagctaaaatatacgcgcctacgcctttaggatcattatcaattactttttcgctgagataataggcatagctgccatcccggtagggatctccgccaagtcctgctacgcttaccgtaccgcttagggtgatatctccttccggatttttacggataaactgtttcaggattcccttgtatcctttctgtgctactccacggtaactagccggcaggtagcctaaacgcatgcctttcgccaacgcatatacgaacatgcaggaagcggaggcttctacatagtttcctgtgctgtcgcctttatccagcacctggtaccagcaaccggttttggcgtcctggtattttttaacggcggcagcggtgcggtttaaaatggcaatgagactgtctttgccaggatcaccggccggataatattccagcgcatctaccagcgccatggcataccagcccattgcgcggccccagaagtgcggcgattgccccgtggttttattggcccagcgctgttcctttgattcatcccaggcatgatataataagcccgtacgggaatcccgtgcatactgctccatgagtacaaactgacgggtaatatcacggaaggcgctgttttcaccggtaagcacggcatactcagcataaaaaggttctcccatgtaaagcccgtccagccacatctggtaaggatagcgcttcttatgccagaagccgccgttgttagtgcgcggttgtccgcgtagctgctcccgcaggtgatcggcagcaatcttatacttattgtccttagtggctttatacaacgttagcagtatccggccgtttttaacgttatcaatattgtaatccgtcagctggtacgtatggatgttaccgttagcgtccacaaaatgatccatgctcttttgtatgtaccggaaatattcctggttgcctgtccttttccacagaccggtaaatccttcgaggatcacgccctggtcgtacgaccacctaaccggcctgccaggctgcatttccagtgagtctttccatatacgcatgaccgtagccgccatgccggcggcgccggtttgggcctgtgaaagtgtagcagtgagcaacagtatggcgaatagtattgatgttttaaaacgcatggtcttctgttgatttggttttagtatcacggtaacggcaactgtctgttgtaatgttttttgtattacgggtatccagcaccgctttgccggaagcggtaagaagatacacatttttgaagtgtatgttttcagcttcctggcactgtatgccttcatcggctttgatcaccaggttactgaggtggatattgctgaccggcatttccggcaggccgcgtatgaacactgctctctttgccccattgccggttacgttattaatataaaaattgcggaatcgcggtgttgcttcggtaactggcagcgtttccacacgtggagccactctcttttcccctgccagtggcaccgggtcttttgcagcgtagtacatatcaaacaggatggcctccccggggatatctttcatgtttatattggccgcataaatatcttccacgatgccgcctcgaccacgggcagttttgaaacgcaacccgatgtcggtacccaggaacgaacagtcggatacataaatattccgggcgccgccagacatttcgctgcctattacaaagccgccatgcgcgtggtatacggtagagttttgtatcactacattttcagtgggcttgcctcttttacgtccctgctcatcacggccggatttaatacagatgccatcatcgcctacatcaaaggtgcagtcgaggatttgtgcgccactgcatgattcaaggtccaccccgtcgccattttgtgcataccagggatttttggcataaataccacgcatggtaatattctcacaaagcagcggatgcaggcaccatgccggtgagttctgaaaggtaactccttccagcaatacatttttacaggaggcaatactcaccatgttgggccggagaaaatctttgatgccggcgtagtcttcaattttactgcctggcttgattacgcctggcaggctggctttcgctcccaggtaagatgaccgggtaggataccaggtagcactgtcttcccccaccagtccgccggaagcaaccagtttgtcccattgcgtggcagtgagctttcccttcttcaccatgcgccaggcatcgccgccgccatcaagaataccactaccggtaatggctatattttcctggttatttgctgaaaccggcggctggcaacgtaccgccgcaagcccttcatatgtagtgctgataagcggatactggtcgaagtcggtggtaaactgtagcaccgcgttcttcgctaagtggaggttcacattatttttgagcaccaccggcccggtgagccacagcccggatggtattaacactaccccgccgcctttattgctgcaggtgctaatagcttcgttgatagcgttactgttgagcgtaatgccatctgctttagcgccaaaagaagtgatggtaaaagtatctttcctgaaatgcggttcataaactaccggtagctcatagcggtatttcccttcaaaaggtgttgtttccaggtaagcggccagcggcaatttcttttcccggatttcaccagcaacaagagcagctatcttagcagcgccatatgcagaaaaatgggtattatctgtaatcccgtccggcagcgtattgtaatgtcccggaggggtggtgcggaacattttctgagaggctgcttcaccttcctttaccagcaaagcggcactgcttttttgcagatctaccagcggcacctgcatcgcattcgctacggaccttaccactgccggataagcaccgtgggtatcttccaaaactccatgcgtaaacttgcggcgcgctaccggtgtaatgagcagcggctgtgcgcctttagcacgggcttcctttacaaagcgctccaggttggttttatacgcgccttccggggcagcatagcgggttgaatcactgatcttcccgtcgttgtgaccaaactggatcatcacccagtcgccgggttttaattgcgctaacacactatcccagcgacgttcatcaataaagcttttagtgcttctgccgttgacggcatagtttttaatgacgatatctttttcaaagcattgcgggaacagttgtccccagccgcgctcaggattatcttccagtggcttgttagccatcgtggaatcgccgatcatgaatatagtaggtttgggaccggctggcgccagtcccaataatgataataaaagtatctggagaattttcattagttatatttatcgttctgcttaaactcctctttattggtcaccgcatcaatctggtcctgcgggataggccgcaccgtatgaaacgactggaaatatgcattggcatccgggttatgcagggcgatccgctcaccgagcttaccggtacgtttcaggtcaaaccagcgcagttgttcgccggccagctcccgcgccctttcatcaaggataaagtcgaggctcatatctgcggctgttaccaccatatctgcttcatgtccggggatggcggcacgtttgcggatcacgttgatatattctgccgctttagctgaattgctcaatttgaactgcgcttctgctgcaatgagatacatttccgcgaggcggataataaatgcgtcccgtgcgctttgctcttcgttcatggatgcccgtgtaggatcatcaaatttatccagggatacataacgggtgcggtcttttccgccgccattttctgtatacactgcattcctgtcgtatatacggtatttggtagaagcgggcagcacatatttgctgcaatagatagccgtatcacccagcttcatacctgcaggtgctgttttgagattattgcaataccacacctgtttgaaagaaccttcgtagcgtgcatccgcagtttcgttgaaaaggtttaacaggaacagcgtaggcatgtaacggttaaatggccgctggttcaggatatcacgctgcatacccggcaggtcgtcgtacttcatggcaaacatcatgtgtgcattattggcgccgcgtgagtgtccgttaggaaacagggtagcatcggtgcgatcatcaaacacgagattcttcatataatttaccgcccagatcacttctttattctgcaggttatccatacgccagagatcagcgtatttgggcaacagcgtatagccgtagctgctgatcactttttctgccaggtcggcggcctgttggttcatgccacgggtgagatacatcctggcaagaaaggcttcagcagcgggtttagttacacggccatagtcagacgtggtagcaggaaggttgttcaccgcctcgcccaggtcgcggaaaatctgtgcatagaaggtatccaccggtgtacggttggcggtagttactacgccagatgtttcggtgagggtaaaatggacaggcccccatgtttccacgatatgccagtaataaaaggcacggaggaaatgcaactcagcgctgcgcacggctcttctttccggcgttaacccggcgccatctatacgtgtgatccctgcattacacaaattaatagcggcatacagctgtttccataaaacactcatcacggaattgctggcctgcaggttgttgtagttggtcatatcaggatacttatcgccggtgccgcttgtccagatatcggtccccatttcggacatgctgtatccttcttcttttccataccaccaacggttataggtatacgctgcatttaccagtgtttcaaacccttcgggtgtggaatatacggcatcggtggtagtaccgccgggattgtattcttccagctgcttgttgcagccggcaagacttccggcggcaaggcacaatatgatgaggtacttatttatattgggtgtcattgttacgttttttaaaatttagaactcaacatttattcctgccacatacatcttagtaagcgggttgctcagatctcctcccctttccgggtcatagtcttttaccttgctgaaggtgaagaggtttttaccggtaacgtataaacgaagactgctcaggtgcagcgcttttaaagcatcggcggagaaagtataaccgagtgaaaggttacggattttcacgaacgaaccatctttatatcccagtgttttgataaaaggcgtaccatctttggaaagactggcattgggccggggataatcgttggatggattttccggtgtccagtaatttacaggcgcactgttttccaatccctgcggatcatattttgctgcatattcggagttgatccactggccaatgcgggcgaaaacataaatattgagatcaaagttcttgtaacggagatcgttattgaaaccaccgctccatttaggcacctgcgcaccaagtatcacgcggtcggatgtattgatcgttccttttccatcctggtccttcactttgatatcgcctggtttgtaaccaaatttcgtagcttccgcagcttctgatgtttgccagataccgattttctcatagtcgtaatatacttttaccggcgagccgataaaccagccattggccacatcgttggtgctgccatctgccagcgctacaatttcttctttattgcgggagtatacgatgttggacgtccaccggaaatcgcttgttgaaatgttcgtagtgttgattcccacttcaatacccctgttgcgggttttaccaatattctgcaccacggtgctcacaccggaagaagtaggcagggtgcgttgcagcagcaggtcttttgtctgcgtgtcataataatcaatgctaccggtgatcctgttgttgatgataccgaaatcgagtgctatatttttggttgcagacagttcccatttaagtcccttgttaccagcctggtcgccaatggtgtaagccatggctgcatttgtatcatcccatgaaaagggtattttactaagatagctcatggtggaataaggatctaccgcatcgttaccggcaataccatagctcacccgcagtttcagatcactgaaaaaggtttgcgacttcatgaacgtttcatcgctgatgcgccatgcagctgctgctgagggaaagaaagcccatttgttgcccggcgaaagcttcgatgatccatccgaacggccagtgagcgacaacaggtattttcctttgtacgcataattcaggcggccggtaaaggaaatgagtttgctggattggtacatactgcgtgcagcgatgccgcttacgttattttgcatggcatagtacaactgcgacggaagcaactgtccttcgccctgcataagcgaggaatcgcgctggtccgacaatacgctggctacgcccgtgacgccaaaggagtgatcgccgattgttttattataggtagccacgttttcccagctgaggtacctccgggtgctgccgttcgactgcgaccgcgaagtggaagcggtagaccggtcgatagagcttttggaagcaaacacgccctgttttgcattttccagtgttacgccaaagttggagcggaacatgaaaccactgaagggtgtcagttccaggtaagcgttgataaatgtacgggtagtgcgggtgttattctggtaagcattcggctgctcatccgccagcggattgatggccgagccgctgttggggaataacaccaggttgccggcagaatcgtacggtatggccagtggaatatacttattcgcctggttgagcgggtcgcggcgggcgctttgttcgtaatacgtaatctggctttgcgcgcctattttaatagcatcattgatcgtttgatcaatgttgagacgggtggaataacgtttgaggtcatccagtttcaataatcccttttcattaaaataatcaaaggagaaatacacttttgttttttctgatcctccggagatgcctgcctggtagtcctgctgtaagccgttatgtaacagcaggtctgcatagtcggcccacaggttatgttgtatttcattcagttcaaaagcgttaaatatttttggatcatcggcctcggtggcccatctgccggtggtacggttagcttcccttttcagggcggtatattcgggtccgttgctcatacgtggatagccatttacttcagacgatccaacataagaactgatatttacacggggtttaccgctggtaccgcgtttggtggtaaccataattacgccgttggcgccgcgggaaccgtagatagcagtggaagacgcatctttcagtacttccatcgactggatatcattcgggttgatgtcctgtatattttcatactgtacaccgtctacaatgtataagggaccgttgctggctttgatggagcggttacctctcaccgttacattcacttttgcacctgctgcgccgctgctgcgggtgatatccacaccgggcagctttccctgtacagattccatcacgttggtagagggtacttttttcagttcttctccttttacggaaaccaccgatccggtaagatcccgtttttttaccatgccgtaacccactaccacaatttcatccagcttcttgttgttgggttccattttgattgtcatggcgacattatccgcggtgagtgtcatcgctgtatagcctatatagctgaataacagctctgtttttttcccttccggtacctggaggctaaaattcccatgtgtatctgtttgggtaccagaagtagtgcctttgacctgaacacttaccagcggcagtggatcgccggtagtggcgtctgtcaccttccctttcacggtacgggtctgtgcaatcgcccaactgctgaaacccaacagcagtaagcaaatgaagtaaattcttttcataacgtttggcgtgagttaaatggcaaataaaagttgtgctatagtaagcgttgattaacgtggtgattaattggtcgaaacaggagctctttcttccgtattgtactgttacaagtctacagaacaatttgttaatggtgaagtttatttacgcaatcgttcccggaaaaatcagtactttcaccataacaagaataccggaaaacatagtccggaagccgttatgaagtatagagcagcaaccataaaagatattgcgcaggcgcttcgcctgtccacttccactgtgtcgcgcgcgttgcgtgacagccatgaaatcagtgccgccaccaagcagctggtgttggaacatgcagcaagactgaactatcatcccaacccgattgcactgagtttgaaagaaaagaaaagcaggtcaatcggcgtgatcgtatcagaaattgccaacagctttttttcacaaacaattaatggcattgaatcggtagctaacgagaagggctatacggtaattatttcgcagagccatgaatcatttgagaaagaagtgagaacgttgcaatacctggcgtcccggtcgatcgacgggttgctgatttcggtgtccagtgccacgaaagacctcacccatctcaaggcgttgcaccagtttggattcccgattgtattcttcgacaggatcatagaagacatcgccacgcacaaggtgatggtggataatttccagggcgcctacaacgctacgatgcacctgcttcaacagggataccggcatattgcctgtattaccaactcagcgcatctctccattacgcgggagcgcgtggcaggatatatggcagcactggagaagcatggcattcagcctcaaccagcgctgatcaaatattgttttcacggtggcatgctgcttcctgaagtaacggatgcagttaaccagctgattaaattaaaacataaacccgatgctatttttgccacgtctgataagctcactacgggttgcatgcgtgccctgaaaaaagcgaaggtggctattcccaaagaaatggcactgacaggattctccaattcagacctgatagaactgctgcatgcgcctattccggttgtgcggcaacctgcttttgaaatggggcaggtagcgaccgaattattactgcaactgatagaaagcaagcgacccgttaaagaatttgaaaccagggtgctgcactccgagttgctgataccatcaaagtaacggggtttattccacccgccaccaatctatatctgcccagccggcatcgtttgtttttacgtcccggctgcagcacaatcccatcttggcgcctatccatctgccggtagtggcggtaaatggttcacccgtggtatggaaagttttcccatctgtgctgtaactgaattggcatatacctcctgcccccacttctaccctgaaaaatatatccgtcgacgttatctctgttatagcggtggctgtttcacgggagcttttgtcagcctgtgtacaggtgaagtacgacaaataaataccattcgcttttttcaccagcgacaaccccgcatagtttgttcccatcaccaggaagctgacacgatccccattttgccgtggtttaaagctcagctttgtggtagcccggaataccggcgccgggaatttctgcaggagtacatggggtacttcccataaattacgggcgctatcgggtatctgtgcggcaaacaggcgcaggctgccttttgccacagacggaaacgcccagccggcagccgggttggcctgccattgccattgcaaccctaaagtgctggcattaaactcatctgattcctgcggcgtggcaaccgggtaacccgcaccggtaaccggtttgcggaaggtcagcaccggttctcctttcccatcgttgtcgttatctgttcctatcaccggccagttgttcacccatttcattggctgcaggtgtactaccctgccgtaagcttccaggtcctggaagtgcaggaaccagtcctctcctttgggtgtttgcacccatgcgccctggtgcggcccgttgacaggcgtacgcccctggtccattacgattttactttcgtaagggccgtacacattttttgagcgcattaccagctgccagccggtggcgactccacctgcgggcgcgaaaatataatagtagccgttgcgtttataaaacttcggtccttcgagcgtggggtgttcatcgtgcccgtcaaataccagcacgccttcatccgtggcttttgtaccggtggcatccagctttttcaccacgataatacttttaataccggcgcggctgccggcgtatgcgtgcaccatatatacgtcaccgttatcgtcccaaagcgggcatgggtcaatcaatcctttgccacctaccaccagttgaggcgtactccacgggccggtgatctgttttgatttcaccacgtagatcccgaagtcggggtccgggtagtaaatgtagaattcgttgttgtgatagcgtatggctggcgcccaaacaccattgccgtgttgtggcacggaaaaatgatcgtaaggaggctggcgcagcaatgcatgcccgataatacgccagttcaccaggtcgcgggaatgcaggacaggcagaccgggaatcgcatcaaagctggaggcaacgaggtaatagtcttctcccacgcggatggcatcagggtcagagtaatccgcatacagcaccgggtttttataagtgccgtctcctttatcagatacccatactttagaaatatccgcggtcgattgtgcgatagcagtggtagcagttagcaggcataacacaccggtgattatctgcataaagaactttaatggtttcataacgtgctgaaaatgtgccggtcaaattagtaaatgacctgcaaaagcaggacgttatttacgcaatcgttcccgttaaactgaaaataactgatatttgtaagaatcagttagccagagaaccatgcaagaaattattatccgtaaagccactgccgcagatttgcctgtattgctggagtttgagcaaggtgttattagtgcagaacgcccttttgatcccaccttaaaagagggcattatacattattacgatatagcggccatgatcaccgcttcgcatattgagctgctggtggcagaagcagccggccagctgattggctccggctatgcccgtatagaggatgcaaaaccctatgtcaggtttgcgcaatatgcttacctgggatttatgtacgtggcgccatcctggcggggtaaaggggtgaataagctgatcattgaaggtctgaaggcatgggcacaatcgcggaacataacagaaatgcgcctggaggtataccatgaaaatacgcccgcaattaaagcttatgagaaaaccggcttcagcaagcacatgctggaaatgcggctccccatatgagtttccgggatttcataaaaaagtggcacaattttcgacaggtggcggggtaaagaacttaaaaccatgaaacagatactcgtagccttagctgcagcagtcgttttcttttcctgcaaaagtaacgctgataatgccgccgctattgaaagtgcaaagaaagccaccatcgattcgatgaataatgtgagtgccatcaaacagcaggtagtggattccatgaatgccttgaaaagcaaccgttcacatggccgcgaaaatgtagccggtacccaatataacaatgaaaccgctccggtggtagccaatacagaagctcccgcgcctgcccccgcaaagaaaaagggctggaaatcgtggagccataccgctaaaggtgctgtagtaggcgccggcgcaggtgcagtaaccggtgctatcgtgaataaagaccgcgtgaaaggcgctgccatcggtaccctgatcggggctggtgtaggtgctggtacaggtgcaattgtagatcacaagaagaaacaaaccgcacaacagtaacaggtaataataatgaagaaacggcgtatcctcacgggtacgccgtttttttatgatatcaatcagcagataacggtaacgctactacgctattggtgtaaccggctatcgcggtgctgaaatccccattcgttcaactgatcccatacaggaataagccgcgcagcgatttcagtaagctggtattccactctcggcggtacttccgcatatacggtcctggtaacaagcccgtccgcttccagctcctgcaggtgcagggttagcatgcgatcggtgatattgggaatgtgttctttcaactcaccgaagcgcagcgttctgttcaccagcttgtacaggatatataacttccacctccccgccaggatatcaatggcataggccaccccgcacacacctgaaatctgttcgcggttcaaatgattggtagacgtttccttgcgctttgccattacttacatttttgtgtgttgcatacaataggcttcaaaaatacaaatgtaacgttcgtggaataattttgtccgcagttatttaaaaaacaacttttatgaagatattaatagtttatgcgcacccggaacccaaaagtatgaacggcgctatgttcaacactgcagtgaccacactcctggacgcaggccatgaagtgcaaacctctgacctctatgccatgcggtttaacccaatttccgatcgtaaaaatttcaccacagtatacaacgatgcttttttcaaacaacaactggaagaacagcacgcctcgcgcgtacatggctttgcagcagatattgcagccgaacaggaaaaaatagcctggtgcgatctaatgatctggcagtttcctttgtggtggttcagcatacctgccatcctcaaaggttgggtagaccgcgtatttgcaatgggcacctcctacgggaacagccacatttatgaaaccggcatttacaccgggaaaaaagcaatgctttcgctcaccatcggcggaccggaagatgcgtatattagcggtggccttcacggcgacctggaaaacatgctgaaacccattcaccggggcatcttccaattcacgggcttttccgtgctggagccatttgttatacatggccccgccagaatatcaccggaagaacgcgcactggcactggaagagtggaccgccaggttaaaacagattgcacaagaaaccactattgaagtaaccaattattaataatgaagatacttatcataggcactaccggcgccatcggcagtaaagtaaaagaggcgttgtcagcaaaacatgaggtgatcagcgcaggccgcagcagcggcgatatccaggtagatcttaccgatgcagcttccattgaaaacatgtacagatccacacccggtatagatgcggtgattgttacggccggctcctccggcatggagagctttcaaaccctttccgaaaaaagtttgctaccgggcatccaatccaaattactcggacaagtaaatgtagtactgattggccagcattacctgaatgaaggcggctctttcacgctcacctccggcatactcgctgacgaacccgcccgggatgccgctgcaggctcgctggtgagtggcgccgtgaatagttttacgatagcggcggccaccgagctgaaaagaaatttgcggatcaatgccgtgagccccggattggcagccgactccgcggatgcaattgcacatttgtttcccggctttaacccggtgcccatgcagaagctggtaaacgcttacctcaaaagtgtggaaggagtagtaaccgggcaaattatccgggtacatgaataagccctatgcggatatcgccgattttactttttcacggtgacaaagcccccacgctaccaggttttctgctacggggagaatagtttgcccgtatggtgtaatggcatacgccacggttaccggtttggtggccagcaccgtacgggtcaccaggaaattgatctccagtagctttagctccttcgataacattcgcgcagagatgccattgatctcccgcagcatttttttaaagtgattgctttgctccgtgcggttggccaggtaccgcagtaactgcagtttccatttgccgctgaacagttcaatgctgtcgcgcatggccgtgagttcttcctcacaggtggcttcccgtatctgccctttgatgttgatcgttgccatataggttctcctcatgtaaccggttacctccggtatacctatagcaaaggtaacccaacatagtaataattttgcgggatgaaacatcaaatgcaggcaatcatattaaacgatttcggcggtgtggagaatttctccatgactaccatgccggtacctcagccaggcgatgatgcagtgctggtacaaattgcagctactgcctttaacccgattgattaccagatcaggcaaggcgctacagaacgcaaacgcatgcactccccggtgctgggccgcgaattttcaggtgtggtagtgaaaacaggcaaagatgttacgcaattcagccccggcgacgccgtgatagcagcatccggcagtatgggctccaatggcacttacgcggaatatatcagcgtgccgcagcacatactggcgcataaaccggcggatattccctttgcaacagccgctgctattccaacgggctcccttacggcattgcaatgcataaacaggctcggacttcctccgcaggcatctgttttgatcaccggcgcagccgggggcgtaggactggtattggtaaaactgctgctgcacgcaggttttacgcgactgctggccaccgcgggcagcgaagaaagtacgcaacagctgatcaacgccgggctacccatctcccaaattatcaattaccggcaaggcggattattgcaggcaatactgcatcagcaggaaggaaaactgtttgacgcatgtattgatctcgtaggcgggcagatgtctgaaacaggggcagcactgcttgctaccaacggtatttaccaggatgtaacagcgcttaccacggcagcagccagggaaaccttgttcaacaaaggcgcagtaatcatgaatatttccaactatgcatattcgcttaccgggaattttaaatattatggagatggcctccggcagataaccacgttattggaaaccggcgccctgttaccttcccccatatggatcactggcggatttagcgtggatactgtacggcagtcgcaccaactgctggaactcaaccagagcaagggccgcaagctggtgatgactgtattttctaatgataacttaatgacggaagggatataacggcatcatgtttgaggcaaggcgcgcatgtggaatcaacttattgaaaatgcggaccacctgcctaatttcctatggaaccttatactggcggggattgcagtcatcacaggatggctgatcaaatatctgttatcgatttttttgcgtcaatctgtacggacacagcaggacttctctttaatacatactatccttttccgccttggaaaagcgtttaactatttcctgccgttgctgctgctcaacatggcaatcccgttaatgcgggtacaccagcaatatgtaccaacgctgagtaaaatagcagaaatagcactgacgctttcttttgcagccctggtgatcggcgccatcaaagtgctggaggattatgtgtaccatacctacgacctgaagaaagtgaacaacctgaaagaacgtaaaatacgcacccagttgcagtttatccgcaaggtgtctattgcgctgatactgatattgacggcctgtattattttactgagcttcgacagcatgcgtaaactcggcgcaggactccttaccggtgtgggtgtgggcggtatcatcattggttttgccgcacagaaatcactgggcaacctgctggccggcttccagctggcatttacacagcctatccggatagatgatgtgctggtggtggaaggcgaatggggacgtgttgaagaaattaccctcacctacgtggtactgaatatctgggatcagcgtaaactgattttaccgattaattattttatagagaagcctttccagaactggacccgcaccggttcagaaatattgggcaccgcgttcttttacctcgactataccgtgccggtggaccaggtgagggccgagtttgaaagactactggatacatccccgctgtgggacaaacgcgcaaaggcgctgcaggtaaccaataccagcgaacgcaccattgaagtaagggcgctgatgagtgctgccagttcaggcgaagcctttgacctgcggtgttatatccgcgaaaatctcgttaagtatatcagggaacgtcaccctgacagcctccctaaaaccagggcctatattgaaaataaggacgaccggcctttgtcagtatagcgatttttccaacacgatcaggtgcttgcattgaataccattttcatagatcggttcggggtaatgggtggtgaaatagtttttcttaatggctgttatttcaaatccctggcgctggtataagtacaattgagcaatgctggagttgcccgtgccaatacaaagctttttagaaccccctgccctggcgcgttgtgcagcatcctgcaggaggatttttcccagcccctttccctggtaggcggggtttacggcaatattcttaatttccagttcgtcgttatctttcaacaatacataggcgccaatcacctgtttctttgtttccagcacatatacgtcgctgaaagggaggtaactgttgatcatcgttacagatggatcggccagcaataacaggtcatagggcatcttctcgtttgtggctaatttccggatagttgtttcttcctgcagggaggtcatcgataattattttgttgctataaattggaataataggtattttcttacaaaccggtcccgggcaacagctacaaataggttcagggaacagattaacaaaatgaatatacaaaaaaaacaggcatctgtgtaaacagatgcctgcaatatgtttgattattgaatagcgatatactggcgttttacgttatgaccataaatttctaccagcgcatccttactggtggcggttgcgccgccgctgatgctgatcgttttttgatcgcctggtaatacagaaatataattatcgctgtaaaataccggtaagatccttttcttgttctgtgcatttaccagtgataggtggttgaaaaatgccacagggcctcctgccggattgctgatagttacattaatactgtcgcctcccgctttcacggccgttagcttcacacctgctgccggcatttgtgctaacccggaataatttcctttggcatccggcaaccagtacaggttttcatctaccacctgctgcgcggcgttcagcaagcgcaaagagaagaacaatccctgcggcgcttttaatttatccaggagcggtttcatattcatgaatggctgcaccgtggtgggtcccacctctacaaatacctgtgtgagcaggctatcgttgccctgcatgtcgtatgtttttaattccagcatcaggtcgcgggcgtattgaaaggtgttatttacggccattaccattccctcttccgggttatacatcacatgcagcggggtggctcctttgcgggtaccatacaggcaggcattggggtcaagatagtaatcatacatttgtccgcgcagggcagtccaggggttttgtgttttccagatgatcacaccggtataccaatcccacatatgtgaactgataccttccattaaaccgcggtactggtcgtagtttactagctgtgctttgttggcccactctcttaaatcatttgtttttccatagggatccacggctttgttataagcgatatacttatggtaatcccatacggcgtcggttttgccggtttgctggttgggcggcaccaggttttccgtgggtaaaaatctttccagtgactcataatcgccggtgcctaccgaacctacttcagagttaaacggaaaggtgcgcgtgctccagaaggtggacagtggctgaatgccgtaaggaccgtcgccgttaccacccagcgtgttgtgcgacatgctgtctgaattggagtagtcgaagaaatagcgggtgccgtccagtgacggaataatagaatccttcatggcggcgaacaaatctgccggaggcgtaatttcatttcccccgcaccagaaagccagcgaggcatggttgcgtaacattttcacctggtcggctacactttcgaggaacagggaatgattgtcggggtatttgcggcgggtccactggtcgtcctttttcatggggtcctgccatctgccgttacagtcgcctgagatccagaaatcctggaacaccagcaggccgtacttatcacaggcttcgtagaactccggtctttccgtaagactgccgccccaaatcctgatgaggttcaggttcatatcgcggtggaagcgtacttccgcgtcatatctttctttagtgaagcggaacatggcatcggaggtaatccagttgccgcctttaataaatatcttctgaccgttgaccgccacttccctgctgccggtgtgtgcattccagtacgtttgaatttcacgcacaccgaattccacggcttcctggtcatccgttttaccgttgtttataaactgcagctgcagctggtagagtgattgcgggccatagccggcgggccaccataacagcggttgtttcagcaacaagtccggtagttgcacgatggcggtggcatgtggcggcaaggctactttctttgtgatgcggttccctgcgagggtgtattgcaaagtaccggtaacaaccctggcagtggcattttccagcgtggctcccacctgcagggtagccggcgcctgtgggccctgtggctggcggacgccggatacgcgggtaatgatgtgcgggtctttaatccttacggcgccggttttttcaatggtcactttatcccatatgccggtgttgcggtcgcgcatgggttggatccagtcccaccccgcggtatactgcggaccattattttttgcgatggtaccatcgcctccctgcccaccgttggggttacccggaaactggggcgggtacacgattacagcgagacggtttttaccgttcttcgccaggaaaggagtaatgttatatgtttggcggagataggcgccatagtgagtggttttatttacgcgatgcccgttcagataaatatcgcagccatcgtttactgcccggaagtgcagccatacctgggcgtcgccggtggccggctgttctgtaaagtcctttacaaaccagtaggtgtaatgatcacggccaacgtgatagatgtccggaatcttttcattgttcatgccgtacatcggatcgggcacctgtttattatccagcatcgtggtgagcaccgtgcctggtacggtggccggcgtccagccggagagtgtatagcctggatctgagagctgctgaccggtaacttttacaccagcaatattgctgcattgccatccgctgttgagttcatatttttcctgcgctgataatcttaaaaaagacaacatcagcaggcaggagatcgttgatttccgaaacatagtgctttttatttttacgggcccgtagttacctgatacaataaccgcaaagatagcacaactgtattccggatcaaagcatgtccatttttttggtcagaaaacaggaaaccccttcgcctgccgtgccggcaggcgaaggggaacattagttgataacagcttactgctgttctgataattcttttactttatccagcgctaatggccatgctttattgaaatagtctttaaactcgtcagccaggtccatttctaccagcaactccgttttgccgttgacgttagtcagcgtataattttcatatgcgccggcccaggcttttactttgtcgctggtgaggtcttccacgccgttgtcaatttcaccgaggtgttgaaacgacataaattcattgggcaccttatccgcaatcctggccaccataccgcggttactgccatcgtggaatattaccttgcttcctttctcccagttggtatctgctttagagccttcagcaaaaggagctgtccactgcggataggaattatcgccccaaagtacttcccatactttttcgcgtggcgcattgatggtagctttaaacgttgttttttccataactattcatttacagggttcataatttgtttattgtatttgttccggtactccagcggggtaagtcctgttacctttttaaacatggtcctgaatgtttttgtatcgatatatcctacgtcgtagatgacttcgttgacgttttttgtactggtttcaaaatcgcgcttggctgcttctatctttatccgctgaatatattctatcaccgtgttaccggtcgattttttaaatcttctttcaaaagttcttctccctatagccgacatatcagacagctgttctaccgtgatcttgtcctggtaactggattcaataaattcctgtgctttacggataggttcgtcgttatgtgctttttgtccttcgaaaatgatgaaaggcgactggctctggcggtctatatcaatggcatatgccttggcggtaaggatcgcaatatccctgccggcgtacttctccacgaggtaaaggatgaggttgagataagaataggcgccgccgctggtataaatacgttcttcttccgtgatgatccggttgtccatcaggtttacatccgggtacatggttctgaactcccgggccattttccagtgggtagcacattgcttgcctttgaggagaccggtagcagcaaggaaaaaagcgcccaggcataaactggccacggatgcgccctgctcgtattgctgcctgatccagggaataaaatcctggttcatggctgctgcgcgcgactgatccccgtgcagggaaggaatgatgatcaggtctgttttctttacatcgtttatcagcacctccggagagatggtaaataaacggttacgctggcttacttcggctgttattccaaccagctgtacctggaacattggctcccggcctttttccgcaaggaagttattaatatccgttaaaatctggtagctgccttcgatgttaactaaactggtgtgcccgaggggaaccaggatggaaatatgtatcatacgctgcaattataatagtttatgccgcaattaccctgagaattgtcgctttacacccctgttacttcccgtaacccttacgatttttgcattatagttttcacacaaaaatccggttaaaaatgaccatgatccatacctaccttactttcaacggtaactgccgggaggcaatgactttctacaaagattgtctgggtggagagctgaagattcaaaccatcggagaatcgcctgtttcagcagaaatacccgcttttatgaagccgtttatattacattccagtcttaccaaaggcagcctggtactcactgcgtccgacatggtgcctgacgcgggacttacagccggcaataccgtttctttattattgaattgcaacagtgaagacgaagccagaactttttatgcccgtctttccacggatggtattcctacgcatccgctggaaagtactttctggggggctttattcggtgggcttactgataagtttggtcttcactggcttattaattttgaaggtaacagccggcaataattatttatttcccgttaaacgctttttccaacgctgcgatatccagcttcaccattttcatcattgcctgcatcgctctgccggatttttctttatcaggatcagtcaacaatttagtcataatggtaggcgtgatctgccaggataagccaaatttatctttcagccagccgcattgcacttcgcttccgccgtctgcggtaagcttcgaccagtagtaatctacttcttcctgggtttcgcaatataccgtaaaggaaacagcttctgtgaacggaaattgcggtccggcgttaatcgccaggaactcctgtccttccaggtgaaaggtagctgcgagcagtgtaccggcaggaattcccataccttcctggtaatatgacttatcggtcacttttgaatttttgaagatagatgagtagaagctgatcgcttcttctgcattcatattaaaccataatgatggggtgatcttttgcataacgatagattagaattttacagattttcatttcgttacaaagatacccgtcgtctttctcttattgaaggtgcaaaagcgacattctttgggggcacttgcgacaattgcgcgcggattttgtctttctcaggattacgctgattttactgattagctggatttttacttttggatttttttggatttttagatttaaaaaaattaagagagatgaaagcggattcgcttttatctcccttaactatattattaaacatattatcaggaaaatctaaaaaaatccaaaagtaaaaatccagctaatcagtaaaatcagcgtaatcctgagaaagacaacctccgcgctgtcagcacttctttgagtcccatcatgagcagggagccggcaccgaagagcagcatcacccagggagcattatggatgccctgcgaggtgatgatccagccgctgacggccgttcccagggtaacacccatgttgccgaaagagatagataagctggtggcaaaccccggggcttctggcgcagcggccaccatgtaggcttgcgctgtgataaagcagggtgtgtgcaggaaaccccatacaataacgagtggtactgcgaacagcggcagatagtaaatacctatggacaccagcgtgatggcaatgagagaggcagccattgtaccggttacacttttgcccagcagtttgccggccaggaagttgccgggcacgccggctgcgccaaacaggagcagcattacgcccacttcgccggtggacatatgatttacttttcccagatagtccgcaaaatagctgtaggtggaaaacatggccgataccataaacacgttcatgatactgctggccaggaaggcgggtttggtgagtattttcagctgcgcgccataagatggtttttctgtagccggcatcgatggcaaaaaggcaaggatggctatcagcgcaatcgcacttacaatggtttgcactacaaacgataactgccagctgttatagatccctgccagccaggtggcaaacgggatagtcgttaccgttgcaatggcaatcccgctcatcacgacggccatcattttatgcgtgtgctttttatcggccgcaccggtagccgcagcgatagccgtggaaatatataccggctgcaggaatgccggcaacatccgcaccaccagtaacagccagaagggaggtgataaggaggacaccacccctgttatgagaaaaatggaaatgctgacagccatcagtgttttacggttacatcctgataaccagagcgtcatcaggggtcctcctaatgcaataaccagcgcgaatgcgcttaacagcgttcctgcctggtcgatagaaatgttgtaatacgccgccagttgcgggagtatcccaataacaccaaattccgtggtgatgatgccgagtaaaccaagacttccgatatatgcgattcctttcatttgctttgctgttgaataatgccggactttttttgctggtacaaaagtgagtatgtaaatcatataaagaaaataatatgatttatcaatcgtcataaaaatatttataacttgcaggatggttaatctggagtggtacagaacatttaaagccgtatatcaaaccggctcgctgacagcggcgtcaaagatgctgtttatttcgcagccgaatgtaagtcagcatttatccgcgctggaagcgcatatcgggaaacagctatttgagcgcaaacccaaactggtgcctaccgattatggtaagctattttatacgcaggtagtggagccattggaaaagctggaaaatgtggaagcggatttccgttatttctgcatcaccaaacaattaccgaatatccacatcggcgccgtaaaagaatatttccaggcagtagtagccaaacgcatcagcgaggtgcaggcgaatattatcattgagtttggcctgaccaaagacctgctgcggcggctgcagaaaggcgatcttgatttcctcattgccacgcagctgatagaagaaaagaacatcatctatgaacccattctccgggaacagttcctgattgtatcccacccggatcttgacaccaaaccatttaaaaactccctgaaaaagaaatcactggatgaagcggagtcgtggctgctgaaacagccatggtttgcctatagcagcgacctgcccgtgatacggcgtttctggctggaaaacttccgcaagcgtcccgctatcaaaccacagtttattatcccggatatgcaaacgatcctgcaggcgatcagctgcggcaacgggcttactatcactgcggattacatggtaaaagaaggcattaaaaaaggagaactgaaagaagtatggcggggcaatgtacccgccagcaatacgctgtaccttgcctacgacaatacccggatggctaccgaccgggtaaaaattgtacgggatctgctgcagctttaaccgcttgctgaaagaaatagtttattttgtagtactgaacgatcatttactatttatgaagctaagattccacctaagcaccctttggcttattttaagcctgtttggcagcgccatgagccaggcgcagtccactcctccccggttccgggttatcgccttttatacggctaaaaacgaccaggcccacatcagctttgtacatgaagccaataagtggttcccggagatggccgcaaaataccagttcagctatgattccaccaacaactggcaaaacctgaacacggcgttcctctccaggtaccaggtagtgatcttcctggacacccgccctgaagacccggcgcaacgcgccgccttccggcagtatatggaacatggaggcggctggattggttttcactttgcggcgttcgcgctcaccccttcggatgtgcctcaaaactgggactggtaccacaacaccttcctgggttcgggttcctatggcagcaatacctggcgccctacctccgcggtgctgcgcgtggaagaccaccggcatccggccaccaaaaacctgccggatactttctccgccgcacccaatgaatggtaccgctggagcaatgatctgcgcaaaaacccggacatcaggatactgctgtcggtagattccagcagtttcccgctgggcacaggtccaaagcagcacgagatctggcacagcggctattatcccgtagtatggactaataaaaaatataagatgctatacctgaatatggggcataacgatatcgactatgaacatcataccaataaggaattatcttccacgtttgcgaatgaaacgcagaacaggctgatactggatgcactggaatggatggggaggaagcaataaaaggctacgcaccggaggtataccggtgcatagcttacggttatttagcctgtaaagtggcgatagtttgctgttgtgctgcaacctgtttatttaaacgttctacgtttttattcagctgaataatatacagggtgagttcttctaccttcttcagcaactgctgatcaaagtcgcccaggtccaatcctttttcaagtacttctttttcggaaggaataccttccaggtgtttttcggttgttacaaaatgctccacctgttgcagggatggcaactcatactccggatgaaatacataatctgcccaggcgccttgctgtaccttcacacggcgcgcgccgatcgtgccttctaccgtgagtttgtaattggctgacgggctggaacttccaatacacatgttgccggtgtttccgtcagctgccataaaatagttagcagcaccacttccgtcggagtgcatatttgaaaaatacaaatttgcaccggaagcgcccaggccaaatgaccttgtggcgccggcaaactcaatagcggaaccattatacaatttcattgatttcttccaggcattggtcgtccaggttgggcctccttccacatccagccgtgctgctgaagtagctgctcccacactgagatttccctgtattgcgatcgcatcagtcggtacaaacggcagcacatttgttacgttatcatcttttactaaaatgagcgactctccacttgcataacctgtaaatgaaaaacctaacatggcatagctattcgctatttcagtcgccagataggttttcccgttataaacaagcgttactaaccttgttatttcattgtagctgatcagcgtacctttattcatattattggctgttgcagtatttatgtcaaccgtccacctcctgtagtatgctacagttcctccccttataccggtaacccttcccatcacatgcatatctgccatcggagttccggtataaatctcgtgcagcaatatataattcaggccttgcgaatcttccgattgcccaacaataggccggttcacataatagttacggccgttatcagatacctgcaacttacttacaggattaagcgttcctatgcctacattgccggtagtaccaatcacattggtttgggcctttacacttgtaaaagcaaatacaaaaagtacagggagtaattttttcatgagattttatttttcagatataaattccgggcagacagaaaacagggcaaggctacgttgcaagtcagggatgctacaataactgaagggtaacgggttaaccattctgaacactttccgtccgggaacaaaggaaaggagaaagaacaaaagtattgctcacacctttgtgttaatctatgcaaaggttgtcttattcaggattaggttgattatactgattactttgattttattttttgtttggagatgggtatttaaaaagagatgacgtgaagacgggatagctcatgcttcacacataccttacacatgctttgcatttactttatacgtgcttttgacctgcttttgatgtggagatgacgtggacttgatcggtaatgtattgtttatcaatacgctatagtgggttttgaaatattctttagacgggattcatcagagaaacaaactggatatcaatgctttagccacattataaagataaacataatcaggcaaaaagacaacagctgcatttttttagatttaaaagatggggaagataaaagcggagacgcggattttgtctttctcgctgattacgctgattatactgatttatttgattttactatttggattttttaaaggatttggggagataaaagcggagacgcggattttgtcttggctcaggattacgctgattatactgattactttgattttactttttggattttataaggattttaaaggatttggggagataaaagcggatatattcgctaacatctccccaaatcctttaaaatcaaaaagtgatcaaatcagcgtaatcagtataatcagcgtaatcctgagaaagacaaaatccgcgcttaattcataaacgcctctatctttttcttctcgtccaatttcacaaactggccatatttatccaggtactcccgggctactgttttgaatccggccttatcctgtttattgagcagatagattgttcttgcccgcaggtatatttcctcgccgggtgcgccgtaaggctttacggcagcgtaaatggcggcccagtcggggttagcgccattatccggtacagcgggcgcaatcaggtcctggtaaataaggttcatcatttttacggccgattgcctggcgcccatagctttatcgatggcttccatgttatcgcggataatggagaagccggtgtcgcgggtgctgccggttacctgcattacataacgaaggtcttcttccgaatacggctgtttcatgaccgcgaaatagtcggctcctgccagggcggcgccatctttatcgccggcctgcacggccagcatagccagttttctcaaaaattccggatcttttttaccatcaatgtactcctgcaacatggcgctgtaaatagcggtgggttctgtgagatcggcgtcctgcgcggcgactgcgggaatggcgcccatgtctttattgaggggtgcatggatttttcttatttcggcaaacggaattttcactacttcacggtcgtaggtgagcagtccgttttgttctccttccacatcaaagggctgggtgtagatgctggcagataagccttgccgttccagtaattgcaggtgctggttcatgaccgcgtatttcgatttcagtgcgcccggcttttcctggatatatccccaggcggtattggtgttccactgatgatcagcgatgaatacaccgataccgccgaattcgcccaatacgcgggctttccccggcatttttatggcgttcatggggttgggataactgtgtacatcggtcagatcggcgccaatgtatgcatccggactcggactgcggagtttttcatttacatacaggtattcgccggagtggccgttgacgaggcgggaaggatcgctgcgtttgatccattccgttaaacgctgctgatcaaactgtccccatttttcgttgaacaatacccaggtagtaacgcagggatagttgtgcagttgagccagcgtttctttgcattgctgttcaaaggcggctttggcgccttccggaagactgtgattgggacttaccatatcctgccataccagcatgccgagtttatctgcccagtaataccagcggtccggttccactttgatatgtttacggatggtattaaagcccattgctttgatggctttgatatcaaatgccagcgcttcatcggtgggcgcagtgtataaaccatcgggccagaaaccctgatccagtgtgccgaggttgaagtaaggtttgttgttgaggaaaatgcggtccactcctttttcatcttttgcaatggatactttgcgcataccgaaataacttttcacttcatctttaacggtattgcctttcagcaatttcacggaaaggtcgtacaggaaagggttgccgggcgaccataacgtggggttttccagcctcagctgcagtggtgcgccgcttttgcctttcactttacctgcgggcttaccgttggcggaggcgatggcttctagggtgtatccggcaggtgcgcttacggtgaggttcagttgttgcttgtctatatccggcgtgaaatttaacccggagatataatctgtgggcactttttccagccatacggtttgccagatacccgagctgggggtataataaatattagcggggttgagtacctgcttgccggaagggcccacgcccctgtcggatggatcgtagatcttcagcaccaggatgttttcaccattctttacagcattggtgatatcgatggtaaacgacgtatagccgccggtgtgaccacccacttctttgccgttgagatatactttgctttgccagtcgaccgcaccaaaatgcagcaatgttctttcgccggcagcctggctgatatcaattttgcggcggtaccacagtcgttgttcgggaagcagtgttttctttacacccgacaaggccgattccagcggataaggcacgagtatttgtccttcgaagttatacggcgctgcttcatcagcgccggtgatagcatattcccagaggccattgaggttttgccagttgccccgttccagctgtggacgcggataagcggtgagtgcattttgcgggctcacttctttcgcccacctggattgaatagcaacgggcttcattttatacgtggtttgtgcctgtagcgggcaaaggccggataataacagcgcagcggctagtaatggtgttctcatcatggagttacttatttctttgtggttaaattgagtggttgacagggttgtgatcttcagttcatcttaatggctaaaacaggtacggcagcaaaatatacataattcccgatgaataaacggacttaacttttaaggtttgttaatctgtatattttgcattttcattaatattatattttacaataatgttatataatcatctctataattaaaaaaataaacaacatctctttattataattaacattttattcataaattatacaaaaacaatctcatcccatggcataattaaaatattactaaaatgaatactataaacctcaaccgctatgatcacatctccgatacctgggatgaaatgtacattgccgataatcacctccgggagcaataccaccggattatcagttacctggagaatgaatctgccaacgacctcaataaaaaagaagaactggcgaaacggctgtttatgagccaggggattacctttacggtatacgacagcggagaagggattgaaaagatctttccgtttgatatcatcccccgcatcatcacctgtgccgaatggacctttattgaaaaaggtattaaacaacgtctgaaggccctgaacctttttctgaaagatgtatataataaccagtttattatccgcgacggcgtgatccccgcctcgctgatctactcctgcccccatttcctgcgggaaatgcaccagctgaatgtaccttacgatatctacattcatattgcagggatagaccttatccgggattacgacggcaccttttacgtactggaagataacctccgcacgccttccggcgtaagttacatgctggaaaaccgtgaaatcaccaagcggcttttccccgatctcctgccccaatgcaaagtgcgcagcgtaacggaatacccgtctattctctataaaaacctgctgtcactctcgccgcgggctgtcgctaatcctaccatcgttttgctcagtccgggtatgtacaactccgcctactatgaacacaccacgctggcccgtctcatgggcgtggaactggtggaaggccgcgacctggtagtacgcgatcagaaagtatacatgaaaaccaccaccggtctgcaacaggtagatgtgatctaccggcgtgtggatgatgagttcatagatccgctggtgttcaaccctaaaagtgtgctcggcgtagccggcctcatgagcgcctaccgcaaaggcaatgtagccatcatcaacgccaccggcaacggtgtagccgatgataaagccgtgtacagctacgtaccggacatgatcaaatattacctgaatgaaacaccactgctgcaaaacgtacctacctacagtttgggtaacccggaacataaggaatacgtcttccagaacatgcacaaaatggtgatcaaaaaaaccaacggaagcggcggctacggcatgttaatggggcatgccgcctcggaatctgaaatagaaaattataaaaaagaaatactgaaagatccccgcaatttcatcgcacagcccactatcagcctgtctaccgccccttgttacctcgatggcatgctgcaaccacgccgggtggacctgagaccttatgccctcgttgggccagacggcatctctattgttcccggcggattaaccagggtagccctgaaagaaggctccctcgtagtaaacagctcacagggtggcggcagtaaagacacctgggtactggcatcataaactaaaacacaagcctatgttaagcagagtagcctccagtttatattggttgagcaggtatgtagaaagaagcgatggtattttaagaatgctgaaaataaactacgcatcttcacaggacaccatccaggaatttacctggacgccggtgatccgtatttcttccggcagaaatgaagctgaaatatcttctatcaaaaacgatagccggtcggtgatcgagtacctgctctttaaccgcgataatcccaattctattatcaacatgatcacgctggcccgtgaaaatgcccggagcgtgcaggaacatattgcgaaagacctctggcagtgcctcaatgaatactatcataccgtaaaagatccgaagctgctctggtatgtacaaaaagatgatcctgttaccgcgctggatatcctcattaagcaggtaatgctttattacggtactgcaggcagtatcatggaaagaggcgaaagcaggagctttatgagcattggtaaatacctggagagaagtatacagtccatcgatatcctggacatcaagtttatctctatctccaataatcccgacctgctcacggatacctcttactggcaacacctgcttttatcgctgggcggttatgagctttacctgaaaacctaccgtaaaggctttgaagcggaaaacgtgctggaactggtcatgctcaacaacgattttccccggtcagcaaaatattcggtcaacaatattcaccggtatttcgaacgactgaaaagtgataaaaatattgaacactataataaattgtcgtttaacatcgggcgactgaacagtaccatcacctacagctccgtaaacagtatgaaagcggaagggctgcatccctatcttgttaagatcaggagtgagctgtatggcatcgggaacctgctgaatgaatactatttcgcaaacgcttaaccatcgcattattatgcctgttttcagaataaaacatatcacgcattacacttatgaaacaccggtgcgggacagtgccaaccagatcattttgtatcctgtaaaagacgattaccagagagtgatcaaacatgatctgagtatctcccgtcacccggaagtggaaacgttcaaagattattatggcaatgaagtaggtattttcacccaaacggatccgcatcatgaattgaaaatattctcggccatcgttgtggaaaccattccgcggccactgcccaccgatgtgctccttcctgccacccaatggcagatgctcgaggatatccgctacgacgtagcatttattgattatctcaaacaggaattttttgaaagcgtggcctctttacggcaaatttcgctggacctgaaagaagacactgatacgccgttcaaaacagcggtgcgtttctgcgattatgtatacacgcatttcgattatatcaaaggagtgacaactgtggacagtacccttgatgagatcctgctgttacaggcaggcgtatgccaggattttgcgcacctgttaaccgcgatgctgcggttcactcaaattccggcgaggtatgtgagcgggtatatttgcccgaataaaaacggtatgcgcggcgagggcgccacccatgcctgggcagaagtgtatattcccgaatatggctggctggggctggatcccaccaacaactgcatcgcgggggagaaccatgtaaagctggcagtagggcgtaacttcagcgactgctcaccggtgaaaggcgtatacagcggcggagcaggccataccctggatgtgacggtatcagtaggttacgacgaccaggaccagtttgatcctgaaccatttttccctgcccagcccgccatgagcagtactgttgcggccgagcctgtaaaaaacagttaccagcgccacctggaagaaatgatgatacagcaacagcagcagcagcaacaatgaattccaggattacaccggctaatggcgggattccgtctgcggagcccgccggcgccggtttggtccgctaaaagccatctgttgatttatatcttaaaacaatttgataattcacaaataaagaaaaatttatatagttttgccttgaccctttatgggagaacgatcactacaactgtcacaacttaaaagagtacaatgcaaagcttagccataaaaggccgctgggatgctttttgtaataccatcagcaaaattccgccgaaatacctgtatgctttatttttattaatggcggtaggcatctcctttcattcctggtattcttcgcaggacatggaaagatggacccgttataataacttcctgatctttaaacacgcattcgcgcacctggtacacaaccaggacctgtacgtattatacgaatctcagtattacgatctgtataaatatagcccatcgtttgccctgtggatgggcgctttcgcctggatgccggacgtgcctgcgttgatttgctggaatattatgaatgtggtggtatttattatcgctatcagaacactaccggtaaagaaagaaaagcaatcgatcctgctgttatttttggctatagagatgatgattgcgctcaccagctcccagatcaacgtattcatcacaggctttttcatcctggcctggcatagcatggaaaataaaaagatctggctggcagcattgctgctggtagtaaccgtatacattaaattatttggcatagtggccatgtcgctgttcctgttatatcctgaccgctggaaagcagcgttatacacggtgttctggaccgttgtcattgcggtgatgcctttgctcgtgatttcctgggatcagctgctgtttctttacaaaagctggggacacctgctggccaacgattactccgcttcctacggcgtgtctgtgatgggatggtggcatacctggtttgatatggatatctccaaacagctgttcatgctttcagcagcggccgtattcatgttaccgttcatacccatcctttataaccgggaatcgaaatttaacctgagcatgctggcttctgtgctgatatgggtagtgatctttaaccacaagggggaatcccctacttatattattgcgctcaccggtgtagcgatctggtattttacgcaggagcggccttccacgttaaatacagtactggtggtgcttacgctggtattcacctccttctcttctaccgatctgatcacgccttactggattgccagaacttatgtagagccttacgccgtgaaagcggtattctgttcgatagtatggctgaaaatagtgctggaaccattttttgctacttccccggagccgggaacgattacagcagagaagctgcagcgcgcagcataaagataaaacgaaagggaaggctggatggccttcctttttttatgcgttttgttttcttacgtatttggtgaggatcacgatgagttgtccttctatctttccttctatttgttctgtattatccggtacgagacggatattctttaccaccgtacccatttttgcatttagggtagaacctttcacatcgagggacctggtaagaataacggtgtcgccattttgcaggatggcgccattgctatccctgtgcaaatccaccgcaccatcgttttcatgatcgccggtagctttcgcccaggcgagcgcttcatcgttcaggtaaatcatttccaggttatctgccgcccagctttcctgttttaaccggttcaacatgcgccaggataccgtctgcacacccggaatttcgctccacattgattcggttaagcaatgccagtgggtactatccagctctgctcttttctcaatctgcgactgacatttctcacagatgaagatacaattatcctgatcactgtaggtctgaggaggcacttcatatacattcagcggttcttctgatttgcatagttcgcacttgttttcactccttgttagtaatagttcgttcagcttcataatatcctttataaaaaaatgtgcacgaaggtaacgttttttgtcccgggaaatgcccattttcttatttgcctggagtgatttaacatacccggctaaaaatgtttacggataaaagcggctgtttcatttattgccatttttccttcttctatcataccacccatttgaaagaagccatggatcatacctttatacagggtttcctgaaccggtaccccgcttttgcgaagcgctgcagcataggctattccttcatctcgcaagggatcatattctgctgtaataaccagtgcaggcggctgtcctgtgagatgctgcgccagcaggggcgcagcatccgggtgttgccggttttgcggattgggaatatataatgaccacgccagctccgctcccgccagatcaaggttcaatccttctgcaaactctttccatgatggcgtttgcagggaagcatcggtaaccgggtaaatcagcgcctggaaccgtaacgcggggccgccatgctcccttgcatgacgggcaattacagcagcgagtgcagccccggcactatcaccggctacgcctatacgatttccatccaccgctaattcccctgcatgatctgcgatccactgcaccacggcagtgccttctttcagtccccggggaaaaggatgttccggcgccagggcatagtccaccgataccaccacacaatctgctgcattggttaatgcacgcaggggcgtatcgtgtgtatccaggctgcccatataaaaccatccgccatgaaaataaacagttaccggcaggccggccttatccgatggcctgtaaatgcgtacgtttacagggccttcagtagtatgcagtgtgcagttttgcaccacttttacagctgcgggtgtgccggccattggtataaaccggtggtaaaaatcgcgggcagccgtaacgggatctgtttgtgcaggagcagcggggatatgattgatatagtctaatgccgcttgtacggtgggtttaaatgccaggtctgtgatcatgtgatgtacttatttgttttatgatcacaaaactggcattcctgtagctataaagaaaataatatagtttattgttacctataagaatatttatacagcaattatggcactacagtaataaataaataagtagccagtatcaccaataacacaattccctgcaggatattggttttccctgcattaaaagaaatgctgatggtaaaaagtgagaggatgagcagcagtgtggatttggcatcaataccgagcgtaattttgaagccaagcgtataagagacgatggctacagccgggatggtgagaccaatactagcgagtgcggagcccagcgccaggttcaaacttgtttgcaaccggttttgtgaagccgccctgatagctgccagtccctccggcagcaggataaccgctgcaatgataacgcctaccagggttttgggcgcacccaggttcaccacaatggtttcaataacaggcgataacttcttcgacagcaacaccactactgccagcgctattaataaaaataccaggctcacggtggtggtgagtccggaaggcggagcagcatgtatatcttcatcacccggcggcgcatctttaggcaggaaatagtcgcggtgacggacggtttgcacggccacaaaaccgccatacaacaccaaagaaatgatagccacaaatatcagctggctgtttgaataaacaggccccgcttcggtagtcgtataatttggtaagacgagggttaaaacggagatcgccgttaacgcgaccaatgcggcactgacaccagcttttataaacgcctgctccttgaaacgatagcctcctataaacaacgacatgccgatgataccggaaaggatcagcataatggcggcgaacacggtatctcttgcgagcgttgagccctggtccgctttattcaacatgatggatacgatcagtgatacttctatcactgtaattgccagtgccaggataagcgtaccataaggctctcctaccttatgcgctactacttccgcatgatgcacggcagataataccacagcgataagggatagtcccatcaccgccgataaaacgccattttgctctcctgcgaatcctaataataccaatccgattagaggactgataagacaccataacgggagcgtaattttccatttcctgtagagaaagtgattgaatgccatttgtttaatttacaaaactttaggcacatggccgcattcagcaacggagagaatttgcaggcaaatgatttatgctcctaagaatatcctatcttcctaaagtttagtaaaaacagtgaacatgttgaaacgtagaaatttcatcaaaaacttaggcctgtccggaaccggattgctactggcctcccgcacattatccatgcccgttagtgcacctgcagccgggaataaactgctccgcttcggcgttatttctgatctgcaccacctgcagttcgggaaatcggaagagccacggttgaaatcctttatggatgcggtaatgaaagctgatccggattttatcatacaatgcggggatttctgccgtccggcaaagtcagagggtatcatgactgaatggaaccggttcagggggcccaaatatcatgtgctgggcaatcatgatatggatgtatgcgacaaagccacgatcatgaaattatggagcatggaaaagccttattactcatttgaccagggcggttatcattttgtggtgatggaccggaattttttgctgaaagaagataaaacactggaagattacaataacggtaactggggacctctcccttctccgctgcggagtttcaccgatgcgccgcaactggcgtggctgaaacaggacctggcagcggcggaatatcctgttattgtttttatgcatcaaccggttttcctgagcgactttttccaggaactcggaaatgcagatgaaatcctggccatttttgatgaagcgaacctcgcagcaaaacaacagggtaaaaactcccgggtaacagctgtgtttatgggtcatgaccacgacgaccggtatggggaaagaaatggcgtacattatatcctgctgaacagtgctacgtatgtgtacaccgaatcaggcgcccatttttacgccgactcactctatgcttttgtaacccttgatccgtcgggatggatgcgtattgaaggccggactacccattaccgcgatgaggtgcccgaaaaaataaaagcgcagtttcccaccagtatcagcgatcacgctatccggttattttcacggaaagagaagccgtgacaacagggcgcattttaaaccggcccggaaacgttttcagccatcagccggtaggcagcaggctgtacaccacctcatacagttcgttaatgcggaaaggtttcgctaacaaactgtcggccttacattggctgatggattcttcaggataattcctggcggagaaaaggataaccggcaactttgcttcgtcaggcgaggatttaatatcccggcataaattccgcccgtcataattacccatggcaatatccatcagcagcaggtcaggagcgaactgcgagatactctgatgaagctttgcagggtcttccagggtcatcacgtccatgttttttctggaaaggacgagggatactgcttcaaggatatcaggattgtcatctacaaccagaatcttccaaatgtggattgttttattttcatgaacattcacatcgggaacgcgttggccatgcctcccacagatcaggctgtaaaggtaaaactgtttttcatttgaaatattggcacagcacgcttttttcccagccttactttgaatggcttcctctactccctgtaataatctttcaggctgccatttggggtgaagctgatgaaataccgctcccggctgccattgatggactggggataccagctgatgctgtttccattaaaaatgccgtaaatatgttcaaggggttttgcgccggcgatatctgctgctttacggtgatagttcctgtatacagcagcaacgctggcaaaactgatctcatcgagaccaaccagtgatttgctgatatcatcgcgcacagacatctgcaccggtttgggttcctcccatttgccatcgttatagttgtattcgtcaatataggcggcgttctgcggatgctgaaccgttacatttattcgtccgtcgttataaaaatgaatggatctgtagagatggatacttttgcctgcaaaggccggcaattcgcgcagcgcgtgttcggcagcattcaactttacggcattactaagaaaatcatggtcgccggatgttgtagtggagttatgtataatcgtggtgccattgcgatgttccacaacagtagtattggtgctggtactcgtactcaggtgggtactggtgctggaacttgtggtggtggtggtttcgtcctgggtagccggaagatctttgtagctgctgtcggtatcactgccatacagggtatcatgtatggattcccggaactggttacaggacatacacatcaccactactactataatgccggtcatcttttgtaaacgcatcttcataattttaatcagctatatcactggcaaatattacctgttgaggattttctttcagataaaaaaccgggacagactcctgcctggtcatgcccagatccaggagcggcactattttttttaacgaagcagtatgggtttttcctgcatcatcctggtagcgcaactcaaagcgtacctgcggctgttcattaatataagtgcctgtttgctcggcagaaactatctgtgcatctgtacgcaagccgtagtacttaagctgcaacgcattgcctggcgtgcctgtaaaaagtttcaacagccagcccaacccgatcccgctcaccagcataatcaatggacataaaataagcggatgatagaaagctataaagcgccagccccgtccgtggttctctaacatataggaatatacgtagtagccggctattgcggcaacaaccagtaaccaggcaaggcacatcatgatgatccggcctgcttttattcccaccgttacgccgtccagggttaaatgcggcactgctttaagtttatcatcaatcaccagcggaacggttttacccacctcataacggtgcagctccggcttggtatcgtttacctgtaactgttcggtgatttccgtgccgcagaaattttcaagagcgcaggtgatctcccgggtaacaacatccttaccttcagcgggtagttccttgctggttaacacacgtgcattctttctcacgccttcttttaaaagacgcaggatatttttcctcatgataaaaggcaatacaatccattttctgaaccagcgctggatcaatatcccccacagtattacagacagcgtcaaccaggtaagcgccagccatggctgcgtgccgccatccccatcacttacgccatacccggtattataatagatgagcatgggaaaagggatcgcaaagaaaagcatgtaaatgaaccagaagtaactccaaaaacctttcattcagctaatttatttattaaatttaagggaaagatgcttaccatctgtaaaagacattacggggttcagtcttttttgtagatcaccttattttcacattcaccgagaatcacgcggccatagatcaccttcgtccagccgttttcaaaaccgtgattattagctatgaggtaacctttattggtatcttttttaatcaccttgtgtgcatcgatgtagcggccttttactttgcaaaacacaatatcgccaatgacgtattccgcttgctttacaaaagtgagcagggtgccgcttttcaaaatgggtaacatagaggagccaaaggctttcatttttcctgtgccggtagtttccaatccggactttaatctttcgtacttgttcatgttgttttaattgattgaataaaaatggatgaccatatagtaaatgatcgtagtgcaggcgcatggagttactgaagccaatatgcgggaacggttaactgaaacgggcaaattcaattataagcatgatggtgaaacactgttgggctacacaagatgggcgggtataacaaatggtatgctgtgaaataacaaaacctgcgggcagcgcaggtatcaaactatttggggatactgccggggcattttctataaagaacaactgccgcaaaagtaataaaattttctattctcccggataaaaaaaacgtgatactgaatttgtatcacgttttttttatgcttttttattttgcaggggtaatgacgatgttcctgaattcaataggaccgtgatctccctggaaatagatcgggccgggttcaccttcattgctatccaatgcaccgccggtaataccgggaatggcggcattgcatatgatagttttgccattggcaacaaccgttaccaggcgacctaccagggtaatatcaaaagtttgccattgaccggggccaagcaccaccatgtcgtttggcaccaggaatccgtataccccaccaaacaggtgactggatggcggatctgttttaggattgtcgatgatctgtgtttcataacggcccctcaggtaaacgccgctattgctacctgcctggtagcggaattccacatgcagcttaaagtcggtgaacttctgttcagagatcaggttagcgccggaatgcgggctggcaaggataccgtccttaacgatccattggttctgacccagggctttccagccggtgaggtcctttccgttaaacagttttactggtttatcccaggttggtgctgccgttcttttaagatccggcgcttttaccccggtgaaagcataggactgtccgtcgctggtatggattgtaccgcttatcccggcatcggttaccgtgccttccagcgtcaggtcgcggtcttccttttcccattgcggcgggatggagaagctgaacctgccgttgtcaaaattcactttggagataggcctggcgctgccgccggtgcttacaaagcgacctaccagggttttaaaaccggaaagctccacttccagccaggagggcttatctactccattttcgctgaccttgatatcccaggcgccaatcagggccccgcctttaacggcttcggtcttaatagccgatacctgtgccattacaccggaaggattagctaatcccagccccatgcagcatatcagacctgcgataatactttttctattcatgttcatgtccatgtttattgaagaaagctataaagataaatatttgatcctgcttcttatagcactttatcgggtttatttaaaccagctcccaaatctataattatcgtgatatttaccggtatcccctcctgtaacatttattccagggcctgcgttaaacatcaaagctcttccccatgcatatttctacctatattaaattcccggttattctcgcggttatcctggtactgggcggatgcacaaaggacaagtgcaccaaaatgatccaaactaaaataaatattcccgttatgatggcactgaccgactattgggcctccatcaaatcggaagcgccaaaggagatcatccttacgggcaaaatctatgtgaaagaccagtatatttttgtgaacgagccctacgccggcatccacattatagataacagtaacccgtcatctcctcagaaagtttcttttatcaatgtaatggggaatatcgatatcgctataaaaggcgacttcctttatgccgacagctatgctgacctgattgtattcaacatcagcgatccgcgcaacatcaggtttgttaaacgtgtgccggaagccaccagtttgccggccaacgtaaacggcctgctggtaggatggcgctataaccgtgacagcatcgtgattggttataccaccagggataccagttattgcgattgcgatccggatcctaacatacaatatcttgccagcgcagaagtggcctcctcttataaaaaacaggccggcaccggcaaaggtggatccatggcccggtttaccatcgctaaagattacctttatactgttaattcctggcagttaaaaacatttgatctctcggatgccgctaacccggtgtttaaaagcctgcaaacctttaatgcctttattgaaaccatattcccttatggtgaatatctttttatcggcagccagaacgccatgttcatttatgacatcactaatccggcagtaccaaccaaacgctctatggtaacacatttcagggcatgcgacccggttgtagtggaaggaaacagagcatatgtaaccatcaggagcggtgcagcctgcgcaggcaatttcaatcagctgcaggtatttgatgtgagcaatgtggatcaacccataaagttgagcactaccgaaatgatcaacccacacggtttaggtattgacaacgggaagcttttcatttgtgagggccagtacggacttcgcttcatggatgccacaaatgctactaacatcaccactgcaaagctggtaacagggccggagacatacgatgtaattccctttgaaggccagcaccgcctgctggtgagcgccagggacggcatttatcaatacaactacagctccatcacaaacccgcagctgttaagcaaaataaacgtaaagggtaatccatattaacaggggctttcctgttaataactattaaaaacagccagtttatacatattatcatccgctggtgtggcaatatacaaccagctttccaatgctacgcgggaagtacaggggccgtaggtaatgagcctgatctttctctttaccgattctttttgcaggatcgataaaacttcctgcaggatttcgcctttgaagggcgtaaacataaaaaataccgttccttcagaatagtcggcttcccgcgcatccacatttataaatgtaacagccggcagatggagtgccgcagcgcaggcccctgcataatcgcagaaggccggctcaaattcaattcccctggtggcgatgccggtgagcagatttacgaggatagccacctgtcccaggccggcgccgatatcgaaaaagacatcttcttttatgaaaggaactttttctaccagttcaaacacgatcctcgctggtgttttctgataataaaccatttcaggttcaagatccctggtctgctccggcattgtttgcagcggggataatccattgataaaaatatcgaggttatcataccccgcttcttccccatgcccattatcatccgggttaatatgcacgtatttattcaccaggtgtttaaacccattcgttgtaaataaggttgtactgatcgttcgctgaagttgctgaaacaggttaacatcaattccttccagcctggactttactttctcagcgcggttcctgagtaccagcaatggatccggttggggcgtgttcaacaggagttcgttaatccgctcaatcacctggaagtcgatgaagtcaatgacctccatacgcagatcaaattcccgctcctggtagagcaccggatttctctctgcttcctcaatatactgttgtagctcaaaaatggtcatctttacaggatcgctgttatacttaaagaggaattactttcctatcacctgttttctatgttccactccccagttaaacaatgagtccagcactttttcgatagatgttccatgctgggtgatggaatattcaaccgtaggcggaaaagtattgtgcacttctctttttatcagtttattcgcttccagcgtttttaattccttcgacagcgttttatctgtaataccgcccacttcctttgatatttgtttaaagcgcttgtttcctgtggacagagaaagcataataagcagcttccatttgccttccagggcatccagggcgtcttttatagcaagtacattatgggggcaaccttcccgtgtcagcatttttttcttttatttctaacgatgttttcccgttactttcccgatggatagcgctatccgatggtatagtactatcagctgtatagcaaatgtagatacttttgctgcataattattaacagccttaaaaaataacgatgacagtcaaaacgaagcgtatcctatctacagtactgatggtcattcctgccatagtacttgttatgggcggagtaatgaaattacttggagcggaacctgcatcagtaatgcaattcctcattaaatcgggatttggcaattatataaaagcacttggcatcacagaactaatcattgcagcgctgctgctttacccggtaacaaataaaaccgggttcctgttagccactagttatttcggcggcgccctgtgcctggaaatatccggtgcacagccctttgcttccgctgtgttcctggttatactctggattgccatgttcttaaggtccagggaaatgtttctgccgttatctatggtgaatagccaataacgcaacagggaacgatccggaaaatgaaagcactatgtcttcagtacaaaaataatggatacagggctttggctttgaggatgcaatggttcttctatattccggattgttaaccctgcttcgctgaacagcgacgcccatgcgcccaatgttctgaaataccattcatagggttgctggaaatctcttttcaaacctttccaactcccttccttccaaccggaaacataaggttcctgctgcgcaattgcggatggatgcaatgtttgaatgaacaccaggccgccgggcacaatgagtttattgatatttttcaacagtgcatccgaatctgttttatccagcagcgcaaaattaatgaccgctgctccgggcttgttccctattgtatatttaccggtggccaggtcattgaaactggctactgcataatgatctccgcccttttcaatggcattttctatcaatgcgcttacagcatccacaccaaaggccgttattcctttgctttgcaaacaacgggtgagccatccttcgccgcagccgatatctattattgattgaatattgtgggaacaaatggtgtttacaatggcatcattagtcgccagtattctcgattcaatttcagcattatcaatagacgcaatccagttgtcggcattggcatgccaggaggtagttatttttgttgactgatccatgatttaattttgatgatgtgataattacttaagcgctctctgcgcgggaggatttatttctataaaaaccttatactaacaaattacgaaatataacgtttcagtccactttgcgggctgaattgcatccatagcaagaacatacttacccattttgtgtatgggctcacacagctgccgttttacctgcatgaccccgtaaacccaatgatagtctgatacatagaagaacctgctccgttgaaaaccgcttctggtatgctaattgcatttttggattttaaatctttattgaataaccaaaaaaacagtttatgaaatcgattcttagcgtcattggtgtgttattgttatcggccatcctttttgcttcttgcagcaaggacaccgatcctgcagacactgatatctttgctggtacattcaggggaaagatcgggtatgttgactcggaaaaaaacatcagccaggacaatggcagcgttttcgttacaaaggttggtacccggtatgacttcagattttccgacggcattcctgaccttaccggcgttcagtttgagcggaaggacgataacacaatggtaagtatgggatcatcaggtaccggtcttattacgatcaataaggacaagctcgtgataggctttgcaagggacggccggtcctggacagctgactgcggcagatagtatgatgtaaataaccctgcaacgttacacgctataagcgacctacatctgtccgggcttaactttttctattttctgtagttaatttaaaaatgatttattacaaggtgcacaaagaagtgccttaaggtcccgggaccgggggatgcagcaatgtgtccgccggttccgggattctgctgattttgatcattattttgtatatattcgtcgtaatctagaatacaaaatactttatgagaagatacgctttaatcattcttttgctcgcttcattttccgggtatgcccagagcacaattaataattacaaatacgtggtgataccggaaaggttcaatttctcccgggaagataaccagtatgggctaaacaccgtagctaaatcgttgctggaagaaaaaggatttaccgtttatttcgacaattcagaaataccaaaagaactggccggtaacaggtgcaatgccctgaatgcggatgtggtgcagaaaaaaggactgtttgtcaccaaccttacacttttattaaaagactgcaaaggcaatgtcatttttaaaagtaaagaaggcaaaagccgggaaaaagaatttgctgcttcctataatcttgctttaagagatgcctttacgtccctgaatgacgtaccatatgcgtatgacggcaccaccgctgaagcgcctcagcaggccgttgcgcctaccgttactcctgccccggtttctgcgcctgccaacacacctgcacctgcggtagcagaaactaaagaagctgctggtactttatatgcacaacctacagcaaacgggttccagttaattgacacctctccgaaaaaagtgctgacgctgtttaaaacctccgtgcaggattattttattgccgatagtgatgcatctcatggaatagtgctgaagaaaaacggagactggtattttgagtactataaagataataagctcatttctgaaaagctgctgattaagttttaacgcggtagttgcttgattttgaaaaagccttcaggtttaacaacctgaaggctttttctttgcatagggagatatctctctaaaaataccttaatcaaaaaatgcctaccttatccactgcaggtaaatagccaccggcatcatggccagtataaacggtacaataacggcaaatgcaataccggagtaattgatgagcgcattatatttcacataatttaaccccagcgattgaaaagcgcttttaaatccgtgcagcaggtgccagaaaagcgaaaagcagccaacaagatatatgatcacttctaccggatgctgaaatttctccagcatcatttcatacaggggcagctcctctccgtgtaaaaactggttggtccggttcggaatccagaaattggaagtatgcaccaccaggaacaatagaatgatcgttcccagcaacgccatgctcctgctataccaggtactgttggcgccgggcttgtttaccaggtatttcaccgggcgggcatcccggttggttttccataaccacaagccctgtacaatgtgcgcaataaaagcaagcaccaatacaatctcaatcgtccggataaccacgttggtggccataaaatgcgcccagatggtaaatgttttgcccccgtcgttataaaagatggccgcattaaccaaacaatgtaccaccagaaaactgattaaaaacaggcccgttgttgccacaaggaatttttttccgatagaacttgagaaaaatcttataaaccaattcatgataaagaatatttttgactgccaaaacagttacagcaggatattattctgaggatacaatttaggaggaagatctttttcttccaacaattcgcgcaattctatttcaatgtcgcggcatattttggtcagcggtacatcgttcgcgctgccttcaaaaggattctcggtactttcacctatttgctccagcgacgtatacatccaggaaatcatgatgctgaacggaaccaccaaccataccatgtgtcctttcatcactccatccactaactcattgaactgatcaaaatccttcagcaatccaaacggcagcagcaggcaaaatagcctgataaaaaaacggttaacgatggcgtattgccgcggatacggactgtttttcaactgctcgcttttagcctggctgatataaaactctttcagccccttttccatttcgagaaactgcgcaatctgcatctgctgctcatcatagcatattcgcagcagcttgccctggttcgacaaaatacgggcagtaatactactggcagccaacacctcctgcagttcttcgttggaaatatattttcccagttcggcttccaatggtgtttccctttctgccacgcgaaaaagtcgctggtactctgtattgtgctttttatcgaccgtttcccaggggcgtgatgaccgcatctcataccgcaatgccgttaaccaggccatatggcggtagatcagttcctttgtggtagccgggctactgaaaaaatccctgctgaatagtccccacgatctgctgaagcttactatagaggtccaaacctgttgtgcttcatttgtgcggttataggtctgcgtatttttgaaacccaccgtaaaagctgtggcagtacctaacaatgccactaccgtccagggaatactgatccattccaggccgcatgtttcgtacagtaccacgggcacaatgctcaaaaccagcaaaacatataccttccttcgtgtccagaagagaaattccccgaatttgtatgatttacctacatgcatatttccgactttcagtttttatattgttcaataaccatcccgtcactgttccccggggccagcgttgaactaaaggtaacaggcgcacattattaggcttccggtgcggatggtacatcctccatgcggatggcgtcgtccaggaattccccgccttctgcggtattctcattgtgatagggcaatatcacctcgggctccttcggttctgtacggccatcaggagtgggtgttgtaccagggtgcagcagatgtgagaagatgttcatgttattatcattttaaaagatgaaaacaggacgggttgcccgtcatgccgaaaacgcttcagcagaggcaatcgatgggccaggcatataattcattaaaaatcagataattaccttctaaccggcaaaagaaatcacacgatatttcgtcatttcacttgcgtacacacgaaatacagtgaatcatcggtggtcgcttgcccccgctttccccacaaaactatttgtacacgtcacatttaatgttatctttgcaactaagataattagttaataagatataaaatgaataccgaggtaatcaaaagaataagaaaattgaaccagcaacattcatacacctctattcagatgcatgaagcagttgcccggaaggccggcctttccggaactgatcataaatatttagggttcttactggagagagggcaaatgactgccggcgaactttccaacatcaccggtttaaccacaggtgcagttaccggcctgatagaccggtttgaaaagaaaaaactggtaaaaagacgatttgcggaagatgaccggcgtaaggtgatcattgagcccatcacccctaatataatggcattgctggcgccactttataaagaattccggagcaagtcagaaatgctgattgcttccttttctgaaaaagaaatcaaagtgattgaagcctactttttaaaggcaattgaaataatgaatgaaacaaccgataagctcaataaaaaataattgaatatgggagttagcatactggattttcacgaaatcgataaaataaaactagcaatggcaggcggcaaaggcgccaacctgggagaactatcccggatggaggggatacaggtacccggtggcttttgcgttaccacggatgtatataaaaaagttacagcgaataatgaaacgtttaattcactgctggaccagctgtccgtgttaaaagcggataacaggaaagctatcagtgataccgctgcaaaaatccggaaggtaattgaagcaatagtcattccggacgatattcaacaggagatcacccgccatcttaaaaaactgggtgaaggacacgcatatgcggtacgctccagcgccactgcagaggatcttcctaccgcttccttcgccggtcagcaggatacctatctgaacatcaccggcaaagaagctattctggcgcatatcagcaagtgctgggcatcgttgttcaccgacagggcagtcacctaccgtttgcaaaatggatttgatcatagaaaagtgtatttgtctgttgtgattcagcaaatgatttttccagatgccgcagggattatgtttacagcagacccggttacttccaacagaaaggtagtgtctattgacgccagcttcggattgggggaagcactcgtttccgggattgtaaatgctgataattataaagtccgggagggcaggattattgaccggaaaatttcttcaaaaaaactggcagttcttgcctcagcggaaggcggcaccaaacagcaggagatcgggccggaacaacaaagtgcgccaacacttaccaataaagagatcagaacgcttgaacggattggaagaaaaattgaagcctatttcggtagtccccaggatattgaatggtgcctgcataaaggtaagttctatattgtacagagccggcccatcactactttataccccatccctgaagcaaacgactccgaaaatcacgtttatatatccgtggggcatcagcaaatgatgaccgacgccatgaaacccttgggattatctttcttcctgttaacaacaggtggcgccatgcacaaagccggcggcagattatttgctgacatagccgccgccctggcatctcccgccagcagaaaaaagatcatatcggtcgtgggacaatcccatccgctcataaaagacgcgctcatgaccatcgtaaagcgaaagggttttattaaatcgttgccggacgataaaaaagcagcggatcagcgtagccgcaataaagtaatgtcgtggacctttccgcccgaattcgaaaacaacccggccattgctgctgatttaatcaaagccagccaggcatccatagaagcgttaaaacagcaaatacaaactaagtcgggcccagacctgtttgattttattccggaagatatccaggaattaaagaaagtatcatttaaccccaaaagtttggatataatcatgatggcgatgcatgccgccacctggattaaccaaaacatgatgaagtggctgggtgaaaaaaatgtggctgatacgctttcactgtctgtatccaacaatattacggcagaaatggggctggaactattggatgtggcagatgtgatccgtccctacccggaagtagtggcgtatttacagcaggcgaaagatgataacttcctggaagggctggtgaagctgaagggcggacaggaagcccgggacgctattaatgcttatctcaacaaatacggcatgcggtgcgcgggggaaattgatattaccaaaacccgttggagtgaaaaacccattatccttgttccgatgatcctcagccatgtcaggaactttgagccgggtgccagtcgtttgaagtttgagcagggacaacaggccgcgctgaaaaaggaacaggaattattagaccggctgaagcaattaccgggaggcaaacgaaaagctgctgaagcaaaacaaatgatcagcctgatccggaactttgccgggtaccgtgaatatccgaaatacggtgtgattaaccgttacttcgtgtataggcaggcgttactgaaagaagcggcacaactggtacgagccaacgttattcatgagaaagaggatatctactatcttttttttgaagaattacgcgaagtggtacgcactaataaactggattacgaggtcatcaacaaacggaaagacgaatacaaattatatgataagctaactcccccacccgttatcacctccgatggtgagatcgttacaggtgagtacaagcacgaaaacatgccggccggggctattccgggcctggctgtctcttccggggttatagaagggcgggcacgcgttatcctgaacatggaagacgcagatatagaagagggtgacatattaatcaccacctttacagatcccagctggacgcccttgtttgtatccataaaaggcctggtcaccgaagtgggcggactgatgacccacggtgcagttattgcccgggaatatgggttaccggccgttgttggcgtagacaaagccaccaggctgatcaaagacggacaaagaatccgggtgaacggaacagacggatatatagaagtattttgagaggagggtaaaaagacctgcaggttacgcaggtctttttactataacaacttatagtgcacctggacggtgttattattcaatttctttacatccagtaactccaggcggttttcaaactccaggccgctgacaagaggtaatccgctcccaaataacacgggttctaccaccaggattatttcattcaccaatcctgctttcataaatgcgcttactgtttgcgtaccaccaatgatcactgcttcagtatgtcctttagcagcgagctgcgctacaatcttttccgggccgtcgctggtaaacaacacattggattgagccggtgtggcgctggtatcgtgcgttaacaccaccagcgaaccttctttaatcggcaggtaatttggcgccaggatgttgtaggtggtttttcccatgatcaccgcctgtgtacgttgacatatcgccataaacccctccccgtactccggcgataaccaatcaggtacatttcttttattactgatcattccattcgcagaagcagcgagataaataatgattttcatttcctaagctttattgtaatgaactaaaatattacatcacaaaaatacgctgatcagatgagtcacgcctcccctgcaaacgacaatttaagggggcatttgcgacagattagtaatctccaaaatgccggcatcagagcacctgatgaagccggatttttcaattatcaattatctttggtattcattcaagcgctgtttttgatcaataaatattagcaatatgagcaggcaaatttttaacaggtcagttaaagttgatgggattgatattttctaccgggaagccggagacaaaaaacacccctccatattactgttgcacggattcccaagctcatctgtgatgtttaaaaacctgatggtagccttatcagacaggtttcacctagttgccccggactacccgggatttggctttagtggttttccggacaaagatctttttgaatattccttcagtaatatatcagcgtatatcaataaattgacggatgaaataaacctgaagtcgttcactatctacctccacgactatggttgtccgatcggactgcggctatgcgtcaaccatcctgaaaagatagcgcggataatagtacagaacggcaacgcttatgatgaaggtatcggtccgcaatgggatgaaacgattgactattggcaaaaccctacccctgagaagaaagcgaaagtttcagcgttcttaagtgaggaaggtgtaaagatgcaatataccgcaggactgccggaggaattgttacccagggttagtcctgagttgtggcagctcgattgggactgtatgaagcggcctggtaatattgatatgcagtttgatctgaactgtgattttgagaataacattaaaatgttcccggttttccaggaatatttccgcactcaccagcctcctgctttgattatatggggaaagtatgatgctttttttagtgtaaaggaagcccattgctacaagagggacttacccggcgcccaggttcatattgttgatggcggccatatggcgctggaaacaaattttgatgaagtgttaaaactgatcattaaattcctggggtaaaatagaaaaaatatgtggtcacacctttactggtattacgagatacgaggtaacgaaacttatagccagcaactattaaccaacgatgttctcagcgttttggaaaataccgggaagttaaaagccaaggggaaccaggaattctgtaacatggaaggtcttccgtggatcaacgttactgctatcaattcgcggaatggcagttatggcagggccgaagatttcaacagcgaatgggttaatttaatcgccatcatcggatcaagatctacacctgaaaatgaaactttttacatcagtttattaactgacattgccgaaaaaataaactgggaattaatactggaggaagacgacaacgataatgaaaacgttgttttaaggaaaaagacaccatagctgtcaattatatgagggccttattaataacgcataaaattgtatatccctctatacccgatgaggataatccaataaaaagacaaagaaaaaaatccatcactcccctccccacagataaggtttaaaaaagtgtcaacccgacattttatttactcttataatcaattatattttttattttagtgtctatctacaactgacatactgttgtcacaacccgtttataactttgtttcaacaaacatccaatacatgaaacaaactattcttgtactggccatcgcaatgatagccctgacttcccacgcacaatccaaaaaaagcaacaatatgtttactgtaaagcccttcaaaatcgatgtacaacaaactgtactggacgatctccaaacccgcctccgccaaacccgttggcccgatgcgcctgaaaacattggctggaaatacggcactgaccccgaatttctcaaaagcctcgtcgcctactggcaaaacgggtacgactggcgcaagcaggaagccgcacttaacaaatttccacagtttacagtggaaatagatggtgtctccattcatttcctgcacatcaagagtaaaaaccccaatgcccggcccctgctgctcatacacggatggcctgattgtttctatcgcttttacaaagccattccgctgttaacggatgattacgatgtgatagtgccttccattcccggtttcggcttctcgggccatgtatccatgaccgacgacggttctgcaaaaattttcgccacactgatgaaagacgtgctcggctacaacagtttcctggtggccggcggagacgtaggcagcggcatcgccaaatccatcgccaatctttatcctgaaaacgtaccagccatccacctctcggacgtagggtatcctaacggctcggaagactggagtactatgtccaaagccgaacaggaatttggacagttcatacagcaatggtggtaccgggaaggggcatattccatgcttcacgccacgaagccgcaaacgcaggcgttcggtctgaatgattcccctgcaggcctggcttcctggatcgttgaaaagtttaatacctggggttcaccaggtggcactattgaagaacatttcacaaaggacgagctgctcaccaatatcatgatctattgggttagtcaaaccattaactcctccatgcgtacttatgccgaaggcgcttatcagcaacttgcttcgggccagaaggtgaatactcctaccggcgtcgcggtatttcccggagatgcaccaacaccacgggaatgggcggagagaaaaacaaatgtaaaacggtttaccgtcatggaaaaaggtggccacttcgctgcattggaagcccccgaattatgggtgaatgaagtggatacgtttttcaaaagtaccccaggaaaataaaaccatagcaatttaaagattacaaaagggggtatgaaaatcccccctatgtatttgaaaaaccatcgtgatccgtacgtattaacatgaaaaaagtaaccatcactttactaaccctgtttagtttttacagccacacacgggcacaggaatttgacattgttacgcttcataataaggtgtctatttgttatgatgcgaacagtaagttagattccattactgcccatcttcttgcatcggatattgaacagatcagtggcttccggccttccacctcagcaggcattgctgatgtaagcggaaatgtgattgttattggaaacattcatgctgaaatcattgcccgattccgcaataagataaacctcgactctttaaatggtaaatgggaaagttatggctaccgcctattgaaagccccgacaaaaaatattaaaaatgcactcctcatttgcggaagcgaccccagaggtacggcttatggcgtgtttgacttatctgcccgtttgggtgtttcgccctggtactggtgggccgatgttaagccggtaaaaaggaaaaaaatttccatcgatataaaagactatacctccgcccctccctccgtaaaatacagggggatttttatcaatgatgaagactgggacctgcagccgtgggcggctaaaacctttgaacctgaaacaggcgatattggcccgaaaacatacgccaaggtatttgaactgctcctccgtttaaaagcaaacctgatatggcccgctatgcacccttttaccaaagcattctttcatttccccggcaatataaaaaccgcggaagactatcagatcattattggctcttctcacgcggagccaatgctgagaaataatgtaggcgaatgggatgaaaaaacgatgggccggtttaattacttcaccaacaaagaaaagatttacagctattgggaaaaccgaatccgggaaagccgtggcattaatgccatttataccctcggcatgaggggcgtgcatgatggccagatggaaggtattaaagatctccgggacgctgttcccatagtggagaaaattatcggggatgaacgggagatgctcgccaggtacatcaacaaagatgtaacagctgtaccacaggtactaactccttacaaagaagtactggaaatatatgatgctggcatgaaggttcccgatgatgtaaccattgtatggcctgatgataactacggttacatacaccgcctcaataataaaacagagcagggacgcagcggtgggtctggtgtttattaccatgcttcctattggggccgccctcatgattatctttggcttagttccacgcatcccggactgatccgcgaagaaatgctgaaagccttcgaaacaggcgccaacaggttgtgggtactcaatgtgggagatatcaagccccttgagtacaacataacgttgttcctggatatggcatataacataaaatcattccgggacagcaggtatgtcaaagatcacctgacgaattgggcaggctctatattcggaaccacccatgcccggaaaattagtaacatgctatgggaatactatcgactggcgttcgaaagaagacccgagtttatgggatggagccaaaccgaaccgactaccccaacaaattataccgcctataatcatttttactttggagatgaggcccggcgccggatagacaaatacagcagactggaggcggaaatgagaaatatccggtcacaaatcaacgttaaggacacagacgcgttttatcagttggtgtattatcccatcgtgtgtgcctcgctgatgaataaaaaatttctttacagggataaaagctacttatacgccaaacaaaacaggttaagtgcatacgattatgcccaattatcttcagatgcttatgaaagtatagtacgggaaaccgcctactataacacaacactggcaggcggtaagtggaagcatatgatgtcgatggagccgagaagtctccctgtataccaggcgcccgttataccgcccatccatatcgacagtacaaacagttgggatatcgctcccgaaggtttagtaaccaaagattcttccctgttaagcacgaccggatcgaagtcgctaccggtttttgatgtatttaataagcagaaatattttattgacatcttcttaagtaaaaatcagccggtagaatggaaagtaaccacctctgataattggatccggttgtccagcagcagtggcgtgttaactacagaacctggcaaaaaagaaatacgaatatgggtggaccttgactggaacaaatttacagggaatgaaaaaatgaccggtcaaataacatttcagggagctggcaggcagatgcaggtaaacatccagggaattaaacgaaatattccggcgctttcaggctacaggggtaaaattgaaaactgtgggtttgtttccatacaggcatctcatttttcccggcaaatgaaaagagggctgcagcattggaattttgtagaaggactgggatataaggacacggtgctacaggctttgccagtaacaattgcagatgaattgccgacagaccctgatgttattaaaagcaaccgttcttatgttgaatatgatttctataccttctcctccgcagatccgggcattactatcttcacattacccacccacccgctaaataacctttatcatttacgttatgctgtttccatcgatgatgggccattaaaaatggttgactataaaacctttggcagaagtgaagagtggaagcaaaatgtattgcgcaacagggctgaaaagaaaattgatatgccgcatctaagcgccggaaagcatcagttaaaaatatattgcatggatccgggggtaatattagatgaaatccggattgatcttggaggattgaaaaaggcgtatagtgccattccgtaactaaggcctcatatcgatagaaagcactgtgaatcacacaaactaaatttcttatttttgcagcaaataaaagcgctaaattaccaccatatgaaaaacgctaaaaaaaaattgtcacccgaacaatcacaggaactcctcagcgtattgaaaacccgttttgaaaagaacaagcaccgtcacaaagggctcgactgggccaaagtacaggcaaagctggaggcaaacccagggaagttatggtcgctcgatgaaatggagctgaccggcggcgaaccggatgtagtgggatatgataaaaataaagatgaatacattttctttgattgttcagctgaaagccccaagggccgcagaagtatctgttatgaccatgaagcactggagtcgaggaaagaacacaaaccggaaaacagcgccattgaaatggctgcggatatgggtatcgaggttttaacggaagcccaataccgcgacttacagcaacttggcaattttgatttgaaaacatcgagttggatcgtaacgccccctgcaataagaaaacttggcggcgcgctcttctgtgatcgtcgttatgatcatgtttttgtgtatcataatggtgcggaatcttactatgccgccaggggctttcgcggatcgttaagggtataattcccataatacagtgagaatggcagaaatagccccccaaaatctcccaaactaccatcgtgcttaataagcttaaggactatctttgaaactgatttggaacacggatgaacatttcagcagcatccaaatctgtattgaaaataaaaatattaactataaaacctttagtttatgaaagcaaaaaaaatctgggcgaatttcagtgtcagtgatttagaacgaaccactaagttctataaacaacttggatttaagccaaacggagcgtcggaccaactcaccagcttcttctttggcggggaagattttatcatccatttctttttgaaggatatacttgaacctgctatgaagggacaaataatagacacccaatccggcaatgaaattattttcaccctttctgttgaaactaaggaagaggttaatgcctgggcaaaagaggtggagcacgccgggggaacaatagtttcacagccagaggaatttggaaagggttattatggtttcgtgtttgctgatcctgatggtcataagtttaatatatttcagatgtagtatcgctgatgagcgattagaaatattagttctagcagataattaaaaagggtgctgtagaaggcaccctttttgttatgtcttaccactggcatctgatcaacatgatcagaatgactttttaaatacttcgaaagcgacaaattaatagctatcttactatccgatcattaatgcgattaccatgacgccaataaaacccatattattattttgttttagcttacttgctttgccagctttatctcagaaccagcaatatacttcagatagcctaaaagctcaacaattaatagccgacaagataaaacagctggaaacctcaggaataatggagtatctatacatgttctcaagtggaggctcccttgttattttgtataaaaaaggacaaagaataaacggcattaggaacttgtcttattataaaccgggatcaaggtttcgtaatgtaagattaaccaagcagcagaaatcaaattataccaagtgtattgataaggcccggatggatacaactataaatttctccggatgctacgatgacgtccatgcatttagcaggattgttttttcagcaaattcttccaaacacagtttaaaagggtcctttacaaccgactgctggcaaaagttggaaagaaatgatttgtatccacttgatgacatctacaaacgccttctaaccaagtattaggtcaaagtctgaggtttgccactgccagggtttcggtatatattttataaatctcctaaaacagcagcctctatttccgtgtctggcaatattttttatgctaaaaattatgcttgtccggctaaagtggatttaacaatcaaggggatggctctgaagaaccatccccttgattaaactaagggaaactcaaggcccaacatcacctgttacaacatccccggcccgtttgtaattggctataataacccctttagaagtcacctggctttctgtcaacgtaaatgctgccgggatcccgccgttctcgaagagcttttttccctcaccaagaatcaacgggtaaattttgaaccggagttcgtccaccaggtcgtgtttaagcaacagttgaacgagttttccgctaccccatacctgaatatctgcaccctccgaattcttcagcttttggatatctgccggagttttgaggaaaatggtattttttcaatctgatttttccatggtctgcgacagtacgtatttggcgccatcattgatgccaggccaaaagtcagcatgttgaggccaataagatgcaaaaatttcaaatgtttttctgcccaaaatataatctgccggtttcagctcttccatcatgatcttgccaaaaagctcgtcaccataagatgaagtccagccgccatacttgaagccgcctgaggtgtcttcctgggggccgccgggcgcctgcataacgccatccagtgtaatcattgaaaaaacagttatttttctcattttactttcttttttacaattaagataaaagttgtttttctgatattgagatctaccggttactttaaaaaattgttcagatagttcaatattgttgttgtctgcatcatcagggtaacatgaccttgtgaaggaacgatggccaattgcgatttgggcattgttcccagatcagcactaacagcacctcccaatgattgatatgtttttgttaactcaattttatccagcccatcattatcaccggatatgattaataccggtgcagtgattttcgaaatattggcctccccgaggttgaatggcaccgcagcgtacgcaatcatctgctccaggaactttgtccattttgttttatcaggcgccacagcgtcataggcagttttcataggggtgttcgcaaaaaactccggcttcatttttttaaacgcatcgcttactacgggcagccaaccggtacttttataggtagccgaaatgatgaccagatttcttaagcgtttaggactttgtatagcaaattcgtaagctatagcgccgccaaaactaaatcctgctacatccgcactgtcaattttcagataatccattactccttccacatcgcgtgctaaagcagcatgcgataattccctgtctgaatacggtgtatgtccgtgtccctgcaattcaatggcaattaccttcctggtttttgacagctcggggatcaattggccccagtttgtattaattgtcataaaagcaccgtgcagtaaaatgataggcctgccctcgccatatacttcataataaactttgatgccattaacaggtgcatagccgctgctggaaggtttcgcttgctgtccgcttgattgcgatgctatagccataattgcaattaacagtattgatttaagaagatgacgtgttttgaatagatttttcatatcgctgtttgaatgttagtttgaatgttattgacaatacaaaactatcattctctccaggatccggcatggggtgaaagcgacaacttaggggtagaattccgacaaaacaagtctgttgtgacaaaaagttagcatctacaaaaaggaggtccctgctttctacttcagccccctttttaagatctgcccggccatcctgaacacgcacaaatgatttgatcccactcacattccgcgaaaacctgggtccctataataagcctgtactcgaagatccatgctctgtgccattgacaactatcctggaaactattctgtaaatactggcactcttcttatgaaaacggtcaaagctcacttcatcctttacataaagtagcatcagcatagcacatgtaagaccaatagctagtcctgcaatactgattaaagagtagattttattttgcgcaagtgtgcgaattgcaatcttgaggtagtttctaagcatataggcaatataagctccctgaacatttcaatgcctatgccaaaatgcaagcatcttattaataattatttatataagtccaaatccaacaaaatgtccgattgagaacatgcggtgtacgtcaacgggcagcgaaaacccagattggaaattgttaatcgagtttatgtatgctcacatctgtaaaataaccaagcgtttccggtccaatccaaagtcctacgcttccacgcagatctttgccctgcttcaggtcattgacaatcaaagtaggttgttcagcaccattgatatagaatttggccgtttcatcttttacttcaattttcactttgatccattcagccggcagcatatcagcataagcctcgtattttcccggtgtttcttcccgtgatctatcccaggggtagcccggcaacgaaacatactgagtcgaatgattcctccgtacctggtcattggcccggccattggttggacgaatgtaaaacaactccattttggaggtatccttactcacccgaaaggcaatgccaataaacccacgtgcgccttccccggcattcacctgtggttgtcccgaaatagttgcttcaatgatgccattatgaaaatcgatatttttgagcaaggcaactgtcttttcgttaatggcggtgttcgtcatttgcaaagccagcgcgtttttgcctttataatctaattgcctaacagttacctgataaggaatgacgttatcaggaacaagggaaagatgctgtgcctgagacgatgcaaataaaaatgcactcattcccaaagtaatcaataaaacttttttcattggaactgattttagtagatatttcaatgctgttatttttatttgaacagtaaagagatgatgtccctgccagattccataaatttcaaaataaatattgccttcccaaaacaggaaaacacccacctatggctaatactcaatacatctttacactatcaatttatcaacctttaaaaatttcttgcaatttaattccaataatctaaattcgccttcgctaaacatattaacccacatcttacttaacaacaccctcgaaatagtatttgaaatcctatagtaaaaccaatagttatcccatacacatcaattataaaataatatgctaacaacaaaaacctttggaaaattatccattatcgccactgtaacggctacactattttcctgtgaaaaagcgcagccagttaagattgacaagttacctgcaggaggactaactgtcaccccaaacttaacattattagcggctgcacctgtgtccacggatagcttaattgcttactggccactggacagttgtctactcgccaatgatgtcaccggaaacgggcataatggtacttcttttagtaccacctttaccacagacaggtttggtagtagtaaaggggcttattatttcaatggcacaagcagttatatatctgtggatgacaagacagatataaaattgcttaataccaactacaccttcagtgcctgggtaaaattggataactatgaatcgtcctggggatccagtattatagccaagcgaaatggtagctccaacgggtatgcctggtcaatcacaggattactgaccacacccggtctcgtttccctgggcactggtggtggatcttttaatgcctacggtacaaaagtagttaccactggtagctggcacatggtttccactacctataactatgcaacgcagcaactgagtatttatgttgatggaatacttgataatattaccaatgccgcaccacctattagtagcactacaaataaattatatattggtagagacgaaatttcgttaccaacaggatacttcatcaaaggagcattagatgatatccgcatttacaggagatcattgactgctgccgaaattcttgccttgtataatcagactactgctccaactagcggtttaatcgcttactggccattaaacagttgctcagcagccaatgatttaacgggactaggacataatggtactgcttataatatcacctacacaaaagacaggtcgggtatcaataacagtgcttcctatttcaatggaacaagcagctacatttctgtagaagataaggcagatatccgattaacagcaacaaacttctccatgaatgcgtgggtaaaactcgatagctataactcgtcctggggttctgaaattttagtaaaacgaaacacatcttctcctggctttacatggtcaatcaccggactgctggcttcgcccattggtaccggttcatttggtcctggtggcggatttgtcaatgcattcggcacacaagtagttgccctgaatagttggcacatggtcagcaatgtgtataatgtaagtacccaacaacttagcatctatattgatggcgtattggataatgttaccaccggtgtgctgccagctaacgctccggcatccaaattatatatcggcagtgatgatctcactcttggcacaaatggctattacctgaaaggggcaatggaagatatccgcatatataacagagcattaagtgcaaccgaaattcaacagttatttactgctgtcaattaatggtaaacactctagtactttgaaacggttgcagatcaggtgatttgcaaccgttttttatttctgcacagccagtcactacaagcgccccggttcattcataattaagctaccttattaaatttgcttcgataatcacccggcgtcatgccgactacttttttaaagatttgccggaacgctttgacgtcaccataacccacctcgtacattacttccaggatttgtttacttgttgattcaaagctccgtttggccgcctctactttaacacgctgaatataatctgccggagaaagctgtgtagcctttttaaagcggcgggtgaagttaatccggtccataaaacaatgctttgccaactgctctactgttaaccggtcaccgatgtgctgctctatatattcctgcacgtttcgtatcatctggtccttatgatccttcaatccattaaacaagataaaaggtgattgggagtttcgatcaatatcgagctgcagtacttttgaacagtaaagcgcgacttcgcggccgctatatttttcaacaagataaagtaccaggttcagactggaatgaccacctcccgccgtatacagcccctgatgttctgtaatgatcctgctggtctgcaagtccagttcaggaaataatgcacgaaaatgcgctgcagcctgccagtgtgttgcacagggtgtgtgcctgagcaatcctgtggcggctaaaaggaaagtacctgtacataagctggccacttcggttcccctgcgatattgtcgtgttacccaatccagcatctttgtacttttttgtatgccgaagtcgtactcatgatcgaagctgggcagcaggatcagatctgttttagtaatattttcgaacggtgtgatatttaactggaaagttccgttcaataacttctgccgaaggtcggtacctgccagttggatatgataataaggcggtttaccctgcgccagataaaactggttagctttctcgaatatttcgatcgctccaaaaagggtacttggttttagtacgccatcagctattaagatcgttacacttttcatattataaaggtaaaccaccctatatgcacaaacaaccccttaaattgctaaatgtacaccccctcggagtcgccggtgcgctctaattttgctttcatgaaagagataaatattcttgtgagcggagcagcagggcaaagcggcggtttaattctgcgggaactggcttcgcgacaacaaccggtccgggccctggcacgcaatatagcaagcgcaaaaaacgggactgatattcccttaattgaatggatcgaaggcgatatgttggccaaagataccctaaggccagccctggagggtgtggagcgcactatcctgatctcatcggcaaatgatcgcatggtggaaacacaatgcacctctatcgacgcctgtaaagaggctggtgtaaatcatgttattaaattttctggtgaagaatcacagcaaggctacgatgcgcagcaatttcgttttacccgtgagcatgagcagatcgaggattatctggaaaaatccggccttcaatggacacacctgcgccccagccagtttatgcaggtatacctgcgggaaacggcagccatcagcaggcatggtgcattgcgcctgcctttagcgtcaatccagatgtcgcccgtcgatttgcgcgatgtagcgaaaattgccgcttccttattaattgatggtggataccacggccggtctcttcgcattaccggaccagaggcgctatccatgtcggagattgcccggatattatctgacaccaccggtaaggagattccttatgtccctgtaagctgggacgaacggaaagcagcattggcagctacaggcatgccgggttactttcttgatgcgcttgcagaacagaccgcagaaagagtaagcaagccgcaagcttttattgatatcagcacacatcaattgtttgatataacgccaaccacatttgcacaatttgcagaacaacacaagcacatttttaagcagcaatgaagaagataagtctgccaacgaattttgcagcgtttatttacaaaaacaaaagcacatttaacaactaaatattatgaaaagcacacagataagttattccgtaaatccggaaaaaaccggtgaacacatcgacctgatacgcggcgtatttgaggaactgaatcgcagtcatctgacagaggtaagctatagttgttttcaaacaggtgaacatacctttatgcatatcgcacagtttggcagtgaggctgcacatcaggcatttaccaacctgccttcatttaaggcattcagtaaaaattcaggcgatcggattgtcaacaagcccgtttcaattgacgtgaaggaaataggtgattacaaaaatagactagcatgagaaaattaattgtaagcagctttgtctcccttgacggcgttgtagataaaccctgggagtgggtcgggtctttttttgatcaggagcataagcaggactcattaacgaagcttaaagatgtcgacctgtttttgttaagccgtcctacgtatgaacattttgcatcgctatggccgaatattaaaggggaggcttatttcgatcacatgaatgcgctgccaaagcttgtggcgtctaagaccatcaaggaagccggatggaatgcgacgatcatcaatggggaagtaactgaagaaattgccaggctaaagcaaggaccgggtaagcatattcttaaatacgggtttggtgaccttgacaggacgctgatgttgcatcatctcatcgatgaacttcagctttgtattattcctgttgcagttgacaaaggccgccgtatttttgaaggtatggacccggaccaggtcaaactcacattgacggatatccgcaattttgagaatggtgcagcgatattaacctatgttccatccggttcaaaaaagcaataagaatgaagcgggagaatacttatttaagttaaaatcaaaggccccgtgctttacattgatcgtttctccctgtatgtttccccgcaaatcaattggttgaacctctttaactttatacccatcagggagctgtacggtacagttaccggatatacctgcctgctcccacaatcgcaaaatggttccgctactgtcaggattttcaccgaatgccgttactaaaacaccggttcttgaaatagatatgcccttcctttttaaaggttggtttccggaggccccttctgctactcctgtcagtaatgacacccgggcctcccaggatttttgtattagattgggtacggtttccgtgtgttgatctgttgcccatatccgaactctttcgctccatgtaccatcctgccaaagaggataattagtgttccacatgttattgtaaagattgacaaataccgatgatcttctgggcatatcatctaaagagaatttccataacccgggctctcccaaactgataaggggagcatctatcggcgcaagcgccactcctgatttgtttgcagccgtaatggcaacacctgaattcaccgccatcaaatacctgttactgccggaaataatatccgttgccggatttatcgcccctcccaggcggccaaccgtgaatgcaggtttatcaacggcaaatgggaaacaaagccaccctccttcaggttgtttgtatggggttttagatgctacaaaccattcaacatccacatacgcttcctgtcgcggaaaagtaaaaacaatagtgtaactttttgcataaccttttgtctcagttgtcgataaaacagctacatcggctattggggtatgctgcaccgataatttccagtcttcaggagtaaaagacagataagggattttgtctgccgacggcatacctggtttacctaaatcatccagcccccacccttccttaatcctgctgtatgcattaaaccatttatccacttcattagcactgaagcgctcatgcaagaactgtcccatcacataggcagaagaattatccaccagttgacgaccagtacttttttcttttaaagatgatatcccgcctctttttaaatcgaaaattgcggtaaagaacggtgtggtgagtgtggtcttttcatcagacgatgtggtttcatttttcagttctttttcggatatgacaacatacccgcccgcaggaacgtctttcacgaaaatggtttttcctttttcccagggtacctccaccattcctgaacgtttccaggatagcggattatatactacgaaacgctttcctgctatatttgtcgattttgccaatgcgtttaaccgggatgtcagttcctttgttacgatattgtttgtattttgaatatactggcgcttttcgtcataagattttaaccattttgttttgcttcctattttggtgttttccgcatcgctattgggcaacccggaatagtccccattcaggggaataggttcggcttttgcttcttccaaccatttcttccagtcatcgccatagctataccggggaccatatccggcattcataccccaggtatgctcactgtataaaaggctttgctcatatgattccgccagcctttgtgcaactgactgattagatacgccccagatgttcatttgtgttgaaagtgcatccagtacagattccaacggacggatattcctggcaatctttgattcctgtgggtttgccatcaggccatgtatccatgtatccggcatatctccggtaacagttggcaaatcaggtttttcggcaataagcgcattggcaaaatcatcgagggttccgaaatggattttaatccccggcatttccttcctggcataggctaaaagattcgctatgtctttttccgaaggtggtccggcgttgtcattcgtcatttgcatcgccagataatttttacatggccagttttcagttggcttgatatcggagccgtacaaagcggtataattacaaagtattttcgaaccatcagggccttgccaccaaaacaattcaggcagacggggatactggctggcaggattacaacccagctgcagaaacttaatacccgcatgattcaataaggttggcaaaacccaggaatgactcggcacatcagtcatttttgcactaatggtcattggtagcccgtacttccgggtgacggcagacgaataataaaggccacgaaccaggtcctcataatcgagcgactccgtttgcattgtaaaaggaagcccatgtaccacaatccggccatccctgatacttttttcaattcttgccttcctttcaggagtttgcagaggaccaagtatctgtgcctgtaacggccagcccggaactgtccaggcgaatcggtgatcttgtgattgtgtggaatttttttctattatttccaatgccttatccatcatttctgtgcgataacgcttgaaaacattctgtggtaaatcggtaaatcctaagtcaaaatgggtcttaaataccacccatacgtctgttactttcgaaatatggggagtagctgtttttcgatcttgtgcacctgttcttgttacgaataataaaataacaacaattaaagcattaactctttttatcataaatggtgtagcttttcatttcagaggctgaccaatccccggatttttgaataccaggaagatatcagcaacaattttcttccccctgtgattctacacttaattcatgcgggaacggcgcactaagctaaatgatatatcccggtaacataccgtcaaaattgacattatcctatgttattttgccccttcaaagctgattttctattttattttaggcggatacattataaatgttccttcgggcaattggtaaaacgacgccggcttttccagcttcacaacactttttgccatcatcccttttatttcgccgtagcctctgtcgctgtaaaccaacaaagccataccgggtattctttgcaggtattcaaacgagggcaaataaaactgaggtagttccgggcagtaccacaccgttgtttccagttttgtatcacccggccttaccgcatccggggtataattgattactgcacgtttacagagatagccggctacagtcatcgtatcattggtcagtgtaataccaccgtgctttttccaccgctccggaaaaccctcaccggcatggtaaacattggtcttcataaattcatcaaaattcatcggaagcgccattttgccccgcaattccatcagccttttgattttgtattctatctgccagattgttttatcgccgttgggcaaaatatcctctgcatacaaatacccgggatgagcataaactaccaaaggtttccaaccggccttttctatccgttcctgctccacgtgcatcggcacttcagatgggctgctggtatctgttgccttaatgtaaaagccaaaatctattttataaatgtctaacaactggttgttttttgtttgggcattgccgtttgtaaatgtcataattgctgataacaagagcaataactgaaagattggttgtgggctcatattccaaaaatagacattatggtgctgacaaatatccctggatacaggtattttattccttgtattactgagtatctttgtaatttgaaagaactataaaagttttgttgcctgccctaaacatcaatattgctataaaaattatgagactgcaaattacacccttcgctattatttcgataatagcactgatagctacgatttattatttacaaggtatacaaaacatacccaaaggcaggtatgggggctatattgtcttgctaacagggtttttatttgtgattacattggtattagatgtaattttcaggcttaccatcaaaagccttctaacaatttggattgtagaagcagtattggcttttattggcctcattgtccttttggtttgacacggaaaatatgaaacagatcattatatccggacttttaatattatcaattccttgtattggacagacagtaactaagacattaaagtatgggggaacttatacttatggaggtaatgttgagaaaggtcgtatcggaacaatttatatttatcccgagacagacagcactattctgttttatattgacttaaatcgtggcgctccttcatacaacacggggtatttatatggacgagtgattattaaaaatgacaacgggacattttatactaaaattgacctcgcagagaatggatgtaaattgatttttaagttttcaagaaacaagttgacaatacagtcaattgaggttaactgtggctttggtggtttagtatatgcagacggagaatttaaaaaaatatcaaaaaagccattggactattttgaggatgtggaaggaaaaaaggtttattttaaaactacaaaacctgaagactacaataaagattaaagcatacaaagcgttgccataaaaggaaagacactattttaatagcatttgctcagtaaagaaagatattgccatagtatgaaaacatcgccatcaaatatcttgatatttcttttctttctaaacacttccgctatggcacaagcagatacttcttttaaccaattcgaaaaaacgtataccgcgtttgttgataacagcacgccccttgccgctttttcggtaaaaaaactaagtcgaaaggaatggaaaaattcgaacacaaaaactgcggataacaaaaacaccttaatcacacctgtatcaaacggagctatcacattaaccggaataagagctgtggaagagatttatacaaccgcaccaaggggcaaaggagaacgtgtagggcaaaccatcgccaccaacctgcaatttaagggacaatattacggaataaaaagattgcttgagataaggataacggaatggaaaccagcggaggttaagctggtatcgtaccgcgaactatggctgaaagtaaaattgctatacccgaatgataatggcgataaggttattgagaaaagtacctacgattatatcaggctaatactcccatttgatgataagcaatagaaaaacaatccacatccatatcgtttggccatacattctacgccacagccctttttctgagtttatgggcgcttatattttagtaaatcggcctgttgcttgtcctcttccgaaagtggtcgtcctgttctcccagtgatggtaagcaattccaaatttggcaaaacgatgtttacataatcggagtcatacgtgacctctgagcctttgggtaaacgatagcctagtaaaatgtaatcgtcggccagcgttcccctgataaatgtgctatcggcgccaatcattacatccccaatacagggccagccaaataccagttgttgatgggtaagcgtaacgttccattcattatgcaaaccaaccctgataatatccgttacctgtaaattaaaaaaacgggcaggttttgataaatgaacggagtcaatatcgttcaattgtgcctctttcctgtagttcatatcaaactccgtagcataaaaaacagtatctccggccgaaaggacaatgccggctgtagtttcgggctgcttcaagatataagtatgtagcattttttgtggccttacctccggtttattgattccattatttattaatccgccctgatcccataccattaccaccatcggaaataacagcacagtagcgccaatacccgaaatccatcttatacccggtttgttatttctgtcgaggcaagcccagagcagtaaaaaagctattggtacagtaatgtaccaataataaaaggtgtaaagcaggtacttcccaaaagggccaaagttaagatccataatttatcagtttattgcagttgcaatagcaagatagggcactattacgtttcctatggtacaggaatcgaatttcctttttgctaaatttaaagcaaataggcaacttaagctgattaaacctattgtcatataaaaatagttttaatcgctgtcagggtgctgttaccacataattaaaaaaatataattgggattattaaaattttgatttaacaatgaatagcattcgcaccacttttctggatcaaatagacaatgaaattatcgagaaaaaagaagctttgatttatttataaatttgaatgaacatcaattatctttttaagcagccggaaaaacactgacatcatctgagataatccgagtctaatccttttaaccagcttgtcacgtcccttactattgtatcatctaactcaaacaatagaaattcaggatatttgactctttgatgttcaggatgtacaagaacaatcaatctatcccggttaacgattaaaaagtcataacaaaaccttataaggtagcctatagcgtcattagctaagccggttgtttctacaacaacaacttcatgattatccaactcatttaagattacaaagataatttgctcataaaagctgctatcactcaaggacagatccggaagattaaatatctgcctcagataatcgattccagtagaattgaacttctttcgacttttataggcggacacttttatagctccttgaaaaaaagagttaatatgagaaactggcggttgtgaggtagagaataattggcgctggattccaggaatagatgttaatatcatatacagagacccatagttcaactgatttttcactctatattcataattttctatcaataaacctcgtatcattttttggcctttactggaagattacttttataccatcctctgcaggatttgcgcctgtaaaattatcattttggatcagtgattgcacaaacgtattatctcctgtttctaatgtatattggatagccgcattcatcctgtgatttccatctgtagtgactgtctttatctatgaaacccgcagctccttgttcgattgccatccactaatttaaactgatcgtcgaataatacaagattaagataagctttgggcgagctctttttctttcgtcagaaatcagtgttctcttttttcctggtcactgtaatctctgttctccggttcgcctgatgatccgcttccgcgcattttaccccgtttaaacaatgattcaccagtcttgattccccatatccacgggcagtcatcctttcattggaaattccttttgtcacaagatattgtacggctgcatcagcccttttacgggacaggctcatgttgtaactgtcgctcccccggctgtcggtatgggcactcagcattatctttatctcaggataccttataagcaccgatgccagggaatcaagtaccgctgtggcatctggagacctgatataactcttatcgaagtcatagtacaagttagtcaaaataaatacctcatcgggttgtggtactccaggcttcggttttacccggtttggcgggggaatgctcgctgcgggaggttcaacgggagacgcctggcggacaaatatataaatatcatcgctgcctttcccgcctggcctgttggaagccaggtagccactgaccgaatctgcagacacaaaataaaaatcgtcgtaactggaatttaacggaggccgcatattcactggttcattccactgatccatagcgccagttacacggaatatgtccaatccgcctatgcctgtatgtcccctactggcgatgtacaagttgccgtccggccccagcacgggaaacaattcatcgtcaggcgtattgatcaccgccccgcagttcctgggcgccagccacccgccggatgtatcgcgaaggcaaaaccagatatctgcaccaccttgaccacccggcctgtcggatacaaaatacaggatgttgccgtcgccggtgatggcggcatggccagtggaccattcttctgcattattgtatgggaatggataggctggcttctcaccgtccgatatatataactccagcctgcgcgtcccgatcttcttcccgtcttctttttccattttcaacctgccttcccggctaacggtaaagtacacggaatccccatgataacaggcaggcccgatatgatacttgcttacatctatcacggaagcaagattgtctatatttagcctgccgggagagccttcggggttgcttagctggaataccctgaagtaaggctcgcccgtttgtcctgataccttctgcgaagtaggttccaaccggttgaaattggaagtgtaatacagttttcctttttcacggaaagcaccccaatctgaataggtggaattaacggcatccaggttttgcaggcgaatgcgccccggggttgtccattgcatggcggaatcgcagccggcaattctatttcgcaggtccctcctgcctttatactggccgtaactatttttggcagcatcatattgcccaagcattttctgtatgtccccaatccttaccaggagagaatcggcagaaggatctttctcaacacagcctgtataagcagcgatcgcctcagggtatttctgcaacgattcataactgtaccccagcctgtagtacaccagcggtttggctttctttgaccgggccaaccgctcgtatatcggtgcagctttgctgaaacgccatgttctaaagtaggtatcagccaattgctcataaccgggctgttcctgccccaggcaaggaacataaaaaaacagcagcaggaataggattgatttaacgggcatgatcgttcatttaaaagtacctgggcgatatctcccttttttgtttgttcaggaacagcaggccgatggatatttcatggctgcccgattgataggaattaagcccgctgacagtgaagtcatatgcatatcccagccgcaaccatttggtggcgtatacttccaccaatgcagaaactgcatcctgtctttccagaccgctttgcaggtttgttttgtcccatatctggaagccagtccggtaagaaacgcccagccacagcatctctttgatcagcataaaggcggtcaggtcaatattagacggacctttaaaatcctctttccaaagaaaagaaggctttaatttgagatgttctcccatattaaggaccgttcccgcccccatgtaaaggtgcggttccctgacgatgctggtaaagagcttgccgtcccagttatatgccttcatgccggtggcctgaagcaggttattgacagatgcggtaatgtaatatttcggcgtatagaacagtacgccgaaggttgcatccggttcgatgtgggtgggcctgcccacggggacacgctcgtcgaaatcgtccacatattccagtacagagccatccagctgatattgcagaataccaccggtaataccgaaacaaagccgcttcgcgccttcttcgtccaacggtatacggtaggtggcgcccatcgctgctgtaatagttttttgcgcccccatttcatcgagcataaaatttccgctcagtgcaagccgctcttccttcgcattggtcagcccgtctatcgaagcacccgtggttaccggtgcgccgtctattcccctccattgcctgcggtggatcacattaaggctggttccacccctatagccggcgtaagccggattcagattcagcatattgaaaatgtactggctgaattgcacttcctgctgggcttttgcaggtaacagatacaacaagccccataatacacacatcagcattttatggttcatatcaactgtttttatctgattaattgaatccatcccgtgtaggttttgatgccctcggggatgcgtaatttcagtacgtagtaatacgttgattccgtaaggccattaccatcccattcgttgtggtagctggagttataatacacttcattgccccagcgattatagatggcgatggaagaagccgggtaattctccaatcctttgatcaccagtttatcgttacggccgtcgccgttcggtgtgatcacattagggatgaacaccagtctgccgccaccgtcaaaaggtatcttcgtggtatccccgcccggtggaccggtaggcgtagtgccggtttcattggtcaccgtatctatcgtaactaatgccatattattgatggaagatattcctgcggtgctgttttttaccatcacctggaagcccgcctgctgcgtgctgccaacggaaaggctgttgaacccgaacagcacattgccgccggtgagtgtgccgccactgcctgttaggtaactggtgttggcaggaatgggatcgctgacgttcacatcagccaacggcacggtaccggtgttacgcacgtaaatgatgtaggtaagcacctcacccggctgggcgctgttatctccacttgcatcccttacttctttccacgtggtaaaatctttcacatccaacctgaatgatgcccttgcgctgacactgcagccaaccgggtaagaggcgctcacttcgtacagggctgcatctgtcacactaacattagccaggttgagtgtattgcctgttacactgctgatcaccacgttgtttttgtaccaggtgaaagcattggcgcctgccgccgtggcggtaagcgtcaggttggagcccgaccatagcgcttcctgtgcaggtacattgagcacgggggcagacgggcctgcaccaacacttacggtgatcgcctgtgcgtcatttgccgcgttttcgcatatggtgttgttgctgacggtcacataatatgtggtagtcgcggtaatgggcggggtggtaaatgttgcgccggtgtacagcttatttgtcagcccggcatcggcataccagttataaatcagcgggctgctgagccttgcaaagtccgtgagccgtgaggtagcggtaatagttaccggagatccctggcaggtgctggtatcttttaaggtaacatccgcagctatggctttataattcacattaacgaatacctgttttgctgtcaacgggctattctcacaaacacctgtcccctgaacagtcacgtaataattggtagaggtagtgagcgccggcgtcgtaaaggccggacctgtagccagtttttgtgtaagtgcaggatctgcataccaattgaaagtcgcgccgggtactgtgctgtttgcattaagcacggcagttccttcctggcaaatgctggcgctgtttacggcaatatcagtagcaacggcattccgggataccattacattaatggcctttgctgcgccggtggggttagcgcatacactgtctcctgtcacagttacataataaaccgtattgcccctaatagcgggcgtcgcaaaagttggcccgtaatccagcaattgggtaagggcggaatccgcgtaccagttgaatgccggtgtatttacagaaggcgctgttacgttgagcaatacattgttcccttcacagatggacacatcgttaccaacaatatcggtggccgcggcaacgcgaaagacttttacaatcgcttccctggcattgccgggtgtgttttcacagagcacatcattctgcatagtgacataataatgtgtagtctgctgtaatgaaggagtagtaaatgtgctgcctgttgccagcaaggtagtaagccctgcatctgcataccatcggaagatggcagtcccccgcactcttgccggaaggttagcgttgagcgttgctgtgttgcccgcgcagataatgcggtctgtagccgcaaggtcttcacgggtactgctccgcttaacagcaatcctgactgtttttgccccgccgggtttattgctgcatacccctgttgcagtcactgacacataataactcgtgatgttatacagcggaggcgtggtgaaagctgcgccggtgaacagtgctcgcgtcagcccgggatcggcataccatgtaaataccgggtttgtcaatgtgctggaggcagtaagcgtggtgcggccgcccgggcacgcagtagtatcctgcaggataatatccgtgggcactgcaaaacgattaatggtaacctttaccggtttaccggcgccgggcagattttcgcaaacgcccggtgcattgatggtcacataatactccgtagtagtattcagggccggcgttacaaaagtggcgccggttccagccagagaggtcagtgctgcatcgcggtaccatttgaaaatggcgccgggcatactactggaagcacgcagtgttgcaattccgtcttcgcaaaaagaggtatctgccacattgatatctgtcgctgtaccaaaacggttgacagttacagtaacctgctgcgcattggctttattgcttacacaaacgttggtgccagccactgtaagatagtaagaggtagtggcggtaggaacaggcgtctggaaagcttcaccggtatacaacaactggctgagcgccgcatcggcataccagttaaataccggttgcgctatcgtattgctggtggccagcaatgtggtgatatctcctttacagatagcgcgtggcgccacgacaatgtctgcagcggttgcattcctgttgacagtaaccgttacctgctgcacatcgccaggaccgttcacacaaacaccttcgccggtaacgtttatatagtaggtaacggatgcgctcaaagccggggtggtaaagcttgcaccagtgaataccaattgggtgagccccggatccgcataccatttaaataccgggttggtgatgccgctggatgcgttaagttgcacattgctgccggcgcagatcacggtatccctgatgataatgtccgccgctactgctttccgcgaaactataatattgactggttttgcttgcggcgggaagttttcacacgcgtccgtgccattcacggtgacatagtacgtagccggagcagaaagggatggtgtggtgaaacttgcacccgcagctaccgggttattcaacccggcgtctgtataccagctgaatacgggattactaatgtcggaactggctgtcatggtcactgcattgccttcgcatatggactgatccgcagtggtaatatccgctgccagggcatgacggttcacggctactgtaacggacagcggaatagttgaaggaccttcgcaaacaccgtttccgcttaccgccacgtaataatttttggtggctgccaggactggtgtggtgaatacagggcctgtaaagatcaggctggtccggtttgcatcactgtaccagttgaataccgggttgctcaactggctatttgccacgagggtagcggtttccccggcgcaaatcgtcatgccggccacggtcgcatctgcggtcacgctattacgttgtaccgttaccgttaccacctttgatgtgccgggatcgttctcacaaaccccggttcccgaaacggtgatataatagttagccgaagcgcttagagcgggcgtggtgaagcttgcaccggtgaacagtagctgattgtgagctgggtctgcataccagttaaataccgggcttgcaatgctactggaagcggtgagctgtacagtgttgccggagcagatcaccgtatccttaacgctgatatcactggctactgctttcctggcaatcgcaatatttactgccttgccattcggagggaagttttcgcaggcatctgaaccattcacagttacataataagtagctgatgtagagagtgcaggtgtggtaaagcttgctcccgccgcaataggatggttcaattctgcgtccgtataccaggtgaacacgggattggtaacagaagagccggccgtcatggtcacggcgtttcctgcgcagccagactggtccgccgcggtaatatctgaagccaccgcatgcctgttcacagtcaccgtaacggtggcaggcacacgctgcggagtggaaggaccttcgcagataccgtctccgtttacagtcagaaagtattgagtagtaatagccagcggcggtgtggtgaaagccggccctgtgaagagcaggttcgttctggcggcatcgctgtaccagttgtataccgggttggtaatattggatgaagccacaacagtacccgttgcccctgcgcagatggtaagaccttccgccgttacatctgctgtagtgctgttgcggagcagcgttactgttactggcttcgcggttccgggttcattttcacaaaccaggttactgctggccgtaacataataggtggtagtgttcactaacaccggggtagtgtaaacggtacctgtgaaaagtaagttggtcagggcagcatcggcataccacctgaatacaggccccgcttccccgcgcaggccgcgggtgagatcggtggtgcttatgacgagagtcgcagactgattcggacatatctcctggttgttcaccagtatatcggcagcagtagcgcggcgttttactccaactgtcacggcatgtgcatcacctgctttattttcacaaacatcggttccttgcacggttacataataaagcgaagtggtagtgatggccggtgtggaaaaactggcgccggttcccagcaaagtggtcagcgcaggatcaccataccaggtgaataccgcacctggcacggtggaggtagcgatcaaggttacgccttcccctggacatgccagggtatcccgtatagttatatcgtttgcaacggctttgcggtttacatttgccaatacagttttggcggtgccgggcagactgctgcacacggaatctccggatacggatacataataggtggtagcggcatccagcggaggtgtggtatatgttgcgccggcacctacctgttgctgtaaggcagcatcgctataccaggtgaatacagcaccggttaccgcgctgctggcggtgagcgtgcctgcctctccaacgcagaccgcctgccctgctactgttatatctgctgcagtactgttccgccggatagttactgttactgctttggctgaacccactgcgttttcacaaaccaggcggctgctggcggtaacgtaataagtagtaatattttgcaatacgggtgtgatgtaggtagtgcctgtaaacagcagattggtcaaccccgcatccgcataccatctgtatacagggcttgcctcactgcccagcccacgggtaagattggtagcattgatcaccagcgtggcagcctgtcctgcacaaatggcctgatcgttcaccagtatatcagcagcagtggcgcggcgctttacaccaacggttacggtatgtgcatccgcggcctgattttcacacacgttatctcccttcaccgttacataataaaatgatgtggtgttaatagccggtacagcatagctggcgctggtactcagcacggtagttagcccgggatccgcgtaccaggtaaatacggcgccgggcacagttgacgtagcatttaaagtaatgccttcgcccgggcatacaagggtatccacaacaatgatgtcggcggatatgccagtgcggttaaccgttacctgaactgctttggcatctccgggcaggctggcgcaaacgctgtctcccgaaacggtgacgtaaaaggtggcactgctatccagtgcagatatagtatagccaggaccggtagccaccttgtgctgaagggaaatatcgctgtaccaattgaatactgcaccctttattttgctgttggcggtaagagtggcggcactgttgggacatatggcgatatcagctgcagtgatgtcatcaggcaaagcggtgcgctgtacagtgagcaccacggcttttgccgcaccctgtatattagcacaaacagcgtctccctgaacggttacatagaaggtatcagtgacggcggtatcagaagtgatatatgtcgggccggtagccagtagaatatgaagcgaatcatccgcataccagttgaacacggggttcttcacggtagtggtggtggctgttagcgtagcgctattgccgctgcaaacagtcttgccggccgcattaatgtccgcaaccgttgcattcctgttcacgatcacattggcgatgtaggcatccccgggccggctgctgcacacaccggttccgcttaccgccacgtagtaatctgtactggtattcaatgcggaggtctggtaatgatcaccggttacgagcggttgcgtaagggctgcatccgcaaaccaggtaaatcgcggatcgggtatggcgctttgtacgataagtacagcagaatctccagcacagatcgtctggccgctgcctgtgatatctgccaccactgcatttctgttcacattcacccgcactctgcctgcattagacggcgcattttcgcaagcatccgtgccctgaacagtaacataataggtaatgctatcctgaagcgccgtggtggtatgattggcgccgctggtaagcggtatggtcaatgcgctgtctgcataccatgtaaataccggattggccaccgttgtacttgccgccgtcaatacaattgtgttaccggcgcatatggtggaatctttcagggccaggtcggttaagtccgccaggctggtaactgtaacggttatacgttttgctgtgcctggcagatttctgcacacattggctccctccgctgctacataatagtttgtggtgcctgttaaggccggagttgtaaagctggagcccaaacccaccggttgagtaagcgccgcatcagcaaaccacgtgaactgcggattggagatcgttggagaaccaacaacaagcgtagcggatacaccgctgcagatgtgctggttcagacctttgatgtcggatgaatcagcattccggttggcggtcacggttacctgtttggcatcgcctggcagaggaccgcaataatcaccgctggatgcggcaacataataggtggtggtattagaagtgggtggcgttacaaatgtattgccagtgcccagcagcgtgttcatgcctgggtctgcgtaccaggagaagttcgtccctggcaggctggaggtggctgtgagtgaagcggtggaaccggcacatatcaccggattttgcacggatacatcagccggagcagtgtgtgggcgtacatctacatttacaactacaggtccggtgccgatggggccaggttggttttcacaaatgccatccgcgctaaccgttacaaaaaattgcttttgactgttcagcggaggagtgttgatcatagggccaacggcgtataactgtgtcagcgaaggatcctggtaccagcggaatacgggattttgcaagttgctactggccgtgagcatggcgctttctccggcacaaatgctggtggaacgtgcaaagagatcggctgtggttgcattcctgtctacggtcacggttacggcttttgccgtattgggcaaattctcacaggaagactggctgctgagggtaacgtaatatgtagtggtagcggttagatgcggggtttcataaacatcgccggtgaatagcaggttagtgagttgcgggtctttataccatttgaatacctttcccgctccggtatgtgaggtacttgcaacaagcctgacgatgctattataacaaatgttctgatcgttcacctgtatgtctgccgctactgaataaggatgtacggcaactgttaccgcctttatgttggaagtaaagttttcgcagacgcctgtaccggttaccgttacataataggtggtggaagcgctgtgggatggagcgctgtaggtgttgccggtaaaaagcaaggtagtcaaagacgcatccgcataccatctgaaaacaggagccggtacagttgacgaggacgccgtgagcgcgacagaagcacctgtacaaatcaccgtatccctgatattgatgtctgccgctgttgcacgccggtttacagtaacctggacaggctgattgccggaagcgcatttatcaactgaatatgcggtaatatagtaggtggtggtaacagttggggtaacccggtttggattgcccaaaggagtagtgcccccggcgtccacgaaatatgcgatgctatcgacattcgtactacccgcggtgatcgcgggaagggtaaggtttacactgtctccctcacaaatggagaccggtgtaacctgtagtgaaggactcagggcctgttgcaggctttctgtagatgtggccacgcagccggtgccggcggtaacgaccagttggtaagagccgctgttggccgctgtaaatgaaggtatcacgatactgtcgatgccggaccgtgtactgccatcaggcagtgtccatatgatattggcgatactgccgatggggcgcgttctcagcacaacccttccgccagggcataccttcccttccgaaacagcaccggaaacacggataagtgaagtagaagcagtattgaacagctctacattcggcgtaacctgtgtaccacatccgtccaggatctgaatggtatagtttccgggagcaagcccgtgaaaatcgggcgatccctggaagggagtatatgaggcgtcgggaacgcccgctggttttaaccggtaagtaaaaggagagctgcccactccttccacatgtaaggttcccgtatcccggccattacacacaaaaccgccggactttagctggtcaaattgtggcggcatgtaaggaggcaacgttaccagcaaggaatccaacgctttcggacagagagagggtgaacctccgtttgtataaaccttcacataataattgccggaagggagattgtaaaatgccctcgcaaaattgctgccagcaggaatcccctgaacaacgtcgccggtctgcgtattaacaagaaaggaattatgagcaacattgcctttggaaccggcaggaacaaaaaacctggcatacgtctgtacatcatagaatccgcaacctttcgctgccggtaccatccttacagagtcaattaccgccctggtgtaagatttgacgaggttcatgctcaaagtgtctgtccggcaaacggggcttccataggatacttctatggaataaaccccgaaaggcatgttctggaaaatatcatttgcggccactccgctgttcattatgtaagtctgtcctatgttcccgggaccggtcagcactttaaaagtaatgggatatggcccgttgctgagtatattttttacgctgatcctgccggattcaagagaacagggcatatacccggttaaagtgaaaataggctgctgtaaagtggattgcgggagagtgatccttgttgttttggaaaaattagcagcgtcgctgatcgttatattatatgttttcccggctaccaggcttggcaggtgaaaagtgtgcgacgacatatttcctgtgaccacccggttgtacgggccaccctcctcctgtatagtaattgtgatgggattgcaaatgcgccggaaagaagacagggtggaactgagataagtcaggtactcgcttccgcacatattacttgcccccgggctgatgatcgtatttactatgaggtctgttggttctacagtataggtataatatttactttccagtgtacaggggttttcaacctgcatcctgacggtttgagctgctgaattatcgtaagcgccgcctacgggtacagccggattgctaagtgccgtccagggcccccaattgccggatagcgccggtgattcgaagcgcgccatgacacttgcataattgaagtcaggccatttctgaccaccactgtatatattcactttctgaccgtttaccgtcagcccgtcgcaggtggcgttgatgaaaaagttgttatagggtgtattatcttcaatatttacagaatcgatcggccggtttgaataagaataatcttccacgacggtgataacgccgctcaggcgagagctgccacaatcatccaaaacccgcacggtgtactgtcccctcgccaggttataaaaaaaattggacgactggtaaggccgcaatacggtggtaccagtggcatccaacaattcatactgatagggggctctccctttcacgatgcttacgctaagataaccttgcggactacattgattgccgggaattgtttgataagactgttcggtacctataaattccagtagctgataaggagaggtcactgatgcattttttaccactggggtagttcccgtatttgcatcgtacaccagcacgagataatttcccgccgggagattattgaatatattactgccttgctgcggcactacaaccgccatgctgttggcgtccagcaactcgtagagcaccggtggagcggtattggtagcagttaccgtgatcttcccgtctgactggcaaacaccatttgttaccgaaatgattacattaggtttcgtctgtgaaaacacaggaaaagttgatatggtagtcaacatcagaattgtcaggacaacaacctggtaaatgcagcgtataccaagtaaaggtatctccataagaaagggtttagtctcacagaaagaaatattacgttcgcggtataaagctgaagaaatgaatgttaaacaacgggccttcagtgtaaccttctatataaaaaaggatggacctaaactgcaggagtaaaggaaaacttcttttaacccataacggccaaatatttctgtccggagcaaatagagatttcttcataaacagcctgttttactgaataggaaaggattatgcccttaggtataagcatgcttacctatcccattccgcttttacagtttggtcacaaatacgataaaacttgatattgctgtttatgccaggagagtatttcaattaggttaacaccaatagccggaatttgtttaaaatggccgccatatttatcaggcattgttaataccgttcagataactttcgcccgaaaagccaataccataggcaatttcactcatgcgcatatcactgcgcaatagtctgaaatgacgacttaaattttcagatttaagtttcccgggttcaaaaatgattacttgtttataaaaccgaagtactggtagaaaaaaataccggtaatcaggtattgtactgacatggttaatttagttgctttgtttaagcaaaaggcaaaaagcttatatcgaatacacataaacaaaaatgttttaagctgcttactaccaaaacataacctaatcattaatatagatgaattttagattccatgataaggtatttctgagattaccacgctatataatccacaaaaaaactttggctgcggatttgactatagaaatgatgatgaaggatttattctttttggaagctgtttatgtagcttctcccgtcgtctatgataaatgcattaaatttcaggcaaacgctcttactgtcgctgatgttgatacgttagagcttactcttgcaaagtactataccagaatgtcaacaagaagtacgccttttggtttattttctggagtgggaataacttcctggggcaagggggacgttgtttttaatcccggtaagatccattggagaagaaaagcaagattggatttccattttttagcggctacaatcaaaaaaatatcaaatttaactgttgtaaagagatattcagtatactttctaaataatagcggttacaaaataaataatgaactcaggtatgtagagttttttccatatggatttgccaggaagtatcaaattgccgctataaaaatatccggcctcattgaagaggtatttgacttaacgatcacaggggcaacttttatagatcttgagcgttttcttgttaagaatggcatcgatgttaaagctgcaaatgaattcctcgattacttaattgaaagtaaggtgctgacctccgctttcgagccgtctcctgttggtactgatattctccaacaaatttcaaataatattaaagcccttatcggtttagatcttcccgatcgcgaaatgggagaattacacgatgctatggactttatcaatgctttgcgctcggatcttcaacacgtaaatgaaaataatacattaggcgtaggggcatacaaaaacttatatcaaaggtctaaattgataatacctaaccaggtcgaaagtaatcttatacaggtagattccttttttgaaggagtagaggaagcagttagtgcggattacaaggtgctgttagcgcaatcatttactttcctaaattcattttttgaaggaaataatcaggataaagaattaaatcttttctcacagcaattttcagaaaagtatggtgatcgctttatgcctctcaacctgatcatggattatgatagtggtcttggttatccagttagcaaaaatttcgggtattcgccgtttgtaaatgatattgactttcaccaatcgcctcgtgaagctataagcatcaaatggaactacagtaatcggctgctttttaaaaaaataatggccggcagggataatcgggcgtatgaaatatctttgacagacaatgatctgccgatcagggaaagacaaacgaacaatctgccgtccacactctcagctcttttcagattgatcaataacgattcgtataaaattcagctggaaggcttttttggtccctcagctgtaaatgcgattagtcgctttgcttacataaaaacagatattgctgacttagcgaaagatattatatcatatgaagaaaatgaactggtaaattgtattgatgttgaaataatacacataccaagcgacaaagctgccaatattgtccaacatccagattttggacaatataatctcgcatatctcgggaactccaacaagtcgggaaagtattcggtaaacattaatgacctctatttaaagtgtatggatggagtgttgttactatggtcaaaaaagttaaagtgttttgtgcgaccaaggcttaattcaatgcataattacagttcgagcaacttacctgtataccgcttcctgtgcgattttcaaaagcaaaatttgaaaaataatattagtttccagtggggtgatcttcttcattgtttcgagtttttcccgcgtgtaacttatggcaaggtaattttatatcctgcgatgtggaagttggatagatcggacctgcattgtttttataaaaatgatggtgataagtcaataactgaattaatagaggagttcgtaaacagattcaggtttccaagatatgtggtcttagctgacggagataatgaactgttgattgactttgaaacgcagatcacattcaggttccttctgaaagcagcaaagaatcgttctcaaatattaatcaaagaatttctttatcacgaagacgaacatacaatttcagccaaccaactcatggggactgtattaatcgatggttcaaaggagttcaaaatgtatcgaaactttccccatgaaaccagaatggagccaggcaatgatgcacccgaagcagaatggctatacttcaaaatttattgtggtgagagttcagcagaccacgtcctcctaaattatcttaaacctgtgacagacttacttattgaagcaggtcttataacgatgtggttctttattaggtattatgacccttactttcatttacgttttagagttaagctgacagatgatagtaacaagggaaaagtttatgaaataatttgccggtatctgcagaaagctgtccaaatgaacctggtttcaaggctaagtacagacaattatattcgggaattggatcgctatggagataaatccatcgacctgacagaaggtatatttcatcttgaaagtattaatttccttgacttccttgttaatttcaattcaaatgaatgggaagaaaagaaatggatgtttgcggttgtctccgttgactcatttcttaacactgctggatttagctcttctgataaagtaagccatttaaaaaaaagtttggatgctttttacattgagttcaacgtaggcaaggaggaaaagaaagctttaaatttaaaatatcgaaaacatagggataagctacaggagttattatcaaatgacaaaaaatatgaccgcaatgattcagatatttctttcattaagcatattgtatcagctaatcaaaagggtatagctggatttttgtctcattttcctgagaaaaaaaaagagaacgctgttttttttagcgaactccgatactttagtagtgttacccacatgactctaaatcgcgttttttcattcaaaccaagaactaatgagatggttatttattactttatttataattactatttatctcatatcgcgataaatagcaaaaaatcatttctttaacagaaataaaagcggatgtcgaaaagctatcagagtagacgcaatttttaaacccagaaactatgttattaaaagaagaatgcaaacttgaaatggatgatttaaagtcattgtcaattgaaaagagaaccgtaacagagttaaccgaatctgatatggcttcaattgatggagggtcgactgtatggtgtttgctggcaaacccagttgctatgttcacactaatccctgaatggtaaacatcctggagataaggtacagtcccttcaaccggtctgtatcttatcttattaggacaaattaccatgcagggcacttcaattcgaacagcataagttggagtatgataatactaataatgattcttatctttaacccggagaagtttaagaaagttgattacagataaagctgctgattggtttaatacaaaaagaatggaagatgggaattaaaattaaacagcatgatccatttgattgtggcgctgcctgtttggttagtgtttgttcttattataaacttaaaatctcaatagcaagcgtccgtagtctaaccaaaacggaccttagaggcacaacggttctgggaatcgtcaaagccgccaaaagtatgggatttatctctacagcatacgcaaatgcacaattgatagatttggaagaacgaaaagagccaattgttgcgcatgtgttcatcagtaggcaaccccattatgtagtcatttataaaactacaaaaaaatatgttaaggtgatggatcccgcttatggtacaatcattaaatatagccatgaagatttcctgaaaatctggagtggaacgctgatcacgctaactccggatgctgaatttgagactggtaattttacccggtcgcatgcttctcacttttggtctcttataaaacctcaaaaatcattgtttctccaggtgctgtttggtggaataatctatgccacacttggtgtttccacctcaatttacgtgcaaaaaattacagattatgtaatccccagctccaataataatcttttaaatttattgacgataataatgattattatcgtggtgatgcaagcttttatcaatctttccaaagagcttttaattatacaaatagggaaactagttgatgtaaaattgatattaggatattataaacacattatttacctgcctcaggcattttttgatgggatgcgtgtaggagaaattatcagccgtgtaaatgacgccattaagatccggagttttataaatgaagtctgtatcagtatctttctaaacggggctattgtcatgttatccttggttttaatggctatttattcctggaaacttgcactgctgatgtccctgattatacctcttgcgattttactttatttcttcagtcatagaattaaccggatctatcagagaaaaggaatggaggcatcggcagttttggagagccagcttgtcgaatcaataaatgcttcaggtaccatcaaaagattgggcttagaaaattatgtgaacgaaaaaacggaaaatagttttatcgtctttttaagaaccatataccaagcttatacttcaaattcttatattaaagtaataagcgacctggtaaataaggcacttatcgttcttctgctttattttgggactttcatggttacagacggtgtaattactaccggagagttgttttccttctatagtctcctggcgtactttaccgcccctctttttgcattaattgcatcgaataaacaaattcaggaagcagttattgcatctgacaggctatttgaaattatggatttaaaaacagaggccgaaaatcagaccagtaagattgatcttcaaactagtatgattggagatattactttcaaaaacgtcacttttcgatatggtaaccgtgcaattattctggataatatatcccttcttattcctcatagaaaatcaaccgcaataatagggaataatggttcaggtaaaagtacaatcatgaatcttttacaaaacatgtatcctattgacgcaggaaatgtacatataggagcgtacaatctagataccataagcaatcactctttaaggaaaatgataggagttgtccctcaaaaaatagacctgtttgccggaactattattgaaaatattacaataggcgagcccgacaggattgattatgaaaccctgatgaaagtctgtaaacagattaacttactatctttcatagaaaaacaatctaatggttttaacacctacattggagaaaatggagttttgctatcggccggccaaaagcagaaaattgctattgcccgggctttatacagaaatcctgaaatattacttctcgacgagccaacttcttcgctcgataagggtggtcatgattatgtgactgaaataatcaggaatttttcgaatgaaaataggacagtcgttgtaatttcacataacctctcaaatatcaatgtttttgacaatattattgttatagatgaaggaaaagtccttattgaaggaggatctcatcaggacttgttgaataattctgctttatacaaggaaattatcagtaggaagtaatatggagagatggaagccagtgatgtcaagcatctaaaagatcttgaatcagaacatactgagctcaaaaaggtaagccgaaacatcgaatccgcaccttgacagactaacaaatagtcccaaaacaacaaagcccgcgactagcgcgagctttgtaatcttccattgaaccattggatattttctattgtgatgctagacctgcgaacctaaagtatgcaacaattgctgacaggataaaaactacaatcaacattgggagcattttgtattctttcttcctgacgtgaacaaccacacctgctaacatgattgagcaaaaggctgccgctgccataggtgtcataattggtgcaatgcctgaaagccatgggactataatgccgatacatcctaataattccagaacccctaaaattcgaattggtattatagacctgctcggtttcaaatgtccgtctgcgatgtgcttttctttacttcctgcaatttttccataaccaggcaaaataaaaaatgcagagagaagtccctgtattatccacaaaattatattcatcttttcattatgaagttaaaaataagctattgaaagcgttgattgatgagcacaataagatgtccggaagacttccaggttgtctcatcgaaagattctactaaataaaaccttctttattcttaacttctgattagccctttctaggctgatctaaccaaagattgacatcttccattctatggagcaatttgtgataaattaggcaaatataataaataactatgcgacgaagagtatcgcaaaacaacagatttaaattatttactgacctctttgcgggaaaagactatagcgatgactgttggtacaatccgattcggattttcatattttagtaaaagctgagtaccctgaaatcggggctataccaaagggactcaactaaaaagaaaagcccgcgaccagcgcgagctttgaaatcttccagtgatccccttgggactacatcaatgccttatatatcgcggcttttcagggttttaaaagttagtgtaaccttttttgttacctcccggaatagcttcatttgatcaggtttgaaagaactttctatccttacaaagatacgaaagaaaagctaaaagactacaaaatgaattaggcttgaaccctacaaccctgtactaccttactttacacagtcctttgacttggttttaacacgcacttaatgccttaaatacaggtttacttcctctactttcagtccagtatattgacaaaactcagaaacacttatgaactgccctggattctttcccaaggcttcacggatacgttgcagcaaaagtcgggaggtccgctcactgcggccggtgatattttctatatcccgggcataaatcaccatgcggtgaggtattaatgtctgcaaattcggcataatcggaatggaaacttttttgggttaaaatgccggtttatgtttggtgtggttaatcacaaatttactgcattctgcgcagatgtgagcctaacgggcttggctatgtaaacagccctttttcttaatcttaaattgtttccaatggcaaaacaaatgggaataattcctttgaaaggtacgataggtaatatcactttttaccaatcaaaggccggacacctggcacgcggaaaaggtggacttaatgccgatcgcattgctacagatcctgcgtttgttcgtacccgtgaaaacggagcggaatttggcagggccggtaaagcaggtaagcttctgcggacggcgcttcgcgcaatacttttgaatattggtgatagctacatgtcttcccgtctaacccgtgaaatgatgaaagtgatacaggcagatgcaaccaatatcagaggacagcgtaacgtcattgatggcgaggctgaactgctgaaaggctttgagttcaatatcaacggtcgtttaggcggtacattgtatgcaccttttactacggcaattgatcgcgcggcgggaacgttaatagtcgatataccgtcgtttattccggtcaatatgttggctgggcctgcaggcgccacgcatttcaaagtgcaggcagccgctgctgaaatagacttcgaggcagaaaccttcgtcaatgggaatgcaagcagtgcagaacttcccatcgacgctaccgcaacggctgccatgaacctgaccgccagagtaacggacaatagcacaaaaccgctattccttacattaggcattgagttctaccaacaggtaaatggagcgctgtacagtcttaaaaacggtgctttcaatgccctggctgtagtagaggtttccggtatgccggctcctcccccgggtccgtaacgaaacgttagcctcgacaagaatgtccaggtaattcttaatctttaaaaagcgttttatggaattaatgaaacgtcttacagcatcaacaccacctttttttaccaaggtgcgtaacataggattgattctgaccgcaattagcggagccttgatgggtatgccagcattgccgttgatcatcgctaaagtagcaggataccttgctgttgcgggtacggtgatgactggagtaagtcaggctgccgtaagtgaaaaaggcggttagtattgcctaaaatagttctccggtttaaaggtgtggttaccttacggattgtttggtgtaaaggggctctcgcgaacagcgagagcctttttttatcctataagggattgtaattttgattttgtcagaaatgcttccactacagccagaacatgcaacttatcttcgggtaataattggtcgaagtgctgcaatttattggcttcctcttctgtaattggtcccttttctgcgtttatcccgttaaccaggtaatcaatggacacgtttaatgctttagccattttggccgccacgtctattgatggagtgataaaatccctttcgtatttgctcacaatattaccgctggtaccgatcaaagctcctaactcagattggtttatattcttctgttttcgcattatggttacacgttgcccgaatgtcatatcaattttttgattgggttaattcaagtcgcttgaagtaatactttaattaacctaaatctatgaagaactaagaagattgcaattacattataaatattaataatgaatattttgtactgataagtaaaatatagcttaaataatgggaattaattgtacataaacatacaaaaaagtacatttaatgcttgttttatattgtaattatacgtacatttatgtatcaataattacaatttagatatatggaaaatcgacacaaaacaagatgtttaacggtaggctccactatccatgagagattggatattgataacaggcatgttcctaaaattaggttgataggtttatggatagagaaagcaggatttaagattggagataaattgactgtagatatcgagccaaaccgccttctacttaacaggatagagcctgaaccattgccacctgtacccgaaaagaaaacacgacgtaagcgccattatctgtaatcacccctttttttgttaaccccgacaaccggacgcctgcgggcggaccgcatctttgatctttccgcccgcggggatcgggttgttacccaaaccatgttttaatgaaaaaactccgaaccagcgaacaacgattgtttgctgaaaaccttgcaaaactattcccgccggtaccgttatctgataacgaattgcatgatacctatacaaggttatgcaactttccgatttacataaaagagtatctgcgccgcgaattaggctggactgaatcccaattttcagaactggtactgccgccacgtccaggtagaaatatgagaccgacggatgaagaattactgaagatccgtataattgttaaagcgcaactctcctacctgttgcgatacctggatatttcaccaagtcttgtatatgcgccgaataacagcagtagcgctgaggtacaagcatacagtcactaggcatctcccgcttagcatttaacccctctttcatttttcaattcttattcatgttgaatgtttatactgacacctccgtaattggaggctgtttcgatattgaattcaaagaattcagcaacgcattatttgaagagttcaaaaatggcataaaacatctggttatatcagatctggtattgttggaactgagacaggctcgcgaggaagtaaccttaaaacttgatgaagtaccggccagttttaaagcagaacataaaaatacgccggaagcagtagaccttgcagaggcatatattgcaggcggagctttaagcaataaaagctttaatgacgcccttcacattgctattgctacacttagcaaagcggaagttttggccagttggaattttaaacatattgttaatctaaaccgaattaaattgtataattccattaacttacagatgggttatgcaatcattgaaatcagaacaccacgggaaattttaaagccaaacgaccatgaaaaaagctaaaaaatacgatgcggttgcagaggtccgtaaaattcgggaaaagttgagcgttaaatattggaaacaccctgaattgctatttcgtgacctaaaaactgccagtgacagttaccataatgaggcaaaagcccgagctgctcacggataaatcttttataggcgctctacagcctaataattaactaatcatttttataacattcctgtcagcgttatctgcctgctttatccaggcagataacgtattggctattattgggtggggccgtggcctggaagtaaccaattatcacgagacggccagttactgggctatcagtgagagcaattaaaaattactgttctatcaaacgcgctaacgtccgggagaatagatgatgggctactacagctgggcttatgatcaaccgatggtcaaagtgataaagctgagcctatattctatcgatgctcccatcatctgttctcacggacgccgcgcgatagtacactgtcgatcaaggtactgacgctggtgttcgcgcagcttattctcccgtcgcttaatcagtgttctgtcgttcagtgctataatctcccgctaaatagcgttactgtcgctcctccccgccgcccatccccccccttccgctgcgctccagagcgcagcggaaggggcgagcgaagcttggtgaccattagccaactgaggtcatagtgccccctttttctcgattaggtctatttagtattcaataaagccactttcagtaatagatttaataaaatatttcttatattagatacctatcattacttcttatgtcactcgacctcaaatccattggaaataaattgatgcgttgcagactgcaattgcaattaactttaatggacgttgagaaaggaacaggcataactagtaacaggataaatttggttgaaaatggtgaaatcgaggcaaccggtgacgagattttgatattttccgacttttataaacaggactataatttttttataagtaaccaaaaattatctgcctctgagcaagttgatatattatatcgacgatttgggaattccttttcaaaagaagatagatgggccattcaagaatttatatatttatgtgaatgtgaacagtttctatgggatcaattcaacaaaaatgaacctaagtttaatttttctcctattggaaattattataaaggtcatggtgaattgggagcagtagcattcagaacattcttaggatattccacccaaactattataaacgatatatattatgaagtgaggaaggctcaaatccatgtatttagaaggcgacttaagaactcgagtatttctggattatttataaatcatccctacgcggggaaatgtatcttagttaattacgaagaggatatatacaggcaaaatttcacactcgcccatgaattaggacacgctatttttgattttaacaatgctattaatatctctttccaatctgattggcagaagaattctgactatatagaattacgagcaaatacctttgcgtctaactttctcattccaaaagaagctttgaaatcactaaatgtccaagaatggactcaagaaattattttgtctgttgcacaaaaattaaaaacaaatgtaaaacccttgctgatctctttaaaagaactaaaattaatagggcagaatgagtttcaaaaattagagagagtaaaaattccaatttttataaaagaggatccagaactacaaaacttaactactaagcgcaaagaagcaaaaatgcaccttcttgaaagaggactttcagcattctatgttcataaatgttatgcggcttatgaggccgggctagtaacagaaagaagaatggctgaaatgcttctcacaaatgaatttgatctcccattaattctggggttattttcactgaaactaagttatggaaattgacattaaaaatttcaacacaatcaatgtagtcgattgctgctccgtatggaacatcctatcatctagccttttatttgctgcatcacaggaagcgaagtgctttttctctattacaaaatacgtcgaatatgagtgtctaacgaaaactcgaaaaactcaaaagaatgaggacgaaatcttacaaaataaacttaaggaacaactaaaaaaatcttccattcaaacatttagtttaagtatttctgatttacaagaggttgaattattaagagaaaggaagaaattaggactaggagagctttcctctatagcctttgctaaacgcacaaaacaggcgatcattacagatgatcagaaagcaagaaaactatcaaaagaggtgttaggactaaataatacacagacaactcctcacctatttggttggcttctgtattatcaacatttgtcagatagtgatttaccattgataattaaagagcataacctatatggagggccattggagttacttttcaatgaggtttaccttcattgcttgcatataagattgatgtttaaagatcagggtgtctgataattagctatcatgatagctaaaataaaatcactttgaataatttttcttatgaacataagcggaatagttaagaatattttagaattcggatttacggagttgacaacaagcgaagatgaatttgtaaatatcggaaaccaattgggcactccaatgaaaagcagaagaaatggagaggtcatagatttgctaaaacctacaacatccataaatgctagtcagcattctctctctcgattgtttggattatccgaatttccatatcatacagatggcgcttaccttttacgcccaccaaagtacatcttacttcgttacaaagaaggtgaagaagaccctacgccaacaattatactaccttttttattttttttgaatagcgacgacattgactatttaaggcgggaatgctggtcagtattcggcaggaattgggggttttattcaagtgttgtgaaccttgatattaatactaaacagctatttttacgctatgatgttggatgtatgaactgcatcagtaaagttagtttaatagaaaaaataattgcatcacaagttagccgaggattatgtgtgaatatttcttggagtcctggaaaaaccttgattatcaataattggatggtattgcacaaccgtcctagtgttaaaatgagcgaattagataaaagaacacttcaaagacttatgatcaatgactaaatttacctccgtctgggaatttgacctattatggtccaaatgtaatgtttacacacaaaaggctattagtgagtcacgtgagagtcctatgtttcctttttggtgtgctcttgcactagagtttttgggcagggctactctttcaaaaattcaccctgtattattggcggaccctagagaaggcgacaacattttgtatgtattcggcttttctaaagctgaaggtccacctaagtccattgcagctaaaactgtatttgatcgatgttttaaaatagttcctggctttaccaaaaaagagctagatgcctgtttaaaattaatagatcgcagaaatgaagagctacatagtggctctgcagcatttgcagattattcaacaaaacactggttggctgatttttataacgcatgcaaaatacttttggaattcctaggatttagcctagaaatactgtttggaaaatctgaaggaagtgcagcagaggaaatgataacagaagttgacactaagcttttgaaagcagtaaaactcagcataagtaaatttgctaaatcattcgcagaattatcggatgctgaaaaagaatctaaactcaaaatgggtagtgaaaaggcgctggagaatcataggagtggcacaaagatagaaaaatgtatttgttgcaacgcagacggcctattggccggcaaggttgtttctgtgtcgcaggataaacttattgatggagatattatttatgaaaggataatccttcccacttcttttacttgctatagttgtgggtttaaactaattgatcatcaagaattagttatcgctgactacggaggacaatttactgaacaggttgtatgggatccatctgattttcatgggatatctactaccgaaattgacccggctgacctttatgactatggaaatgattgatttctgctaatattacttcttgggccaaaatgcgtgtttgaaatcttctggattatatggtgggatttcattaccacttttaagttggcgattggtccattccagtctctctatcatatatgggatccatcgttcatcgcggaataggtgcaaaaaatgatttatcgctgttggttcctgctcctcggaaatcagtaaatatactaagtatgacaaagaaatgcctttccccgaaatagcattagtatgaccatgatcagacatgaaaatctcagcaaatcttataatatctttttttctggaatttaggtagtgatttaactgaagtatatttgttatttgtaagtggctcaattctttaatatcctttagacggaatggaattttccgatctaatcttgatttaacggattcagtgatacctttatcaacctcatctattattggattaactttataaaaagcatctaaagattctttattaagatctactttttctggatgtagaagtatttctcgctcgagtatagatctataacgagatagatttgacttcagtcgagaaaattcaatgtcagctgtttccaatagtgccgcgatacgagcgaaatcacgacggataatgtcaggtatttcctcaactcccttataaccaatatcgtgctcaatttccgcccatgcatgctgcagaattgaccgaatctgtatctcgaaagaaaaatctttgaaaggtcggtattcagttaaagcagctcgggcatcagatattttcacaacatagtgaagtgatagatagccaaactggtcaaatttcttcatgcgtttatccactgaattttccttgtccaccataaactcccgtgcaacaagatccgcgacaacatcaacctggtcttcaaacatggtaataatcctaatcccaacaaggtcagtaatctggttgagatccgtatacttatttttgattttaatcttggtctccaaactatctttggtttttactcttccagaaatcgtatgcacaggaatgtcactagatgcacacaggtcctgaatcaaagctcttacttttcgctccatagattgcaactctttgacagaaccttgatatgctgttaaaatcccgttgaaggtactcatggataagttattaagagtaattttattttatttcaaaatagagaacgtttcttgaaacatcacattcctatctatcacatagaattaatcaaatgggagaagtgaagaacctgataaagcacccagccacttaatagtaattaacatacatattctcaaatttacatgattaaagtttatttatgtaaatgaccttccgtagatagttcgaattaacatattctccatgttaaggtcctcaaaaacaaaaactatagccactagattaattaaacttaacccttccattgtaaggacatatgccgtaagcttctggatacagccaattacctgatgcggccactattgggacatcagtcagaacaactaaaaatcactgccggctcaaacacgttagcatctgggagaatagataatgggctagtacagctgggcttatgatcaaccgatggtcaaagtgatacagctgaacctatattctatcgatgcccccatcatctgttctcacggacgccgcgcgatagcatactgtcgatcaaggtactgacgctggtgttcgcgcagcttattcttccgccgcttaatcagtgttctgtcgctcagtgctataatctcccgctaaatagcgttactgtcgccccgccccgccgcccatccaccac

SEQ ID NO: 17 - DNA, 78574 bp, Chitinophaga pinensis
  source 1..78574: mol_type = genomic DNA
ggaatttattttgattttaaaaagatttggggagatataagcggatatccgcttatatctccccaaatctttttaaaatcaaaaatgatcaaatctgcaaaatcagtaaaatcagcgtaatcctgagaaagacaaaatccgctacaataatttcatctcgtcaatcaaccgcgtacagcccgcgtatttgtccacgataaacagtacatagcggatatccaccatgatattccggcaaatggaagggtcgaagttaatatcgctcatcgtaccttcccaggtgcggtcgaagttcagccccaccaggtggccgtacgcatccagcgcaggactgccggaattaccaccggtggtatgattggaggcaatgaaacacaccggcatcttgccattggcgccgtaacggccatagtctttcttcttataaagttctattaaccgggcaggcacatcaaattcataatctcccggaacatatttttccatcacgccatccaggtaagtatagaaatcgtagtgaatagcatcgcggggattatagccatctacttttccgtaagtaacccgcagcgtgctgttggcgtcgggatagaagctttttttactgcccattacatccatttgcgcctgcatataagtgcgttgcaggttgttgatgttcgactgcagatccgccagcgggcggcttacattatccacataacctttgcgcatagccattaccagccgggtagccggatctttccacatctgcgccaccaccgtattatagggttgttgtacaaaagcggttagtttatcgatagaggttaagccggatatcgcatatagtttatcagtcaatgcgcggctgtctttgttgttttcctgccagatctgtgcaaactccgcccctgcaaattgcgccggaacgcctttggcatacaaggcaatcaggctcacagccacatcatgatctacctttgcattgtaattctgataaaatccctgcatagatgcgaggaactgctgccgcatggtttcatactgcgcttctcccctttcatgcacatcgttgaggaaggtgatgaggcggtcgccgacagtgaacagctccacattttttaccagctcactgtaatagtcgcgggcctgtgcataaggttgcacctgctgatagtacccgttgagcgaatccagtacgccgttgtacttttgcttccataccgggttgctttccagctgctgccggtaaacatcttcatactgtagttttttacctacgccgttggtttgctttacgccctgcatttctcccatccatttcttccagtagttggcggtgccggcgaatttagctgcatactggatttttatctgcgggtctttccgcatgtagctatccataattttgagggcggcatcgcgcatttccactttggcggcatcgagcacctctacggtttgctttactccttcggagggcagatattcggtggtgcggccgggaaaacccatcaccatagtgaaatcattttgtttcactcccttcagggaaatggtaagggcatatttaggctttaaaggcacattatcctttgaataaggcgccgggcggccatccttaccagcgtagatgcgaaacatcgaaaaatcgcctgtatgacgcggccaaacccagttgtcggtgtctgatccgaacttaccaatggaagaaggcggcgcgcctaccaggcgtacgtcgcggtaagtttccgttacgaacaggaaatactggttgccctcataaaaaggctttatcatggtttcctgccagctttccctgcgggcattctggcggatttcgttcaaacgtttgtcgatagccgactgccgctctctttcgctcataccgggcgttacatcctgcagggcggctttggtcacgtcatcaatgcgtacaatgaaggtggcaaacaaaccggggttaggcagttcttctgccgccgactttgcccagaacccgttttccaggaagttattttgtaaggaagagtgcttctgaatggcgtcataaccgcagtgatgattggtgagcagcaatccctgctcagagatcacttctgccgtacaaaaaccgccaaagctcacgatggcatctttcaggctgcctttgttaatattgtaaatatccgcggcagtgattttcatgcccattcccttcatctctttttcattaagaccggaaagcagctgtggcagccacattccctcggtggcataagtgtgcccgccaagtaccaggagtaccaataaaagcaccggtttcacgattcgttgcaacatatctgatattctttttataaaagaggcaatttactataattcggggagcagcgaaaagataaccccatgtttccgatcattcatcgacataaacccgcgatttacagagaagacagctattatccggctggaaagtcagaatttcagccctatatctatctgtcgcaaatgttccggttaaaatcttcggtagtaatagcacacattacagggtggctgatatgcctgagtttacccctgctgtttgtcagtgggcaaacgggcgaccgcaaagcgctctctatcttattctcaacagattacctggtattcctggtaacgtatgtagcactgttctattttcataccaccttcctgtttcccaggctgtacttccggaaacaatatgttctttacttcctgtctgttttactgttgctgatcatggtcaactatatgcggccctatgatcacctgttctcgttgtcgcatccgcgtggagaaatgccatggcgccagcaaatgccgcccggggcagcaccaggcccgcggccggaaggaatgcggccacccggccgaccacacaggcccatcgacattgtaagcgacttccttttcctgctcaccattgcactgagtatcgccatcgaaaccacacgccgctggcggcaaaccgaaaaaagagcactgtacgcagaaacccgcaaaacccaggcagaattgtcctttctgaaagcccagatcaatccgcacttcctgtttaatacccttaacaatatttactccctcgctatcacacgcagcgataacaccgccatgagcatcatgaagctctctaacatgctgcgctatgtaaccgaggatacgagagatgattatgtactgctggaaagcgaaattgattgcctccgggattatattgatctccagaaactccggctcaccactaaaacgaaagtcaatttcgcagttaccggcagcccgggcattaagtgcattgccccgctggtactgctacccttccttgaaaacgcgtttaagtatggcgtcagtaatcacgaaccgtctgaaattaccatcctgctacaaacgtccgaaaacaggatccacttttactgcagtaataaattattcagaatggcgccggacacaagccgcacgggcattggcatttccaacacacggcaaagactggaacacctctatcccgataaatacgaactgcagatcagtgaagataacggcgcatattctatttccttacaattacaggtataagcgatggagattaaatttattgtgatagacgcctgccttacaggtgatcaaaacctatgcacaggaatttccctggctgaaattacagcatacttttacagatgccatttccgcagcggaatacctgcggcagtattaatatcatcggggaatgccatctgcgtagttcctttcagtttatcattcacgtatacctgtgcatgaatatgcgttaccctgccttcataccagcccgggtaaatggaagtaaatttaacctgcccggctgtatccgaatactgcaatcccctgcagaaaaccagcgcggtattatcctgcgtaccgaggtatccccggttgctgtagccggaataataaccatccttatcgcaatgccagatatctaccctcgcgttggcaagcggcttgcagctgttgttggtgttcagaatgttaatggtaatgtgcaacggggtacctgttttgccatcggtgatatccacgcgctgaatggaggagcccctgctgttgtagagtggatagggaccatctgtttcttccggggaaacggtacaggcgccgctgctgctatctgttccgggatcggcagcatcactttttttacaggcttcaatcagcaccggcacagcggtagcgctgataaacagttgtttcaggaattgtttacgggagttttccatctcatcatttttgatctgctataaaggttttgattatgtaacagatttacaaaaaagatagatgaaccggccctatgtaccggagaatagcatttccggagcggaaataaaatcccggctccggaaatgttttaacagattagctcatgcaacgattagtgatacagataattaagcgcaatgatatcattggcattaaatgtacggttgccgccattggagcaggccagcatccaggagttggcatccggtgcagaaggagtgcccggaatatatactgcgcctacgttgcttgcgccttcgttggtggcagtaccgccgcagctgtaggaacggtccatgtaatcggtatgacgcataccaatgcagtgaccaatttcatgctggataacagaacctacatacaatacgttgggattagatccgtaggcgtactggttggtgttcatcttaatggtgccatacggattaccaccgctggtaggaaatccggaagaaccgagtgtgatgtaaccaccgcttggtccctggttaaatcctctgatggtaatgtcagcggcgccgctggttacacgctgaaaggtcatgcgcagccccagcctgttgtaacgtgcaatggcagtgtcagtgcctgcgataaaggcagtacctaaactggtcaccttaattctgataacgcggggtaatgctgtaaccaggtaattagtgcggtactgttctgttttggccacccgtaaaacagggctcgtaacggtttctttcaactgtgcagctgtaagcaggatgtcaccttccacaaggtagccatcttcggtttttaccacgttctctgtgctaaagccatttgctttaatctgggctaacacttctgctgacacgggatcgggctgcgcttctttttgtgcgccgttcttctgacaggacgcaaagaggaaagccgctgccatgcagcagagcacaggaattgattgtgttctcataattcagatttttggttttggtttagaaaaaaaagttcagatttttggtttagattttaaaaaaagatatccctgtcgcctgttttttcaaacaggccactgttaacaacactaaatgcccgcgctgatctgtggctgaataagacgcggaataaaaacaattgcgtactaaaagcacattgttttttttcttcttattgccgcaaacgcgatcgcccagctttgattatcttccggaaactgcagttgtgatactgtgctctcgttttcggatacatacaacagctaatatgccctgctatggcatagcatcagtttttaatgggttggtagtgattcagtaatgccggttatttccggtgactaagatttgctctatcaattaagaaactgtgtaacagattcagatcgttgttcagatttagttgaattttatattaggttttcctctttcaatattacaacattcgtttaatttaaaaaaaatattttgttttagtattgataaaaaattgtgttgaaaatctaaatacagtagctttaggtagcaacactaaaccaaaatcactcacccgttgtcgacacctgcatgcggataataccctctaaaatatggcccttgctgtttttgcagctttgttatttttactatgctgctgcacagcgatcacactatcccgacagcctggtgcaacggtatgctaccgatacattttcattgcaacggaaaagtggtcctttcctggtgaagtttgcaaaactgccaaatgagtcaaagctgcagcaatggggacttgtacagcctctctcccgctatcattacatattacaacacgtaccggaagatagtacgctcgtatattgttacagtgcaggttataattttaaagcaagcattccgctgctgcaacaactggaacaaacatccgcgcgggatagcatcaccatacaggtgtcgtgccacccggcagaaaagcaattaatgtatgcccgcgtgcagtcgtactccacgcagtaccacgtagccagggcaaaggttaaaaagcaggactggcccttgtttatcagtcaggcggccatacagttcgcagaccttatccggcgaccaacccctgaaattattatcaataccggcaacctggcagtgaaccggatccctttcgcacaacagcaatttccacttatcacaggaaaacgtgtaaccgtttccgttaaagaagatttatttgataccactgatatcgatttacagggacgatatattccttcttcctataattcctccctccaaaccgcgcatgctttgataatggctacgctgattggcggcgcgggcaacagtggtgcaggtggcaaaggcgtggcgcctgaagtaaagctgagttctgcagactacaacagcagtctccttccggatgatgatgcctattatcaacaatccggcatcacggtacaaaatcactcctatggtaccggcatcgaaaattattatggcgccgaagccgtggcctatgatcagcagatttatgaagcagatactttagtgcatgtctattcttccgggaacattggtacatcaccagcctccggcgggcgttaccagggcattacagggtacgctaatttatccggcaattttaaacaggctaaaaatattattgtcagcggtggtacagatggcgccgcccaactgatcgcactcagttccaaaggcccagcctacgatggccgcattgtcccacatgtaaccgcttatggcgaagatggcacctccggcgcagcagcgcttaccagcggtgtggtggcattactccaggacgcctggcgtatgctgcacaacacgtccgtttccgccgccctcatcaaagccgttatcattaacagcgccttccggcccgcaggcgtacatccatcatttggcagcggatatggcaacctgcacgcatatggcgctatcaaaaccatacaggacaaccgcctcctccagggcagtgccggcaaccatacggctacgtccttcaacatcgctgttccggagggcatacaggaggtgaaagtaaccctgtgctggaatgatccaccggccactgttaataccgttaaagcgcttataaacgacctcgacataacagctaccaccgccgacggcaaaacctggctgccgtggacgctgagcacctatccgttaattgattcattattgctacccgcaaaacgtggcagggatagcctcaacaatacagaacagatcagtattgaaaatccggtgcccggcaatgtgcgggtgcaggtatccggcgcacaggttactgccggcacacagcctttctacctggcttatgaactggtgccggtaaaaaccttccagtggcaaaaccccgccacaggcactacggcagccgcaggacaggcattgccgctgcaatgggaaactacgtatagtggtaacagtgagctttcctacagcagcgacagtggccgcacctggctccccattgcacaaaatatcccggtagaaaacgggctgtataactggaacgcaccggatattttcagcccggtgatcctgaaactaacgttaacggatacctcgtttatcagcaaccctttttacatttcgccggcactcaccatgcgcgcaggatttaactgcatagatacggtactgctgtactggaacggacaaccgggcgcaactgcataccagttgtacaccatgagcaatacggcgctgattccgtatagccaggtccatgatacttttgtttttatccccaaggctacggcgtcgtcgttgtattttgcagtaagccccgtcgctgcgggcggctggacaggcatccgcagctatgccgttaattacacgcaacagggtgtaggctgctatgtacaaaacctgctggccgatcctactaccgataataaagtagccctgtcgctcacactgggcagcacctggcaactccaaacggtttactgggagcggtttacacgggaaggctggataacgctgcaacaacagcccgtaggcgacgccatgaactttaactacctcgacgacaccgcaccggaaggactgctccgctaccgggtgaagttgctcacctccaacgggcagtatatttatgccgacccggttactgttaccatcattgcaggcaatcatatcttacttttccccaaccccgtaagcagccagttcaccgttttggatggcaccccacgcagccgccaactggtaattacggatatgagcggacggatagtattgcagcggaatcttgaggatatccaggaaaaggtggaagtgcagcgcctggcaaatgggatttataactgtagtatttatgcagataataaacggatctactccgcacagtttgtaaagcagcaataattgctgcacaatgccgggttatgatgagcttcctgctaaacaaaacagctgctccggtaaaccggaacagctgttattatacttacaatgagataagactacaggtgaattgcttcgccgtaagctacttctatggcgtcttttacagattcgctcatagttggatgcgggtggatggaatccagcacttcctggtaagtagtttccagtttacgtgctaccactgtttctgcgatgatttcagtaacgttggcgccgatcatgtgggtacctaaccattcgccgtatttggcgtcgaagatcacttttacgaaaccttcagtggcaccagctgcagaagctttaccggaagcagagaatgggaatttacccactttcacttcataaccggcttcttttgctgccttttcagtataacctacagaagcaatttcaggtgcgcaataagtacagcccggaatgttcatgtagtcaattggttctggtttgtgcgcatatttcttttcattgtatgcgatagcttccacgcagatgataccttctttggaggcaacgtgtgcgagggcctgaccaggcaccatatctccgatagcgtaaacgcccgggatatttgtctggtaatatttatcaaccaatacacggcctttgtcggttttgatacccattccttccaggccgagattttcgatattggcagcgatacccaccgcgctcagtaccacatctgcttccagggtgatttcgccggtttgggttttcacttttgctttcacaccgttaccacttgcttcaacagcttctacagaagcgttggtcatgatttcgatgcctttctttttgtatatcttttccagttctttggagatgtcttcatcttccactggtacaatgcgcgggaggaactcaacgatggttactttagtacccagggttgcgtagaagtaggcaaattcaacaccgatagcgccggaacccacaacgatcatggatttaggctgctgagggagggtcattgcttcacggtagccgattacattcttaccatcaatcttcaggtttggcaactcacgtgcacgtgcgccggtagccaggatgatatgttttgcgtcgtgtacagtggctttaccgtctttatcggttacttccacctggcctttggattttacctttccattgcccattaacacgtcgatcttatttttcttcatgaggaactgaacgcccctgctcattttatcagcaacaccgcgactacgtttgatcaccgcctcgaaatccacttttgcatcaccgatcgtgataccatagtcttttgaatgctgtgtatattcaaaaacctgtgcagtttttaacaaagccttcgttggaatacagccccagtttaaacagataccacccagactctctctttccactactgcagttttaaatcccagctgagaagcacggatagcagccacatatccgccgggcccactaccaattacgattacgtcgtatgccatattgtttaatttttaaattgaacttgccaaaggtaaataaataagcagaaagcacaaagcctattgcaaaaagccaccggagcggagattacggggatgttttgcaacatttaccgctgtaatccgcgctccggtggcttttatactaaaatcttatactatcgcagatctactacttccacgccagggtaatttttggcatcgaaagtaaaggtagcatcgctcaggttggtatttggtgtaaaattggtgatttcgtaagtataatggttaccattcttctcaaacaccttcatcctggcaatgctctggtttttcttatctacagaaacaatcaccttaaatatagtcttagatttatctgtaggcgtcagttccacattctggaacaccttacctttttcctgcgtttctgcttccagtttgtacaggtaatctttatcgtagaagttggtgaacagtttggccggtgtcatggcgccactgctctgatccacgttattaatagttacttcattcacatctttcgcgtatgtccaggaagttttgttatcgctgatgatttcctgtcctggcagcgttactttatatttagctcccttcaggtaaacagtaccttttttggaatcagacacgctgttattagcgccttctacttttaatataaaattagcgactactgtttttaatgacttaaatttattactaacaccatccagaacggtttttgcctttgggtcggaagcgcccttagattgtgccatgccgctgaaaatgataccactcaacaacattccggttaatacaaatttcttcatcgtagttttttttagtttgtgctatccaacaaagacaaatgccatgccggtatagccgtgtaggtttttacagggtgcaaaattcattatatttcctgaaaaagggtaataaattccgaccgccttaacatattataacaaattattaaggatttcattcagctcgctttctgttttcaccagcacatccctggccttgcttcccatattggggcctacgatgttggcggcttccagctggtccatcaggcgccctgcacggttgtagcccagcttcatcctgcgttgcaggagggaggtggatccctgttgggtggtaacaatcacctgggcagcctcttcaaacagcggatcccggtcagcgatactcagttcgcggccatccgggtccttgtcatccacgtattccggtagcaggaaagcatcggggtagcctttctggttaccaatgaattcagccacgttttccacttccggcgtatccacgaaggcacattgcaggcgtaccagttccccgttgaaggaaaccagcatgtctccctgccctatcagctgttcggcgccgccgatatccaggatggtacgggaatctatttttgaagataccttaaaggccacgcgggccgggaagttcgctttaatggtaccggtaatgatgtttacagaagggcgctgggtggcaatgatcaggtgaatacctactgcacgggccagctgggccaaacgggcaatcggcatttccacttccttgccggctgtcatgatcagatccgcaaactcatctaccaccagcacgatgaacggcaggtagcggtggcctttcagcggattgagacggcgttgcgtaaacttaccattgtactcacggatgttgcgggtaccggcttctttcagcagatcgtaccgcaggtccatttcaatacacagggcattgagcgtgtggatcacctttttggtatcggtaatgatcgcatcatcttcaccgggtaatttggccaggaagtgtttctcaatgagcttgtataacgacaactccacttttttcggatctaccaatacaaacttcagctgggaaggatgctttttatacagcaatgataccagcaaagtgttgataccaacggatttaccctgacccgtagcacctgccatcagcaggtggggcattttggccagatcggcaataaagttttcgttgtcgatctttttaccaatggcaatgggcagatccatggtgctggtctggaatttttccgaggccagcatatttttaagagatacgatggttttcttcacattgggtacttcaataccaatggtaccctttcccggaataggcgcaatgatacggataccgagcgccgacaggcttaacgcaatgtcatcttccaggtttttaatacgggagatacgaacgcccgcagccggcacaatttcgtacagggtaacggttggtcctactgtggcactgatcttctgaatggaaatatcatagtttttgagggtatcaatgatctggttcttattcttttccagttcagcggtatcctgcacaatcactttgtctgcattatgattttccagcagatccagggtcgggaacttataatctctcagatccagggacggatcgtaaggatctaccggttccacgggccgtgtgggcgctatctcttccacttcgtcttcctcgtcctggtaagtgggttttatttcgaaggccacttctaccggttcccctttctttttgctgacaggggcaagcggttgttcgggcgtttcttctatatacaataatggtcccggatcttcttcttcctcttcttcctcctcctctgcaggctgcccgttttcgtaagcaggttcggcaggcaggtaagctgcatgggcagaggggatcacggtgatgtcttccctttccaccaactgcataggtggcaggtcttcctcgtcttcttccggttccgcatgcggcgggattaccattacgccaccgtcgtcgcggagaccgtttttacgtgcgtcttctttcgccgaggcggcgggtgttgccgcagtggtttgcattacaggggccaccggtgatgtggcgggtatgggtttgggtgcttttacttttttctccggccatttgaagtcgaagttgaatttccagataagccaggagaagccaacaaccagcaacagcagggcggttcctgttttgcctacgaagccggtggtccatttattcagggcatcgcccagggcgccgccccaggggaaatcgccgccgccgatggcaaaggccattgtcatgctgataaagagcacaccaaacaggatatattttatactgcgccagatacggaatacccggcggccaacgatgaaatttacgccgatgataaaaaagaagtagcagaacaggtaagcggcaatacctacgccataaaagaagaagttatgcgatacataagcacccaggcggccgagcaggttatctacttttacatctccaaaaaataattccctggtagaataatggaaaattttatcctggtcatcttcccaggtaaaaagataggaagtgaaagcaataaagcagtaaacagacaataaaagaaagaacacgcccagtaccttgtgggtgcgctcatcttttaccagctcttttaccttcacctcgggctccttctctttcttcaatacatccgggttcggtgcggggcctttcggtggtttcttgctttccggtttttcggttttcagtttattcttggacatattataatttcagatttgggactacctgtcctccgacggcggcaactgtaagatccagtgtgccataaactcgggaaccaggggatcaatggtttgctccagctctccgtattcgttcacttcacatgttttgcagcgctgaaacaaatggtttaatccatcaaacttacggattgttgtgagcagattaccattttcgttcaatgcgcgttcaatttctttcagattggcggtagcatccacctgtatatctgcggtgccgttgattgccataaacggacatttgatctgtttcaggtaggtcagcggcttatatcttaataacgaaatagtttccggactcatattggctctccgtattaattcatcctctgtttgtaccttcttaacgtcttcgcttgaattacggtatatatcccggagaatttcctgtgcccttggcgttatggctacgatgtcgctgtcgcttgccaggaggtcccagtatggcttcatgcgtgcctgttctgccaggatcaggctatccggtttgccggccactttccctttggcgaaagcttgctggtcgatcagttcccggccgcttatgcccactcctgccatggatattacaaaggccactcccggattgtttgctgccactatttgcgccacaatagcgccttcgctgtgtccgagtacccccatccgcgaaatatccacatccttcctggctttcaggtatttcagcgcggtgagcgcatcgtgcgaaaaatcgtagatatcggatgtataaaaatcgccggtggaagcgccaaatcccctgtcgtcgtaccgcagggtagcgataccgttacgggcaaaatagtcggccagcaccaggaaaagtttatgccctgctatttcctcgttcctgtcctgcggaccggagccggagagcaataacactacaggatacttgccctgagctgccgggcggatgaacgttccggcgagtgttacactgtcttttatgttattaaacctcacctgttccgtgtaatacgggaaaggcggctttggttcctgtggtcttttgtacatctcgccggccgtaatttctttccggccaaggtcggcatgactttgatcatcgcccaacccggtaatgcccctgaactgctttgcagccgggtcccatacaccggtaaaagaaaaccgcatcccgtctatacgcagcaacagggtatccttgcgatacacgactgtttcaatctcaaactggtcgtcgtccgacatttcgggcagctggagtgttcctttatagccctcgccgtcttttgccaggtctacgatcatacggtatttatccccgtaatatagtttaaaggtgccgtaccatttaccggcaatatttgcattatcctgcgccattcccactgaccctgtcagtaaactcacgatcaacacccaaaaacctctgtacatatacgagaatgctttatgcttttaattttaagactcctgccagcaggcagatccagccggcaataaaaaacacgccgccaacaggcgtaatgatgccgatgcctttcagacctacgttgccggtagttttgagcagcgtcatcagatacagtgaaccggagaacaggatgatgccgataatgaagcatctgccagcccagattaactggttaccgggcacatgagcaaataagatgccggtagcgattaatgcaaatacgtgatagaactgataagtaacccctgtctgaaaagtagatacggtttcgggaggcaccagctcttttagtttatgtgcgccgaatgcgcctaaaattactgccaatgcacctaataccgccgcccaaactaaaaaactcttatgcatattagaaattttgcgtaaaggtatccaatgaaatattatcagatgtaattatatgcttcgattgctggtaaaaaggaagacgctctgccattttcttctctacaaacccggtcaggtcttcatcttccagaccggcaatcaacggccgtttgaattttttacgttgcaggcgttccaccattacatctacagaagggttgatccagatggtagtgccatgttcgttcataaaatccatattctcctggaaacagggcgtgcccccgccgcaggagatcaggaagttttcctgctgggataactcccggagcagctgactttccttttcacggaaataatcttcgcccttgctggaaaaaatatcagcaatggtcatctcctccgcttccacaatcacttcatccagatcgtagtaaggcagttgccagtgatccgccagttgtttaccccaataggattttccggcacccataaaaccgagtaaataaatcttcataaataacgcgacagtgcttaataaattcgttcctcacgcaggatgagtccatgccaggcataggtcattttccataatatattgcaaatataaccgggtatttgtatcctgtttgttaaaatcggcggtgatgaaaccggcctgttgaaaaacaaagggatgcaatttcatattctccttaaaatcaacgcttccccggccataccatttaaacatcgcttctttggcgctccagcagattgttttatgcgacagctcctgtttgggatcgataaacgaccgttctgaaggcgacaggaacttgtgagacaccagttctattttaggttttacctcttcaatgtctatgcccaccgctgctttggtactaacgatagcggcagcataatcgccgcaatgtgaaatggagaagtggtggctatcacctgccaataccggtttacgggtatgtgtaaacataatttcctgaatggggaattccgggaaaagcgttaccagcaaatacctgcccgcaaaatgctgtaagcgtttatgcggatggtgaatagcccggctgatgcttaccttttcctggaaaaaattttccgtttctgttatcttccatacacccagcttcgtttccggatcaatttgtatcgttcgtattaatggcatatcttgccaaattaaagcaaaaaagcagaaaaaacagcttttggcagcaggtctttcactaaatgccaacagctgaaaaataaaagctaacaatacagctcactaaaactaaacgaacctaagcatgattctgtcagacaaacggatattggaggaaattgaaaaaggcactatcgttattgctccctatgaccggaaatttctgggtaccaattcttatgacgtgcacctggggaaatacctggctacctacaaagaccgtgtactggatgcgcgcaaacacaatgaaattgatcattttgaaattccggaggaagggtttgtgttacaacccggcaccctttacctcggcgtaacagaagagtataccgaaacgcatgcacatgtgccgttcctggagggcaaatccagcaccggccgcctcgggatcgatatccatgccaccgccggtaaaggcgatgtaggattctgcaacacctggaccctggaaatttcctgtgcacaacctgtacgcatatacgcaggaatgcccattggccagctgatctactttatggtagaaggcgaagtagaaacgctctataacaaaaaaggaaatgccaaatataatggtcgcaccataaaaccggtggagagcatgatgtggcggaatgaattttaaataaggaagcagtcagcagccgccaatggctaactgctgactgctattttcaactcatgtgcttctgtaatggtgggcacttccagcttcctgaccaaccgttccatggctgccgccggcactacttcctcccgctgccggttttgctgtaacagcttcgctgccggcacttccacatacacaattgttaccgctgcctcatacgttgtaaaaagactgatcacctgttccctcatctgccgtgtaatgttggtggcgttccatacaaaggattttttttcccggagatagatcctggcttgttccttcgcagcctggatcactacaccattgccgcttttatcagtaggacttattttcatggtttgccggatatgatccagggagatgaccggcaggtgtttataatgccgctgtatatacgtgtctttccccgcgccaggtaatccgctcatcagtatgaccggtgtttgcggcgtttcaaagggcacatagtccggtgagctgccggtttttaacaggtattccatgcgcgcctgcggtgtggcaaacgggcgtggttgtccccagcagttattttcccggcacaactcttcgaagcaatccagccggtagagcaggtctgcctgatcggcacagttgcgcccaagcgcatcggcgcgggccagcaatgccagcagctgtgtattcacttccaggctggcggtgatcagcgctttctgcggatccggcttttcaaagatccatagcggcaggccgtggtacctcaccagtttggcgatttgctcgcggacaaggaagggcgccggcacatccccgtaaaggatttgccgggcccgcgcttctcctttgcgggcatgacccgcagaagtgatgcgaccatccggttcaataaccgtagtgctgtatttttccacgtcgtgcagcagtgcggctgcccacagcagttcctggtctgccgccggcaattgccggtagcccggcaactgttgcaaggctgccagtaccatctgcgtatgtacggccacgttaccttctgcgtggtgccgcgcgtcctgcggaacttcctgcatcacgcgcacccattcaaatgtatgttccaggtgcgaccagtttttattttcactgagctgccacatagttacctccttcattatttaacctggcacggcgccaatggcgggtccagtgctggtctgtttttacatgtcctttgcggacatacttaaacacgttgtctgcaaaatcgcttaccgcatacccgttggcattgcgggatacaatgccttccatggtagcgggtttaccggtatgcacgtcgtgcggatcaaaggcgccggaaccgtttaccagccccagtatatcacgctcaaactcctggcgtgtagccggcggcgttatacgctttacttccggcaccaccggcaggccgagcattgccgcgtagaattgggtttcctcccaactgagccactgctggccttcccggatgccgaatatataaaagtgatgatccaggttgcggtattcaatagaatgtaccgcgtaaagattttcgaggaagatctccaggtcacccaggtcgttctttatgctttgccagtagcggcggatgctttctgtccacggcgaagtagtgggcgctgcatgtgagcgcgcaaataccccgtaccgggataagcagttattttctccgtccagtttttccgtatggatcagcaccggtatctgctgcaacgattgccagtattcatattgaatacggtcgtcgctcgtagtgccgggcgaaaacggataatgccaggtacggccatatttctgagaaattgccatgtcatcagggtttaagttaaacaatagtttcacaggccggttccgggatggaacggcgaaaggaatgatttaatatgcctgtgaaattacatggctcaagtgtttgcagtttttaatcaagtacgccgcaaaagtaaagaaaataattaaatagtatattacacaggcttttgaaaacaacaacaatcatcttctgcaaatgaaaaaattccttctttgcgcaaccgccgcagctgccctggcagcctgtaataacggcaacagcagcaaccaaaccaagggtaccgacagtacgctgaaccaggctttcagcgcctaccaggcacattttattgacgccctctggaaagaaaaccccgactgggctaccagtgtgggctatcataaatacgactcggtgctggtagtgccggacagcgcggctgccgcagcgcgactcgcatttgcgcagcaacaactggattccctgaaatcctacgatcccgctgcattgaatgacgccaataaaattgattaccagctgatacagaactacctggaatcggtacaatggggtattaaagagcagaaaagcaacgaatgggacccatcttcctataacgttagtaacacgtttgcctttatcttaaatgaaaactacgcgccgctggaaaccaggctacgcagctttggcagcaggttgaaaaatatcccggcttactacgaagccgctaaaaaacagatcaaagatcccgtaccggaacttacttcgctggcaatagaccagaacaacgggggcatatcggtatttgaaaaagactttgcagattcgctgaagaaaacgggtatcccggcagcagagcagaccgccatgctggccagtgcccaaactgccaccaaagcgatccgtgattacgccgcgtggctgaaggcattgaagccggagcatccgcgcagcttccgtttgggcaaaacgctgtacgatcagaagtttaaatttgatatccagtcgtcctttactgccgcgcagatctatgattccgcgatagcacgcaaagcttttgtgcatggtgaaatgacaaagatcagccgccagttgtggccgaaatattttggtaatacaccgatgccatctgattcgctggagctcataggccgtatgatcgatacgctttctgtgaagcatgtgaagccggaagagttccaatcggccatagaaaagcagctcccttcgctgattgcgtttatcaaagaaaaggacctgttgtatattgatccgtccaaaccattggtggtacgtaaagaaccggcttacatggcaggcgtggcaggcgcctccatcagtgcgcccggcccctacgacaaaggcggcaacacctactacaatgttggcagcctggaaggatggccaaaagataaagcagaaagttatttgcgtgaatacaatcaatacatcctccagatactggatattcatgaagctataccggggcattatacccagctggtgtatgccaaccaatcgcccagcctcattaaatcgctcatgagcaatggcgccatgattgaaggatgggccgtatatactgagcagatgatgctggaaaacggctatggtaataacgaacccgaaatgtggctgatgtggtataagtggaatctgcgcaccgtatgtaataccattttggattacagtgtgcatgtaaaagatatgagcaaggaagatgcaattcatttgctgaccaaagaagcgttccagcaggccgcagaagcagcaggtaaatggaagcgggtgagtgtatccagcgtgcagctgaccagctatttcacgggttacaaagaaatcattgatctccgcgaagcttacaaacagcagcagggcaaggattacagcctgaaagcgtttaatgagaaattcctgagctatggcagtgcgccggtgaagtatattcgccagttgatgctggctcattagcggatgttgtctttctcaggattacgctgattttattgattttaaggatttgaacactttggattttaaatgatttggggagatctgagtagataatttaagataaataagcggataaaagatttggggagatatgagcgggtatatccgcttatatctccccaaatcatttaaaatccaaagtgttcaaatccttaaaatcaataaaatcagcgtaatcctgagaaagacaaaatccgcgtcaggtgtcgcacgtaacatcgtcccagaactggttcctgtagttggtgagccagttgagggcgtagtgccgttcgtatacgatgccgggatgcagcggttctttttcgcctttcaagcgggcgtctacacaggcccagttggcgcggtagtagaggtcgttggcgtcgagaatttctgtggcgctgcgcaattctgtggcgccggccaggaatgctgtgggatcggaggcagggccgcggaagggaaaggcttcttccggcaccatatcgaggttgcagagggcgtccatttcgccgagagacggtacttttttcaatgcccagagcaatacccagatgtcttcacacttccaggtttcccgtgttttggcgtcttcctgcggatcttccaggaaggctctttcggcgggtgtggttttatcccagagctgatgttgttgcaggtagctgataacggtggggctttcgaggtatccgaaggccacggtgtttacggcggcgagtacggctacccgttgggctgtttctgcggcggtgcggagcacgacttcctgctcatcgcggataacaggaaggttgacggttgttttcacctgcatttcctgcaggagctgtatgttccgttgttttctttctgttgcggcggaggaaggcgtgtcctggttatcgaaataccgtgcgttgatatttacggtgagattggtagcggtagaatgaccatttacatcgagcagcagtgcgccggttttatcccagaagccttgtacttcggtgttgaagatgaagttattttcgcagaagaagatgccatccagttcgtcggccaggtccatgatggcggcccggaggtcgccgttgaaggagggtgtggcgaggataacgatttccgtattgagcgtcgctacttttgcgagcagcagttctttcagggccgggttttctgccggcagctgctgtacaaagccgtacatgccgagcaggttggtggttaccgggtcgtcgttccgtaccagctggtaaccgggcgtggcgcgttgccggtagttgatggtgagggtatgaccttttcgcagcagttttttccctgatgtgatggtcagttgttcccaacggttcgccggtccgtttactttcactgcctgatctccaaaatgcgccctcatacgggtcaacactttctccatttccacctcatgcgtatagagcgtacaattttccatgctatttctttcgagggggcaaaggtagcttaaagcggttaaagatggtaccggatttgccttattacaggaaaacggacgacatacgcatatttattccaagcataaacattttcatatgagtaagcgatcattgcctgtactggctgccttcctgttgtttatagctgcgagctgcgtgccgccgagacgtccccggccgcctaaaccaccccgcccccgtgttcaggttattttgcctttttcgctcccggccggttctgcagcaggtggaggattttattcagcttaaccgggtcgttgatgtaaggcgacaggtcgaacagttctactttccggaaggccaccgggtgactttcgctttgcagggagatagagccttcggataacagtttaccatcttttaacagtcctggttgcggatgggaaacattgcccccgcccatttgcggtttattgtatacaataacagtatcgccttctacaatgtgtttaataacggagtcgcgcagcaccagcgcttccgcgcgcacccaaacatcgccctggtatgttttggaggtggaactgatgcaatggtctttgataagttttccattcattaccacattggtgcccggcgtacacaggttggccgtagagcggggatcggtgccattaccgcccagtaattgttcttccagcgaaatggggaagtcctggtctttggtcatgctggcggcagtttgtccgtgcagcatgataccactgttacggaaagcccatccggggccgccttttacctggtcgccggtaaatttatattctactaccaccaggtaggcagaaaagttctttttatagaagatgtgtccatattgttccctgaactcgtcataattttcgtagctcactttcagcatgccgctgtctacccggaaggtattcccgaaattatcgttcaggtcatgcccggttattttaacgtcccagtctttcaggtccttgccattaaagagttttaaccatttattgggtgcaatttccttctgtgctgagctatggaggccggccagcagtaatagcgcggtgagtgcttttttcatgtgttcttttatttaccgggttaagatagcctatcgctgagagaaatgcaagatgtggttggcatataattcgtgctgccacaatcatatttactttcttatgaaaacactgttacgtatacttcttcctttgggagtactgattagttccgttgcttacggacaggaaaacggcaactggcaaaacgtgctggagcagcaattacaggtattggccactgcggcgccggaggactggccaccgcggatagaaacgcttaccgcattggcggaggcgcatccggaggaatggctgctgcagtattatgcggggtggtcggctacacagttatcgtttaagtcggataaagcggctgccgacgcgttgtgtgaaagggcaggaccttttgtgaagaaggcgctttccatgcaaccgggtaatacggaaacgctgacattgatggggtattggctgtctgccaggatcaatgctactccttcccgcggggtttccctgggcagccagagcaggagttatgcagaaaaggctattgcggctgattcttcgaatccgcgggcatggctggtaaaagcgttgaatatttactatacacccgctatttttggcggcggtaaacagcgggctaagccgacagtagatattgtggcggccaagttcgccgcattcagaccggataatgcgctggcgcctaactggggtcagcagatctttgatgcgctgatggcttcctaccagtaagcatgttttccccttgtgagcgtagtgtgtaagaaattacgcaccgtatcggatgtgccacaggaacataagagaagccatcatatttatcttgctaaatatcaataaattagatcatttaccacaaaagtgcagggttttagctgtaagttccccaaactgtatatatgagttccttaacacaacaacttagttttcaagatccacaacaaccaaaagcagggtccatatatgatagctccaatatcatcaatgttacacccgaaggccggattgtctctattttttccggtgcatggctgctcggcagcgccatcagtaaagtagataaatcgcctgtatccagtcttttaaaactcctgggagccggttacctgttatacagaggtatcagcggtaatgacctggtaaatggatttctgggtaaacggaaaccggataagcatactgcgtctgtaaatatcaggactaccatctctattgataatccgaaggaggaggtgtattatttctggcggcagctgaacaatcttccggtgtttatgaagcatttgcagtcggtagaagaaacggatccattccactcgcattgggtggtaaaggggcctggtggcattggtacgctggagtgggatgctgaaattgtgaaagaggtaccgggagaactgattggctggagatctttgccggggtcctctattgctactgcgggcagggttaccttccgggaaacctttaacgggggaactgaaattgatgtgatgattacctaccggccaccggccggatatgtaggctccgggctggcctggttgctgaatccggcgtttgaaaatatgctggtaaaagacatcaaacgtttcaaaaattatatggaaaccggcgagatactaaagtagttttacccaataaaaaagcggagataatgaaccatctgtttgttatctccgctttttttatgtgaactatcattacgacaatgcttctcttctgaacctgttgtaaacgccctgacttttattaatcagtttcagcactctttggcgggcgtcgtcctgcaggccggttatttcgtgttcgaatacttctttcagatccgacagatcttctccgccttttcctaccaggccattgatcttatggcgccaatcatctgctgttgttttgatttttttgcgggttttatcgccgctatcaggggctgttaataatccaattactaaaccggtagttaggccggctatagcacctgcaagaaatttcgttgtagacataatttctggatttttatggtttaacaaatgatttgtgtgcatggttcattcacacggtaaccagaaattttcaaatatcaggccagtaaaagtaatgagcgaagatccgatcttaaagaaatgttattgtgtaaaataaagggaggaaaaaccacctgctaagagagagtaaatgtaccagtatcaatatcgtgaaaattcgaagggaacgctatccaggacaacatcagagttgacattgtcccggcaggtggataagataagcgtattagataatggaatttataaaagtcaaacggagcagtaaaataattacattctggtatttttcaaacctttttgaaagaaatgaaataataaattttattaaaaagtaaatcctccccggaaagtaaataccagagaggatttgtgtgttccggcacaatattatacaatagtcttatatcttcggtataatacctttttagcctgaatatctgaaaagcaccaggtatgaaaacggaatgttaacaggaagataacccttgcgtataccttaagaatacctccattatgctttgactacgctttaaacacgctttatccatgcttcatccacgcctttgaggtggacttgatgtggacttgatgcggaggtgaggtggacttgatccggtctactttgcatccagcatattggaaaccaggcggttaaagtcggcctggaattgttcataatgctcacctgttccggggccggaaaagccggtatgaacctcctgcacgttcccttttttatcgataaagacagtggtagggaagcctttgatgccagtgagctgcgggagcgttttctctcctttctcaggatcagcgggcgttacgccggtgatcagtaccgggtagtgcacatcaaaacgtttcaggaagccttccagcgcatgtttcgacttttcgaagtcggtggtgcgttcgtaggccaacccgatcacttccacgccgcggtctttgtttttctcataccatttgctgaggaagccggtttcgtccatgcaattagggcaccaggaacccatcagggtgatgatcaccactttatttttgaagcggtcgtctttgatactcaccttgttgccgttgagatcggggaaggtgaaatccagttgttgctgaccaggtttcatggtggcgatggttctttcgtcggggagtttggcggtatcatttttcacggccgaccagtactcgagtccgtcgccgataccagcgaagaagcgaccgtttgtgatgctgtctttccccacgcgggcggtaaacaggtaggcgtgggagccgtcgaaggtagaaaggcgcagggtatcgccatccaccacgccgtccaggaagcggtagtcgccggtggtggtgaggaacgtgccatgcacggtgttaccggattgtttaaactcaccgatggcggtggaaggggctttgtccttatcttttgcagatacgaactgtgttacccagcggccggatacattggcggtggccggtgtatttacggcgaagcgttctgctttgcctgcgacggcagagaaaggaatgcttacgtccttatcggcgaggtgcctgatccaaagtccttctgctgcgctgtcggaggtgagcttcgctttaaattccgagtcgaagaagggcattttaatcaacagggagtcgccggttacagacacttcatctaccagtaatttatctgtcgcattcagcacgtacagcacctttttaccagcggtagtatcttttacttcaaagttgaaaacgatgtctgccccgtcggtgcggtgcagtttggcctgccacacaccattggcggggtttttagtagactgaccggtattgcaggcggtgaaagccaggcttatacccgccaggaagatgcttaattttttcataagactacgtttgtgaatagttcctttcgccaaagagcaggctgccaatacgcaccagggtactcccttcctgcagggcgaggtgatagtcggcgctcatgccaatggacaattctttaaaggacgcttcgttgttaaagtaagtggttttaacggatccgaataactcgcggagctggtggaactcttcccggatctgtgtttcattggaagtattggtagccatgcccatcatgccggcaatgcgtacctgtgaaaaagcggatggactggcctggtatgtttgcagcagttgctgtaattcctgcgtatccataccaaatttcgtttcttctgctgcaatgtgaacctgtaacaggcaatgaatgatgcgctgatgtttagcggcctgtttattgatttcctgcaacagtttaagactatccactgcatgaatcgtatgcacaaatggcgcaatgaatttcactttattggattgcaggtgaccaataaaatgccattctatatctgccggtaaaagtgtttgtttttctgttagttcctgtacgtaattttcgccgaagatcctttgtcctgctgcataaaacgcagcgatatcttccactggcttcgttttggaaacggctaccagccgggcgtgatgaggatggagccggtcgagtacttcgtggtatgctgctaaattgattgccatcgcgcaaagatagtgcgaattttgtctttctcaggattacgctgattttactgattttactttttggattttttggattttataactgattaaaatattagggagatatgagcgaatatatccgcttatatctccctgatctttttaaaatccaaaaaatccaaaaagtaaaatcagtaaaatcagcgtaatcctgagaaagacaacctccgcgaaaatctacgctaagatgctccggctgataacgatgcgttgtacttctgaggtgccttcatagatctgggtgatcttggcgtcgcgcatgaggcgttctacgtggtattccttcacgtagccgtaaccgccgtgaacctgtacggcttcggtggttacccacatggcggtttcagaggcaaaaactttggccatagagctgctaagggtatagtcctggtcctggtctttatcccaggcggctttgaggcataacaggcgggcgccttctatgcgggtggccatgtctgccagcttaaactggatggcctggtgctgggatatttctttaccgaatgcttttctttctttggaatatttcagggccagttcatatgcgccgctggcgatgccgagcgcctgggaggcgatgccgatacgaccgccggcgagggttttcatggcaaatttaaacccgaagccgtcctctcctatcctgttttcctttggcacttttacgtcctggaacatcacgctgtgggtatcgctgccgcggatgccgagtttattttctttggcgccgatagtgataccgggcatttctttttccacgatgagggcgttgatacctttacttcctttttcaggatgggtttgcgccattaccaggtatacgctggccgagttaccgttggtgatccagtttttggtaccgttgagcaggtaatgatctcctttatcttctgcgatggtacgctgggaggtagcatcagaaccggcttcaggctcactcagcataaatgcgcctattatctgcccggaagccaggggcaccaggtatttctgtttttgttcttctgtaccaaaagcttcgagaccccagcaaacaagggagttattcacactcatcaccacggaggcagaggcatctatcttagaaatttcttccattgccagtacatatgagattgcgtccagtcctgccccaccatacttcgggctcaccatcatgcccaggaagccgagttcccccagttttttgatctgttcagcagggaacttctggtgttcatccctttctatcacacccggcagtaattccgcgacagcaaagtcgcgtgctgccttttgtatcatcagatgctcttccgtcaattgaaagtccatggttttaattttatgtggtaatccactcaaattatttataaatcatcagctaaaaaaatagcccgattaaaattcaacgttgtcaaccagaacaggcgaaatattgaacaaatcgctacaataacgctactgtattggatttgattcagatattatatacaagtttttcaccattacacgttctgctgctttgggcgttcacataaaatcctgtagcttgcctgtaatgctatttttatgaagaatattaaaataatagaagtaaaatcggaaataggagcaggtacgcgtggcgccagtttgggtgtggatgctattaagattgctgcgctggactttatgagcaacttttttgtacactttcccaccgaggccattgaaacggaaaataagctattgtttgaacctattgaatcgccctatgccaaaaggatcaaaggcacttttaacatgtacgagcgtatcagcaagagtgtatgtgaaacggtgaaagcaaactggttcccggtattgctttccggcgaccacagtactgccggcgcaacgattgcaggcctgaagatggcacatcccaaagccaagctgggcgtgatctggatagatgcgcatgctgatctgcatacgccttataccaccccttccggtaatatgcatggtatgccgctggctacggctattgcggaagataatatggattgcaaggtgcatgacctggatgagaatactgccaaaatgtggaatgccttaaaaaacattggcaaaatagcgccgaaggtacttccggaagatattgtatttatttccctgcgggattatgagaaagaagaagattacctgatcaagcaatatggtatgaaggtgatcactaccagtgaagtacgccggaaagggccggaaaatatttcccgttccgtgttccgttacctgagtgattgtgagtacatctatgtttcttttgatgtggacagtctggatgcttccatttccaagggcaccggcacgccggtaagtaatggactgagggagcgggaagcggaggatctgattgccaagttcatgcagcaccgtaagatctgttgttttgagatcactgaagtaaaccctacacttgaccgtgaaaacctgatggcagaaattgcctttaatattttacagcgcagcgtgaatgtgctgatgatgaactgatgtttgttataatttaaagtaggcgataagccagccggtgacttcgctgtagctgcggatccctttctcttgtttattagctttgaggtagcggtcgtacagcagggaggaatacgcatctacttttcccgtatagggttcataaaaatcgatgatcgctttatagtcggcttttacgccgggaagcgcccttttccagatgttgcgggcgagggtggtatcgcggagggcgagctgacggacgctataaagaaacatatcaaaattggcggcataacggaaatggctatccggaatgctggttgccgccaggtaacctacaaagttcgcttcttcttccggtgcataccctatctggtgtgcaatttcatgacaggaaacaaatggcagcaatacatccggaacggtggtattgacctgtgcttcgttggtaaacgggttaaggtagccggtaacaccggggtaattaagccagtgcccgaacatagccggttttatgctgggtgctttataacgcagggctggccaggttttggcggctgcgtcgtaagcggcgacggctctttcaaaaacaggtttgccggtggtatctgttttcatagtgccggtggtatcgccggtattggttttttccaggttgacgagttgcagtaatgtatccgataattgataaagctgttgcgtattataagtgccggtaacaaggtgtgtatcgcgggtgagtgagttgcgttcgtagttaaaaccccatagcacgaggaaggcgagatacacactcagcaggaactgaacaccgcggagcagttgaaaacccagggcttcccagcgtgcgcggatgagtttataacatagttttaacaaatagagtattcctccgataatccaggcagtatatattacatcgccaatactgaatggaactatacctgttacttgtctgaacgccaaactactccaatcgtaccacctatggaagtagaaatcgctgaagcggttactccaggcgaataatccttttaacaatagtatagccgtaagtgttagtacaatacggacgattttctttttaatccggacttttgtctccatataatgtggcggaacatgatagatgaaattctacaaaaacagttaagcgcagcactttccgaacatttgaaagtaaaaatacatattaatgatgcaaaaagcgtgcatggtggcgatattaacgaatcttttcgtataggcaccaacgaggggtatttttttatcaagatgaacgatgcggggaagtacccggatatgtttaagcaggagtatgcggggttgctggagttgcaggctgccaaagcgctgcatacgcccagaccgctgggttacgggagtgtgaacggaagggcttacctgttgcaggagtttttgacgaaggggcaggctgtagctgatttctgggacgactttgccgtttcgctggcgaagcagcatcgtgtaacgcggcctcattacgggtatgcgggtaccaactatataggaagtttgaaacagtataatacgccgtacagcagctggccggtgttttatgcgtttaaccgtttattgccactgatccgaatggcttatgaccagcagctggtagaccggcagctggtgcagcaggtagagcggttgtgccggcggttgccgcagatattcccggcagaggcgccggcgttgctgcatggtgatttatggtcaggtaattttatggtggggagtaacgggcgggccagtgtttttgatccggcggtgtattatggtcacagggaaatagacctggcgatggcgcggcttttcggtggttttgacacgcggttttattatgcgtaccaggccgcttttccattgcagccggggtggcagcagcggataggcatttgccagttatacccgttgatggtacatttcatcttatttggcggcagttattacaacagcatgaaagaggtgctgcaatcgtattgattattcgccgggggaatcgataaagtcgcgcattttgccatattcttcttccacgagcggataatagcggtttacatcttcccgaatttcatcaaaaagccggcagatttctgtgctgtgcagttcctggttgacgcgcagataattttccagttcctgcattttggcgctgatccaggtgaggcctaccatagcaaaattcggctttagtttatgtacctggaatttcatggcttcccattcgtggttatccaccattacctgtagtttggtgatttcatcccggatggttctgataaaaatttcaaagaggtctgcggcataggaaatattgctctcatagagatctgtgagatatttgacatccaaatcgttgttaaactcaaatccgcttaagttctgcacttcttccattattagttctgtttcgtcttcgttgagatatttattaaaaatctgtaatagctgatccggtgtatagggcttggtgagtatatctgttattccggcggcccttgccatggtggcggtgctttccattgctacggcggtggtggcgattaccggcgtggccacattcggttgttcctcatctccccttattttttgtgccagttccatgccattcatgccggggatacggatatccatgaggataaggtcgtattgccttgattcgaggaaccaggtggcatccgggccatttgtggcgagctggtagttgatcttatatttttccagcaggctcatgatatagcgcaggttcatctggttatcttccactaccagtacccttgcgtcttcaaatgagcgttgcaataatttcctgctcagtttaccggcatttgccgtgagtggccggcggctatccaggaaggggatattgaagctaaagcaggtgttaaagccggggagttcttccacggtgatggtaccaccctgaatttccaccagttgtttaacgatggcgagtcccaggcctgtgccgccgtatttctcgcggatatcgccttctgcctgtttgtagctccggaagatgagttccagtttatcctttttgatgccgatgccggtatcagatacccggaagcgtatccagagtttattttcctgccagctttcctgggtagcggtaatggcgatgataccttcgttggtgaacttctctgcattacctaacaaattgattagtatttggttcagtagtacatcgtcgccaataagccaggtatcgagcgcagcgtccagttcggcggttattttaacggggcggcgtcccagtttgagttcaaaagtgttgcgtaatgactggatcagttcccggaggttgaattcgcgttggttaacctgtatttcgcgggcttctatgcgtgaaatatcgagaatatcgctgacaatgcccagcagtatgccggaggaatttttgaggatattgacatattcctgttgttgcgggtccaggtgggtttcttccagcaggtgtgccatgccgatgatggcattgagcggtgtgcggatttcgtggctcatgctggcgagaaaatctttctgggcgcgctgggcttcttctgcctggcggcgggctgtttccagttcctgctgcagttttttctgatccgtgatatccatgtggatgcctgctccgccggtgatgttgccgtggcggtcgtaaatattggtggaactggcgagaatccagcgattggagccatctttcagctttatttccatgtcgtatacgaggggtacattttcatcgaggcgttttttgcggagggcgcgggcgaaggcgcggttgttttccggtacaaaaacgtcggtgatgttcctgccgatgagttcctgttcgttatagccggagaggcggcaaaagctttcgtatacgcgggtgatattgccttttacgtcggtttcgcacatagcggcgttgagattattgaggatgaccctgaatttttcctcattgcgttttatttcttcctggacattgtggcggcgggtgatatcgatggcctgccagatgctgccactgaaaatttcgccgttaaatacggggaggtagttaatttcccagatgtggccgttgcggaagggcacttcccagccgaaccagggctttttttcccggcggagggatttcattttggcttcaagcggcacataatcggccaccattggtttgaggtagcggatcagttcagggtatgagcagttcagggggatatttccatccatataccggctgaatatgtcatttacccatatgcagcggtgcttttcgttggtcacgagcaggcctgcgctggtgctgttgagccaggcggttatgggcagggaaaagaggtccggtgcgccatttaatggcacgccggtactaccagttattttcttactgtattttcctgtggccttcatcgttttgatggaatggggatacgggttttcaataaattcgttgaattgtgaaaatcaggtataagataaaagctaattacgtacctttgcgcctcacgcctggatgccacaacatcaatatggctgatattttatgatataaatatatatataaataagatatcgttggtgaacaaatttatgaaatttttgcaattgcaaatatttaattacctttgcatccctctaaaagtgaggatattgatatgaaaccactccgcgaatttgatatagcctttgttggattaaacccaggggaacattcatttcactatgctatcggggagcgtttctttgataatttcgaggagccgagggatttcagtgattgtgaggtgagtgtaaatctcactttagacaagaagagtaacttcttcttactgaaatttgcgataggtggtaaggtaaccgttacctgcgaccggtgtggagagccctttgagatgcagctatgggatgattttaaccagatagtaaagctggtggagaatccggaagagctggcaagtggagaagaagatccggatgtatcgtatatactgaagacagagagccatttgaacgtggcagaatttatatacgagttcatccatctgagcattccaatgcaacgtatacatcccgacaatgcggacggcaaaagcgggtgtaatccgaaagtgattgaaatgctggagcaaatgaaccagcaggcaaaagaaaacgataacccaatctggaaaggattggataaatttaaggacaattaaaaattaaataaaatgccaaatcctaaacgcagacattctcagcaaagatcagcaaagagaagaacgcattataaggcggtagcggatacattaagcacagacagcgcaaccggtgaagtgcacctgagacaccgtgctcattgggtggaaaacaaactgtactacagaggaaaagtagtgttggaaaaacagagcgcagctaaataataaattattttactatttttacccgagctaacaagaacaaaccttgagttacatgagaatcgggcttgatatgatgggtggcgatttcgctcccacagaagcagtaaaaggagtaaaattatatttagacactgttgcatctgaggtgcatctggttttaattggagacgaacaacagttagctcctttaattgcagccgcacagctggaccaatcaaaatattcagttgttcattcatcccaggtaatcgggatggatgaacaccctaccaaggcgctgaaagagaagccacaatcctccatctctatcggttttcatttattgaagaatgaaaaaatagatgctttcatcagcgcaggtaataccggcgccatgatggtgggcacctattattccattaaagccatagagggagtgcaacgtcctactatatctactctggtaccccgtgaaaacggcacgtacggcctcttgcttgacgtaggtatcaacgccgactgcaaacctgaaaacctggcacaatttgcccttctcggatccctatattccaaacatattcttcaggtacccaatcctaaagttggtttactgaatatcggcgaagaagaaggcaaaggcaacctgcttgcgcaggcaacttacccgctgttaaaagaaagcaaacaaattaatttcgtcggcaacattgaaggaagggatatcctctccgaaaaagcagatgtaattgtatgcgaaggctttaccggaaacatcgtacttaagatggccgaatcattccatgaaattgcgctgagacgtaatatccaggatgactacatgaagaaatttgactctgaatcatatggcggtactcccgttttaggcgtttccaaaccagtaattattggtcatggtatttcccaggaaactgcctttaaaaacatgatacaactgtcgcagcaaatgatcgaaagtaaactgctggaaaaaattaaagaaagctttgtagcgaaagacgacgcacaacagcagtaaacagcaagaaattattttgaagacgctctggtattccagggcgttttttttgcgtatacgatcgccttcggcgattttaaattgtcttggagcaggattacgctgattatactgattttaaggatttgaacacttttgattttaaaagatcggggagatatgagcgaagattgctgcgaattttgtctttctcaggattacgctgattttactgattttactttttggatttttttggattttaaaaagatcagggagatataagcggatatattcgctcatatctccctaatattttaatcagttattaaatctaaaaagtaaaatcagtaaaatcagcgtaatcctgagaaagacaaaattcgcagcaatcttcgctcatatctccccgatcttttaaaatcaaaagtgttcaaatccttaaaatcaatataatcagcgtaatcctgagaaagacaaaacccgctgcattagcgcccttgcagtggcagctttacgtagaacgtagtgccttcgttcagcttcgtttcgaaccagatctcccctcttgcctgttcagcgatgtttttacacatggccagtccgaggccggtgccggacgacttggtggtgaagttgggaacgaaaatgcgggattgaatctctgtggaaatgccttcgccgttgtcggatacgctcacgatcacgtgattgtcggacgtcatttgcagccgtaccacgatctgtcctttacggtcgtcggggatggcctggatggcattcagcaacaggttggtgaatagcctgttcatctgggttttatctgcaaatacataaaaatcgtgtgcgggttggatgtaggtaacttcacaatcttcatgcccctggtacaaggaggtgagggaatacaatacttcattgagcaggaattcttcgttgttgggttcaccgatgcgggcaaaggcagagaaatcggacgcaatattagacaggtgttcaatctgttccaccagtgtgccggctactttgcgcgacaactcctttacattgggagaatcgccggcgatagcgcgttgcaggtattgaatgcttagcttcatgggtgtgagcgggttcttgatttcatgggctacctgccgcgccatttcacgccaggccccttctctttcgcttttagccaggcgtaccgcacttacttccagcttgcgcaccattttattgtattcttttaccaacgcgccgatctcatcatctttatcccattctatttcatcgttgcgctgacccaggtttacgtgccggagcttttctgttaccagcgagaacgagcgggtgatggaattggtgatcagcaacgccaccattcccgcaatgaggaaaatgaaagcgttgaaattgatgagggccacgaggaagttggagatctgctggttcaattccgtttgtgtggcgaaataaggaacgttcaggtaggcgatcacttcatgtgtatcatgattgcgcaacggcatgtaacccgacaggaacggcatcaccccaatgtattctgtatggataaactggatctgttccaaccggtataagctgtagaaggcctgcggatctatcttcgtggagattaaacctttatcggtcatcatcggctgcgtggtttgctgcaggttgccatcacggtcgtagatattaatatccagggccctttcattggcaatatccgagagggaggccgacagctttttcatcagttctgaatcatacatatcccctacctggtccaggtcgcgttggttttccaataccttttccacatctttcgatacctccctcatggttttgctgagcctttcccggttctgcatttccgagcggtagataaagaatttgatggtggtgatacccaatatcaggaaggagaaaataacaacaaagatgatggtgccatgtacttttttgcggatgctgatattgatcagtgcccggaggttgctgatccgcattcttgctttgatgagcaggtcgaatgctttatatacggcgatgatgagcaggaacaggcagaacatgtaggcgaacagggtgatgaattccacgaacatcctgttttcctttaccactatcactactttttcgggggtagcgcggtagatcagttctgaataacctttgatggattttacggtaacatctgcggctggcagttcatgcgcatataaacggaccgggaacgggaagtcattgttattgcttacgagaatgcctttatcatatacggcaaatgaataagcgcctgcgtattcgcggcccggatcgctcatatccccttccaccagcagttccggataaagccgttcgctgcttaccggctttggcgccagggtgtataccagccagccggtaacttctccgttggcgttgtgaaactctttttttgcgatatagctgtagtcgttgaagctgcgttcataataatacaggtcgttgccgggcaccagtgcaggagaggcttccgattcggtaaatatctgccggttaaaagttaacaagctaacggtatccgaagaaaacagggaggcgccgttttcgtcatatgcataaatgttcacccggaagcggctcaggtagccctggaagtatttgggcaggaggagggtgtcgaacgccgacttacggtggatcctgctgctgcggtcctggaaaaaaaactggatggcctcatcatgttctatctttttaccgatatcattcagcagcatttccaggtaaggatccttttgcttggacaggtcttctgcgagcttctgacgggcatacagctccttatgattgttataatgtaccagtgcgccggaggtggtaatggtgagcaggaagagccagaagagaaagggtacggtagccatactgctttcaaagcgatctgcgagaaagtcgagcagcacgatgtaaatcagcagccagatcaccattgtaaccgaaaacggcagttcggggttatggatacggaacagcagccagatgatccctacagccgccagccaaatgtatttggtgcggtactggaaattggtgagttcattcagcaggtagttgatgatctgggagaagaacaaaaagctgaaagatataaagcccagtaccatgaagccgataatgctgtagatgatactgtattctgtaagactgaaggggttggtaacatcgaaagaaatcttggaatctattacaaggctctggatgaggtctgccaggaattgctccacgatatagaggatcaggctggcgatgatgatcaccacgctttgcgcccatctttttttgagcaccggcgggttgatagtttttacgtgttcccggaagaagaggaccatccagaaggtgagtaatacgttgatcagcagatcgccgagtgagtaaaagatttcatcttttgcatagatcctgggatcgaagatattgagttccttcaggttaaacggaaacgggtatacgtagctgagcacccgcataccgaacacgataaggaacaggaacaggaagccatacagcgggttggtgctttttgccagcagggtggcaaagaggttgaggaatatcagtacgcagatacagcccagcacccgcagcaatatgctcaggttgttggaggggtgtacgtgcatgccggtgttgtaatcgaggaagaacagcgtttgttcctgcccgttatttaccggcaggataatatgttccggcaccaccagggcgggttgttcccgcaggatgctgtactcctctcccagttcttccttgtcataaaagtgattgacgaggtagttgttcttaatggcatattccatgcggacgggaatggctgccaccaggtattgggcgtggcccggggctgatttcaccctccgggtgatgacttcgtaatagccatttttcagcttcatgaaccgctcgccgttttccagtgacgtttgcagttcttccggctgtacctggctggtattccagaacgtaagccagatgccggtgttattggaatcgtaggcaaagaggtagtactccatgccggtaagtttgtccagtgttttctggtcgtagctgcgccggaggagggaggcggtgaggccggtatctttaacgagtttttcgaatgttttttcgcgttggtggatactcttttccatgctgcgcttcacgccttgcggggacgagtagtacgaccagtagttactgaacaggaaagcgaaggtaaacaaccaggctgcaatgatcaggagatagccatgtcgcaggaaaaaaagccgtatttctttagtatcgatcaatgcgggtgtattaaggaactatttataattgctctgtggctttcaccttattccagagtgtatccatttccgttaaggtcatatcgttgagggtacggccctgttccagtgccagtacttccattgcctggaagcggcgctgaaactttttattggtgcgttcgagggcattttccgcgtcgatattaaggaacctggaatagttcaccaaagagaacatcacgtcgccgaattcatcttccatatcatttatattcccgctgctcactgctgcttccagttcatttacttcttcttttaccttatcccacacctgtgcggtattatcccattcgaagccggtttgtttggctttttcctggaggcgcatggcctttacaagcgcggggagcgacaggggaacgccactgagcacggattttttaccttctttcagtttaagcttttcccagttttgttttacctggtcttccgtatcggcttttacatcgccataaatgtgcggatggcggtggatgagtttatcgcatacgccgtttatcacgtcgtttatatcaaatttttgctgttcagagcctattttggcgtagaacacgatatggaggaggatatcccctagttcttctttgatggacttccagtcttcatcggtgatggcatcggccagctcataggtttcctcgatggtgagctgacgaagcgtttgaatggtttgcttgcggtcccaggggcacttttcccttaaatcgtccatgatctgcaggaggcgatcaaatgtagctgtcttttccatattttgtaaaaatagggatcatttggggattttaatattcatagatgattccgggcaggaacgggtccggagaaccaaatgcggacgtgtaaaaatggggaatactttttcttggtaaaaaggccattttagttacatttgcgagctattaaatggtagcgatttcatggtttggagatggtaatttttgtaattattgtggttacaaaaccggcatctggcaatcaaaaaatcccaaaatgtattgatttatgaatccgaaacacattgcgcttatttcatcggagttgggtatttccggtaaacaggcagaaaacaccatggccctgttatctgaaggctcaacggttccattcatcagtcgttaccgtaaagaggtaacgggaagtctggatgaggtgcagataggccgtattgaagacctgcagaagcgttataaggaggtggatgaccgtcgtgattttattatcaaaacgatcactgagcaggaaaaaatgacgcctgagttattatccaaaatagaaaacacctgggtactggcagagctggaagacatatacctgccttacaagcctaagcgtaaaacccgtgccacagtggccattgagaaaggcctggaaccgttggctaccctgttgtttgagcagcaggacggtgatatttcggcggcggaaacatttatcaatgagcaggtagctacgtctgaagaggcgttgaaaggggcacgtgatattattgcggagtggatcaatgaaaacgcggagtgccgtgataagctgcgtaagttatttgccaataccggcaagctaacgtctaaagtagtagaaggaaaagaagccgaaggcgataaatataaagactatttcgagttttcagaagatctgcgggagatgccttctcaccgggtgctggcaatattgcgtgcggagcacgagggtatcctgttcagctctattgcgccggtagaggaagatgccaatgcattgatcagcaaacaatttgtgacaggtaaaggcaaggccgcagaacaggtaaccaaagcggcggcagatgcttacaagcgtttgctgcgtccttccctggagaatgagttccggacggctgcaaaagaaaaagcggaccaggaagcaatcgaagtatttgcggaaaacctgcggcagctgttgctggcagcgccactgggaccaaagggcgttattgccattgacccgggttacaggacaggttgtaaaatagtagcgctggacaaccagggcaatatgctggacaacgatgttattttcccgctggaaaaaaattacaaaagagatgatgcagaagccctgctgaagaagtgggcagctaaatatgataccgaagctattgctgtgggcaatggtactgcgggccgtgaaacagaagagtttgtgaagaagattgattttggcaaaaagatcaatgtgtttatggtgaatgaaagtggcgcatctgtatattctgcttcagaggtggcccgtgaggagttcccggagcatgatgtaacagtgcgtggcgctatttccattggccgcaggctgatagatccgctggccgaactggtgaagatagatccgaaagctattggtgtgggacagtaccagcatgatgtgaaccagtcgtcgttgaaacagagcctggaccgtgtggtggtgagctgtgtgaacaatgtgggtgtgaacctgaatacggcatccaagcacctgctggcgtatatttccggtttgggcccttcccttgcggagaacattgtaaagtaccgtaaagaaaacggcgcattcagcaaccgtatgcagctgaagaaagtgcaccgtttgggagataaagcgtttgaacagtgcgcgggctttttgcgtattgagaatggcgataacccgttggataattcagcggtgcatccggagcgttatgacctgatcaaggaaatggcggccaaacaacacagcactgtacaggatctgatgggcaaagaagagctgcgcaagcaaattaacccgaaggattatgtgagtgccgaagtaggtttactgactttggaagatatcctgaaggagctggctaagcctagccgtgatccgcgcgacgagatctctatttttgaatatgccgaaggcattcataagatggaagatgtgaagccggggatggtgttgccgggcgtggtgaccaacattactgcttttggtgcatttgtggatattggtgtaaagcaggatgggctggtgcatatttcccatctctccaataaatttatcagcaatcctaatgaagcggttaaattgaatcagaaagtgcaggtgacggtactggaaattgatgtggcgcgtaagcgtatttccttatcgatgaaagacaacgagaaaggcggtggcggcggttcccagcagcagggagccagaagggagtcccgtggcgagcagccgcatcagcagaagaaggtgaataagccggccgctaaagaggcgccgctgaacgacttccaggctaagctggccgcattgaagaataagtttgataattaagataaagaaagaaggaaggccggtggtcttccttctttctttcagcgttcatatttctgcatccactgcaggaatttttccgggtagtcggtatctcctttttcgctgaagagcatgagacttctgttcacagtgaagccgatataaatgatgtcccggtccatatctatggcaataacagcttcatcgtagcctgattttccgggcatatatccttcgttaaaaagtattttattttccacttctatgggtggcgttacttttaatctttcaaaaaaagatttgcgggctttacctatcagtgcgttaagcctgcttttcagtggctcggcttcaaaaaggctgctttccatggcgtatttgccatcgaattgcaggaaactgttccaggaagcgaccatgtctgtctggatagtatcgccaccagcgatcatggtatcggtaggtggcaggttagactggtcggccagtacaatcgcccttactttctgggcggggctattacatgcaaacgcgcagatagtgagcgataaaagcgatgcaacaggaatccttctcgcactcatggttaaattttttttgtgatactaaagggggcgaacaacaactaccgggtaccacttttcccggcagttaacagcattatttatcagtggaaggttaacaagtcacatattaaaaataatggttttcaataaagttccgggctatttgcctttaaatacaggaggtcttttttcaataaacgcctgcatgccttccttctgatcttcagatgcaaagagaagataaaaatttttacgttcaaaatgtaatccttcttccaggctggtgtcaaaagtttttaaaatggcttctttggccatttttagggctaccgggctcatggcggctgtttccgcagccagttttatggcttcctgcaggaacagttccacgggcacgatacggttaataagtccggcccggagtgcttcttccgccgtaataaagcggccggtgagcaccatttccatggcgagggcttttcccacagcgcgggttaggcgctgggtaccgccggcgccaggcattacgccgagttttatttccggttgtccgaagcgggctgtttcgctggctacgatcatatcgcagagcatcatgagttcgcagccgccgcccagggcgaagccgctaacggcggctataatgggtttctttatttttttgatagtgtcccaggtactgaactgatcgatattatacatgtctatggccgatttcccggccatttgtttaatatcggcgcctgcggcgaaagctttttcgttgccgctgagaacgattacccgcacttcatcgtccgcatccagggctttgagggcggctctcagttcgctcatgagttgcaggtttaatgcattcagttcttttgggcggtttaattggatgtgggcaacatagggcgccacttgctggtgtatgataataaattccggttgcatcttttaaagttaaagaaatatcataaacatcagtaaaatgtagatgaggaatacgatgcctgttgacatgccataagctatgctcagtacaatacctttcagcagggatttcctgaagctttgccggtagttattccacagcgccagcaccaggtaaatgaagatgatccaccagcctatggtcataaagatatcgttatggaaaataaattccaggagaagcccagtgaggccgataataaagctaaaggaatgcaggtggatggcaaaaatggcgtggtcggcatacagccattttttctgtttgcggtacatccatgtcatgaacagggcaaaaagcggcagcaggacaaacatcaacttgggcacattatggttgaacatttcaataatggcctttttggagtcttctccatatttctggcgcacgccgataatccgccggtataccgacttttctgcgccgtgaaggcgtgccgagtccggcaattgccgttgcgccgcatcaaattcttccacggtatgatagcggttcatattcttctttatactggtgggagaagaatcagagagggcctggtccagggtttcaatgcctgtttttacgttatccccgttgtttacctgggccagggggcgttccgtaacgaattcgccggattccttttcgttgccatgtggcaatgtaaacaggccaaaaaagaaaacgaaggatataaatacgtataattttatcgggttgacgtagcgtactcttttgccagccatatattcccgggaaaggaatcctggtctgaaaagcaggtatttgagggtagtgaggaactgggaatcgtaatgaaagatatctgccacgaagtgtttaaccaggtgggtgaatgtttcatgtggtacggtattttcctgtccgcagtgtgtgcaataccgttcagggacttctgtgccgcagttcaggcaatttttctccttacgtaaaggttgtgatttcaagagatttagatatttttggttgtaacagcaggcaagataaaaaagaaatgacgaattatagccggataaggtccggttaaaaaattttaatatgatttttgcgttttacctttgaacattcaaaaatcagcgattttacgggcatgaagaaaacgatcctactggcactgagtatactggcatttgcggccaggggttttagtcaatattacttccaggacatttacaacacgcagcaaacggtagcgactatggcgctgctaaaggaaaacaaggtaaaaacgcagcaggtgctgacgctggatgcagatatgcagccggaccgggacttccgttgtgaacgcaacctgaatcccacgtaccggcagatgagggcgcagactcagtccagctccaccggttattcggctatgacttctacgttttctgcgaaggggcagttgaccagaacagtagacagttccggtgcaagtgtgactaccacgcagtaccgttacgacgaaggggggcggctgcaatatatcagcagcacttccattgcgcgagatagtaagcttcgttttgatgaaagccggacgtaccgttatgatacggcgggacggttacagcagttgatacagcgtaagggcggcgactccacggtggtagcgtttaaaaccgacagtgcggggaatgtgattgaagagctggatacgcgtcgtgggacgaagatctattataactacgacaaggcggggcggctcacagatgtgtaccgttatcagcctgcgaagaagcgtatgttaccggactatatttttgagtataatgcacagggaaagctggtgaagatgactaccgttaacgcacaaacgtcgtcgtatacaatctggcagtatgaatatcagccgaatggattacctttgagtgaaacgtgctatggcaaagggaaagagttgttagggatggtgaaatacggctatgagctgaatccctgatgcagtttaaaaaaaaggcattcgtaaaatattttaattcaacgttaaaaaaattttgcagcttcgaaaagattcctatctttgcaatcccaacaaaaaaagttcttattaataacgcgaaagtagctcatttggtagagcacgaccttgccaaggtcggggtggccggttcgagcccggtctttcgctctgattattccctacagaccctggtggtggaattggtagacacgcgggacttaaaatcccgttcgcagcaatgcgagtgacggttcaactccgttccggggtacaatgcagaagtgacacttctgatggaaaggtctcatcgaaatcgatgagacctttttcttttaaaatcaatgagttaaacctgaagactccttcgatagtagcggttcgatatagcctctctttaaacaccagattatgtttgaacaccttcttaattaaagattactttcttgttaccttacttttagtgtttttaaactttccttgaaatggtcctttagcccgtccttgcattcagtaactaatggtccacctgtttttcagaaaaacttaaaagctccataatgtcctccatcatagtatgcaatttctcacctggaaaattatcgctcttatgatgctggcatctgtaatacagataatatttatttctaccttttgaataggctgctgtcataggagtagcacatcaacacctcacaatacaggcagccggcaactggcaaaaagtgcaaataaaaaacgctttcatataaaaacgctcttaatattcggacgtaaattagctggtgcaggcaggccaaccgaaggatactattaatttttacaaacaatctttaccagcactgttatgccagtgggcttccggtgttcaattctatcccgtttatgacgcgaatattggcaattattatcagtttcatattgatccccgatctatgtttttcacaaaatggtatcctacacaaccgggcttccaaaataattacaattaccactcctgatcaaaagctttccatcaggatcgactattcaaagggatgcattattaaacaggtaaacctgaaaaataaaaatacgatatcatcttcgggtgtatacaccagtatcactgcaggaagtggaaccgcctcatctgctgatcaaacaggcgatattaaaataacaaataccccgaaaggcatatcgctaagtggtatcacctacggaaccggggcgcttcaaattaaagaaacatgggactttaccagcaaaggagataaaataacctgggatattacccgcaactatagcacaacaaccgacctggaagacatggcctttccaaaatggaattttacagatctatccgtttggaaaggaggaattattgataacggcgggatggtttggtgcaaatacctaaaacaaattaacgatacctatggcgttcataccggtggcgtaacattctggaatgctgattcgggagatgcgttaaggatatcgcctcaaccaggaagcgcgaataaaatggcttcaaaatattcccacagcgaaaatggcgagttcacttttacacaattgctaactgattccgatttgcagcaacgccatcacctgagccgcttcgtatcacaaaagtacgatgtatttgctcccttccaggtaaaaaaaggacgcgtaaagctaagcctggaactacaatacattgattacaataaggaatatgcaagaggaacgcttcccggtattgatgcaacagcagtacgcgagcttttaaatacaaccgggcggtatggcgtggtagacaacaatatagtaggcgcaaatggctggctcaccaactggaaatgtctccatgagccattttttgcgcagatcgggatggcattgaatgatccacactatataaaaaacctgggtgcaacattggaccaggaaagagatcaggcgatgttaaacgacggtcgtgtgttatcccgctggcataatgtacccggcgatgaaattcccggcacatataacccgcaaacaggctattatgaagccatgtggggatataccattgattcacaaacgggctatgtgatcaatacaagcgaactgtttgagttgaatggtgacctgcaatggctgcgtgcacatcaagcaagctgtgaaaaggcgctggactggctgataaaacgggattccaacaacaacgggatctatgaaatgatgaataacggcgtagcggaaaaaaaggcaagcgactggttagacattgtttgggcaagctttgaaaatgcttttgtaaatgcgcaattatacgaagcattaacgctatgggccaaatgtgaaacgattttaggcaatcataaaatggccggccattattcagcgatagccgcccgtcttaaaagtgcatttaataggccggttgatgaaggcggcttctggtcgccggccaaacaacagtatgtgtactggcgtgataaagacaacaccattcatggcgacaacctggttactcctgtaaattttgctgccattgcctttggattatgtgacgacaaggaacgcataaaactcattcttgatcaaatagaacaaagaacaacagcagaacacctgtttcactggccgctttgcttcgattcctttaaaagagaagaggcaagcgatggcaactggcctttccctaaatatgaaaacggggatatattccccacatggggatatcttggtatcaacgcctacgtgaaatatgataagcacattgcgcttaaattcattaatcatctccttgatcagtataaaaaagacggactctcttcccagcgctacagcagaacaacccagcttggactaggggatgatatcctggctggcatctgtaccagcattacagcgttataccaggatatttacggccttcgtccaaaatggaacaggatggggctggaacccaatatgcttgaaaccctgaacggaacgaagttttcatatatccacaggcataccgtttatcaccttgaattgagcgttaatgattatttaatgagcaccggtagcttttctgtaaaaagcagcgaaccttttggtgcggataaaagcgggaacacgcttaagttctaccctggtaataaagatactgcgcaactcctggttcgtgcagatccgggcaaccgtattgacatgaaaattacttcgtggaagaatgatgtatttgcatggactatttcatcacacggcaactatcaattcaccattaatggattgcaatcaggctcaaaatatgaagtagtaacaaacaaagatattacccggcttcaggcgaataacaatggcagcatttccctgaataaacattgtagtatgcctgttaacttttccatcaggaaaacatctcattaagctcctcctttcaatccaacataaacatataaaaccggggccctgaaagaaccccggttttatatgttttacacagtttatggaatgtactttgaatcagcattacctgatgggcctattgaaccccggctgtataaatcagcgggttctgtgcatcatcatccagcagatccccgactttcaacctggttacctgcgcatcacttaatatattctttatgccgttaaatctagcgccatcaggcatataagcgcaggtcatcgccctgcggaagccattggtcatattggctcctgcgccgtgtatcgttaaaccattatgaaaagaacagctacccgccttcatgggtgcagcaacagcgcttttagttgcaagctgtgggtaaacctggaatattgcatccatatttttcccgataccctggttttcaaaaccggtttcatgataagatccgggaataaaatacagacaaccgttttcatttgtagcgtcgtctaaagctacccatattgatagtgccctcttatcggtgaacgaccagaaaggcgtatccaggtgccacgaagtaggattcgcccagggacgttttatgagcacctggtcatgccagatccgggtaccatcccaccctgctaattctgcggccattttgcccaatctctcatcaagcataatctgccttgccgcatcgtttgtttgccagatattaatcatctggtcaaacacctttccaaaatattcactttccttattgatcccgtcgtcttcccccatttttttatcactaccaggcattttcctgccatccctctgttcaacggcctccataataacctgccgccaatgggaaagttcttcctggttaagaaagttctcaattaataaaaatccatcttcccgataagattgaatctgcttttgcgtgagtaacgtgttcatatatctgcaactttttttgaaaaatatcaggcacaccaggcaaatacctgcaggcccatagtattattattttgcctgtattaacttaacggggcctaacaaaccagcgtcatatttactaaaatcgggcacacctacccagccccaggtgcggagcttgcccagatccgatttcatccacatttcattgaccatcaggttcccgacccgtattcttattttattttctccctcctgcaggtatttggatatatcaaatacaaagggcgcccatagccggtctccaacgggtttatcatttacaaacacttccgccatatattttacatcaccaaggtcaatagaagtccgggtatttacatctttcagcacaacaggtatttcataatcaatatatcctgaatactgctgaagtccataagcataccaggattgcagggtgcagtttgctttactgccaacaataaatttcaacggggcagtcagcgtctgctcacttttgacggcccttgcaaacgacagcaatcgtgcatcagcaggcaagtcaattgacgccgcagccacgtctgtttttacgccatccatccaaaccgttgtgccaatcatattatcagggaacactactgtttttgcaccaactggtatattgaccctccagtagtggtaaccggtggcatcattatcctttatttcatccttctgcccatccccgttccgtttttgcgctgtcataaaactggtatacttccattttgagtcattatatgccaacaacataagatcttcatttaacccgttgtcggctaacgtgaatgaagtggccgtggttttataaacagtgtctttccccggataactgatggtccatttatcatcgagcttaatttcttttaaatcagattcatgctgtaccaatggattcatatcgcttgttccgggctcaaatacaagccaataaccttcataaggttgtaaagtcatttttactttgttatatcccttctccttcacgtatgcaacgggtgtacgttccccggtttcacaattccatatctgcgccatgccatcgccatccctgagccaggctgaaaaatttctcacggtatcggagttattggcaagccagtaaaagtggttattggaaatagttctgtgagcagtgtagagccggcctgagttttccaacctgatttgtggcctgaccctttcattcaaagcagtaaccattttactcagcctgtctttgtctcccgacagatcaataacattgggcaaccgctttaatgcattcatctggctaataaccaacgcatctttcatacctttctccggcgatccttctggtgttgtacccaggagcagcacaacgcctccctttttagcaaattcaagtatcttacctgaaacggcatgagaaataacacaagccggtggaagaacgatcgccgaaaagttgtggtcattaatagtgatctttgcaccgctattaatggctcctgtttttcctttatccaggtaatatttatcagcgattaaaaagtcgatgttatttttatttaattctctcatagcatcggaatacacctggttgatctcgagtgaaagcgtatcccagacttctttgccttccagcaagccaaaattttcctcatgtgtaaaaaagccttcagcatttgcccagatactttcaagcgggtttaccaggagaacatccgccacaagcttactttgcctgttcacaaaagcagtccgcctggaaaagtccgtccagttatgcaaataaggccaatatggattttcggtaaaccaatccggcggatacggatcctgttcaattttccggttaacgttaattccatgtggcaccacgtggttaataccaaatgatgtaatagcattaatggtcattttcatcatagcgggtgtttgctcccatcctgcaacgcccataatttcactcataaaaggacgatcttccaattcggctattgtttgcacttccttaaaatcatgaacatcctgcgatttcattaaaagacaatctgttccgggcatagttgctgttcttgtaatgcgcataaaatcgcccatggcggcagtttgtaacaacaatgattcttcccacagattggagatgtaatacatattgtattgtttgagccagttcaccaaaggctcaaagtaacatttgttatatacgtctgaaacaacatcaaaccaatcacaacgggcttttgcaaacaaaccgttgttgtccttttctgttaaaaggggaagccataaacgaatatcctggtttttcatttccttataccgtttggcaagatattctgaccacgccatacgccagccatagtcgccttcattgtcaacaaaaacgccaggaattgttttccccatatcatttgcaaaatgtttggcatactgcgcgtgaacaagcgggatgaaaacttccattaatctgggatcgagatagttaactttcccaccgtcaattccgggatggaatctttttgtgtaagtatacaccacccattcgcccggtggcgccgtccatttgaaatggcttccttctccaatgatccgcagcgatgaggcatcaatggcattgccggctattttacctgccacggcaaaatctgttgaatcataataaacggtcgatttccccgttaccttataccgtttccaatccaggtattttgcctccagctcaggatgctgcgctaatacccgtcctgctgcctgcccacttggccagtcgtattcatcacaataacccagggtaaatcctttgttccttgctgcctgcatagcattcccgaaactgctgaaccagggtttttccaggtattgcttatatggcaatgaagaaaatgccgggtttaaacgatccattgaaccccggggatgtgcatatccggggttcagtccctgcttcatcatttcctctgccatagtagccgtaaaatgctcatccctgatggtatcatcccagaaccagaaagtatggggagcatagaacattggggggctaacaaacatttgttgaaccgttttagggtcgctatattttttttgccattcagattgcccggatatattcaaagtaattgtcagcaagcaaccggtaaaaaagatgttcagatatgtatatttcattattgttttgagttaataactggtatgaatattattttcaatagaaatccatcaatgctacacgcgatattaattatagccggggttctgcactaacttatcgttcttattcatttcactccttgcgattggtaaaaagtaggccttattatcccactttccacttgtgatctccacgggggtaatatcaggaatggtggcagttgtatgatcgggattcagtttgtacaccaccttaaccccatgcattgggtgataggcttccggcccgatcatccagcggcgcacatcaaaaaagcggtggttttcgtacaccagttcaatacgcctttcattccggtatcttgttgacaaggctgcgccggcatccattacatcaggcatggccgcttttttcctgatcatattaatgtaggtgcgtgcttccgcctcctctcccaatccaatacaggcctctgcataattgagtatgatttcgctgtaacggatgaagcgccaggtgaggtcatcctggtgatttacatacatatcggttttgcggtttataaatttaagcatacaggtaccggtattattataaccgcctccataaaccacgctgttcctgctatctaacccatacgtatacacgattttattagcggcggcatcccacttttcccaggtacctacctgcaaaactcctacgggatcggctgccagtaagctggatggccttgacctgaaccttgccccttcgtataaaatggaagcataaaaacgcgggtccctgtttttatatggttcgaggttctgtgcagggttggttctggagaatttagtgccatcactcatttcataagcatctaccaattcgctgggggcgccgtttgtttcaataccgccatatccatttgggaaaacctgccagtagtcaactccctggcttacggaggcattgtaataacgaataaagatgtcttctatactattttttgagataaacaggtcctcataattctgaacagcctcctctgttgatgcaggaccgggctgatacaaaccatatatgcccaggtctattacagccttagcggccgctttggctgcctgccagcgttgcttcctgtcgccatctacatatcccaggagctcagggttggaaaacccggaaaatgttgtattatgaagatcgctggccgcataaagcaatactcttgatttaagcgccaaagcggcgccttttgttactcttcctttgttgacacctgtattcaccaggggtaataatgcagctgccttatcacattcaccggaaataaattgcacgcactctgcatagctgttccgggcggcggaaaagttgtctgttaatttataggatttcgtaaccaggggtacaccgccaaaataactgatgagcaactgataataccaggcccggaaaaaagtggcttcgcccttcaacctgtcttttagtgtaacgccatcaatcagcgccggatcatccggcaatttgtctatattttccaggaatatattgcagtcccggatagcgctgtacctgccgttccagtcgccccagcctgcattatcaggcgacatcagcatgttgctcatattataatcatttcccgcatcatagcatcgggcctcatctacagccagcgaagtcatgaagaacgaccaggggttctggttataaatgctgttcatgttcagttgtatgaggttgggatcagaccaaacatccgcttctgtaaattgcgtggaaggttttgtatcaaggaaacttttgccacatgatgttagcagcagtgacataaacccgatagcgatatatattaagtttgagtttctgtaattcatacactttgattttagaatgttgccgttaatcctacgttagtggttttgttcaatggatatacttcactgttcacccaaatggagcctggagcgtcgtcaggagattcaggatcgaaatccttcatctttgtaaacgttaaaaagtttagggcgctgacatagagcctcagcgattgtatgcctattttttgcgcaatgccggatgacaggttataaccaacctcaaagtttttcaatcttaaataatcactgcttctaacgaagtaggtattattaggttccccatctgtcatccaatatgcgccaccacgctcccatactctcgggttaacagcacttggatgttccggtgtccagcggtcttttacaaggttgtacataaaattcccgacacctggcccgccggaaaaagtccggtaggatctttccgcaccggccgctccctggaataatacatttgcgtagaagttcctatactgtaaatcgatactgagcccgccggtaaatgttggtatggtagttttgttgcttctaacctggtcctgtccatcaatctgtccatcgttatttacatctttgaatataatgtctccggggcgggcgcctgtccaatgagggtatttatcaatcgctgcctggtctgcgaatacacctattgcctggtaatacaatcttgcgttcatctggttgccggtagacttctgatagtcgggcacgccgggtgtttcatcccagaacctgatatgattctttgcccaggcgccgttggcagacacctggtatttgaaatcgccggcactaccgcgatatgatgcctgtaattcaaagcctttgttaaccacttccccgatattttcctgcggcaggcttaatccggcagaacctggcacagaagcgtttcggtaggccaggatattggtacgcaggttgtagaaataatcggcgcttaccgctaatttattattgagcagttccacatcagcaccgatattggattgattggctacttcccaggtaaccccggcgtttggaatacgtaatgctttcaacgcctgttgcggaacattttcattaaatacataaccaccattgtagccataggttgtaaggtattgatagggccctatccggtcgttacctgtttttccccaggagcctcttattttcatttcattgataaaagcgatattatctttccagaatttttcattagagatcctgtatcccagggatatccctggaaaaaaaccaaattgcctgccggccggatcaaaaatataagagccatcgtacctccacacaaattcagcgagatactttgcgtcataggcatagcttagtcgtccgaaataatctaacctgcgggccacaccggatgatcctccattatcttttaattcattacttcctaaatccagttcgtcaagaatatcgctggtatagtttctcctgaaagcccagaaattcatgttatcaccggcaatacgttccgccgcaaaaagaactttaatatcatgcttatcaaaaaccctgtcataatttaacagcgcattgagggttacattagaattgttatccatccactgttgcagtcgcggatcagtgtttcctttcttggatgctaccagcagcggagttccattggcatctaaacttgttttatcccaggtatagaggaaccatggctttctgaattgtttggtactgacaatagttctgtccattgctgcattacctgttaacgacagtccttttatccatggaatagtaaccacgagccttacattactctgaaaaatataacttcttgatttggtgtaccccgtggcatctgtaaccagcactaccgggttagcgccatattcaatatccggtccgggcaagccattaggccatctcgcgggccaggtaggaaaagacctgtttaatgcccagaaaacattttgtgcctgatcggcgcttcccccgttggcgccgccgcctgaatagttcctgttttcctgccgcccaaccacatcaaaacttaaatggatgttgttagtaacttttgcgtcaatattactttgaaaattagtctgcgaatagttggtagctccgtccctgaaaatcccgtcggtaaaattcgatccaagtgaaatgaaatactttatggcctcagcgccgcctgacaatgttaagttgccatagcgttgcggggaatttttcctgattgtttctttaaaccaatccgtattgggatgcccccagggatcagagccatccttatacttctggatatcttctgccgaataaggcaatgggtcgccgggatgataagcagcggaaatttcattctgtaactgtgcataaaggggcgcatccgccattttgggaagaacggtaggtgtattccatccctggttcagggagaattgaatggtgggcttaccggatgcgccgcgtttggtggtgacaaggataacgccattggccgcctgtgatccgtatatcgctgcagacgcatcttttaagatcgtaacagattcaatggtggcggggtccagccgttccaggcttctgccggcaatgccgtcaacaaccaccagcggggaattatcgccaagtgtattggccccacgtattcttaaggtggatccgtcatttccaggctcgcctgttctggtaatagccaccaaaccaggtaaccggcctgctaaggaattggagaaattacctgccggtgatttaaccaggtcgcttcctttaacagaagcaatggagcctgtcagtgtttcttttttgcgggttccgtatccaaccaccacaatgtcatttaacctggcattgcttggggtaagcatcaccgttagtacctctccatctttcatggctgttacctgtttcacttcatatcctatagaagaaaaaagcaggactgcacccttagcaacgctaatcttaaaggagccgttttcatcagtggttccaccggcagtcccgccttttattcttatagatacattggaaacgggttgactgctgtctgacacaacattaccgcttaccactattttttgctgagcaaaggaaatttgtgagatgcccaaaaggaatagcaataaaaatgatgctttgataggcaatagagaatcaaattgcttgtttaacataacatgagattttggttttaaacatcgctggtagtggaattatttacaatttagaaatgacggttactgctgtgcggcggcaggccgacaggtggttgatgcattcataaagattaatttttcaaacgtgaatttaacccccggttgctgatctacagccggaatgaaacgttgatatcatcacaaaaagtgctacttttatatgaaaactttctatcaaaaattttccgccataaaacaatttaaagtcagtcggaactttaatatttcagtaatcatctatcctgtttttcaattaagttggtaatgcaaagtaacctgaatctaaaaggtgcagtgataaattctgatggaatcatttaactttttgacacaccaatgaaaaataaaaggaatcaaaatgtcaattacctgacagtaaatgaaacagacgaactgtggggattatacaccactactattggtttccaggttatatcgcccaatagtgactaccctcctaaaagccatccttcggcatattggttcagtcccaataccggaagggtattgcaggaatacatcctgctgtacattacagaaggagaaggttcatttgaatcggcaagctgcaagctaactaaagtcgttgccggtactatcctgttgttatttcccggcgaatggcatacctaccggccgcttaaaggcaaaggatggaatgaatactgggtgggttttaatggcagttatatgaaacagttaaccggtaatcttttcttttgcaggaaaagcccggtctataatgtgggatttaatgaacagattgtggccttgttcaaccagggtattgagacagccaattaccagaaaatggcctaccagcaggtacttgccggtattaccagcctcctgctgggcttcatcctttacgctgagaaaaacaactctttcagagataaagccatcatcgctcagattgataaagcaagaatgatgatgcgtgaaaaaaccggtgatgatgttactcccgaatccatcgctaaaacgctaaacattggctattcctggttcagaagagtatttaaacagtatacaggattttcacccgcacaatatcaacttgaaataaaattgcagaaatcaaaagaattgctggccagtacgattttaccggtaaaggaaattgcctttcacctgaactttgagtctgccagttattttgtaacgttctttaaatcaaaaacgggattatcgcccggtgaataccgcgataagataaaaggcaaataaagcgatgaaacataattacctgcaacggagtttcattcaacggcaaatgttttacgataagtattaggagaaaggccaactttcttcttaaagatcctggagaaataataaatgctgtcgaaccccgtttgatctgcgatttcctccacgttaagcaatgttgattcaagcaattcttttgccctctctatgcgtaaatttaaatgatattgattaggcgacagccccgttactgctttaaaattcttcctgaatgcagaatatcccataggcaattgccgggcaagttccgggatatctacaggctgctccagtgattcctgtagcaggaactttgctttcattattgccttttccagcgggctatgatcatattgtttactgagcgatatggtattgaccaaaccgagtatctgaagcgtcaaacccgcaatctgttgtgagtaacctacaagcgaggcatttacaacatcaatcatctttttaaataataccagcatatctctatccagccctgttttgatacatggccgattgggatcaaaaaagccctgtttcatcagttgatcaacatagtacccatgaaagccaacccaatattcctcccatcccgagcggatatccggcctgtatcgatgccatactcccgggaaaagaaaaaaacaggttccctcctcaatttccaccggctcggttaatgccgaacagcatgttccttttccttttgaaataaatatcatgtaatagtccgtcagaatccttcccctgttccatgtaagctgatggctttggggatgttcttctttgggataacgttcattcggtgttacttttgaataccccaccgtagttacataaatcccccatttctcctcgattggacctgtattcagatatttaaaaaagttattacccattgaattatcttttctcttaaatattggtggcaaccggcgttattaaaggagggaaatatttccgccgatcaacagcataacgtgttaaaagataaagttagcaaaaatgccttagcagataaaataatgtggaactgaatacatgagggttattgttgtggagcaattatatctctcagcagatgcatcataaataaattcacttcccattgcgaagctaccggggtattacccgacgaagtagtccacatataaggcggtggcccaaactccgttgtaatggtaagcagggatatcccttcagcttctttttcccggatgatccaggaccataggccggtaaagtagttcagcggctccgcccattccggcagtcgtggatcaggtatctgcggtccttcaggaaaacccacacgggcatgtatatgtacggtgcgtctgattgcttcgttaaccgtttctttgaatccttcaagatagctttctgtaacacaaacccagtgtgagaaatcggcggttactttcatggaaggtcttagcttaaacagttcttttgcattccccgggctgaatcctattcttccccggtgcgtttcatgcgcgataacaatattattcttcgctgaaaaattttccgccgcatcaataacggcaagttgttcattgatcgtgaagaaatctcttcctgaatgcgaattaataattaccggttcacattccattgccgcattcagatgatattcaaagctcctgcaaaaggtttgtatatctgcacctttcgcctgatgttgttgcacaactattggtaatcccagttctttgctacgtttgataaataccttcctgtcatttttattttcgggcagccaggaatccacgccgtcatatcctgcggatattaccttttcgagaaaagcctctacggggatgttttcgtggccccatcgtgtacaaaggatttttatctgcatgttatcaactaaaggctttggatttgtgagaaattgcttcaatagggtagaactttagcttacaaaaataggtggtggagtcaccggtgaagaaacataaatgagatttttcttgtgttttctgacatttctttggggaacgactgtgacgataggcagcatgattgttgtggatcgatcttattaaatggtaaactgatacacctcatcttttgacagatcctgccagatcttatattttataataatcgacctttccaacagccaccgtccaaaaatatcctgacttttccagatcctgatccattacctcttttgctgcttcatatgagccatctgctttcatttcagcaatagcagctgctatatcagtgggaactgttgctctccaaactccaacagaaatttctaaaaaagaataactatatggtacttcaaagtcatcaatttctccgttattttcatttgttagcaaagctacaagctcattagccggaagtttaaaagggttgatgccataaatattgaattcggaattttcagaatagggtccctgacattcgataaattccagtaaaccattcttatcaagatcaaatctaacatccaaattattataaaaaacctgattttcttcctcgtaatccgggttaccaagtaaacttataagatcattctttgtttgaccaaagcttatcttactttcatttattataattccgtctaatggtttcaatgtaattctgttcatagctttttgcaaaatagactctattttaacattaaaattttatttaagcatttaaagtttttaccaaacatcccccgcagcctcatttccccgatagaagataatgaccaatctaaaaattattaactattttcgttcactaagtcgtgtgctcgcatattgagcgataggaaaaattatagtccggtgcattacccggaagaaaccggcatctaaattattgcgtcacagcaactgttcagacatttttgatataccctcctgcgaaagctcctattttcaaaattattttttaagatgaactgttaacggtataggattgagcaacaacaatttaaatacggaaccggatgagcgggagacactgaaactggttgcactgggggatgaacgggcatttagtcgcatcgtcagaaagtactcccaggtaatctatccctacctgctttattggcttaaatcgcctcaactggccgaggaagtggcccaggatgttttcctgcgcctctggaaaaacaggcacaaattaccggatatcagcaatttctcaggctatgtatatgtggtttcacggaactgcgtcaactcccagtttgaacgcggattattagaaacagctgcgccggatgtggctcaaatcgatctggcgctgaccaatcctcaaacagacctggagactaaagaactggccaccattatggggcaggccattgaatccctgccaccacgacgcaaagaagtattcctgttgagtcgcaacgaacagttaacgtacgaggaaattgccgctcggttggggatttcgagaagtacggtgagagagcatatggtggaggcattagtcttcctgcgaacttatttaaaaagaaatgccgggatcattatcaccctgttatgggcgttaattaacctgttgtaaagagatgattaaataattaccagattttttttattcccgacccgtcctacccttctttaaaccgggtctttattactgattacaatgactgaagagcaactgacatattattttgacagatacgcccagggaaacctgagcaaagaggagcgtattgtgttcgctgacctgctcaaagatccggctaataaggacatggtagcgcggatgctggaccaggattggccactatgggaaaacaatcaacaggatttttcgcaggaaattgcccgtattgaacagggggtgaccgccaggatttatgctgaccaatccctcccagatgtgcgtcctgtacctcgtatacattccctgaagaaatggggccgggccgctgcggtattgattctgtttggcgccggcacctatctttattcgacctccaaaaagacggcaggggatttcgtaaaaggaaaagcaatgcccactcctgatattttacccggatcgaataaagcactgcttactttatcagatggaaccgctattacactagatagcgctgccaggggcgccattgcccaacagggtaattcttcggttgttaaaacagccaatggcgaaattatttacgatgtgaaggggcactccgaaggcaaagtgatgatgaataccatgtccaccccgcgcggcgggcaataccgcctcacgcttcctgacggtacaaccgtatggcttaacgcggcaagtgctattaccttcccggctgcatttacagggaatgagcgcaaagtaaaagtaaaaggggaagtgtatatagaagtggcgaaaaacgccaaaatgcctttcatcgtggatgttgacgggcaaaccaccgttgaagtgttaggcaccagtttcaacattaatgcatatactaacgaaggtatgattgccaccacactggtggagggtaaggtcagggtgttggcgggtagtatagcagctgctgctgcatcatccgaccggcagcttacgcaccaggcggtaacgctgcgtcctggccagcaagccttacagccggataacaccaccaccatcaccattaattccggcgccgacctggaacaggtgctagcctggaagaagggcattttcaacttcacgggcaggccgtttcaatccatcatgaaagacattgaacgatggtacgatattgaggttaaatatgaaggaactattccaacaaggaaattgaaaggagaaatggacaggggcgttcaattaactgatttgattcgctttctgcagggattcggcctgcatgtggaactgaagaacagaacattggtcataggagaaaaataaataaatccctgtcagccgaaatatgatatatactttgccggcagccaaccaccggaacagatccgtgtatacgtggatcacctgttccggacgatgaatatactgaataattatcccggcaattccctcttaaaagggccagcatatacaattccttactcaaaacgaaaagccaatgatggggaaacatcattggccgggtagtttaggtaacattcaaaacaaagtctgcacagactgcttattaagcacctaaaacagttccaaaggtatgacaaaaactgctttttgtggatggccctcccgtgggggtatccgtcaagtcaccaaaatcttgttagtaatgaaactaactgcattttttcttacagccgcttttctcaacgtatcggccattggattttctcaaaatgtaaatttctcgggcaaaaatgtatcgctcgaaaaaattttctctgttgtaaagcaacagaccggctacctgtttttataccaggaaactgatctatcagcagccaaacctgttaccgttacggccaccaacgagccactattacagttccttgaagaggtgttccggaaccagcctttaaagtacctgattagcagcaaaaccatcagcatatatccggttgcagcgcagcccaccggaaataaggttacaacggttggtgagcttgcgacatttcctttcagcggcgttattcttaaccgcgacggggaagcgctccccggcgccagcatcgttatcaaaggcaccagaacgggtactgcaacaaagactgatggctcgtttaccatcaacgttaatgcaggcgatgttttagtgatcagcaggattggatatggaagcatagaattaaaaatgacctccgccaccaatgctgttgtagtgtcttacccggctggcaaagctgacggggcagctcttaaaaccggtcaatccatctcttccggttcaggcggttttaatttaatactccctccatctgtttctaaacttgatgaagtgcaggttattgcttacggcaccaccacacaacgttttaatacaggcagtgttagcagtgtgaaagcggaagacatcgagcggcagcctgtaagtaacgtgctcgaagcattgcaggggaatgtaccaggacttttcatcacgcgttccagtggtaacgctggcagccagatgaatatttccatccgtcaacagcaatccatcccgctacccaccggcaataaaagtatgccgctattcattatcgatggggtgccattcgtggaaacgccatttgccagtgcaggagcctccggtgaaatagatcccatgaactccatcaaccctgccgatatcgctgagatatctgtattgaaagacgccgatgcaactgctatttatggctccaggggcgctaatggtgttatcctggtgaccacaaagaaaggcaaaacctccgaaccacatttcgatttcaatatttatacaggcgccggtaaagtaaccaactatttaccgatgctgaatctttccgattacctggctatgcggagaactgctttcgctaatgataaaataacacccggtttttcaaacgctccggatctcactatctgggatacaacaaaatccaggaatttccagaaagattatatcggcaataccgccaatcaaacagaggttaccggcgcattttcgggtggcagtcaatatttgcgttaccgcttttccaataccttccggcgtgaaacgacggtatttcccggcgactggggatacaaccgctattcatcccacctgagtatagacaatacgtcgcgcaatggtaaattcacgctggccgcttcggccatgtataccaaagaatccaataaccaggtggccagcgacattacccggtcggtgtacatattaccacccaactatcccgtgcataaccccgatggcagtttaaactggacaggtggattcaccaatcctgattcctacctgttgcaatcggccaggttcaagtcggataaccttttagcaaatgccactttacgatatacgatattggcaggattagacgcaaaggtgagtcttgggtataataaaatagctcaaaccaacgaaacatatcttcctaaaacctcccttgacccgaatagtggctcaggtgaatcagcggctacgtatacatccgactatattgaaacctatatcgtggagccgcaactaacttacaacagatcgctgggtgggggtacactgaacgtgctggtgggtggtacctggcaacaatccagctttgcagaaccatattatgtaagagccaccggcttctccaacgataagttgatgagctcctggacagcagcttctgatatcactttcaaaagcagcagctttaaagaatacaaatatgtttccgcattcggacgcatcaactatgtactgaaagatcgctatctgttcaacctcaccggccgcagggatggctcttcccgttttggtccgaaccgtcagtttggtaatttcggctccgttggtgcagggtggattttcagcagtgagcagtgggtaaaaacagccattccatggttaagctacggtaaactcagggccagctacggaacaacggggaatgaccagatcccggactacggatacctgtcgtcctatggcaatcttttttatcaatatggtagcgcaggaatttatcctttgcgaagcgccaatcccaattatggatgggagtccaaccgcaaactggacattggcttagaaaccggattcatagaggatcagctcttcctttcggcttcctggttttcgagtcgtactgataaccagttggtgactgctcccctctcttcccaatcgggattttcttcctttatcggtaatatgccggcattgctgcaaagctccggatgggaatttgagttgaaaacaaagaatatcaaccataaaaaattctcctggagcagttcttttaatattaccatcccccgtaataagctcatttccttccctggtttaaaaacaaccgcctatgcttatgtatttattgagggacaacctatcaacacttataacggctatcattatacaggcctgaaagatggaattgctaccatcgcggatctcaacaaggatgggaaatttacaaccggcttgttagaaacagcaaacggagattaccagattatatcctccagtattcccgatttctatggcgggttcagtaactcgctcaaactcggcaggtttcagttggatatcctgttacagttcgtgaaacaaatcaaatcttccgttcgctccgcagtaggaatgcaaccgggtggattgtccaatcaggacgacaaaatcattactgatggcttcaagccatctacgttgtccggcagtgacgctacttatgcctataaaaattactacctgttttccgatggaaactattcagacgccagttttataagacttaaaaacctgaacctctcttacgagcttccaggttcctggacaaaggcgatccggttaaaatcagccggggcatttatcagggcgcaaaacctgtttaccatcacccgttacctgggatttgatcctgaaaccgccggtgcagtattaccaccgttaagacaaattgccgctggtatccattgctcactttaaacaatagggaaatgaaaaaacaatgctttttatatacttgtatcgtgttattggccgcctcgctcctgaatggttgtaagaaactgatcgagatagggccaccaaaagaccagctggcttccaacagtgtattcctggattcaactacggcggaagcagctatgatagggttatatgccagtgtggcgaacccgaatccgggcaatgatttgggcacttccgttaccatgttcaatagtatgtcggccgatgaaacgtacgcatatgccatgaattattacgatgattttacgaataactccttaactcccatgatctactacgtagatggtttatggagcaccatgtataaaaatgtgtacatcgccaattccgttatcaccgggatggctgaatctcccttatctgaatcatacaaacaaagggctgccggggaagcgaggttcctgcgggcattatgctacttttacctggtgaatgaatatggcgccgtgccattagtgttgtctactgatgtaaacagcactaccacgcaaccccgtgataacgtggatgccgtttatgaccagatagaaagagatcttacagatgcgcaaaaagtactgcctgccaccttagacatctatggcggcatgcgtatacgcgctaccacctgggctgccgatgccttactggccagggtatatctttacaggggaaaatggcaactggctgaaagcatggctactgccgtcattaacaatccgggaatgtttagtatgaacgactccctcaaccaggtgttcttagctaacaacaaagaaggcatccttcaatttgtaaatggtatcagcagttcatggatcgccaacaacttcgttccttcttcattcagtacaacgcctaaatttgtaatcaacgacagcctctataataattttgaacccggagacaggcgaaaaaccagctgggttggctataaaagctatggaggtattaactatccctaccctgcaaaatacaggtatatggcaggtgtgggcgcagtggaatataaccaggtattgcgtttgacagagcagtttttaatccgcgctgaagcccgtacacaacaatccaactacatacaggcagcagctgatcttaatagcgtccggttaagagcaggtttatccaacacgaaggccaacgacaaagccacgctgatggctgccattgaacatgagcgccgcattgaattcttctgcgaatggggacatcgctggttagatctgaaaagattacccggcatcaataaccctgctatctccagggccgacgaagttttatcgcagctcaaaggaggccagtggcagtcgacagatgttctttatcccattccgcaatctgccattaattctaatcgaaacctggatcaaaacaaaggatatttctagcgccaggtaaaaaccaaacatatgatgcgttatcaattattcaggcaatggctgcctgctgccctgctcatgaccggaacggtcgcagcaaaggcacaatccggacaagcaaagccgttcatactaaaggggcagataactgccccgcagtaccctgtcaaactttatcttcaatacgagttgaatgataaagagcgggcaactgattccgctacgctgcaaatggatggacatttcaccttcagcggcaagctgagcagaccggtatctgcaaagctgtacatgatgccaccgggtggtaagtatgtttcacgaaatttctacctgcaacctggaaaagtagacatccacacaaccagttccctggattcagctactgtgaaaggcagccccaatacggctgtcctggatgaatttgttcaacatggaaataagtacgcaaatacttttacctccctgaatacaagagcttatttcaaccgtggactgaaagattccctgctggctattaatgcggagcaggaacaggtaagaaagaaatttgatgaggaagtagccggtatcatcaggcagcacccgaacgcctatgcctcctgggacatggtttatagttaccgtatagctttagatcctgaaacggttgcccctttattcgaagcgcttagcccggcgtttaaaaattcggcagatggaaaagctttggcaaaacagatcgctaatgtcaggaaaataatggtgggttcgcccgctccggattttatgcaggcagatacagatggcaatgccatcaaactgtcttccttccggggtaaatatctgctggttgacttctgggccagctggtgcggtatctgccgcgcagaaaatcccaacgtactgcgtgcctacaatgcttacaaagacaaaggcttcaccgtattgggcgtatcgatggacgattcgctgcaccgccctcaatggatacaggccatccgggatgataatatgccctggcaacaggtatctgacctgaaaggaagaaataatgaggctgccatccaatatggtatcaagggaatcccgcagaatgtactcatagatcctgaaggcaggataattgccaaaaacaaacgcaacagggacctgatgaacaccctgatggaaatctttgaccgggggcataatatgcgaatggatggagagataaaaggcgagaacgacagcatcattgtttttaaatattacaaccgcaatagttaccaaaacgatacggtgtctatccacaacggcaaattcacctggcttgctgaaatgccggagccacagcgggtgaacgccaccatccttccaaaaggtgaacagcttagcttcttctccgatatcgggtacctgcagttatcagctaatatcgattcgttgccaaatttcacattagagggctccgatatccaggatgaagccaatgccttttatgcaactaccagggaacttagtccgcagcaaaaggaattgctgcaacaactcacggatgcctcacaagaggaaaggtccaaaataggagaacacttgcttaccctgacaagaagccggtatacggctagcgttaaggactatgtagagaaacatcccctcagtttattttccttgcaactggtaaaggatatggcggaagatatgtcggggccccgatataacactgtttacccgctttatgcatcgctgccggaaataatccgtggaacgcccactggcaaaaggatagcagggatgttaccgttgatgaaaagaagcgccgaaggcgcaatgattgcagatttgtctcaagccgatagcagcggacaggaaatttccctttccagctttaaagggaagtatgtactgatagatttctgggcgagctggtgcgggccttgccgtgccgagaatccgaatttgctgaaagcatacaatagttaccaatccaaagggtttacaatcgtgggcatctccctggatactgatgccagcaagtggaagaaggccatcaaagatgatcaactgccctggacacagttgtctgatctgaaaggcagggaaaatgccattgcaaagtattacaacgtgcggggcataccctggaatatcctggttgacaaggatggtaagatcgttgctaaggatttaagaggctttgccttggaggagaaactgctggagttgatcaggtagatgaccggttttattgccttatgtcttcaaaaaatgaattatttaattatattattaccttcatgtatgaaacaaaacccaacggtattatatcagcatgaagcgaatgaataaacgggagctgctttttatatgtcttcttataatttctttttcctgcgtggcgcaaagccagggaggctttgtggggtttggtcaacttcccgtaaaaaccccggattcgctgttgcagcgactaaggcaggccggtgatattaaagcaaaaatgcttgccacggagcctttaatggcatttcatgctgctcacggcacaacagattcggttatcttttactcccaacagatgatcgacgcgctaaacaatagtgatataaaggcccgtgacaagctcccctatcaatccaccctgtaccacactttagcgaaagcttatagcgaaaaagggttgtatgatgaggcgctgcgctattacctcgaaggcatccggtatgcagaagcgctgaacaatggtgctgctgtcaacgaaaataaactgggtatcgcaaatgtatattttgcccggaatgaacacaacaaagccattggggcatataacgatctgctgaatacctcccatgatgagcaactgatacatattgcgtatcaacaactgggcattatctacctggagagaaaagatctcgtgaaggcaaaagcctatgcggagaaggcgatcgtattcttccggcaggaacaccagttaaaaaacgagcttcaaacaaaattaatcctgggtattgtcgctgaacttagtcagcatacagaagaagcattttctatatacaacgaagtaaaaaaccacgcagccgccaaccagttttttgatctatatattaacgcaggtcaaagattaggtgatcttcttattgctgagaaagaatatgaagatgccaaacggttactttccatggtatatgcaaatgccatccaatggaacgacatgaaggcgcagctaaaagtgttgaatagcctgcgagccgtacacgcagccactggcgactataaaaatgcctatgccatcatgacgcagtacatgggtatttccagggaaatactggatctgcaaaataaaaaagagatcaatgagctggaaataaaatatcagaccgttcagaaagaaaaagagattttaaataaagaaaacgaactgcaacatcaaaaaacaataaaatatagcctgttaataggattcctggtgatcctgttacctgttatcggcctgttgtatatgtattaccagaagttgcaggcgcaaagcaagctgaatgccaccatggatgaagtgaatcagcaaaagatagccgtgctgttaaaagataaggaactggcattgctgaaagcctctgtgagcgggcaggaaaaagaacgaaaacgaattgcagaagaactgcatgacagtattggcggtaaccttgccgccattaagcttcgccttgcccatcaaaataatgtgactggaataaaagaggtgataaaacagattgatgacacctatcaccaggtgcgtgatctttcacatgatctcattccacagaagttcaataataccgggtttacagaactgattgccggttatctcaggcaatttgatgttccggggaacgccaaaatatctttccaagcttatcccagggaagaaatagatcttattggcaccacgctgaaagtggaaatctataagatcatgcaggagctgatcaccaatacccaaaagcatagccaggcatcgaaagttgaaatacaactgacaaagatcgatggtttgctaaagctgttgtttgaagacaatggcaaaggttttcctgtagaaaccaccaaatatggcattgggtttcagaatatacgggagcggttaaaattatttgatggggtgctttctattgactcctttccgtcgaagggcaccgtaatagatattgaaatatccttaaaaccagaatggtatgaagcataatattattctagcagatgatcacaaattattcctggaaggtcttatcaggctgatagaaaaggacgaaaacctgcatatcctgtattatgcgcataatggcaagctggtgatgaattacctggaccagcatccggatgagcaggtagacctggtaatcacagatatcagcatgccggatgtggatggcatcacgctgaataaccacattaaagaaacacggccggaaatctgcacgctggtggtgagcatgcacaccgacaataatatgattgatgcccttattcagcatcatgtggatggtttcctatcaaaaaatgcagattccgatgaatttcttaaagcgataaagatgatcctgaaaggtgaaaagtacttttcagacgctgtaaaacagggttaccttaacagtgctttttacaaggaaaaagaaacccttgaaatgctgacctcgcgggaaaaggatgtgctgaaattaattgcagaagaatacaccacccaggaaattgccgataaactctttttaagcaagcataccattgaaagctaccgcaaaacacttatcctgaaattaaaagtacgcaacctggcaggcctcaccaggtatgctgtaaagctgggactactcagctaaccccctgaaaacagggtattgattttcactgaaaaccatgttgttgcccggcatgcgacggtatacctttgtttcaaataaaacgggatgatagttttttttggaatgagggaaaaaaagatcggcctgcagccagtgtatcagcactcctgcaatcattgttcgcagaggaaaagtctgcacatacaaacgaactgcgtttaccttcatgtgttctggatacctgtctttcccatttataaaaaagcttacagcatttgcagcagttgccggcaggcattagccagcaacgccatgcctccggacttacatacaaaagcccgcgaactaaaaaaacaagcgaaagttccctggtacctgtttaccggttcgggccttgtaatgctgttcatcatttttgcaattttcatttctaatactaaaaattaatcaccatgatttacggaatctctctgatcttattaagcatcattgctgtcccttccctgatactatccagaaaacccaacgcaaaggaattgttggaaaaagtagaaccttaccagggatggataggcattattttctgcttctgggggatctggggtgtagtaactgccgtactccatatgggctggcttaccgccgctccgatttggtggaccacattaacagctggcagccttgtagaagcctgcctgggttttttactcggatacccgctcatcaccaaattattcctctccaaaagcgaaaaggcgatggaaaaggcggtacagatccgggcgaaaattgcccccaaacaaggtaagctcggcatattgggcattatcgtaggcgtatggatgattgctgcctctttgatctttacgatagcgtaggaagttattcttcagcaattcaaaaataaaaccaatgaaaaaaatattattggccgcaatgatgctgtttgcagcattgtacagccattcacagggaaaagagagttccattgaagtcaggggcgttgctaaaatagacagggagattgaatcctacctggtagattttgctatagcagccgaatatggagaaggggaagggaaaaaagcttttgaagatcttaagaataccttttttgccaaagcgaaagcggcaggctttgaagaaagccggtttaaagaagataaaatgggataccaggcgttgcaatattacagggaaggcagcttatacacatttgaaacccgtaacaaagaagaacttttaaaagttgttaaactggcaaatggagtggtggtgactatcgtaagcacccggttaagatataaacctgttaaagacagcgaaaaactatacgctactgcattcagcgacagcaaagaaaaggctgccaccattgcaaaggccatcgataaaaaattaggtgcggccattaccgtgacagatcttacctcacctgaatcagtatctgaagaaaacttctactataagccggtaacagatcaatattactatctgtctgttaaatttctgatagagtaatagtgatttgctaccggcctgccattcattgttattaccccaataattaagcgaataaaaaagaagaagctgtctcataaataaatgaggcagctttttcattttaggctttaaggatggttttatccacaatttgcagttgaaaaaaagggaagttgtaagtgtttacgcaccagaagttattgtgtaa

SEQ ID NO: 18 - DNA, 59323 bp, Chitinophaga pinensis
  source 1..59323: mol_type = genomic DNA
aataacttctggtgcgtaaacacttacaacttccctttttttcaactgcaaattgtggataaaaccatccttaaagcctaaaatgaaaaagctgcctcatttatttatgagacagcttcttctttttatcgtgttgcttcgtacaccgggtaatctgtatacccatgtgcggcccctccatagtgtaaattccgttcgggtttatttaatggccagtcgttttttagtcggtcagcgagatcagggttggcaataaaaggttctccccatgcagccaggtcgatgatgccgtcagttaagtactgctccgccttttcccggttcatgccacctgccagtatgatcacgccgttgtattgttgtctgaaacgttccaggaagccgtcgggtaaagcaaagctgcctctcgattgctggtccatgatatggatataggcgatgttccgcttgccgagttcagtggccaggtagctgtaagtagcctccaattcatcatagtgcggcatttcatgcaggccaccatacggcgtaagacggatcgctactttccccgcaccaatattcgcaatgcacgcatcgatggcttccagtaaaaagcggctgcggttaacgatgctgccgccatattcgtcggtgcggttattcacaaaaggattcaggaactgttcaatcaggtaaccattggcgccgtggagttctactccgtcgaagccggcttttactgcattggcagcggcattggcaaaatcctgtaccactgcttttacaccttcggtagttaaggctaccggaacagcgcagggaacaaaagcttcctggccgttttcattgtaggcccatgcatgcgagttggcagcctggatgttggaagcgcctacaggtgcagcaccgccaggttgattggtggtatgcgacacgcggcccacatgccacaactgcgtgaatattttactgcctgctgcgtgaacagtgctggtaaccagtttccagccttccacctgcgccggtgtaaacaaaccgggaatatgcaatacgcccgatgctgtaggggagatggaagtgccctccgtgatgatgagtcctgcgttggtacgttgccggtagtacaacgcattcatttcattgggtattccgttaggattccgtgcgcgtgtcatgggcgccatcacgatcctgttctttaatgtcaggcctttgccggtatatggttcaaataatagcatgggttgtttttttaataatcggataatcggtataacctgccgcactgccaccaaaaaatttcgacctgtcaggctcattcagcggcaactggtgttgcaggcggtaagggagatcgggattggcaataaaagggcggccaaaagcgatgaggtctgcccatcctttctgcagcgcttcttccgccctggcaacggtatacttgccggcgtaaataagggtaccggagaaggcttccctgtaagcttccttaaaagccaccggcatcacgggtgcattgtcccagtcggcttccgcgatgtggatataggcaatgcctatgtcgttcaataccttggctgccgcgatataagtttcttccggatgatcgtccatagcgcccatcaacgtggtcaacggggcctggcgcacgcctacacggtgctttccgatggcatctgctactgcggttaccacttctttcaggaagcgcaagcggttttccagcgaaccgccgtattcatctgttctgtgattggtttgtgaatcgatgaactgctcaatcaggtagccattggcgccatgcaattccaccccgtcgaagccagctgccaccgcatttttggcggcttgcgcaaaatcactgataatagcctgtatttcggctttggtaagctcgcggggcatagagtgctggagcatttccccggcgccgttttcggctccttttcctgtgggatcggcaaatactttcacgccttctgccaggataggggaaggcgctaccggcgcggcgccgttttcctgtatggagatatgtgaaacccgccccacatgccacaactgggcgaagatgaggccattattggcatgcacggcgtctgttacctgtttccagcccgctatttgctccgggctgtaaatacccggggtccaggcgtagccctggccctggcggctgatttgtgtgccttctgatatcagcaggcccgccccggtacgctgactgtaatattctgccatcaatgcggtggctacatcgccgcgggccgctctggatctggtcattggcggcattacaatcctgtttttcaggtgaagtccgcctagcgtatattctgtaaaaagcatcgtcttcgtattttgataaggcaaaattcttccaaaatttattattatcataattatttaacttatacctttgtatcagaaaaatgatattatatgggactcaacctggaatggctccgtaccttcaaatccatctatgaacagggcaccctcaccggggcggcacaggagctttttatttcgcaaccaggcgtaagcctgcacctcaattccctcgaggcatataccggctataaattatttgatcgctcggccaaaaaactggtgcctaccgaaaggggaaaagtgatctataattttatcgaggaacctttactcaaactggaaaatgcagaacagctttttcataaaagtaccagggccgacagagccaccatcagcattggtatgtgctttgaaacatttcaatatacactggagaaatatattgccaccctgccctttaacgtcatcatcaaattcggcgactacccgcaaatgatcaacgacctcgataaaggattgctggatcttattatcacaccgcaaaaaggggatcagaaaaacctggagtttaaacctttttcaaaagaaagaattgtactggtggccggtggcaaaacagatatcaaaccactgaacgctttactgaagaagaaagatctcaaagcagcggagaactggctgaaagaacagctgtggtacagcaccgcggcggacatggagcacctgaaacgattctggcagttcaacttccatcatcaaatggattttaaacccaactacattgttccgaatatctgctctattgtgcgctgtctcagtggagaaaccggtttttcagtagtacccgactttttgtgcgcccgcgaaattgaaacaggcagcatgaaactggcgtgggaaggagaatcgatcatggaaaataccctgtatttcggtacacggaagaaaacaatgtatgcggcggaaatagataaagtacaacggatattttctacagaactatatagtccttcagtcgtgaatagttacgctggcagccaccagtgatttaatatattcagtaggtgtaaggccggttatctttttaaaatactggttgaacgatgacttggctttaaagccgcaatcatacgccagtgttaacacgttcaccggcaacgctttttcattcatgaaacggatctgttccatcgcccgccggatacgccattcattgatatactggtaaaacgacttgccggcataactgttcagcgtttctgaaatatgatacttgctgatcccggcgccctgcgcgagtttatcgaggttcagctccgcatccgtaaatatttttgttttatgaagataagcttccagcgattgtaacagcagccgctgctcatcagtactgagatgcattttgcgggaaggcaatacctccgctgctggtccggctattactttcaccggctgcgtgcccatgatccccacatacttgtacctgataatcaccaggcacaccactaacagtaaggaatatacgatatctctgcagataatattatacgagccatccagcatatgcgccgattgcgcggttttaaatcccaatgaaataatactgataatgcccagcaggtaactgatactgttgatcagcttcttctcctgcggcatatcaggtaattgtttcgcaatgcggagtgataataccggaaacaggaaacccaacaccatcatcagccatgtggtggtttcattgtagtaatacaatacagcatgaccggcatccgccgaccacatcaacacgcataccaccgtaagatagcccaccgcgccaagcataaacggcagaaaaacataccaccgcgaagcaggaataaacgcggtatcccgccgctgacaggcatataaatacagcaacggaccgtagcaaaaaccgataaatgtattcatctgcgtacgcacttcggggtcgttcacaaatgaataaatgcaaaacttgatagcgagatgcgcagcaatactacacagcaacaggatcagcagaaaatctgctttactgcgcaacttactgctgcctagtaaagcaactgcggtaagtgcctgaaatgctccgatggcaataacatatatcatagtgcggatatgcaccgaaagtataaaaccaatattaccggaatgttaaacctgctgcatcggatggctggtgatccatttggtaatgatttcgtaacacatgttaatgtattgggtttcaataaaagtgagtacgtttaaaacagaaaatacgcctacgcgtagcagtagttggatgcggtcgtagtcatcatcagcaagcctcacttttgttgaaaaataccttcatatggatcgcatttttataccattaaaacgctcccgttactgcacattactggttttactggtaatggccggcacggcaaaggcacaaaccatcaagggaattattaacggcagggaaggacacctgcccggcgcttctgtacaaaccgccggaaccagacaaggcacctccaccgatctgaatggcgccttcaccatcaacctacacaccaccggtaaagtaacattgctggtatcttatataggacacgaaacgcaacgactggaactaaccgtaaaacccggtatcaacgacgccggtaatatcacgttgtcgcccaccggcggtaaactgggagaagtactggtaaagggaaccatggcgccttccacggtgaaggccctcagcattaaaaagaattccctcgccatcatggatgtaatcgcggccgatgccattggtaaattaccggaccgcaatgccgccgaagcggtacaacgtgtacagggagtggcggtagcccgctatcatggggaagccgatgccgcgactgtgagaggtacgcccttcgcatggacatccacccttttcaatggcagccgcctgccaagcgccaacgtactcggtaaccgtaactcggtgctggacgccgtgccctcagaaattatccagtatgtacaggtggccaaagccatcacaccagacatggaaggcgacgccattggcggttccattaatttcatcacccgcatcgcccccgctaaaagaacactcaatgttagcgcggcaggcggttacaatactttttcaaaagacgctacctacaacgcatccctggtatacggagatcgcttttttaaagataaactgggcgtcatgattgccggcgccatctgggaccgccagtggggaacagatgcgtatgaagtggcctacaataccggcctgaccaatcccgcacaacaaaaatctatcagcaccgtcatgctgaaacgatatatgggtaagcgccagacctatggcgccaacgtcggacttgaatataaattcaattcctccaataaaatattctttcgtggcctgatggataaattcaacgatatccgcccggtatatgaatcctatgtggattacaataacagccgctatcagtacaactaccgctactcttattaccagaccgtactcaacggcggtgaactggggggcgaacatcagctgtcttccaaagtgaaaatggactggaccgtcagcgactactacacaaaatatttcctggaaacaccgcccaccaacaataataaaggattacccatcgctactttccgtcagaaaataaacggcgggtttaataatctttctgcagatgggaaacggtactggggtttcgattcaccggaaggtgtgggcggtgatccgctgcactttgatgccggcatcaaaaacagcggggaagtaatggacccgtcgaaactcactttgcagcagttagtaattgcgcaactggatacaaaagaagaagataaaacggcacagctgaacttcaaagtgagcgcctcttcgcgggtaaacctgaagttcggcgccaaataccggcataaagaccgcgccggtatgtatggctccaacatcgtatatctccccggcgctgcactgggcattcccaaatcgccggacctgctgccgctgaacacactccagcgcaccgattttccggtacgtggcggcttcttccagggactgaaaggtaactatgatcagttcatgatagatcccatcaccaaacaacagctgtttgatttgtatgatactgccaccctgcggaaaaacggctttgccgactacacttctaaaaccaatgccaccaacatttatacgggtacagaaaatgtagctgccgcttatgccatggcagaaatcgatctcacagataaattaaaaatgattgccggtgtcagaaatgaatacacggcatttacattgcatggctccaaagccactgctgaaggcactccaaaagtaaccaccattacaccggctaccgtcaaaaacaattacaacgcgctgctgcccatgatgcacctgaaatacagtatcagcgaccaggcaaacctgcgcgccgcttatacccgtactttcatccgtccaaatttcacggatctaacccccggcgaatctgtggacaacaccggctccaacgtcaccatcaccaaaggaaatcctgatctgaagccaaccttctccaataacttcgacctgatgggcgaatactatttcaaaaatattggtctcatttccggtggtgttttttataaacagatcagcaatgtaatttttgccaataaaaattattacacggagaatggcgtgaactatgtagtggcacaggcaaaaaacctgaacaatgcaacgctcgccgggctggaagcgggtatcaacaaacgcttcgattttttaccgggcatcctcggtggattgggcgctgagctgaactacacgtttatcagttcttcggtagaagtacccagaaccgtgagcggaaataagatcaccgataaaacaagtctgcctaaccaatcgcgtcacctttttaacagcatcctcttttatgaacgcaatggtcttatgatccgtattgcaggcaattaccgtggcgcatctgtggaaacgatcaaccagcagctgggtaaggatttttatatctggacagataagaactttaccgtagatgcttccgctactgtaaacatcacctccaaaatacgggtgtttgcagagctgaacaatatcaccaacgaaccactgaaaacctatatgggtgacaagcgccgtgttgccgccgaagaatggtatggcagtcgtggtcaggctggtatccggtgggacatcatcaaataacatcatctctcaaaaaaaataacaaatacaatatgaaaagaataatgctggtactggctatagccttacccatggcaacctttgcccaattggccgatagtgcacaaagagttgtgcgcatgcagggagcggttaacttccgcgatgtaggcggatataaaacaacagatggtaaagaagtagtgtggggtaaagtattccgctctgctgatgtaagccacctgacagaccaggacctcaccgtactggagcagaaacatattcataccgtcatagatttccgtggggtaaaagaagccgctgcggcgccggatcatttgctgccaaaaacggattacctgctgtgccccgccggcagcgatagtttgccaggtgctgcacaaatgggcgaaattattaagaagggtaatttcctggagaagttttacggcaacacccaatacctgggcgatcgttataaaccattgtttcagaaactgctggtgttaccggccaatgaatccatcatgtaccattgcaccggtggccgcgacagaaccggcatggctaccgctttgttcctttatgcattaggtgtaccgcaacaaacaattgaagccgacttcaccgccagtaacgtatacctgttgcccatgaataagcggatgttccagggtatgcaaaaaagtacaggtatggatgaagaaaccatccgtaaagcactggaactgaaaccggaattgctgcacagcctttttaatgccattaaaggcaagtatggcacggtggaaaatttctttgagaaagaattaggtatcggggaaaaggagcgggcgatcctgaaagagaagtacactatttagcagtaaaagcggagggatttccctccgcttttacttattccttcattccttttacaagggccacaatcgctaagccgcacatcgccataatggcaaacgaccagcgtaaactggtagcctgggccactaatcccaccagtggcggcactatcataaatccaagatagccgatggtggaaatggatgccagcgtttgcccgctgttggtgctcttcgagcgtcctgccaaactaaatacgagcggcactacacacgctacgcccagtccggcaaaaataaacccgataccggcagtaaccggataaggcagcaaaatagccagcaataacccgctgaggatgaaccagccactatacagcagcattgatttaatacccagcctgttgacgagcctgtcgccgataaaacgcccggtggtcatggctaccatgtatataccaaatgcagccacggcagtggatttagtgctgccaacaattttttcaaagtatagcccgctccagtcatacatggtgttctccgtagccatacacgcgaagcagatcaaagaatatttcaataatgatttatcaggaagcgcaaaggccgctctttttactgtttccctcaccggttggtccggtaatgtttttggataataatagatagtgaataccagtaataaaacactgatcatcagcaaatgataggaaggcgccacgttcatggtcaccatcaggtatccaatagctgcccctgcgaagcccgccacgctccagatgccgtgaaaggtggtcataatagattgcgggaacaggtgctgtacctgtaccgcctgcgagttcatggaaaggttcagcaggttacgggcagagccaaaacaaaataataccagcgccagctgccagatactggtggtgaaaccaggcaggctcagtatcaggttaaacaccatcgcgccaaataccatgatcttcctggcgctgaatagccccagcagcctgccggtaatgggcattgtaagcatcagcccgataggcagggctaataacaccaatccgaactgcgcctcgtttaaatgcaattgttgtttgatagagggtatcctggaagcccaggaggagtaacctaatccggagatgaaaaagaagacggagatagcgatgcggtattgcctggcatcggtttcattttgaatatttgctaacatgatctgcgctcacacacctgtttgtggcatttgacgacgcaaaattaggcaaatccggggagaaatggccttggaaatgcaggggattgtattttaccgtttaaacaagtcttccatcgttacttcgttctgaatgattcctgttttatatacattgtctttggtaccgtaagtagtcaccattgtaaggaacaaagtcttttttgtacccgtcttttccttaaaaacgtgcaatttgttttctaattcagtagcataggatttatcaatagaaaatgtggcatttgaaaatttcatttcacagacattgatacagccgtcctgcctgtcaagcagcaaatctatttgggcacctttttcttttttttcaggtgttgatctccaggcagattcttctgtatagacaccggagatccccaaagcatgtttaatctggttggtgtgcttcaggcaaataccttcaaaggcgctaccgctccagctcttccatgactgagaggtcgacagtttcatccaggtcccctttcctgttgccctggtatgctcaatgaatttgaggtagaataagctgtattcatcaattaatttataaaccccatcccgtgtatttttttgaaatggcatatacatattcacaaaagcggactggatcagctcatcaagcagcctcgttgtggtaccaccagtgtgcaggttacaggctttaatgatctcttttcttgttaaacctgacggctttgccgccagtgcctttacaactgtgatatggcggtcagccatttcaaataatgagtgatacagattattgaattcacctataagcagtccgtcctttgtgaaacacaggcggtctatggcctgcgtggcactttcccctcttgtgatctccttgaggtaatgcggtactccgccaaaagccatatatatctgcaatatttggtatgtatccagattcaccgatttactgtggagataaaccgatgtttcataaagggtaaaaggtagtaaacggattttttttgtaatccggttatgcagtcctcctttgttattaacaattttctgaatcatccatgatgctgcggagccacagatagcgactatcagttgaggttgctttgatccccatgaattccagaaatattcaaatgcggataaaaaaccagatttgtgagaacttagccagggaaattcatcaaaaaatatcaccttcttttcctttcccagtaacggtgtcgaaaattttatgagcagaagaaatgcttccgtccaggttttcggaaccgcaggcggtatgggggaatttaatgcaatggcaatactgtttctgaaattctccagctgttgttgaacagaggcattatgtacgcctgagaattcgcaaatgagctgtttatgataaaactgccggatcaggaaggtttttcctacccttcttcttccatatacagcaacaagttctgcttctttagaaactaacgtctgctgtagtgtctttttttcgctctccctcccgatcagtttttccatattgaaatagtttaatgttttgatagttatggctgcagatatatctttatccgcagccataactatacaaatatacatacttatggctgcagatcaaaatatatccgcagccataactgctaagatgctgttttttccgccaggatgtgggagtggccgggagccgctgttgcctgtttctccatggcggctttgaatgaagcattatctcggcaacaggtacttaaatactgttatctcattgataagagatcacaaccgataccccacagtaacagataaattcctgtttttataatcccgttcggaataagtagcctcctccttaatctccccgatatttatcaaacccggctcatagtttacccccagagaaaaccttttatattccacccccacaccggagcttatcccgaaatccgttcttgataaagggtgtcgtgtatccccgaatgtatccgttgaggttttttcataatcggttttcccggacgagtgaactgttttgttctttgttacctcttttcccccgataccataagcaatataaggtcctgcatttataaacagccgggtactggaagtaagcgggagtttatacccgataagaagaggcaactgaagataagtttgattggttattattttgctataggtgatcggcgcattgccgccgccaatccacctttcagcactttcgtgtatggtccctttgacggtgagtgaaacaccggatcgtaaataaaccgcatccgacaggttgtagtctgtaataaatcccacctggaatccgggcttactctttttgtctccaataatatagttcactgtttcattggcattcgacaggttaaacccggcgtttactccaaacgtgaagggtttgtgttgtgcagtcacctgaagaactgatagtagtattacgcaggttgaaataagtaatttttggacactcatgctacagtataaatttatcttcatccgggaataggtttaaatccagcgcattgtaagcgctgcggaataaaagtaaatattaaaagttcttttcctggagaaaaaaaggcgcttcttatcaaggatgtttttcttccgcgtatgcttaacatcattatttgattgaaatagtacaacatttggaaaagaaagtgtcattaaagtattttatacgtccgtacttttagtgtcctgataacactcgtacgaacgttatgaacaaaactacttttacaagcagtacttacgggacttccagccttctttgccaaagaaaaaagcaatccggatcagcactgcatcatttgatattatatcagctgggcttaacaggtattacaggtaagcataagctgcggattaaaaaagtaccggtttaaacatctcctgagtcagccagcaaccaagtcattattcacatataaaaacagttcaccggaaacacccgtttccggaaagggaatctttttgcctatctgtactacacaatttaatatgaccgttatgaaacgatgccttctttttattttctttctcacgctgatagtaccactgggtacttatgcacaacagcaaacagtaacaggagtggtacgggatgccaccaccggcatagctttgccgggcgtaagcgtacaggtgaccggcactactgccggcgcggtaacagatgccactggtaaataccagttgaatatccccgctaatggcacgcagctcagctttactttcatgggatacctggccaaacaggaaacccttgctggtcgccatacgatcgacattcaactgcaaccggataccaaagcgcttggtgaagtcatcgtggtaggatatggtacgcaacgcaaatccgatcttacttcttctattaccaaagtagatcttgccggtgtaaaaagcgcaccggtaacgggcgtggaacaggcattacagggccgtgcagccggtgtaactgttacgtctgcatccggcgtccccggctcaccggtaatggtccgcatccgtggaataggaacggtaaataataacgaccctctctacgtggtagacggtgtgccggtaagtggtatgaactatctcaaccctgctgacatagaaagcatggaaatcctgaaagatgcttctgctaccgccatctatggctcccgcgctgccaacggcgttgtgctcatcaccacccggaaaggtaaagccggtaaatcacagatcacgctggatgcatattatggtctcaacagtccgtggaaagattataaaccagccggccgcgatgaatacctctacatggtaaaaaatgtgtacggcgaaactaccgatcagtataaagatgcactggcacagtataataaaggatataatactaactggtggaaagaaacggtgaagaagaacgcccctgtgcaaagctataacctcggtgtatacggtggcaccgacaaagtaacctatgccatcagcggcgggtacttcgatcagaaaggtatcatcgatccctctgattttaaccgcatctctttccgcgccaacacttctgcgaaagcaaaagaatggcttactatcggtcaaaacctcagcatctccaacgaacaaacaaatgtaatcggtgatgaaatccccggtatcatgggcaacatcattccctacgatccgctgatccccgtgctggacccatcaaaagaccagagcgatccatacagcaaatgggctacctctgccaccgtattcggcagcagccctaaagccatcctggcaagggaagtaggcaaacgaaatacactgcggatggtaggagatgttttcgccaacgtaaacatcctcaaaagcctcgtgtttactacccgcttcggattgaacatttcccgcgcagatgaatggactttcagccctacttattatatgaagccgagcgacctgctggaaacgccgcaggccaattcttcaaaggcatctaataattattacaactggacaaacacgttgaactggacggagacattcggccagcatcgcctgaatgtactggcaggtatcagcgcggaacgcagccgtgacacctatcttaatggcagcaaacaaggccagctgggcaacgaagaaaactactggttcctcgatgccggtaacatgaacgacaaaagcggtggcggcgcagcgcgctggtcgctgatgtcacagtttgcacgtgccaactacagctacgccgataaatatttgttctccgcaagtgtgcgccgcgatggctcctctaacttcggtacagataaacagtttggtgttttccccgccgtttccggtggctgggtgatcagcagggaacagttttttgaagatatggaccttgcctggctgaccaatgtaaagttgcgcgcaggatggggacaagtaggtaaccagaacattcccaacggcgcctacaccacgtttgtagccaacagcctgggtcgtaactacctgcttggtaacggtacatccgtggtaatgccgggctactctatggataatcttggcaacgggaatatcaaatgggaaacagcggagcagtcgaacgtaggactggaactcggattatttaaaaacagcctgaaaattgaagcggaatattttaaccgcaaaacaagggatatgctcatcgctatgccaactgcctccatgtttggcgtgccttatccctgggtgaatgccggtaatgtaagcaacaaaggctttgagctttctgcgaattatgaaggcgatgctggtgcaatacactatgctgttggtggtaatatttctacctataaaaatgaagtgctgagcctcggcggtggtcagccatatgtggaagacgtaggctggcaactgcgtgtactcagtttctccagaacagcagaaggccatcccatcggtgaattctatggctggaaaacagatggtgtcttccagtcgcaggctgatgtggacaactacaagagcagcaaaggcgaggtaatccagcccaatgcaggccccggcgatttccgcttcaaagacctgaacggcgacggcgtgatcaacgatgcagataaaaccgccatcggcagcccgcaccccaaatttacatacggtgccaatatcaacctgtcgtacaaagcatttgacttttcgcttttcctgcaaggcgtttccggaaataaactgttcaatgccaccaaatatttaacaaagcatccgcttggctttaacaacgtggaggccggcgctgcctacaatgcctggacaccggaaaatcactccaacgaatatccgaaaatgtcggtgaacgatccgaacgataactaccgcgcatccgactggtatgtggaaaacggcagctacctgcgcatcaaaaatatccagctgggatacacgctgccggaagcattgatcaaacgcatgggactacaacagttacggatatacgtagctgcacaaaacctgttcaccttcacaaagtataccggtctggatcctgaagtaggcgcttaccagttaaacagcagcgaccagaataaaatgtcgcgtttgatgggggtggataactacacttatccacaagtgcgcacgatgcaggtaggtgcaagtttgaaattctaataactttttaactgacaagaaatgaaaaggctgatatatatagcattaccggcagcactcttactgggcagctgttcaaaagattttatcaaaggcgacgtgcccgccaaaacagacgtcaaccagttctatagcaatgcaaaggaagtaaacatgggcctgatggacgcctatgatgctttccaggaagaagaatcacaactggcccgcttcgtatatggcgatatggccagcgacgacgccctgaaaggcggtgaaaccattggcgacggcccggatatggaagccctggtggaatgccggccactgtctaccaacgactggtcctataagctgtggacacaatgttacaaagccgtcacgaaagcaaatatcctggtggagagtattgataccaaagcggattttaaaggagatgaaaccacgaagaaccgctaccgcgcagaagcacagttcctccgcgccctgggctactattacctggcaatggcctacggcgatgtgcccctgttcaccaacggcgttaccaactacacacaggtagatccgaaaatgatgatcaggaaaccggtggcagatgtatgggcgcaggtggaaaaagacctgacggaagctattcccgcactttatacaaaacaaaccattccttcttcggagttggggcgtgctacgaaaggcgccgcacaggctattctcgcaaagtcactgatgtttcagaagaagtatgatgcagccgtgccggtattatcagacctggtaaagaacggaggctaccagctgtcgccaactttcaattcgctgtggcgtccgggtacgggcgatttcaacgccgaaaatatttttgaaatcaactataccaatacctggaactggtccagcgatggagaaggcgctatccgcaatgtatacgaatcatcccgcaacacctggggctggggctttaaccagccaacacaagacctggccaatgagtttgaagcaggggacccacgtatcatttatacgcttacctattccaaagatattttccaggcaaaaacacctgcggaacaggtggaagaaaagaattccatcaacaacgtatatcagtaccattcctataaagtgatgatgttgcaggccgaacgcgacggcatgaccaccggcggcgccggcatgaacgaaaaaattgtccgcctggcagatatgtacctgttgtatgcagaagcactcgtgcggtcaactgccgctaaagatgtaaataccgccgtattttatctcaacgaaatacgcaaacgtgccaacaacacacctaaagccgacccggtgcgtgtaaagcaacaatttaccgttgctgccaacaccttgccgatgcgcgtgtataccagcgatgtacaactgctgaaagatattgcgcatgaacgccgcgtagagctgggcatggaaggcgttcgtctgtgggaccttatccgtacagataataccgttgcactggatgcttactacaaaaaatggggcgccaacggatatgaagcaaggggcgatctgaaaggaaaattctatggtacctggatcagcaaatttgccggtggtaaatatccgaccttccccattcctcaaaaagaaattgacctgtcgcagggcaacctgaagcagaccagtggatattaaatcatgtttatggagtatacaatgaaaaacacagccctgcaggtagaacagctgcaggcacaatatgagcaactggtacgacgcaccaatgaacctgcgggtacatacaatggtatttatgacaggtataagtatcccgtactaacggcagcgcatataccttatttctggaaatttgacctgaatccggataccaatccattcctgcaggaacgtatcggcatcaacgcggtgttcaatgccggcgctatccggctgaatgataagttttacctcgtggccagggtggaaggcagcgaccgtaaatctttctttgccgtagctgaaagtccaaacggtatcgatcacttccgcttctgggattatcccgttgagctgccacaggtggccgaccaggaaaccaacgtatacgatatgcgtttaacacagcatgaagacgggtggatctatggactgttttgcgtggaacgcagggatccggctgcagcaccgggcgatcaatccgctgcggtggcgcaatgcggcattgtccgcaccaaagatctccgctcctggcagcggttgccggatctgcaaacaccttccccgcaacaacggaatgtagtgctgcatccggaatttgtaaacggcaaatacgctttttatacccgtccgcaggatggatttattgaagccggaaatggcggtggcatcggcttcggactggcagacgatattaccaacgctgttattcacgaagaacaactgctggataaaaaagtataccacaccgtatatgaagcaaagaacggtttgggaccagcgcctattaaaacaagtaaaggctggttacatttagcccatggcgttcgcaacaccgccgcaggcctgcgttacacactctatgtatttatcacctcgctggaagaacccaccgaggtaatacataaacctgccggctatttcatggcgccggaaggcgaggagcgtgtgggagacgtatccaacgttttattttccaacggttgggtaacagacgaagaaggaaatatctttgtatattatgcttcgtcagatacgcgtatgcacgttgccgttaccacggtggataaaatgctggactacgccatcaatacaccggcagatggttttacgtccgatagtaccgtacaacgtatatgcgaacaggtgagtaagaaccagtcatttctgtaatgtttaaatgaacaacatgaagttaagaaccatcatcactgctgcattgatgggcgccataccggcgctcgcccagcagcagcctgtcgataaaaaggctacaccggaaaccaggcagctgctgcataacatgtcggcgctgctggataagggcgtcatcctcggccaccaggacgacctggcctacggcatgcaatgggcctacaaaacagacgagtctgatgtgaaaaggttaacggggcagtaccccggcgtgttcggttgggaactgggtcgtctggagaaagacagcacccataacctggacggtgttcctttcgattctattgtggtatatatgaaatgggtatacgaaaacggcggcatcaatactttcagctggcatttcaacgacccggttacaaaagccaccgcctggagtactgatccgaacacggtgaaaagtattatccccggtggtgcgcatcacgcggcttacaaagcttacctggataaactggccgtttatcttcataaaataaaaaataataagggaaaagaaattcctttattgttccgtccgtttcatgaacataccggtaactggttctggtggggcaaatcgtcctgcacaccggaagaatttaaagccatctggcagttcaccgtcaactacctgcgcgatgtgaaacaattgcataacctgctgtatgcttattccgccgcggattttgctacagaaaaagaatacctggaacgctatcccggtgatgcctatgtggatgtgctgggctttgatgcttattgtaataaagacgtagcctattttgtaaaagatcttaacaaccggttaagtatccttcagcaaatagccgccaaacaccacaaagtgccggcactcaccgaagtgggtaacatcaatacgccacaggcggagtggtggacaaaaacattcctgcccgtactggaaaagtataagatgtcttatgcgctcttctggcgcaatggaccaaaggaaggcgctttcataccttacgaaggtcaggtgagcgcagcagattttattaagtttgccacacaaccgccggtgattttactgaaccagttacaaaccaccgctgtttataaaaaatagcaggttgttttcaggacaattatatattttgtaggggagagatgattaccgtggaggtaatgatttctcccttttctgtatttaaatgtccacgtgttatgtccttctttaaatatattatcagctgttgctttctttacctgcctgtagcggcgcaggtaccggttgacctccatgcgtacaagccctctggcgaagtaaaggtaagcgtagcagatcaacagctcaccgctgtgtggaatgccggcgctaatacacaagcgcgtattgtactgaacatggaacagcaaaacccgcttattcacagcctcagctggaacaccggtaaaaaagaatggcagcaggtggcatccggtttgcaaccggtatttttccttaccaccggtaaacgcgacctggtttcacaaaacggatggaatatcttctttgataaaacggataaattaccacgtactacttacccggtacagttgcagaaagacagtgtaaccgttattacagatggctcccgcacggtattgcgggtggcaggtgctacggccggtccgtttaatggcgtggtggaaataaccctttacaacggcagcgggctaatgaatgtagccgccgtgatgaccacccaaaaagattccaccgcgatattatacgatgccggactaacggccacggatataccctggcagcaaattcaatggtccgatcccaaaggcgtgatgaagtcagtgccggcagtagcgggcacacaaaataccaacgtcgccgttaaataccgcaccatcatcggtgaaagcaaagccggcagcctggcgttgttccccgcgccgcaccagttcttttacccgctggataattgcttcaaccagtccttcacctggtacggaaataattataataaagatgcacccggctatggtatcggtatccggcaggaaccggcaggagataaaagatgggtgccctggtttaacgcgcctccaggcacggcgcagcgccttcatttcttttgtttgctcagtaacaccccagcagggcaaacgctgcagtatgttcgccgttatactcacagtgacgtctatacgccgcttcccggatactatacgatgagcagccattttcaccaggagcataccgccgatgtgttaaataagctgccgatgcccgaaattccggctttcataaaagcttttcgtgaaacgggtgtgaatattgtccacctgggcgaattccatggccccggccatccgcgtggtccggaaggtgaacgcttcctggaacagcaaacactattcaaagagtgcgagcgattgtctgccggaaattttttactgctcccgggtgaagagcccaacaacttcttcggtggccattggatgaacatctttcccaaaccggtttattgggtgatggatcgtaaacgggcacagccttttgtaaccaatgatccaacttacgggaaagtatatcgtgtaggcaataaagaagaaatgctgcaactgctgcaaacggaaaaaggcatggcctggactgcccacgcacgcaccaaagggtcaaccgggttccctgataaatataaggaagaagcattttttacctcgccccagtttatgggcgccgcctggaaggctttgcccggtgatctttcacagccttatctcggcaagcgggcactggatctgctcgatgatatggccaactggggcctgcacaaaacaatgattgcagaagcagatcttttccgtatcacgccggaagatgaactgtacggacacctcaacgtaaactatcttcaattggatcggttgcctgcttttaaagagggttggcagcctgtgctggatgccatgcagcagggaaagttttttgtaaccaccggtgaaatactggtacccgcttttacggtaaatgggaaatcttccggcaataccatcgccgctgcagagaagggaactgtgaaagtaactgccagctggactttcccgcttaactatgcggtaatcatctcaggtgatggaaaagaggtttaccgggaaaaaatttcactgcatcagacacattctttcgggtccactacatttacatttaataccaacctggaaaaccgtaaatgggtgcggtttgaattatgggacgttgccgccaacggcgcatttacacagtgtgtgtggataaagtagcgggatgtaaatccgcttcgttgatcgctttaaattcgtctaacggggatgaacatacggaacagcaataatcttccggtaactcactgaaggcagtaccctcagggatttgctgttccggatcaccggcatcatcatcatacaccgttaagcacacctggcattgatgtactacccgttcaacagcggcaacaggcgccagcgattgctgctcggttacataatgctgtaatacatccgcctcgctttcccgttcgtaaaaagttctgcacagcgctacaatgtaaggccccaggtgctctttggaaacaccttcgcggtataacaacaactgcgcggagttggcgttgtaaccggccgtatacagaatgtcgtaacgctgcatatacttcagcttgctgccatgcttgttttcctgcttacggatcaccaccgttccaaaaagacttgccggccggttaatccttacactgaagcacaaaccataggtgcgtacatcggccgtatcaaagtaacggatgatatgacgtttcagcacaagcccgtcttcacagttgtcttccacctgccagtttaattcattcgccgcatggcgcacattgataccatatttccccaacacataatcccagagcttacggtgagccggttcaatattttttatgatcagcgacttccacggtgtggcatacaattgcccgatgcgtgtttccaggcaaatggtacatacttctttcaaaaaagctatcgggaaatcttcatcccgccggtaaatacctaaccagtaactattttcgaacttattaaaaccttcgtagtatggtaaatggaaagccggcagatcaggttccttctccttcgggcggccaatatagctcgctacctgtttcacctgctggtacacttcctccggggtatcgccttcgttgatactctgctccagttgcttgctcatggcagcaatgttattggtatagatcagctccggccaggcgtacagctgctggcttcccggcatgcggatatacaggtaccagtaatgcaggctgcctgaagagatccagttgatatgcccggtgaacaacggtacaaatgtttgctgactatcgcagatattgattttcagtgtgggcgtatagtcgaagccgttaaatacatctttataaattccttcactcagccagctgtcgtggataaagatgccggcagcagggtaggagctcatgatattaggctggtctgctatgggcaactgtttatctgcgcagttcttcttaaaggccgctaaatttttatccggtatatccaccagtaattgttgccgtaagccaaagcgcacatgcgtagcctgcgctgctgcagctgtttccagcagctccagcaggtatcccggtgaaataatgccaccggtgaaattaacgggtaaagtatgcgtgtgtttagccataattatacaagtgctgccacggttttctgaatcgatttttccagcagggtctttatttctgatttgcagctgccacagcccaaaccggcgccggaggcctggcaaagctgttgcaggttatcgcaacctcctgctatcttctccgtaatatttccttcgcccacattgccgcaggaacataccagcctgccaattaccggtgttcctttcttacctgaacgaagtaactccagccgcttatctgataactcaatcttttgctggatcagatccctgaattctgcaaactccgatttgtcgccaatcaggatggcgcccaccagccggtcctggtgaataatacatttcttataataacgtttcgccttgtcaataaaaacaacctcttcataagccgggtctttcggtgtttctaccataccaagcgaacaaagatcagtgccatgcatcttcaggatgttcataaacagggaaccctggtaataattgctgatgtcgccgttaagataacgggccactacttccgcctgctgctctgcagcggcagtgatgccgtacaaggtgccattgaaagcagcaatctcgccaatagcataaatttccggatcactggtctgaagatattcattcaccactacaccgcggttgcactccagttgcgccgcctgggccagttctatattaggcaccgttcctatagacattaccaccgcctggcagggaatgtacaaaccacttttcagctggatgccttccagttgatcctgcccggagaaacggttaatttcatcattgtaataaatctcaatacccctgtcggtaagttcttcataaagaagctgcccgcccagtgtatccagttggcggtccattaaccgggaagtgcgttgtataacgccaacgtctatattaatttctttgagagatgctgccagctctatccccaataatccacctcctgctatcattactttccctttggaaggatctatatgttgtttgaaggcatctgcatccatccgcgtgcgcatggtgaaaatgccggggatgggcggaatatcccgcagcgtggctgcccggctgccggtggccatcagcaggatatcatacgtatgtactttcccgttactgtcggtgagcaacttattggtacggtcgatatgcgtaatactgacgcccctgtgcaaggtaatattataggctttttcttctgcacgggtcatcttcaccagctgtttccattgctgggtaccgctgatataatccggaagcattacccggttgtaaaacggcaggtcctctttactgaacaccactatttcatctgaagtgtttagttcccggtacgactttacaaatccgcaggcgccggccccggcgcctattaccacaattttttgtaccggcttccggtagcgtgctacctgtaccgccgcatatttaaaatccggctgtttggaaatcggatcaagcagtggactagtcaggttattggcgcggtgaagatcgttttgaaggatttttccccagtgcatcgggaggaagacaactccttttttgatggtggtgctaagctgggctttcacccgtaccgtaccgcgttcattggtaacggtaacaatatcgtctgccgaaatgccacgttgccgcgcatcttcgggatgtatttcaaggaaggaggaggaaatatgctgcttcagcttacttaccttacctgttttactcatggtatgccactggtcgcgtatgcggccggtagtcagtatcagcggcagctcatggctgagcggctctgacctgttgtcatcgtcaaaactatgtatcaccgccttttcatcaggggtgtaaaaccggtggtcgcggaacaggcgcggcgtgccgttgcccgattgatagggccactgcacgctgcgctgcgcctttataatatcatagttcagttcacttacatcaatattggtaccggcagtaagccggcaatgttcgtcgtatatttctgatacattcgtatagtcgaacccgtgataccccattttttgcgcaaagcggcaaataatttcggcatccggcaacgcttcgccaggtgcatcatttactttggagagataactgatgcggcgttctgcattggtcatggtgccttctttttccgtccaggctgcggcgggcaatactacatctgcatagcgcaatgtttccggtttgctggaaatttcctgcaccactacgtactttgccttttgcagtgctgcttcggcaaagcgggcgtcgggtaaactcaccagcggattggtacacatgatccatatggctttcaaccgtccgtcgttcagtgcggtgaacatctcggtggcagtaaggcccggcttatcagaaagctctgtgcctccccagaaagcctgtacctctttgcggtgcgccgggttgttcagtacccggtgggcaggcaggagattggataaaccgcccacttcgcggccgcccattgcgttgggctgaccggtcagggaaaaaggaccgctgccgggcttgccgatatgcccggtgatcaggtgcaggttaataagactaagatttttatgcacacccaccgagctttggttcagccccattgtccagaaggtcatgaaaccagtggcattgccaatgtaatctgctgcccggtgaatatcttctgctgcaacaccgcaaatggccgccgcttcttctatggtgcgttccatcacggtatccttgtacttatcaaaaccattggtatgcgcttctacaaaggagctgtccgtaaagccggcagtgatgagcgccctgcctatggcatgatgcaatacaatatcggtacccgggttcacctgcaggtgcagatcggcgagcgcacagctctgtgtaaccctcggatcacttacaatgatcttcatggcggggttggctgccttcgcagcttctaccctgcgccataaaataggatggcaccaggctggattagcacctgccacaaagatgcagtcggcctgctctatatcatcataggtgccaggcactgcatcttctcccaaagccattttataagcagctactgcactgctcatacacaaccgcgaattggtatctatattgttgctgccaataaatcctttgattagcttatttactacatagtattcttctgtaaggcattgcccggatgcgtagaaggctacggcatccggaccatgttttttgatgatggctgcaaatacagcagcagttctttccaatgcctggtcccatgtaaccctttgccgtggaaggttacggtgataccgcatttcaggatacaacaacctgtctgatgtatccatcacggtataatgcaggttcatacctttggaacaaagcatgcccttgttaaccgggtgtgttttatcaccttccacatgcagcttgccctgccggtctttatgtaccactattccacagcctacgccgcagtaacaacaggtggttttgaatgatgcttgcatgctaaaggtttttacaatgatttatgataccgctaccggtgttcttaccggtgcttcctcgctggcaggctgccgggtaaagcgtgtgagcattacaatacaggaaatgccaatcaccacataaccgatatacgtgaacgcctgtacgtagctgatgctgtctgatttaaacaggaagccgaacatcatcccgcccaggtttcccccggcgccaacaataccgcttaccagcccggcatttttttcgttaataaaaggcacaatcccataagtggcgccatttgccattttcaggaacagtgcaaagctcagcatcgctatgatagctactaccagtgatcctgcctgcgcaaataacaataatccgattccttccgccagcagcatcagagccaataaccatcctttccctttcatgccaaatctggcgcctgccttgtctgaaataatgcctcccaatgcccgtgcaaacaggttcataaaaccaaagatgccggcccagaaccctgcgctgccctgcgaaagttgaaatgtatccacaaaatgtaaagaggcaacgttatcaaaagtgatctccatgccaaaacacattccgtatgccattgtcagcgcccagatgcgccagtcggccaacaccgaccaatccgttttattatcttttttattataaccaatctcatcaaaatttccgttaggcgtatcttttgtataacggtaatacagatacgctacaccgagcatcatcactcccggcagtatcatcgcatagcgccacgcttcgggcttggtataaccaaaaccaacaattgcggcaaatatcaccggcatcaccatgttggtaacgcccccgcccaggttgccccagccgccggtaatagcattggcggtgcctttgatggcaggggcgaacataagggaggtgtgaaactgcgtaataacaaaagaaccgcctataacgctgatggctaaacggaacagcataaaggaagtatagtcttttgataaccctaccaggaataccggcaacgaacctatcagcagcagccggatggcggttttgcgtggcccccaggtgtcacagagccggccaatgatcagccgcgctatgatagtgccggatacggaagcaatgatgatattacctacctgcgatttggttaaaccaagatccgtgcggatggtaggcatcagcggcgccaacccgaaccagccaaagaagcaaacgaaaaacatgagccacgtaatatggaacgtgcgcatctgtatggtatcaagactgaatatttttaatttttctaaaggagcagccatgtgttgcgtttttacaggttatttaatcaggaattcgggccggatattcaccgatatgtatacccagttactgtttggagcagcgttctttacatttttaacagtaggagaagacagggtagcagtactccagaagtgactgtaacctgcttccaggcctatcattttggtaagtgtgtaatttgctgttacatctgcttctgttccaaactgtttattcatgcccgttacatcggctgcactgaaaaactcgtgtacgtcgccggtcaatgcccaacgcggtcccggctttagttttgtttttacgtaataatcctgtaatcccttattcccaaatccgctggccacatagaaataatccatattaccccagaacttatgcggggtgccatacagcggatcaaaatcaggactggtataatctgccccggcgccggcgctgaaagttttatttacactataaaagaaagaaccggaaagtaaactgccgctcaccgtttgtccgttcccgttggtaccaaactgatgatacgcggcagctgtataggtaaatttgttaaatgcctgtgtgtaaaacaacccggtggtcatacgggtatttaccgcgccttcatatacttttacggccacatgctctacactgtcgatgtggtattttgaaaactgatccgtcaggaaaagaaaagataagttgcctttgttcagcttcctggatacataagcaaactccaggcttttgtacatgttgccgccattggtatttgcggtataattaccgggaggcgtggcattgtacacactgccgctggcattttctttattctggttaaacgcggcgcccacatgcagggtccacgcattactttcatactttaataccgctgcatcgtgccggcggccctgctgcagccagtcgagattacccagcaaacggctgtcgtcatacaccagttcctggcggccgattttcagagaaaggctcttattcttcaccacagtatctgtcagcaatatttctgcccaggcttcatgcagcataaacccgttattatccggggtggtagtacggttaatggtggatccgtcttgtccccatacgcgtacatcctgtactgtcaatcccagcttgatccggtaagcgctgaatccggccattaaccgggtgcgctgggaagtaaaaaaagctggtgcggcgccttcaggctgcggagcgccttgtccgttacgtagttcggtgcgggtcctgagttgcgcaccgagagagagctgggcatagccgtactgcgataacagcagtccgggaagtatcaacgataccttgcctggaaaccattttttcatgtaactttggttgattttgaatgagccaatcatttccggatcagaaacccggttagcctgccagctaccgggtttcgtttttttattatacacctgccatctccatctcagcttctacgcctatatacaccatgtcgtccacgatctttacagggtaggtagtgagggaacattcgtgttcatcagacaggcaacggccatctttcagggagaatgtttttttatgaaaaggacaggctactttaggctcgtcttgtacagtgccggtcatgccgcggctgagcgccatctgctggcggtgggggcaaaggttctgagtggcataccattcatttctgcgggcaaaaaagaacagtgctatctgctcctccttatactttacgcaaacgccgccattggtaggtacatctgatgttttgcaggcgaggaaccagctggtagtagttgtgtgagtagtagacatagcagtatattttttgtgtaaagagattatttccattctgcggctttcttctgggcgcgcatcgtttcaaattttacagtagggtctttatcagccggtgcatttacgaagtgcgagaaacgtttacgcaactcaggattttccaccacttcgcgccactcgcatttgtagttgtcgaccagcaactgcatttctgattcgagctgggcggcaataccaagactgtcattcaacaccacattgcgtaaataatccatgccgccatccagcttgttgagccaggtagctgtacgggtcagcggatcggcagttttgatgtaaaacatcaggaagcgatcgatgtattggatacaggtttcactgtcgatatctgatgcgagtaattgcgcatgctgcggtttggagccgccattaccgcatacatacaggttccagcctctttctgtggcgatgatgccaaagtctttcgactgtgcctctgcacattcccggatacaaccggaaaccgccgatttaattttatgcggcgcccgcaatccgcggtagcgttcttctatccggatagcgaaactcacactgtcgtgcagtccgaagcggcaccaggtagagcctacacagctttttaccgtgcggagtgctttaccgtaagcatgaccgctttcaaaacccgccgcaatcaattcttcccagatattgggcagatcgctgagatgcgcgccaaacaaatcgatacgctgtcctccggtgattttcgtatagaggttatatttagtaccaatctgaccaatcactaccagcttttccggcgtaatttcgccgccgggaattctcggtaccacggagtaagtaccacctttctggatattggcgaggtagcggtcgttggaatcctgcgcagtgtcgttgcctttgtcaaggatcatgtcgttccacaaactggcgaggatggaggcaactaccggtttacatacttcgcagccttcgccgttgccgtagtgatccagtacttcatcaaaggaacggagtgattttactttgatcagatccagcatttcctggcgggagtactggaagtgttcgcaaaccacgttgcggatatatttgccctgtgccttcatggtggcggtgatcaggtctttcaccatcggcgtacagccaccacagcaggtgccggctttagtacatttctttacttcgtccagcgtttcaaaaccatcggttaccacctggcagatggcgcctttgcttacgctttcacagctgcagataatggcttcatccggaagggccgtaacaccggcgccggtatcagcactgccgcttctgttacccagcaataaatcttccgggttagccggcagggccagtttgtttttggtggtttgcagcagcatgttgtaggcagctgcgtctcctattaatataccacccagcaggaactggccgtcatgggtaatgttgatccttttgtaggtgcctttaaatttatcttcaaatactatactgtgacagctttccggggccgggaacgggtcgccgaagctggctacatccaccccgatgagttttagtttggtactcatatcgaaaccggtgaaggctttggcttcaccggtgatatgagaggcggccacttctgccatttcataacccggggccaccaggccatagatcatgttgttgtaaagtgcgcactcaccgatggaatatataaaggagtcacttgtctgcatctgttcgtttaccacaatccccccgcgcggaccaacggtgatgccggcagcgcgtgccagctcatcccggggtttaatacccgcagacactaccagaatgtctgcttccaggatggtatcatcggaaaactgtaatcctgttatggcctcttcacccagtatttcacgggtgtttttgccggtaagcactttcagtcccagactggccagcttgttctgcaggatagaggagccttgttcatctatctggcgtggcatgaggcgggaggaaaactccaccacatgcgtattgttaataccgaggtccaggagggctttggcggcttccagtcccagcaacccaccgcctattacggcgccgctgctggctcccggggcataagccttcatcatttccaggtcttctatcgtgcggtaaatgaatacgccttttttatccatgccgggtaccggcggtacaaatgcggccgagccggtggccattacgaggtaatcgtaggtttccacgatacctttatatgactgcactgttttattaatacggtcaatctgcaataccgggtcgcccaggtgcaggcggatgccttgctctacgtaccagtcggcggtagcaagtagcaggtcgtcggctgttttgccgtcaaaccaggaggtgagatgtacgcgatcgtaggcgggacggggctcttctccaaatacaaccagttcaatcggggtgtcggcagatttggaaatgatcttctcacaaaatttgtatcccaccataccgtttcctattactactattttcattcgattatatttaaggatcagaaatcttgaattatattataaattaattaatataatagtattttttgctttggagatgatttttaaggtaggcgtatgatgttaattataaaattaagcgtttttgttttaattttaggcatgcatagctgttaaataatcacataattttaaatatcatatgtatgcaggtatcaaatccatttctatctttagtaggagcaggacccggagatcctgaaatgatcacgctaaaagcgattaataccatccgccaggccaacgttatattatatgatgcattggtaaacgaatcgctgctcacttatgcttcgccaggcgcggtaataaagtttgtaggtaaaagatatggctgccatgcgctctcccaacaggaaataaaccacctgatcgtggaaatggcattggcccacggccatgtggtccggctcaaaggtggtgatccgttcatattcggcagggcggtggaggaaattgaaaccgcgaggaagcatgggatcaaagtggctattataccagggatctccagtgcagtagcagtaccggcatctcaaatgataccgctcacctgcaggggcacggcggaaagcttctgggtaaccaccggcactacccaaagcggcgatatttcgaaagacattgccttggcggcacagtccaccgccaccgtagtgattttaatggccatgagcaaactggaagcgatcatggatattttccgggcacacggcaaggcagccacgccggtagccattatccaggatggcaccacgccgcggcaaaaaatggtgacgggcaccgtaaaggatatcacctggcgggcacaggcggccggtatgggaaatcctgctattatagtggtaggagaggtagtaaagctgcaatccctgctggcagatgaaacattacaacaattacaaaacagtaatacgatacatgaagaaagataaacagggctgtgatggtaaaacttgtctcctttgccggttatccctgaaagagtgggccccggcaacagcgttgtaccggaaaaacttttcgttgaacaaaggagaaaccctgtttaaagaaggtgataaagtagaaggtatctactttatttatgaaggccgcatgaaagtgcataaacactggggctctgaaaaagaactcattgtccgctttgcacaaaaaggcgatatcgttggtcaccgcggcataggcggtacggaacaccattatcccatatctgccactgccctggaaccggtaaaagtttgttttatagagatggacttttttcaggcatctcttaaaatcaatcacgacctgctgtatgaactgatgctgttttatgcacaggaactgcaaacgtccgaaaagcagatgcgcaacctcgcacatatgtccgttaaaggccgcatggccaatgcactgatactgttgcaacaaaagtttggctttaacaaagacgggtttattgatcttgcattgagtaagcaagacctagcctcctacatcggggctacttatgaaaccactttccgggtgttgaatgaattaatagaggaacggttggtagcagtttcaggaaaaagtatcaccatcctgaatgaaaacaagttgctcaggctcacagaaaccagtgcctgagggcattcccggatcaagtccacctcatcgtcgtatcaacgccgggcttacttcccctcaatccccattaaacaatatacttccgcagtttcttctcatttaatatcgtaatcgcccttccctccgcggtaatcagtttctctgccataaattcctgcaaattgcggtaaatcgtttcataggtggtgcctgcaaaagcggcgagatcctggcggctgatcgtaaaatgaagcgccttatgcaaccggctgagttccagcaaagcatccgccagcctcccttttacatccatatgcaccaggttgcgcatcttccgttctgcctcctgtaattcatcggcataaaattgcatcagcttcaatgccaggttggggttcactttcagcgatgcctcaaaaaacgacagctccgtataacataccgtggtatcttccagcgcagtggcggaaaccgtatacagccgctcaccgctgcctaacccccggtgcccgaggatatcccccttttgtgcaaagcggacaatgagttctttttcagagccccattgcttgtgcacctttacgttgccgtcatacaaaaaaaagatcccttttaccgggctgccctcctggaaaattgtttcattcttcttataaaaaagatgctgcctgtgatccgataccgccgcaatccattcgggaatgctgtactggcataaaaaacaggtgttcagatcgcaggttccggcttttttcatgactgcaatactagtgtttttttgtgtttttggaagaaaaaataggttttaatatgatttgaatcatatttttgcattgttttaaagatataattgtcattttgtatagtatgaatcataaaaaagagcaaaagtttgccggaaatatgtcaaggagggtattttacctgagcctgcaggcatgtatcaacgccctggttataggcgtagtggcaaaagcactggtgttgctgatcagtcttattaccaacctgtcgttttacggtaaattttcatttgaagaagcagggccggccggaaaccacctgggtatgatcgtaataatagttcctatcataggtagcctgatagtaggcgtgatggcgcgttttggcagtaaagccatccgcggtcatggtatcccggaagccatggagaacatcattggcaatgaaagcaagatcccgccggtgattaccttgctgaaacccatatccgctgctatttctatcggtacgggcggtccctttggagccgaaggccctatcatcgccaccggtggcgccattggctccttcaccggccaggtgattcacatttcttctgcagaaagaaaagtattactggcagccggcgcttgtgccggtatggccgctattttcggcagcccgctggccgctatcctgctggccattgaattattattgttcgaattctccccccgctcagtgattcccgtggccataggctgtatcgccggcgccggtatgcacatcctgttgttcgacagcaacccggtttttgctatgccccccatccccgcggtaaccgatattgccctggtcacctatgtgctaatgggtgccgtaataggtgtagtcgccgcttacgtgtcaaaatctgtttatttcgtggaggacctgttcgagaaattacccatccactggatgtggtggccggcactcggcgccatcgcggtgggcgtgatcggctacttcgccccgcacaccatgggagtgggctacgataacatcaaaacattgctaaccggcaccgcaccgctggcactgctcgtatcactttgtatccttaaatatctttcatgggtgatttccctgggtagcggcacttccggtggaacgctggcgcccctgtttaccattggtggcgcctttggcgccttactgggcgtggccgtaatacaattattccccggcagcggcatcaatatcgccacggcagcgttgatcggtatggccgctatgtttgccggcgcttcccgcgcattgctcaccgccatcgtattttcactggaaacaaccgggcaaacacatggccttctgccgctgatagctgcctgcacagccgcttatttcgtatcgttcttcctcatgaaaggcagcatcatgacggagaagatccgccgcagaggcgttgccaccccggaagagtatacgcccgatatgatgcagctgattaatgtggcggccgttgctacacaacctcctgttatattgcaggagcaaatgacgcaagcgcaggcagaccagttattgcaaaccgtcttttatcactaccgctacttgccggtaacagatagcgccgggcagtttaaaggctatgttaacaggcagcagttgtcggccggaagcaatacgcctgtccgcgggctcctggagtcatctgcaccatacctgtatcccgccgataatatcaatctcgttacagaactcttcgatagctacccgccggatatcctggcggtactcgacaaaggaaagaaattgacaggcatcgttactgccgatggcgtgctgagaacctatggtgaacgccgcaaggccaccgcaaagtatcactctgctttctatggcaatacccgcctgctgcggttaatggcccggggaaaacgattgctggcacgatcttaacctgccggcattaaaggttgaaatacgggtccgctcttttgagcgggcctttttttataccgggtaaaatattcctccgcactgtccgtcttcgtataaaagcttcttaactttaatacatgcagcggaaattaccttccatagaagaaagaatacaacactcgcagaacttccggaacggggcgtttcagaacctctccgttacgccgatgaaacctgacgatgttacctattttaccatgctccgcaaagtactgcgacgcccggcggatgttcgccccccgggagcgatgccttccgtacacaccaacctgaaaacattatactcggagaaaccggtggtcatctggtttggtcattcgtcgtacctcatccatgtaaagggctttaatatattggtagacccggttttcagcggcagcgcatcccccatgtcatttatggtaaaggctttcccgggagcagatgcctatacgcccgctgatatgccggaaatagatcttttgatcgtcactcacaatcactatgatcatcttgataaaaaaacattagcacagctgaaaccacatacaaagcgcatttataccagccttggcgttggtcacgacttacagcgctgtgtggcaacaggcaacaacgtgacggaaatggactggtgggaaacccgtgaaattgctacagacatcaccctaacggctacgcctgcacggcatttctccggccgcggattcaaaagaggtggcagcctgtggtcttcttttgtactggaaatttttgggtataagatttttatcgggggagactcgggatacgacacgcatttcaaagccatcggtgataaattcggtcccttcgatctcgtgatactggaatgcggacaatacaatgattactggcctttcatccatatgaaaccggaagaaaccgtgcaggcggctgtcgacctgcaggcaaaagccctgctgccggtgcactggggcaaatttgtgctggccatgcacgcctggaatgattccccgaaaagagtgaccgccgccggtgcacaaagaggattgctggttactactccccgcataggagagccggtagttgtaggcgcacattatccgcaggaacactggtgggagtaatacctatatccggaaactcaccatttccacaatgccttcaccgggtgcatgaaacagctgattgcccccggtgagtcttttttccgtttcgcacaaaggctccactgtttcaagtatgccatccagctgatacagcaatcctgctatgtctgcacggttattcacattgatgggccggccaatatagctttccagcacctcttttaccgctttgtgatgagacaaaaaatttacaggcacctcttcctcagataaagaataatccagcattacctggttgtgccggaactgcgttttaaatagttgcatcacctgcacaaacgcctggttggggatgtagtgaagcacaccctcaaaaatgatgatggccggaatctcttcgcggtagccattttttaataatttattccatagcagcgccgtatctgttatatcgcatttgatgaaagcgatcagcggattgccaggaataatttcttcgtatagccgttgcttttcttcaatatacccattgtctacttctatgatccggctgatctgctgcgggtagttttccaggagatataaagataaagggtccagtccggcgccgagcataattacctgttgtcctgcaaattcagggatgcgcctgtgcaacatcctgcggatgctctgtttgcgcaggcagatcatatctgtaacaaatggatattgccgtttcagctcatcatataaaccactggtttcactgaaatcgatcgcttccatatattgttgctgcagtggagaggtgtacaattgcatggctgcttccagcaccaggcgggaagtggagggtacttttaattttccggtcattttgaggtgcatttacaataaagctaatatagcgcaatgcataggtacggcagggttattttaatatgaagcgtttataaacgattcataataaggtatctttaataaacaaaatggtagcatcattgtttcattaaaaatgtcaacaactcagcttatgcagccacgtatcgcatcactcagcaaactggaacaggacggaagaaaaatctcccggttgcctttctcgatcaggatcttactggaaaatgtattgcggaaccacgacaacttcgccatcactgatgaacacgtggaaacactggtgaactgggatcctgcgggaacagacaacgaaataccttttaaaccggcccgcgtgctgatgcaggactttacaggcgttgccgctgtggtggatatcgcttccatccgtgcggaagtgatccgcaaagggaaagacggcgctaaaattaacccggccataccggttgacctggtggtagatcactccgtgcaggtagattttttcggaacagactactcctacacaaaaaatgtggcctatgaatatgaacgtaataaagagcgttaccagttgctcaaatgggcgcaacaggccttcgataattttacggtagtgcctccgggcatgggtatttgtcaccaggtaaacctggaatacctcgccaaaggcgttattaaccgtgatggttggctgtttcccgatacattggtgggcacagactctcatactcccatggttaacggtatcggcgtattgggctggggcgtaggtggtattgaagccgaagcagctatcttaggccagcctatctatttctcctgcccccaggtgattgggctgcggctcaccggccggttgacggaaggcgttactgctacggatatggtgcttgccattacacagctgctgcgtaaatatggggtggtcgacaaattcgtggaagtatttggcgacggtctggacttcctctccgtgcctgatcgcgctactatctccaatatgtcgccggagtttggctgcaccgttacctattttccgatagatgcacaaacgttgcaatatatgcatcgcaccaaccgctccaaagaggatattgcgcaggtagaaaactattgcaaagaaaatatgctctggcgtcatggcagcgaagaaatcacctatacggatatcattgaagtggacctcgggcaaatacaatccgctgtggccgggcctaagcgcccgcaggaccgtatcctggtccgtgatctgcacaatgagtttgaaaccctgctcagcaaggaattcaagcgcatgtacacgcctgaaggcaaacggcgtgataccgcctggctggcggaaggcggttccggcaccacctttacctacgaaatacagaagcacgtggaagaagtagcggtggaactcgactatcttaaatccgtacgtattaaactgaaaaatgaagaatatgtgctgagcgacggcgccatcaccatcgccgccatcaccagttgcaccaatacttccaatccaagtgtaatgataggggcagggctggtagcaaagaaagcgatcagtcgcgggttatatgtgaaaccctgggtgaaaacaagcctggcgccgggttcacgggtggtaaccgaatacctgacgcgctcgggtttactggctgaacttgaagcattgcgttttcatattgttggctacggttgtacttcgtgtattggtaacagtggtccgctgccgcctgccattgcggaagcggtggaaaaaggcaacctggtggtggcatcggtactttccggtaaccgtaattttgaagcaagggtacatccgcaggtaaagatgaatttccttgcttcgccgttgctggtagtagcttacgccattgccggccgcatcgatgtagatatactcaccgccccgctgggctatgaccctaacggcgaaccggtatacctccgcgacatctggcctacacaacaggaaatcaatgataccgtagcggccgcagtaaagcaggaagactttgaaaacatctataaggtaatattcgacggcgacgaacaatggcgcggtttactggcgccctcgggcaaagattatcactggagtaacgactccacctacatccgggaagcgccgttctttaaagggctctctgaatttccgtcttccgtggaagatgtaaaagacgcacgcgtgttactgaagctgggagactctgttactacagaccatatctcccctgcaggctcgtttaaacaagacacgccagccggtaaatacctgctggaccggggcattgatccgcgtctctttaattcttatggctcccggaggggaaatcacgaagtgatgatccgcggcacctttgccaatgtgcgtattaaaaatgagttgtcacccaaagaaggtggctttaccactatcattccatccggaatggtgttgcccatttatgatgcggcacagcaatatgcggccacaaaagtgccgctgatcatactggcgggaaaggagtatggcagcggttcttcgcgcgactgggcagcaaagggcaccaatctcctcggcgtaaaagcagtaattgcggaaagctatgaacgtattcaccgcagcaacctggtaggcatgggcatcctcccgttcgagtacctggaaggagaaaatgcagctattttaaatctaaccggaacagaatcatataccatcagcgatatctccaccggtcttgttcccaacaaaatactaacggtaacggctatcccggctgaagggccgcccattattttcaaagtaaaatcaaagctgaactccctgatagaaatcgagtattatcgccacggaggcattttacagtatgtgctgcgggcgtttcttgagaaggcttaaacgcgaattttgtcttggctcaggattacgctgattatactgattagctggatttttacttttggattttataaaggattaagggagatagcagcggatatattcgctgttatctcccttaactattattgaatcaaaaaatcaaaaaaaatccaaaaagtaaaaatccagctaatcagtataatcagcgtaatcctgagccaagacaaaaactcgcgctacctgccccgcgaaaattccaggatcttccggcggttgcctaccagccacactacatcttcccattcaaatgcggtttcggaagcggggttgaggattttctcgccgccgcgggcaatgcctactacgagtgcctgcgttttttcccggatgccggaaccgcggatggtctgacctttgaggccattgtgttcatccactacgatgctggtcaggccgatgttttcgtcagctacatcgtcgcttctttctacgttgagggtgttaaccacacggttaaattcctccagctgcgcttccgtaccaatggcggtaaggatgtcgtgcggaaataatttctcatcgcgggtgggtgcgtagatggtcacattgcctcttttaatggcgcctacgttaatgccgtacttttcccgcagctgcagatctatcagcggtttatccaccagggtagaccagggatcaatttctacttcagatacctgcgcatcccagggcagtaaatctgctgccgtagccttattattggctgcatcggcagtttcacgggcattcagattggtcaggaaacggctttcaatacggttataatatttctgtagttgtgaacgcaacaccagtagcacgcatgccaatataacggcagtacccattaacgcctgccagaacggaaagtactggtttaccaggaaacctaccagcagtacggccaccacattacgcactacttccaccactaccagcggaccgtgattgtatttggaatccagccataacgccttataggaattgctcgaaattttctgcaccatcaaggcccagataaatggcgacatcatggcaataccgatgatcacactcagtaattccgccaggaacaggttcttcacatatttaatcacaaacggaccgatataataggtgttgagtaagatcacggcgaacatgatcactgcattcagtacaatcacttttacataactgcgcaatacaatacgccagtcgctttccgcctgtaaggtttgtgaactggcactgtaccggttaagggtagttagccagcgaccagggatgatcttctccaaccagttataaaatggcacggaaaacttgatcatgtaaggtgtagtgaaggtggtaatggccgaaacgcccactgctaccgggaaaaggaactcgctggttactccgagggaaagccccagtgttgcaataataaaggcaaattcacctacctgcgccatactcatacccacctggacagcctgtttcagcggctgaccggataacaacgctcccattgtggtggtgaaaaatttcccggtgatggttaacaacgttatccacagtaccggccaccggtattctacaatcatctccgggttgataagcatacctaccgatacgaaaaagatagcgccaaaaagatcttttaccggttgtatgaggtgctccactttttcagaggaggtggtttccgctatgatggaacccatgataaaggcgcccagctccgcggagaagcccactttggtggccaggatcaccatgcccaaacagagcgctatactcagtatcagcagggtttctccattgaggtagcgttctattttcttcagtgcggtgggtaaaagaaaaatccctgccaggaaccaaaccgccaggaagaacatcagcttggcaatggtaaacagcatctccgttccttcaaatttccggctcaccgccatcgtagataataataccatcatgaggatcaccacaatgtcctctatcaccaacacgccgaaaactattttggtaaatgactttttcttgatacctaattcttcaaaggcacggataatgatagtggtagaggaactggccagcaaacctccgaggaacaggctgtccataaaaccccagcccatcagtttaccggtaaaataaccggcaacagtgatcagcgctatttctacaaatgcggtaatggtggcggtaccccccacccgcattagctttttaaaactaaattccagtcccagtgaaaataaaaggaagataacaccgatttcagaccaggtttttatcccttctgcatccccgatagtaggaaacagtttgaaattgggccccactataaatccagcgatgatataccccagcaccatcggctgtttcagccgtttaaatagtaatgtaataactcccgccgctcctaatattaatgccaggtcaatgatcaatgatggtagatgcatacagtaataatcgatttaatgtttcgtgtgatgtacttttatggcgctgagaaatcagcgcacatatgtgtcagatgccagtttccggacctttgaatattgctaatatattatttttccggcggggaagcaagattaagtttggctaccgctccttctctgcctgtatctgcgctacatatctcgacggtagtatcccgaactgtttctgaaaattctttccaaaattagtcagggaagcaaagccgcaaagctccgccacttcattcactttgtatgatccggtggataataaagacgctgcttttttcaaacgtgcgatattgatcagctcatgaggcgtaagatcggatatcgcttttattttacgatagaaagtagggcggctcatgttcataaaatctgccagctgttccacatcgagatcaatgttattgagatgctggttgatcaggtcattcagcttttccaggaattgttcatcggcgctggtataggccatgctgcgcagatgcaccagcggagtactggcataataggattttattttatgacggttgctgagcaggctcgcaatttgcgcctgcaggaattcaggtgagaatggtttttcaatataagcatcggcgccgagttcaagcccttctattttcgattgcattgtattgcgtgccgtaagcaggatcaccggaatatgactggatacaaaatccgacttaataatacggcatagctcaaagccatccattaccggcatcatcacatcactgatcaccagctgcacgggctgctcctgcaataatagcaaggcggcctgcccgtcgcgcgcagtgattactttatatttatcttccaggtcgtctgcaatgaaagaaagtatttcttcattatcatctaccaacagtatcagcggcttgttttccatttgctcaggttaaattctatttcctggtgaacaggcaaagtaagtgaaaaaacatttagtgtcccatcggtcggcagcaactcgaggctacctttgtgcagcagcgttaatgatcttgaaagggatagcccgatacctgtaccggatttatcggccgtggccttcgcacggaagaatggctcaaatattttgtccttcatttcagcaggaataatgtatccgtcgttcttcaccaggatagtaaaagtggcatcgttttcatccaccggctgcaggtgtatggatgctttggtagcggcataccggatagcattgttgatcagattgcccagtatcttatgtagagcttccgcatctacataagcaaaaaaatgaaggcttgataactctattttaaaccggatatcctgctgctccgctgctggcgtaaatcgcagatggttttctttcagcagctcagaaatatcagtacgcacaaaattcaggctgaaaccattgatctctgttttgcggaagtcgagcaactggttggttaactccagcagccggtcggtattgcgttccatgatgcgcaggtttttctggatcagtggtacctcatcggatttgcggatcaccttttccatcggccccttgatcagcgtaagtggtgtccggatctcatgcgcgagatgtgtaaagaattcaattttcgcctggtataactctttttctttttcatgctccagcaattcaagctgccgtttctgcttttgctgcgcacgctgatgataccaccggataataaaataagccaggctgcatagcaggacgatgtaggcggcatatgcccaatagctggcccagaagggtgggaggataacaatagtaagcacacgcggcgtaatgctccagctgccgccactgctggccgacttcaccataaaccggtaagtaccgggcggtaatttggtaaagaacgccttccggttagtttccaggtaagtccagtcacggtcaagcccttccattttatatgtgtaagccgtcatctccggggaagtgtagctcagcgccgcaaagttgatgctaaaagaggattggtcgtgcgataaaacaatcgtatccgtcaggaaaatagattgtttcaggatgtcgcccacctgggcttctttattatacacctggaagccggtaatatatacgggtggcagataactgttacgcacaaacgactcggggttgaaacggatcaatccttttacactgccaaaatacatattgccacaactgtctttataagcggaattataattaaactgatcatttaataaaccactggctttagtatataccactgcattttcagtggcgggtgtaaaacacgccagccctttggaagtagttacccacaggcggtcgctcttgtcttccaggatagaaaatatcatattactaaggaaaccatgccgggtgttgtaagtcgtaaaattattacgctgccggttgtacaaacaaagaccatcatctgtggccagccataaacgatggtggctgtcttcaaaaattctgttcacgcggttgttgctcaaactggtgctgtcatgtgcatcatgcaggtaaagccctttcttccccgtgcggcggttatagaaatataatccgtccctcaccgtgcctaaccagatagtgccttccctgtcttcgaaaacagccgtataaaaaatataatgaggtacttcttttacggtattaaattcatcacgggaacggctatactcatataatccccaggtagtacatatcagtatattatcgttgctggtacgcagcaagctatagataaaaccactgtgcagctgatgtggcccgtcacccggtgcatagtgccggataaattttccgctggggatatccatgacatccaggccatgctcgaaagtgcctatccagagggaatccccggtaaccagtaaaccatgaagattggtatgcgataaacccggtgcatgtttatccaaaggccggatggccgaaaaactgccatccgatgggatgaacttattcagccccccatcttcggtacctatccacaaatgaccatatttatcgggatgaatctctctcactgcgttaccactgagagaagaagaacctgttttcggaaatagcttttcgaaatacgtataaggttgtggaaaataattggtgccgccaaagtaagtgcctacccatatgccgccttctttatctttacaaatattataaatggcattatcagaaacagagtaaggatcatcataattttttttcaggttgatgatcttaccgcttttaatattatagatatagataccggattccgatgcaatccagtattcatcatcgttccggcggataatgtccctcacatacaattcaataccggctgtatccctggaaaggaaatcttcgtaggcacgtgtccgtgtattaaacagttttaagccctgccctgcggtacatgcccagatggtatccctgcccattggtacaattttctggatagcataggaattgggtttggcagaatgtgtgaagagggaataagtggtaaaattgtttttgtcgtaatgatagaccgccatattgcccgccgaagagcacaaccagaggcgtccttcgccatccaggcaaacagaggaggcgtcccggaagccggggacttctgtcagacggtcggttgctgcctggtagcgaaacaggcggcctgcggatataatccagatatttccctgcctgtcttttgtgatggaccgtacttctccctccgtttttctactcagctcgcggaactgttcattacgcggattatatataaatacccctttgtccgatcctacatataacaggccgtcatcgtcctggaacaggcagaggatgtagttgccaccaatacttcccggctgctctgttcgcctgaatacccggaaggtgtaaccatcgaaccggttcaagccgtacatcgttccaaaccacataaacccctgtttgtcctgcagcgtgcagataacggcgttgtgcgacaaaccgttctctacctggtaatgtacaaaaccgggcgactggctatatagcgccccgcttagcagcagcaacatgaacaggatataatagcggatttttggcatgtgttcgtttagtggaaagcttaaaactaatggtttttccgctaaaacccaccaccatccggctaaaagctaaaatgatacaaaagagataaaaattgagataaatgggcaaacaagtattcagcggatagtctttctttggagaagtgtgttaagcgtgaaatatacacttaaataagccatcttctaaatccatgttatgaaaagtagccaactactttcactggtatttttactgtttatcagcgggatatgccgtgccacttctgaggataccactggtatgttcaaaaatcctttgctgagctccggccccgatccctgggtggtaagccacaacggtatgtattattatatgcataccacaggtcataacctggtgatgcggaaaacaaaaggcatgtcggcgttggcgcaatccactcaaaaagttatatggacaccaccagccaaaggacccaatgcgagggatatctgggcgcccgaactgcaccgtttaaatgggaaatggtatgtgtattataccgccggatcgtctgatagcattcatccgcaacacacatttgtgctggaaaatacggccgccgatccaaccaccggcagctggactgataagggacagatcaccgatcccgcccatccggagcacttcgccattgatggcaccctcttacaatataacggcaataactattttatctggagcgggcataacggaaaagatgcggtacaacgcctgtatatcgcccgcatgaaagatccctggacactggcctcttcaaaagtagaaatagctgcgcctcaatatccatgggaacaaaacgggataaatgaaggccccgaaatcctccggaatgccaaaggagaaatcttcctggtcttctccgcatgcgggtgttggacagaaaattatatactcggtatcatgaaattaaagcctggcgcagatccgctgctgccggccagttggactaaatcgcctgatcccgtattgcaaagcaagccggagaacggcgcttatgcaccaggacataacggtttctttaaatcgccggacggaaaagaagactggatcatttatcacgccaactcaaaagccggacagggatgtggcaatcaacgtaatccccgcatacaaaagatcacctggaatacagacggcacgcctttttttggcgaaccggtgaaaataaatacatgggtcactaagccttcaggagagtaaaatcactttaagaaaatatatgaaaaagaagtacctattttttgcactggcacttggattgggcagcagtacagcaatagcacaacaacaggattggaaaatagtgggaggtaagatcgctacttcctggagcgaacaggtatcgccggcagctacgttgccggaatatccgcgcccgcagctggttcgcggcaactggaaaaatctgaacggattgtggaattatgccatcaaagcaaaagaggaaagtcaacctaccatctgggacggcaaaatactggtaccctttgctgttgaatcagcactttccggcgtaggccgtactgtggggaaagacagcatactgtggtataacaccacgctcacgctgccttccggtatgcagggtaaaaagatattgctgcactttggtgcatccgactggcgtactaccgtatacgttaatggcaaagaagccggcagccatgaaggcggctttgatccatttaccttcgatatcacgtcattagtaaaaaagggtaaacaggaaattgcagtaaaagtatgggaccccaccgacgatggcgatcagccaagaggcaagcaggtgaagcgtccggaaggaatctggtataccccggtaaccggtatctggcaaacagtatgggtggaagccgtagcagatacttacatcacttctaccaaacaaacacccgatatcgaccaggaaacacttacggtagcagctaatgtggaaaacttaaaagcaggtgatgtagtaaaagtaaccgcattcgatggtggtaccaaagtagcagaaagcgccatcaacggagaaaatgctgtattgaaaatagcttcgccaaagttatggtcgccggaatcccctttcctctacaacctcaccctcacggttacacgaaaaggcaaggtagtagacgaagtgaaaagctatttcgccatgcgtaaatcttccattggaaaagatgccaatggcgtagaacgcatgctgctgaacaataaattcgtattccagtatggcccgctggatcagggctggtggcccgacggattatataccgcccccacagatgaagccctgaagtttgatatcgcacaaaccaaagcaatgggctttaatatgatcaggaaacatattaaagttgaacctgcacgctggtactattactgtgatcagctgggtgtgctggtatggcaggacatgccgagcggcgatctcggaaacggctgggagccacgtcccggtattatcgggcgtggcaccgatcagcatcgctcagctgaatcagaaagctactaccggaaagagtggaacaccatcattgatgaattatataactatccctctattgtagtatggacgccattcaacgaagcatggggacaattcaaaacagtggagattgcagaatggaccatgaagaaagatccgtcccgcctcgtgaatactgccagcggcggtaacttttacccggtaggacatatcatcgacctgcataactaccccgagccagcaatgccggatccggccatatatggcgataaacgcgccatcgtgctgggtgaattcggcggactgggattgccggtgaacggacatgtatggcagcaaaaagataactggggataccagagctttaaaaacgaggaagatctttttaaacgctacagcgggttcaccgacagattggaagcactgatcaaacaaggactatcagccgccgtatacacacaaaccaccgatgtggaagtggagacaaacggcctgatgacctacgaccggaaagtgcagaagatgccactggacaaactgaaactgattcatcagaaattgtataacccggccttggtaactataaaaccataatgatggaaaagcgaaagttgtttggcttattgatgctttctgctttttttgttggtcttatcccggcggatgcagcgcatccgccgggtgccagggctgacaccaatacctttgtggcccccgtttaccaggcccttccactcggcgcagtaaagccacagggctggctgctgcaccagttgcaaatcatgcgcaacggaaccagcggccatctcgatgaagtatatggtaaagtgaagaacgacaacggctggctgggcggaaaaggcgacggctgggaggaaacaccctactggctggatggcgcagtacccctggcctggctgctcaacgacaaagaactgaaaagtaaagtactccgctatatcaactggaccctcgatcaccagcggccttccggttattttggtccgctcaccaaaaccgagcgggaaaagaatatagccattggcgttagtaatgccgccgacggcgacgactggtggccaaagatggtgatgttgaaagtactgcaacaatattatacggccacaaatgatccccgtgttttaccttttatgacgcggtattttcactaccagttgcaggtattgaaatcctgcccgctgggcaaatggacagaatgggccacctcccgtggcgctgaaaacgtaatggtagcccaatggctgtacagtatcaataaagacaaacaactgctggaactggcagcactgctgcaatcacaggcatttacctggagcagctggctcggcaaccgcagttgggtaatagatgcggctgcacagcaaaacgaccagcactggatgcgccgtcacggtgtaaacgtaggcatgggactgaaagatcccgtgatgaactaccagcgcaccggcgacaaaaaatacctgcaggacctgcacaccggctttaccgacctgatgaacctccacggcttgccgatgggcatcttttccgccgatgaagaccttcacggtaacgcacctacgcagggaactgaactgtgcgccattgtggaagccatgttttccctggaggaaattatcggtatcaccggcgatcctttatatatggaagcattggaacgcatgacctttaacgcactgcctacacaaacaaccgacgattataacaacaaacaatatttccaggtagccaaccaggtgaatatcaaaagaggcgtattcaatttttccctgccgttcgaccgggaaatgaataatgtactgggtatgcgcagcggttatacctgttgcctggccaatatgcaccagggctggacgaagttcgcctcacacctgtggtatggcgctgccggtaacggcctcgcggcgcttacttacagtcccaatgaagtaacggctcaagtaggaaagaatcatacccctgttaccattcacgaagaaaccggctacccgtttgaagatcagatccgtttccggatgaacatgcgggagccagttgcctttcccctccaactgcgtatccccgcctggtgcgatgaagcaacaatactactcaacggccggaaattacgttccgaaaaaggcggccagatcattaccctgaaccggagctggaacaacgatgatcagctggtactgcaactgcccatgcagatacgcacttccaactggggccgtaattcacgcaccgtggaaagaggaccactcgtatatgcgttaaagttagaagagcagtgggagaaaggacatgatgaagtggaaggcgattatttcagtgtttaccccaaaggtgaatggaactacggcctgcctgaaaagatcatccgcgagccggcaaagtacctgaaggtgagcaccgtgaaaccggtaacagacacattcgtatggaacctggcacatgcgccggtaacgatcaccaccaccggtaaacaactccctgagtggaaactggtggatgatgtggcgccccaacccgtaacagaccggaacggtatttataaaggtaaagtaaacgacaaagaaaccagtattacactggtgccctatggttgcaccaaagtgagaattgtagcattcccggtagtgaaataaacaatagcgtagcatatttcaaccaaaaagacagcatgtaagactgataatttaataagaccacacaaacatttgttatgaaaaaacgattacgtttccgcaatttaatccggaaggtgataccgggcggctattgccggctattcacggtattgttgctttccttgggcctgatggcccatgctgcgcctgcagacatggtgattaccggtaaggtaacagacgataaaggaataccactggtaggagtaacagtgaatataaaaggcaccaataaaggaaccgccacagatggcggcggaaattactcgctctctgttccggaaaacaacgccgtactggtattttcctatgtaggatttctgaaacaggaagtaccattatcgggcaaaaaagtagtaaacgtacaactggaaacggatagcaaaggattgggagaagtggtagtggtagggtatggtacacaaaaaaaggaatccctgacaggcgctatctccggcgtaaccagcaaagacctggaaagggtacacgcttctaccgtgagcgccacgctggcgggtaaaataccgggcgtgtctttccgtatgcccgacggcagacccggcgcaggcgccaacatccagatccgtaatttcggaaatgccctgtatgtaattgacggtattcagaaagatgccggccagttcaacaacatttcccccaacgacattgaaagcatcaccgtactcaaagatgcttccgccgctatttatggcgtaagggccgcaaatggggtagtagtggtaaccaccaaaagaggtaaaatgggagcgggaaataccattaacgtagatgcctatacgggatggcagaactggtcgagattccccaaaacggtaaatgcctatgagtggatgctcggtaaagccgatgccgaaatgaatgacgaaaacccgcatacagatatcacaagggaggaactggagaagtggaaagcgggaacagaaaagggatacaggagtttcgactggtacgattttattatcaagaaaaatgccccgcagaattctattaatgtgaatgctacgggcggttctgaaaatatcaactactatctttccctcacacgcctggatcaaaaatcggtgctgggaagagaatttgattttaaccgtaccaatatccagagtaacgtggatgccaaagtggcgaagcgtgtaaaagtaggcgtacagatcaacggtcgtattgagcaacgcgataaccccggcgttcccggcggcgacgactattgggcgccccgcttcgcactgttccgcaacaggcctacagaaagggcatacgccaatgataacccgttgtacccgaatgatatcggccacaacacggagaactgggcggtacagtcaaaagccatctccggctattggacggaagactggcgcgtgctgcaaaccaacttcaacgctacttacgaaacacctatcaaagggctcacactgaaaggaatgtattcctactatttcgctgacaagctgatgaacggtcacgaatatacgtacgatacctacacctaccaggaggctacggatacttacctgcgtaccggcggaagctccaatccctggagggaacgcggcacgcataaagtgctggaaaacgtattgcagggccagatcaactataacaacacttttggtaaacataccatcggcgctacattggtgtctgagcgcatcaaacgccgggagctggatgtgtgggtgcatgcagtgcctaaaagcaacctgctgccactgatccagttttccgatatggatacttacaatgacaacgactggacagaagcccgtgtgggttatataggtcgtttaaactatagtttcagtgacaaatatttcctggaagtagccggccgttacgatggctcctggaagtttacaccagataaaagatggggcttctttccgtctatctccggaggatggaggttaacagaggaaccttttgttaaaaacctgctgggaggaaattctattctcacagaattgaaattaagggcttcctatggagaactgggtgacgatgatattggtatcggcgcctacgactacctgcccggctatacgtacggcacgtctactgtaatcctggatggcaccattatcaggggctcccgcgataaaggtgttccaaacgaccgtctctcctggtttaccagtaaaattgctgacgtagggctggattaccagttgtggaatggaaaaatatccggctcgctcgatttcttcaaccgtaaacgttccgggttacgtggccgcaagtacgatgtactggtgccaagtgaaattggctacaacctgccggatgaaaatgtgaacagcgattcacagcggggcggcgaattctctgctgcctataacggccaggcaggtaaagtgagctttatgattggcggtaacgtatcttattccagaagcaggctgctcgaaacctataagccgatatggggcaactcctgggatcattaccggaattccattgaagaccgctggaatgggatctactggggatatgaagccatcggccaattccagtcgcaggatgaaatcaataaataccctgtgaatgtggacggacaaggcaacaaaactttgttaccgggagatatcatctataaagacatgaacggtgacaacgtgatcaataacctggatgaaagacctattggctatcaaacaacaggtaaccctaccgttaactttggtttaaacttcggcgtaagatggaatggttttgattttgcagccgacttctccggtggttccatgtattcctacaatcagaactgggaaatgagatggccctatcagaatggcggcaacctgcttaaacagttctacgacgatcgctggcaccgtgaagatccttttgacctgaacagcaaatggattcccggtaaaaacccaccactgcgattcaacaagggcggtcatagtaactataacaaggcatctactttctggttgcataatgtacgttacctgcgcttgagaacaatggaaattggctattctattcctcagcaaatactggacagaattaggtttaagaaggtaagggtatacgtaaatacctacaacctattctcgttcgataacgtaaaagaccttggaatagaaccggaaatagcagacgagaacgggttgcaatatccgcagaataagctggtaaacattggtttgaactttactttctaagtaattaataagattcgttatgaaaaaaagtttgttatatataggtctttgtgtactcgctttgaatacgggttgcaacagggacaaagacttcctggacgtgccaccgtccaacatcctgcagaatgagcagttatggaatgatgaagggctcatcctttccgtactcgccgatctgtacgaccgttacccggacaggcaaacagatgttgagaattcgccgataccttcaatggtggtacaaaccatagataactggggcgagtttgcccgctttgatgaggccttcgcatctgaaagcggccagtactggcggcatagcgccagcgactatccttatgtatttcccggtatgattgtaaaaggtggacgcgaagtgacctattgggattatgcgtatatcagggagttgaatatattcatcgaaaagtgtggagcctccacaaaactgaaacaggaggtaaaagacaggtttgttgccgaagcccgttacctgagagcggtggtatattttgaagaagtaaaaagggtgggcggtgtgccgttgatattgcaggcaatggagtatgactacaaaaacgatcctgcttatctgcaacatccgcgtgcgaaagaatcagagatctatgattttgtgatcagcgaaatggatacggtaaagaaatatgtgcctgcaagccccgtgagtaaaacccgtgtaactgtagggctggcgctggctaccaaagtcagggcggcattgtatgccggttctattgcaaaacacggcgcagaaacaccgcaggtgtcattgcccggtggagaagtaggtatccccgtttcaaaagcaaatgcttattatactactgccctgcaggcagcacaggaactgattgccaccggcagttattctttgtacaaaaagaattcggataacatcacgcagaattttgtcagtctgtttatcgacaaaggttccaatccggaagtgatttttgcaaaggattacaaattgcagagcggacgtgtgcaaccctggaccttgtggagccagccacgttccaatgcagaagagcagcagggcggccgtttaaacccgtcgctgaatctcgtacagtcgttcgagttactggataatacttttgccccgcttcccatcaatgcggcaggtggcggttatatgtactatagtgatccgatggatttgtttgccaacagagaccctcgtttagccgctactgttatgttacccggatctgaatttaaggacaagaaagtagatatatgggccggttatattaagaaggatggcagcattgttacgggtgacaacttcggggcaaaagccaagctggagccgaatggaccggatgtgcaggtagttggatttgacgggccggtaaataacctggagttcagcgcccaatccggttttattatccgcaagtatatggatcccaccgttggatcgggccgtataggcactcaaagcgaagtatggtggatccgttaccgttatgcagaagtgttgctcaatgctgcggaagcagcgtttgaactggggcaggcaggtgtggcagccggttatatcaacgaagtacgtgaaagggctgggttcaaaaccccgctgacggctgggcaaatcaccttcgaccggattgtgcatgaaaggaaagtggaactggcatttgaaggtcacgaattctgggatatgaaacgctggcgcctggcacataaggtatggaatggtgtgaaaacaccattgactactacacctggcactgcaactgcggtaagtaaccgggtatttgccctgtggccttacaaggtatacgatccgggaggcgccaataatggtaagtatatatttaagcaggtattgccgggagcggttacttccgcgcatctgttccggatgggaaattattatgggtatatcgatgacgatatccggaataataatcctaaaatagtaaagaatcctaaccagtaaagcgaattattatgagaactaaaattcagtatatcatactcattgcattaggtatattttctgcctcctgtaagaaagataactacaaggcaccctccagtacttttaatggaagactggtataccagggagagccggtaaatgttagttacaacgatgtatattttgaactctgggaacctggttggggaaaaagcatacccatcaacgttaatgtaagccaggatggttcattttccgcattgttgttcaatgcggcctataagctggtgattcccgcttcacagggccctttcaggtccattccggacaaaacaaccaatacagacaccataccgttgacgatctccggcagcctgcaacaggatatcgaggtaatgccgtattacatgatccgttctccgaaatttacagcagtggcgaaaaagctcacggctacctttagtgcggaaaagatcattaaggatgttaatgcgcgggatattgagcgggtattcctgtatgtgtgtaaaacgcagtttgtggatggtcgcaatagcattcaaacagccgatatggccggtggcgatatcgttaatcctgcgaatatcagtctgcagctggatataccggacgtggtgccggcacagccttccgtatttgcacggattggtttaaagatagcaggcgtagaagatatgcttttctcccccgtacaggagattgcactgtagagaatgatgaacaaacattcacatgaagctgtctcataaataaatgaggcagctttttcattttaggctttaaggatggttttatccacaatttgcagttgaaaaaaagggaagttgtaagtgtttacgcaccagaagttattgtgtaaat

SEQ ID NO: 19 - DNA, 56322 bp, Chitinophaga pinensis
  source 1..56322: mol_type = genomic DNA
ggctaatttttgctcaaaactgtattttctgcgtttatccataaaaatgccccctaaaagtgtctaacttttagggggcagtacatatatccgcttctatctcccttaatcctttataaaatcaaaaagtaaaaatccagctaatcagtataatcagcgtaatcctgctccaagacaatttaaaatcgccgaaggcgatgctacgcctgtttcttgcgctggatggctttttctgctgctgcaacgatgtgatctgaatcgaggccatattttttcagcaggtccagtggtttaccgctttcgccgaaggtatcgttggtgcccacgtattcgatgggaacgggtgtatggcgggcggctacctgtgcgatgctgtcgccaaggccaccgagtacattgtgttcttcggcagtaacggcgcaaccggtttttttcagggaagcgattactgctgcttcgtccagtggtttaatggtgtggatgttgatgatttccacgctgtagcctttttcttccagaactttaccggcttcgatggcaatccaaaccaggtgaccgcaggcgaataaggtgatatctgttccttcgtggaggatctgtgctttacccacttcaaatttctggtcttccgcggtaaaattgggccatttcgggcgaccgaaacggaggtataccggtccttcgtagtcggcgatggcgatggtagcggctttggtttgattgaaatcgcaaggtacgatgacagtcattccgggcagcattttcatcatgccgatatcttccaggatctggtgggtggcgccatcttcacccagggtaagtcctgcgtgggaagcacatatttttacgttcttgttggaataggcaacagactgacggatctggtcgtatacccttccggtagagaagttagcgaaagtagtggtgtatggtattttaccgccgatggttaagcctgcagcgatgccaatcatgttggcttctgcgatacctacctgtacaaagcgatcggggaattctttaataaaagcgttcagtttcatagaaccgagcaaatctgctgtcagtgcaactacattggggtttttacgacctacttcgagtatgccctcaccaaacccgccacgggtttctttttcatttagtggttgaatatcttttaccattgtggtctttttaaaaatgaagcgtaaatgtaaacattaaaaaatgaggatcctagttactcagtactttattacgcaggctcacttcccattgccaggcggtgcgcatactgtcttcgataccaatttttggctcccagttcagcttttccttcgccttactgttattggcgtaaatagagatcacatctccttccctgcgtgggccggtggtgtagtttaatttgatgccggaaattttttcaaatgctttgatagcttccagcacggttacgccgttgccggtaccgaggttaaacacttcacagttgctggtattgtggtgttctataaggtattggagcgctttcgtgtgagcggcggcgatatccattacgtggatatagtcgcgtacgcaggagccgtcgcgggtatcgtaatcggtgccgaataccgtcatttttggaattttaccgatggcggtttgggtgattacgggaaccaggttgtctggttttcccagcggcagttcgccgataagtgcagatgggtgtgcgcctaccgggttaaaatagcggagcaggatggagttggtttcatttacccggctatagtcttcgatgatttgttcacccatttgtttggtacgggcgtatggagactgggcttcgccgagcggtgtttcttccactaccgggagggctttggtattgccgtaaaccgagcaggaagaggagaatacgaggttgggtacattgtattctttcacgcatttcaacacattgaccagcgaggtgatattgttctgaaagtacatcaggggctcgtttacagattctcccactgctttcagggcagcaaaatggatgacgccaacgatatcccggttttcatgaaataccgcattggtgtcttccaggttacaaagatctactttgtagttgcgtaccttttttccggtaattttttcgataccatctaataattgggtgctgctcctgatattactgtctacagatactacatcaaatccattattgatcagatctacaatagtatgcgcgcctatatagccacaaccacccgtaacaagaaccttcatgatatttcagatttacgtttatttgatatttcagaaaactttttgattgagcaccgtttcgaggtaagctccgtagccgcttttcagtaaaggttttgccagatcctttagttggccggcgtcaataaatcctttacggtaggcgatttcttcgatacaggctactttaattccttgtctttgttctattacctgtacaaattgggatgcctgcatcagcgagtcaaatgtgccggtatccagccatgctgttccgcgtggtaagatagaaacttttaattttccccgctgcaaatattctttatttacatctgtaatttcatattcgccgcgtggactgggttgcagatttttagcgatttccactacttcattatcgtagaagtagagtccgggtacagcgaagtgggatttcggttgtgtgggtttttcctcgatggacagtactttcatgtcctgaccaaattccacaactccatacctttccgggtcggatacctggtaggcatatacgatgccgccgtcggggttagtgttatgagccagttgtgtaccgagtcctgccccgtaaaagatattatcacccaataccagtgctactgtgtcctggccgataaattcctcgccgattacaaaagcctgggccagcccattggggttgggttgttccgtataagtcaaattcagtcccagttgttgaccattaccgaagagccgttgaaaagccggcagatcgtgtggggtggaaatgatcaggatatccttgatgcccgccagcatcagggtagacagcgggtaatagatcattggtttatcgtagaccggcatgatctgtttgctgatagcatacgtaatggggtgcagccgggtgccggagccgccggccaggattattcctttcatttgcaagatcaatttttgatggtcactaacttaactcttccgatcagaagaaaaccgcacaaaaatagcggctctctttcaattggcgtcttttttttataaaaaaagctctccggaggttacggagagcttttaaaagtatctgttggttcacttttttaaatgaacaggtttacgatgaaataggtgactgcggccagtaatccactgatgggaatggttaaaacccaggcccacagcagtgatacggtaaccccccaacgaacggcagataaccttttggtagcccctacgcccatgatagcacccgtaataacgtgggtggtactggcgggaatacccaggtgttccgtgaggaagagggtaatggcgccggaggtttcagcagccacgccttccagcggggttactttagtgatacgggttcccattgttttcacaattttccagccaccgctcatggtgccgagtgcgatacaggtaaagcacgccagcggtacccagtccggcatttccttgaggctgccgatatagccggcagataccattgcagcagagatgatccccattactttctgggcatcgttactaccgtgaccaaggcttaatgccgcggaggaggccagctgcaggcgtttgaaccagctttctgcccggtatggatttgccttacggcagatatttacaatgatgagtgttattataaaggccaccaccatacctatgagaggcgccagtacaatgaaatacactgtgggcaaaactttgtggaaattgattacgtcaatattgccaccggaggcggttacagctgcaccaatgaaaccacctatcagggtatgcgaggagctggagggaattcccagccaccaggtgaagaggttccaggtaatagctgccaccaggccgcaaaggattactttcagcgtgataaactgctcaaataccgagttggctacggaattggctactttaaactcaccgatgtagtatttggcaacaaaaaaggccacaaagttgaatactgcggcccagagtactgcctggaaaggcgtaagcactttggtcgacacaatagtggcgatagagttggcggcatcatggaaaccattgatatagtcgaaaatgaatgccagtatgataataattactagtaaagtcatgacatcaggagaattatgcgttcagaactgtattcccctttatcaggagtacttgataataatggtttctattacgttggcgcagtcctcgcacttatcggtagcgatttccagggcctggtagatttcacgcattttaatcagttctgcggcgttctgctctgtatcaaaaaggtcggcgatagccatatcgtagatatcatcagcatggttttccaggctgttgatctttacgcaggcatcggtaatgatgcgcatattctgcatattgcgcagttcggggattgctttggcaagttccagtacacccaggtggatcagttccgccagtttgcggatgctgtcgttgatgtaatgtactttatagagatccattcttttggcagaaccatggatgtaatctgccacatcgtccagtgttgccgccaggtagtgaatgtcttcacggtcaaacggagtgataaagttttgtccgagctctacaaatatgcggtgtgtgtaatcgtcgtttttgtgttccaggcgttctatcaggtgtaccttatcctttctcacagccagatctgtggtggctaccagctcattgagcacagtcgccatttctaccagattggaagctacgtcttcaaacaaagaataaaatacccggtctttcggcatgaatagtttaacaaaagaattgaagcctcccatacgtttgagtttataaaatttgccgcaaaaatagctttcagaatctatcccagccagtaaaaaacgtgaattaataattccttaacactggattaatataaaagtaatatagcgatttttcctttgcatagaaaattatactcataaacaggctgcctacaacctgtacatacaaacctataatgtcggataaacgcccattagatatagccgtaatttcagatgttcatctgggaatttacggctgccacgccaaagagctgattcagtacctggatagtatcgacccgcggatattggtgctgaatggggatattatcgatatctggcaattcagcaaacgctattttccaaaggcgcataccaaagtgatccgcaaaatcctgaagatgatcggcaaaggcaccgaggtgtattacctgacaggtaaccacgacgaggccctccgtaaatacgcagggtttgagctgggtaactttacgatcgataataagctggtgctggacgtagatggcaaaagacactggttctttcatggagatgtgtacgatgtaaccatgaaaaactccaagtggctggccaagctgggcggaaaagggtatgatctgctgattatcctcaaccggctggtcaatcatgtgctggaaagcatggggagggaaaagatgtctttctccaaaaaagtaaaacagggggtgaagtcggccgtaaaattcatttccgattttgaacaaaccgttgccgaaatagccgccgataaagagtttgatgtagtgtgctgtggtcatatccaccagcccctgatcaaagaaatgcaggtgggcgataaaacaatcacctatctgaattcgggcgattgggtggaaagtcttacttcccttgaatataccaaccagcaatgggccctgtaccaacaccccgttacccggaagggcaccgtacttgcagaggacgacgatgatggactcaccgactgggatgctacccgtattattaccttccccggctcctgattttttctttcttattattacatttaaatattttaaatatatttatatttaaatactattttcacaaaatcataacaagcgcttaatattaaattaaaagtagactactaagtttgccagagaaataattaagtgtgacgatagtggcacatttagataagcaagaaaaacagctagatgaaagtattgaagttacatcctttaatgacgatctccctattgcaaatgcagatccagcgtttgctttattgtaatgtggccgtgtatgtgcgtaattcgcttgccaatacatttgatacattaaaagacgcaggttttgaagaagatgttctgattgaatatcctatcgatgaaacactgagtttgcgggagtttgaggaagaagtggaagaaaggttcaatttttcactggagttgtgcaacaaagacaacaaacccttcatgaataaaagccagcacttattccagattgcctgcccggtagccgacagaaacacagaccgtaattaccagctggatatttcccttgacatgctgacgaataataaccgtcagtcgccccagcaaaatatgtggtaattatttgttcgccctcttttatatcctctcagctgacccggcttatcttctctttaaaattaactacgcgaaaaaccttttatcaattaacattctcgtaatgccccgttaacactgcggtaatgtagtgccaatacttttgccatcaaatattaaaacggccttaaaaccgtattaaaatctgattaaaaaattattgtgaaacgaatctcttctatacttatctggacactgttagcgtgttgctccttcgccaatgcttcctttgcagctgatcccgccaaaatcaccggtaaggttaccgacaagaaaacaggtgaagccatcatcgggttaactgtagtagtagctggtaccggcaaaggcgcagtaacagatgtggaaggaaggtaccagatttcagttgaacccggcacttataccctggagtttaaattcatggggtaccagacgaaatcagtttcggaagtaatcgtaagtgcaggtaaacctacgtacctggacattgtaatggaagaaagaagttccaaaagcctgaaggaagtggtaatcaccggaacggccaaacaggaaaccatcaattccctgcttacgctgcaaaagaataccaacacagtagcacaggtagtatctgcagaagccatccgtaaatcgccggacagaaataccggagaagtattgaaacgagtatccggcgcctctttgcaggaaggtaaatacctcattgtacgcggactcgccgaccgttataatcaggccacggttaacggcgccctgttgtccagtacagaaccagaccggaaaacattttcctttgacctgtttccatccaatattgttgaaaacatcgtcatcaataaagcagctgtacctgaattaccggcagaatttgcgggtggccttgtacaggtaaatacaaaagatatcccttccgaaaatttcctgacagtattggccggtacgggttttaataccatgtcggccggaaaggactttaacacttataaaggcggcaacaaagactggcttggggtagacgatgataccagaaagctcccgtcttcctttccatctaccaaagccggttatgatcaactgtcaacagcagataaaattgctgtatccaaatcattcccggatatatggtcggtaaatacaaaaacaacaccgcttaactctaatttccagattgccggcggtatcaataaaggaaaagaaggtaaccgttttggtgcggtactgtcgctaagctacaaccgtaacaaccgtaatttcgatacttaccgtaccgactttgataatgacggatcccggatctacaactattacgataaaaaatctactcagaatgtattgtggggcggacttgctaatttatcctaccagtttggcaagaataagatcagcttcaaaaacctgtacagtgttaattctaccgtggctaccacagtaagaactggtaacgatattccatccgaaacagatgtacgcgcttatgaattgggattcaacagcaaccgcatctatacttcgcaattatccggtgagcatttctgggagaaagcaaaggtgaagatcaaatggaacggcagctacaccaacatgaaacaggatgtgccggatcttcgccggttgggttataacagcattgccggtaagaatgatttttatgccaatatatcttccggtggttccgctacccttactggttccggccgtttctattccaaactgaatgataatatttacggtggtatcctagacctgagccggtttgtgaaaatcggtggccggcaacaacaggtaaagatgggttacctggttcagagtaaggaacgtggtttcacgccacgtgcgcttggctacaccctttttgatgccggcgatccttatgcacatgacctggtgcgcttaactcccgataaattatttgcaccggaaaactttaccgaccgcttattgcggatggatgaaattaccaatacgccggatgcttatggcgccaatgcgctgctcaacgcaggttacctgcagtttgataacaatatttatgagaaatggcgactggtatggggggtgagagtggagaactttgaccagtcgattaaatataaccagaacggaccacagaataataaaactacggtaacggatatattaccttccgtgaacctgacctacctgctgaatgcaaaaacaaatatccgtttcagcgcatctcaaaccgttatccggcctgagttccgtgagcaggcgccgtttgccttctacaactttgatctcatggctaccgaatccggtaactctaacctgaagagaagtaaggtgaccaatgtagatctgcgctatgagctgtatccccgctccggagaagtattaaccattgctggtttctacaagcactttgaatctcctattgaaagattttacaatagtggtgcgggttctgttggtttaacctacctgaatgctcctaaggcgaatagcgccggcgccgaagtagaatttagaaagaatctcgattttctgaatcctgataatgcaggattctggcattctttcacggtgttttctaatgtggcctatatctataataaagtttctttcgaaaaagataaagtgctgaaagcacggcctatgcagggtcaatctccttatgtgatcaatgtaggtttacagtttgaaaaagaatctaccggtactgtggcgaatgtattatttaaccgaattggcagaaggattttcattgtaggtaacgacacggagcctgatgtatatgaagcgccgagatctttactggacttcatggtagcgcagaaggttttccgtaaaggagaaatcaagctgaccgtaagtgatatcctgaatcagccggctaatttttaccaggataatgacgacaacggcaagtacgacaaaacatcagacttcctgagaataagtaccaaaggcggtaccaatgtgaatctttctttctcttataaattctgataaagagaagcgtaataataggaatagtagattttaaaaattgcatttaatttcaatccatctgacatgaaaaaaattctgtttcctgtaatgtttttggcggtgattatctcatcctgcggcaaagacgatgatcctacaactccgccaccggctcagccagtagacatgactaaggctactattgaaagaaccagcgataacagtgaatttaaggaatctcctgaaacactgccaaagcagatcacttccaatactgttttgaaaacaggtaaaacttacctgctgactgattttacttttgtattgaacggtgcaactattaaaatagaaccaggtgttaccattaaaggatccaagtctccgaataaaggtgcgctgatcattaccaggaatggtaagattgatgcacagggtactgctgccgctccgattgtatttacatccagccaggctactcctaacagtggcgactggggtggtattatcctgttgggtaatgcgcctaacaatggtgcaaaagacggtattgccggcttacaggccattgaaggcggtgtaaatgaaacggctactggttacggtttacatggtggtaccaaagctgatgataactccggcatactgaaatatgtcagagtagaatatccaggtattgcctttgccgtaaacgatgaaatcaacggtgttacttttggtagcgttggttccggaactaccattgattatgtacaggtaagctattccggcgatgattcgttcgaatggtttggtggtacagtaaattgtaagcacctgatcgcttatcgcggcacagatgacgatttcgatactgataacggtttctccggaaagatccagtttggcctggtactgcgtgatgctgctatcgctgatttcggtccgagcggtgcttccaacggttttgaatctgacaacgatgcggacggtactaccaaaacgccgcaaactgctgctactttcagcaacatgactattgtaggaccttacgctaacgccgctccggctgctactgctgctccttacaaaagaggtgcgcatatcagaaggaacagtaaaatttcaatattcaactctgtatttgttggctggcctgttggcttgtttgtggatggtgcgctgacagaagcaaatgctacttccaatgcactggagtacaagaataacaccattgccggtagcccactggtggtagctgctggtaccgcaacatttaattccctggcctggttcagcactgcagcatttgccaataaaacactggctgctgttactgatgtgaaactgaccaatactgggtatactacttttgatccaagccccgcagctggttctccgctgttggctggtgcggatttcaccaacgcgaaattaggtggtggcgcttttactaccactacctatgtgggtgcagcagcagcaggtgacacctggtttaaaggctggaccaaatttgcagataaatagtatttatttaaatttcataaactgtaatcttaggccgcccgggtttttacccaggcggctattttttatttgcccagtttagccatatacttctccggtgctttttcaaacacatttttgcaggtagccgagcaaaaatgcagggtatctgttttatatactgcccattctttataactggtatcgtagggcatttcacaaacggggtccggaagtttattgactgcaatagctgctggtgtttcggcagcgggagcagtagtattttcagcgggcgcctgcttttgtgcgcaggcaaacaggaataaggcgctacacgtaatgaatatatatttcatagaattttttaacgaaggtatagataaaaaagaattacggatttgcgggagatagtgaactgattacacttcttccaacaaatccgtaatactatatagtaattgcagcagttattttaccagatcactacccgttctgcttccggcagcaccattttattgcccggagcgcagccccatgcagcctggaattcagccaggtgaggcagtggtccgttgatgcggaattttgccggtgagtgcggatctgtctggatctggttgcgcagggcagcatctgtgatgttgccatgccatacctgtgcccagcccaggaagaaacgttgctgccaggtaaatccatcaataggtttgggttcccctttaccttcaaacgattttacgagggcgtgataagcaagcgttaaaccacccaggtcggctacgttttcaccgatggttaaggcgccattgattttgaaaccaggcagcgcttcaaggccgccgaagtagtcgatataacgcttggtcagtttatcgaagttcttgcggtcggcttctgtccaccagtttttcaggttaccttctgcatcgaactgtgagccctggtcgtcaaagccatgggtaaattcgtggccgataacggcgatgataccgccatagttgatggcatcatctgcattaggattgtagaaaggaggctggaggatacctgcagggaatactacttcgttgtttaacgggttgtaatatgcgtttacagtttgaggcgtcataccccattcgcttttatctaccggtttgcctattttatcaacattttctttgtgtacgtataagcttgcggcgattacattttccaccagtttacctttttctatattgatggaagagtaatctttccatttgtcggggtaaccgattttataggtaaaggaagcgagttttttgtgtgccatttgtttggtagaatcgcccatccaggtgagtttatcgattctttctccatatactttacgcacgttttcgatcatttcagatactttctgtttgctgctttccgggaagtactttttggcaaacagtttacccagcggcatgcccatttttccatcggtggagcggatagcgcgttctgcgcgggttttctgcgactttttacctgtcattaccgtaccgtagaaatggaaattttcattatcgaaagtagcaggtaaataaccggcaaactggccgagcagctgccatttggaatatgttttcagtgtttcgagtggcgtagctttcagcaaagcgttggctttggtgagataggtcttgttctggagcacgagggtatcggttttgatatcctgtttagcggcgaagttttcccagtcgaagtcgggcgccagtgttttcagttctgagaaggcggccctgttgtacgttttaaccggatcgcgcagttctacattgctcagctggatagcggcgagtttggtttcaaaatccaggatggtttgtccggcgcttgcttcagggaaacctgccagtttaaacattttatcaacgtgactaacaaattcgctgcgcacatttttggtagcggaatcctgtctttcgtagtagcttttttcaccaaggctcaggccatcctgtgcctggtaaagcacattcattttactgtttttggcgtctgcgtctgcaccaaaaccggtaaaggaagataccccgattttctggagttcaccggttacgctggcccagtcggcgagtgttttaatggcggcaatcttatcgaggtagggttgcagcggagtgatgccgcgttgttcgatagtagcggtatccaggaaagatgagtaatagtcggcgatctgttgttcttctgtgccttttttcaggtctgttttgctggtaatttcagcaatgattcctttgaggcgaacttccttgttttctttatcgagaacgttaaacgctccccagcggctctctgtagaagggatggggttgttttttttccagttaccattcacgtagttgtcaaaatcatcacaggctttgtaggaagaatcgatatcagccaagttaaaagcgggcaccttggtggtgtcggccgtttccgcctgctgcgaggaactgttggaattgcaggctgcaaatgtaaccatggcagccagcaacggtagttttaccgcattggttttgttcatatttaaaacaggtttagtatcctaagttatggaaaacgggtcaggttgcatgaaaggttttttatgaacggcaatcgccgccatgatggctgttgccgatcaaatcccggaatctctaaataattaggtaggtttgtgttacgtaaattaacatataaatggatttcaggtttaaattgtacagggttaccacggctatagtattgatgatatccggtattttcacattcatgctcttgtccagcatactttttctgggtaccaacttcgggtcaattgtattcctgctttctatgggggcctgttttattcatagcgttttatcattatatcttcagcggagcctgctattaccggaaattccgctgaaagagagtacgccgggtggcatgagatttatgggtacaatagggctgatatttgctgttctgctcattttgtcggggttaaccatattgctggttacgccggagcagatgaaggcggagatcgacaatctgccgccggatcagcaggcggcggttaaacaaaccctgatagcgccgataggcgttttcctgctggtggtgggaagtttgatcgcattgaatatagggttgtcgttccggtatctccgtcagtggctgcaattgcagggcgggaggagcgaagaacatgaagaataaaaaacggagttatggaaaagcgggagatagccaacagggatgatatcatattactggtaaacagtttttacgataaagtaaaagcggatgatctgatcggctttatttttaatgatgtagcaaaggtagactggccgcatcacctgcccattatgtataatttttgggaagggattctgctggacggcggtaattacaagggaaatgtgatggatcctcattttaaactgaataaactgatcccattggagcctgcctattttgaccgctggctgcaactgtttgaagccaccgtcgccgaaaattttacgggagaaaaagccgcactggcagttacccgcgcccggtctgtaaaagggatcatgtcgtttaaaatgaaccagatcaatcatcctggtaccggcaatcaaattccgctcgttaacccgggcaataaacaataaaccaataagtgtagtatgcaaccattagcggagcggttaagaccggtaacgttggatgaactggtggggcaggagcatcttaccggcaaggacagtattttaagaaaagcgatagagcagggaatgattccttccatgattttgtggggtcctcccggtgttggaaaaacaactattgccaatatcattgcacatacattacaggtgcctttttacacactcagtgctatatcggccggggtgaaggaagtgagggaagtgatagaaatggccaggcggcaacagcatgcggtgttattcattgatgagatccaccggtttaataaatcacagcaggatgccctgctgggcgctgtagagaaagggatcattacgcttatcggcgccactaccgagaacccctcttttgaggtaaatgcggcggtattatcccgcagccaggtgtatgtattgaaacctctcggcaacgatcagctgatgcagttgctgcaacaggccatggaacgggatgagtggctgcgcagtaaaaatatcgagataaaggaaaccagcgccctgtttaatatttccggcggagacgcacgtaaactgctcaatctttttgagctggtggtgactactttacgggaagatccgcttgtgattaccgataaaaaagtaatggacatcgcccagcaacgggtagctatctacgataaaaagggagaacagcactacgacattatttccgcgtttatcaagtccatccggggcagcgatcccaatgcggcattgtactatctcgcccggatgatcgacggcggagaagatgtgaaattcattgcccgcaggctggtgatcctggcgtcggaagatatcggcaacgccaatcccaatgcacagttgctggccaccagctgcttccaggccgtaaacctgatcggctttcctgaatcaaggattatcctgtcgcaatgcgttacctatctcgctgcttctgccaaaagcaatgcagcggttgctgctatcagcgcggcgcagtcggtagtcgctaaaaccggcgacctgcccgtgcctttgcatatcaggaacgcccctacgaaattgatgaaagagatggactatggcaaagggtatgcatacgcacatagttatgaaaacaattttgtgatacaggaatttctgccggatgctatcaagggaacgaaattttatgatccgggaaataacccgcgtgaaaatgaattgaggaattacctgaagagtttgtggaaggaaaaatataattattaaagataaagtattaaagacaaagcggcctgttcagtttgctgaacaggccgctttgtctttatgcaggcgttacttcccggatacttctccaatacttctcggatacttctcagatacttaggagtagcgtatgtgtcgtactccctatacagtccccatacagtccctatacagtccccatacagtccccatacagtccccatacagtccccatacagtccccatacagtccccatacagtccccatacagtccctatacacttccgatacactccccatacactcatgatacactcctcatacactccctatacacttcccctatttgaaatgcaaaacaccttcctggaaatagtaactcacttcagcagttgaaatgaggttgtcgaggaagtcctggagtttcttttgtttgttaataatccctgtaaagcacttcttccctactgcggggttatctatcactacctgtacatcgtaccagcgctgaagggtcagtgcaatttcctgtacgggcgtattgtaaaatatatattgtcctttcatccacgacagcacctgccgctcatcaaaagcagctacttgtacaggcgcaccggcagtaacccgtgcctggtaaccgggcttcaatcctacggtttgcgtggacgtgcgcatgtttacacttccttccaccagtgcaacttttactgctgcggggtcataggagttgatattgaaagcggtgcccagtacttcaatggctgcgccgccgggcaaatgcacgataaaaggccgcgaagcgtctttggccacctgcaggtaagcttctcccctgatctctatttcacgggtgttgccggtgaaattcaccgggaaatgcgcggtggtagctgcattcagccaaagtatggagctgtcggataactttacctggtaatccattccggttggaacgctgatcgtactccattgattgctggcgcctccctgcagggttaataccttcccgttgttatgaaagcgggcatctccggctacaatagcctggctgccgctaccagtaagatcaatttccttgccgtcgtcaattttcagcagaatggctttggccggcgccgtagcggcgatggatttttggtgagtagccccgggcaatttcaggtacagcaaaacggctgttgcagcggcagcaatgccggctgccatgccgatataccgggtgattttttttctccgtgcttttttcaactcattgtgcaggttggcccattcctcgcgcgtatccagtttctccatcattaccttgcctttgccaacagagaagagctgctgcatttcctcccacatcacctgtacatcttcctgttccgaaatcaggcgctgtagcaacagctcatcttccggatcaatatgattgtccagtttatctatcatcaggctttttatttcttctgcagtatggtccatatattttgagctcaaagcattttctttcgtaaaaattgcagggcgcgggatagtactgttttaacagtattaatgctcacccctaactctgccgctacatcattacggcttttcttttctatgtaatacaactggaagatccgcgcggtttttggcggcaattccctcattacctgtaataaatgatcggccctctgctgatattgcaaggcctgatcttcgtctccgtgtacttttattacagcggtatctgactgtaccgcatattgatatcctaattctttctgctcgcgcgacttctctgatttttttaaattaagacacctgttgcggacgctttgggtcaggtatgcttttatggatagaatatcttccaggttttgtttatgccacagatcaataaatatttcctgtaccacatctttagcctgctgctcatccctcagcaggtaaaatgcctccattaccattcttctgtaatgaacagagaatatttcaccgaatgctttctggttttgttctgacatcttatagcagcaatctaacgaggaacaggttggaatttctcttacaaacctaaacaaaaaaaatattcaaaacagtataaaaaatttgtcacccgttacggacaaaagttgtctatagaacaaatttcacgtacttgaaaaactgaacgtatgccacattatgtacgaggtgcttttatttttctattgtcatgtttttactttatcccggccagtggccaattaccgtcagacaaaatttcattgaatgtcaggaatgtatcgttaaaggaaatttttaatcagattaccgcaaaaacgggctacgacttattttacagcaatcagcagatcaacgaccagcaaaaggtgtcgctgaacctgaaggaggcggctctccaggaagtactgaaagccgtattgggaaacggttttacctggcagtaccgcgacaaggtcatttacattaaaaaaaaggaaggtctgcccccggattccacgcgcaatgcgcctgcattaacggatactgttatgcgtatttcggggaagatcacagaccagaaaggcgtactgctgcccggcgcctccgtgaaactgaaaggcaccgacaagggtggcgttaccaatgaaaaaggggaatttgacatccccgatgttacgcacggcgcggggatactggtggtatcttatatcgggtttcaaagccgggaagtagccgtcaaaaaccgctcgcagatcaatgtaagcctgatgggcgaaggatctaccctgaacgacgtactggtaataggttatggtacggtgaagaagaaagatgtgaccgcatctgtatcctctatctcaaaggaagccatgtcggagagaacattgttttccctggcagatgccatgaaaggcaaagcagcgggtgtgcagatcacccagaacgatggcacgcctggttctgaaagcaccatccgcatccgcggggccagctccatcagtggcggaagcacacccttgtatgtaatagatggggtgatgcaggaaaatgccaatgatattaacccgggagatattgaatccattgagattttgaaagatgcttccggcactgctatttacggggcccggggcgccaacggcgttatcatgatcactaccaaaaccggcaaggcaggaaaaacagtggtggaactgtacgccaacaccggttttcagacacccggccacctggtaggcgtaatggacgcttcggagtacgcgcatgcccgcttcctggcttcggcctatacctatacgcccgcagatgccacagatcccaataagccgggcacagaactcaccggctacacctattaccgggatgccccactgggcagtcccgccggtttctggggagtagccaccgatgaaacgtatcacgactggtacaactataataaccccgattcaacaaataccgactggcaaaaggccatgtttcagaacagcgccatacaggaataccgtattatcgcttccggaggctcaaaagacacgaagttttcttttatgggcggttacctcaaccagggaggactgatcgtttacagcggctatgagcgctttaacgggcggtttaattttcaacagaaactatcacccgcggtaaccctgaccagcaatatttccggcagccggactactatcaacggttttatctccggttcacagaacggcggcatcacctccaatagtgttatcaccagtatgttcagccagcagccggtaaagccgctcaccttttccgatattgaagataatgaaggggtggaaggttacatcagcaccaatccctattcgctggcaaagaatgttaccaataaaagatccaatgccgaatgggtaacacgcctggcgctggactggaacattaacaggcatttcacctttcgcacaaccgccaattattctgctgtaaataccaatacagatgcctattatcccaagaatacatcttccggcgccaagtatggcgggcgcgcagtgctggcgagaggcgccactgataaactgatgaatgaaaacctgctgtactataaaggcaatataggcagggaccacagtattaatatcatgggcggcgctatctttgaacagaacaaagcaagccttgttaccgccgaaaaccagcattacgatatagagttgctgggaccatacggcctgggaaacggtaccgtgccggtaatacctacctataacattaccaaatggacgatggcctctttcctgggaagggcggagtacagttaccgccaaaaatatatggctacacttaccatgagggccgacgggtcttcccgcttcagtaaagataacaagtggggctacttcccttctgccgcagtagcctggagagccagcgatgaaaagttcctgaaacctgtacacgcaatcagtaacctgaaattccgcgcaagcctggggcaaagcggcaatacggcgatcccgtcttacctgacactatctacgattactacctacttttccccgatggatggtaacactcccgattttggggtagtggtggaaagacctgaaaacgcttccctcaaatgggaaaccaccacacaggtggatgccggcatggacctcggattatggaatgataaagtaaatattacggccgactggtacctgaagcggactaaagacctgctgatacaacaaatcacgcctggttacagcggctacaggagttcatggaataacctcggttccatccagaacagcgggttcgaatttaatatcagctccccgctgattacccgggcgcaatttggctggaacctggatgctaacattggcgttaaccgctcaaaggcggtggaaataggaccggatctgggtctcgatcctgccgtggtagcgggaattggtaccaccgctattatcaggaacggtcagccgatagggcaatggttcggataccaaaccaatggcattttccagtcgcaggcggaaatagatgcatcggggcttaccgttatcaacggacaggccatcagtaaaatacggcctggaaccaggaagtttattgaccagaacggcgacggtatcatcaatgcagccgaccgtgtggtgctgggacagggacaaccatcctttaccggcggcctcactaattcactccggtataaagcatttaatctgaatgtggtggtgcagtacagttatggcaataaactgtacaatgccaacagggtggcaatggaagccggaaggagcacaaataatatgtcgaaaggatccgttaacgcctggcgtccgtctttatatgatatgacatcaggggaactggttgaaaaagggaatccgaataacagctaccgcatgcccggtagcccggaagaattgctgatgttatccgactggatagaagatggcagttttatccgcctgagcgatgtaaccttgtcctatcattttactgcgcggaatgtagggaatatcacgctttttgtaagcggtaaaaatctctggatcagcacaaaatactccgggtatgatccggaggtaaacacccgccagggaggtttcggggacctgatgccatcattggactacgcctcttatccacgctccagggtatactcattcggtttaaaagctcaattctaaatgttatgaaatcagctattatacttgcatgtacgatcgtacttttttcttcctgtaaaaaatttctggaagaaaaaccgcaaactcaatataccaccgacaatttttttgttgataagtccacactggaagcaggaattgtaggaatgtattcttctgcaaaagacctgttcggcgtatacaccaataccccgttgttcatgacagaaataggtacagatgaagccatgttcaaaggaacttccggcgtacgttttaatttcgaccgttatactttttctgtaagcgaaggatcgatctatgaatactggatcaggcactatgaaattgcggcaagggctaatattgttattgatgctgccgctaaagttgccaccatctctgatgccgacaggaaagtgattacaggagaagcccgttttatccgcgcctttgtgtacttccggctggtacaggcttttggggatattcccatcatagagaagccaatcagcggaaaatttgattacggtcttccgagacgccccctcaaagaagtgtacgacttcattctcagcgatctcacctttgcgtcgcaggatggtgtgctgacaacccaaaaaacaaacgacggacatgccaatcaatgggccgccaaaacgttgctgggcaaagtatatctcaccatggcctctgcaaaggaaaccgcgctcaccaaacaaacgggcaaagtagatggctacaaggatatagcaatggatgtaaaagcgttgtatacaaaagcctgggaagcgctgaaggacgtgaaagataacagtggtgcggatctgctgccggtgtacggagatgtgttcaaaattgagaataaaaatgtgaacagggaatcgttgtttgaattgcagttcagtccggtcgttccttatggcacacagtggaccaaggaatatggtatggcttatacaggcggcctggtgaatggtaacccgctctactataccaattctatggccggcgtgaataacctcgtgtatgtgccgaagttttacacctactacaagaaaacgccgaaagacgtggattatgataaaagaagggtatggaacctttccgattccatgatcaatgtggcgaataatgcaccgtctaaattaacgtatatctggacttcgccctactcgccggatgcttacaaccaaactatcctgggacgctgcggcgttaccaaataccgttggggggcttcatggcaaaccacttcgcaatacctgtattccaattgtcccaacaatgtgattgtgctgcgctttgcagatgtgttgctgatgtttgcggaagcggattataaaatgaacggaaccatttcagcagaagggctggctgcgatcaacaaagtgaggcaacgcgcccgcggactggatgccagcggtgttcctgttaccgccgcacaaacgccgggctttaatgactataccgctgcagatattactaccgatgaaatactgatggaacgagcccgggagctttgctttgaatttcaacgctggttcgatctcgcgcgtacaggcaggtttgaggcattcctgaaaaagaaccgggatgccggcaatacgaaaattgtaaatacagccaccagttttgatccggcaaagcattacctgtttcctattccacaatctgaaatagacttgtctaccaacaaagaaaactttaaacaaaacccgaattactaaaatgaaagtaagaagcgtattaatcaaatggatcattggaatgatcttgccattttctgttagcgcgaatagtatggcgccggctgaatatgatgtggtagtatacggcggcaccgcgtcgggcgtaatggcggcggttacagcggcgcgtgaagggcttaaagtagccatactggaaccaaagaagcatctcggcggcatggtcaccggcggcctttctgcgactgatctcgggcgtaaagacgtgatcggcggatatgcgaaagaagtataccagcgctgcggtaaatattacggtctcactgatacggttgcctggtttcctgaaccgcatgtagccgaaaaaatattaaacgatatggtgaaagaagccaacgtgaccgtattttttaatcaccgcctgaaagaaaagaacggcgttaaaaagaaagagggaaaaataaccgcgattaccatggagaacggcgcttctttttctgccaaagtatttattgatgccacctatgaaggcgacctgatggcgttttcaggcgtatcgtatatcgtgggccgggaagcacagagtttgtacgatgagtattctgccggtatcagggaaggctccggtaccaggagcgcttttgaaaacgggaaattattgcctggcatccagccaacacctccggggccaataggcgccggcgataagaaaacccagtcttataacttcagactttcccttaccaacaataaagcgaaccaggtaccttatcctaaaccggccaaatatgatcctgccaggtacattgaactttattattcaactatggatgccattgaaaaactgggcgctgcggaagccgctgcaaagctgttccctggcatgggaaaaatccccaacagtaaagtagatcttaacatggcggattatgttggtggcaactgggattatcctgatggttcgtataagcgcagggcagcaatatggcaggaccatattgattatgtagcggggtatgtttatttcctggcaaatgatccacgtttgcctgccgaattcaggaatgtgtttaatcaatggggattatcgaaagatgaatttgcagataataataactggccttatgagttatatgtgcgtgaggcccgtcgcatgactggtgattgggtgatgacacagaaagatgtgatttcagaaatgcagaaacccgatccagttggcctgggctcctatggcctggatgtgcatcgtgtgcaagggtacgccgacagtaaaggccgtctcaaatatgagggcgggttacaacgtaccgaacctgaacggatgaagcatattccttaccagataccttaccgcgtgctgttgccaaagaaaaaagaagccggcaatttactggtaaccgtgtgtatatcggtaagtcatgtggtatatgccaccatccggatggagccgcagtatatgatcatggggcaggcagcaggcgcagcggcggcattggctgtcaaggaaaataaagccgtgcaggatgtggatacgaaagtattgggtaataaattaatagcacagggagctaagctggagtcaaaaataaagcaactcagcgacttgcctgcaccagcgtcaatagactaaaaatgcgagtatttatctttttattgctgttctggctgccggcccatgctggctggtggccagggcaaaaagcgccacggtcaattgtaattgctgccataaaacatccttcggatatccgtgaaatgaacctggcgcaatctgttgccgggctggctgcacaggcgctgaatgaaggcgccggcgatgaaggtgtgtggattgaaacatccaatcccgactacagcgtttattttcattcactggtagcaagattaaaggctaacgtgccgggtacgtttactccctggcaactggtagaaagatacaaggccaggggaattatcaaaggttacatcctgtatgatttcaacaggaatgataactccgttaaccttgctaccatttacgctgcccttaaaaaaggagtgctgatagatattacacaggaagccatggtcagcagtaaggggctgaaaaaattatatgatgccaccaaagcagattttaaggaagccactcttcatgccttactgccggagctgaatccccatgcgctggtgattgccaacccggcttattccaataacagggattacgcgattgcgcagaaaactatggtttattatggcgtggatactattttccaatccattatcaggtgggtgaagccgctttctccggtaataggatggaataagggagaagaatttaaacacgtagaaccttgcaccagatggggtttgatcaatactgcttcggattggtgcatgaacctggcattgttatcgataccgccggtaaataaattgccgcagatccggtctcttgatccccggaaaattaactgggaggagcagctaaactatcatgcctttgtaatgagcgacggtgataacatgcagtggacattcggcaattttatacacaataaagactattggagtaacccctataatgaagatatcccgatgtcgtttaccacttgcgtgcttaaccttgcccaggcgggcagcgatgtatatacctgcctggcgaagtcccagcccaaacacaactccatagtggagtatggcgccggctattattacccggatctctttgccaggtcaagaccggaaccagctaagctgctccgggaatatgccggtatgatcaacacagagatgaaaagaaccggcgcaaaagttttcggatttatctgtaaagatgtttcgggtgagcaggcgttggaagcctacaggatctatggggaagagatagaagacctcaccggtatgatagccgtacagtattcgccttataatggcggttatggaaaagttttctgggtgaaaaataaaaaaggaacagagataccggtagttacctgtaaataccagctatgggccaacctgagcaagcaaggctccggtgatccggtgccgctggcagactggataaacaacgacaacgcatcatcttcttcaggaagcaaacaactgaactggaccattgtacatgcctggtcgcatttcagcgacagtgccacacatcattccattgttactaaagataaaagcattactaccgcccaacgcggcgtaacaccggttaaatggacaaaggatctccttgataaaggaacaaaggttgtttccattgaagaacttttatggcggatcaggatgcagcataatcctgcagaaacccgtaaagtggccggtattcaccaataatcaactaaacattatgcaaaagagtacaaaggcaggccagctgctttccatcccggtgattgtagcggcgttgggttattttgttgacatctacgatctgctgctgttcagcattgtgcgcatgccgagcttaagggccctgcacgtggcagaaaatgaattgatggaaaagggtatttacctgatcaatatgcagatggcggggatgttgctcggcggcattttttggggagtattgggagataagaaaggacgactgtctgtattgtttggctctattcttttatactcggtggccaatatcctgaatggttttgtgactacagtagatcaatatgccctgttgcgttttatagcggggatagggcttgcgggggaactgggcgccggcattactttggtggcggaaatactgccaaaggaaatacgcggttatggtaccgccattgtagcgtcagtaggtgtgctgggagcagtgctggcctattttatagcagatcttttcgactggaagatcgcttattttattggcggcggactggggttggcattgcttgtactgcggtttaatgtatttgaatcgggtatttttaaagaagtaaaaaaagcacaaagatcacgcggtaatttcttctccttattttcttccggtaaaatattttttaaatacctgagatgtattatgatcgggttacctatctggttcgtgatcgggatcctgattactttttcgccggagttcggaaaggctatcggtcttactacagctgtggaagcaggaaaagcggtgatgttctgttatatcgggctttcgctgggagatatgagcagtggcttgttaagccagtatttaaaaagcaggagaaaaacggtgcttatttttgtgatgctcacctgtgcggcgatagttgtttacttaagtcagcggtcgcagagtattgttgtcttttactcactgtgcggttttctggggtatgccattggttactgggcgttgtttgtaacgattgccgcagaacaatttggtaccaatatgcgggcaacggtggccactacggttcccaattttgtacgtggcagcgtgaatatttttacgcctgcattccttttgctgaaaaatcattcaggcgttaccgttgctgcgggtatggtgggcattattaccattatacttgcgctgctggcagtatggaagatggaagaaactttctccaaagatcttaactacacggaataaattattatctcttcaaaacatatataatgaggaagaaaaactttcttttactggcgggtcttattttttcgatagctgcaaagtcgcaggaaacgtatgatatatgcgtgtatggcggcacctccgggggtgtaatagcggcttatacggcgaagaaaatgggaaagtcggtattgctgattgagccggggaagcaccttggcggcatgtcatccggcggactgggatacactgatatcggcaacaaatatgcggttaccggtttgggtattgatttttaccgcagggtgggtaaacattacgggcagtttgagtcctggatatttgagccgcatgtggcagaggatgtatttatgcagtatatcagggaagccaatgtgccggtgctttaccagtcgaagatggtggcggcggtaaaggaaaatggttttattaaggagatctcagtggagagcacagcggctccatcgaagcaacaaaaacatatccgtgcaaccgtgtttattgactgttcctatgaaggtgacctgatggcaagggccggtgtatcttatacggtaggaagggaatcttccgctgtttacaacgaatcgtacaatggcgtgcaggtgcagcctcctgctacaccgcagcatggtaaccaggtacccgacggcgtagacccgtataagatacccggcaatccatccagtggcttgctgtggggcatcagcaacgccaggctggcgccaataggaagcggcgataaccatgtgcaggcttataatttccggatctgtttaaccgacgatcctgctaatcttatacctattacccgcccggaagattatgattccagccggtatgaaatattgccccgctatatagcaaagctcactacacctaatgatatccgggagatcctgaaatttgacctgatgcctaatcataaaacagacatcaacaatggtggcggcttttctaccgacatgataggcaggaattgggaatatccggatggaaattacgctaccagggaaaaaatccaaaaggaacatgaactgtacaacaaggggctgctgtattttatcgggcatgatccccgtataccggacagtgtgcgccggtttatgctgaactggggataccctaaagatgaatacgctgataacaatcactggagcccgcaaatgtacatcagggaagcccgcagaatgcgcggcgtatatgtaatgacgcaggctaattgtgagcggaaggaagtggtaacggatggtatagggatggccgcatatggcatggattctcacaatacccagcgtcttgttattaacgggatggtaaagaatgagggagatgtggaaaaaggcggcgccggtccgtatcctattgcttaccggtcactgacgccgaaagagaacgaatgtaaaaacctgctggtgcctgtttgtttgtctgccagtcatattggttatggctccataagaatggaaccggtattcatggtactggggcagtcggccgcggtggctgctgcgtttgcggttgacgggcacaccacggtgcagcaggtagatgtaaaaaagatacagacattgctggctgcaaatccattgatggatggcagcacgccagagatcctggtggataatgatgatgctgcccatgtggaaatcaccggtaagtggtcgcttaaaaaaggaggcacttacggtccttctgctctttattcttctgaaaatgacgagcctaaatccgtaaaatttataccggaagtgaagaaaggtggaaactatgacatctatacctatgtgttgccgcggataaataatgtatctcccgctaccaaagtaatggtatttgatggcagtcaatccagggagataactattgttaaagagaaggtgattgtaaacggtcagaccagcggtgaatgggtacatttagggaaatttaatctgccggcaggcaaaaaagccggcatcactatctccaataaagaagcgggtggcgtgattgtggcggatgccgtattactggttcccggaagatagtatgcttatactactctctttctttatctaaaatttcaaatgattgttctatcctttcgccgttttcatctaccagtgtaataatatgtttcccggctgcggggtgtagcgccatctggtgaaactctgtggtagcgcctatgaagttgttatcgaggtgccagaatattttagtggcattgttccggtgagtggcggtaaagatggtttgaccaggctttccgtcgatttcaacgggcacgaatatacgcgcccctggccggggatagatcagttccataggcgccttatcctgtcccagtgaggcgaggcaatccggcttatacggcggcagctgctgataatagtttttgctgcggtagtaatactcctgtgagggaggcaatacaaaccaggatttatgctgcatgagcgagggtgattcgcaggcttccgttacgcgccactggccggttctgtcgagatgcaccaactggtggtacggacacacacctgccctgatcccggcggccggtacataaatggaatctttttcatcgcatagttcgcctgcacggaagccgcttttgcggcatacctcaatttttttcagttgctgataaggcgtgttagaccagccgctggtatgcaataaacggaacacatcaaagagaatgggcgcggcggtggatacccctatcaggccggggcggccttctccgtcggcgtttcctacccatacccctactacatattgcggcgttacgccaatcgcccatccgtcccggaagccgaagctggtgccagttttccaggcgatacgttgggaagaggagaactgctgccacaacaattcttcgcccggccgcatcacttcagtcattgcctgaaaggcgtaccagatggagcccgcatccagcaggccgtctttactcaatccgtatttcgacgggcgttggatattaagccggtaattgggaggatgaatatcatccatatcgtacttacctttatattgatccatgtgtagcagtgtacgggccatgctggcatacataccgcacatttcccacagggtggtttcgccgccgccgaggatcagtgataagccatagtggtcggctggtttgttgagggtggtgatgcccattttttgcagcagggaatgaaaccgttcgtagcggtattgctgcaacatacgtacggcggggatattgagggatctggccagcgcgcgggaagccggtaccgcgccatcgtaaccgagatcaaagttttgcggcgaatagccggctatctgcgtaggaatatcggggatcagtgtattgggcaatatgaggccgtcgttgagcatggcggcatagagcacgggctttaatgtactgcccggacttcttctcgcctgcacaatatctacatgactttccagctcgggatctgaagggtgatagatgttgcctacatacgccagggtgttaccggtttctacgtccagtaccaatacagctgcattattgatgccgttcgccttataagcattgtgataacgttcggcgatggcggtggcgttatgttgcaggtcggcctgcagggttgttttgatgcgggtaggttcgtccgtttgctgttgcaggtaatcacggcggaacaggtccagcaggtgcggcgcttcctgtggcaatggtaagggctgatccggcaggggttctaatttcgccagctggcaggtaatgctgtcgatggtgcgctggcgatataatttattcagcagttgatttcgtttattcagcaacgttaccctgttgcggccgggatgtaccagcgcgggactgttaggtaataccgccagtgcggccatttcgccccacgacaataaatcggccttacggccataataccgccaggcggcggcttccagtccaactacattgcccccgaaaggtgcattagcagcatataacgcgataatcttctttttagaggccgcaaattccagccgcgtggccaacaccgcttccatcatcttttgccagatattgcggggctgattgcgcgacaagcgaataacctgcatcgtgagggtgctgccaccgcttacaacttttctgtcacgggcgttttgattaatagcccggcctatggcgataggatctatgccccagtgataatagaaacgtttgtcttcatatgcgacgatacacttttcaaatttatccggcacatgtgcattgtacggaaaccgccattggccatccggtgcaatgctggcgttcagcagatcgccgttgctgtcttccagcacataggaggttgggctggtaaagagttgtttgggtaaacaaaaatagtaggcaatgagcacaacagcggccgctgcgagccaccacttttttttgatgcaccattgtttaaggatatcaggcttcattatttttttatgcgcgttcaaagataagttaacttattgttttgaacggctcgtatatctggtagtcagggtgtaatcacaggttgctctctacacattacttctgcccctcttcacctttaaaatccctgatggtctttccatcataacgatacactccgtttacagatccaaaccaaatacttccatcgttagcttccagaatcccaaagaacattgggttatacgttatttcggttaccgttggcctctgatcaggcaaagacctttggtcataccgggaaagtgcccaggcttgattgcgcaggaactttccgtcgtaccggggaactgccaaagcctggctatgatccctctctgaactagtccagatattaccttttttatcctcaactatataaccaacaaacttctgtgtgaaatttgtaaatgtactgccatcatagcgccaaagaccatcagatccgccaagccagatattaccttttttatcttcgattatggaacgaacattcttaaaaggtttgtcctcatgggtaaaaacggagaatgtttttccatcatacacgaaagtattgcctcttgtagcaaaccaaaacttacctgttttgtcttcaataatagcagtaacttcataagggggcctctccggaaaagttttccccgtccggtcctcattcattacatctccattgatgatataattccggaaggatttcccatcgtaacggcttgctcctccaaaaacaccgaaccagatgttgccttttttatcttcataaatactaccaacatcattattgagaagtctatccctggtggtgaaattttgaaaggatttcccatcataataataaacacctgaaccaatagagccgaaccacaagttgcctttactatcttctaaaacagaaaaaaaacgggccgtactcactttactggtaatattggtaaaagattttccatcgtatcgaaaaactccctcccacgaggcaatccagatgttgccctttctatcttgcatgatatttcgggtgatggatgtaggtccggttttaggttgtccgtaggaaaccttaaagatgcctgcgacaataaagacgccaaggaagattgtctgaataattgttttgttagatttatacatcattatgtcaatttgttattgataatgtatttatattgtatcaaccaggttgtctttctggtgggcaaccagctccacgatttcgcctttgcggggctcaaagttgatccggcgaaattactttgatatctttcagtacagggagcttggattgtaaataaaattgtaaactttgtaaataataacttgacactatgcaccttggtcaaaatctcctcctggggaaacgcaaatacctgttgggattgatcctattcttgtttgtctccgtcatctgcgtggctttcatgatgggtggaagtgacgattttgatatttccagaagggaggttttacttcgccggatcggacatgaactacttttacagtcgggcgacagtacctcaagggtgctcccggtaaaaaagatcgctgaaaatgaataccggatcacgtttgagaatgatcttacttttcaaccggactccctggtgaataccactcggcgtttgctggccaaagacccgctcgcacgtgattatgttgttaatgtgctgaactgtagcaactccagtgtagcctatggatacgctatctccaaaaatacaaaagatgatattgtaacctgtatgggaagaaagcagcccaaaggatgttacatgatcaatgttaaattcaaaccggtgggtataaatactgcaaagaatggatatctcctgggcagcctgccgtttttagcatttgttggttttctttttttgagatctgttaagccgcggagacctttacctgagaaaagcgctttacctggggatgatcaggatacgggcatcattactttaggttcggttttgtttgatgcgaagaatcgtaagctcataattgatggaaagacgatagacttaaccggaactgaaacccgtgttctacaaattttcgcgttgtctcctaacgagactatagagagaagccggctgcagaaagagatatgggaagatgaaggtgttattgtagggcgtagcctggatatgttcatatcaaagcttagaaaaaaactggaatttgatccgaatatcaaaattgtggttatacgaggaaaaggatataagcttgaagttaactcttaataaaaattctctcaccaattttctcttacccgggaattgctaaaacaaaaaagccctgcataactgcaaggcttcttttctaagtcggggcggcaggattcgaacctgcgacctcctgctcccaaagcaggcgcgataccgggctacgctacgccccgtctccgacgctatgtagcgggatgcaaatgtaggaaataaatatccacaaaaacaaatcctcctgaaaaaaacttcagtgatgatattcatttattgacaggcgcaccggaaagtatatccctcaccgttaggccgggtaacaaacggaatacgggaatactgatgccgtatttattgcacagttctttaatgctccggtcaatgagttccgcgctgtacctggaggagaaatgtccgaggatcagctgttttacgcggatatggcttaccatatccatcacttcttccagtttgctgtgcttattcttatgcgctactattttcacatccccttcactggctagaaacgtagcttcatggatcaggatatcggtgccatcccagcgttccatatcctgcacaggcgtatcgcccgaatagccaaccaggttggttcttacttccattgtggtgctttcttttcctcgctccataatgatttgccggatcgtttcggggggaagcgctgccagctccggcttcactttttgtttcacctgcattaccttatagctcaggctccggatgatgtgcgcatcggtagttacatgttcgttacgcacaggaataaccactacatcgtcttttacccatatttcatcgcccggcgctaccgccctccattgtgtactggcaatatgaggatcaaaatttttggagaatgcttccatcgccggaaaagaactgctgtcccttggataacagattaccggcagtccatcccgtgcattcagctggtttagctgcagcaggcccgttaaatgatccctgtccgcatgagaaataaatacatagttgatcttcctgcttttttgcaaaagtgcagccgttaatccatctcccgcatccattaaaatacccagttcttccaggaagtaccaggtggaaaataaggcggtagagtagcctgatatcgttagcttcatcagtggttcttagttatgttataaagatagacatatttcacagactctccaccagtaggtataacgacaaatctgatatggttaaaataaacaaaactgaatctgttttatttgccttttatagctgaattttacggtctcaatatttgttctatgatgcagataattaacagtacacaggaagatatcgatgtaatctttagtctttatgaagccggcacacaacttcaaaagaaaattgcacagaagcactgggagggatttgaccaggcgctggtggaaacagatatccgtgaaaagaggttatggaagataatggaggacgaccggattgcctgcatcttttctcttacattccaggatccctttatctggaaagagaaagatcaagatccggccatttacattcaccgtatcgccactcatccggacttcaggggcaatggttatgtaaagcatattgtacggtgggccagggaatatgcggtaagtatcgggaaaaactatatcaggatggataccggcagcggcaatgataagctgaataactattatgtaagctgtggctttaattatcttggcgtggtggcgccggtggcgagcgatgagttacctgcgcattataagggggggacttccagcttgtttgaaatagtgctgtaaggcggttatgagagtatacataattaaaaaaggctttccgtaaacggaaagccttttaaatgctaagtcggggcggcaggattcgaacctgcgacctcctgctcccaaagcaggcgcgataccgggctacgctacgccccgaaatcccttcttagtccgcatcttctgcattaacagctgcccttgcggcaatacctttgcttcaattgcggagtgcaaatgtaggaaaatgtttaacataaaaacaaatttttttaacaaaaagacgcaaaatataatagaatgccctgctacgctggattacacgaggtgacaattttctcaagaaagtaacaaacctgtgaaataagatcgctcaaagcgcatccctttccggaaaaatttattcggtacgcaagctttttaccggattggacctggccgctttgatcgattggtagctgacggttataaaggagatgacaatggcaataacaccagccaacgcgaaaaaccaccagcggatgctgatatgataggcaaaattctgcagccatttattcattacccaccacgccacggggaaggcgatcagcaaagcaaataccaccagctttaaaaaatctttcgacaacatccctacaatacccgctacgctggcgcccagcactttcctgaccccgatttccttaatacgtttttgtgtggcaaaagtagcgaggccgaaaagtcccaggcaagacaccattacagataacacagagaaaatattgaaaagctttcccatgcgctgctcggcgaggtataagcgcgacaggtcttcatttacaaaaccgaaagaaaatgggaaatcgatatatacctgctgaaatacttttttcatcgtcgccaggctttgctgcatattggcagccgtagtccgctgtacaatataccctgtgttcccgttaaaattgccggaactgccgttcctgataatcagcggttgtatgggctgttgcactggcttgaagttaaaatcttttactattcctatgacaatgcctgtacggctatccatggttattctcgttcccagcgcagtttccacgtttagcttcattgcttttatggccgtttcattgagcacatagttattttcatctcctttaaaatctttggaaaaaaacctgccggcctttaactgcatcctgaaagtatgcacaaaatgatcatccacccacatttgcggaaataccaggtttgcctgtgggtcctttccttcccattcaaccgaacgggtaccggtgggcagatctgtaggcaggtgactgataaaagtataatcatctatctccggatactggctcattacagctttcagcgccacctggttccgctgcaggtcgcccaggcggggaatcggtacatacaggaggttttccttgttgtaaccgatatccatggtccggataaagtgtagttgtttatacactacaatagtgctcactatcaggatcactgcaatggagaattgcacgatgatcaggctgttcctgaaaaacgttttcctgccatgcagcatctttacacctttcagcactttcaccgggttaaaagaagaaaggaacagcgcggggtaacttccggaaagcaaacctacacctattgctattcctaaaagacccgccatgaattttatattcaacaggttaatggagatggatttcgctgccagctggttgaacaatggtatcaatgcccatgctatcaccagcccgataatcagggagataaaagataataataacgcctcacttaaaaactgcattacaagttgcgaccgcaaagcgcccactgttttacgcatccctacttctttggcccgttgcccggacaaagcagtggacaggttcataaaattgatgccggcaatcagtaaaataaaaaccgcgatcagggaaaagatctttacttgttgatagttaccctggccggctacatcgagcatcaggcgggagcgcagatgcacatcctttagcggctgaacgtacaggaatccatttgttttcgttatatccaggcggcggtaaagcgcctggatctgctgctgtaacgatgccagggctgctggtgtgccactgaaatgatcatccatcagcaggtaagtatatacatcaaaattaccccatccctgttccaggttgatggttctttcatagagctgaatgggaagcaacatatcaaactgcaggtgcgaattacggggaatatctttcagtacacccgttaccagcaggttattgccattgtaatcattgtcaatgtgcagggttttgcccatggcattttccgggctgccaaagtacttctttgcactgctggcggtgagtaccacgccatcgggcctggagagcaggctggacgcgtctcccagcaaaaggggataatcgaagatgcggagaaaattactgtcggcgtagtaaatgtttttctcctcatacttttgattatttactgttaccatgctttgcagggcggccagccgggtggcgttctttacgcccggaacagcttccctgatggccattgcagccggtaccggcaccactgctgctgctatatcccctacacgggccgttaggcggtaaatatgcccggcattggtgttaaagcggtcgtagcccagttcatcctgcacccacaggaaaataagaatgctgcaggccatgcctgtagctaatccaaaaatattgaggccggaaaataatttattcctgaaaaggtttctgaaggctgttttcagataacttttgaacatacgggtgtaagattgatctgttttgtgaaaagccaacaaggtgccagatatgaaatatctttatgctagataattatactttaaagtatttataatgtgtccggttttaaaccataaaatgttcatttttaaagctgttttgtcagcagattgccggcataatccgctgcaaaaatctgcctcttaatttccgcaaaaaatatttgtccaatagtccggatgtcattcgtcataaggtcgtaaacaacatcattcaacgttaaaattcagaaaaatgaaagaattcatgatgatcttccgacatgcaccggaccccaaccgggtgataagccccgggcaaatgcaggccatcctccggcagcggcaggactggatcggcggtatcgccgcacaggggaagttttaagcactggtcaactggggcaggaggcaaaaacgctccgggccgataacgtgatcaccgacggcccttatgcagaagtaaagaaaatagtaggcggtacctgattgtaaaggccacttcactggaagaagcgatgcagctggttgatggctgtcctattcttcttgcaggcggccatgtggaagtaagggacattataaaaatgaattaacacaatcatcaggtccggtgtataacgatcttcttcctcaactattcaaaacagagtacagcaaaattattgctgtactctgtaaactatttggccttccgcacatggaaacggcctaaaaacaaaacaaaagattacctcagaagaaataaaattttcagcgaaaagatagctgccgatctgaaactgcaccggccaccaccggaggaaattgatattgatctctccgccgccaatattcaggacagccagttgaaaatgatgtttgccatctgtcacccggctatccctgcggaagcccggatagggctttctctccgtatcctgtgcggctttggtatcgaggaaatagcggccacttttttaaccggcaaggaaacgatcaacaaaagattgttcagggcaaaggaaaagctgagaacagaaaaaataaacatcgaattgccggaagaagcggatatcgcccaacggctggataatgtgctgaccactatctacctgttgtttaatgaaggctattattccactacgcaacaccaggtgctgcgcaaagagttgtgcctggaagctatgcggctgaattattttctgttggaaaatacgcctaccaatacgccagccgtaaatgcattgatgtcgctgatgtgtttccacgcctctcggtttgaagccaggaccagtgattccggcgcgtatattttatatgaagaacaagaccgcagtctgccggcatcgatgatggaaaggcgctgcaatattttgccagcgctttgcaactggcaaaaacggctgccgataaaaatattatttcgcaatacatgcataaaatcaggagcaattccacgggtaaatagtctctttatttttggacttacggttatcctgctatgtcaaataaatcagtcttttaccggctaaaatccttgcattaccgggagcattttcgtatcttcgttgctgcttaccggaagccatcagacagtcttttttaatcgtaaaacagctactttttttgccactcagccggtggttattgcccggttgttttcaactgcttttattgcatgtaaaaacggtatctccggatacaggaggggattatttgcttttaaagtagcagtggcaggaagaataatcatatggaagaacaaattattacagagaagccggcgtttagagaagcgcttaaattctggtttaaattaggatggataagttttggaggtaccgccggccacattgccattatgcatgattatttagtggaccggaaaaagtggatcagcaacagtaagtttctgcatgccctgaatcattgtatgatcctgcccggaccggaagcacagcaattatccatttatatcgggtggttgctgcatggcagaaaaggggggcttgccgccggtatcttgtttgtattgccatcgatgttcattttacttgggctaagcattatttacgtgctctttggcaatatcccgtgggtaaccgctatgttcgccggattaaagcctgctgtgattgccctcatccttatcgccatgttcaggatcgggcagaaagcgttacacggaccactgcattacggcgtggcggcgctggcatttgtatgtattttcttcttcaatatttccttactggccatcattggcggcgtagttgttattggtatcgtcacgcgcatgatatggcccaccgcattacaacaccaggaaaaaaatacagcaacaaccggagatgaagaacatatgtatgtgctgaataaaaacaccgtatcgcccggagaaggcttccaggcacggcggctcctgaaattactgggtattgcctttatcgcctggctgcttccgtttggactgtttttgttgtttttcagcgactttactttctggaaaaatatggggttgttcttcacacaaaccgcgtttgtgactgtaggcggctcgtatacggtgctgccttatgtggcgcaatacagtgttacaaaactgcactggctcagtaagctacagatgatcgatggttttgcactggcggaaacaacacccggtccgctcatcattgtattatcattcgtgggttttatggccggttataaccattttggcggctctttgtggatgggtacagccggactgctcgctactacctactttacctttttgccctgtttccttatgattttcgccggggctcccctgattgagaaaacgcacggtattgacatcatcgaaggcattcttggattaattaccgccgctgtagtgggtgtgatactaaatcttactttatatctcgggaaagatgtgatttttccgggtggcattttattcagcaagccggatatcctggcgctggtatggatgatcgtatcattggtgctgatgctgaggtttaaaatgaatattttatacctgattgggttgagtgtattgtatggagtgtttcattatttgttatacccttaagggtataacaaattttcattcgtcacttctgctttcttaactcatccagcgccaatgccgtcaggtcttctgttattttcgtcggtgaattacaatcacagttactcattccaattacgtaaatatcttcaccgggaatataaacgcccattgttttgaacccgaatatactgccgccatgttccctggccggcatcccttttatttccctgatgtgccagccatacccataggcaaactcttctccagtgttcaatttatacttcgtaaaagccttttgggttgttgctgcattgagtaacagatgctgattcaaagcattctgccatttcagcatatcgccggtggtggacatgagcgaaccagatgaaaaaggaacactgaaactgatcatcgttttattcacgtatccatattcctttttgtgatacccgtatgctctttttttgatgatttgtctgtcgctgcagtagtaagattgactcatcccaactttatcgaaaatatgtttcccgataaaatccttatatgtctctccggaaaccaattctatgatatatcccagcagcacataccccgaattattatacgcaaacctttctcccggtgcaaaatcagctggttcgcttttgaaaaaattgaccatcatttcaggactcatatctttctgcgcaatcgtcgaaagagatttcatgctggtgaagtccttaatgcctgaagtatgggtcaataaatgatggatcgttattttatttcccgaaggataatcggctatgtatttggagacaggatcctttacacttaatttaccttgttcctctaacatgagaatcgctacagccgtaaattgtttggtcatggaacccaactggaacacgttctccggcgttaaattcacgtctgattccaggttagccttgccgaacgctttctgataaatgggcttcccattttgagcaaccataaatacagcaccggggccatctttgtcattgaataatgttagaatcaaactatccatcctgctttcaaggctttgtgctgaagcaatattgagcgaagtgcaaattatcagcgatagtaacaatagggtatggatcaactttactctagtcattgagatttgttaaatgtgtcctgaatcaatgcgcctggcattgattttaaaaatacacgaatgagtccaatgatctatgaaaatgttacgtaagtggaaatatttgggatgaaaaggatcaaaaccatgcagcagacattatctaaaggcttttaactatgtgctaaatctttcgatttatttaacgggctatgaggggcaaagttcgaacctgtttaatgaaaatttacgagagattatttgctatttaatgaatagtcgataatattactaattgaacttatttatcaagtaactaacacaatccgacttatgaaatatttatttagttttctcttcttgctctacgcaatcactactctaggacaagcatcctttcctaaggggtttaaattaataaaaggtgacaatactaccggagaagacgataggtactctaatgggaaagatgtttttcaaatgcatttctttttcagagcatatgacagcgattacaactggaacgatgataactataaaaaattcatggcagaagcctttggctacccaatgtatcgaactacagacagtctcttgtggggcacaggaaaaattggcgagtattattcctacgtagtcgtagactggcacggtgaaatatttgagcttgtttccgattacaatgatgcagacttttccttctattcaaaatggcttctttcttctataagagcgtatcgtaaaaaaggaaaagtatttatgttcccgacgaggtaccatttgtattacaagcccagggtttaactataagcctaaacagattaagttattttgtcagggtactatgtttggaattaaaaagcctctaaatctttcgcttctttcatgaaatgatagtctttttacaaagactagttgtcttcatgtaacaacattgaagtaaatacttcttgcattgatataagaagtatttacttcaatgtccggaatattaaaacaccgcttcaggataatcggtatatccattttcacccccactatacaacgtatcgcggttgatttctgacaatggcaaattatatttaaagcggattgccaaatcggggttggcaatgaatggtgcaccaaaagataccaggtcggctatgccttctttcaggatggcattcccgctttcctgcgtaaagcccaggttagccatcaacctgccgctgtagtgatagcggaaatggctgaaataattatcctgcaatacttctaccggggtacctgttaaagtttctgcaggcccaacaatgtgcaggaaagcgagattgtagtcattcagttttttaaggatgtactggaacatggggatagtttcttcatccggcgtcacaatgcctacatggctatatgcgaccggtgtaaacttgatcgctacccttgtgctttcccatacttccaggatgacatccagtatttcaaatataatacgtgcacgattttcaatactgccgccatactcatcggtgcgatgattagtggccaggcttagaaattgaggaattaacatgccagcctgtgcatgtacttcaacgccatcaaatcctgcttctttcgcattcttagccgcctgcctgtaatcctgtatagtttgtttaatttcagcaacggtgaactcgcggggcgtttgtgtatctttaaagccctggggtgtataagaatgattttgcggattaatggcggaagggcctgccggcaattcaccatcaaaaaaatccggatgagatgcagcaccaatatgccctaattgagagaagattagtcctcctttgttgtgtactgcctgggtcaccagtttccatccttcaatctgctcctgcgtataaatgcctggcacattaataaaaccaatagacttcggattcacccaggtaccttcactcagaattaagcctgctgaagcgcgttgtgcataatacctggccatcaatggtgtaggaaccaggcctttattggtggcacgtccacgcgtaagtgacgccattaccacccggtttttcaatttcaaatcacctatctgatattcctctaacagaggttgtgctgtatttcccattgtttttttaaggcaaacttcgggcatatgccccagcgttacaatatgggaaaaactaataccatagggataaatttatcccattaaggaattaaaatacaatgcctatttttgaataaagtgaacagcatatgtatgaaagaaagactcccctcacaatagattgcggactgcacctgactaaagaagtgctgaatggcaaatggaagccagccatcctccgtgctatttcgatggatgtaaagcgtcccagcgagatactacgcttatttcctggcgccacccgcagggtgctgaatgtacaactcaaagaattggaaggacatggcatgatagagaagaaaacctacccgcaactaccgcctaaagtggagtattcgcttacggagatcggctgttcactgatgcctattattgatgccatgaaccaatggggtgatgctaatcgcagctttttggagaatgttattaagcaagcacctaagattagcgaaacatcaaaatcgacatgccagatttatagacatatgatggtagcgcgtaagatcggataaggtttggtagtgggattgctgcccatccagtctcaatccctcaaatcaaaaaagcctttaaatctttcgatttgaaggctttttccttgcggagagagagggattcgaaccctcgatacagtttaacccgtatgacggtttagcaaaccgttcctttcggccactcaggcatctctccattatttccctgaaggggttgcaaaaataggaaaagttttatattctccaaaagcaaattcggttttttacaaaaaaacttgccctaagtatataaaaatccgctgaaaggcggtccccatgcgggtgaacatgaaaaagccgtgcagttgtgcacggctttttaaaataggttctcagggctaaggccggctttacatggccgccagttgtactttctgttgcaattcaattacactgtcacggaagttattgtcagtatccatcaggtcctttacggtttgacagctgtggataacggtggtatgatcgcgtccaccaaaatgttcaccgattgttttcagggaatttttagtaaatgatttagcgagatacatggtgatttgcctggcctgcacaatttcacgtttacgtgttttttgcaacagcttatcataaggcacatcaaaatattcgcagaccattttctggatactctcgattgtaatttctttggaagatgtttttacaaaagatttcaatacgcgcttcgccagttccaggtcaatttccttacggttcagcgatgattgtgccagcagggaaatcagtgcgccttccagttcacgtacgtttgtctggatgttataggctacatacttcactacttctttcggcatttccagtccatcgttccgcatcttcatttccaggatttccatccgggtttcaaaatcggggatctggatatcagcgctcagtccccagcggaaacggctcagtaatctttcctgtacgccatccagatctttaggcgccttatcagacgttaggatcagctgcttgccggattggtgcaggtggttaaagatagcgaagaaggcgtcctgtgttttctctgcgcgggcaaagaactggatatcatctacgatcaacacatctatcaactggtaaaagtggataaagtcattgatgatattattcttggagtgatctataaactggttaatgaatttctctgcacttacatataacaccgctttgttcggatgtatacgttttacatcattgcctactgcctgtgcaagatgcgtttttcccaaacctactccaccatatattaccagcggattaaaagaggtgccaccgggcttttcggccactgttttacctgcacgtcttgccacacggttactgtctccttctacatacgcatcaaacgtataattgggattgagctgcgagtcaatctgtacccttttaatgcccggaataacaaagggattcttaaccgggttgtgaatcgttaaaggaaaatctacttcattgtctttctgaggtttggtaaactgcgtgggcatgtttactgttctgggatgctgatgtggcgtaccgttctctactacaatgcgatactccaaccgggcttctttacctaattctctcttgatggtttttcctaacaatcccacataatgctcctcaaggtattcataaaagaattggctggggacctggatggttaaaacattgttttcaagtttaatgggtttaataggttcaaaccatgtcttaaacggctgccattctactatatccctaattatattaagacacttttcccaaacttgttcgcaagttttattcattgagataaaaaaaattagttgtttcttaattaaggatgcttagttctcgaattcgaaattccccaacgcaggaagttgaaaaattttcagacaggacgacgaatatctgtagaaaatgttgaaaaaaaaaatttatctacccttgtttatattctcctgattacagagtaccaaaacccctttttccactactgctgtggctttacagcccagacgtgacaaggttttcattactataaaccccattgattaacagcacctttatcttttccattctcctttttatcataaatatggatatataattgataaaataatattgtatcctttctctcaaaaaaaaccgttcactgataagtcatgagatattcacactttttcgggagagggtgcaaaactatgttagtatctccatttaaaaaaatgtattaggggatagtaattgtgaaagtatttatttatatccacgcgcaccggattaataaaaaatatttgtccgcactaagccgaataccttatctttgacccttctgaatttaaaataatttttctatgagttttgaaattaccggaaagctgattgtgaagtacaacacggtacaacgtagcgaaacttttaagacaagagagttcgttattgagaagtccgacgacatcaatggccgtgttatcaacaactatataaagtttcagtcggtgcaagaccgcactggtattgtagaccggttcaatgaaggtgaaaacgttaaagtttatttcaatatcaaaggcaccagatgggagaaagatggtaaagtgaattacatcaccaacctggacgcatggcgtatggaatctgtaatggcagcacctgctccgggcgcagatcctcagcctaactacaatactccacagatgcctgcaggcggcggagatggcggcgacgacctgcctttctaagctgaaagcatcacacaaaagctattgaagcgaagatataagcggattacatccccttatgtcttcgctttactcattttatacattaccccgcatttgctatctttgccgcagttttaggataaacacctaaccgctaatatgatacaacaaatatctctcaaattactgccggccgatgccgcctctcatacaaatatcatacagcacgctgctgccgcactaagtgtaaagcctgccgagattacaggattcaatctgctgaaacgctctatagacgcacgttccaagcaggtattctttgtccttaccatacaggtattcattaacgaaccttttggagaaaggcaacacacccatccggtatatccatccctgccagccaatgcaccacgggtgctgattgcaggcgccggacccgcgggcctcttcgccgcattgcggctcatagaagcaggcgtaaaaccagttatactggaacgcggtaaagatgtacgcgcacgacgccgtgatctcgccgccctcaataaaacaggtatcgtaaaccccgactccaactactgcttcggcgaaggcggcgccggtacctactccgatggtaaactatacacccgctccaataaacgcggcgatattaaccgcatcctcaacatattcgtacacttcggtgcagaagataagattatgatcgatgcacacccgcacatcggcaccaacaaactcccgcatatcatcaccgctatgcgcgaacaaatcatcaacagcggcggagaagtacacttcgaacaaaaagtaaacgccatacaaatcagcaacggcgcagttacaggcgtgcaaaccgccaccgggcaaatatttgaaggcaaacaactcattctcgccacaggccactccgcccgcgatatatttatcatgctccaccagcaaaacattttgctggaagccaaaccctttgccctcggtgtgcgcgtggagcacccgcaggaactcatcgacaatgcacagtatcattgccaggtgcgtggcgaatatctcccgccagccagttacagcctggtagaacaggtggaaggccgcggcgtattctctttctgtatgtgccccggtggcataatcgcccccgcagctaccgatcccggcgaactggtagtgaatggctggtcgccttccaaacgaaacaaccccttcgctaattcaggcatggtggttaccgttgatgaatccgactttgcaccattcgtacatcacggcccgctcgcagcgatgtactttcaacaggcggttgaaaaacaggcgtatcatgccggtggcggcaatttcgtagcgcccgcacaacgtatgaccgactttgtcaataaaaaagtttcagcctcgttgcctgaatgctcgtatgtacctggcctcaacagcgtggacctgcgcagcgtattacccaaagtagtacaccagcgcctcgccggcgcctttaaagcctttggccgcaaaatgaaaggatactacaccgaaaatgctgtactggtggccacagagtcacgcacatcttcaccggtacgcattccccgcaacaatgatacgctggaacacccgcaggtggcaggtctttatccctgcgcggaaggcgccggatatgccggagggatcgtatccgctgcaatggatggcgaacgcgtggccgccatcattgccgcaaagttgtcgtaacgatattccgacttatttattggggattaatcactaatttttcaccatgaacctactcgaagtcaaacacctgaaaaaacattatgacacccacaaagcggtggatgatgttagctttgatatacagcagggcagcatctttggattactggggcctaacggcgccggtaaaacaaccctgctccgcatgattaccggtatcttctaccccgatgaaggccagatcattttcaacgggcaaaaattcaacccggaaaacgatgtgcagtacatcgggtatatgccggaagaaagaggtctctataaaaaaatgaaggtaggcgaacaaacactctatctcgcccagctcaaaggactctcccggaaagaagcggtacagaagatccaatactggtttgataaattcgatatcaactcctggtacaacaaacgggtcgatgaactcagtaaaggcatgcagcagaaagtgcagttcatctccactgttctgcatcagcccaggctgctgatcctcgatgaacccttctccggcctggaccctatcaactccaatctcattaaacaggaaattttcaacctcagtcagcaaggtaccaccatcattttttctacccaccgcatggaacaggtagaagaaatctgcgaccatatcatgctgatcaacaaaggccataaaatactggacggcagcgtaaaacaaatccagcaggattttaaacagggcctttttaaagtaggcctgggcacgatgcctaatcctgcacaaatggctacttatcactttaacattgtgcaaacacatgataaggcgtttaccgtaaaaatgaatgaagacagcagcaccaacgatatcctgctgcatttcatccgccaggacattcctgttacatattttgaagaaatccttccttctatcaacgaggtatttatcacccaggtacagcaaaccgaaaacagcaacgcccccgtagctgctttgccgctggcctgattaacctgctacttatggagaaaatctggctcattataaaaagggaattctttacccgcgtgcgtaaaaaatcattcctcatcaccactatactggtccccctggcctttgctgccatgatcattgtgcccatccttttatctacttcttccagcgaacataagctcattgcggtggtagacaaaagcgggttgtttgaaaacaagttccccgattccaaaggcgtatatttcaaatacgtgcaaaaccagcccatcgatagcctcaaactgcattacagtgatctcggctatgaaggagtgctgtatatccccgagtttgatatcaacaggccctccggctttgaattttacagcagcggccaggcaagcatcaccatagaaaacagtatcaacaaggatatcaacagcatcattgaaaagaagcgcatgcagctgcaggggattgaaccctctaaaatggatgaaatcaggtcggatgtggaagtaacctttaaaaatggtaaggacgaaaagaaaggcagctcctgggtgtcttatggagtaggctacgccagcgggttcattatctactttgtgctgttactgtttggtacctccgttatgcggggtgtgatggaagaaaaagtgagccgcattgcagaagtaatgatctccagcgtgaagccttttcagctgatgatgggaaaaattgtaggcatagccgccgtgggcctgctgcagttttttatatggggtatcttcattacagccatatactccctgataccgctgttcttttcacctgaaagtatgcaggcagctgccgcccagggcaacccggcgcaaacggctgaaatggtgcacagaatgcgggaagtgataggcagtatcaactggagcttactggtaccttgctttgtgttgtacttcctgggaggttatctcttttactctgccttgtatgccgccattggcagtttggtcaacgaagatgcctccgacgtgcagcagctcaccattcccgtaacagtgcctatcatcattggtatcatgattatgatgaaggcagtacaggaccctggtagtccgctcgcggtatggggcagtattattccattcacatcgcctatggtgatgatggcgcggctgccttatggcgttcccggcacagtaccttactggcagctgatattgtcgtttgtttgtcttattggtggctttttgggtactacctggttagccggcagaatataccgtacagggatcctgatgtatggaaagaaaattacgctgaaagaagcgatgaagtgggtagtaagaaaaccataaaaattttgtgagatggttaccggggcggttgctccggtaaccaatcaaatatcgaagctatttaaatggcggatggtttccctgaactccgtccatatttccgccaatacagctgccgcaggctttatatcatgtatcagtgcacttacctggcctatttccagttccccttcttcgaggttaccttcaaacatgcctgatttggcgcgggcgcgtcccagcaaggttttcagggcatctatatctgcgccgttatcctccgcctgccgcaccgcctggtaaaaattatttttgataaggcgcacgggcgccagcttctttaaacttaacatggtatcgccttctttggcatttaccaccgcctgtttaaaatttatatgggaagatgcttcgggggttgctacaaaacggctgcctacctgcacaccggatgcgcctaaggcaaatgctgctgccattgctttcccggagcctatgcccccggctgcaataaccggtatttttacctgttcgcatactgccgggatcaataccatggtggtggtttcttcgcggccgttatgcccgccggcctcaaatccttcggccactactgcatctacgcctgcggcctcgctttttaatgcaaaggctgcgctggataccacgtgcactaccttgatacctgcggctttcaataccggtgtccatgtttttggattcccggcagaagtgaacacaatttgtaccccttcttccaggataatatttatcagctggtcaatatccgggtataataacggcacattcactccgaaaggcttatcagttgcctgtttacacttttgaatgtgctcccgcaatacggcaggatacatacttcccgcgccgatgaggcccaggccgccggcattactaactgcgctggctaaacgccatccgctcgcccagatcatgccagcctggataacaggatattgaatattgaataaggaagtgatacggttgttcataagcgaatatactatagcttgatgctgccggtattatcccaggtctatttcggtattatcgcctatgttcaggctctggctcaatccgcggatattggcgtcgctgcctatcagggaagatttcaatactacttcatacaggttgctgaaagagccgataatagaatcctttacaatagagtagttgatcacagtattatcaccaatggccacattagggccaataatggcgtttttaatgttacagccttcccctatgcttaccggcgggatgatgatcgtattttcatatggtaatacgggattgctggccagtttatatttcttcaggagaatagcgtttgtttccagcagcgtatctttccggccgcaatcgaaccagttggatactttgaagccgttgaactgcacaccgtgctcaatcatacattccagggcatccgtgagctggaactcatcgtgcgactttatcctgttgtcgatattgctttggaggcagtcgtacagctgctccgtttccttgatcttgtaaagtcccaccagtgcgaggttcgacttagggatctgtggcttttccactacgcgggtaatctttccctgttcatccagttcggcaacaccgaagttacgcgggtcgtctactttcttcaggcccagcatcgagtaaggagaggcgatcacttctttaaagtcgcattcacagatggtatcgccaagtacaatcagtatttcatcattacccactacatcgcgggtaagggataaagcatgaccggtaccttcgcggctgttttgctgcacaaagtggcaggtaagctgcggatacttcttttctacgtaatgctggatcttttcaccaagatagcctaccacaaaaacaaattctgtgatacccgcatccaccaactgatcaataatgatactgagaatggttctgccggctaaaggtattaatgctttaggctgtgtatatgtatgtggacgaagcttggtgcctgcccctgccactggtattattgccttcatttagtgttgtagttaggattagctattgctgctcgaatgcggcgaaattaacataaaaagcggaaagcataaagcagaagcctttatgcttgcaattgatccggctttaatttatttttgcaccaaatttaaggcaacatgcaaagagaccagcaaatatttgatttaatcggccaggagttggagcgtcagcgccacggcattgagttgatcgcatctgaaaactttaccagcttacaggtaatgcaggcgatgggacatgtgatgacgaataaatacgccgaaggttatcctggcagaagatattatgcgggctgtgaaattgtggaccagagcgaacaactggcaattgacagggctaaagaaatatttggcgctgcttatgtgaacgtacaacctcactcaggggcacaggccaatgccgctgttatgctggctattctgcaaccgggcgataaaatcctcggactggatctgagcatgggaggccatcttacccacggttcttccgtaaactactccggaaagctctaccaacctcatttctacggtgttaacaaagaaacaggcctggtagaatatgataaaatggaagaaattgccaaccgcgaaaagcccaaactgattgtttgtggtgcttctgcttacagccgcgactgggattacaaacgtatccgcgaaatagctgaccaggtgggcgcttttgtactggctgatattgcgcacccggcaggtttgattgccaaaggcttactgaactctccgtttgctcattgccatttcgtaactaccactacccataaaaccctccgtggtccccgcggcggtatgatcatgatgggcgcagatttcgaaaatccgttcggtctgaaaacaccaaaaggcgaaacccgcctgatgagctctctcattgataccgctgtattccctggtatccagggcggtccgctggaacatgtaattgccgctaaagctgtttccttcttcgagatactgtctgacgagtacactgtatacgccaatcagatcctgaaaaatgcgcagtccatggctaaaagctttgtaggcaaaggatatgaaatcatttccggtggtaccgacaatcacctgatgctgattgacctccgcaataaaaatatctctggtaaaaaagcggaacaaacactggtaaaggccgatatcaccgtcaataaaaacatggtgcctttcgacgataaatctgcctttgttacttccggcatccgtattggcgttcccgctatcaccacccgtggtatgaacgaaagccatatggggcagatcgttgactggatcgatgccttgctgctggatgcagacaatgaagggctgatcctcaaggtaagaggcgaagtgaatacgtttatgcagcagttcccgctgtatcccgagttgtaggcggattttgtcttggctcaggattacgctgattatactgattagctggatttttacttttggattttataaaggattaagggagatagaagcggatatgtactgccccctaaaagttagacacttttagggggcatttttatggataaacgcagaaaatacagttttgagcaaaaattagccattgtgatggcagttgagaatgattatcaatccgttagt

SEQ ID NO: 20 - DNA, 54411 bp, Chitinophaga pinensis
  source 1..54411: mol_type = genomic DNA
ttcgagaatatatagaatattataataacgatagaatcaaattaaaactaaatggcttgagtccaatacaatatcgaactcaagccgcctaatcaaaaaagtctaaactttggggagcagtacatatactcgcttttatctcccttaattattattttaagaaaatctaaaaaatcaaaaaaaaatccaaaagtaaaaatccagctaatcagtataatcagcgtaatcctgagccaagacaaaatccgctatttccgcttcaggaacacgaagccgttcttctcaccaatcacctccaggttagggtggcgccggtaaggctcactatccgtaatacggcaaatgaagtaggcgggcttgtcgatccggccattcaggagccagtcttcgttgtaatagtttttattggaatgtggcaactctcttgaatagtaatgctgcgcataactgtggtatcccaacgcctttacatatacgtctttcccttgcagggaaatgaaatagtctatggcagcgcgctgtgaataggcttctatcttgggcacaaaatgtactactgttacctgtatcaccaatatggaactgataagcaaacacatcaatcctttgctgatcttccggcgtatcagtaatacactgcttataataacaagtataatataacccgcgccatatccggcttctgctaccgaccagggcacggctgcctgcaggttggctaccgcgaatttatcaccgatgtacgggatcagcatgtctttgtaaacacctaccagtggcaatactgcaattgccaatccgagcacaataccgatgaaaagtatcagggcaatattccagccacgcagccgctgctttccttcagagagcaggtatacctgccaggccgcaagaaaagacagtgggaaataacacagcgaagaataatgtacaatctttgtttttacaatagagaaaaggatcagtactacccagaataacacccacatccatactttgaaatccttcagttcaatggcggcaggagtggagtagatcgtttttttcctgctttgtaaataggtgaaaagaaacgtgctcgccggaaaacagcctatcagcaatacaatccagtgataatagaaagggccgccatgaccggcatcttccgtagtaagcaggcggatctggtaagccacaaattcattgacaaaccaccagccatgcgctgcaatctcatatccaaaccacaacagcgtggtaatacaggcaaacaaggcaattaaaccaaggtgggaaaaccggatactgatctttcctttattccagatccagtatatcaacaggcacaataaagctaccagtatggctactggtcctttggtcaatacagccagtccgaggaataagccactgagaatggccatacggaaaggtttatggttatacccgatgcgataggcaaagtaaatggaaaggaagatgaagaaattgaatgtaggatctatgatacctgacttaaaataaaaatgcggtaaccaggagcccgcatataccagcgcccaccagaaaccgaatctttcatccactgtttttttaccgatggcaaataaactgatcagtgtggcaatgccgatgatggcattaggaaaacgggcagcaaaatcatttaccccaaaaaggtgcatacttcccgcctgcatccatataaataagggtggtttttcccagaaaggacgaaaatcgatctgcacctggctgtagttgtggcttacaatcatttcgcgtgctgcttccgcaaagttgatttcatcccagtcgaataaatgtacggccccaagaaaaggtataaatagtaaagcggccaccagggcaatcaataggtatttcattgaaagtatttaaaaaattggattacgaacggtcagcttgtgaccgttcgtaatgatgccttgctatgtggtggcattggcctgtaaaagcgcctctgcacatacttccggcgacgacctggtgtcccggaaactgaaaagtccatacacgatgacagtacttaaagttcccacaatgctgccaacatatacatctataaagaaatgctgcgccaggtaaatgcgggaataaccggcgccaagcgccattattaataacagcaatcccagctttttattgcgcacaattacggccagaaaactgaacatgccaaaagccgctgcggagtgaccagaaggaaaactgcaactgctgtgcacattaacccatctgaccgtatgcaccagcgtagccgtttcatctccgaaataggagatggggcgtggtgcattataataatgtttggccatctgtactacgatggtgaccagcagcagcactgccagcccgataaagaatagcctgaaccgctgggttaccagcatcaggaacagcactattccaaacataattccgtcaccgaggtaggtaagcccggtaacaataacatcgccccagccggaatgttctctgttaatactgagaaacaggtcccgttggctgtaagtggctaacatcactccgcccactattagccatagcaggaagggcagaaagaaccaggagttctttctgaacagtgtaaacagcgttttcaagtctgtaggttttaaattgtaggttgctttaaatctctttaagaacttctttctttctaaatctttgtaagaacttttttatttgttgaataacgcgaaaatagtactctttattaaaaagctgtgagtcattcatagccttaacaataaggaaacctgcaatggggagtaacaccatatttgacagccacatgcccgaccaggtgaacatcacgccatttctcgccatcttttcacctatcatgaaaaatacgttaaaaatcacaaagaagatcacggcaaacaccagtggtgtgcccaatcctccttttctgataatggaccccagcggggcgcctatcaggaacatcacgatacaggcagcagcaagcgtgaatttacgctgccattctactttgtgcatcaggattacaccatgcttgtcttcaaactcctgggtaggctgttcgagggcgctctgcgtttcacggacattctgctctgctctttccaatacggtacggaggctcttctccggtataatatcttcaaattcttttgctttcaacggcggggcgctggcagcccaggcggaatccttccatttgaagaaagggtaacgtacagtaacatacgaatttacggtcttactgtactggttctctattttctgcagggaatctatcgctacatccagttgccttacgttcagcatttgctggttggaggcaaaaagatccatgttgaggcggttaaaagcaaatgaactcaggtcaaatgctttgctgtattttttaaagcccagcctgatcatgtcgccgggaaccgtgtatccgcggttgttccgctcttcataacgccagccattgtccaggatgaaatacaggaaacgcttgttggccgtaagtaccatctgtcctttttccgcgaggatgatgcggtcgccgccaccactctggtggtcgaagatcatcacctggtggatggtttggttgtctttatccttttgggctaccttaatggtatagccgggaatatctttataaaatacgcctgccttgatattaaaggctggcttggagttggtaatgtcgtagagcagtgatttggcctggaggttggcaaccgggatcacatagttggcaaacaaaaaggccaggaaagcgattacggagcacaccagcagcagcgggcggataaagcgcaacagggaaatgccggaagattttaacgctaccagctcgaagctttctcccaggttaccaaaggtcataatggaagacagcaacactgcaaggggaagggccagggttaccagcgtggcgctggtataggcaatgagttgtatgatcacacccgtatccaggcctttacctaccaggtcgtccacgtatttccagaggaactgcattaccagtacgaataaggtaacaaagaaggtagctacaaagggacccaaaaaggtttttataattagtttgtcgagttttttcactgataatgcggtattaaaaagatggaatcccgatcttcgtattctactggccaggatactcctaaacggtaaagttagcacgaattcacaaaggagtgttagggagaacctgaaaataccgttaaaatttatatggaaagttttgaattaacaccggaagaagcagccgttatagaaagcacgcactttattcttctgaaaaacagtgcaatagggaaggtaatggtgttgatggggaagctgcaggaagcgctggcagcgtacgaccgtaacagtagtttcccgtttaagcctgagtggctgctgcagggcggtaaaatttcaaagggggagcagtacaaggggctgccctgggtaatgctggactacccgcgttatttcagtaaaacggaagtttttgcgtttcgcaccatgttctggtgggggcattattttagcgctaccctgcacctggcaggtaacgtgaagcgctattacagtcctgttcttgaaagcagttacacaaaactggcggaagccggatttcaggtatatgttcaggaagatccctgggagcatgatttcgaaaacggaaattactgtttcataaacaccttaagtttagatgagtggaagacgctgattagccggaacgatttcatcaaagtggctaaacctttcgtgatcggtcattggggcaaaataattactgatgtagtggaggcctatgctgcgctactcaatatacttgaaaataaaggggcttaactgccgatgcggtggaagagatctttcacctggtattcccatagttgactttggtccttcacttctttcttctctgcgaaatcttttactaccaggatagtttcattcgttacttcagaaatttgtatgcggaactcaaaatattcctctttgggagcatgcgtccagtgcagccggatgtactcatcctcttcctgttccagtacttccgcttcttcagcagtaccgttccatgaaaaggaaaaaacattatccctgaaatcaaccctatcggcgaaccattcctgcaaaccggcaggggtcgataagaattcatacaggataccgggtgagcaccttaccggaaattctaactcataaagcactttcttagacatctctcaaataattagtaaatcaatatcatccagttgcaattatagaaaatattttactctgtcaaaataatttacggtttttttttatagaatacataaaaactttacacgtcttaataaaactatatatattacatttataataaatataaaacagccacatatgatagcgctgtctgcttcgcctctatagtggcgaatttccgcgacatttgcaagcccttaatgatcaatcgattttatttggaaatgatttaaaaacaatagattttttttggtggctatctaaaaaaagttatttttgtcaggcattcatcaaatcttaactttttattaacctgtaactgttccgactctatgtcaatgcgccaacttaaaatcactaaatccattaccaacagggaatcacaatccctggagaagtatctgcaggagattgggaaagtggatttaattacgccggaagaagaggtaaacctggctatccggatcaagcagggcgatcagagagcgttggagaagcttacaaaagcaaacctccgctttgtggtatccgttgcgaaacagtaccagaaccagggactgtcgctcagtgacctgatcaacgaggggaacctcgggttaattaaagctgctcaacgttttgatgaaacgcgcggttttaaattcatttcctacgccgtttggtggatccgtcagtctatcctgcaggctttggcagaacaatccaggattgttcgcctcccgcttaacaaagtgggcctgagcaacaagatcagcaaagcgtactcccagctggaacaggaatatgaaagagaaccatctcccgatgaactggctaccatcctcgaaatcaatacggaagaagtggaagcaaccctcggtgttgctgcccgccacgtatctatggacgcgccttttatcgacggggaagataactccctgctggatgtactcgaaaacccgaatgccgttagcgcagacgaagaactggatcaccacgattccctccgccgcgaaatcgagcgctcactctctactttaacagaccgtcagaaagatgtgatcatgctgtacttcggcatcgccgttgaacatcccatgtcactcgaagatattggcgaaaaatttggcctgacccgcgaacgcgtacgccagatcaaagacaaagccatcaccaaattaagaactacctccaggagcaagttgctgcgcaactacctcggataacgcggatgttgtcttactcaggattacgctgattaggctgattaccttgagtttttagttgattttgtaaagatttttaaagattagcgaagatggctgcggtaaatccgcaacggtcttcgctaatcttttttaatcccaaatgatcaaatccgggtaatcagcctaatcagtgtaatcctgagtaagacaaactccgcgtaagacaaaatccgcgagaatccgcaaaaaaatatacttttgcagtccgtttaaaataccaacaatgtttgaatcattatcagagagactagactccgcgtttaaacagcttaaaggggaaggccggatttcagaaataaatatcgcctctaccgttaaagagatccgtcgtgcattggtggatgcggatgtgaactataaaattgccaaggaatttacagataaagtaaaggataaagcgctgggagaaaaggtattaacagctatttcgcccggacagctcatggtgaagatcgtaaaggacgaactggccgaacttatgggcggcaccgaagcagaattcgacctcaaatccaatcctaccgttgtactgatcgcaggtttgcagggttcgggtaaaaccaccttctccggtaaactgggcaacttcctgaaaacaaagagaaataagaaacccttgctggtagcagccgatatctaccgccctgcagcgatagcccagctgaaagtactgggcgagcagataggggtggaggtttacagcgaaccggaaaataagaatgccgttcagatcgctgaaaacgccatcaaacacgcgaaagccaataacttcaacgttatcatcatcgatactgccggccgtttggcggtggacgaagtgatgatgaacgaagtagccgccgtaaaagctgcggtgaaaccacaggaaatcctgttcgtggtggattccatgaccggccaggatgcggtaaataccgccaaagcgttcaacgaacgcctcgactttaccggcgtagtgctcaccaaactggatggcgatacccgcggtggtgcggcactgaccatcaaatacacggtggaaaagcctattaagttcgtaagtatgggtgaaaaactcgataccctcgatgttttctaccccgaacgtatggcccagcgtatcctcggaatgggggatatcaccaccctggtagaacgcgcccaggaacagttcaacgaagaacaggccaaaaagctggaaaagaaaatccgccagaaccagttcgatttcgacgatttcaaggaacaactccagcagatcaaaaaaatgggtaacctgaaagatctgatgggcatgatccccggcgtcgggaaggcagtgaaggacctggacatcagcgatgacgcttttaagggcattgaggccatgatcaactctatgacgaaggcggagcgtgccgacccggatatgatcgacggaagccgccgcaaacgcatcgcaaaaggcgccggaaaaaacatccaggacgtcaaccagttcatgaaacagtttgaacagatgcgccagatgatgaaaatgatgaataaatttggcggtggtggtaagggtttgaaaggaatggtgagataaacggatcagattgatataaatattttttgcaaataccaacttactgattacatttgcatccctaattaaacaatatttcctaactcgcaaaaaataactcgacttatttatgccagtaaaaatcagactgcagagacatggcgcgaaaaaaaggcctttctattttatcgtagtagccgacgcccgcgcaccaagagatggtaaattcatccagaaaattggtacttacaatcctttaacagttccggcttccatcaacatcgataccgaaaaggcattgcgttggttgcagaaaggtgcacaacctaccgacactgttagaagaatcttgtcattcaaaggtgtattgtatttgaaacacctgttaagaggtgttactttgaacctgttcgacgagcctactgcttaccagaagttcgcacaatggcaagctgaacacgaacagaaagtttctgcccgccgcgacggtcacaagaaagcaaggattgctgctccaatcgtaagaaaggtagaagacactccggctgctccagcgactgaagcaccagcagcagaagaaggtaacgaagcataaaacggcaacgttttaacaatacctgaaaaaggaaatatttgcaactgcaaatgtttccttttttaatttttgttaatagcctcatcagcaatcagttacctgatccgctaaagtccgacagcaaaaaattatgagtaattatttcagtataggtaaactggcctccgcgcacggtttgcagggcgacctggttttaaggcacagcctcggcaaaagatccgcgctgaaaggtgtaaccgttatattcctggaagagcggaaaaacagcttcattccctactttatacagcaggtaaccgtaaaggatacagaaagcgtatacatcaagctggaaggtatagataccaaggaagccgcacacaaactgatgcccgctcaggtatacctgcaggaagaagacttcaaacaacaaaccgcttcctctgcacccctcgctttgctgggatttgctgtggaagaccagcaatatggccccttgggcactattgaggaagtcattgaaatgcctatgcaggtactcgtaaaagtattcatcaagggcaaagaagccctgctgccggtcaatgagcagtcgctggtgaaagtagacaagaagaaccagacggtacacctcaacctcccggatggtttgattgaattatacaccggttgatctgacggattcaactgttataaagggcacacaatcatgcgaatagatataatcaccgtattaccggaattgctcgaaagcccgctgtcacactctatcatgaagagggcacaggcaaaaggcttactggaagtacacgtacacccgctcaggcagtactccaacctgaaacacaaccaggtagacgactaccagtttggtggtggcgcaggaatggtaatgatgctggagcctattgtgaatgcgattgagtcgctccaggcaaaagtgcagtacgatgaggtgatctatctcacccccgatggcgaaacgctgaaccagaaaatggccaaccagctgtcgctcaaaggcaatctgctcctgctttgcgggcactataaaggtatcgatcagcgcatccgcgatcactttatcaccaaagagatctccatcggcgattacgtgctgagcgggggagagttgggcgccgccgtactggtggatgccatcggacgcctcctgcccggcgtgctgaataatgaaaccagcgcccttacagactccttccaggacaatttactggcgccgccggtatacacccgcccggaagagttccgtggatggaaggtgccggaaatcctcctgagcggagatcacaaaaagatcgacgaatggagacaccaggaatcagtagaaagaacaaaacaacgcaggcccgacctgttataacgtaatgatacataggtcatatagagcgctttaccatttgacagggataatttcttgatttttaatttggtaaatgctatttcttgacttacttttgcactcccataaatatttgaaagatgaacgcaatttcgtttgttcacgaacaactgacagctaacaaacagtacccgaagtttaaagcaggcgacaacgtcactgtcaactataaaatcgtggaaggtaataaagaaaggattcagtcctttaaaggtgatgtgttgaaaatccagggtacgggatcaacaatgtctttcactgttagaaaaatttctgatggcattggtgtggaaagactgtttccgctttactctcctcatatcgatggtatcgtgttgaacaaggtaggtaaagtaagaagagctaagctttactatctgcgcgaacgtgctggtaagaaagcccgtatcaaagaaaaaagggtttagtataaatacagggaaatttgttaaaagcgggaccattaccggtgccgcttttttcgtgtgcttaaaatggtattaaaactagcgcaggattgcccataacggtaaaaaagccgattatatctgctatctttgttgactgaacttttaaacattgagaagatgactgctgtttttttaaattcatcatttttgatccttcaggacattggaatgtccgagctgctgttgattgccgtggtagtattgctgctcttcggaggtaaaaaaattcccgaattaatgcgtggcctcggtaaaggtatccgcgagtttaatgacgcaaagaacaatgtgcgccaggaaatcgaagaaggaatgagggaaaagcccgttcaggctgcagcaccggccactacagatgcaccacataccagcactgaagaagctccactgcccaaagtataaattgtagccaactccctaaaggagtatttttctgttaatttaatttaactggtttagtcttgtctgaattcagcagtataatcactttccataaagcattatacgccggcagcacaagctgtgcggagagggtgcgttattacctcgaccgtatagctcagttaaaacacttgaatgccttcctggaagtatatgaagaggaagccctggagaaagcgcgcgagcttgatacccgcctcaaaaacggggaaaaattgggcgcactcgcgggtgtggtagtaggtattaaagatgtgatctgctataaaggccataatgtaagcgccgcttcccggatactggaagggttcaattccctgttctctgccaccgccatcgaaagattgctggcagaagatgctattatcatcggtaatctcaactgcgatgaattcgcaatggggtctaccaatgaaaattctgcctatggccccacgctgaatgccctggataatacccgcgtaccaggcggctcctccgggggctctgccgtagcagtccaggcagacttatgccaggtaagtctcggtagtgataccggcggctctgtccggcaaccggccgacttctgcggcatagttggcctgaaacccacctatggacgtatttcgcgctacggactcatcgcttacgcctcttcatttgaccaaataggcatttttggcaagaatattgccgatgtggcgtcagttctacaggtgattgcgggtccggatgagtttgatagtactgcttcccaaaaagaagtaccggattataaagcagacctggaaaacaataaaacattcaaatttgcgtatttaagggatgcacagtaccacgatgggctggacgcagaaatgaagaacggctatattgatttctttgaaagtttgcagtctttgggtcatacggtatcaggaaaaagttttgaatacctcgaccatgtagttccggcatattatgtactgactacagcggaagcatcctccaacttatcccggtttgatggggtgaaatatggacacagaaccgctgaaaagaacctggatctgacagaattttacaaaaaaagtagatccgaagggttcggaaaagaggtaaaacgtcgtatattactggggacttttgtcttgagtgcgggctattatgacgcatattatactaaggcacaacaggttaggcgtcttgtaacagaaaaactcaacgatatattagaagaatacgacgccattttaatgccaactgtgccatccacagcatttaaattaggggagaagactgatgaccctatagctatgtacctggctgatatttatacggtactggcaaatctggcaggggttccggctatatccgttcctttgtaccggcattcaaacggaatgccatatggtgtacagatcatcacaaagaagtttagcgaagcaaacttgttacatatagcgcatcaattgatggctaaggagcaggttactgttgtttaaaataaattgtatgagaaaaatctttttactactgctgttgccagcaataagtttagtgagtgtgagtgcaatggggggcaatagcaatcctaaagagatggcgtatccggtattttcacccgatacctctgtagtaaagctgaatcacaaggtacgtttaccaaaagatactgctttattgccatcgccaacatccgtggcagtgaagaaagctgcacagagcctgcctaacaccattcgcagtgcgaaagtgtatgaacagatcaacaataacctggttgccggttatgtaagtaactatgccacccggtatagtcagcatctgcaaatcatgatcgataaaggacaaccctatttcaatatgattgaaaaggtgttccgcgataatggtatccctgaggaaatgaaatacctcgcagtaatcgaatccagctttaataccaatgcccgttccagggtaggagcagtaggggcctggcagtttatggccggaaccgcccgtatctttggtttgagcgtaggtaagaaaatagacgaaagaaaagatttctataaatctaccctggccgctgcccagttccttaatcagctgtatgcacagttcgacgactggttactggtagttgccgcttacaactgcggcgcaggtggcgttcaacgcgctatcaaagccagcggacgtaccgatttctggggcatgcaatacttcctgcctgcagaatcacgtaaccatgtttacaaattcatcgctaccggttatatcctcgataagttcaataacttcttcggtgtaagtgaagataacaccatcactgtaaatgtgcctgtagcggataacctgtctgctcccgttgcgagaggcccgttaacagaagaggagatcttcaatacggtggaaatcaatgtaaccggcaaataccgcctggaagcaattgcaaagaaactggatatgaacgtggccgaattggaccgcttcaacccgggcttctccaaagcaatggccagcgccgaaaataactacgacctgcgcatccctaaagaaaagatgaagcagttcatggcagaaaaaaatgaaatgctgaaagaatctgttcagatgaccctggacgataaagcagtaggtgtagataaatccaaattcccgccgccggtgaaaatggcagaaaagaataccaccgctaaaaaagcacctgctaccagcagcaaaaaacattattcttccaaaaagcatcattataccgctaaaaagaagactactgctaaaaagaaaactaccacaaagaaataatcacccgcaagggtatacgaaataaaaaagagaccggtgatcatcactggtctcttttttttattatcaataatctcatatcagatagtaagcaggcctttacgtttttcactaaaggctaccaggtccagtaacggtccggtcataaaggtggtggccagcgccatcagcaccatcatggcaaatatctccggcgataagatccccaggtcaaacccgatattcaataccaccagctccatcaatccccgggtattcattaatgcgccaatagaaaccgactgccgccagctttgacccattaaacgcgctgtaatggtactgcccccaaattttcccgctacagccaccagcatgatcatcccaaatactacccagagatcaccctggttcaataaaccaatatgcgttcttaacccggtatacacaaagaagataggaagcagtagtaatacgctcacatcttccagcttatctgtcaatagctgcctgatattggtgccatgcggcatgatcacacccgccaggaacgcgccaaacaaggcatgtatcccaatcacttctgccacccatgcagatatcagcagcataaaaaatatcagggatactgctgctttctgatggcctttcgccatttgtgcctgcatggttctgttcagccaggggcggacgagcagtaacatcacggctacaaatgcaattgccagtaaaatggtcacgagggcgctcactatcccgccagcgttcacaatggccaccactaccgccaggatacaccaggcggtaatatcatctgcggcagcgcaggtaatggccatgatgcccaggggcgtgttggttagtttccgttcctgtacaatccgcgccagcaccgggaaagcggtaatgctcatggcgatgcccataaacagcgcgaaagataaaaagctgacattggcaggagcaaactgtgtaaaaaggaaatatgccagccaaacgccaaggaaaaaaggaataataatactggcatgactgatcatcaccgcgtcatgcgctttattcctgattttactgatatccagctccatcccaacaataaacataaagaaggcaagtcctatctggctgaggaactggaggtttttcaacgaatctgccggaaataaaaagccggaaaatgaaggcgccacccaacccagcagggaaggacccagcaacacacccgcgatgatttcacctaccactgccggttgcttcagtttattggcgatcagtccgaatacccgcgctgccagcatgatcaggatgatttgcaacagcaacagtcccagcgggtgtttcagattttccaggtagcgccaccagccgccggtggccatagccgccgctgccggtgcaggagtgataaccgtgtgcgcattcaccggtaaagattgtcccttctgaaggattacccatatcagcgccgcaaaaatgccaataatcacggggtaccagagaaagcgtttagtcatgacaggaaattattaatggttagctgcaagatataaaaaagcaaaaagctattacggggatagaccgctgcagcaagttaaatcttcgcatacggttatcgctgtaatagctttttgtggatataattagccggcagtttagctgatagcggcaattcccggcagttcttttccttcaaagaactccagtaatgcgccaccaccggtggaaacataacttactttatctgcaatcccaaactggtttactgcagcaacagagtcaccgccgcccaccagggagaaagctcctttggcagtagccgttacaatggcttcggccacgcctttggtaccagcctggaaagcagccatttcaaatacgcccattggtccattccataaaatagtattggaggcagcaatggtttcgctgaaaagggctacagacttaggacctatgtcgaggcccatccatcccgcaggaatattatcgttggaaacttcctgggtatttgcatctgctgcaaacttatccgctgcaatggaatctaccggcagtaacagttgtacgcccttttcctttgctttggctaccagttcattcgccaggtccagtttatcattttcgcagagggagctgccaatttctttgccctgggctttcaggaaagtgtaggccataccgccgccaatgatcaggttgttggcacggtccatcagggtttcgatgatcaggattttatcgctcactttagcgccgcccaggattgcagtaaagggagatgctgcgtcgttgagtactttttgtgcgctgtttacttctgcttccatcagcaaaccgaacatacggttctctggtgcaaagtattgtgcaatcactgccgtggacgcatgtgcacggtgagcggtaccaaatgcgtcgtttacgtatacgtcgcccagtttagagagctgttcagcgaatgcggcatcacctttttcttcggctttgtggaaacgcaggttttccagcagcagtacttcgcccatttgcaggtcggctgccgctttttctgccacaggacctacgcagtcttccgcgaatttcacggttgcgccaccaagtaaggaaatgaggtggtataccaggtgtttcaaagagtatttatcagtaggaccatcttttgggcgacccaggtgagacatcaggataacggcgccgccatctttcaggattttctggatggtaggaactgctgcgcgcatacggttgtcatccgtgatctcgaatttatcattcaggggcacgttgaagtccacgcggatcaaggctttgcggccgttgaagttatagtcagaaaatttgctcataatgtatcaatttaagataacgagaaggggtaaattaaaaaaccgcggtaccaacagcgcaaagcgagtatataaccaggtaatgctggccaattgctgctatggtgtagttccgcggaatttaaaggctcccggtttgcaccgggagtacctgttataattattatttgctgatcaaaccggcgaagtacttcacagtacgcaccagctgagatacatagctcatttcgttatcgtaccaggaaacggttttaaccatctggtgctcacctacagtcagtactctggtttgtgtagcatcaaacagggaaccgaagtggataccgatgatgtcagagctcacaatttcatcttcggtataaccgaaagattcgttggaagcagctttcatagcagcgttaacttcgtcaaccgttacttttttattgaggatggtagtcagctcagttaaagaaccggtgatggtaggaacgcgttgtgcactaccgtccagtttgcctttcagttccggtaataccaggccgatagcttttgcagcaccggtactgttaggtacgatgttggccgcagcagcacgggcacggcgcaggtcacctttcggatgcggcgcatccagggtgttctggtcgttggtgtaagcgtgaacggtggtcattaaaccggtagcaataccgtagctgtcctgcagtactttcgccataggagcgagacagttggtggtgcaggatgcgcaggaaataactgtttcgctgccgtccaggatttcgtggtttacgttgaaaacaatcgttttcagatcacctgtagcaggagcagaaataacaacacgtttagcgccggcagtaaggtgagcggccgctttatccctgtcagcaaagaaaccggtacattcgatcactacatcgatgttatgttctttccagggaatttgagacggatctctctgtgcatatatcttcacatcttcaccgttcacattgattgcgctttcagaatgcttaacgtctgcatcgaatctaccctgtgctgaatcgtatttcagcaaatgcgccagcacgttggggctggtgaggtcattgatagctaccacatcaatgccgggcattttgtaaatctggcggtataccaaacggccgatacgaccgaaaccattaataccaattttgagagtagttcccattttacatcgtgatttgagtatgaaaaaatcgagagcgaatttacaatcaatacccttattaatcaatataattttaggttatgaaaatattttttggaaatttagaataacatcctacatttgcaatccgaaaatgatgcgccgcgttggtcaaggggttaagacgcctccctttcacggaggagtcacgggttcgattcccgtacgtggtacaaataaaaagggttcttccaaacagaagaacccttttttatttacgctttctcactcttaaaaaagcttacgcctggttgaatccgtcagcccatctttgtgaagcagcacggagattcctttcattttcatataaggaacgctcaggtaaatgaatccctgtctccctgcttcaggtccccacgaattttttgctttataatagatattgccgtactggtctttcagcttgccggtaatatgcacaaggtggtcgtctgtagtgctgaaatcctcaaaggaagattgccgcatttcctgggtcactttcttttccggccgggcttccgtaagtatcagctccttatcttcctgcttttcaggtaatacagctaattctgcagtaaacgtcggctcggtcccgtccaggtcgagggcgagggaaaaccctgcttcgatcgcgtgatctatgttttccataaattcatcgaggggcaggttgtaaaaccgttcattggcccagttcgccgggatactcagcacaaagggtttatagaaaggaacatgcgtaaaagatgtaatggtgaggtaattacccgggtttaactgcgtataggcaagaaagctcatagaggtgtatgtctttccttcatacgggaattcatccggcgcctttcctaaaaaactatccagtttggcaggtacttcctttttccatccggtgcccagcttattggcagggtcagcatatttttttacggtgctttccagctctttaaacatcacggaatggttatgttccgtatgtccgtttagcagaccggtatataccgtttgcggtaataccccgaattcaactgagctgatgatgggatcatgattaaggccgccttcagtaaagcgcgcagtgccttgccgtaggatataattcctggctttcagtaaataggcgcatctcacaaaatacatttccgaaagatcaattttttctcctttcaaccggatgatctcggactccaggaaggaagtggtggaaaaactccaacaggtacccgaggcgttctggctgataaccggtaatgcaggaacctccgttaaaacagagaaaacgtagctgctttttcgctgcggcaacgtagcagccttttcaggtttactgttacaggcctggatagcgggcagcaaaagcaggaataataaagcaagtagcagatcttttttcataacggggcttaccatgtttcttttctctttttcagataataataatacccggcgaaacctaacgacaagctgaaggccagcatgcctgctgaaagccatccggatggaaagctgttcactactgcgcaaccgataccggcactcagtaacaggaaaaaatatttcgctgcatagtctttactttccacaccaatccgcagcatcttttctacttcagtgacatcaatcccccggctgatcatcttgcttttaagacgataattaagcagcatccggatcagcgttagcaaaaaaaccgttactacatagaacagcaggatgatgatgacggtacggataattacatcgggaacataggtgccattggcaagcgtgaaaccgccatcagcacttccggaagccgtgtgcgcatttaaaaaacggactaaaattattttcctcatctgcgtaaattgtttagtagtgatgaagccggcatgcccctgatgcgttatttatcattagaccttcataccggttttcaggttgcagttttactcaagatttaatgtcctgatctttttccggtaagtgttatatagttccataaactgcatgatcaatacgccggatagcagcaacaatcccggtacaaggcccaccgcagcgatgcccgaaaagatccagctgatcgtactccaacacgctattaaccctgcggccaccaggccgatggcgccaaacagcaagccatatagatacaaggcctcttttctgtcgggcgcactagctgcagacaacagatcaggaatgagatgcgctgtttcgaaatccggtaagggaacttcgctttctttgatatggctatacagcatttggtaagtcctgatctgcatttgacagtggaggcaatccgcaatgtgtctggcagccgccgggtccgcgaactcttcaagtgcatagcgctggagctgttcttcacttaaatgtatcttgctcataaatgctcttttgagtaataatcaagtaatcgttccttcaatacttttcttgcgcggaacaaatagtttttaactgttccggcaggaagtcctgtgatgttcatgatctcatcaatactgagctcttctttatgaaataaagtaataagtgtacggtagacaggtggtaacgcagcactaagcttttccaggatctctgctctttctttcagggaaagtagctggctggcatctaatgtatccttgttgatttcctgccaggcgctttcgcgtaaaagcaatttatcatcatcaggaatgtcggtcagctccggcctgtatttttgcaaatggtctaaacaggtggtgtagctgatttgcgcaacccaggtagacagccgggattgaaaacggaatttcggaagatacctgaataccttgagatagatatcctgcattatgtcttttctgtccgacgggttactgatcatcttaaagataatatttgctaccagtttttcggtgctgcggagcaatagggtagccgcatgagggtcgccctccatgattttttttatcatgtcttcatccgaaagaataggagggcgccctgggtacatcgtatatatcagacgtcataaacaaaaaaaggttgcaggaagcagttgtttctaatgccgggtttctcagatttcttccaagtgtttaacaaagatcttacccgttcagtcattttatatgctacgaaatatctgttggatattattttaagagaatggataatgccaggcgaacttccttgcggcaggtaagatgctcttatttttaggtatctttagagatcaagttgtctgctatgaaaaaaaagaaagtcgcttccctgttggtgagtatgcatccgttacaacgggtgctggtaagtttgggattcacgctcctggtgtttattgcgtttttattactgaagataacaatgcatccgttggtgctgactgcattgttatggaatatcttcgccatttcctatatcaccaccgggtggattgtttttttcaaccgtaccattgaagagatccgcacctgggcgaggatagatgatggcagccgcactttcgttacattaacagtggtagtagcatctgtagcgagcctggtactggtgttgttaatgatgttgtcaaaagagctgaccggtctttcaaagatcctgtatctcccggtggccgtttccggcatgctggcttcatggacaatggtacatactacgctcacttttcattatacccatttgtattacgacgatgcagaagatgacaataccaaacaggcagaaggactggagtttcccaaagaaaaaaaaccggactatatcgacttcgcttatttcgctttcgtgatcggtatgaccttccaggtttccgatgtggaaatcaccggcagagtgatccggcgcacggcattggcgcatggtttattgtcctttttgctgaacacgtttgtagtagcattaacgataaatttaattgcaggattgaaacaataagtcggcctggctaccgtgttttcttcataatcttcttacctttgataaagaatcgaaaaaaagttttggtttgtaaaacattttcctatctttgcaatcccaaacgaaaatgccgcgttggtcaaggggttaagacgcctccctttcacggaggaatcacgggttcgaatcccgtacgtggtacaaaaaagaaggacttctgcaaagaagtccttcttttatttcagacattttatgctcattcccccgcgaaagttttgctacaaagttgcctcctgcaacaaattcacaacaacatttagtacatttattccaacagcactcctttccctgaaactgaaatgattaatggtcctataaaggcacacgaccaacgatggcaaactgtagtcaggtatagcttttacctgctgtggatgatattgtccctcaccaacgccaatgcccagaaacggggaaatgctacctacaacttcacccacctcgatatcagcaacggcctggccagcaaccacgtttccgcagtaatgcaggaccggaaagggtttatttggattgccagcaccgcattacaacgttacgacggcactaacctggtaacagtggccagtttcgacagggtacccggctctatctattacgacgacatttgcctttgtgaagataaaaaaggccgcatctggatgggaacacccgataacatccgggtatatgaccccgccaccgaccaggtaagagccctcctggtagccggcagggacgtccggccggaaggactgcaatgcagccagatcctggaagatcatgatggcgtaatatgggccaccacgcacgacggactgctacgcttcgatgaaaagttatttcactttcagaaagcgtccatcatccctgaagaagaccgcatccagatgatggatgccatcatggaagacgaaagcggtaacctctggatcagcggaaaacacggtgtatatatccttgaccgccaacggaaaaatttatacaatgccgccaataacccgcagcaactgccggtactcaacatcgataataccttcaagaaaatatttaccgatccctatcaccaggtatggctggccggcagacacggacttttgtataactacgatcctgcttcccgccaactctcgcattataccttcgatgcgccggaaggcaaaaaatataatgaagcctatgatgccatcttcgacctggtaaccgacagcgataaaaacctctggatagccaccgaaaaaggcggcatattccgctataaccgcgaactgaaacgctttgatctgaacatcgccgccgacaatgcagacgaaaaaggatttcattatacctacgaagcgaattgctttctcagcgaccgcgaaggccacctctggatcggtaccgacctgggaataaatatccttagcctgcacaacaaaacattccgtatcctcgacaacagaaccactttcgccaacacccaacaacacctgccggcaacggaagtaaccggcgttttccaggcttccaacggcgatgtgtacataggatactggggaaaaggcttcagtcgcttaaatgccaacctggaactgatcagcaactatgtacacgacaatggcgaccccgcatacacactcccggaggaacgcggactggtatggactttcgcagaactgaaagacgggaccatcctcgtcggacaggaaaatgcatttgtctcgctgtttaatcccgccaccgggaaattcataaaacacctcacgtcgcccgtactctacgaacaaacaatactcaacctgaaaccacaacacgataccaccgtttggataggactatacaaacgcggactcgccagctggaacccccaacaaaatacttttcaacactatcatgaaataacagattccctgaaaagacccgtttctgtaatggatatcgttccggatggagattccctcctgtggctcggctccagcagtgcaggtcttatacagtttaatacccgctcacgccgcattacccaccggcaaacatttgaactggatgcaaaagtatacagcaatattacctccctccgccgttttaacgataccacattactggccggcaccgatcacggactctgggtttataacacgctgcgccatacttataaaccgctcctcattaacactaagctgtttgatcagtgggtactgagcatggaagaagatgggccaggcaaaatatggtttaccacccaatacggattttatcgctatcatgtggcagacaaccgggtggaaaccttcatcgagggtgatgatatcatcgataacacccgcaaagtaagacgccgcatcgtaaaactggatgatggcaacctgctcgtaggcgcttctgatcatattgttaccttcgaccccaccagcctgcgcgtagcgccgccaccaccggatgttactattgtaaaccttaaagcactcgacagtattgtactgatccatgccgcactgcaggacagcgtgccggttacactcagctataaacaaaactttatcagcatagagtttaaaagcctgcaataccaccaagaaaagatccggtattactatcagctggaaggcgtagatgaaaactgggtgcttactgacaatttattggtagcaaaatataccaacctgcctcccggtaattataccttccgcgtgcgtgccgtaaataccgcgggcaccttctctgaacatatcactgcattacagatctttattaaacccgccttctggcaaacctcctggttccggctattatgcctgctgctggcagcttcactggtatacctctactaccgccttcgcattgcaggtattaaaagagaagcaaaacaacgcgaagctattcaacaacaaattgcccagctggaaatgaaagcgctgcgcgcccagatgaacccgcactttatttttaatgcgctgaactctatccaaacctttatgatgaaaagcgaaacagaacaggccctggcctacctgagccgcttcgcaaaactaatccgcaacgtactcgataattcacaactcaataataccaccgtagcccaggaaatcagtgtgctggaaaattatatggaattggagaaactccgcttcagcgacgagtttgaatacgaaatcatcgtcgaccccactctcgacgccaacatggtggatgtacccaccatgatcattcagccattcgtggaaaatgccatctggcacgggttactgcacgataaagggaaaggcaaagtaaccatcacctttaaaaaggtagatgaccgcattttatgtaccatagaagataacggtatcggaagagaaaaatctgcagccatgaagcgcctgagcaaaccccgtcaccaatcccgcggactgcaaattacccgcgaccgcctctctctgtataacagccgctttaatgtggatgccagcttcgatatagaagacctgacagatgaagaagggaaagcactgggaacaagggtgaacctgtggttcccgtttgtggaagaatagcaaatgggaaagtagcaagccttcccatttgccggaatattttaggcaagaccggtttcataatgccgttccggaatttcaatatccaggaagccttttttaaacaaccatgccttgaagatttgctgcacatcatactctccatgtaccaggaaaagttttttcacctctttcggatgctgacacgccagccactggcttagatcttcatagtcgccgtgcgcactcatagaacggatcacgcctaccgccgcatttacatggaaacgggtaccataaatagatacctccttggctccgcgcatcagcttaccaccgagcgattgcggctcacaataacccacaatcaggatggtattacgggcattgtcgatgttgttggcgatatgatgcttcacacgcccggcttctgccatgccagatgcggaaatgatcacgcaaggttcctggcggaaattcaacgctttggattcatctaccgttttaatgtaatgcagcccggggaagtcaaacggatcatcatcctttttcagaatagcagccacctccctgttaaatacttcgggatgcgctttggtaaccgcagttgcttctgtcgacagcgggctgtcaacaaaaatgtcaaccttcggcagcttgcccgccagttgcgcattgttcaacgcgtacagcaattcctgtgtacggcctacactgaaagccggaatgatcagcttccctcttttttccatacaggtttcccggatatgccgcagcagctcagcatcagcgggagcggcgtctgcatgcagcgtgctgccataggtagattctatcaggatgtaatctgcctgtggaaacacctccggcgatttcagtatcgcatcgttatagcggccaatatcgccgctgaaagagatctgctctgttttaccgttttccgtgatacgcaggtgtacagacgcggcgcccacaatatgcccggcgtcggtgaacatcagctgtatgtccttatcaatgttcgtccaggtacggtaatccatgggcttcaaccggtcaatggccagtttggcatcatctacactatacaacggctctataaaaggaagtccttctttcgccatttttttattggtgtatttcgcatcatcgcgttgtatttcggcagagtcgagtaacaatatttccgccaggtcacgggtggccggtgtgcagaaaatatcccctctgaatccaagtttcaccagtcgcggtataagaccggaatggtcgatatgtgcatgcgacaacaccatatacgttacttcctgcggatcaaaaccaaagtccctgttaagagcatctgtttcatgacccatgccctggaacataccacaatccaataaaatctttttgccattcttaagtgtgatcaggtgctttgatcccgtaacagtgcgtgcagcaccatgaaatgcaattttcatatctgaaatttagcgtgaacggagttcaacattttacgatttacatttaaacgaccaggtgatcgcgaaggaggcaattaatatgccgtctttatccctgccttcactatgcagggttactgtttctgcagaattatcatttaacgcccgctctatagtagccctcagcagcggcagttcggagcaggtaaaggtggtaaggccagtcgccttttttacaaaagtagattccatgccggtaacgagcatggatacacgccgcggagcgctgcgcacatacatcatggcgggtaaaccggtgctgagttctgccgccatcgccaggcaggcaaagtaggtagacctgaacgggttttgcgacaaccaccggaaaggaaccgtggttacacagctattggttgccagtgattttaaccgcacccctgaaagccaggctgccggcagcttccagaacaggtaggccgaaaacttaaacggatgctgtgcaaacttctgaaaagattgcacagcatccgtattaaaagtggtaatgccgttatccatgacgatgctattcgttgatataatgggaaggctgcaacgcagcgggtgaccattgtttcaggaactcctgcactttctttttatcataggtatctgccgattccagcaaaccggaattctgcgtatgcagccggttacctttcgcatccagtattaccagcaccgggaaaccaaagcgctgtggataacccagctctttcagcacaggcaggttcttgttttccttgctgtagttaagatgatacactacataattatcattcagtgccgctttcagctcggcatcatcttctataaatttatataatcgtttacaccagatacaccagttaccaccaatttgcagcaacacatgtttctgttcctttgctgccttttttaccgcagctgccatatctgccttggcatcagcagcaggattgtaaatatgctccaggtcatgtgtttgcgcctgtgtggcaggaatcgcaaatgccatactcaataacaacgtccaaacaaacttcttcataaaaaacaattaatcaggatatctaatttacactatattttgcacatactgctggatggccagctgggctttggcagggtcctgcaactgcaaaagaacaatatctttcagctgttgctgcaacgccggatcatataccggcacacatacctctatcctgcgatggaggttacggttcatccagtcggccgaacccatatatacttcttcctggttattattatggaagatgaatacccgcgcatgttccaggtaccggtctacaatacgcgtaatgcggatatttttactttccgggatatccggcacgaggcaattgatactgcgcacaatcaggtctatctgtacgcctgcttcgctggcttcatacagtttactgatcatccctctttcctgcaggttatttattttgatgatgatcctgccgggtttcccttcttttacgtgaacaatttcccggtctatcaacccggaaaaacgcgttgtcatattaaactgcgctaccagcaaatgctggaactgtaaaaactggtaaccggctggttgctccctgctttgaagatagaggaacagcagttccatctcccgggtaatttccttatgcccggtaaacaaaacatgatcagtataaaaacgtgcggtgctttcattaaaattaccggtagcaataaggccgcaataatcccactggtatccacggttacgttttaccagtgctgttttggcgtgtactttcatgcccggaatactataaataagttttacgccggcatccttcattttctttgcccagcggatattattggcttcgtcaaagcgcgctttcaattccacaaacaccgttacctttttcccgttcttagccgcgctgataagcgcctgtgcgatctgtgaaccggaagcaatgcggtacagcgttacatatatttccgctacatccgggtctgcggcggcttcgttaaagaagcgcaggatgtaatcatatcgctgataggggagatgtaccagcaggtcctgttgtaatacgaggtccagcaaccggtcggtagccacaatggctttgttttcggcaggtattactttgggataatccacctgttgtaatcctgccggtgcgggcaggttagccaggtctttcagattatgataacgtccgcccattacctgttcatcctcctgtacatcaaactggatggccaggaaatgcagcagtgaccgggaaatggcggcgtcatacaggaaacgggtaggtacgcctaactcacgtttacggatcaacgtttccacttcttccaggatatcgcctttcatttcgtccatatccatttcagcattgcgggtaagcttcacactatgacagctttccaccgtatagcccgggaaaaggtaggacaaatgagcacggataatatcgtcgagaaaagcaatgtaatgaataccatcgagcgacggcagctgctgaaaacgcggcaggtcggcaggaatattcacaattacaaattcctgtatgcccgtattattttcaggtaccagcgttaccgccaggtacagctgattgttttcaagaaataattttttatgtttcccattgagccatactggttgcaaataggccagtacagtagtaaggaaataatattttgtaaaggagagatgagcagtttggaaaggttgattataatacaattgtacgccctgtgcctgcagatcgggtaacacgctgccggtgaagatctggccgtattcctgttgctgccggtttatttcctgcagcacctgttgtaaggtatcgctgctgatggattcattttcaccggctgccggatcattttccagtacccggttaattgtaagtatagccggcattctcacccggaaaaattcatcgaggttggaagaaaagatggaaaggaatttaatcctttcgtatagtggtacctgttggtctgccgccatcaacaacacccggtaattaaaggataaccagctgagatcgcggttatataaaggaacacccatgaatcattatgcttttaccgggaagaaaattgctgcaatcaggaaagcgaatacagaaatgataagaccaaacatgaaaatattataggaaatacgcagcagtttgtatttatgacccagcactacgccgaggtaataaatgtctcttgtcatgctgctgtacaggaattcagagtcatccatcatctgttttattccccactggtattcttccaggtgcatcttataaaagttgccaaagaacaggaggttggcatctttcttttcgatatccgctttggtgaagatgccgctggttacattcgggcgggtggccagcaccgaaaagatgaccgtgagtactgccgtgaaaaggaaaataatagacgggatcaccatattcggataatcttccagtcgccttaccagcacgctcaatatcaccgaaatgataatggaattcaccgaaatcatgatatgcgctttgctgtcggccatggagctgaggcggatatgattggtggaagtggttctgaacatcgtttccacgccacgttccgatttgccggctttgtccttgcccttgtcttttttctttttttcagtggcggtagcaggcgcctcgccggaaacgtctgtaccgggaatggcggtgacagcggtgatattattttcagctgcttcttttgtttttttctccagcttctttttcagcttctccaggttctcttctttctgttgtttaaacaaagtttgggcatagtcggtccagtaatgatggtccgttaaaaaggtaatatttgtattcagccatttgatggcgggaatatcggtttggtaggtgagctccatttcgtgccggagcagtttgttccggtcggggaactctttggaccccaggtgagagaggtcggcgtcacaaacaatctgttccaccaggttgtgcggcgactggggcattttggtagccaggatagcgccctgcaccatcgactgaacattttcaggcgcctgttgttgctgtaagaattgcagggcctctttggcgccgttttcttcgtgggcgctgccttcgcccaggagatacccggcgtcatgaaaccaggcagccacatatactgccgctaattcgtcgtcctgcaggcggtaatgagccgcaatttgcccggcagcctgtactacctgttgcgtatgtacgagattatgataaaccaggttagggcgcgggtgttgctgatactgggctaaaacatagtcccgggctgcatctataatagcattcttttgcataaggaagacgaaaattaagataaggaactgcgaaatacgctgtttactttgtactttttatcgtactaataacggtatgttcgctatttcgcgtattacaaatcgcaaattgagcctaagttactgcatttttgagttaaatttatgccataaagttacactatggatgtccgcatcgggttaatatttctccttttcttactgtcatgtaatctgagcgacagggaacaaaaagtatacgcctctccccgtggttacgatttaaaagagccggtacgctaccgggtcagggaatctatgcaggaaatctcgggtatagaattattccccgatgagcacaagatcatggccattaacgatgaggaaggccgcatctaccagctggatgtattggcaaaagaaccttatccccattttaaatttgcaaaagacggggattatgaagatatctgtcatacagatagcggctggtttgtgttgaaaagcaatggctccctgttccaggtccacggcctgttcaccgacagcgtttacagcgatcatcacaaaatgcccaaaacagggaagaaggagtttgaaaccacctactacgattcggctcataacgggattgtgatgatctgtaagaactgtgaagatgataaacgccatggcgtaaccagcgcctaccgcttcgatctggctaccaaaacatttgataccacagctgtctataaattcaataaccaggaaattgcccgcctggccggttctgatatgcggttcttcaaaccatctgcagcagccattcatcccattgaaaagcgattgtacatcatcgcctcagtaaacggactgctcgtaattgccgatcttcagggtcacgtgcaggaagcctacaaccttaaacaccgcctgttccttcaaccggaaggactggccttcgcgccaaacggcgatatgtatatttccaatgaaggcggatacgacggtaccgccaatattcttaaatttacctacaagaccaaatgatcagatcaaccatcatctatattgccctgctaatcttcacaggtactgccacctacgcccagtcgccgcaggtagtgaaacgtgtaatccttatcggcgacgccggggaattgcacgacaacggcaaaaactccgtagtggatgccgtacgcaataccttcgacctccaggacagccgcaataccatcctcttcctgggcgataacgtatatccgcacgggttacccgactccgccagcagcaagttccaggtggccaaagaaatcatcgactaccagatcaacctggtacgcggtaccaaagcccaggggtatattattcccggtaaccacgactgggacaaaagcaaacccgatggatgggatattatccgcaatcagcaacagtatgtggattcccaacacctcgataacgtacagtttgaacccaaagaaggatgccccggccccatagaagtaaagatctctgataatatcaccctcatcattatggatagcgaatggtgggtgttcccttatcagaaacccggactggaatcctcctgcgattgtaaagacaacgacgagatccttacccggctgtcggaaatagtggctaccaaccgcaacaaactgatcatatttgctacccatcaccctttccgcagctacggcatccacggaggatattatacgatcaagcaacatattttcccgctaacagacctgcgccccgcactgtatgtgcctctgccggtgataggttctatctatcccattgcccgcggcgtttttggtaccccggaagatattcccaatccaaagtaccagcagatgatcaaaggagtggaagctgccctgaagccacatggccccgttgtatttgtgtccggtcatgatcacaccctacagcttataaaagatcagcagaacgcctatgtggtaagtggcagcggcgcaaaaaataaccgcgtaaaaaaaggcgctaaatccctttttgccagtacagataacggttttagcaccatcgaattaatgtccgacagcactgtgcgcgtccagtattatacggctgataacggcgcacaacccgttttcagtaataacctgttccgcctgcaggacattccgcaacaggcgcttacctatactccgccggcatcactgcctccctttatcagggtagctgccgatacacagtatgtacaggtctctaactttcataaaaaattgctgggagaaaattaccggaaagtatgggccaccccgttgaacttcccggtactggaccttaaaaccgctaaaggcggcctgaagatcctgcaacgcggcggtggaaaacaaacacactccctccgcctggaagacagcaccggcaccgaatggtccatgcgctccctgaaaaagttcccgctggcagctattcctgaacagctgcgcgaaaccattgcccgcgaagtagtacaggaccagatctccgccgccaacccctacgccccgctggcagtaagcgtattggcagaagccgccggcgtgccgcacaccaatcctacttttgtatacctgcctgccgatagctcgctcggcatctatgcaaacgactacggaaacgaagtattcctctttgaagaaagggaacccgttaccggcagcaacgataaaacttacaacacaccaaaggtactggcaaagatctggggagataatgacgaacatatagatcagaaatccgtgctccgcgcccgcatctttgatatgtacatcatggatttcgatcgccacgatgaccagtggcgctggtataaggaaaagcacaaaggagaagaattttattacccggtaccccgtgaccgcgaccaggcgtttttcctgaacggaggttttattccccgccaggctgcccgcccatggttcatgccggctatccagggcttccggaaaaacatcccggatatcaatggcttcaacttcagcacccgttacttcgatcgctctttcctcaacgaaatggatgaagaagattggaagaaacaaacagataagcttttaaggaagatgaccgacagcgtgatcaacgctgctgtaaaagcttttccagatactatccagtcgctggtagggcccatgatgatagaaaaattatctgcccgccgtaacatcctggaaaaaaatacactgaaatactaccgcttcctcgccaaaggcgttgacgtgccggccacagaaaagaatgaactcatctccgttgaaaaacaaccgggtggtaaagtagcactggatatattcaagatcagcaagaaaggagccgttcagcaaaacatctactcccgcaccttcgaccccactgtaaccaaagaggtaaatgtatatggcatgggtggcaacgatcgctttgtgataaaaggcgataacgcaacacccatacgcatacgtctcatcggcggcaaggaggcagatgcctatatcgacagcaccaccagcagggcgggcaaacgggtacgtatatacgatcagcgatccggcaaagatagtttcgccctcaccggcaatgaacaacgccgcctgtccaacgatcctgctaatatcaaatataaccgcagcgccttccaatacgaaaaaacaatgccgttactggccggtggctacaaccgcgacgatggtttgctgctcggtgtaggcttgtctattacccgccacgcatggcgccgggagccgttctccaccaaacacctgttcaccgccacccacgcagtagccacgcgcgcctggaacttccgctatgaaggagaatatacagacgtcatcgggaaatcagacctgctgctgtttgcaagagcgaaagcgcccaacaataccatcaacttcttcggatatggaaatgaaaccgtattcgataagtcggataataaaaccatttcctactatcgcgcacggtataacttttatacagcagaagcattactgcgtaccagcataggaaatcatatgaccattgcgtatggtcctacattcaataactacgcttttaataaggatgaaaaccacgaccgtttcattaccgacttcaaagacaacggcctggattctgctggtatctacgccaataaagcatatgccggtggtaaaatagtggctactatcgatacccgtaacaacaagatcattcctacccgcggtatcctgtggactaccacctacgcaggtaactttggtgtaaatgataacagtcacaatactacttcgctgcaatcggatctgagcttatacatgagcttccgcatcccggcaaattttgtaatcgtcagccgttttggtggtggtaaactttgggggaactacgagtacttccaggcactcaccgtaggcggcgttcaaaacctgcgcgggtaccgcaatttccgctttgccggcgacgccagcgtgtataacaatacagaaatacgcgtgaagttattcgacctgaaaacatatctcctgccagcaggcgtagggctgatagccttcaatgatataggccgcatatggcgggaaaatgaaacctcccacgtatggcacgatggatatggcggcggcgtttatattgcgcccatcaacgcgctcatcatcaccgcagtggtagggcattccaaagaagaaacagtaccctacataacctttgggtttaaattctaaataaaaaaagaggccggctcatttgagccggcctctttttttgtgtcacccaacgggcaacgtatcctcgcttcacagcggagcttccatatttactttcacgcggagcgctttcaatccactcacaccttgtaactcttccaggtccagcatttcaatttccggcaacagtattttcttgctttgcaggaaagtgatatactttttcagttcttccatttccctcacataagagtataccattgcaatggtaccaggctgcgttaaccgctcgccggtatcttttatgtgtactttatcaatgcgttttttgatgatctcataacgcacattgtaagcgccttccacatcaaaccggcgttcatcgctgcggaagctgatggtaataggagcgctgtgcatcaggatcatctgggtggtttgcagcggcacttttaatttaggccccagtttatgtgtaagtcttgcgatatgcgccatggaggaaagctgccacaggcgcaggttgcgcaggtataactggtcaaacttcttttcctgggcaatcgactgcccaatataaatagtatactccacgccatcggtacggtacttttcaaagtagcaggggaaagaatgctggatatactggcgttctttctccaggtactggctgatggctgtgttgatgctggctaaactgtcttcgtactccctccggtgatgataaacatgtccttctgatttgtccatctgggcaaaatagctggccagtaagggtttcagatcttcattatcttcacagagatgttccagtacaggctgtatctcctggtccatgaattcattcactttcaggtcttcgcccgcctgcaggctgttactgagattgtcgagcaggtcatttgttttaaactgcagctcttccagtaaaggcaggtgaatggttttaccgatggtttcaagggtatcacggatcagttccagctgttcctgcaaatcctcgcggatggcagtgccttgctgtacagatgagttgcggatatccacagcgccataaagcgggtatacctcatcaaagctgatgctttcaatatctttcctttcttcttcgggtgtcagcaggtaactccaggcagcgtctacaaacttccattctacggaaggctgtaatgcggtaaactggtctttgatcacttcattcagccggttctcgaggatgttcatgctgcggttcagcatgagcaccagcaggggataggtgttttgcagcttccacagcgggtcagccgacaagcggttgggagtggaagaggccagctccagcacgcccagtatttcctttttatgggtgatcgggagtatcagaaaactccggatgttcttgatcggcaaatatttcaggaatgcgtggggcgcaatagacgcctcatttacatccggaacaatcagcggcgcagggttttgctgcgaatgctccagcagcagctggaaaaagtgttgctgttgttttttgttgccaacccccaggattggatcggtattggaaaattgttcttccagcacattcttgccattcactttagggaaaggtaccaggtgggcggttacatcaggtatgcccaaaataaccgggatcattttttccagggtacggtagctctctacctcgttgctggcgcgcatgttcatcaccaggctcttgatattattgagcgtttccgattgggttacatctttcacggtccagataacaaagccttccaaagaaaacatactggtaggcaacaactcctgcagggcatccggcgtgatctgcttggaacagaacatatcatagttcagatgcggcagttcaccgtttacctttacatccacaaacctgggatcaatatttactttcacataacgtttaccaccatccggcgtttccagcgtatggatgatatcgttcttatagttcatgggaaagtggaataccttttccaggattagtttatataaccaggtgatcttgtctttttttacctgtgcaatggaaatgccgtccggaacggccgataactcggagccgttttctgcaaatagctgtttaaagagatcagaataatggaagatggcgaacttaaacggaacacctatgccataaatgtctttgctggaatccgtggtcaccgggaaaatggcggctatcaatagatccaggtattccttataagcgctcagatcaccattgccgggaatgggtttaagtatttccgggttactttcaaatttatcaatgatcagtttatagaaagacgaacgggcttctccttcatgtgttaccttttccttcagataattgaggaagggtacgaatgatatattggattcaattactttatcatcgttaaatataccggggtgtgcagttaaaactttcatattatcgtacaattataaccaaaggctgtccttttagtgccagtaataaattcttattacaatttacagtaaaacattgcaggaataacagaggagggtactaatgtagacgcaaaggtaggggaaatattgtatcaatattgaattccgggattcaggtatttgtcaaatctggtatacacctgataatcaaatacctgaatccgcagaaatccggaagatttattgcaattcgatctggtttttgagcagatcttccaaagtatcacgcttgcggatcaggtgtggtttgccttcttttaccagtacttccgccggtttcaggcgggagttaaagttagaggacatttcaaaaccataggcgccggcgttataaaacaccaggtaatcgccttcccttacctcattgatcttacggtcccatccaaaagtgtctgtttcacagatattacctaccacggtatagatccgctccgtgcccttcgggttggaaatattacggatcaggtggaacgcctcgtaaaacatcggccggatcaggtggttgaagcctgaattcacacccacaaatacgttggcggtagtttgcttgatcacgttggcctttactacaaagtaaccgctctggcttacgaggaattttcctggttcaaaccacagctgcagcgggcgcacgtatgatttagcaaagttgttgaacgcttcgctcagttttttgccgagcaggtcgatgtctgtttcaggatctccctgttggtaagctaccttaaagccgctgcccaggtcaatagactccaggtcagggaagtgttgcaccatttcaaacatcacttccacgccccgcaggaacacgtctacatccttgatttcagagccggtgtgcatgtgcaggccggttactttcagtttagtagaattgataatgcgttcgatatgccgcatctggtggatggaaataccaaacttactatcgatatgcccggtagagatcttaaagtttccgcccgccataatatgtgggttcaggcggatacagatcggataactgccaccgaacttgttgccaaattgctccaggatggagaggttgtctatattaatgattacgcccaggtctttcgctgcaataatttcctgcaggtccacacagttaggcgtaaagatgatattcttcggatcaaagccagctctcaggcccagttgtacttcctggatcgacaccgtgtccaggccgcaaccaatagaattgatgtacttaaggatattgatgttggtcaatgccttacaggcgtagaaaaagcgggtgtcagacttatgaaaggccttttgcagcttttcatactgggttttaatcttttctgcatggtatatatataccggggtaccaaattcttctgctactttcacaaggaaatcggcagtaagtacgtcgctttgtttaggcattgaaaatccttagtttaagaatgaggatgcaaaattactacgcaaaagtgagaaattgtagaaaaaagggagaatccccggtagcggaggtacttataagcaaattaacgtctttatggagcaatacagatttgacagaacagccttcaaaatcaagacatacgctgagtcggacgcggataatgttgatttaagcctttccctggaagagcgggttcgccaggcgtggtatttaacatcaaaagcctatggttttgacctgaataacccaccacggatggataagactgtattttcatgtagaaaacagaaataataaggtggcgagtgttctctgatatggaatatagtcctaggcattatgctggcgctttgtatggtagctctggtatctgtggaatttatccactgccctggttttgttacaaaatgaagtcaaaacatggcttgttttgtcacaaattaaggataaatttgggcttgttttatgacaaatttgaaaaaaaactattcctggtatgtcatttaaaagaaatattgaaaaataccttaatgtctggaagttaagtgataatcgaaaaccgcttatcatcagaggagcacgtcaggtaggaaaaacaacactgatacgagattttgctaagacttatcagtatagaattatacttaatctggaaaagcctaatgatcggagttattttgaagattttaatgacgttcaaactattctggaagcgttgttattagcaaatgctattccttcgtctgctattgctaatacactcctttttattgatgagattcaggagagcccaaaagttatccagttgttacgatatttctatgaagaattaccgcaacttcatgtgattagtgccggttctcttttagaatttgccatgcaaaaggtaccaagctttccagtaggtagagtagagtttttatatctccatccattaaattttcaggaatacctggaagcaataggaaaacaagagctgatagaacatttacacgcagttccggtaagggcagttgctcataagttgttaatggatgctttccatcgctatgcaattattggtggaatgccggaagtaataaaaatggatgttaagcagcagaatctttcggatttaccaaggatatatgaaagtatttgggggacctataaaagtgacgtggaaaaatatacatctaatgataccgaaagaaaaattattaaacacttgatggataccgccccgttgtatctcgacgaacgtgtaaaatttcagggttttggaaattccaactaccggtcaagagaggtaggagaagctttcagaacacttgatgatgcaaaaattatacgattgatttatccaactacagatttgcacccacctctaaaaacagatctaaagaagtcaccacgtctacagtttctggatactggtttggtcaattattctcttggtatccaattagaaatgttagctatggatgatctgaatagcgcgtacaaaggcgctgttatacctcatttaataacacaggagcttatatctcttcaaagtatttcagcgcataagcctaatttttgggttagggaaaaaacacaatcaaatgcagaggttgacttactttttacctatcaggatttggttattcccatagaaataaaatcaggtagtacagggagcttgaaatcacttcaccaattcattgacgcagcagatcactcatatgctattcgtatgtatgctggtgtttttaaggtagaacaagccataacccctaataaaaagccctatctgcttatgaacttaccatactatttaggcacaagtttgccactatatattgaatggtttgtccaacagaaactttaatgtattgcccgatggttgaagtgtagccggttttcctcagattagcttgatatgttttagcaaggacttacactactcctcttcatccccttccataaacccttcaatactcctccggtctttcttcgtgggccggccaatcttactctgtcgcttacctgtctgaaacacagacgcaacaaaggcgggcgccagtttatcctcatcaggagtggtatctatataatgtttaatggcttcactatacggcacccggttggagataacgctcaccacttcaatcacccacttacgggcttcgctcctgatctcaaatttatcccccggatttacgggcttagcggctttcacagaggagccgttcatcttcactttaccgccgtcgcaggcatctgcagcctggctgcgggttttaaacaccctgatagaccagagatatttatctacgcgtactttttcggtattactcatattcaaaaactttaagccggcggcaaccggagctgccgccggtttggctatttactcatctccgcaaaaaatttgtggaaataaggaatggtttcaatgcctttgtaataattggctaaaccatacttctcgttgggagaatgcaggttgtcgctgtccaatccaaagcccatcagtactgttttcagccccagttccttttcaaacagtgccacgataggaatactaccgccaccgcgcaccgggataggatctttgccaaaagtagcgtggatagctttgtgcgctgccttaaatgccaccgagtcgattggcgtaacatacgggctgccgccatgatgcttggttactttcaccttcacactcttaggtgcaatggcttcaatatgtttggtgaacagatctgatatttcgtgccagtcctggttaggaacaaggcgcatggaaatcttggcaaatgcttttgatggcaatacggtcttggaaccttcgccggtataaccaccccagataccatttacttccagcgttggccggataccggttctttcgatagtggtaaatcctttctctccccaaacatccgctacacccaggtcttttttatattcttcttcatcaaaaggagcggcattcagcgcggtcctctcttctgtacttagttcctgcactttatcatagaagccgggaatggtgatgtgattattttcatcatgcagggaagcaatcattttcgcaaggatagtagccgggttagctacagcgccaccgtatacaccactgtgcaggtcgcggttaggaccggttacttccacttccatataagccagtccgcgcaggcccgtatcaatggaagggttttccaggctgatcatggaagtatctgaaatcaataccacatccgctttcaggcgctctttgttatctttcaggaagatgcccaggttagcagaacctacttcttcttccccttcaatcataaatttgatgttgcagggaatcgtgttggttttgttcatggtttcaaaagcctttacatgcatgtaaaactggcctttgtcatctgcactgccacgggcatatatattgccatctttaattacgggttcaaacggaccgctgtgccacagctccagcggatctgcaggctgtacatcatagtggccgtataccagtacggtgggtaaggaaggatctatgatcttttcgccataaacgatcgggtgaccagcagtctgacatacttctactttatctgcgccggcttcttccaaacgtacttttaccgcttccgcacattgctgggtatctttattgtgacgggaatccgcactcacagaaggaatgcgtaacagcgccagtaattcatccaggaaacgatctttgttctctgcctggtaatctttccaaacttgcatgattctaggaaattaagttcacaatgtggtgcaagttaaaggaaaatcaacatttacagatttagatagtttcgaatggtagtccatgccgttttagagagaagtgaaccgttatcacttcccgtttgaataacatccaatacacgatactctcccgtttgtcaatctcaaaattctgaccggataccctgctaagcttttatcttattttcagtaaaaaaattaatctattatgggaaaacaagtcggaataatcagcttcacgggcaagctgggtaacctgatcggttaccggaggaacgggcaatactttgtccgcaccatgcccgaaacggtgcggcaaaccgccgctacccggcatgcatcgcgggatttcgggatcgccagcaggaaaggaaaactgatccgccaggctgtcactcctcacctggatatcacccgcgatggctcattggtgaaccgcctgaacaaaacgctgatctcagcaggagaagaccaattgcaaatgttaaccggcttccggttcaaccggcacgccggcgtggagcaattcttctgccagcagccggtgatctcacccgccggggtggtaaccatacctgggcaaaccttgcggccggaaggcacagccacccacctggaagtgaaggccattgccgttcgcatcagtttcctggagcgacgcataacaggcagccgtactgccactgtaatgatcggtatggacacgcatttccgggatatggagctggatgtaacgttgccgggaaaaggaacattgctggtaatactacaggtaagaagcttcaacgggtcgctggcatcggccaaccgccggttcatagcggcaaacatactcggggtggtcacaccggcagtcacaaaacagcgggcgaccattataccggatataaggaaagtaccccgttataaagaagcgcgcgggaagaagtacaatactaccttgcgtatacctcatatggtgacggtacaccaaagggaatgagcagatgttttcctgatcaagtccaccttgcgtgcaaggcaaaagtaaggcataagcaggcctgtccccattttccaggaacgcctcgttatcttcactgcctctaataatgatcaggaaattagtttctgtcttaccaggaactccagtttctggtttacatcgagcaatttggcggttaactctttattctctttgcggagggcgtacacttcatatgccttttcgatattgtgtttcaactcctcttcattccagggtttggagaaatatttataaacctgtcctttgttaatggcatctactaccgcgttgatatcggcatagccggtcagcagcatgcgtataggctcggggtacttttccagtattgattcaaaaaactctatcccggttgtctttggcatccgctggtccgagataatgatgtgaaattcctgttctgccagcagcttttccgcgtcctccgcagaactggctgtaaccacgttgtacagccttctgaatgaagctttgaaagcattcagattgtgtatttcatcatcaatatagagaatatggatgtgttgtgcactcatttaagcagacttagttccaagttattgataataaatgagttagaaacaatgaaactttcgatatcgattttgtatccattctgccccattcaccttaaatcttacggtaaaacgttcaatgttttacgctcaacaaaggtacatataaacatactgttttatgatgaatatttcaaggatgaatgaacttttttaaaaaatagccgtttccttatccaatagcgatttagtgggggagtttccatattttcgtgtagttatgaaaagcgcgcgttaaccgctttttttatagcgttcaccggtgaaaaaactacttacaccggcaagcgtaaaatcgggaataccttttgcacatttgccggcacttaaaacttaaatttaaattcagatgaaaacaggaattattgttattgtagtactcgcgttgttggtcatgttaggttgtggtaaatacaacggcctcgttactaaagacgaaaatgtgaaaaataaatggggagtggtacaaagtagctatcaacgccgtgctgatctgatccctaacctggtggccaccgtgaaaggcgccgctaatttcgaaactgaaaccctcgaaaaagtgatccaggcacgcgccagcgctacccagatcaaagtagacgtgaatgatctcagccctgagaaaattcaacaataccaggctgcacaaggacagttaagccaggcactgggccgcttactcgccgtatctgaagcctaccccgacctgaaagcaaatgctaatttccagaacctccaggctcaacttgaaggaacggaaaacaggattaacgtagcccgaaatgacttcaacgaagcggtaaatgcttacaacagctccgttcgtactttcccaaacaacattatagccggtatcactggctttaaacaaaaaggttatttcgaagcagccgcaggtgcccaaaatgctcccgaggttaaattctaaaacaacccttacaagataagctgtctccgggatgctggtgtaataccggcatcccccggaacagcaatccaaaaattatattcagcatgcgcattttcccttttaaacgaaaagagattttttcagaaacggagaaagaaagactcgtgcaggctatccgggtagcagaacggcttacttccggagaaatcaggttgtttgtagaaagccattgcagctatgtggatcctatggacagggcgaaagaagctttcgtgtcactcgatatgggaaaaacaaaattgcgcaacggcgttttggtatatgtggccatcaaagaccggcagtttgctatcctgggcgaccagggcatacatgaaaaagtaggcgacgaattctgggtgaaggaagcagcattgttaatcgaccactttcagcgcaatcgtattatcgatggcatcgaagcatgtatagcggaaataggcgcctcactccgtacctttttcccgcatgaagccggtaatgatgcgaatgaactgcccgacgatatcgtcttcggcaaataaaagccactctttttaaaacgattttagctttgatacaatgaggatactacgctggtttttaccgggattattaatgatggcgggtttgctggcaaatgcccagaatataccgccccggcctaatcctcccactttagtcaatgactttgcaggcgtgttgctgaaaacggaagatgatgccctcgaacaaaaagtagtggcctatttcgacagcacctccacgcaaatagcaattgttacactcaagtccatcggtgactacgatatcagtcaggtatcattaaaaatattgcgcgactggggaataggtaccaaaggcaagaacaatggtatacttattcttgtttcagtggaagacaggaagatcaggattgaaacaggctatggcatggaaggcgtagtacccgatgctaccgccaaccagatcatttcacagatcataaagccagctttccgtgaaggacactactaccagggcctcgacggcgctgtggaagccattcagaaagcagccgccggcgagtaccgtgcagacccgcggcaaagcaaacccggcgtcagcccgggagccgttttcctgatcatcatggtaattgtgattattgtttccatcatcggccgtggcggtggcggaggcagaggtggcggtaccacctataacagacggggcggatggatatggccggtaatcggcggtatgggaggcttcggcagtggcagcagcggaggcggatggtccggtggtggaggaggtggcggcttcggtggcttcggaggaggttccggtggtggcggtggcgccagtggcagctggtaagagcaggaaaactattttatgtcatatttgcatgtgttaaatggagatgctacccttgccctgttccggcaaagcaaggtaccgggagagatagtggtgtgccgggaaatgatgtgcgaaggcaaagtaaaatatacaaaagacctcacagaattctttgaaagccgcgccaagcatctcgaattccattacggaatcgataagcaaacctattataccaatgtggtacaggagctggagaaattagcactctccggctccgctgcagatgaaatcgtattgtggtttgaatatgatctgttttgccagatcaatatgctgttcatcctttactatctcagcagccggcttactatccttccccccattaccctggtagacctgcaccatcaccccactgcggatgaattcccgcagatatttgaacaacggacacagcttcaagctgaagacctgctttgggccgccgacgtatgggacgcctggtgccttagcaccccacaagcgctggaaaccatcagtaagctgcccgccggaaatcttaaatacctgcccgaagctatcactgcacatctcaaacgcttccccgatatcaataccggcctgaacaccattgaaaactatttcctgctccgcctcgtgctcggaagctaccgctggtacgacctctacatgcttttctggaacgaactcgaaatatacggcttcaccaacttccagctcgatgttctcatccaccgcatggccaatgccggcgtcatcgaagaacacgaccaaatgctgaaaatcaccagcctgggaaaggaaatactggaagaagaagaaaactacctcgactacatatcactcgaacaccgctggctcggaggcgtaaaactcgccaacaccccctggcgctgggacccacaactcaacgccctcgtggagattgaagcgtagattgtcgcggattttgtctttcccgctgattacgctgattttactgattttactttttttgattttttttagattaaaagatagtgggagataaaagcgatgttctgcttctatctcccattatcaattataaaaaacaaatcaattaaaaatcaaaaagtaaaatcaaaaaagtaaaatcagtaaaatcagcgtaatcagcgggaaagacaaaatccgcgcacgcattatttaatacccgctttgatctcctccgacgccttacgcagatagtccgcctgtttcagcagctcgtcgcggttagcgccggttacggcagtggcttcctgcgatttgcttttgctgatttcctgcatccagttactgatgtaggtgcttacctgtgagttattaaattgggcggtcatggcttttacctggtccacaccttttgttacagcaggggtgttgttgatcttggataagaagcccaggtagtcgaaagctgcattcagcttgtcctggccggaggtttcatcaaattttgttgccacaaaagtaacatcggaagcgttgcctttcctggcatatacacctgcgatagcatttaccagcttgcctttggtatcactttccagctgtttggcgatgttgtatgctttttccagatccagggtggctaagccttccaggccggcggcttctacagcataggatttgtcttttgttgctgcttcaaacaaagcggcgtactgcggatcttttagttcacccagttgcagcagtgctgctgcacgtaccagggagctgggatcttgtttggcaaggttcgccaaaacaggcagggcggctgttttcacagctgcattgctcaggttcagctttccgatggcatacgttcttaagccgtgatatttatctttcaacgccagctgcaacagtttcactgcttcaggattggtggcctgtgcatctgctgcttcatctatagcaatatggcggtccatataattaggcgcgtgggcatattgataagcataagtgctaaacgcccggtggtcgtctatcttggctaaaactaccttatctgcatctacatttaccaggtctggtttagccgtgtaagagaaggtaaaggaatcaacccggtgttccatgaagatgttatgcctgtttgctttgccgccttcatagatgtcaatggccatggggatgtgccatactttatcttctttctggatctgctgtaatataacggtcaccgtgttggcggcatcattatacttatagctgatatccagctgtgggaagcctttaccaaaataccattcgttgaagaaccagttcatatccctgccggttacttcttctacagctaaacgcagctgatgcgcttcggtagctttaaaggcgtttgttttcaggtaaacgttcagggatttgaagaaggcagaatctcctatggcattgcggagcatgtgcaggatacggccacctttctgataggtgatctggtcaaacatatcttccttgtcgtgataatggaagcgtaccaggtctttatcgccggcatactgcaccatcgacatatacgactgtgccgcttccaggctgtgttcatcggcagcgtccttaccatatttatgttccagccacaggtattcgctgtagtctgcgaaggattcattcacagtaagattgctccacgactctgcggtggccaggtcgccaaaccagtggtggaacagttcatgcgcaattacgccttcattgtagttgttattgtccagcagctcccggtccgttttctgtataaactccccgtgaagagtggcggtggtgttttccatagcgccggaaacgtagtcgcggccggtgatctgggagtatttcacccagggataatcatatcccagtattttagagtagaaggtgagcatttcaggcgtattaccaaaaatgtttctggcatatttctcaaaaggcttttccacataatagcttacttctttgccgcgccaggtatcttttacaatggcatattcacctaccgccatcataaacaggtaaggggagtgggggagatccatcttccaggtatctgtacgggtaccgtcggcattatttttctggcttaccagcttaccattggaaagggtaacatatttcttttcaacggtcatgctgatttcctcggtgcacttctggttggttttatcgatagtaggaaaccaggcagaagagctttctgtttcgccctgcgtccatatctgggtgggctttttaggatctttgccatcgggattgataaaatagagtcctttggcatcagaaatagcggcgcttccctttactttgagttcatcgggttttgctgtatagctgatatagatgatatatgattcggtggctttgtagcttttatccaaagcgatgtgcagttggaggtcgtcgtagctgtatttcagcggactgcttttacctgctttaactacggccacttctttaatatccatgcctttggcgtccagggtgagggagtcggtggcataaaaatgcggtttgagggttatccaggctttgccatagaggtaccgcttggcgtagtcgaaacgtacgtccagcttagtgtgtaccagatcgttcactttagtggcggatgcgcggtagatctttagtgcggggtcttcctgggcagctttgtcagattgggccatcagggaagtgctcatcccgagtccggctattcctccgatcagcatccccatcagggattgcttcagatgtagattcatgtaaaagactgttttaaacaaatgtatcggcttgcgccaattaaaaagagtcaaatttaaacaaatgggccaaatatgaggtaagtggttaaaaatgctatttttgttgagcttacaggccaataaaacagcattatgatcaaagcaatagtgaatggtaaatctacatttgccgttaataacgattccaaacttacctgcgataaccaggaagtggactggtcggcagtaaagctgcctaccggcgattacagcgttataatggacggccgcagctaccaggcgcaggtgttgaggatagagaaagatactaaaaccgtggtattacaggtaaatcagcaacagtttgaagtggtgatagaagaaccgatcgaccagctgctggcctccatggggatcaaggatgcgatgaccaaaaaggtgaatgacatcaaggcaccgatgcccggactggtgctgaaagtgctggtaaccgcaggtcaggccatcaaaaagggcgacccggtgctgatcctggaagccatgaaaatggagaacgtgttcaaggccgcctcagatgctatcgtaaaggaaatcaaggtaaaagagcgcaccgccgtggaaaaaggtgaggtgctgatcgtgctggaataatatttgcacaaggacagttttataccaatatatagtatgcatctcaaatacaggacagtaatattcgtatgggcatgtctgttactatgcggccggctgtgggcgcaggaacaactccactacgtgtatattcagagcgagaagggacagccgttttatgtaaaacataacggcaaagtgctgagttccaccgaaaggggctacatcattatcccccggttggaaacaggtacggcgcccattacggtgggttttccaaacaaagaatccagggaagcacagtttaaccttagaataacaaaaggtgatcagggctttctgctgaaacagtccggcgaagccggttattctttatataaccttcaaactttccgggaactgaaatcggatgccggcgaaacggcactggcagcagcgcctcccgccgcagattccattgtgccggagctggacacggccaaaaaggaaatgatgaccaacctgcagaaagacctggaaactacttttgccgataaagcaattgtaaccggtcctgctaaaacagctcccgctaaatcaggcaatccttttgcttctgcgctggataaggtagtggtaggcggcgacgacaggaatgagccggagccagagccggaagtaaaaaaagaggcagctcctgcggaagtggcgccggtggctgccgaagcagaggtgaagaaaccccggaagaagcgtaataaaggagaaagagagcctttaacagaagaggaacaggcgattttgagcaatgtattggcagaagaaggtaaaaccgccgccagcgaagctgctgtggcagctgaatccaccaccgctcctgccggagaaccggtgaaaaagagatccaagaaacataaagcaaaagaaggagatcctgactttatagaattccaggatgatgcggcacctgcagcagcagctgctgctactacggaagctgctgcgccggtagtggtggaagtgccggtaaccgctacagaagaagcgccggtgcgcgccaaaaagaagaagaaaaagatctttgatgatacagagcatccggcaaatatcatcaccgattccagtggctatggcattgctgttacagaagaagaaccggtaagaagcaaaaagaagaagaaacgtaatgaagaagaagtggcgactgcagatgcagcaggagcaccggtgggagcagaagtggcgccggaaatgacgaccgctgaaaagaagaaagccgatgcacgcctgatcaactcagattgcaccaatgtaatggacgatgatactttccgcaaggtgttacgcaaattcgtagctgccagaacggataacagtatgatcgaagtatttaagaaacaaacccgcaactattgcctgcaaacagttcaggtgaaaaccctggtacagttgctcacggcggatgatacgcgctatcgcctgctggatacagcctattccaaaacagtggataccgagaaatatggctccctggaaacccttttaatagatgactattacaggggccggttcaaagccatgttgcataaataatataaccttcattattacggagttataggaagatggatcacaggatcatctgactataactccgtaattcattccggatagtccgtaattctttattttcgcccccatatgaacaggtactttattgaagttggatataaaggggcgcagtacagcggtttccaggtacaggaaaatgcacataccgtgcaggcggaaatagaccacgcgctgagtacattattccgggaaaagatggagagtactggctccagcagaaccgatgccggcgtaaacgcgcaacagaacttcctgcattttgatacggaattgcccctgcatccgcagttcctgtataagatcaacgccattttgcccgatgatatcgtgctgcgggccatctaccaggtaccgccggatgccaacagccggtttgccgcattggcccgctcctatgaatataccttatatacccgcaaagatcctttcctgaaagaccggggctacttttttccttataagatggatatcgctgcattgcaggaggcagcagaagtgattaagggttatagcgactttaccactttctcgaagcgcaatacacaggtgaagacttatatctgcaatattaccgagtcgtactggacggtagatggagaacgtatagtctataacgttacagccaaccgtttcctgcgtggtatggtacgcggcctggtgggaacgatgctgagagtggggcgcggtaagctttctatggaacagtttaaggaagcgatagagagcctcgattgtacaaatgctgactttgcagttcctccgcagggtttgtttttaatgaaagtaagatatcctgatgggttgctgcagccaataagctttgatcgtcaataattctttgtctctgtaatcctttgcagcagagggttacagagaaagataaaaaatagtcgggctaaaaagttggaagtgtaaaaattccgcctacctttgcgctccgctttgatagaaagcgcgcatacaaaagctctttccgacactatatttctacacttatttcatcatggcggtacagccgtaatacctggtatcagtgcttctgcgatcagccaccatgaaaaaataaaatttgaaaaaatctttaaaaagatttggtagaaaacaaaagttgattacctttgcaaccccaacaacaacggggcaacaaacggaaagcgaaagttgcagaaaaaattgaaaaagatgtatggcaaaagagccacggagatcggatctcagacatcagcaatgatcatataagatggtcaaaagttctttgaaagattggaaacaacagcacgaatctaagtagtgatgcttaggttcaaacaggtaatgtacagctaaacataattaataaagatccgattgatttcgagagaaattagtcag

SEQ ID NO: 21 - DNA, 53863 bp, Chitinophaga pinensis
  source 1..53863: mol_type = genomic DNA
tcgagaatatatagaatattataataacgatagaatcaaattaaaactaaatggcttgagtccaatacaatatcgaactcaagccgcctaatcaaaaaagtctaaactttggggagcagtacatatattcgcttttatctcccttagttattattttaagaaaatctaaaaaatctaaaaaaatccaaaagtaaaaatccaggtaatccttaaaatcagcgtaatcctgagccaagacaaaatccgcgcattaaacttcgctccaatctccgcgtcttatgaacaggtttttatttatattcaatgaaataaaacctgttaagaaccatttaacctatggccgtttcacaggacgataaatcactcttggcattataccgtatacctgatacaaaggaaaaagggtttacccttattatccaaaagtaccaggaaaggctctactggcatatccgcaggatggtaatggatcacgacgatgccaatgatgtgctgcaaaacgtttttattaaggtgtggaaaaacctggaaaacttccgggaagatgcccagttgtatacctggctgtataaaatagccaccaacgaaagcctcactttcctcgagcagcaaaaacggaaaacgtcggtttcattgtctgatgtggaaaacggcctaagcaacaaactcagggcagatccgcagtttgatcccaataaactggagtggaaactgcagcgcgctatcctcagtttacccgataaacaaaggatcgtatttaacctgcgctactatgatgaaatgccctacgaggaaatgagcaaagtgctggaaacctcggaaggcgccctgaaagcctcttatcaccatgctgttaagaagatcgaagagtttatccgcaatggctgaccataaattttacaaatatttattttaagtaatttttaaagaattttgccaaaagattaaaatcacattaaactattaataccgtttactgtctaaaaaacagcaaatatgaacaggcagacctacataacaaatgaattaatgcaaatagcgccaggcaccaactggccggcagaagtaccatttacggtaccagcaggctattttgaacacctgcccgccgctatcctgctgcaaattcaactggaagatctgcgttccggaacagccgctgttccaaaccagccgccaactattcctgccggctacttcgaaggattaccacaggccatcctgcaacggatccaaacggaagaaggaaccagctccctcacctccgttcacacggaactggaagccatttcgcccttcctcgcggcaatacccaaacagacgccatttacagtacccaccggttattttgagtccctgcgggccagttccagccccgttattccactgcgggtagcccaccggaaccggaccgccacctggttgaaatggaccgtagccgcctgtcttaccgctttcatcggtagcagcgccctgctgttcgtgatcaacaacaacaaccatcataatgctatagaaaaacaactggaagacctgaatgaccaggatatcgttaattacctgcaaacccacactgatccctttgataatgaagctttcttcgccagttccgcggaaataaccccggtgcaaagtcagctgaaagaagcagttccactggaagccatcgaaaattacctgcaaaagaccgatttatcaaaggaagtgttacctgaaaataaatgatgaaacatctttactttatatggattacaatgtttgtgctcctcacccatgccggcgtgagtaaggcccagcaaaacccgtcggaaagtgccgccgaaaaaataaaagccatacaggtccaatacctggcccagaaattaaacctcaccccggaagaagcccagaaattctggccggtttataataattatacccacgaagtggaacaactgatcgcagaacgccaccagaaaagagaccaggaaaaattagccaccgacaacgccgatgatgccgcccggaaaaatatggacaaggaactgaaatacgaaaaacggatgctggacatcaaatcacgctacagtacagaatttcagcgtgtactccccggtagaaaagcaggcatggtgtttaaaagcgaaagagaattccggaccatcatggtaaaccacctcaatacccaacgcatgaacaggatgggcggaggcccaagaagacgaccataaaagaattacggggaactaccccgcaattcccccttactctattatttataatgtgcccttacttcactcaccagccccttttcattaatcaccatcatctccgtacttaatttatcattgatgcttttataataaagcacaatagaattcaccccttccaggatatggtataactcaaaatgcagatcaggataggcttccagcccacgggtaaagtaagccttcaggttctctttcccccggatacaaccggtaggatcattgttgattcttttaattaacggggaatagaaaataacatccgcatcgtaatgcgacatgatctcgttgaggttgtgggaattccaggcctgtagccaggcttcaccaattttggtcaaactttccattgtcgttttttttcacaatgtaagccatccgccggcacaactatttgcagaaaagatcagtttccattttacgccactgcaatggcgttactttaaaacagcggcgaaactgccggtaaaaatgggtcacatcttcaaaacccgtactgtaagctatttccgcgatcggctgttctgtggtgcgcagcaggaaacccgccatctgcagccgcttctccagcacccaatgcatgggggaactatgatagatatcccggaaacggcgtttcaatgtggccgtactcatatgccccatagcggccacgtcttccaacagccgcacctccgcaatcccggtactgagcttctccatcacctccggaagcgggtacatggccgctttggcaagcatggcacttattgcctcctcaccggaaataaggtgaagcgcgtgtgaaagtatgttgtaataatcaggtgtggtaagggtatcgtctgcaaagtggcgcaacagcgattgtgagaagtcgtgccaatggctgtttaccggcagtgtagttaatgcccggccaactgtatgagctttatttcccggctttttaagcaagtccaggatcatttcatccgggatcacgaggtttatacttccgtattgccgctgtggctgcaatatctctgagcaaagcaggcttccggccggaatcaccatcgcatccccgctgcgcaggtaatgtacctgcctgccgtcgtacattcttttctctccctgtactaccaggttaagcaccgtttgcggaatatacaactcatgcgtggcctgatcgcggtaaacgctatacgatgcccagttccggccctgttgctcccatgttttattggtatgctgtcctgtaagtgacaagctgtcaaacggcgtatacatcttgacatctcataaaatccaaaaaattccggtaatcagcaaaatcagtgtaatcctgagtaagacaacctccgcttaaaacttagcaaaaggttctttggtatcatgataaaaaaggaatgtccagccttcctgtttgccgcgctccaggaactcctggcggagctccatactgcgcttgccatcgtaatcatatttggctgcaaaccggcttctcatctgggatatctgtggcgccacatctcccccgaaaaatattttatctgctccatcatctaccagaaatacctggtgataaggacagtgaccaccggtcacttcgtaatgaatatacccgtcgatagtcccgttaccggttgtaaacaccacgttatcccgctgttgtaataacataatatcttcagagagataagatttgccggagtgctccacggcgtaaagcatttcctcgttgtttacataatacgtagccccggggaaattgagcgtgcgttctcccgtgataggatcttctgaagaaacgccgccggaatgatctttatgtaaatggctcatcaacactttggtgatttccattgggttgatgccattgtctatcaggtgctgatggatttgcagtacgccatcggggttacgaaagcccagcccggtatcaaataaaatataatcgcggtccgtgattacaaggaacggctgtatttcaaccagcaacgaaccatgcgggcgatcctgcatgctgtctgtccccagcttaaaaggaaaaaatttcttggtcccgtctacggtaaatgacccttctgataatggaataatacgtgccattttgcaaagatactatcttaacaccatctgccggtcggcatccagccgcaacagtataaatatcagcatggtaaaggtcatcagggaagaaccgccatagctcaccaggggcaggggaatcccgatcaccggcgcaagcccgatcgtcatcgcgatattaatagccaggtggaaaaaaatgatactggctaccccataggcatagactcgcgtaaaggtcgatcgctgtcgctccgccacaaaaatgatccggaaaagaagggctacatatatacccaggaaaatcacgcttccgaagaagccgaaatcttctcccacagtacagaagataaagtcggtgctttgttcaggcacaaaatcgtaacgggtttgggtgcctttcaggtatccttttccccagaagccaccggagccaatggcaatcatactctgcctggtattgtaagtagccttcggatcgttttccttacccagcattacttcgatacggcgtacctggtagtccttcagtactttggtaaatacaaagggaacgatgaacatcacaaatagtccgcagaaggcgtatacccccaggatcagcgcgagcttcgatcgctttcgttttatttcgcgccgcataaagtagatgaccagcgcggtgatgaccgtaaaaataatgaagagtatcgttcggtccaccaacagggccgacaacacgagtacaattcctgaaaaggcgattaccagcagtacgccgggcaatccttcgcggaacatcaccaggaaaaaggaaaaatataccagggccaatcctgtttcgtcctgcaaaatgatgataccggcaggtatcagggccaatgcagcggcaatcagtctggatcgtagtttcgtaaaatcagtttcctgtgacgacaggtatttggcgagcgccaggttggtacaaagcttggtcagctccgccggctgaaactggaatccaccaatcaccagccaggaatgcgatcccttcacatctttaccgatcccaagcaccagcaatagcagcaacagcccgcctgcgtacatcaggttggccgtagccgtaaaaaatttactgtctgtaagccatattactgcagccagtacaatggacacaccaaaccagatcagctgtctcgaatagtttttacttggatgaaggatatcctgccacacgttatcatcaccccggtattccgcagcaaaaatggacatgatgcctatgatcaccaatgccaggtacaggccaactattggccagtcaatcccttgtgtcagtttggcttgcgagcggttcattattgattaatcggtttattcgatgattggttaaggcttgttcttcttaataacagcattctgattcaatgaatccaaatgcgatttagccagcatggcctgatctattgttactgtttccattactgatttcaacagcggctgacgtttggtggagatactgtctttcaggtatttctccatcatcaaactggcaataggcgctgcatacttggcaccaaaaccggagttttccactatcacggcaatggctatacgtgctttttcagcaggagcaaaagccacaaacaccgcgtggttcttcagttttgttcttacaccgtttacaataccatagttttctgctgtaccggttttaccgccaacggtaataccttcaatctgcgcaatacgcccggtaccactttccaccacgtctgtcataccatgaataaccgcgctgtaggccgtatcagagatatgcgctacatcgtgcttttgtttgtatttatccaggagatgggtgttatcgttatcaatgctggctacaaaatgcgggatatagtaggagccgcggttagccacaatacacatggcattggccatttgcagcggcgttagcagcaattcaccctgaccgattcccaggaatacggatgtacacgagttccagctgcctttgtaccgggcatcgtaatattttttatccggtaccagtccgcggccttcactgggaatatccacccctatcttatgcccgaagccaaagttgttcatatagtcggcccacttctgcataccgcctaccttgatccccccaaacttacctgcatccacactcaaacggtatacatgcgaaaaataggagttacaggaatgcgatagtgccaggcggagattagccgcgtgaccagcatcgtggtgttcgcatttgataggtcttgagcagccgtagtaagcgccgccacaggggtatccgaagctgggggtaattacgccttcatcgagtcctaccagtgcgatcatgggtttaaacgtggagcccggcggataggtagcctggatggcacggttaaacagtggcttggtggtatctgtataaagtttgctgaaattggcgcttcgatacgaacctgtgagcaggttaggatcgaagctcggaccgcttaccatggccaggataccgcctgtttgcggatcgatggccacaatactgcccgatttgcctttcattaatttttcaccgagtacctgtaattcaatgtccagggaaagccgcaggtttctgccggctactgccgcactgtcaaactccccgttttcataagctccctgcggtctgttcaggttatctttaaccaggtattgtatacctcgttgccccatcaatacggtttcataggtcttttccagccccgtgaatccaagatagtcgccggagctataagaggcgtaagtaccagtatcctttaacatggccggggatatttccgctatatacccgagtatattagctgcggccgaataagggtaggagcggatttgcctgggtaccagttcaaatcccggctggaagagatacatgctttcctgtagctgcccgaatacttccggcgccagcaggggagcgaaaactgattgtcttacccggccatttttgataatggcggtaacgatccgtttcctgaattcttccttatctatttttaaaatattacagagatagcctgtatcgatgctttttacactggcaggggttactacgaggtcgtataatacgtcgttgccgaggatgctgcggttctgccggtcgtagatgataccccggcttggataaatgactttacgaagcacggcattggcatccgccagcttggcgtatttcttttccactacctgcagaaagaataacctggtgatgatcagtattaccatcccaagtataatcatctgtattactctcttcctgggctgattgaatactgacatgctattaaggacggaattattttaagttacaaacctacgttaaaaagcagaaactatttcttcgagaagaacagcaattcatacagcacaatcaggaaaagactggccaatgttgaagagacgatcttcatcaccaggtataacgggttgcccataccaaacacttccaacgtaaagaaaagtgcatggtgcaggaataccaggatagcggcatagatgagaaactgggacacacccatactggtcatcgaaggcgttttctgggtagtttcaaaacctccctgtggtgacaggatattgataataaacggacgcagataagcaatgaacacacaggcggcagcatgcatacccggcgtattcataaacatatccagggaaagccccatcagcaatcccaggagcatcagcccggggcgtggcagattaaaaggcagcgcaaggataaacagcatataaagataggggctcaccagctggtgcaacaatatttcattgagcacaaacacctgaatcagcagcaggagcacgaagcggattatatttcttaacagtatactcatttaatcaacttatacgttgaatcttccaatctttgttgttcttctttcaacaggttttctatcacgtatacatattgcaggttgaagaaattggtagccaatttcaaccggatagtaaacgaggtgctggctttgtctcctacggcaatgctttctacatagccgatcggaatattttcagggaacagggcagagaagccgctggtcaccacggtatcacctttatgaattttggcgcttttcggcacgtctttcagcagggcatagccggcgtcttcaccatcccagtgcacggaacccatttcttttccctggcccaggcgggcgctgatggatacagaattggatttagagagcatcgacaataccacggagtagttgtcgctcacacttctcaccacacccaccacgccgctgctgctgataacgcccatattaggacggatcccctgcaggctgccgcggtgaatagtaatatagttgacgggtttgttaatggagttgttgatcactttggcggagaagtactcgtaccggcggatctgcgtgccaacaacgcggtgggcggtatcatcactgtattgccggatggtgtcggttttgatcccgttggtggttatcatactgtcgtagctggtacggagcaggttgtgcaggcgcatgttttcattcaccaagctgtcgttggtcgacttcaggtgaaagtaatactgtacattattatacttgtcatataatttaccgctgatatcatttgcggaactgaggtaggcggctcgctgaaagttgttatgctggaataccaataccatacaaatcacttccagcagcagaaataagaagaagttaaaatatcgcctaaagaaaatgattagatttcgcacaagcgcgcactattttaggatttggttatccggataccctgtaattccctcccaatgggatgaataacaaaatatccggatcacaaatagttttattgcatcaggaacggatacttacctacatgctttaaggcaataccggtacctcttaccactgcgcgtaacggatcgtctgctacatgcaccggcaatttgattttttgggtaagacgtttatccagtccgcgcagcaatgcaccgccaccggtcaggtataaacccctgcggtaaatatctgaggccagctcaggaggcgttgtttccagcgctttcaggatggcttcttcgattttaaagatagatttatcaagggcttccgcaatttcctggtaagataccatgatttgcttggggatgccggttaccagatcccgtccgttaacaggaatatcatctggtgggttatccagttctttcagggctgatccgatgtggatcttaatctgttcagcagttctttcaccgatcaggaggctatgatagcggcgcagggcttccatgatatcagccgtgaactcgtcaccggcgatacggatactctggtcgcaaacaatacccgccagtgctattaccgaaataccggtagtaccaccgcctatgtcaatgatcatattacctacaggctcttctacatcaatgccgatacccagggcagctgccattggctcgtgcaacaagtatacttcctttgcgccggcctgttcagcagagtcgcgtacagctctcttttccacttccgtaatgctggaaggaatacagatcaccatccgccagcttggtgcaaacaagggctttttggggtaaaccatttttatgagttccctgagcattccttcagcggcattaaaatccgctatcacgccatctttcaggggacgtatagtacgaagatattcgtgtgttttttcgtgcatcatcatggccttttttccaactgccacaattttgccactagcccgttctatcgctacaatggaaggctcgtccactaccacctggtcattatgaattatcagcgtgttcgctgtaccaagatcaatcgcgatttcctgcgttaaaaaattaaaaaatcccattgttgatacggtcaaaaattagaatgcaaaaatgaataattccaacgaatatacgatgcaaaaaatggatattcttgcaataatacagctaaatattaaaaaaagttatttgttgtacaaacggcatagtaactgctctctttatgctccgaccagatgaacgggataaccccgttttaattgttcctactgcctaaaattgtgcctttacaagtcccgcttttcaattgtcctgtaccagtcctccctactgtaaattaactccggctaacgtctaaacaaattcgtacccgatatccctgcggtataccttaccatcaaatgcaatctgctccgctgtttgtacagaatgagccagtgccatcgacaggtcagacgccagtgaagtaatggctaatacccggccgccgttggtcagcacctcatcgccttcctgccgtgtaccggcatgaaacacgatctggtcgcgggtaggcgccggaattccatggatcaccttattcttttcgtatgcttcgggatatccttttgataccagcatcaccgtagcagcggcacgctcgtcggcgtaaatcgtttgcccgctcagtttgccggtcattactgcagtaaacagttccaacgcatcattcttcaaacgtggcatcacaacttccgtttccggatcgcccatacggcagttgtattcaattacaaagggcgaaccctctacattaatcaggccaaaaaacacaaagccatgatacacaataccttccctggaaaggcctgctatcgtgggccggatcacttcatcctccacttttttcataaacgctgcatcggcaaacggcaccggcgataccgcacccataccaccggtattcaacccaaggtcaccttctccaatccttttataatcctttgcttccggtaatatcttataggtatgaccatcggtgatcgcaaatacagacaactcaatacccgtcaggaactgctccacgactaccgttttactggcatcgccaaacttggccgacttgatcatctgctcaaactcctcggccgcctcttcataagaagttgctatcaccacacccttaccagccgccaggccatcggccttcaatacaattggtaaggagtgctgctgaagataggccagcccttcctcataattcttttcactgaattcacggtaagcagcagtaggtatattgttccgctgcataaacagcttggcataagccttactgccttccagctgggcgccttcctttgaaggacccagtaccgggatatgctgtaacagttcatctttctgaaagaaatcatagatcccgtttaccagggcctcttcagatccgggcaataccaggtctatcgcattatccaggcaaaaggtctttatcttatcaaattcacttacacccatgttaacgttcgtgccgcattgagcggtaccagcattacccggtgctataaatagttgaccgcaaagagtgctttgtgacattttaagggccagtgcgtgttcccggccaccacttccaagtaatagtatgttcatatgaattgcctaataaatgcagatgcgaaagaaagtgcaaagaaagatcaaaaaaccgcaaaaaatgagcatttataccatttttttacgcagattaacgattttatttaacttgccatatttaaaggttcacgaaatctgaaacaactattgctaaaactaaccaatttatgatgcaaactactgttgcacaagagtcccctattgcctctgagaagggccaccctaaagggctctcagtattatttgccacggaaatgtgggaacggtttaatttttatggtatgcgggcgttacttacgctcttcctggtaaatgcactggctttctctgaagcagattcctctatcatttacgggggctttctcggcttatgttatctcacccccatgctgggaggatacatatccgacaggtacctcggtaacaggaactgtatcatattaggcggttttataatgggcgttggccagctccttatggtcctcagcgccaccatctatgcctccaatgtggaaacagccaaaaccatcgtttggctcgcccttttcatcatcatctttggtaacggcttctttaaacccaacatctcttctatggtgggccagctgtatccgaaaaacgacggccgcctcgattccgctttcaccatcttttatatgggtatcaacatgggcgccttcctcggaatgctcatttgccctatcctcggcgacgtaaaagtagacggcgtgagaatggtcagcgctttcaaatggggcttcctcgccgccagtatagccatgttcaccggaaccatcctgttcttcttcctgaaagataaatacgtggtaaaaccaaccggtgaagccatcggcgccaaaccggatttctccaaagtttctgccgtaaccggcgaagccgataaagccaaatttacaaccagcgctatcctcggtgtactggtgttaatggtggtactgttcttcggcatccactacctgtcgctcgatcccaaccccatcaaatcatgggtgtatccttttatatatgcagccggtatcagcctcgctgtactgatccttaccgataaatctattaccaaggtagaaagacaacagatcaccgttatctacttcgtggcctttttcgtgatcttcttctgggcctgcttcgaacaagccggttcctcccttacctttgtagctgattaccagacagatcgccgcctcttcggctgggatatgcctccttccttcgttcaaaacgccaactctattttcatcatcgtatttgcattgcccttcagctggttatggctcaaattacagcaacgcaacctggagccgatctccccgatgaaacaatcacttggattggcattactggcgctcggattttttatcatcgccatacaaatgaaaaatctcggacctaatgagaaactgggcgtaagctggttgatcctgatgtatcttttccataccctcggcgaattatgcctgtctccgataggtttgtcactggtatccaaactggcgcctcaccgtttctcctccctgctcatgggagtttggttcctcgccaatgccgccggttacgcactggccggcaccctgggcgcattgctgcctccaaccctggataaatacaaactcgctactgataacggtattgacctgaaagctatcctggatggtaccatcaccgctaccgcacagcaaatggataaattacaggaacttaaactggctacacattacccaaccttcgcaggcttcaccatccacaacctctatgagtttttcatggtgtttgtaatcctgccaggcgccgcagcggtgctgctgttcctgtctaccagcttcctgaaaaaatggatgcacggtatcaggtaagtcaaccttattataaaaaggaaaggagggaagctgataactttcctcctttccttttttaaaagtaaattcattgcttataacatctctacctgtaaatccataaacgatcttatgtccgataacaacttcaaaccctttgtttcacccggcgtacaaatgaaagaatttacgctgaaatccattttgctgggctgtgtctttggtatcatcttcggtgctgccaccgtgtacctggcgctgaaagcaggtcttaccgtttctgcttccattcctattgccgttatcgctattaccttagggagaaaatttttcaagaccaccattctcgaaaacaacatcatccaaacgaccgggtctgccggcgaatccatcgctgcaggcgtggtattcaccctgccgggattcctgttcctcagtgacggcggcggcacacagttctttaattactttaccatcctcatcctggccatcttcggtggtatcctcggtacgctgatgatgatcccgctgagaaaatcactgatcgtaaaagaacataaaaccctgccttatcctgaaggcaccgcctgcggtgatgtgctgatagcaggagagaaaggcggcgactttgccaaaaccgccttctacgggctgggctttgcttttgcctatgccatccttcaaaagattctgcatgtgattgccgaaacaccggaatacatgaccaaacaggccagtaaatttttcccttccgccaaactcagcgccgatatcaccccggagtatatgggcgttggttatatcatcggaccacgcattgccggagtactggtagccggcggcgtactgtcgtggctggcactcattcctttgctcgcatcattgctgccggcagatgtgatcgccacccagctggtcaaaataggctacctcgctaatttgcaaacaccgggcgggcagggcgactggaacccgctcacccatacttttgcagattattcttccgctgtttattatgcatacgtaagacaaatcggtgccggagcagtagcagcaggcggtttcatcaccctgctgaaaaccatccctactatcatttcttctttcaaaggaagtatcggcgctatcaaagatggctcgggcaatacagacgagaaaggaaatgtacccagaacagaaagagacctcagtttgaaagtagtgctgttcggcagccttgccctcatcctgctgatggctttcttaccacagcttccaggtgattctatcggcaaaaaattactggtaggtctgctggtagtggtgttcggcgccttcttcgttaccgtatccagccgcattgtgggcctcatcggctcttccaataatcctatttccggtatgaccatcgccacactgatgggcacctgcctggtattcatcgcagtaggctggaccggcaaattatatgaaccaatggccctggtggtaggcggtatgatctgcattgcagcggccaatgccggcggtacttcccaggacctgaaatcaggctacatcgtaggcgcaacgcccatgtaccagcaaatagcactgttcattggcgccattgtatcgtctgtggtgataggtttaacagtgaagttcctggataagcctacggcagatatgattgcgcacggggttactgaacacgcaatcggcagcgcatactatcctgccccgcaaggcacgctcatggctacactggcgaaaggtatcctttcatttaacctcgactggcaatttgtattggtgggtgtgtttctggcgataacgatggaactatgtaatattaattcgctctccttcgcagtaggcgcgtatcttccattgtccactacattgcccatctttgttggcggcgctatccgtggtgtggttgatcacaaacaaaagaaagccaataaaaaattatctccggaggaagaagaactgggcaaaggcaacctttttgctacaggtcttgtggcagggggcgccgttgccggcgtgatcatcgccatcctcgcaggtttcgactggtcggccgtcattcttgccaaactcaatagccaacagctgctcacaaatatcctcgggccgggtgggtactacataataggatgcgccttttttgcgtttatgggctggtacctgtaccgcaccgcccgcaaagcctagatccaacttttcaagatcaataccgatgccggtaacagggtgtaacaatccattaccggcatccgtttttattttttaaatgtttaatttagccgggattaattaaaactgattataatataacctatgcgcatattagttaccgcaatgctcagcgccattgttttactgggcatctcctgcggcaaggataaagatgatagccgccaacgcagatttatatcattgaagctggacgaccgggtttatctttcagaaaatccaaaaggcattatcaccctgccaaatcttacggatgaaaacccggacaatgattatcctactatggaaatcaccggccagagctataacggggatgtgatcacctttagcttagctaccgcatccatgcccttcaaaccaggcgtatatcccgctacccagaaaggaaacggtttactgattgccctcaacagcacttactacaccaacctcacctctgcaggaagcactgattttcaaatcaccatcacgcatatagacaacctcaacgtagaaggaaccttttccggaacactcaaagacgccagcggcgctggcggaacacgcgttgttaaaaacggcgcgttcagagcgatgattagtcaacagggccagtaggcggagggatcgccttcggcgattttaaattgtcttggagcaggattacgctgattttactgattggcttgatttttacttttggattttataaaggattaagggagatataagcggatattcgcttttatctcccttaattattattaagaaaaatctaaaaatccaaaagtaaaaatcaagccaatcagtaaaatcagcgtaatcctgctccaagataatttaaaagcgccgaaggcgctacacaaacgacaaatgcgggtacgttgccttcagcaccgccttgtcatcagcgcccagccagttggatagcagcgtggcgtatacgcttttgaagtcaacctggtattgcaggtccccgtctttcaggttaagcaggtctggaccatcattgataagtccgggttgctttaaactgccgcccaccaggaacatattattcgcggtgccatgatcagtacctccactggcgttctgacttactcttcttccaaattcagagaaagtcattactaccacatcttcaaaacgatgattcgctttcaggtcatctgtaaatactgttaacgcatcgctcagctggccaaataaacgggcttgctggtcctgctggtttacatgggtatcaaaactgccatgcgacacataatatactttggtattgatatccgacatcaccaggttggcaatggtgcgcaggttccttcccagctctgtattgggatagggggcagaagatttatatgttttaaactgttgctggatataggctgcggaagaaatggtttcacccatcgttttatacaggtaatccgcattattatgatgatcgttatcaggagtatgttgctttaaaagctctgcaaaatatttatcattactggtgccgtaaagccttgcagggtctgtcatggcaaggcccttgtcgctgtcgcctttcagcgccaggctcaaggtatcatctatttccagcgcctgtgttggtttatcgcatcccttgcattgggcgtcgagataacggcctatccagccatccgaccagtactcgttcgactggctcgcggaatgccagatatccatggaccggaaatgcgagcggtcggggttaggatagcctacgttattgagaatacccagcgcgccgtcatcatacagggtcttcaatcctttcagtgcagggtgtattcccaggtcgtcattcagggaaagggctgcctccctttttatgcccagcgccgggcgcgccttataataaatatcgttgcgatagggaataactgtattcaatccgtcgttaccgccggatagctggatgatcaccagcactttgttgcccgggggcgccagatgccctctttccagggctttcaggaatttcggcatcatcaccgcggcagaagccagtgaacccacctgtaaaaaacgacgcctgttgagaatcagcatagcataacttttagcggttagtagttaacacaattgatattccggtgtactcatcacatcaattgttaccgttttaatatagttttcgcggctgctgctatcagcatatttttccagcagctggcggcttatattaccgggctgctgtaataaaacaccggcaatttcatcggcaagccgctctcttggcaccttttcgtaaccagccacgtaagggtcccaatttatatttgcgttcaccttctttgcgaattgccgcttcaggaaatcattgatctgcagcgtcattttatagttagcaccttcgcccatttcaggagtcagctctttaggcttcacattaaacgcctgcgagtataatattacctgtggcacacgtagccggaacatcaggctggagctgtcgatccagttccgcccgccaggccagccggcaacattgggcggataaaaaagcaactgacccaatacccgctgaaacaacaacatcacttcttccttttcaaacgtcatggggatagttctgcggatgcctgccagcaattccacgggcgattttatccggttgccaatgatatccggactgtaaaaccagtcggccataaatatttcccgcatcagggatttgatgttgtaacccgactggtaaaacttttccgacagcgcggtaatacgtgcttcatcaggggtttcagacacaaaatactggtatatttttgcggtaatgaacctggcggtatgccgttgctccaaaagtattttcagtacatcatctccattaaaatttccctgtttgcccaggaaatttttcacaccgtcgtcatgctgtttttgccggaaaacaaaagtgcctgtttcatcaaagccccatccggtaaaggctcttgccgcttctttcacatcctgttcggaatagttgcctcttcccatcgtgaacagttccatcacttcgcgggcaaaattttcgttgggatgttgtttacggttctgctgattattaagaaattgcagcatagccgggcttttagataccgcaccaagcagatctccaaaattgccgagtgcattttcacgcactaccgacaacaactgctgattaaataatacattttgcgtacggcaggcgaaatgcccatgccagaaaagactcattttttcgcggagaggatgctcgctctgcaccatggcatttacccaggatacattcaggtctttaatgccctggtcattcatttgccgcacacttttcttttcctccggcgtcatcgttttctgcttccggtaatccggaagatcatctgcggctactacatccacagaagtaactgacgctcttgcagggccgataagtatcttattcacaattttttcccgccttttgctttcccagtgagagatcacggggagggtttctccaaagccagcgcgccaggcgagatgttgcatctgaattttacgggcaacttcagccataagcattaatttatgatgagactatcaaatgcagaacgggtttaaccaatgaaaggcttctcacagaaataattaccgggaacggttgttaacggaacctccacacctggtaactgcttcctttctcaaaaacactttcttccaatggcagggtgagaaaagcatctgctttaagcaaactggccagatcgcccgaaccctggtagggctgcggtatggccagcagcacgccattgggttgtgattgcagctttaccggcaaataatattccaatgcggcgtcaaaaataactttctccgatagctgtgcatagcaaggctccggtaaggccgctcccatagctgattgtatccacgcgtgaatgtacctgtaaaaacacataaagcccgatacggggttgccgggtaaggcaaacacaacgggaccgtcattaaaagtaccaaacaggaacggcttgcccggccgctgctgtactttgtgaaatacctgttgcattcccagctgttgcagcacagcaggcaggtagtcaaacatgcctgcacttaccgcaccggagctgatccaaatatcggtttcgtccagcagtggctggagctggtctttcatggctgcttcatcgtccaggaggtgtacataacgggcaggaacacccatttctgccagtgaggccaacaggctgtatacattggaaatgcgtacctggtgaggttccggcgtttcgtgtaccgctaccaattcatctcctgtagcaattaccaccacacgcgggcgcttgcttacttccaccgtggtctggcccactgtggccagcacaccggcttcagccgggccaatacgggtaccgggtttaatcagcaccgtgccggcatccacatctgaaccttttttatgaatattctgtcccttcttcacggcgccctgaatagtaaaacgccggaacccttcgtgttccgaaggtgtaaggtgttcatactgaacaacggtatctgtcatttccggtaaaatggcgccggtcatcacttctatacaattggcagtattggaaagctgcagctgcggagtgcctgcagcctgtacatcttccacgccaaaaatatgctgcccgcgggcaaagctgtcgtagttaacagcaataccgtccatcgttacacggtcaaatggcggaaagggcctgtcggccagtacaggctcccgcaaaatacggccggcagcggattcaaacggtaccgtttccgtaccgaggtcccgcacagtttgcatcacagcctcaaatgcagcagcaacagtcaacatcattttgaattacttttgtatcaggtgaacttgtttaaatttatgcttttatgtccaatgaatcaagtaatgctttttcacatctgaacgagagcggccagcctgcaatggtcgatatcagcggcaaactggatacttatcgtatagccgttgccgagagccgtgtttatctcccgcaggtgatacgcgaccagttccagggacaggacatccaaacccgcaaaggtggcgtgtttcaaaccgctatcatcgccggtattatggccgcgaaaaaaacaccggaactcatcccgctttgtcataccttactgctggatggctgcgatgtacagattcacctcgaaggagaagaagccattatccgctgcaccgtaaaaaccaacggtaaaacaggcgtggaaatggaagccctcaccggcgccagcgtagctgcacttaccatttacgatatgtgcaaagcgcttacccaggatatggttatccgggaaacaaaactcatcagcaaaacaggcggcaaacatgactataaccggtaataaagcgccactgaaaggactggtgctctgcggcggcttcagcacccgcatgcaggaagataaaagcagcattaactatcatgggatgcctcaatggcaatacctggttactttactgcaatcgttgctgccggaagtatacatttcctgccgtggcgatcagcaggaacattttgccggttaccctaacctggtaccggattcggtgccttttggcgggccatccgccggattgctgagcgcacacgcgctgcaaccggaagcagcctggctggtgcttgccgttgacctgcccctgctcagtaaacaaagcctggagctgcttatcacccaacgtgacgtcaccaaagcggctaccacttttgtgagtccggtcaacgatttgccggaaccactcattgccatatgggaaccagctggtttaattgcgctgttggaaaatgtaaccgccgggaaaaactgcccgcggaaaactatgctgagtaacagcatcgcgcttcttaaaaatccatatgcagcagaacagtttaatgccaacacgcccgaagaaaaggcggaagcattgaaggacctggagaaataagcaacgggatattattcaatcattgcaggactacacaatttcaccatctgcaaaaaactcctttttccagataggtaccgtttctttgagggtgtctatcgcaaattcacaggcgtcgaacgctatgccccggtgagcagaagccactgctattaccactgcgaggtcgccgggatacttatccccaacggcatgcagcatggccaggcgctgtacatcccatttttccgctacctgcgccgctattttctgcatttcagaaatagccatcgcctcataacattcgtaaaataattttaataccggccgttgtttggtgtgattacgcacagtaccggcaaaaattacctctccgccgcattccggcgcctggatgaaggccagcgcttcctccacggtaatggtatctttaatatctattaatatttccatctcttaaatactaaaactgaaactatactcaacctccgcttaccggcgggatcaccgcaatttcatcctggccgcttatctcctgtgtatcagcagcatacgtccggtttaccgctatcatcacggaacggagctgctgcaacgacggatatacctcatacaaccaggctttcaaagtggctacatctgtaatatgttccggcttttccagtaccggcacaccagcaatatcctttgctgctccaaacaataatatgcccatacattgtaaattgttagttaaaactacaatatagcccgataaagtagtaattttaatacggcagaaaatcaatttatgaaaatacggttaagaggcaacagcataagatatcgcctggataaagcggatgtggaactcctggaaacaacaggaaaagtggaatcaattacgcatataggcgccggtaccctccatttctgcctccggggaaaagatatttccgaccccatcataaagatggaacacgatggtgtacacctgctgctcccgcttccccgtcttgctgcctggtacgcacccgaccaggtaggttttgaactgatcctgcccaacgccgatggatcatcactgactatcctggtggagaaagattttaaatgtcttacagacagaaatgaggacgaaagccagtcattcgataatccgatggcggggaaaaactgctgataaatgctaacagatgcacatcatcgtatcatagactacgtacgcttgtcggtaacagaccggtgtaacctccgttgcacttactgtatgccggaaaatatgcattttgtgcaacgcaaggcattacttacggacgatgaaattttacggctgctgcaaactctcgcaaccgccggtatctctaaaataagaatcaccggtggtgaaccttttctccggccgggcctgatgaccctcctggaaaaaataaaagccattccaggtatcagcgaaatagctatcaccaccaatggcgtcttaacacaggcatatatccctgctttgcagcaacttggcatcacgcatatcaacctgagcctggatacgctgcaagccgaccgcttcctgcaaatcacccggcgcaaccggttttccgcagtaatggacaccctgcaaagcctgctgcaacacaacatgcaggtgaagatcaacgccgtggtaatggaaaacgtgaataccgatgaactaaatgccttcaccgcacttacacgtgataatgcactgtccgtaaggtttatagaagaaatgccctttaacgggcagggacatacgttttcaggtatcgtatggaactatcataaaattttgtctgtaataggcgagaattatacgctgcaaaaaatagcggatgcgccacattccacttctctcaattatcacatccccggccataaaggcaatatcggcgtaattcccgcttatagccgcactttttgcggcacctgtaaccgtcttcgtatatccgctaccggtagtatgaaaacatgtttgtatggcaacgatgtgttaaacgtaaaagagatgatgagagatgaactgcagcaacaccttctgctgccggccatacaatcagccatccatgcacgttttgccaatggcttcgaagcagaacagcatcataccgaaaaaaatatggaaagcatgtccgtaataggtggttaactattatttacttcagcaacatctgcacacccgcatacaggatcagcaacgccgtagcaccagccacccacctgggattcaacactctcgcactcagccgcgcaccaatctgtccgccggcaataaccgccagcagcaaaggccctgcaaacttcacatcaaacacaatggcatgctttgccgcctgaccgcataaaccggcaatagaatttacgagaataaaaaaactgctcaagccggcaatatttttggcggtgtcgtatttgcccaaacgcagcacgggcgaaagatagatgccgccgccgattcccgtcataccggagagcaacccaataccgccgccaataatcccatacgctacaccattccctttattggcagggataatcggctcttctttctcaaaaaacaaacggtagcacatcagcaccgccgccagcgtaagcgcaagtcccagcaacaggaaaaaggtagcctgcttcataggtaagtaactacccgcaaaagccagcggcacgcttaccagcgacaactgccacgctttttttaaaggcaggtggccgcttttgtaaaaatgataaacgccgccggtcaccactgctacattacacagcaaagcagtagacttcatcagctgaaaatctactgcccagaaaggcaacgacaaaatagccaggtagctggaaccgccgccaaaacctgcagcagagtaggccaatgccactataaaaaagaggatacaaagttcagggatcacggttaataggtttgcatctggtgatcaataacactggcccaggcatgaataccgccttccacattgtatatacggttaaagcctagttccgttaaacgttgtgccacagcgcgacttcgcatgccgtgatgacaaagcaccgctaccggcacatcatcagggatagctgacacctgctgtaatacacgccccatcgggatatgcacggattgcggaatacggcagatctcccattcatcatcttcccgcacatccagcagcatgaaacgggtatcccgctgcaaccagtcgtttaattgctgcacagataaagattgtaccccttccagttcacaaacagtttgctggtagtttgcctgcagggccgtgatttcccggttggctgctaccggggtgatattaaaggtaagatgggtattgttcagggtgtcaatggtcatcagttggttgcgcagcggtgtgccgataccggtaattactttcactgtttcattggccatataacagccgatgatacctggcaaaacgcccagcacgcctatgtcgttgcagttcagcatttcgccgctttccggcgcctccgggaaaatacagcgataggtggcgccctcctggtagttaaatacgctcagttggccttcgtatttatagatggcgccgtataccagtggtttgccggtaattacacaggcgtcgttcaccaggtagcgggtgccgaaattatctgaaccatccacaatgacgtcgtattcccggaaaagcgccaatgcattatctgtagtgagccaggtgtcatgtatcacgtgggttatctccgggttcagctgctgcagccgttttacggcctgttctaccttggatttcccctggtcggcggtagtatataatacctgtcgttgcaggttggtgatggaaacaacatcatgctccacaatacctattttcccgactcccatggaggtaagatattgcaacacgggtacaccgaggccaccggcgccgattaccagcacttttgcctgttgcagtaatgcctgttttgcggagccaaatccttccagtcttgtttgcctgtcatatctgtccatactgcttcatttagacactaaaattaattgtattcgggagaagttttccggtgttttttgggagaaggatttcctacacctccggggtgttgcaggcagcttgtcagcgttttaattccaggtacatggttaccaggtctacataactgccgtctttctgcctaatgccattgggcaggcggccacattccatgaagccgaaattgcggtacagctgcatggctttttcattggtggaaaaaacatgcaggtaaatcaggcgcagtgcggggcgcgattcagtccaccgcagcatggcggtgagcaggcgccggccgatacccatattgttccattgcttttccaccgcaatgcctatttccgcggtatgcgcttttttatgcaaaccggtgtggtttacgttgatagagccaatgatctggtcctttacaacggctaccagcaggagctggttaggattatcggtgtaagactggatataatcctcttcagacgcaatgtccagctccatggattcactgcgggtaaagagcaggtaatccatttcccgggtcaggcgctggaaactggccagcagcgctgctgcatcattatgttcgggagggcgaatgatgagttcgtcgccggtgggcaggaaatgtttcataatagaataccggtggaaattacgaattccaaacgacgaatgacggatttcaggcaattgttagcgggcattactccgtttacaatctccctgcgaatccgtcatccgttaaagattatccgtaatggcttatatcttgtggctgccgaaataggtttgcagcacggttggtatctgtatgccttccgcggtttggttgttttccagcaggcaggccatgatacgcggcaatgccagggaacttccgttcaaagagtgcagcagctgcggcttaccattgttttctttgaaccgtattttcatgcggtgggtttggtaagcttcaaagttgctcacagagcttacttccagccatttctgctgggcagcgctgtatacttcgaaatcgtaggtaatagcagaagtaaagcccatatcaccggcgcataaacgaagaatgcggtaaggcagctccagctggttcagcaacgcttctacgtgcgctaccatttcatccagtgcctcataagatttatcgggatgtaccagttgcacaatttctactttatcaaactggtgaacacggttcaaaccacgtacatctttaccataggaaccggcttcacggcggaaacaaggcgtatacgccgtcatcttcactggcaggtcggtatcttttatgatctcatcgcggtaaatattagtcaccggtacttctgcagtgggaatgagataatagttatccgccgttgcatgatacatctggccttctttatccggcagctggccggtgccataggcagatgcttcgttcaccaggtatggcggcgcatattcagtatagccgttgagggtattataatccaggaagtattggatcagcgcgcgttgtaagcgggcgcccctatttttgaagacaggaaaaccactgccggtaattttgttacccagctcaaagtcaatgaggtcgtactgtttggccaggtcccagtgtggaacggcgcctgcatacaggtcaggaatttttccacccttgcggatttccacgttttcttccggcgttttaccggcgggcaccatcgcagcgggcaggttaggaagtttcaccagggcatcctgcaatgctttttcggtggcattcagctcttcattcacagggccgaggcggtctttcaaagccgctacagcagcacgctgcgcttctccttcttcctttttcccctgggccatcagtttaccgatttctttggataaactgttcacctgggcctgtgtttcatcgtattcgagggttaacttcttgcgcttgtcatccagcgccagcacttcttctactacttccagctccttgaaattcttaaatgccaggcgctccaataccaactctttattttgacgtataaacggtacttgtaacatgttgtatgatcaaattttagcaaatatattaaaatagcttaactcaggtacttcccgacaatgggcactctgcggcctacaccaaaggctttggaggatacccgtataatagggcagaattgatttctcttgtattcattggtatttaccatctttaaggcccgcgaaaccaatgcagcatcgaagccctgagcaactatttcgcgcggtccctgacggcgctctatgtactgataaagtatcctgtcgaggatcgcgtagtccggtaaactgtcgctgtccttctgatccggccgtagctccgcagaaggcgctttgtcaataatattggccggtatgatctctttctcccggttaatatatcttgccagtgaatatacctgcatcttatacacatctcccaaaacgctcaatccgcccgccatatctccatataacgtaccataaccggtagacagctcactcttattggatgtattcagcaggatataaccaaacttgttggataagcccatcagcaggttaccccgtatgcgcgactgcatattttcttctgccacattaaatggcaatcctttgaaataaggctccagcgtggttaagaacgtttcgtaaatgttgttgatacggataacatcatgcgggttatccaggttttcggatagcgctacggcatcatctacagagtgactggtagagtagggagaaggcatcagaatagcccgtacattttccttacccaacgcatcgcaggcaatagccagtgtaacggcactgtcgattccgcctgaagagccgaggatggcctttgtaaagcccatcttaccaaaataatctttaattcccaacaccagggcatcatagatgcgatcaatattatggtcaaacaccagctcggtgagcggcgtaaaatcaacaggtttcactggtggcaagtggctgccaaccagcttttccaactccatgccgcccatcgcttcttcaaagtaaggcagctctttcactacattaccctgcgcatcataaataagggagcctccgtcaaatacaatttccgtttgggaacccacggtattgcagtaatacatcgggatcttatatttcaatacattggcgagaataatttctttgcggtcttcatcatgatcataatcaaacggagaagcggagaggttaatcatcacatccggttcctgtgcaattagctggtccatcgggcaaacacggtacaggggattatctcccaggttccagatatcttcacaaatggtaacagccagctttttgcctttaaacgggatgatattccattcaatagacggttcaaaataacggtattcatcaaacacatcataggtaggcagcagcgttttatgcaccacctgttttacttcgccttcatataaaaaccaggcggcgttaaacaggtctttgccctcccgttgcgggttgcgggccggaccgcccaccagcacggcgatatctttggtatgtgcttttataacatctatcgcatgatagcattgtgcaataaaatcttcaaattcaagaaaatcacgcggaggataaccacatacacataactcggaaaacactaccaggtcggcgccctgcgcctttgccgcatggatgccgtcgatgatctttgccgtattcttttcaaaattgccaatatgataattctgctgtgccagtataatattcatggtaaaaatattcaattaaaaaagagggaaaactagaaaaatacaccaagccggagagcaaagctattcatattcacccttccgtcgtcccatttgccgttacgggttacgtccacaaaaccgttctggtaggtaatgcctgccataccagtaagattggcgcccagcggatattctatgcccgctcctaataacatgcctatgttgatacggttcatttggggtaagatattcaccttatcataggtttgccccatcgacactacatctgcgcggccggtgataggaaaatccaggtaggtgccaaactgtccccagaaaccgataccaccttcatccggcaaggttttcagcttcaatgccagcggtatttctatataggaaagcttcatattatactcagcaggattggctttataatcgcctaaacccttacctgcatcatatttcagcttgctgccggccagtaatacctggaaccccgacgaaaatgcataagtaccttgttcgttcagcttaaaatcggccatcagtccgaagttcaggcctgctttggcactgttcctgtttacgcccgattcctgtggcttcaggatggaaaccatcgggctcacggtaaatccaagctttactttttccctgaaagaattaccgccatattgcgccatacctgctttcgccactcccattatcgccagtaaaaagatgatcttcttcatagatgatgctaattcgtaattttttataatacaaggtaaataataattttaccttagatgagttttaagaatgatgcaaagttacattaataaatataccctgctgataagttgcgtggcagccctgctgggtaccgcagcctgtaattccggtaataaagcgccggacgttagtcatatagccatgaacgttagtttatcgcgtttcgactccgccctgtttactattgataccaataatatacaacccggactggcaaagctgcatgaagcatacccggtattcctgcccctgtatattacggatatccttaacctgggcgcgtattccgacagcaacgcagcggtacagcaacaactgcacctgtttttaaccacacccgatttccgccagctggaaaaagcagtatctgccaaatacggcagtcattccacactgaaaccagaactggaacagtgtttccgctatatcaaatactatataccttctttccgtccgcccagagtagtcacttttatttcgggtatcgccaactatggcgctatcacagtggattctatcctgggcattggtttggatatgtacatgggagaagattttccaccctacgcacagatccccgattacccggattatatggtgcaccggtttgcccctcaatacattaccaccaactgtatgcaggtaatccagcaacagttgtatccccctgcgcgtaaaaacgggaacctgctggaacagatgatggaggccggtaagcaacaatatttcctggacaaagtattaccggaaacaccggatactatcaagctgggatatacgaaaagccagctggactggtgccgggaaaacgagcgcatgatctggcagttttttgtgcagaataacctggtatattccagcgactggcagcagatcaatcattttattggcgatggcccgtctacacagggaatgcccgagggcgccccaggcaaaattgccaattttgtgggctggcagatcataaaaaagtatatgagtgaacacaaggatgtgaccttgcagcaattaatggagtcaaaagaagtgacggagatcttcaaagcctcgaagtacaggccctgagaaaggattacaggctaaacgaaaacgggtattaattcagtttaaagggaacgaccatctggaactcaggaattttcacttccagtattttcttgtccagctggttttccatttgataagtaccgtacatcttgccgatctcagtccgtaaattggatcccgagacgtactgataagtttcacctggcgccagcagtggttgaacacctacaacaccttctccttctacttcacggtgtgtgccattggaatcaataatgtaccagtgacggcgaagcagtttgatagggaaaatgttgttgttctcaatggtaatacggtaagcaaacatgaattcgcttccaataggatttgaataatccggctggtagaatgtttccacgctgatggtgatgccctctgttaccttcttaaccataaaatcaacctttaacgtaaaaataagaaaaataaaaccagtggctggaaattttctgactttaacgattctttagactatttcaatatcatccagtatagcaggatcttcctctgaagccctggcggccacctctaaagcgttattatagtagcccctccgcaggtattcggacaaatatctccataaaaatccaaaaaagcccagatgctggtattgtttgatatgacaagcttcatgccgcatccaggctgtatccgctaaaaagcgttcccgggacgccccatgcaagtggatggtgcggcccaggaccatggctacagactgcacccgcatgaagcgggcggctgttttggctaaccatgaattttcacgtatgcggcattttattttttccaatctttcttcccgaataacgtaaatctacgggaaatattgaaaccccaacggaattggccctgtaaccaggaagtagtggtttcaggaataaactgactttcctgtatggcagtggagttggtgaaagtaatgctgaatacgtgacccccggtttctatttccagtccgacggccagcgggttgtaaaaagagatgcccttcgcagatttgaaatagtctttgctttcctgggaacggaacggataatagtattctgccagaagtcccatccttttgctgagcttcagcctgccggccgctcccagggcaaacatattattcatgtccatgtatgccacgtggttacggtgcacgtaagtaggcgacagggtaagtgataacttgtcgccaaatttcctagatacaatagcctgggccacatacataagccggtcggccccgtcttcaaaataagccgccgaggttttatccgtggcagaaggcatcccgctgataacggcgttaccaaatacggccagcgataacgggatatggttatcagttgtttgctgtaaaaaacggtacttcaccagtccttcgtacaactgctgcaaatccccgctgcccttagtccggctgatacccaccatgaggtcgtcgctcaccccatattcaaaagcaatgcggatatcggttgaattatctgtaccgaaaaacgttttggtaccgccaaactcaccaccggcatcgccgaaacggtgggtaacacggaaatccagttcgtgcctgcgcagcatttcggtcgactgcccctgtacaatgcgggtacttttataggtatcccgcactttggtatgaccggtggccgtagaatcaaaaagcttgtcgaggctctgtgcatgcgcacatacagagagcacacagcataataaaatggttgatatatacttcatggattgatgttgttatttactgtaaggtgtataaactgcattaaccgtaacggctactacttctgctacattttgcactaccagggaaggtatcttgataccgtgatcggctacacgaacattaaaggtggatacagcggtaagcgttgtgccctgtgcagtaatagtgcctttggcggtgtagctcttttctaccccgtgaatattcagtgtgcccgtaatcgttaccgggtaagtgccgtctttgctgaattccggtgattcattgatctttcccttgaattctgcaaacgggtatttatcactttcgaggtaattttcgttaaaatgctcctgcatcagcttctttttaaactggaaagaactgataggtactttaaaaaaaacttccttcgtttttgtgttgagtgcagaagcgcctttatctgttttagcttctatatcctccaatggagaagacgaaaaaaatgataaacgggtatttttgcaggagtaaacatcctgtgcagatgcagtaacaaccggtagcagggcaactgcaaaaagcaataagtatttcatgtttatcttttttaggttattgatccggaagtccttttgcgatccagcaggcgatagagtcttttaaaccctggctgagtgcgggaaaagacattgattgtggcatatctgcctgcggaccggttacacgggcctcaaaaacagtacggttggcattaataaacgttttcaatttagcagcggtggaaaaatctgccagagcgggcgagttgccgcccggatgacagccacggctggtacagttagcttgtatgatcgcaaaaacggtggctgttgtgatatgggctgcatcacagtctaccccgccacttaccggcgcaggggcctgttcatttttacaggcagccagcagcaggcatgccattaaaaaaagcttgttccttgtcattggtctttcaaatttgattgtagatagtaagtacgggatgatgagagaattggttgcttcacaggcagataaaattctgctatattacatgattaaccacttatttttgtaccaaataagatctgaccgtgaatattgaacaactatacagcatctatgagcagcatcgctccgtacaaacagatacccgtaaactgaaagccaatgatattttctttgcgctgaaaggaggcaatttcaatggtaacgaatttgccgcccgggcgctggaaatgggcgccgcctttgccgtggtagatgaagcagcttattttaccgtaccggataaaatgatgctggtagacgatgccctcaccgctttacagcaactggctttacatcaccgcaaacaattaaatatcccgttcctggccatcaccggtactaacggtaaaaccactacgaaagaactgatcaatgcagcattgtctgccggattaaaaacatatgccaccattggcaatctcaataaccacatcggcgtacctcttactattttaagtatactcccgggcgtagaaatagccgtagtggaaatgggcgctaaccaccaacgggaaatagccggttattgcgaaattgcgttgcctacccacggcatcattaccaatatcgggaaagcacacctggaaggctttggcagcgaagaaggcgttaaaaaagcaaaaggggaactgtatgattttttacgcgccaacaatggcaccgtattcgtatgcaacgattatggttacctgcttgaaatggcgcacggcatcccggaaataattacctatggcagcagcgaagccgattacgtaggcgaagccatcgccgacagcgccttcctggccgtggaagtacggggcagcagccaggtaggatttatacaaacacaactgacaggcgcttataatttccccaatgtaatggccgcagtagcggtagccagccactttaacgtgccggaatcagcgattgcaccggccattgcacattataccccttccaacaaccgctcacaggtaataaaaaaaggcagcaataccattatcatggatgcctataatgccaacccctccagcatgagagccgctattgaaaactttgccggcatccaggctgataaaaaagtgctgctgctcggcgccatgatggaacttggaacagatagcgttaaagaacaccaggacctggtaaacttactggaacgcacacactgggaggcagtggtactggttggcggcgactttaaaaaagtaacccacccgtacatcttcctcgaaaatgccaccgaagccggaaaatggctacagcagcaacagtaccaggatacacatatacttatcaaaggctcccggagcaccggtatggagaaagtgctggcctgataaccaggggcgattcagcaggcagacccaaagcgttcaaaatatttgttaacgatttcataattgtattatttttaatacttcaatctgtcatttgaactttaccaaaatctgaatcgcaatgcacaaaaaaatctggcattaccttattagtatgctttgctgcgtactattgatccctgctgccctgtttgcccaggaaacaaccgccgatatagccggtattattgtaagtaaagaagggcctgttcccggtgcaagcattactgctacccatgtgcccaccggcacaaaatataacaccgtttcccggaaagacggccgttataatttacccaacctccgcgttggtggcccttataccttatctgtttcttatattggctttaaagacgagaaacgcgacaacattttcctgtcgctgggacaggatttcaaatcagacatcaacctgcaatccagtaccagcaccctcacagaaatagtggtcacttctgtaacccagaacaaagtgattaacagggcccgcaccggcagccaggaagtaattacccgctcccagatggaccgcctgccaacgatcagcaggtctatgcaggacttcaccaaacttacaccttctgccaacggcctgaatatcggcggcagaagcaatcagctgaataacatcaccgtcgacggcgccaacttcaacaactcatttggtttgcagcccacactcggctcccaaacagcatcccagcctatcagcctggaagcgctcgaacagatccaggtaaacgtatctccctatgacgtaagacagggcggcttttccggcgccggtatcaacagcgttaccaaaagcggtaccaacacgttcaaaggagccgtgtatacctacattcaaacacccggattacaggggttgaaagtaggcaacgccactgttcccaaacccgactttaactataacctgcgcggcttcaatgtgggcggcgccatcatccccaacaaattgttcttcttcgtaagtgcagaacaggaaaggattaaagcacccgctaccagcctcgtagccaacaaacccggcggagtagccggtggcaacgtatcacaggcagtagcagatacactggatgcacttaaacaattcctgatcagcaaatacggatatgatcccggcgattaccagaattatacctaccgcacgcaaagtgataaagtaacactgaaggtcgactggaacgtgaatgagcataacacctttacatttaaatacagttacctgaaatcatttaaagatattcctgccagcaacagtggcgctcccggcggcggtgctgttggaagtggccgccagcccagtgctaccggtcttcctttcagcggaagcggctataccatcaacaataacttcaacatttttattgcggaactgaatacccgcatcggcaaccgcgcttccaataaactgcagatcggctactccgccatgcgcgatttcagaaatgctttgtcacaaagtaattttcccctcgtggatatcatgaacggccagggcgccagctataccgccttcggatatgagccgttcacctataataacaagctcaataccgatgtataccagctgtctgatatcttcaccatgtacaagggaaaacatgaaatcacgataggaacacaaaactattataaaacgttcctcaatggcttcgctccaaactacaatggcaactaccgctttaatacactcacggatttttatgccagcgccaacagcaacctggcaacggcttcccgttatgcagtgtcttatgcaactaccaaagacggatcctttccatacgcaaaaatcaacatgctggaactgggcgcgtttatccaggataagtggagtgttaccaacttctttaccttcacctacggattacgtatagacgtaccagttataggcagtacattctctaaaaatgattctctcactgctttgactttcagggatggagtaaaggtagatgtaggccaggcgccaaaaacaacaccgctcctgtcgccaagaattggatttaactgggacgttacacatgacggaaaaacgcagctccgtggtggagcaggtttatttgccggtccgccgccagctgtatggctgagcaaccaggcaggtaacaacggcgtacagtttggatcgtttgtagcgcaaacaagtgccactgcgcccaccattccttacccgttcagtgctgatccgaatacttacaaagctggtacagaaggacggttatcttcccaatataatatagccgttaccgataaaaactttaaatatccgcaggtattaaaagcaacactggctgttgaccgacagttaccatggggcgtaatcggtaccctggaattcaactattccaaagatatcaatgcggtatatttccagaacgtaaaccttcctactgcagggtttcaactggatagcacccccgatcaccgcacacgctataattcttccaaaatatacgcaggcaacagcctgagtaatcctaatatcagcgatgccatcctgatgcgcaataccaacaagggctattcgtattttgccaccatccagctgcagaaaaacctgcctaatctttacctgagtgcagcctatacttacagtaaatctcgcagtgtaaatgatggcggcagcatcgcacaaagcaactggcgcgatcgccccgttgccggcgatcctaatgccaatgctctgggctactccaattactacatgccccaccgtatcatcgcagccgctacctaccgctttacctgggcgaaacatttcgctacttctgttggtgttgtgtatgaagccgctccaagtataaacggactttacagcaacacttcctatacttacaacggcgacgtaaacaacgatgcttccggtggtaacaacgacctgatctacattccaaaaaccaggaacgatattaaactggtgccggttggttatggcgacaaaacctacaaccccgctaccaatgcagataaacgcaccgcagatatcatctggaatcagctcgataattttatcaaacaggataactacctgagcggtcaccgtggagaatatgcagaacgcaacgctgtagtattacctttcgccaaacgcatggacctgaatattacacaggacatcttcgtattcagcggcaaagagaaaaccaaacacacgctgcgtatcagtttcgatatcatcaactttggtaacttcctgaataagcgctggggtatttccaaaattccgaacctgccctctttcctgaaatacgaaggacaatacaaagacgcttccggcaccgctactgctaccgcagcctactccttcccttacctggatgcagcgaaccagattccgctcaccagttcattcagagacaataccggcactatttccagatggcagggacagcttggtatcaggtatatgtttaattaacgcggattttgtcttggctcaggattacgctgattttaaggattacctggatttttacttttggatttttttttgatttttagattttcttaaaaataattaagggagataaaagcgaatacatccgcttttatctcccttaatcctttataaaatccaaaagtaaaaatccaggtaatccttaaaatcagcgtaatcctgagccaagacaaaatccgccagggatacaatttatcggagtaatagtgcgttaatattttttgaaattaatccctctatttgtgagaagtggcttaaaaaaaagacctgcaagctaaaaaacccgcaggtgttcataacctatgccaactttagagtaatctttaaaacttaaactgttagaatctataaagcctaagtcttgtaatattttgagtattgatgttttttctattttgtatataagagataacgtaatggaaaatgtatttgttcaaaaattcgtgaaaaaattttggtcttaacattttgggcccttctttccggggtatctctctattacttacggaggataaattcctttggattgctaaaatggaaaaaaaattaaaaaaaatattattatttaaattttaaatatataagtaaatgcttacttgatatcctggcaaatttctatcaaaaccccgttgctgtgcttaggatgcaggaaacagatcagcttattatcagcccccttttttggtgtttcctgtaataaaacaaacccttcttcctgtaaccgtttcatttccgcataaatatccggtacctcaaaggcgatgtgatgcatgccttctcctttcttatccaggaactttgcaatagcgctgtccggccctgtggcttccagcaattctattttggtttcgccctgccggaaaaaggcggtctgcacctgctcgctgtccacctcctcctgcttgtaacatggcgtgttcagcagcttttcaaaaagcggaatggacacagataatttattaacggcaatgcctatatgttctaccctgagcatgtttataaatattaatagtggtacaaatccggtatccgtaccgctttccggaatatgcttaacccggtaaaaatagaacttatgttgtaaatttgttaggcccggattttaatataaacagaaagacattatgctgcagctgcccgtttacctcgataacaatgccaccactccctgcgatcccagggtagtagcggccatgttaccctatttcaccgaaatattcggcaacgcagcaagccgcagccacctcctgggatgggctgccgaggaagcagtagacaatgcccgtgaacaggtagccaaactgattggggcaacacctaaagaaattgtctttacttccggcgccacagaagccgttaaccttgccattaaaggagtgtatgaaacatacgccggcaaaggcaatcatattattactgccgtcaccgaacataaagccgtcattgacacctgcaaacacctcgaaaaacagggcgcacaggtaacctggcttccggtaaaccacgaaggacttatagacctcaacgaactggaagcggctattacgccccaaactatcctgatcagcctgatgtatgccaataatgaaaccggtgtcatcaaccccatacgcgccatcagcgatattgccagaaagcatggcgtattatttatgacagatgccacccaggcagcagggaaaattccggtagacgtaaacgacgatggtatagacctgcttaccctcagcgcccataaaatgtacggtcctaaaggaacaggcgccttatatgtgcgcagacgttccccccgcgtaaagctcaccgcacagatcgacggaggcggccacgaaagaggtatgcgctccggcaccctgaatgtgcccggcatcgtaggactgggaaaagcctgcgaactatgtatggaagaaatggcggccgacacacaacgcatccttcccatgagaaacaggctggaaaaggctttgctggaaatagagcaaacatatttaaatggcgcccccggtcagcgcctgccacatacctgcaacctgtcatttaaatacgtggaaagcgaaaccctcatgatgggcttcaataaaaaaatcgcgctttcctccggatcagcctgtacctccgcctccctggaacccagttacgtgctgaaagcaatgggcctcagcgacgacctcgcacacgcctccctccgctttggactgggaaggtttaccaccaatgaacaaatagattttaccatccaaaccattacagacgccgttgcccaactaagaaccatcagccccatatgggaaatgtataaagatggcgtggacctctaagtccacctttcccccgggtcaacgccgtagatactccgtacatactccccgtataaagccccttaaaaacctcccatacaatagccggaaaggtaatagcgtttaccctatatttgtatctttactaatatcctaatccttacaaactgttcatgctagccatctttaagaaagagattaaccagtttttcagcagtgttaccggctatgtagccatcatactgtttttactggcgaatggattaatgttgttcgttttcccggaaaccagtttactggacaccgggtatgccaacctggatccgctgttcaatctggcgccgcttatttacctcttgctcataccggccattaccatgcgctgctttgcagatgaatttaaaaccggtaccatggaattgctgagcaccaaaccactcaccggctggcagattgtaatgggtaaattctggggcagcctgctcattgtagccatctccctgcttcctaccatcgtttattattttgctataaaacaattgagtgtagataaccagctgcttgataccggcggtatcattggctcttatatcggacttttactgctgggggcaacattcaccgctaccggtatctggtcttcttctttaaccaacaatgccatgatcgcctttctcattgcactgtttacctgctttatactttataacggattcgatgccgtcagcaaaataccggcgttcagcggcggagccgactactacctgcaaatggctgggattaaattccattacgcctccatcagtcgtggtgtaatagatagccgcgatatcgtttattttatcagcatcataggcctgatgctctatctcactaaattatccctgcaaagaaaactctggcaaaacggttaatgaccgtccttactaaacaacatggctacacgaaagaaatacatacaacgtgcaatagcagttatactggtactcacgggcattaatatagcagcagcttattttcatggcagatgggacctgacagcagaaaaaagatacacgctcaccgccagcacccggcaaatgctccgcaaactggacagcccggtggaaattgaggtattcctcaaaggcgattaccccgccagcttccgtcagctggcacaatccacttccgaactgctggaagagttccgcgaatacggtaaacaaaacctccggtttacatttatcaatcccggacaggggctgacggactccgcacgcatgaaattcctcggtgaactcaccgcacagggcatcatgccgtttaatatgaaagtgcagcaggaagccaacgacggcttcgctgaaaagctgatcttccccggtgcactggtgcattacaaaggcaaaacggtaggggtgaatctcctgaaaaaccagggcgggcaggatcccatgcaaaccatgaacagctcggaagcgttgctggaataccagtttgcctatgccatccataaattgcaggaaaaggaaaaaccactcatcgggtacatgcttgggcatggagaatcacttggcgccgaagtatacgacgccctgagtacccttcaaaacagctacggcctggataccctcaccctgcaggccgcttcctacataccccgcgattttaatgtaatcctctttgccaaaccggcaggcgctttctctgatgcagataaatttaaaatagaccagtatgtaatgaacggcggcaaagtgctgtggttcctggatgaatccagcgccaccatggacagtttacacgaacacccggaattttttgccatggatcgcgggctgaacctggaagacctcctgttccgctacggcgtgcgcattaaccaggacctggtactggacctgcaaagcgatgtagtgccgctggtagtaggcaatgtgggcaaccggccgcagatacagccgatgccgttcccatacttccccatgctgatgcctaccaaagcgcatcctatcgtaaaaaatctggatatggtgctgagccgcttcgtaagttctatcgacactataaaaaacgacgccatccgcaaaaccatactgctcaccacttccaggaacagccgtaccacgcgcctgccggcacaggtaagctgggacatcgtaaaaacacagcccaatccgcgcgaataccgccagaaatacctgcccacagccgttttgctggaagggaaatttacttccctgttccgcaaccgcgaaaatcctgatgcggtaaaccagctgtttcacgcatccgggcaacctttcagggaatcatccgatactatcaacaaaatgattgtggtaagtgatggcgatgtaatttccaatgccgtatcccgcaaggaaggcccgctgcaaatgggcatcaacgaatttaacccgggctttgcctttgccaataaagagttttttctcaactgcctggagtatctcagcggcaacagcggtatcatggaagcccggaacaaggagctgacactgcgtttgctggatggagaaaaaatccggcaggaaaaaaccaaatggcaggtcatctgtttcctcgtacccgttgggctggttttgctatttgccatggtattccagtttatacggcaacgtaaatttgctgaataggctgaagtgctgtaagacactggctttcagggcatacaacagtggccgcttcctggaaatggcaaccttaaaccggaaacctagctgccgttttcctatctttgctgctcataaaatgcaaatcacgtgggaaaaacagaagtaacatatctggtattttttattgtgatcatcctggcagtagtatttgaccttggtttttttagtaagaaaaatacgaaaacaagcctgaagactgccctgtggcaaagcattttctgggtagttttatctatgctcttttttgggttcatgtggctggaagacggcgcagaacccgccatcagctttttgagcgcatacctgatggagaaatccctgtcgatagataatatctttgtatttatactcatctttagtttttttaaaataaaagaagagtactattccagggtattgctgataggtatactaatggccattattttcagggctttatttatctggctgggaattgagctcatagaaagatttgaatggatattatacatcttcggtgcttttctcatttataccggcattaaaatgtttgtcacaaaagaggatgacgaatttaaaccggaagaaaatgcgatttaccgttttatgaataaatacatgcgggtaactacagaagagccgaaaggcaaatttgtgatccgtaaacataataaggcatatctcactacgttatcactggttgtggtgatgctggcagtaacagatatcttatttgcggtagattctataccggctgtatttgccatatcacgggatccgatggtagtatatacctctaatatatttgcggttttgggactcaggtccctgttctttttactgaggggagcggtagataaatttgattatctgccccagggtattgccatcgtcctggtttttataggactgaaaatgctggcagagtattttttgcacaagcacaatattcatataccggtatacgtatcattgatagtgatagtgctatgcctgggaggttccatcctctattctctctatcatcagaaaaaagaattaccggaaggagaagtgaagtaaaaagcagcgcagacattaattttgcagcagctaagtgattattcaaacctgataaacgtgtataacgcagccagcatcaacaaaactttgaaaggggaattgttgcaagagaccggattttctgaaattgaccatcttttattggacagcaggaagctcagcttccccgaaacatctctgtttattccattggttagcccgcggcgcaacgcgcatcaatacattgaagaattgtaccgcaaaggggtgagcaattttgtggtgagtgaacaagtgccactggagaagtatcctaaagccaacttcattctcgtaaaagacaccctgcaggcgctgcacgcactggtggcctttcaccggcaccagttccatatacctgttattggcatcactggcagcaatggcaaaaccattgtaaaggaatggctgtaccagctgctggaaaaagattacaatattgttcgcagtcctaaaagctataactcccagataggagtaccgctttctgtatggcaaatgaaaccggaacaccagctggccatctttgaagccggcatttcacaacccggtgaaatggtgaacctcgaaaaaattatccgtcccactatcggcatcttcaccaatatcggggaagctcacagcgaaggattcttaaatatccgccagaaaataaatgaaaagctggtactgttcgctaaaagcgatatcctcatttactgcaaagactatctcgctctcaatgagtgtgtgctggcctttcacaaccaggtaggcaaaaaagaaaaccaggaaggcggaccggaattgttttcctggtcacggaaaaccgatgccgacctccgggtaaccagtgtggataaacacgataaccatacccgcatcgatgccctttacaaacaggaacccctgcatttccagattccttttgtagatgaaggttccatcgaaaatgccattcactgcctggcgctcatgctgtacctcggcaaggaacaagccgttatccagcaacggatggatcagctcagcaatatcgccatgcgcctggaactgaaacagggaatcaataactgctcggtgattaacgacagctacagcctggacctcggctctttaaccattgcgctcgacttcctccagcaacagcagcagcacgctacccgcacggttatcctcagcgatatcctccaaagtggcaaaagcgacgccaccctgtatgaagaagttgcagacctcctgcaaaagaaaggcatcaataaattaattgctatcggtaaaaatataggcagggagaaaaaaagcttccagcagatagaaggcctgaaaacacagttcctcaccaccaccgatgaatacatacaacaattcaacgcagatgatttccagaatgaaaccatcctggtaaaaggctcccgcatcttccagtttgaacgcatcggcaaactgctggaacaaaaggcgcatcaaaccatcctggaaattaatctcaccgctatttcccataatgtaaagctgtaccagtcgctattaaaaccaaacaccaaattaatggccatggtaaaagcgttctcctatggcagcggtagctttgaaatagccaatctcctccagttccacggagtcgactacctcgcggtagcctacgccgatgaaggagtggagctgagaagggccggcattaccatgcctatcatggtgatgaacccggaacctgccagtttcgacgccatcctccactggaacctggaaccggaaatttattccatgcagatcctcctgcagtttatggaggaaatcaccacagcaggcaaaacggagttccccgttcacatcaagctcgataccggtatgcaccgcctgggattcgtgaaaagcgaaattgccgaactggcgcaaatactcaccgccaccccgctaatgaaagtgcaatccattttcagccacctggctgccagtgaagatccttcaaaggatgctttcacacagcagcaaggccgcctgttttatgatatgagccatgaactgcagaaagcattgggctatactgtaatccgccatattgccaacagcgccgccatcagtcgccaccccgacctgcaactggatatggtgcggctgggtatcggcatgtacggcatcgacagcagcaacggcatccaggaccagcttcgcaatgtaagcaccctgaaaaccaccgtagcacaactaaaacgcctggaagccggcgataccgtgggttatggcgccaaatgggaagccaaaggcccggcagtgactgctaccgtgcgtattggctatgccgatggctacccacgcagactgggcatgggcgttggtaaaatgctggttcgtggcaaactggcgcctgtagccggtgtagtggcgatggatatgctcatgctcgatgtaacacatatccccgacgtagcggagggagacgaggttattgtttttggccaggatttgtccgtacaggacctctccacctgggctggaaccattccctatgaaatattaacaggaatttcacagcgcgtaaaaagggtatatttccaggaataatgatattgcaggcttcgactttgaaataaactattatttttgataaaattctaatatcagttgaaatatcgtcacgtagtatttatcgttatcctgatcctggttattgaccagacactgaaattctggatcaagacgcatatgtttatgcaacaggagtttgtgattttccccaattggttccggatccattttattgaaaatgaaggaatggcctatggtcttaaattcggaggcgacttcgggaagatccttctcaccatgttccgcctggtagctgtagtggtgggctttgtgtacatgaaaaagctcatcaaagaaaaatacagcaccggcctgctgatctgtggatccctgatcctggcaggagcagccggcaacctgatagacagtatgttctacggccttatttttaacgatagtgtagggtatgaagtagcgaagtttatgcctgccggcggcggttatggcagcttcctgcacggtcgcgtggtagatatgttatacttccctatctacgaaggctacctgcctaaatgggtaccgtttaaaggcggcgactacttcgtgtttttccgccccgtattcaatgtagccgatgcagctatttctaccggcgtaatcacgatcctgctgttccagaaacgcttcttcggaaaacacatgcagcctaaagccgttgaacactctgatgctgtagcaaaagatcccgtagcttaattatcaacttatttatatagaaagcgctcaccggtggtaagcgctttttttatgctattactttaaagcataggaagatgaccggcaaaatatccgtctttcatcttccaaaatcttctgaaatttccgcaaaatgcccgaaattggatttatactaagatacctgtaaaccaaaatcaggattatttcaccgggggcgtaaacctatttcaggacgtgacagtgtatagagagtgtatggggagtgtatcatgagtgtatcatgagtgtatcatgagtgtatagggagtgtatgggaactatatagggactataacacatacacgagtcctaagtatccgggaagtatcagagaagtatccaagaagtatcacagaagtatccccgcatattaaacatagttataaagcgacgcatccaataaaaaaatgtggccttccaagcctttcacgctgaggaggttacaaacgcaactgctgttcccaccgcagttccggacacacctttttccaaataatcaccccatttgctttgaaatgaaaaatacccggattatatttgtctactaattctatagactatatgataataaattttacaaatcattcattttcagtacgatgttgcggcatgacatcgtaaaaaggtccccttatcattttctcattccagaatcaataatgtttacagcacatgcaaaagtttttaatgctggcaaaatacctgttcttaatattggcattcagtccggcactggtacatgctcaacttaacggctcttatgtcattcagggcaaaattacagacgatcatggggcagcccttccaggcgcctccgtacaaatcaaaggcacttccttcggcgctcaaacagataccaccggccgctttgaagtaaccaccaattctaaattcccgctgaagctggtcatcaggctcataggctatcaaccccaggagtttgaagtaaaaagcagcagcagcaaactggccatccagttatatacacaatcactattggtaaatgaagtagtggtgtccgcttcccgtcagcaggaaaaactgctccgctcaccagttgccatcgaaaaactggacatcagggcgctgaaagaaaccccttcttccacgttctacgacgccctcggtaacctgaaaggcgtgcaaatgaccaccgccggccttaccttcaaagtattcaacacccgcggcttcaacgttcccaacaacttccgctttatgcagctggtagatggtgtggacaaccaggcagccaccctcggcgtgccactgggtaacgccatcggacctacggagcttgatatttccagcgtggaagttacacccggcgcatcttccgccctgtatggcatgaacgccatcaacggaatgtccaacctcatcactaaaaaccccttccaataccagggcgtaagtgtataccagaaagtagccgtgaaccacgttggcgacgacggtggcgcaaaattactcacggaaacggctgtacgctatgcacagcaatactcttcctggtttgcctggaaaattaacctgagctacatgcagggtaccgactggtacgctgataaccacagcgacttttccccgcaatccaaagccaaccccgactttccacaactcagcggcgccaacaacatcgccaacgatgcctggaataaatatggcgataactccaacctccaggttatcgataaagacggacgtgcctacaatgtacaccgcaccggctactgggaaaaagatatcgtgggcgactttaccgttaagaataaaaaagccgacgtgtcttttaacttccgcttaccccacaaactggaactgtccgcgtcttaccgctacggggaaatggacggcttctttcaacgtggtaaccgtatcggcctcagaggcgtaaccgtacaaaacggcaaactggaactcgtacaccccgacttcaccgtgaggtcgtacatctccattgaaaataccggcgattcctataacatgaatcccctggccgacaacctcgaaaaatcattcaaaccagataaaaaatggctggccgattatacctccggcctgaacaatgcgctcactgcaggctccgacctggtagccgcacatgccgccgcccgcgcctttgcagacgccggcagatggacgcccggcactcccgcttttgatgcacaggtggccaaaataaaaagtatcaacgactgggatatttaccctacttccaagaaccctgaaaataccagtggcggcgccgctctcctgcaaaagagccggttctaccacacagaaggtacctggaacctgcgtaaatacatccatttcgcggatgtactggtaggcgccgattaccgcacctatgaaatcatcccggacggtaacaacttcgtggatttctcccgccccgccgacaaacgcaaccaaccaggcggtaaacacatctggtacggtaaatacggcggctttgcacaaatcagcaaaacattcttcaacgacgcattaaagctcaccggctccctgcgctacgataaaaacgaacagttcgaaggtaaagtaaacccacgcatcgcagcagtttacagcatcaaagacaaacataacttccgcctttcctggcaaaacggattccgcttcccttcactgtttgaagcgtactccttcgtaaacaacggccaggtaagacgtgtaggcggactcgcattcattgaagaaggactgggttacttcaaaaactccttcctcaccagctccgtagatgcgtttggtgtagcggtaaataaaaccatcaacgcggaacacatctccaaagatgctgccgccgcaaaaaatgcaggcgtattgaaagtggccaacctggatcctatcgttccggaacagatcacctctttcgaagccggttataaagcggtattgctcgataacaaactctttgtagacatagatggatactacagctcctacaaacatttcatcggccagattgaagcagtagtgcctaaaacaggtaacgttaacaatcccgatcaaacagtgctgaaccagatgctggataagtctttacaggatcgctaccgcgtatggaccaacagtaaatccaccgtaaacaactacggtttcgctgtagcagttacttatgacctgtataaaagctacaccatcagcggtaacgccaactacaacaaactggcgcaggataaaaccaaagatgatgcgttgattcccggttttaacacaccagactggttcaccaacgtaagcctaggtaaccgcaatgtgtacaaaaatattggcttcaacgtagtatggcactggcagaatactttctactggcagaacctttttggtaatggcgacgtgccttcctacaacactgtagatgcgcagatcacctaccgtgtaccaaagatcaaaacatcctttaaactgggcgcttccaatatcctgaactccaagtacttccagtatgtgggaggtcccactattggcggattatactacctggcgttaacatacgacaatgtgttccagcggaaataataaataatagttgctgagatacagggatgcagcgatatcgctgcattcctgtttttaaaaaactacctaaaaataactggtatgactacacgtacaacagccgttgcaggcaccgttaccgaaaagccgcagtcctccttcaaatggtggcagataggggttgtatcgttgttgatagtcaccgcgctgattgccctttattattacgaagtaccggatgccgtacagggaaatgtacgccggttctttcactccctctttacaacagagctgctgttttatattgtggtgggattatgcgcgcaactggtagacggcgcattgggtatggcatacggcgctacctcttcttctttactactgggactgggcgtatcgccttcagtaagcagcgccagcgtgcatgtggcagaagtatttaccaccggcgcttcagggtttgcacattttaaactgggcaacgtaaataagaaactgtttttatgcctgttgatcccgggaatgatcggcgccatttccggcgcttacctgttatccgacaagattgacggggatgtgataaagcccttcatcagcgcatacctgctgatactcggtattatagttatccggaaaggcatccagaaaaataaaagaaaaaccaaaacaaaaagactcggaccattggcgtttgccgggggatttatggacgccatcggcggcggaggctggggccccattgttacttccaccttgctgagtaaaggccgtaccgtacattataccatcggttccgtaaatgcagcagagttctttatttccctttccagcgctgccaccttcctgatcttcaccggcatctccagctggcaggtaattgtaggccttgtaatcggtggtgtgatcgcttccccttttgctgccatcctggtgcggaaaataaaacggaaaccactgatgattatggtaggtgtcctcattattattctgagtctgcgtacaattgtcgctacgctacttcacctcgtttaacaatatgccttctttttcaaaactacgtatattgttcagcgttacctctgctatttgtgtgagcgcttcttttgtaaaaaagccctggtgggcagttaccagcacattagggaaggtagttaatctggatagtacatcgtcctggataatacttccggagaagttctgaaaaaacaagtgttcttcctgctcatacacatctattccaagtgcgccgatatggccatctttaagcgctgccactaccgaagccgtatctattaatccgccgcggctggtattgatcagtactacgcccatcttcatagatgcaatagcattcgcattgatcatatgccgtgtacgctccatcagcgggcaatgcagcgatatcacatccgactgtgcaaaaatagtatccagcgacacatactttacgcctgattccaacagttcttcattctcgtaaatatcatgggcatacaccttacaaccgaagcccagcatgatcttgcaaaacactgaaccgatattgcctgtccctaccacgccgattgttttaccaaagagatcaaaaccttccagtccgttcagcgtaaagttgccatcacgtacacggttatacgatttatatattttccggttcagccccaggagtaaggccaccgcatgctccgccaccgcatggggcgagtaggccggcacccgcactacctttataccggctgctgctgcagccttgagatctacattattaaacccggcgcagcgcaatgcaataagacgtacgcctttttgctgaagcacgctgatcacagcagcattcaccttatcattcacaaatacgcagatcacgggttcatcttttatcagggcggcattatcttcatttaactgcacttccaggaaacggaaacggtgctcctcctggtggttaccctggttgaagtaatgaatatcgtatggctgcgcgctgaaaaagactatatccatgatcgtggtgcttgtttgcattgaaggtaataaaaaaagaagctgtctcataaataaatgaggcagctttttcattttaggctttaaggatggttttatccacaatttgcagttgaaaaaaagggaagttgtaagtgtttacgcaccagaagttattgtg

SEQ ID NO: 22 - DNA, 1801 bp, Chitinophaga pinensis
  source 1..1801: mol_type = genomic DNA
gaagctgtctcataaataaatgaggcagctttttcattttaggctttaaggatggttttatccacaatttgcagttgaaaaaaagggaagttgtaagtgtttacgcaccagaagttattgtgtaaatttaaggatggcaagaggtaaaagcttatcagtagcatttaaaagcacccatcagaatcaggggatgttatttcctccagatctgaatgaattaatatcatcagatcaccctgttcgtatagttaacgatatcattgatcagattgatatcagtatgttgcttctgcaatacaaacccggaggagccagcagctatcatcctcgtatgctgttgaaagtacttgtttacgcctatgtaaataatatatatagtagccgtcgtatagaagaggcactacatcaaaatatttactttatgtgggttagcgggatgaataagcccgatcataatacggtaaaccgtttccgaagtggtcgtcttcaaaagacgttgcagccaatttttacccaggtggtgcacttattatgcgccgaagggcttttgagcataaaagacttgtatacagacggtactaaaatagaagcgaatgccaatcgttacagctttgtctggggcaacagtataaagcataataaggagaagatcagtaaacaattaaatgagctgtggaagtatgcccagtctgtagcagcagcagaactggacgacgatactgacccttccggctttaagaagatagacagtactaaagtgcaggcaacgatagctgctattaatgaagcattgaaggataagccggttgataagaagatgcgtcaaaagttaggttatgctggaaaacactggccggccgcccttgataaatatgaacagcaggagaagatattgggaccaggaagaaatagctacagcaaaacggatactgatgccacttttatgcgtatgaaggaggatcacatgaaaaacggtcagcttaaacccgcctataatttacagattagtactaacaatcagtatatactctcttacagccttcatcccaaccctacagacaccgctactcttaaagatcatctttcacagcatatcaagcagcttaaaacaaagccagctaatatcactgctgatgcgggatatggcagcgagcagaattatcagtggctggaggataagcgaattactgcttatgttaaacataatcagtttgacaggcatcaaaataaaaacatacgttataaaaaacgatttacagtagatcagcttgagtatgatgataagaaagataggtttaaatgccccggcggccagatcctaagtagaaagcgaacctataaaagtcgttcccgggccggctatgagcaaactatcactcaatatcaatcccgcaattgtgatggctgcccacttaggggagattgtcaccaacaaagcggcaatcggattatagatgttaatcataattacagaagacttaaaaaccaggcagagaaacgattaagaaccaggcgtggcatccagaaaaggaaacaaagatgcttcgatacagaacccgtatttgctaacattaagcataatcatcattttaagagatttatgcttagggggatagaaaaagtaacagtggaaaccggattactcgctcttgcacacaatattagaaagaaaatagcttgctaaagcaagctgacattaactatttattctcttaaaaaacacctgatcatcataatgattattaggccatcttttggctaaaacaaagaagctgtctcaattaattatgagacagcttct

SEQ ID NO: 23 - DNA, 1720 bp, Chitinophaga pinensis
  source 1..1720: mol_type = genomic DNA
tcaaaagttctttgaaagattggaaacaacagcacgaatctaagtagtgatgcttaggttcaaacaggtaatgtacagctaaacataattaataaagatccgattgatttcgagagaaattagtcagtatcaaaacttctttacaatggagagtttgatcctggctcaggatgaacgctagcggcaggcctaatacatgcaagtcgaggggcagcacaggtagcaatactgggtggcgaccggcaaacgggtgcggaacacgtacgcaaccttcctttaagcggggaatagcccagagaaatttggattaataccccataagaatgtgatctggcatcaggtagcatttaaagatttatcacttaaagatgggcgtgcgtctgattaggtagttggtgaggtaacggctcaccaagccgacgatcagtaactggcgtgagagcgcgaccagtcacacgggcactgagacacgggcccgactcctacgggaggcagcagtaaggaatattggtcaatggacgcaagtctgaaccagccatgccgcgtggaggatgaaggccctctgggttgtaaacttcttttatctgggacgaaacacttcttttctagggagcttgacggtaccaggtgaataagcaccggctaactccgtgccagcagccgcggtaatacggagggtgcaagcgttatccggattcactgggtttaaagggtgcgtaggcggacatgtaagtccgtggtgaaatctcagggcttaaccctgaaactgccatggatactatatgtcttgaatgttgtggaggttagcggaatatgtcatgtagcggtgaaatgcatagatatgacatagaacaccaattgcgaaggcagctggctacacaaatattgacgctgaggcacgaaagcgtggggatcaaacaggattagataccctggtagtccacgccctaaacgatgattactcgacatacgcgatacacagtgtgtgtctgagcgaaagcattaagtaatccacctgggaagtacgaccgcaaggttgaaactcaaaggaattgacgggggtccgcacaagcggtggagcatgtggtttaattcgatgatacgcgaggaaccttacctgggctagaatgcagtctgactgatgctgaaaggtgtctttgtagcaatacacagattgtaaggtgctgcatggctgtcgtcagctcgtgccgtgaggtgttgggttaagtcccgcaacgagcgcaacccctatcactagttgccagcacgtcaaggtgggaactctagtgaaactgccgtcgtaagacgcgaggaaggaggggatgatgtcaagtcatcatggcctttatgcccagggctacacacgtgctacaatggtgggaacaaagggctgctacctggtaacaggctgctaatctcaaaaatcccatctcagttcggattgaggtctgcaactcgacctcatgaagctggaatcgctagtaatcgtatatcagcaatgatacggtgaatacgttcccggaccttgtacacaccgcccgtcaagccatgaaagccggggggacctgaagtcggcaaccgcaaggaaccgcctagggtaaaatcggtaattggggctaagtcgtaacaaggtagccgtatcggaaggtgcggctggaatacctcctttttagagctcattatcctgagagctgttgtttccttcttttaaatttatttg

SEQ ID NO: 24 - DNA, 1448 bp, Chitinophaga pinensis
  source 1..1448: mol_type = genomic DNA
tgtactgctccccaaagtttagacttttttgattaggcggcttgagttcgatattgtattggactcaagccatttagttttaatttgattctatcgttattataatattctatatattctcgaatgtccttttccagtgtaattattgaatcatattttttcagataaaacaactctgacttcaatattgaaaagaacccctccatggctgcattatcgaggcaatttccttttctggacatactttgcctgattctattgcccttaaatagtcgttgccaggccttcatttggtattgccatccttgatcagagtgaataattaattttgatttttccggcagcttagacaaaacattttttagcatttctacagtctgattaccattgcaacgtctatccaatgtatagctgattatttcactgttatataagtccattattggtgataaatacaatttttctcctgctacactaaactccgttacatctgttacccatttctgattgggtttgccagcataaaaattacgttgtagcagattcggagctattttgcccaactcccctttataggatttgtacttctttacttttaccagtgatttaatccccaattctctcatgattcgcagtacagttttatggttaacaatgatgccttgttttcttacagccagcataattcgcctgtagccatatctgccttgatgatgatgatagatctggaggatttgagtttttagatttatttttttgtcttgtcgctttttttgataatagtaaaacgtacttcttgccatccctgctgcttttaaaagcagatcctggttgtaatcgtgccttaattccctgatggcttttgctctttttgctttttgttttgagcttgttcttccttcattaaggcatccaacttttttaggtacgcgttttccgtgcgtaaccattcgttctcggctttcagtgccgctaattcttgttgttcaggtgttaagttctgttcaacttgcgatgttttatgtttcatgggttgttttttttgaccacttcccatcattagcaatccctggcggccttcacgcttgtatatacatagccaattataaatggtagcagcacttgagataccgaaaatagagctggcctccatcaaagataagtccttatttaaaatcttctcaaccactttgatcctgaatttactcgtgtaaacctttaaacctacctgcaactttaagcccacttcacccgcgattcgataatgctcaagccattgctggatacaaaaacggctacatccaaaacctctcgccactgaactaacggattgataatcattctcaactgccatcacaatggctaatttttgctcaaaactgtattttctgcgtttatccataaaaatgccccctaaaagtgtctaacttttagggggcagtacatat

SEQ ID NO: 25 - DNA, 1337 bp, Chitinophaga pinensis
  source 1..1337: mol_type = genomic DNA
ggcctcagtaaaatggtacaaccaactgtttaacaaaaacacagggccctgcaaaatcgaaagatgacgtatagagcctgatacctgcccggtgctggaaggttaaggaaggatgttcggagcaatccaaagcttctgactgaagccccagtaaacggcggccgtaactataacggtcctaaggtagcgaaattccttgtcgggtaagttccgacctgcacgaatggtctaatgagttgtacactgtctctaccacgagctcggtgaaattgtagtatcggtgaagatgccggttaatcgcaacgggacggaaagaccccgtgaaccttcactacaacttaacattgattttgaatgccagatgtgtaggatagttgggagactatgaagcagcttcgccaggagttgtggagtcatcgttgaaataccaaccttctgttatttagagtctaatccctgcaaggggagacattgtttggtgggtagtttgactggggtggtcgcctcctaaaaggtaacggaggctcgcaaaggtaccctcagtacggttggtaatcgtacgcagagcgcattagtataagggtgcttgactgtgaggcaaacaagccgagcaggtgcgaaagcaggctaaagtgatccggtggttctgtatggaagggccatcgctcaaaggataaaaggtactccggggataacaggctgatctcacccaagagctcatatcgacggtgaggtttggcacctcgatgtcggttcgtcacatcctggggctggagaaggtcccaagggttcggctgttcgccgattaaagtggcacgtgaactgggttcagaacgtcgcaagacagttcggtccctatctgttgtgatcgttagtaaattgagaggacatgaccttagtacgagaggaccgggtcgtacataccgctggtgtatctgttgtgccgccaggtgcagtgcagagtagctatgtatggataggataaacgctgaaagcatctaagcgtgaaacctgcttcaagatgagtttacttttaagggccgtcggagactacgacgttgataggttacaggtgtaagggtggtaacatcgcagccgagtaatactaattgcccgtaagctttaattttttaaatattacgttaaagagtcttagaatacaactttcccgatatgttatcttattagtttgctgtaacagcaaaaaagatcttatggtggttatgccgagggtgttcacctcttcccattccgaacagagaagttaagcccctcatggccgatggtactgcaatatcatgcgggagagtaggtagctgccatacttattaagagaa

SEQ ID NO: 26 - DNA, 1203 bp, Chitinophaga pinensis
  source 1..1203: mol_type = genomic DNA
cggtatctaaggagtatttagccttaccagatggtgctggcagtttcatacaggattcctccggtcccgcactactcaggatactacacgtccatcagaatttctgtctacagggctatcacctgctacggctcatctttccagatgattcaacttgatctgactttctaaaagtagtcctacaaccccggacagaattgcttcgatccggtttgggctcttccccgttcgctcgccactacttagggaatcattatttattttcttttcctgcaggtacttagatgtttcagttccctgcgttggcccccttgcgggtaatacaccttcagtgtactgggttgtcccattcggaaatctacggatgtaacgatcgtttgcatctccccgtagcttatcgcagcttaccacgtccttcgtcgcctcttagatcctaggcatccaccatgcgctcttattcgctttaaaaaatttagtatttagatattactatcttgaatacaacttgcatttcccaatatgtcaaagaacttttaaccactgactgctcttacgagctttcatttgtgcgattattgatgatgtgtgagatctgatccctgtgactctttagtcaaacatcttcttgttattattataagaacttatactctgtattgtattgtttgtgttggggttgcaaaggtagtgatcttatatttaatcaccaaaactttcttgaagtattttgcatctttaattatcttagtatcaatgacttgtctattgggaaagtgctattaatatctccgataatcaaacccctattttacaaagaacactagcttttttgaagcggatggcaaagatatgccctttatcattcgcaaacaaaactatttgagttttctctcaaactatttttcaatcttatttcaaattgttttcaaccttatggctgagtgtaattttataatccgtgtgaggatcattgctttagagtaaaaatgtactgacgctttatgaaattatctgctctttagcagatgcgtctactcttaaagaaagaaaaagccttagtgcaaacgcaccaaggcttctcttaataagtatggcagctacctactctcccgcatgatattgcagtaccatcggccatgaggggcttaacttctctgttcggaatgggaagaggtgaacaccctcggcataaccaccataaga

SEQ ID NO: 27 - DNA, 1175 bp, Chitinophaga pinensis
  source 1..1175: mol_type = genomic DNA
tatacctacaccctttaacgcactattccgtaagtgcgcgatcctttcactactccgttactccatcgaatttatagcaggtactggaatattcaccagtttgccatcagctacacctttcggctttgcctaaggacccgactaaccctgatccgattagcgttgatcaggaacccttagtcttacggcgataagatttttcatcttatttatcgttacttatgcctacattttcttttctaaacgctccagcatgtttcgcaacacaccttcgatgcagtttagaatgctcccctaccgtctaataccttaagtattaggcctaaagcttcggttatatgtttgatgcccgattattttccgtgcccaaaccctcgaccagtgagctgttacgcactctttaaatgaatggctgcttccaagccaacatcctggctgttttaggatttgaaccgcgtttgatcaacttaacatatcattagggaccttagctgttagtctgggttatttccctctcggccatggaccttagcgcccacagcctcactcctggagattatattatagcattcggagtttattagggtttggtaggcggtgaagccccctagcccaattagtagctctacctctataatacgtctatatccaaggctgttcctaaaaacatttcggggagaacgagctatctctcagtttgattggcctttcacccctatccacaggtcatcccatagcttttcaacgctaatgagttcgggcctccagttagttttacctaaccttcaccctgcccatggatagatcacaaagtttcgcgtctacccccactgactgattcgctctgttagaacttgctttcgctacggctccggtactgaagaccttaaccttgccagtgaggagtaactcgtaggctcattatgcaaaaggcacgccgtcactcattgctgagctccgaccgcttgtaagcgcacggtttcaggaactatttcactctcctgttcggagtacttttcacctttcccttacggtactggttcactatcggtatctaaggagtatttagccttaccagatggtgctggcagtttcatacaggattcctccggtcccgcactactcaggatactacacgtccatcagaatttctgtctacagggctatcacctgct

SEQ ID NO: 28 - DNA, 860 bp, Chitinophaga pinensis
  source 1..860: mol_type = genomic DNA
ccgcagttacggtcagcgtggccggcgctacctggaacgactggctcaccgctgctgccgccgtgtaattggcgtcacctgcctgtgtagcgcttatggttacattgcccacgccggtgatggtaacagtgttgccgctcaccgtagccggaccggcggttacggtgtaagctactgttaatcctgcatcgctgttggcgctgagcgcaaaggccgcatcgccatatgttttgttagagatagccgggaaggtgatggtttgagatgcctttgtaatagtaagcgatccacctgcaaagttaaagtcgtagttagcggctgttaatgtgcccgcagtgaccgtaatcggataaacaccaggcgcactgttgatatcggcagtgtgggtaatggtggcatcaccacttactacactgctgttttcgttgtttacaaaaccggtaatgatataatccggtgttggattagtttgtttgtatgccctgtttttatcattagccgttaccgttagggtggctttggcaacgttgaaagtttgtgtgacctgcgtggccggtgagtagttgccgttgcctgcctggtcagccgcaatggtaacgctgcctgcgccggcaatggtaacggtgttgccgctgatggtagccggaccgcttaccacgctgtagctcaccgctaacgtactactgctggtggcgctgagcgtaaaggcggcgtcgccatatgttttgttagcgatagcggggaaggtgatggtttgcgaggtgagcccaacagttaaggtaccattcaccggtgtgaagatgtaattggccgctgtcaacggagttacatccacagtaatagggtatgcacccggcaca

SEQ ID NO: 29 - DNA, 703 bp, Chitinophaga pinensis
  source 1..703: mol_type = genomic DNA
cagagaagttaagcccctcatggccgatggtactgcaatatcatgcgggagagtaggtagctgccatacttattaagagaagccttggtgcgtttgcactaaggctttttctttctttaagagtagaggacatacagttcttttataatagcaggtcactgctaacaggatgacaccgccaggctaggcaacaacctaccactacacttttacggttcatcatatattcctgaaaatcaggaataatacattaagcaacacgcttaatatcaaacttgaaatacaggaaataaacagcaattaagttgaaataatttttgctgcgaatgataaagatgttatctttgccatccgcttcaaaaagccagtgttctttgtaaaataatgggttgattatcaaacgactatactgcactttcccaatagataagtcattaggattgagataattaaatataaaaaatgttgtaaaatgtttggtgattaaataaaagatccctacctttgcaaccccaacacaaacgatacgaaaaagttcttctaaaaataacaaagatgtatggcaaaagagccacagagatcggatctcagacatcagcaatgatcatataagatggtcaaaagttctttgaaagattggaaacaacagcacgaatctaagtagtgatgcttaggttcaaacaggtaatgtacagctaaacat

SEQ ID NO: 30 - DNA, 700 bp, Chitinophaga pinensis
  source 1..700: mol_type = genomic DNA
tcttatggtggttatgccgagggtgttcacctcttcccattccgaacagagaagttaagcccctcatggccgatggtactgcaatatcatgcgggagagtaggtagctgccatacttattaagagaaaagtcctggtgacataccaggactttttcttttctttctctctatgtttaagaaaaggggatcattccagatctgtcggaaaatacactcaacaataaggttgaatacaaattgaaattgacttaaatagtttttgctgcgaataataaagattctatctttgctgtccgcctcaaaaatatgtagttctttgcgaaataagggtttgattatcgaagatattaatagcactttcccaatagataagtcattgataataagataattaaagatgtaaaatactttaaaaaagttttggtgattaaataaaagattattacctttgcaaccccaacgcaaacgacgcgaaatacaagcaaaagttcttctgaaaaataattaaagatgtttgactaaagagtcacagagatcggatctcagacatcagcaatggtcatataagatgatcaaaagttctttgaaagattggaaacaacagcacgaatctaagtagtgatgcttaggttcaaacaggtaatgtacagctaaacataattaataaagatccgattgatttcgagagaaattagtcag

SEQ ID NO: 31 - DNA, 513 bp, Chitinophaga pinensis
  source 1..513: mol_type = genomic DNA
ccgcagttacggtcagcgtggccggcgctacctggaacgactggctcaccgctgctgccgccgtgtaattggcgtcacctgcctgtgtagcgcttatggttacattgcccacgccggtgatggtaacggtattgccgctcaccgtagccggaccggcagttacgacgtaagttaccgtcaaccctgcatcgctgttggcgctgagcgcaagggccgcatcgccatatgttttgttagagatggccgggaagctgatagtttgagatgcctttgtaatagtaagcgatccattcgcaaagttaaagtcgtagttagcggctgttaatgtacccgcagtgaccgtaatcggataaacaccaggcgcactgttgatatcggcagtgtgggtaatggtggcatcaccacttactacactgctgttttcgccgtttacaaaaccggtaacagtataatccggtgttggattagtttgtttgtataccctgtttttatcattagccgttaccgttagtg

SEQ ID NO: 32 - DNA, 496 bp, Chitinophaga pinensis
  source 1..496: mol_type = genomic DNA
aaagccgaaaggtgtagctgatggcaaactggtgaatattccagtacctgctataaattcgatggagtaacggagtagtgaaaggatcgcgcacttacggaatagtgcgttaaagggtgtaggtataggtttggtaggaaaatccgccagacttgctgaagcctgatagtacagcaaagcttcggccgcgctgatagtatccctaatcagacttccaagaaaaacttctaaggttcgtttatagcagcccgtaccgtaaaccgacacaggtagtcgagatgagtattctcaggcgctcgagtgatccgtggtaaaggaactaggcaaattgacgctgtaacttcgggataaggcgtgccgcagtgatgcggcctcagtaaaatggtacaaccaactgtttaacaaaaacacagggccctgcaaaatcgaaagatgacgtatagagcctgatacctgcccggtgctggaaggttaaggaaggatgttcggagcaatc

SEQ ID NO: 33 - DNA, 372 bp, Chitinophaga pinensis
  source 1..372: mol_type = genomic DNA
tccaccatgcgctcttattcgctttaaaaaatttagtatttagatattactatcttgaatacaacttgcatttcccaatatgtcaaagaacttttaaccactgactgctcttacgagctttcatttgcgtgattattgacgatgtgtgagatccgatctctgtgactctttagtcaaacatcttcattaaagattgaaagaacttatgtgcatggcgcctggcgtgtagccatttgcgttagcagcaaataaatttaaaagaaggaaacaacagctctcaggataatgagctctaaaaaggaggtattccagccgcaccttccgatacggctaccttgttacgacttagccccaattaccgattttacccta

SEQ ID NO: 34 - DNA, 360 bp, Chitinophaga pinensis
  source 1..360: mol_type = genomic DNA
tcttattcgctttaaaaaatttagtatttagatattactatcttgaatacaacttgcatttcccaatatgtcaaagaacttttaaccactgactgctcttacgagctttcatttgcgtgattattgatgatgtgtgagatctgatctcggtaactctttagttacacatcttcattaaagattgaaagaacttatgtgcatggcatccggcgtatagccatttgcgttagcaacaaataaatttaaaagaaggaaacaacagctctcaggataatgagctctaaaaaggaggtattccagccgcaccttccgatacggctaccttgttacgacttagccccaattaccgattttacccta

SEQ ID NO: 35 - DNA, 352 bp, Chitinophaga pinensis
  source 1..352: mol_type = genomic DNA
cagttcaaatctgctcgggtctacaatgattacgggggattagctcagttggctagagcacctgccttgcacgcagggggtcatcggttcgaatccgatatcctccacttaatcacctttgttcttttaatattaaataagatgtttgactaaagagtcaccgagatcagatctcacacatcatcaataatcacacaaatgaaagctcgtaagagcagtcagtgattaaaagttctttgacatattgggaaatgcaagttgtattcaagatagtaatatctaaatactaaattttttaaagcgaataagagcgcatggtggatgcctaggatctaagaggcgacgaaggacg

SEQ ID NO: 36 - DNA, 325 bp, Chitinophaga pinensis
  source 1..325: mol_type = genomic DNA
gtaattggggctaagtcgtaacaaggtagccgtatcggaaggtgcggctggaatacctcctttttagagctcattatcctgagagctgttgtttccttcttttaaatttatttgctgctaacgcaaacggctacacgccaggcgccatgcacataagttctttcaattttttattaagccaagttggttatggactgaatcggttagtgagatagtatcagccaaccttgtctgataaacagatccgtagctcagcctggttagagcactacactgataatgtaggggtcagcagttcaaatctgctcgggtctacaatgattac

SEQ ID NO: 37 - DNA, 324 bp, Chitinophaga pinensis
  source 1..324: mol_type = genomic DNA
cagttcaaatctgctcgggtctacaatgattacgggggattagctcagttggctagagcacctgccttgcacgcagggggtcatcggttcgaatccgatatcctccacttaatcacctttgttctttaatattaaataagatgtatggcaaaagagccacggagatcggatctcggacatcagcaatgatcatgtaaatggtcaaaagttctttgaaagattggaaacaacagcacgaatctaagtagtgatgcttaggttcaaacaggtaatgtacagctaaacataattaataaagatccgattgatttcgagagaaattag

SEQ ID NO: 38 - DNA, 290 bp, Chitinophaga pinensis
  source 1..290: mol_type = genomic DNA
tagtatttagatattactatcttgaatacaacttgcatttcccaatatgtcaaagaacttttaaccactgactgctcttacgagctttcatttgcgtgattattgacgatgtgtgagatccgatctcggtaactctttagttacacatcttcattaaagattgaaagaacttatgtgcatggcacctggcgtgtagccatttgcgttagcagcaaataaatttaaaagaaggaaacaacagctctcaggataatgagctctaaaaaggaggtattccagccgcaccttcc

SEQ ID NO: 39 - DNA, 288 bp, Chitinophaga pinensis
  source 1..288: mol_type = genomic DNA
gtaatcattgtagacccgagcagatttgaactgctgacccctacattatcagtgtagtgctctaaccaggctgagctacggatctgtttatcagacaaggttggctgatactatctcactaaccgatccagtccataaccaacttgacttaataaaatttaaaagaacttatgtgcatggcacctggcgtgtagccatttgcgttagcagcaaataaatttaaaagaaggaaacaacagctctcaggataatgagctctaaaaaggaggtattccagccgcaccttcc

SEQ ID NO: 40 - DNA, 280 bp, Chitinophaga pinensis
  source 1..280: mol_type = genomic DNA
aaagccgaaaggtgtagctgatggcaaactggtgaatattccagtacctgctataaattcgatggagtaacggagtagtgaaaggatcgcgcacttacggaatagtgcgttaaagggtgtaggtatatttttggtaggaaaatccgccagagatgctgaagcctgatagtacagcaaagcttcggccgcgctgatagtgtccctaatcagacttccaagaaaaacttctaaggttcgtttatagcagcccgtaccgtaaaccgacacaggtagtcgagat

SEQ ID NO: 41 - DNA, 266 bp, Chitinophaga pinensis
  source 1..266: mol_type = genomic DNA
tacaaccccggacagaattgcttcgatccggtttgggctcttccccgttcgctcgccactacttagggaatcattatttattttcttttcctgcaggtacttagatgtttcagttccctgcgttggctctccttgcggagtaatacaccttcagtgtactgggttgtcccattcggaaatctacggatgtaacgatcgtttgcatctccccgtagcttatcgcagcttaccacgtccttcgtcgcctcttagatcctaggcatcca

SEQ ID NO: 42 - DNA, 264 bp, Chitinophaga pinensis
  source 1..264: mol_type = genomic DNA
gttcgtttatagcagcccgtaccgtaaaccgacacaggtagtcgagatgagtattctcaggcgctcgagtgatccgtggtaaaggaactaggcaaattgacgctgtaacttcgggataaggcgtgccacagtgatgtggcctcagtaaaatggtacaaccaactgtttaacaaaaacacagggccctgcaaaatcgaaagatgacgtatagagcctgatacctgcccggtgctggaaggttaaggaaggatgttcggagcaatc

SEQ ID NO: 43 - DNA, 261 bp, Chitinophaga pinensis
  source 1..261: mol_type = genomic DNA
cttaataagtatggcagctacctactctcccgcatgatattgcagtaccatcggccatgaggggcttaacttctctgttcggaatgggaagaggtgaacaccctcggcataaccaccataagatcttctttgctttacagcaaactaataagataacatatcgggaaagttgtattctaagactctttaacgtaatatttaaaaaattaaagcttacgggcaattagtattactcggctgcgatgttaccacccttacacc

SEQ ID NO: 44 - DNA, 257 bp, Chitinophaga pinensis
  source 1..257: mol_type = genomic DNA
gctgaaaggtgtctttgtagcaatacacagattgtaaggtgctgcatggctgtcgtcagctcgtgccgtgaggtgttgggttaagtcccgcaacgagcgcaacccctatcactagttgccagcacgttatggtgggaactctagtgaaactgccgtcgtaagacgcgaggaaggaggggatgatgtcaagtcatcatggcctttatgcccagggctacacacgtgctacaatggtgggaacaaagggctgctacctg

SEQ ID NO: 45 - DNA, 255 bp, Chitinophaga pinensis
  source 1..255: mol_type = genomic DNA
tcaagcacccttatactaatgcgctctgcgtacgattaccaaccgtactgagggtacctttgcgagcctccgttaccttttaggaggcgaccaccccagtcaaactacccaccaaacaatgtctccccttgcagggattagactctaaataacagaaggttggtatttcaacgatgactccacaactcctggcgaagctgcttcatagtctcccaactatcctacacatctggcattcaaaatcaatgttaagtt

SEQ ID NO: 46 - DNA, 255 bp, Chitinophaga pinensis
  source 1..255: mol_type = genomic DNA
tgcctagttcctttaccacggatcactcgagcgcctgagaatactcatctcgactacctgtgtcggtttacggtacgggctgctataaacgaaccttagaagtttttcttggaagtctgattagggatactatcagcgcggccgaagctttgctgtactatcaggcttcagcaagtctggcggattttcctaccaaacctatacctacaccctttaacgcactattccgtaagtgcgcgatcctttcactactcc

SEQ ID NO: 47 - DNA, 255 bp, Chitinophaga pinensis
  source 1..255: mol_type = genomic DNA
cggtatctaaggagtatttagccttaccagatggtgctggcagtttcatacaggattcctccggtcccgcactactcaggatactacacgtccatcagaatttctgtctacagggctatcacctgctgcggctcatctttccagatgattcaacttgatctgactttctaaaagtagtcctacaaccccggacagaattgcttcgatccggtttgggctcttccccgttcgctcgccactacttagggaatcatt

SEQ ID NO: 48 - DNA, 255 bp, Chitinophaga pinensis
  source 1..255: mol_type = genomic DNA
tctcagtgcccgtgtgactggtcgcgctctcacgccagttactgatcgtcggcttggtgagccgttacctcaccaactacctaatcagacgcacgcccatctttaagtgataaatctttaaatgctatctgatgccagatcacattcttatggggtattaatccaaatttctctgggctattccccgcttaaaggaaggttgcgtacgtgttccgcacccgtttgccggtcgccacccagtattgctacctgtgc

SEQ ID NO: 49 - DNA, 255 bp, Chitinophaga pinensis
  source 1..255: mol_type = genomic DNA
ttcaaatggaaaaacagatgaaagaaaaagctatatatttatgagagttctttgagtgcgccaggttgcggatggtaggtgagtccgtggggtctgggagtggggaggtatatcgttatgggtttaatgggaaggagaatgataatgatgtgaagggagaagggaatcagatagactacggcatgcgtgtttacgacccacggatagggaagttcctttctacagatcctctatcgaaacaatatccacactata

SEQ ID NO: 50 - DNA, 250 bp, Chitinophaga pinensis
  source 1..250: mol_type = genomic DNA
tctaaggagtatttagccttaccagatggtgctggcagtttcatacaggattcctccggtcccgcactactcaggatactacacgtccatcagaatttctgtctacagggctatcacctgctacggctcatctttccagatgattcaacttgatctgactttctaaaagtagtcctacaaccccggacagaattgcttcgatccggtttgggctcttccccgttcgctcgccactacttagggaatcatt

SEQ ID NO: 51 - DNA, 221 bp, Chitinophaga pinensis
  source 1..221: mol_type = genomic DNA
atcggttagtgagatagtatcagccaaccttgtctgataaacagatccgtagctcagcctggttagagcactacactgataatgtaggggtcagcagttcaaatctgctcgggtctacaatgattacgggggattagctcagttggctagagcacctgccttgcacgcagggggtcatcggttcgaatccgatatcctccacttaatcacctttgttcttt

SEQ ID NO: 52 - DNA, 191 bp, Chitinophaga pinensis
  source 1..191: mol_type = genomic DNA
tgttttcattgtttacaaatccggcgatggtgtaagtgagcggcggattattagcgccgtatgttttttgcttatcatccgcagttacggtcagcgtggccggcgctacctggaacgactggctcaccgctgctgccgccgtgtaattggcgtcacctgcctgtgtagcgcttatggttacattgcccacg

SEQ ID NO: 53 - DNA, 168 bp, Chitinophaga pinensis
  source 1..168: mol_type = genomic DNA
acggacaaatcgttacctggctatgggagaaaactgcaggtcctgcgggaggaaatctttccgccgctaacgcagccaaaacaaatgtcaccaacctgcaggcgggaacttatacgttccggctgacggtcactgataacgatggcgctaccagcaatgccactgtga

SEQ ID NO: 54 - DNA, 148 bp, Chitinophaga pinensis
  source 1..148: mol_type = genomic DNA
tcgtaacaaggtagccgtatcggaaggtgcggctggaatacctcctttttagagctcattatcctgagagctgttgtttccttcttttaaatttatttgctgctaacgcaaatggctacacgccaggtgccatgcacataagttcttt

SEQ ID NO: 55 - DNA, 141 bp, Chitinophaga pinensis
  source 1..141: mol_type = genomic DNA
tttttgcttatcatccgcagttacggtcagcgtggccggcgctacctggaacgactggctcaccgctgctgccgccgtgtaattggcgtcacctgcctgtgtagcgcttatggttacattgcccacgccggtgatggtaac

SEQ ID NO: 56 - DNA, 140 bp, Chitinophaga pinensis
  source 1..140: mol_type = genomic DNA
taaaaaagctgctgctaagaaagctgctcctaaaaagaaagctgctgctaagaaagccgctcctaaaaaagctgctgctaagaaagctgctcctaaaaagaaagctgctgctaagaaagccgctcctaaaaaagctgctg

SEQ ID NO: 57 - DNA, 132 bp, Chitinophaga pinensis
  source 1..132: mol_type = genomic DNA
taaataatgattccctaagtagtggcgagcgaacggggaagagcccaaaccggatcgaagcaattctgtccggggttgtaggactacttttagaaagtcagatcaagttgaatcatctggaaagatgagccg

SEQ ID NO: 58 - DNA, 130 bp, Chitinophaga pinensis
  source 1..130: mol_type = genomic DNA
aaaagaagctgtctcataattaattgagacagcttctttgttttagccaaaagatggcctaataatcattatgatgatcaggtgttttttaagagaataaatagttaatgtcagcttgctttagcaagct

SEQ ID NO: 59 - DNA, 128 bp, Chitinophaga pinensis
  source 1..128: mol_type = genomic DNA
gggggggggggggggggggggggggggggggggggggggggggggggggggggggggggggggggggggggggggggggggggggggggggggggggggggggggggggggggggggggggggggggg

SEQ ID NO: 60 - DNA, 128 bp, Chitinophaga pinensis
  source 1..128: mol_type = genomic DNA
tttttttttttttttttttttttttttttttttttttttttttttttttttttttttttttttttttttttttttttttttttttttttttttttttttttttttttttttttttttttttttttttt

SEQ ID NO: 61 - DNA, 128 bp, Chitinophaga pinensis
  source 1..128: mol_type = genomic DNA
agaagctgtctcataaataaatgaggcagctttttcattttaggctttaaggatggttttatccacaatttgcagttgaaaaaaagggaagttgtaagtgtttacgcaccagaagttattgtgtaaat

SEQ ID NO: 62 - DNA, 1525 bp, Chitinophaga pinensis
  misc_feature 1..1525: note = ADNr 16S
  source 1..1525: mol_type = unassigned DNA
aatggagagtttgatcctggctcaggatgaacgctagcggcaggcctaatacatgcaagtcgaggggcagcacaggtagcaatactgggtggcgaccggcaaacgggtgcggaacacgtacgcaaccttcctttaagcggggaatagcccagagaaatttggattaataccccataagaatgtgatctggcatcaggtagcatttaaagatttatcacttaaagatgggcgtgcgtctgattaggtagttggtgaggtaacggctcaccaagccgacgatcagtaactggcgtgagagcgcgaccagtcacacgggcactgagacacgggcccgactcctacgggaggcagcagtaaggaatattggtcaatggacgcaagtctgaaccagccatgccgcgtggaggatgaaggccctctgggttgtaaacttcttttatctgggacgaaacacttcttttctagggagcttgacggtaccaggtgaataagcaccggctaactccgtgccagcagccgcggtaatacggagggtgcaagcgttatccggattcactgggtttaaagggtgcgtaggcggacatgtaagtccgtggtgaaatctcagggcttaaccctgaaactgccatggatactatatgtcttgaatgttgtggaggttagcggaatatgtcatgtagcggtgaaatgcatagatatgacatagaacaccaattgcgaaggcagctggctacacaaatattgacgctgaggcacgaaagcgtggggatcaaacaggattagataccctggtagtccacgccctaaacgatgattactcgacatacgcgatacacagtgtgtgtctgagcgaaagcattaagtaatccacctgggaagtacgaccgcaaggttgaaactcaaaggaattgacgggggtccgcacaagcggtggagcatgtggtttaattcgatgatacgcgaggaaccttacctgggctagaatgcagtctgactgatgctgaaaggtgtctttgtagcaatacacagattgtaaggtgctgcatggctgtcgtcagctcgtgccgtgaggtgttgggttaagtcccgcaacgagcgcaacccctatcactagttgccagcacgtcaaggtgggaactctagtgaaactgccgtcgtaagacgcgaggaaggaggggatgatgtcaagtcatcatggcctttatgcccagggctacacacgtgctacaatggtgggaacaaagggctgctacctggtaacaggctgctaatctcaaaaatcccatctcagttcggattgaggtctgcaactcgacctcatgaagctggaatcgctagtaatcgtatatcagcaatgatacggtgaatacgttcccggaccttgtacacaccgcccgtcaagccatgaaagccggggggacctgaagtcggcaaccgcaaggaaccgcctagggtaaaatcggtaattggggctaagtcgtaacaaggtagccgtatcggaaggtgcggctggaatacctccttt

SEQ ID NO: 63 - DNA, 930 bp, Chitinophaga pinensis
  misc_feature 1..930: note = Tryptophan 2-3 oxygenase
  source 1..930: mol_type = unassigned DNA
atggttacaacagaaatcgccgaaaaaattcaacggctggaagaaaagtatgccgccatgggccagaacctgtcatcctacctggatggccttctgtacgcggactacctcacttattgggattatattcagcttgatgtattgcttaatctgcaacatccacgcacaccaattcctgatgaaagaatattcatcatctatcaccagatcacggaattgtatttgaaattatcgttgcaggcaatcgaacaaatcagccttgcacctgtactgtcagctgagatatttaaaacccagcttaaaaggatcaacaactatttccacagtcttatcagctcatttgaaataatggtagatgggatggacaaggaacagttcctgcaattccgcatggcgctgttacctgccagtggcttccagagcggacaattccgcatgatcgagatctgctctacccggctaaacaacctggtatacgaaccccagcgcccggaagtggaaggccaggaactgaaagacgtgctggacaaaatctactggagaagcggcgccaccgaactggctacaggtaaaaaaacgcttaccctccgccagtttgaactgaaatatatggataccttcctgaaactggccactgagtacaaagacagtaacctgctggccagctataaaaagctctcccccgcggaacaaacggaattaatccccctgttaaaggagtacgatctcaatgtaaacgtacgctggccgctgatgcactacaaatccgcggtaagatacctgcataaaaggccggaagacattgccgccaccggaggcaccaactggcagcaattcctgcctccaaaaaataaacgcatcgttttcttccccgaactatggacggaagaagaactcaacaactggggtaaaattgctatgggcgagtaa

SEQ ID NO: 64 - DNA, 1209 bp, Chitinophaga pinensis
  misc_feature 1..1209: note = Tryptophan synthase subunit beta
  source 1..1209: mol_type = unassigned DNA
atggatattgcgattaatactggcaactccaggtatcaggtggataagaatggctattatggcagatttggcggggcgtacattcccgagatgctgtatcccaacgtagaggaattacagtccaaatatctcggcatcctcagcgatcccggttttcagcaggactttgaagccctgttgcgggattatgtaggaaggccttcccctttatattttgccaaacgtttgtctgaaaaatataaagcgaaaatttatcttaaaagagaagatctgaatcataccggtgcacataaagtaaacaataccatcgggcagatcctgctggcgcaacgcctgggcaaacgccgtatcatcgctgaaaccggcgctggtcagcatggcgtggccacggctaccgtatgcgcgctcatgggcatggagtgcgtggtgtatatgggcagcattgatatagaaagacaggcgcccaacgtagcgcggatgaaaatgctgggagccaccgtagtgccggccaccagcggcagtaaaaccttgaaagatgctaccaatgaagcgatccgcgactggatcaacaacccggtagatacacattatattttgggcaccgctgcaggtccgcatccatatcctgatatggtggcccgcttccagtcggtgatcagcgaagaaataaaaaaacagctgttggagaaaaccggcagcgagaatcctgattatgtactggcttgtatcggtggcggcagcaatgcagccggcgcttacttccattacctcgacagggaaaaggtaaaactggtagccgtggaagctggcggaaagggtgtacacagcgggttttccgcagctactacgcagctgggcaccattggtattatccatgccagcaaaacattgctgatgcaaaccaacgacggacagatcgtggaaccacattccatttccgcaggactcgattatcccggcatcggacctatgcacgcccatttgtatgaatcgggccgcgcacagttcctgtcggctaccgatgaagaagccctggcggcggcttatgaactgagcctgctggaaggaattattcctgctatggaatcggctcacgccctggctaaactgaaagacctgcccctgaatactgatgatgtagtggtggtatgcctttccggccgcggggataaagatctggatacctatatccgtcacatgaataaataa

SEQ ID NO: 65 - DNA, 774 bp, Chitinophaga pinensis
  misc_feature 1..774: note = Tryptophan synthase subunit alpha
  source 1..774: mol_type = unassigned DNA
atgcaaaatcgtattgatcaactgtttgctgttaagcggcacaacgttttaaatatatattgtacggctggctttccgcagttaaatgacaccctgcctgtaatgaccgcattacagcaatatggagcggaccttattgagctgggcatgccattctccgatccgctggccgacgggcctgttatccaggacagcagcactaaagcgttgcagaacggcatgagcctgcacaaactgtttgaacaacttaccggtttcagggaccgtatacaggtgcctgttatcctgatgggatatttcaacccggtattaacttacggtgtggaagccttttgcgcaaaatgtgcagaagtaggtgtggatggtatcattgtgccggacctgccaatggccgaatatgaaaatgagtacagaccagtgtttgaaaaatacaacctgcacctgattttcctggtaacgccggaaaccagtgaagcacggatccgtaaaatagacagtctgagcaaaggctttatttatgccgtatcttcttcttccaccacaggaaaagacaaggatatgaaagaccagcaggcttattttgagcggctgaagcagttgcagctcacaaaccctgttttaattggttttggtataaaagataaagctacttttgatacggcatctgcttatgccaatggcgctattatcggcactgcctttatcagggccattgagcacagtaagaatattgacgaaacggtgaaaacgtttatttcgggaataattcagtaa

SEQ ID NO: 66 - DNA, 804 bp, Chitinophaga pinensis
  misc_feature 1..804: note = Indole-3-glycrol phosphate synthase TrpC
  source 1..804: mol_type = unassigned DNA
atgaagaatattttagcagaaattgttgctcataaacacatcgaagtagctgcccgcaaattgcagcgcagcgcgcaggacctggagcagtcgccggccttcccgagggaaacattatcgctccgccatttcctgcagcagccggaaaaaacgggcattattgcggaattcaaacggcgctctccttcgaaaggagtgatcaacggcgatgtaactgttcaacaggtaactaccgcatacacccgttacggcgcttccgggctgtcggtgctcaccgatgaaaaatatttcggtggttcttccgacgatctgcaacaggcgcgtagcttcaaccagatcccgattctgcggaaagattttgtgatagatgaataccagatactggaggcaaaggctatcggggcagatgtaatactcctcattgcagaatgcctggatgccgcacaggtagcacacctggctgcttttgcacataacctcggactggaagtattactggaagtacacagtgaagcgcaactggaaaaagtaacggcacatacccacctggtgggcgtgaataaccgcgacctgatcacgttccaggtagactttaaccgttcctgtgaactggcgccgaagattccggcggataaagtgaaagtggcggaaagtggtatcaatgaccccgctgctattgtaacactgaaagccgccggattccagggattcctgataggcgagcatttcatgaagcaggaagatcccgcacgtgcctttgaaaattttgtacaaacactcagcgatctgcagcataaatcataa

SEQ ID NO: 67 - DNA, 1725 bp, Chitinophaga pinensis
  misc_feature 1..1725: note = Phosphoglucomutase
  source 1..1725: mol_type = unassigned DNA
atggatataaatattcaaaacaaagtagcgcaatggctcaacggtaattacgacgctgaaaccgttgccacactgaagaaaatgcaggaaggaaaccctgatgacctcaacgacgccttttaccgtaacctcgaatttggtaccggtggcctcaggggcatcatgggcgttggcaccaaccgcatgaataaatatactcttggaatggccacccagggcttcgccaattacctcaaaaaaaccttcaccggcgaaattaaggtagccattgcacacgacagccgcaacaatgcccgctttttcgcagaaaccgttgccaacgtttttgccgccaacgacattaaggtatttctttttgaaagcctgcgtcccacaccggaactgtcttttaccatccgtcacctgcgttgccagggtggtgtggtactcaccgcctcccacaacccaaaggaatacaacggctacaaagcctactggaacgacggcgcacagctggtgccgccccacgataacaacgtgatccgtgaagtagagaacatcgcctccccggatgaggtaaaatggaccggtggtgaagccaatatcaccctcatcggccaggaaatagacgaagcttaccgcaaggaactgctcagcctgtccatcaatcccgatatcaacaaacaacagcacgaccttaaaatagtatacacacctattcacggtaccggcatcacccaggtgccccagctgctggaacaatacggctttaccaatgtaaccattgtacaggaacaggccacgccggatgggaatttccccaccgtagtgtaccctaacccggaagaatccgaagccatgagcctcggcctcaaaaaagccaaagaactcgatgccgatattctcctgggtaccgaccccgatgccgatcgtgtaggcattgccgtgaaagacctcaaaggagaatggatcctgcttaacggtaaccaaaccggcgtactgctgtttaactacatcgtggaaagccgcaaaagcaaaggactcgccaaagcaaacgactatattgccaaaacagtagtaacatccgacctgatcgatgtattcgctgccaaaaacaatattacctgctataacgtactcaccggcttcaaatggatcgctgacctgatccgccgtaaagagccggaggaaaacttcatctgcggaggtgaagagtcctatggctatatgattggtcagaatgtgcgcgataaagatgccatcgcctctgtagccatgatctgtgaaatggcggcctatgcccgcagtcacggcaaatccctgtttgaacagctgatcgacatctatgtacgctatggctattacatggaaagtttgatttctattaccaaaaagggaatgagaggcgcggaagaaatcgccgaaatgatgcgcggataccgcgaaaatccaccggttaccatcaacggatcaccggttgcaacgctgtacgactaccagctgcaacagatcagggatattaaaaccggcgacaccaaagcgctggatctcccgaaatccaatgtactgcagtttgtattggaagatggcagcaaaatatctgcccgtccctccggtaccgaaccaaaaatcaagttctacttcagcgtaaacgcaccactggccagtgcaggagactacgacaaagtgaccgctgaactgaatcagaaaataaatggcattattcaggatctgaaactgaaataa

SEQ ID NO: 68 - DNA, 1383 bp, Chitinophaga pinensis
  misc_feature 1..1383: note = Phosphomannomutase/Phosphoglucomutase
  source 1..1383: mol_type = unassigned DNA
gtggcactgatcaaatcgatatccggcatacgcggaaccataggcggtaagcccggcgagggactttctccattagatgtggtgaaatttaccgctgcctacggcacctggctgagccggcaaacagacaaccgtaaggtggtaataggccgtgatggccgtatttccggcgaaatggtaaaaaacctggtagtatccaccctcaacgggctggggattgatgtgatagacctcggtttatccaccacccctaccgtggaactggcggttacaatggaaaatgccgcaggcggtattattctcactgccagccataaccccagagaatggaacgccctgaagctgctgaacagcaaaggcgagttcatttccggtgaagatggtgcacagttgctggaaatagccgaacaggaagactttaatttcgcagatgtaaataagctcggctcctacaccgtcgacgattcctatctgcagaaacatatcgacctgatcgtgaactacccattggtggatgtgcctgccattaaagcacgtaacttcaaaattgtggtggatgcggtaaattctaccggcgctatctttgttccacctttgctgaaagcattgggtgtggaggaagtagaagtgctgtttgcggaagtaaacggcaaattcagccacaatccggaaccgctggcagaaaacctgaccgctctttccaatgaggtaaataaatccaatgccgacctcggtattgccgttgatccggatgtagaccgcttgtgctttgtttgtgaagatggaagcatgttcggcgaagaatacacgctggtagcagtagccgattacgtgttaagcaaaagaaaaggtaacaccgtttccaatatgtcttccacacaggcgttgaaagacgtcaccctcaagcatggtggagaatacaccccgtctgcagtaggtgaagtgaatgtggtaaagaaaatgaaagacaccaacgcggtgatcggcggagaaggcaatggcggcatcattgtgcctgacctgcactatggccgtgatgccctgatcggtatcgggcttttcctgagccacctggcgcacagcaaaaaaagcatcaaagccttacgcaacagctatcccgactatttcatctccaaaaataaaatagagctggataaaggcgtggatgtaaaaactatcttcgaaaaaatcaaggttaagtataaaaaccagcctttaaataccgaagacggattgaaaatagagttcgacaaagactgggtacacttgcgcacttccaatacagaacccatcatccgtatatacgccgaaagccagaatgaaactacggcagacaatatcgccaaaaggatcatgcaggacattaaagaatttatgcactag

SEQ ID NO: 69 - DNA, 969 bp, Chitinophaga pinensis
  misc_feature 1..969: note = dTDP-glucose 4,6-dehydratase
  source 1..969: mol_type = unassigned DNA
atgaccggagcttccggctatataggcagtgtgctggtgccgctgcttttatccgaagggcataccctgcggttgcttacccggaaaccgttgccggaaaccaccccggagggcataactttcgtacagggggagctgttagccgaagcggctatccgccagctcgtagcaggtgcggatgctgtgatacacctggcggcagtcatttcggtagatgaccggcccgataaaaacctttttcacatcaatacggagggcacgcggctgctggccgccgccgcacaacaagccggcgttaaaagattcattcacctcagttccgttactgcttacaaccaggcgccctatgatgaaccgatgaatgaaagccgcagcgtggtaaataccacgcggcacggttacgactattccaaagcggtatcgcaggccattgtgctggaatataacggcagcggcatggaagtggtggtgctggcgccaacagccgtaatggggccgttcgaccggcaaccatcgctgataggtaaagccatcattaatatgtataaaggaaaaataccggctctttttcccggtggtgttgatttcgttgatgtaagggatgtggccggggccattgcaagcgcattaacgcggggaaccgccggcgctgtataccttctgagcggcgaatgggtatcacttgtgagcctgaacagggaagttggccggataaaagcacggccggtaacgctgcgggtagtacctttatggcttgtattcagcatgctgccatttgtgagaatgctggcagtgatcagcggcggaccgccgttttatacgcggcagtcggtgtacaacctgatttacagcagcaaaaaaattgatcattcaaaagccgccgccgaactcaatttcaggccgcggccctttacggaaacccttcgggataccattgattggttcaaacaaacaggcgctatcaaatga

SEQ ID NO: 70 - DNA, 1023 bp, Chitinophaga pinensis
  misc_feature 1..1023: note = Alginate biosynthesis protein AlgA
  source 1..1023: mol_type = unassigned DNA
atgatgcagcatattctcctttgcggtggctccggcacccggttatggcctttgtccaaccaacaaacgcccaagcagttactcaccctgttcgacggctatagtcttttacaactcgctttccggcgaaaccgttttgcctgtaataaagtaatggcgattgttaatgaacaacagtccgaaattgttcaggagcaactgatgcaggcaggcgcagctgccccggtatgcctggccgaaccggtaggccgtaatactgctgctgccattgccctggctgcctttacagcggagccggaaaccatactactcatcactccggccgatcacctgattggtacgcccgaccgctatgccatggccattgaaacggccggcctgctggccgcgggaaatcatattgttaccatcggcctggtgcctacacgcccggacaccggatttggctacatcagctactccggtcatgatgtgctccgctttgtggaaaaacccgaccgcgccgtagcagaagccatgctggccgccggcggcttcctctggaacagcggcattttctgctgtaaagcacgcatcatgctgcaggagctgcaaaaacatgcacctgctatctatgaagccgctgccatcgccgcggaagaatggaaacaaaccggtgtgttgtcgaaagaaagtatggaagccattccttcagatagcatcgactatgccgtgctggaaaaaagtgacatcgtaaaagtagtgcccagtaaaatggactggagcgatgtaggcagctacgaagcattggcagacgcattgtcgcaacactaccagtacaggaatcaccaggcggtttttattcaaagcgatccgcataaaagtatggtaatcggaaaagataaattggtcgcattggtgggcgtggaaaatatggtggtggttaatacagaaagcgcactgctgatcatgcagaaaggaagtggacaggatattaaacaactgcatcaatgggtaagggaaaaccgcccggagctgctctaa

SEQ ID NO: 71 - protein, 309 aa, Chitinophaga pinensis
  REGION 1..309: note = misc_feature - Tryptophan 2-3 oxygenase
MVTTEIAEKIQRLEEKYAAMGQNLSSYLDGLLYADYLTYWDYIQLDVLLNLQHPRTPIPDERIFIIYHQITELYLKLSLQAIEQISLAPVLSAEIFKTQLKRINNYFHSLISSFEIMVDGMDKEQFLQFRMALLPASGFQSGQFRMIEICSTRLNNLVYEPQRPEVEGQELKDVLDKIYWRSGATELATGKKTLTLRQFELKYMDTFLKLATEYKDSNLLASYKKLSPAEQTELIPLLKEYDLNVNVRWPLMHYKSAVRYLHKRPEDIAATGGTNWQQFLPPKNKRIVFFPELWTEEELNNWGKIAMGE

SEQ ID NO: 72 - protein, 402 aa, Chitinophaga pinensis
  REGION 1..402: note = misc_feature - Tryptophan synthase subunit beta
MDIAINTGNSRYQVDKNGYYGRFGGAYIPEMLYPNVEELQSKYLGILSDPGFQQDFEALLRDYVGRPSPLYFAKRLSEKYKAKIYLKREDLNHTGAHKVNNTIGQILLAQRLGKRRIIAETGAGQHGVATATVCALMGMECVVYMGSIDIERQAPNVARMKMLGATVVPATSGSKTLKDATNEAIRDWINNPVDTHYILGTAAGPHPYPDMVARFQSVISEEIKKQLLEKTGSENPDYVLACIGGGSNAAGAYFHYLDREKVKLVAVEAGGKGVHSGFSAATTQLGTIGIIHASKTLLMQTNDGQIVEPHSISAGLDYPGIGPMHAHLYESGRAQFLSATDEEALAAAYELSLLEGIIPAMESAHALAKLKDLPLNTDDVVVVCLSGRGDKDLDTYIRHMNK

SEQ ID NO: 73 - protein, 257 aa, Chitinophaga pinensis
  REGION 1..257: note = misc_feature - Tryptophan synthase subunit alpha
MQNRIDQLFAVKRHNVLNIYCTAGFPQLNDTLPVMTALQQYGADLIELGMPFSDPLADGPVIQDSSTKALQNGMSLHKLFEQLTGFRDRIQVPVILMGYFNPVLTYGVEAFCAKCAEVGVDGIIVPDLPMAEYENEYRPVFEKYNLHLIFLVTPETSEARIRKIDSLSKGFIYAVSSSSTTGKDKDMKDQQAYFERLKQLQLTNPVLIGFGIKDKATFDTASAYANGAIIGTAFIRAIEHSKNIDETVKTFISGIIQ

SEQ ID NO: 74 - protein, 267 aa, Chitinophaga pinensis
  REGION 1..267: note = misc_feature - Indole-3-glycrol phosphate synthase TrpC
MKNILAEIVAHKHIEVAARKLQRSAQDLEQSPAFPRETLSLRHFLQQPEKTGIIAEFKRRSPSKGVINGDVTVQQVTTAYTRYGASGLSVLTDEKYFGGSSDDLQQARSFNQIPILRKDFVIDEYQILEAKAIGADVILLIAECLDAAQVAHLAAFAHNLGLEVLLEVHSEAQLEKVTAHTHLVGVNNRDLITFQVDFNRSCELAPKIPADKVKVAESGINDPAAIVTLKAAGFQGFLIGEHFMKQEDPARAFENFVQTLSDLQHKS

SEQ ID NO: 75 - protein, 574 aa, Chitinophaga pinensis
  REGION 1..574: note = misc_feature - Phosphoglucomutase
MDINIQNKVAQWLNGNYDAETVATLKKMQEGNPDDLNDAFYRNLEFGTGGLRGIMGVGTNRMNKYTLGMATQGFANYLKKTFTGEIKVAIAHDSRNNARFFAETVANVFAANDIKVFLFESLRPTPELSFTIRHLRCQGGVVLTASHNPKEYNGYKAYWNDGAQLVPPHDNNVIREVENIASPDEVKWTGGEANITLIGQEIDEAYRKELLSLSINPDINKQQHDLKIVYTPIHGTGITQVPQLLEQYGFTNVTIVQEQATPDGNFPTVVYPNPEESEAMSLGLKKAKELDADILLGTDPDADRVGIAVKDLKGEWILLNGNQTGVLLFNYIVESRKSKGLAKANDYIAKTVVTSDLIDVFAAKNNITCYNVLTGFKWIADLIRRKEPEENFICGGEESYGYMIGQNVRDKDAIASVAMICEMAAYARSHGKSLFEQLIDIYVRYGYYMESLISITKKGMRGAEEIAEMMRGYRENPPVTINGSPVATLYDYQLQQIRDIKTGDTKALDLPKSNVLQFVLEDGSKISARPSGTEPKIKFYFSVNAPLASAGDYDKVTAELNQKINGIIQDLKLK

SEQ ID NO: 76 - protein, 460 aa, Chitinophaga pinensis
  REGION 1..460: note = misc_feature - Phosphomannomutase/Phosphoglucomutase
VALIKSISGIRGTIGGKPGEGLSPLDVVKFTAAYGTWLSRQTDNRKVVIGRDGRISGEMVKNLVVSTLNGLGIDVIDLGLSTTPTVELAVTMENAAGGIILTASHNPREWNALKLLNSKGEFISGEDGAQLLEIAEQEDFNFADVNKLGSYTVDDSYLQKHIDLIVNYPLVDVPAIKARNFKIVVDAVNSTGAIFVPPLLKALGVEEVEVLFAEVNGKFSHNPEPLAENLTALSNEVNKSNADLGIAVDPDVDRLCFVCEDGSMFGEEYTLVAVADYVLSKRKGNTVSNMSSTQALKDVTLKHGGEYTPSAVGEVNVVKKMKDTNAVIGGEGNGGIIVPDLHYGRDALIGIGLFLSHLAHSKKSIKALRNSYPDYFISKNKIELDKGVDVKTIFEKIKVKYKNQPLNTEDGLKIEFDKDWVHLRTSNTEPIIRIYAESQNETTADNIAKRIMQDIKEFMH

SEQ ID NO: 77 - protein, 322 aa, Chitinophaga pinensis
  REGION 1..322: note = misc_feature - dTDP-glucose 4,6-dehydratase
MTGASGYIGSVLVPLLLSEGHTLRLLTRKPLPETTPEGITFVQGELLAEAAIRQLVAGADAVIHLAAVISVDDRPDKNLFHINTEGTRLLAAAAQQAGVKRFIHLSSVTAYNQAPYDEPMNESRSVVNTTRHGYDYSKAVSQAIVLEYNGSGMEVVVLAPTAVMGPFDRQPSLIGKAIINMYKGKIPALFPGGVDFVDVRDVAGAIASALTRGTAGAVYLLSGEWVSLVSLNREVGRIKARPVTLRVVPLWLVFSMLPFVRMLAVISGGPPFYTRQSVYNLIYSSKKIDHSKAAAELNFRPRPFTETLRDTIDWFKQTGAIK

SEQ ID NO: 78 - protein, 340 aa, Chitinophaga pinensis
  REGION 1..340: note = misc_feature - Alginate biosynthesis protein AlgA
MMQHILLCGGSGTRLWPLSNQQTPKQLLTLFDGYSLLQLAFRRNRFACNKVMAIVNEQQSEIVQEQLMQAGAAAPVCLAEPVGRNTAAAIALAAFTAEPETILLITPADHLIGTPDRYAMAIETAGLLAAGNHIVTIGLVPTRPDTGFGYISYSGHDVLRFVEKPDRAVAEAMLAAGGFLWNSGIFCCKARIMLQELQKHAPAIYEAAAIAAEEWKQTGVLSKESMEAIPSDSIDYAVLEKSDIVKVVPSKMDWSDVGSYEALADALSQHYQYRNHQAVFIQSDPHKSMVIGKDKLVALVGVENMVVVNTESALLIMQKGSGQDIKQLHQWVRENRPELL
